European Patent Application EP 4 470 558 A1, published December 4, 2024. Title: CORONAVIRUS DERIVED POLYNUCLEOTIDES AND THEIR USE AS VACCINES. Applicant: CONSEJO SUPERIOR DE INVESTIGACIONES CIENTIFICAS. Application EP. The sequence listing filed with the application follows.

SEQUENCE LISTING (50 sequences)

SEQ ID NO: 1 - DNA, 29903 bp, Coronaviridae
  misc_feature 1..29903: note = SARS-CoV-2 Genbank: MN908947.3
  source 1..29903: mol_type = genomic DNA
attaaaggtttataccttcccaggtaacaaaccaaccaactttcgatctcttgtagatctgttctctaaacgaactttaaaatctgtgtggctgtcactcggctgcatgcttagtgcactcacgcagtataattaataactaattactgtcgttgacaggacacgagtaactcgtctatcttctgcaggctgcttacggtttcgtccgtgttgcagccgatcatcagcacatctaggtttcgtccgggtgtgaccgaaaggtaagatggagagccttgtccctggtttcaacgagaaaacacacgtccaactcagtttgcctgttttacaggttcgcgacgtgctcgtacgtggctttggagactccgtggaggaggtcttatcagaggcacgtcaacatcttaaagatggcacttgtggcttagtagaagttgaaaaaggcgttttgcctcaacttgaacagccctatgtgttcatcaaacgttcggatgctcgaactgcacctcatggtcatgttatggttgagctggtagcagaactcgaaggcattcagtacggtcgtagtggtgagacacttggtgtccttgtccctcatgtgggcgaaataccagtggcttaccgcaaggttcttcttcgtaagaacggtaataaaggagctggtggccatagttacggcgccgatctaaagtcatttgacttaggcgacgagcttggcactgatccttatgaagattttcaagaaaactggaacactaaacatagcagtggtgttacccgtgaactcatgcgtgagcttaacggaggggcatacactcgctatgtcgataacaacttctgtggccctgatggctaccctcttgagtgcattaaagaccttctagcacgtgctggtaaagcttcatgcactttgtccgaacaactggactttattgacactaagaggggtgtatactgctgccgtgaacatgagcatgaaattgcttggtacacggaacgttctgaaaagagctatgaattgcagacaccttttgaaattaaattggcaaagaaatttgacaccttcaatggggaatgtccaaattttgtatttcccttaaattccataatcaagactattcaaccaagggttgaaaagaaaaagcttgatggctttatgggtagaattcgatctgtctatccagttgcgtcaccaaatgaatgcaaccaaatgtgcctttcaactctcatgaagtgtgatcattgtggtgaaacttcatggcagacgggcgattttgttaaagccacttgcgaattttgtggcactgagaatttgactaaagaaggtgccactacttgtggttacttaccccaaaatgctgttgttaaaatttattgtccagcatgtcacaattcagaagtaggacctgagcatagtcttgccgaataccataatgaatctggcttgaaaaccattcttcgtaagggtggtcgcactattgcctttggaggctgtgtgttctcttatgttggttgccataacaagtgtgcctattgggttccacgtgctagcgctaacataggttgtaaccatacaggtgttgttggagaaggttccgaaggtcttaatgacaaccttcttgaaatactccaaaaagagaaagtcaacatcaatattgttggtgactttaaacttaatgaagagatcgccattattttggcatctttttctgcttccacaagtgcttttgtggaaactgtgaaaggtttggattataaagcattcaaacaaattgttgaatcctgtggtaattttaaagttacaaaaggaaaagctaaaaaaggtgcctggaatattggtgaacagaaatcaatactgagtcctctttatgcatttgcatcagaggctgctcgtgttgtacgatcaattttctcccgcactcttgaaactgctcaaaattctgtgcgtgttttacagaaggccgctataacaatactagatggaatttcacagtattcactgagactcattgatgctatgatgttcacatctgatttggctactaacaatctagttgtaatggcctacattacaggtggtgttgttcagttgacttcgcagtggctaactaacatctttggcactgtttatgaaaaactcaaacccgtccttgattggcttgaagagaagtttaaggaaggtgtagagtttcttagagacggttgggaaattgttaaatttatctcaacctgtgcttgtgaaattgtcggtggacaaattgtcacctgtgcaaaggaaattaaggagagtgttcagacattctttaagcttgtaaataaatttttggctttgtgtgctgactctatcattattggtggagctaaacttaaagccttgaatttaggtgaaacatttgtcacgcactcaaagggattgtacagaaagtgtgttaaatccagagaagaaactggcctactcatgcctctaaaagccccaaaagaaattatcttcttagagggagaaacacttcccacagaagtgttaacagaggaagttgtcttgaaaactggtgatttacaaccattagaacaacctactagtgaagctgttgaagctccattggttggtacaccagtttgtattaacgggcttatgttgctcgaaatcaaagacacagaaaagtactgtgcccttgcacctaatatgatggtaacaaacaataccttcacactcaaaggcggtgcaccaacaaaggttacttttggtgatgacactgtgatagaagtgcaaggttacaagagtgtgaatatcacttttgaacttgatgaaaggattgataaagtacttaatgagaagtgctctgcctatacagttgaactcggtacagaagtaaatgagttcgcctgtgttgtggcagatgctgtcataaaaactttgcaaccagtatctgaattacttacaccactgggcattgatttagatgagtggagtatggctacatactacttatttgatgagtctggtgagtttaaattggcttcacatatgtattgttctttctaccctccagatgaggatgaagaagaaggtgattgtgaagaagaagagtttgagccatcaactcaatatgagtatggtactgaagatgattaccaaggtaaacctttggaatttggtgccacttctgctgctcttcaacctgaagaagagcaagaagaagattggttagatgatgatagtcaacaaactgttggtcaacaagacggcagtgaggacaatcagacaactactattcaaacaattgttgaggttcaacctcaattagagatggaacttacaccagttgttcagactattgaagtgaatagttttagtggttatttaaaacttactgacaatgtatacattaaaaatgcagacattgtggaagaagctaaaaaggtaaaaccaacagtggttgttaatgcagccaatgtttaccttaaacatggaggaggtgttgcaggagccttaaataaggctactaacaatgccatgcaagttgaatctgatgattacatagctactaatggaccacttaaagtgggtggtagttgtgttttaagcggacacaatcttgctaaacactgtcttcatgttgtcggcccaaatgttaacaaaggtgaagacattcaacttcttaagagtgcttatgaaaattttaatcagcacgaagttctacttgcaccattattatcagctggtatttttggtgctgaccctatacattctttaagagtttgtgtagatactgttcgcacaaatgtctacttagctgtctttgataaaaatctctatgacaaacttgtttcaagctttttggaaatgaagagtgaaaagcaagttgaacaaaagatcgctgagattcctaaagaggaagttaagccatttataactgaaagtaaaccttcagttgaacagagaaaacaagatgataagaaaatcaaagcttgtgttgaagaagttacaacaactctggaagaaactaagttcctcacagaaaacttgttactttatattgacattaatggcaatcttcatccagattctgccactcttgttagtgacattgacatcactttcttaaagaaagatgctccatatatagtgggtgatgttgttcaagagggtgttttaactgctgtggttatacctactaaaaaggctggtggcactactgaaatgctagcgaaagctttgagaaaagtgccaacagacaattatataaccacttacccgggtcagggtttaaatggttacactgtagaggaggcaaagacagtgcttaaaaagtgtaaaagtgccttttacattctaccatctattatctctaatgagaagcaagaaattcttggaactgtttcttggaatttgcgagaaatgcttgcacatgcagaagaaacacgcaaattaatgcctgtctgtgtggaaactaaagccatagtttcaactatacagcgtaaatataagggtattaaaatacaagagggtgtggttgattatggtgctagattttacttttacaccagtaaaacaactgtagcgtcacttatcaacacacttaacgatctaaatgaaactcttgttacaatgccacttggctatgtaacacatggcttaaatttggaagaagctgctcggtatatgagatctctcaaagtgccagctacagtttctgtttcttcacctgatgctgttacagcgtataatggttatcttacttcttcttctaaaacacctgaagaacattttattgaaaccatctcacttgctggttcctataaagattggtcctattctggacaatctacacaactaggtatagaatttcttaagagaggtgataaaagtgtatattacactagtaatcctaccacattccacctagatggtgaagttatcacctttgacaatcttaagacacttctttctttgagagaagtgaggactattaaggtgtttacaacagtagacaacattaacctccacacgcaagttgtggacatgtcaatgacatatggacaacagtttggtccaacttatttggatggagctgatgttactaaaataaaacctcataattcacatgaaggtaaaacattttatgttttacctaatgatgacactctacgtgttgaggcttttgagtactaccacacaactgatcctagttttctgggtaggtacatgtcagcattaaatcacactaaaaagtggaaatacccacaagttaatggtttaacttctattaaatgggcagataacaactgttatcttgccactgcattgttaacactccaacaaatagagttgaagtttaatccacctgctctacaagatgcttattacagagcaagggctggtgaagctgctaacttttgtgcacttatcttagcctactgtaataagacagtaggtgagttaggtgatgttagagaaacaatgagttacttgtttcaacatgccaatttagattcttgcaaaagagtcttgaacgtggtgtgtaaaacttgtggacaacagcagacaacccttaagggtgtagaagctgttatgtacatgggcacactttcttatgaacaatttaagaaaggtgttcagataccttgtacgtgtggtaaacaagctacaaaatatctagtacaacaggagtcaccttttgttatgatgtcagcaccacctgctcagtatgaacttaagcatggtacatttacttgtgctagtgagtacactggtaattaccagtgtggtcactataaacatataacttctaaagaaactttgtattgcatagacggtgctttacttacaaagtcctcagaatacaaaggtcctattacggatgttttctacaaagaaaacagttacacaacaaccataaaaccagttacttataaattggatggtgttgtttgtacagaaattgaccctaagttggacaattattataagaaagacaattcttatttcacagagcaaccaattgatcttgtaccaaaccaaccatatccaaacgcaagcttcgataattttaagtttgtatgtgataatatcaaatttgctgatgatttaaaccagttaactggttataagaaacctgcttcaagagagcttaaagttacatttttccctgacttaaatggtgatgtggtggctattgattataaacactacacaccctcttttaagaaaggagctaaattgttacataaacctattgtttggcatgttaacaatgcaactaataaagccacgtataaaccaaatacctggtgtatacgttgtctttggagcacaaaaccagttgaaacatcaaattcgtttgatgtactgaagtcagaggacgcgcagggaatggataatcttgcctgcgaagatctaaaaccagtctctgaagaagtagtggaaaatcctaccatacagaaagacgttcttgagtgtaatgtgaaaactaccgaagttgtaggagacattatacttaaaccagcaaataatagtttaaaaattacagaagaggttggccacacagatctaatggctgcttatgtagacaattctagtcttactattaagaaacctaatgaattatctagagtattaggtttgaaaacccttgctactcatggtttagctgctgttaatagtgtcccttgggatactatagctaattatgctaagccttttcttaacaaagttgttagtacaactactaacatagttacacggtgtttaaaccgtgtttgtactaattatatgccttatttctttactttattgctacaattgtgtacttttactagaagtacaaattctagaattaaagcatctatgccgactactatagcaaagaatactgttaagagtgtcggtaaattttgtctagaggcttcatttaattatttgaagtcacctaatttttctaaactgataaatattataatttggtttttactattaagtgtttgcctaggttctttaatctactcaaccgctgctttaggtgttttaatgtctaatttaggcatgccttcttactgtactggttacagagaaggctatttgaactctactaatgtcactattgcaacctactgtactggttctataccttgtagtgtttgtcttagtggtttagattctttagacacctatccttctttagaaactatacaaattaccatttcatcttttaaatgggatttaactgcttttggcttagttgcagagtggtttttggcatatattcttttcactaggtttttctatgtacttggattggctgcaatcatgcaattgtttttcagctattttgcagtacattttattagtaattcttggcttatgtggttaataattaatcttgtacaaatggccccgatttcagctatggttagaatgtacatcttctttgcatcattttattatgtatggaaaagttatgtgcatgttgtagacggttgtaattcatcaacttgtatgatgtgttacaaacgtaatagagcaacaagagtcgaatgtacaactattgttaatggtgttagaaggtccttttatgtctatgctaatggaggtaaaggcttttgcaaactacacaattggaattgtgttaattgtgatacattctgtgctggtagtacatttattagtgatgaagttgcgagagacttgtcactacagtttaaaagaccaataaatcctactgaccagtcttcttacatcgttgatagtgttacagtgaagaatggttccatccatctttactttgataaagctggtcaaaagacttatgaaagacattctctctctcattttgttaacttagacaacctgagagctaataacactaaaggttcattgcctattaatgttatagtttttgatggtaaatcaaaatgtgaagaatcatctgcaaaatcagcgtctgtttactacagtcagcttatgtgtcaacctatactgttactagatcaggcattagtgtctgatgttggtgatagtgcggaagttgcagttaaaatgtttgatgcttacgttaatacgttttcatcaacttttaacgtaccaatggaaaaactcaaaacactagttgcaactgcagaagctgaacttgcaaagaatgtgtccttagacaatgtcttatctacttttatttcagcagctcggcaagggtttgttgattcagatgtagaaactaaagatgttgttgaatgtcttaaattgtcacatcaatctgacatagaagttactggcgatagttgtaataactatatgctcacctataacaaagttgaaaacatgacaccccgtgaccttggtgcttgtattgactgtagtgcgcgtcatattaatgcgcaggtagcaaaaagtcacaacattgctttgatatggaacgttaaagatttcatgtcattgtctgaacaactacgaaaacaaatacgtagtgctgctaaaaagaataacttaccttttaagttgacatgtgcaactactagacaagttgttaatgttgtaacaacaaagatagcacttaagggtggtaaaattgttaataattggttgaagcagttaattaaagttacacttgtgttcctttttgttgctgctattttctatttaataacacctgttcatgtcatgtctaaacatactgacttttcaagtgaaatcataggatacaaggctattgatggtggtgtcactcgtgacatagcatctacagatacttgttttgctaacaaacatgctgattttgacacatggtttagccagcgtggtggtagttatactaatgacaaagcttgcccattgattgctgcagtcataacaagagaagtgggttttgtcgtgcctggtttgcctggcacgatattacgcacaactaatggtgactttttgcatttcttacctagagtttttagtgcagttggtaacatctgttacacaccatcaaaacttatagagtacactgactttgcaacatcagcttgtgttttggctgctgaatgtacaatttttaaagatgcttctggtaagccagtaccatattgttatgataccaatgtactagaaggttctgttgcttatgaaagtttacgccctgacacacgttatgtgctcatggatggctctattattcaatttcctaacacctaccttgaaggttctgttagagtggtaacaacttttgattctgagtactgtaggcacggcacttgtgaaagatcagaagctggtgtttgtgtatctactagtggtagatgggtacttaacaatgattattacagatctttaccaggagttttctgtggtgtagatgctgtaaatttacttactaatatgtttacaccactaattcaacctattggtgctttggacatatcagcatctatagtagctggtggtattgtagctatcgtagtaacatgccttgcctactattttatgaggtttagaagagcttttggtgaatacagtcatgtagttgcctttaatactttactattccttatgtcattcactgtactctgtttaacaccagtttactcattcttacctggtgtttattctgttatttacttgtacttgacattttatcttactaatgatgtttcttttttagcacatattcagtggatggttatgttcacacctttagtacctttctggataacaattgcttatatcatttgtatttccacaaagcatttctattggttctttagtaattacctaaagagacgtgtagtctttaatggtgtttcctttagtacttttgaagaagctgcgctgtgcacctttttgttaaataaagaaatgtatctaaagttgcgtagtgatgtgctattacctcttacgcaatataatagatacttagctctttataataagtacaagtattttagtggagcaatggatacaactagctacagagaagctgcttgttgtcatctcgcaaaggctctcaatgacttcagtaactcaggttctgatgttctttaccaaccaccacaaacctctatcacctcagctgttttgcagagtggttttagaaaaatggcattcccatctggtaaagttgagggttgtatggtacaagtaacttgtggtacaactacacttaacggtctttggcttgatgacgtagtttactgtccaagacatgtgatctgcacctctgaagacatgcttaaccctaattatgaagatttactcattcgtaagtctaatcataatttcttggtacaggctggtaatgttcaactcagggttattggacattctatgcaaaattgtgtacttaagcttaaggttgatacagccaatcctaagacacctaagtataagtttgttcgcattcaaccaggacagactttttcagtgttagcttgttacaatggttcaccatctggtgtttaccaatgtgctatgaggcccaatttcactattaagggttcattccttaatggttcatgtggtagtgttggttttaacatagattatgactgtgtctctttttgttacatgcaccatatggaattaccaactggagttcatgctggcacagacttagaaggtaacttttatggaccttttgttgacaggcaaacagcacaagcagctggtacggacacaactattacagttaatgttttagcttggttgtacgctgctgttataaatggagacaggtggtttctcaatcgatttaccacaactcttaatgactttaaccttgtggctatgaagtacaattatgaacctctaacacaagaccatgttgacatactaggacctctttctgctcaaactggaattgccgttttagatatgtgtgcttcattaaaagaattactgcaaaatggtatgaatggacgtaccatattgggtagtgctttattagaagatgaatttacaccttttgatgttgttagacaatgctcaggtgttactttccaaagtgcagtgaaaagaacaatcaagggtacacaccactggttgttactcacaattttgacttcacttttagttttagtccagagtactcaatggtctttgttcttttttttgtatgaaaatgcctttttaccttttgctatgggtattattgctatgtctgcttttgcaatgatgtttgtcaaacataagcatgcatttctctgtttgtttttgttaccttctcttgccactgtagcttattttaatatggtctatatgcctgctagttgggtgatgcgtattatgacatggttggatatggttgatactagtttgtctggttttaagctaaaagactgtgttatgtatgcatcagctgtagtgttactaatccttatgacagcaagaactgtgtatgatgatggtgctaggagagtgtggacacttatgaatgtcttgacactcgtttataaagtttattatggtaatgctttagatcaagccatttccatgtgggctcttataatctctgttacttctaactactcaggtgtagttacaactgtcatgtttttggccagaggtattgtttttatgtgtgttgagtattgccctattttcttcataactggtaatacacttcagtgtataatgctagtttattgtttcttaggctatttttgtacttgttactttggcctcttttgtttactcaaccgctactttagactgactcttggtgtttatgattacttagtttctacacaggagtttagatatatgaattcacagggactactcccacccaagaatagcatagatgccttcaaactcaacattaaattgttgggtgttggtggcaaaccttgtatcaaagtagccactgtacagtctaaaatgtcagatgtaaagtgcacatcagtagtcttactctcagttttgcaacaactcagagtagaatcatcatctaaattgtgggctcaatgtgtccagttacacaatgacattctcttagctaaagatactactgaagcctttgaaaaaatggtttcactactttctgttttgctttccatgcagggtgctgtagacataaacaagctttgtgaagaaatgctggacaacagggcaaccttacaagctatagcctcagagtttagttcccttccatcatatgcagcttttgctactgctcaagaagcttatgagcaggctgttgctaatggtgattctgaagttgttcttaaaaagttgaagaagtctttgaatgtggctaaatctgaatttgaccgtgatgcagccatgcaacgtaagttggaaaagatggctgatcaagctatgacccaaatgtataaacaggctagatctgaggacaagagggcaaaagttactagtgctatgcagacaatgcttttcactatgcttagaaagttggataatgatgcactcaacaacattatcaacaatgcaagagatggttgtgttcccttgaacataatacctcttacaacagcagccaaactaatggttgtcataccagactataacacatataaaaatacgtgtgatggtacaacatttacttatgcatcagcattgtgggaaatccaacaggttgtagatgcagatagtaaaattgttcaacttagtgaaattagtatggacaattcacctaatttagcatggcctcttattgtaacagctttaagggccaattctgctgtcaaattacagaataatgagcttagtcctgttgcactacgacagatgtcttgtgctgccggtactacacaaactgcttgcactgatgacaatgcgttagcttactacaacacaacaaagggaggtaggtttgtacttgcactgttatccgatttacaggatttgaaatgggctagattccctaagagtgatggaactggtactatctatacagaactggaaccaccttgtaggtttgttacagacacacctaaaggtcctaaagtgaagtatttatactttattaaaggattaaacaacctaaatagaggtatggtacttggtagtttagctgccacagtacgtctacaagctggtaatgcaacagaagtgcctgccaattcaactgtattatctttctgtgcttttgctgtagatgctgctaaagcttacaaagattatctagctagtgggggacaaccaatcactaattgtgttaagatgttgtgtacacacactggtactggtcaggcaataacagttacaccggaagccaatatggatcaagaatcctttggtggtgcatcgtgttgtctgtactgccgttgccacatagatcatccaaatcctaaaggattttgtgacttaaaaggtaagtatgtacaaatacctacaacttgtgctaatgaccctgtgggttttacacttaaaaacacagtctgtaccgtctgcggtatgtggaaaggttatggctgtagttgtgatcaactccgcgaacccatgcttcagtcagctgatgcacaatcgtttttaaacgggtttgcggtgtaagtgcagcccgtcttacaccgtgcggcacaggcactagtactgatgtcgtatacagggcttttgacatctacaatgataaagtagctggttttgctaaattcctaaaaactaattgttgtcgcttccaagaaaaggacgaagatgacaatttaattgattcttactttgtagttaagagacacactttctctaactaccaacatgaagaaacaatttataatttacttaaggattgtccagctgttgctaaacatgacttctttaagtttagaatagacggtgacatggtaccacatatatcacgtcaacgtcttactaaatacacaatggcagacctcgtctatgctttaaggcattttgatgaaggtaattgtgacacattaaaagaaatacttgtcacatacaattgttgtgatgatgattatttcaataaaaaggactggtatgattttgtagaaaacccagatatattacgcgtatacgccaacttaggtgaacgtgtacgccaagctttgttaaaaacagtacaattctgtgatgccatgcgaaatgctggtattgttggtgtactgacattagataatcaagatctcaatggtaactggtatgatttcggtgatttcatacaaaccacgccaggtagtggagttcctgttgtagattcttattattcattgttaatgcctatattaaccttgaccagggctttaactgcagagtcacatgttgacactgacttaacaaagccttacattaagtgggatttgttaaaatatgacttcacggaagagaggttaaaactctttgaccgttattttaaatattgggatcagacataccacccaaattgtgttaactgtttggatgacagatgcattctgcattgtgcaaactttaatgttttattctctacagtgttcccacctacaagttttggaccactagtgagaaaaatatttgttgatggtgttccatttgtagtttcaactggataccacttcagagagctaggtgttgtacataatcaggatgtaaacttacatagctctagacttagttttaaggaattacttgtgtatgctgctgaccctgctatgcacgctgcttctggtaatctattactagataaacgcactacgtgcttttcagtagctgcacttactaacaatgttgcttttcaaactgtcaaacccggtaattttaacaaagacttctatgactttgctgtgtctaagggtttctttaaggaaggaagttctgttgaattaaaacacttcttctttgctcaggatggtaatgctgctatcagcgattatgactactatcgttataatctaccaacaatgtgtgatatcagacaactactatttgtagttgaagttgttgataagtactttgattgttacgatggtggctgtattaatgctaaccaagtcatcgtcaacaacctagacaaatcagctggttttccatttaataaatggggtaaggctagactttattatgattcaatgagttatgaggatcaagatgcacttttcgcatatacaaaacgtaatgtcatccctactataactcaaatgaatcttaagtatgccattagtgcaaagaatagagctcgcaccgtagctggtgtctctatctgtagtactatgaccaatagacagtttcatcaaaaattattgaaatcaatagccgccactagaggagctactgtagtaattggaacaagcaaattctatggtggttggcacaacatgttaaaaactgtttatagtgatgtagaaaaccctcaccttatgggttgggattatcctaaatgtgatagagccatgcctaacatgcttagaattatggcctcacttgttcttgctcgcaaacatacaacgtgttgtagcttgtcacaccgtttctatagattagctaatgagtgtgctcaagtattgagtgaaatggtcatgtgtggcggttcactatatgttaaaccaggtggaacctcatcaggagatgccacaactgcttatgctaatagtgtttttaacatttgtcaagctgtcacggccaatgttaatgcacttttatctactgatggtaacaaaattgccgataagtatgtccgcaatttacaacacagactttatgagtgtctctatagaaatagagatgttgacacagactttgtgaatgagttttacgcatatttgcgtaaacatttctcaatgatgatactctctgacgatgctgttgtgtgtttcaatagcacttatgcatctcaaggtctagtggctagcataaagaactttaagtcagttctttattatcaaaacaatgtttttatgtctgaagcaaaatgttggactgagactgaccttactaaaggacctcatgaattttgctctcaacatacaatgctagttaaacagggtgatgattatgtgtaccttccttacccagatccatcaagaatcctaggggccggctgttttgtagatgatatcgtaaaaacagatggtacacttatgattgaacggttcgtgtctttagctatagatgcttacccacttactaaacatcctaatcaggagtatgctgatgtctttcatttgtacttacaatacataagaaagctacatgatgagttaacaggacacatgttagacatgtattctgttatgcttactaatgataacacttcaaggtattgggaacctgagttttatgaggctatgtacacaccgcatacagtcttacaggctgttggggcttgtgttctttgcaattcacagacttcattaagatgtggtgcttgcatacgtagaccattcttatgttgtaaatgctgttacgaccatgtcatatcaacatcacataaattagtcttgtctgttaatccgtatgtttgcaatgctccaggttgtgatgtcacagatgtgactcaactttacttaggaggtatgagctattattgtaaatcacataaaccacccattagttttccattgtgtgctaatggacaagtttttggtttatataaaaatacatgtgttggtagcgataatgttactgactttaatgcaattgcaacatgtgactggacaaatgctggtgattacattttagctaacacctgtactgaaagactcaagctttttgcagcagaaacgctcaaagctactgaggagacatttaaactgtcttatggtattgctactgtacgtgaagtgctgtctgacagagaattacatctttcatgggaagttggtaaacctagaccaccacttaaccgaaattatgtctttactggttatcgtgtaactaaaaacagtaaagtacaaataggagagtacacctttgaaaaaggtgactatggtgatgctgttgtttaccgaggtacaacaacttacaaattaaatgttggtgattattttgtgctgacatcacatacagtaatgccattaagtgcacctacactagtgccacaagagcactatgttagaattactggcttatacccaacactcaatatctcagatgagttttctagcaatgttgcaaattatcaaaaggttggtatgcaaaagtattctacactccagggaccacctggtactggtaagagtcattttgctattggcctagctctctactacccttctgctcgcatagtgtatacagcttgctctcatgccgctgttgatgcactatgtgagaaggcattaaaatatttgcctatagataaatgtagtagaattatacctgcacgtgctcgtgtagagtgttttgataaattcaaagtgaattcaacattagaacagtatgtcttttgtactgtaaatgcattgcctgagacgacagcagatatagttgtctttgatgaaatttcaatggccacaaattatgatttgagtgttgtcaatgccagattacgtgctaagcactatgtgtacattggcgaccctgctcaattacctgcaccacgcacattgctaactaagggcacactagaaccagaatatttcaattcagtgtgtagacttatgaaaactataggtccagacatgttcctcggaacttgtcggcgttgtcctgctgaaattgttgacactgtgagtgctttggtttatgataataagcttaaagcacataaagacaaatcagctcaatgctttaaaatgttttataagggtgttatcacgcatgatgtttcatctgcaattaacaggccacaaataggcgtggtaagagaattccttacacgtaaccctgcttggagaaaagctgtctttatttcaccttataattcacagaatgctgtagcctcaaagattttgggactaccaactcaaactgttgattcatcacagggctcagaatatgactatgtcatattcactcaaaccactgaaacagctcactcttgtaatgtaaacagatttaatgttgctattaccagagcaaaagtaggcatactttgcataatgtctgatagagacctttatgacaagttgcaatttacaagtcttgaaattccacgtaggaatgtggcaactttacaagctgaaaatgtaacaggactctttaaagattgtagtaaggtaatcactgggttacatcctacacaggcacctacacacctcagtgttgacactaaattcaaaactgaaggtttatgtgttgacatacctggcatacctaaggacatgacctatagaagactcatctctatgatgggttttaaaatgaattatcaagttaatggttaccctaacatgtttatcacccgcgaagaagctataagacatgtacgtgcatggattggcttcgatgtcgaggggtgtcatgctactagagaagctgttggtaccaatttacctttacagctaggtttttctacaggtgttaacctagttgctgtacctacaggttatgttgatacacctaataatacagatttttccagagttagtgctaaaccaccgcctggagatcaatttaaacacctcataccacttatgtacaaaggacttccttggaatgtagtgcgtataaagattgtacaaatgttaagtgacacacttaaaaatctctctgacagagtcgtatttgtcttatgggcacatggctttgagttgacatctatgaagtattttgtgaaaataggacctgagcgcacctgttgtctatgtgatagacgtgccacatgcttttccactgcttcagacacttatgcctgttggcatcattctattggatttgattacgtctataatccgtttatgattgatgttcaacaatggggttttacaggtaacctacaaagcaaccatgatctgtattgtcaagtccatggtaatgcacatgtagctagttgtgatgcaatcatgactaggtgtctagctgtccacgagtgctttgttaagcgtgttgactggactattgaatatcctataattggtgatgaactgaagattaatgcggcttgtagaaaggttcaacacatggttgttaaagctgcattattagcagacaaattcccagttcttcacgacattggtaaccctaaagctattaagtgtgtacctcaagctgatgtagaatggaagttctatgatgcacagccttgtagtgacaaagcttataaaatagaagaattattctattcttatgccacacattctgacaaattcacagatggtgtatgcctattttggaattgcaatgtcgatagatatcctgctaattccattgtttgtagatttgacactagagtgctatctaaccttaacttgcctggttgtgatggtggcagtttgtatgtaaataaacatgcattccacacaccagcttttgataaaagtgcttttgttaatttaaaacaattaccatttttctattactctgacagtccatgtgagtctcatggaaaacaagtagtgtcagatatagattatgtaccactaaagtctgctacgtgtataacacgttgcaatttaggtggtgctgtctgtagacatcatgctaatgagtacagattgtatctcgatgcttataacatgatgatctcagctggctttagcttgtgggtttacaaacaatttgatacttataacctctggaacacttttacaagacttcagagtttagaaaatgtggcttttaatgttgtaaataagggacactttgatggacaacagggtgaagtaccagtttctatcattaataacactgtttacacaaaagttgatggtgttgatgtagaattgtttgaaaataaaacaacattacctgttaatgtagcatttgagctttgggctaagcgcaacattaaaccagtaccagaggtgaaaatactcaataatttgggtgtggacattgctgctaatactgtgatctgggactacaaaagagatgctccagcacatatatctactattggtgtttgttctatgactgacatagccaagaaaccaactgaaacgatttgtgcaccactcactgtcttttttgatggtagagttgatggtcaagtagacttatttagaaatgcccgtaatggtgttcttattacagaaggtagtgttaaaggtttacaaccatctgtaggtcccaaacaagctagtcttaatggagtcacattaattggagaagccgtaaaaacacagttcaattattataagaaagttgatggtgttgtccaacaattacctgaaacttactttactcagagtagaaatttacaagaatttaaacccaggagtcaaatggaaattgatttcttagaattagctatggatgaattcattgaacggtataaattagaaggctatgccttcgaacatatcgtttatggagattttagtcatagtcagttaggtggtttacatctactgattggactagctaaacgttttaaggaatcaccttttgaattagaagattttattcctatggacagtacagttaaaaactatttcataacagatgcgcaaacaggttcatctaagtgtgtgtgttctgttattgatttattacttgatgattttgttgaaataataaaatcccaagatttatctgtagtttctaaggttgtcaaagtgactattgactatacagaaatttcatttatgctttggtgtaaagatggccatgtagaaacattttacccaaaattacaatctagtcaagcgtggcaaccgggtgttgctatgcctaatctttacaaaatgcaaagaatgctattagaaaagtgtgaccttcaaaattatggtgatagtgcaacattacctaaaggcataatgatgaatgtcgcaaaatatactcaactgtgtcaatatttaaacacattaacattagctgtaccctataatatgagagttatacattttggtgctggttctgataaaggagttgcaccaggtacagctgttttaagacagtggttgcctacgggtacgctgcttgtcgattcagatcttaatgactttgtctctgatgcagattcaactttgattggtgattgtgcaactgtacatacagctaataaatgggatctcattattagtgatatgtacgaccctaagactaaaaatgttacaaaagaaaatgactctaaagagggttttttcacttacatttgtgggtttatacaacaaaagctagctcttggaggttccgtggctataaagataacagaacattcttggaatgctgatctttataagctcatgggacacttcgcatggtggacagcctttgttactaatgtgaatgcgtcatcatctgaagcatttttaattggatgtaattatcttggcaaaccacgcgaacaaatagatggttatgtcatgcatgcaaattacatattttggaggaatacaaatccaattcagttgtcttcctattctttatttgacatgagtaaatttccccttaaattaaggggtactgctgttatgtctttaaaagaaggtcaaatcaatgatatgattttatctcttcttagtaaaggtagacttataattagagaaaacaacagagttgttatttctagtgatgttcttgttaacaactaaacgaacaatgtttgtttttcttgttttattgccactagtctctagtcagtgtgttaatcttacaaccagaactcaattaccccctgcatacactaattctttcacacgtggtgtttattaccctgacaaagttttcagatcctcagttttacattcaactcaggacttgttcttacctttcttttccaatgttacttggttccatgctatacatgtctctgggaccaatggtactaagaggtttgataaccctgtcctaccatttaatgatggtgtttattttgcttccactgagaagtctaacataataagaggctggatttttggtactactttagattcgaagacccagtccctacttattgttaataacgctactaatgttgttattaaagtctgtgaatttcaattttgtaatgatccatttttgggtgtttattaccacaaaaacaacaaaagttggatggaaagtgagttcagagtttattctagtgcgaataattgcacttttgaatatgtctctcagccttttcttatggaccttgaaggaaaacagggtaatttcaaaaatcttagggaatttgtgtttaagaatattgatggttattttaaaatatattctaagcacacgcctattaatttagtgcgtgatctccctcagggtttttcggctttagaaccattggtagatttgccaataggtattaacatcactaggtttcaaactttacttgctttacatagaagttatttgactcctggtgattcttcttcaggttggacagctggtgctgcagcttattatgtgggttatcttcaacctaggacttttctattaaaatataatgaaaatggaaccattacagatgctgtagactgtgcacttgaccctctctcagaaacaaagtgtacgttgaaatccttcactgtagaaaaaggaatctatcaaacttctaactttagagtccaaccaacagaatctattgttagatttcctaatattacaaacttgtgcccttttggtgaagtttttaacgccaccagatttgcatctgtttatgcttggaacaggaagagaatcagcaactgtgttgctgattattctgtcctatataattccgcatcattttccacttttaagtgttatggagtgtctcctactaaattaaatgatctctgctttactaatgtctatgcagattcatttgtaattagaggtgatgaagtcagacaaatcgctccagggcaaactggaaagattgctgattataattataaattaccagatgattttacaggctgcgttatagcttggaattctaacaatcttgattctaaggttggtggtaattataattacctgtatagattgtttaggaagtctaatctcaaaccttttgagagagatatttcaactgaaatctatcaggccggtagcacaccttgtaatggtgttgaaggttttaattgttactttcctttacaatcatatggtttccaacccactaatggtgttggttaccaaccatacagagtagtagtactttcttttgaacttctacatgcaccagcaactgtttgtggacctaaaaagtctactaatttggttaaaaacaaatgtgtcaatttcaacttcaatggtttaacaggcacaggtgttcttactgagtctaacaaaaagtttctgcctttccaacaatttggcagagacattgctgacactactgatgctgtccgtgatccacagacacttgagattcttgacattacaccatgttcttttggtggtgtcagtgttataacaccaggaacaaatacttctaaccaggttgctgttctttatcaggatgttaactgcacagaagtccctgttgctattcatgcagatcaacttactcctacttggcgtgtttattctacaggttctaatgtttttcaaacacgtgcaggctgtttaataggggctgaacatgtcaacaactcatatgagtgtgacatacccattggtgcaggtatatgcgctagttatcagactcagactaattctcctcggcgggcacgtagtgtagctagtcaatccatcattgcctacactatgtcacttggtgcagaaaattcagttgcttactctaataactctattgccatacccacaaattttactattagtgttaccacagaaattctaccagtgtctatgaccaagacatcagtagattgtacaatgtacatttgtggtgattcaactgaatgcagcaatcttttgttgcaatatggcagtttttgtacacaattaaaccgtgctttaactggaatagctgttgaacaagacaaaaacacccaagaagtttttgcacaagtcaaacaaatttacaaaacaccaccaattaaagattttggtggttttaatttttcacaaatattaccagatccatcaaaaccaagcaagaggtcatttattgaagatctacttttcaacaaagtgacacttgcagatgctggcttcatcaaacaatatggtgattgccttggtgatattgctgctagagacctcatttgtgcacaaaagtttaacggccttactgttttgccacctttgctcacagatgaaatgattgctcaatacacttctgcactgttagcgggtacaatcacttctggttggacctttggtgcaggtgctgcattacaaataccatttgctatgcaaatggcttataggtttaatggtattggagttacacagaatgttctctatgagaaccaaaaattgattgccaaccaatttaatagtgctattggcaaaattcaagactcactttcttccacagcaagtgcacttggaaaacttcaagatgtggtcaaccaaaatgcacaagctttaaacacgcttgttaaacaacttagctccaattttggtgcaatttcaagtgttttaaatgatatcctttcacgtcttgacaaagttgaggctgaagtgcaaattgataggttgatcacaggcagacttcaaagtttgcagacatatgtgactcaacaattaattagagctgcagaaatcagagcttctgctaatcttgctgctactaaaatgtcagagtgtgtacttggacaatcaaaaagagttgatttttgtggaaagggctatcatcttatgtccttccctcagtcagcacctcatggtgtagtcttcttgcatgtgacttatgtccctgcacaagaaaagaacttcacaactgctcctgccatttgtcatgatggaaaagcacactttcctcgtgaaggtgtctttgtttcaaatggcacacactggtttgtaacacaaaggaatttttatgaaccacaaatcattactacagacaacacatttgtgtctggtaactgtgatgttgtaataggaattgtcaacaacacagtttatgatcctttgcaacctgaattagactcattcaaggaggagttagataaatattttaagaatcatacatcaccagatgttgatttaggtgacatctctggcattaatgcttcagttgtaaacattcaaaaagaaattgaccgcctcaatgaggttgccaagaatttaaatgaatctctcatcgatctccaagaacttggaaagtatgagcagtatataaaatggccatggtacatttggctaggttttatagctggcttgattgccatagtaatggtgacaattatgctttgctgtatgaccagttgctgtagttgtctcaagggctgttgttcttgtggatcctgctgcaaatttgatgaagacgactctgagccagtgctcaaaggagtcaaattacattacacataaacgaacttatggatttgtttatgagaatcttcacaattggaactgtaactttgaagcaaggtgaaatcaaggatgctactccttcagattttgttcgcgctactgcaacgataccgatacaagcctcactccctttcggatggcttattgttggcgttgcacttcttgctgtttttcagagcgcttccaaaatcataaccctcaaaaagagatggcaactagcactctccaagggtgttcactttgtttgcaacttgctgttgttgtttgtaacagtttactcacaccttttgctcgttgctgctggccttgaagccccttttctctatctttatgctttagtctacttcttgcagagtataaactttgtaagaataataatgaggctttggctttgctggaaatgccgttccaaaaacccattactttatgatgccaactattttctttgctggcatactaattgttacgactattgtataccttacaatagtgtaacttcttcaattgtcattacttcaggtgatggcacaacaagtcctatttctgaacatgactaccagattggtggttatactgaaaaatgggaatctggagtaaaagactgtgttgtattacacagttacttcacttcagactattaccagctgtactcaactcaattgagtacagacactggtgttgaacatgttaccttcttcatctacaataaaattgttgatgagcctgaagaacatgtccaaattcacacaatcgacggttcatccggagttgttaatccagtaatggaaccaatttatgatgaaccgacgacgactactagcgtgcctttgtaagcacaagctgatgagtacgaacttatgtactcattcgtttcggaagagacaggtacgttaatagttaatagcgtacttctttttcttgctttcgtggtattcttgctagttacactagccatccttactgcgcttcgattgtgtgcgtactgctgcaatattgttaacgtgagtcttgtaaaaccttctttttacgtttactctcgtgttaaaaatctgaattcttctagagttcctgatcttctggtctaaacgaactaaatattatattagtttttctgtttggaactttaattttagccatggcagattccaacggtactattaccgttgaagagcttaaaaagctccttgaacaatggaacctagtaataggtttcctattccttacatggatttgtcttctacaatttgcctatgccaacaggaataggtttttgtatataattaagttaattttcctctggctgttatggccagtaactttagcttgttttgtgcttgctgctgtttacagaataaattggatcaccggtggaattgctatcgcaatggcttgtcttgtaggcttgatgtggctcagctacttcattgcttctttcagactgtttgcgcgtacgcgttccatgtggtcattcaatccagaaactaacattcttctcaacgtgccactccatggcactattctgaccagaccgcttctagaaagtgaactcgtaatcggagctgtgatccttcgtggacatcttcgtattgctggacaccatctaggacgctgtgacatcaaggacctgcctaaagaaatcactgttgctacatcacgaacgctttcttattacaaattgggagcttcgcagcgtgtagcaggtgactcaggttttgctgcatacagtcgctacaggattggcaactataaattaaacacagaccattccagtagcagtgacaatattgctttgcttgtacagtaagtgacaacagatgtttcatctcgttgactttcaggttactatagcagagatattactaattattatgaggacttttaaagtttccatttggaatcttgattacatcataaacctcataattaaaaatttatctaagtcactaactgagaataaatattctcaattagatgaagagcaaccaatggagattgattaaacgaacatgaaaattattcttttcttggcactgataacactcgctacttgtgagctttatcactaccaagagtgtgttagaggtacaacagtacttttaaaagaaccttgctcttctggaacatacgagggcaattcaccatttcatcctctagctgataacaaatttgcactgacttgctttagcactcaatttgcttttgcttgtcctgacggcgtaaaacacgtctatcagttacgtgccagatcagtttcacctaaactgttcatcagacaagaggaagttcaagaactttactctccaatttttcttattgttgcggcaatagtgtttataacactttgcttcacactcaaaagaaagacagaatgattgaactttcattaattgacttctatttgtgctttttagcctttctgctattccttgttttaattatgcttattatcttttggttctcacttgaactgcaagatcataatgaaacttgtcacgcctaaacgaacatgaaatttcttgttttcttaggaatcatcacaactgtagctgcatttcaccaagaatgtagtttacagtcatgtactcaacatcaaccatatgtagttgatgacccgtgtcctattcacttctattctaaatggtatattagagtaggagctagaaaatcagcacctttaattgaattgtgcgtggatgaggctggttctaaatcacccattcagtacatcgatatcggtaattatacagtttcctgtttaccttttacaattaattgccaggaacctaaattgggtagtcttgtagtgcgttgttcgttctatgaagactttttagagtatcatgacgttcgtgttgttttagatttcatctaaacgaacaaactaaaatgtctgataatggaccccaaaatcagcgaaatgcaccccgcattacgtttggtggaccctcagattcaactggcagtaaccagaatggagaacgcagtggggcgcgatcaaaacaacgtcggccccaaggtttacccaataatactgcgtcttggttcaccgctctcactcaacatggcaaggaagaccttaaattccctcgaggacaaggcgttccaattaacaccaatagcagtccagatgaccaaattggctactaccgaagagctaccagacgaattcgtggtggtgacggtaaaatgaaagatctcagtccaagatggtatttctactacctaggaactgggccagaagctggacttccctatggtgctaacaaagacggcatcatatgggttgcaactgagggagccttgaatacaccaaaagatcacattggcacccgcaatcctgctaacaatgctgcaatcgtgctacaacttcctcaaggaacaacattgccaaaaggcttctacgcagaagggagcagaggcggcagtcaagcctcttctcgttcctcatcacgtagtcgcaacagttcaagaaattcaactccaggcagcagtaggggaacttctcctgctagaatggctggcaatggcggtgatgctgctcttgctttgctgctgcttgacagattgaaccagcttgagagcaaaatgtctggtaaaggccaacaacaacaaggccaaactgtcactaagaaatctgctgctgaggcttctaagaagcctcggcaaaaacgtactgccactaaagcatacaatgtaacacaagctttcggcagacgtggtccagaacaaacccaaggaaattttggggaccaggaactaatcagacaaggaactgattacaaacattggccgcaaattgcacaatttgcccccagcgcttcagcgttcttcggaatgtcgcgcattggcatggaagtcacaccttcgggaacgtggttgacctacacaggtgccatcaaattggatgacaaagatccaaatttcaaagatcaagtcattttgctgaataagcatattgacgcatacaaaacattcccaccaacagagcctaaaaaggacaaaaagaagaaggctgatgaaactcaagccttaccgcagagacagaagaaacagcaaactgtgactcttcttcctgctgcagatttggatgatttctccaaacaattgcaacaatccatgagcagtgctgactcaactcaggcctaaactcatgcagaccacacaaggcagatgggctatataaacgttttcgcttttccgtttacgatatatagtctactcttgtgcagaatgaattctcgtaactacatagcacaagtagatgtagttaactttaatctcacatagcaatctttaatcagtgtgtaacattagggaggacttgaaagagccaccacattttcaccgaggccacgcggagtacgatcgagtgtacagtgaacaatgctagggagagctgcctatatggaagagccctaatgtgtaaaattaattttagtagtgctatccccatgtgattttaatagcttcttaggagaatgacaaaaaaaaaaaaaaaaaaaaaaaaaaaaaaaaa

SEQ ID NO: 2 - DNA, 27789 bp, Coronaviridae
  misc_feature 1..27789: note = SARS-CoV-2-[3,E,6,7,8]
  source 1..27789: mol_type = other DNA
attaaaggtttataccttcccaggtaacaaaccaaccaactttcgatctcttgtagatctgttctctaaacgaactttaaaatctgtgtggctgtcactcggctgcatgcttagtgcactcacgcagtataattaataactaattactgtcgttgacaggacacgagtaactcgtctatcttctgcaggctgcttacggtttcgtccgtgttgcagccgatcatcagcacatctaggtttcgtccgggtgtgaccgaaaggtaagatggagagccttgtccctggtttcaacgagaaaacacacgtccaactcagtttgcctgttttacaggttcgcgacgtgctcgtacgtggctttggagactccgtggaggaggtcttatcagaggcacgtcaacatcttaaagatggcacttgtggcttagtagaagttgaaaaaggcgttttgcctcaacttgaacagccctatgtgttcatcaaacgttcggatgctcgaactgcacctcatggtcatgttatggttgagctggtagcagaactcgaaggcattcagtacggtcgtagtggtgagacacttggtgtccttgtccctcatgtgggcgaaataccagtggcttaccgcaaggttcttcttcgtaagaacggtaataaaggagctggtggccatagttacggcgccgatctaaagtcatttgacttaggcgacgagcttggcactgatccttatgaagattttcaagaaaactggaacactaaacatagcagtggtgttacccgtgaactcatgcgtgagcttaacggaggggcatacactcgctatgtcgataacaacttctgtggccctgatggctaccctcttgagtgcattaaagaccttctagcacgtgctggtaaagcttcatgcactttgtccgaacaactggactttattgacactaagaggggtgtatactgctgccgtgaacatgagcatgaaattgcttggtacacggaacgttctgaaaagagctatgaattgcagacaccttttgaaattaaattggcaaagaaatttgacaccttcaatggggaatgtccaaattttgtatttcccttaaattccataatcaagactattcaaccaagggttgaaaagaaaaagcttgatggctttatgggtagaattcgatctgtctatccagttgcgtcaccaaatgaatgcaaccaaatgtgcctttcaactctcatgaagtgtgatcattgtggtgaaacttcatggcagacgggcgattttgttaaagccacttgcgaattttgtggcactgagaatttgactaaagaaggtgccactacttgtggttacttaccccaaaatgctgttgttaaaatttattgtccagcatgtcacaattcagaagtaggacctgagcatagtcttgccgaataccataatgaatctggcttgaaaaccattcttcgtaagggtggtcgcactattgcctttggaggctgtgtgttctcttatgttggttgccataacaagtgtgcctattgggttccacgtgctagcgctaacataggttgtaaccatacaggtgttgttggagaaggttccgaaggtcttaatgacaaccttcttgaaatactccaaaaagagaaagtcaacatcaatattgttggtgactttaaacttaatgaagagatcgccattattttggcatctttttctgcttccacaagtgcttttgtggaaactgtgaaaggtttggattataaagcattcaaacaaattgttgaatcctgtggtaattttaaagttacaaaaggaaaagctaaaaaaggtgcctggaatattggtgaacagaaatcaatactgagtcctctttatgcatttgcatcagaggctgctcgtgttgtacgatcaattttctcccgcactcttgaaactgctcaaaattctgtgcgtgttttacagaaggccgctataacaatactagatggaatttcacagtattcactgagactcattgatgctatgatgttcacatctgatttggctactaacaatctagttgtaatggcctacattacaggtggtgttgttcagttgacttcgcagtggctaactaacatctttggcactgtttatgaaaaactcaaacccgtccttgattggcttgaagagaagtttaaggaaggtgtagagtttcttagagacggttgggaaattgttaaatttatctcaacctgtgcttgtgaaattgtcggtggacaaattgtcacctgtgcaaaggaaattaaggagagtgttcagacattctttaagcttgtaaataaatttttggctttgtgtgctgactctatcattattggtggagctaaacttaaagccttgaatttaggtgaaacatttgtcacgcactcaaagggattgtacagaaagtgtgttaaatccagagaagaaactggcctactcatgcctctaaaagccccaaaagaaattatcttcttagagggagaaacacttcccacagaagtgttaacagaggaagttgtcttgaaaactggtgatttacaaccattagaacaacctactagtgaagctgttgaagctccattggttggtacaccagtttgtattaacgggcttatgttgctcgaaatcaaagacacagaaaagtactgtgcccttgcacctaatatgatggtaacaaacaataccttcacactcaaaggcggtgcaccaacaaaggttacttttggtgatgacactgtgatagaagtgcaaggttacaagagtgtgaatatcacttttgaacttgatgaaaggattgataaagtacttaatgagaagtgctctgcctatacagttgaactcggtacagaagtaaatgagttcgcctgtgttgtggcagatgctgtcataaaaactttgcaaccagtatctgaattacttacaccactgggcattgatttagatgagtggagtatggctacatactacttatttgatgagtctggtgagtttaaattggcttcacatatgtattgttctttctaccctccagatgaggatgaagaagaaggtgattgtgaagaagaagagtttgagccatcaactcaatatgagtatggtactgaagatgattaccaaggtaaacctttggaatttggtgccacttctgctgctcttcaacctgaagaagagcaagaagaagattggttagatgatgatagtcaacaaactgttggtcaacaagacggcagtgaggacaatcagacaactactattcaaacaattgttgaggttcaacctcaattagagatggaacttacaccagttgttcagactattgaagtgaatagttttagtggttatttaaaacttactgacaatgtatacattaaaaatgcagacattgtggaagaagctaaaaaggtaaaaccaacagtggttgttaatgcagccaatgtttaccttaaacatggaggaggtgttgcaggagccttaaataaggctactaacaatgccatgcaagttgaatctgatgattacatagctactaatggaccacttaaagtgggtggtagttgtgttttaagcggacacaatcttgctaaacactgtcttcatgttgtcggcccaaatgttaacaaaggtgaagacattcaacttcttaagagtgcttatgaaaattttaatcagcacgaagttctacttgcaccattattatcagctggtatttttggtgctgaccctatacattctttaagagtttgtgtagatactgttcgcacaaatgtctacttagctgtctttgataaaaatctctatgacaaacttgtttcaagctttttggaaatgaagagtgaaaagcaagttgaacaaaagatcgctgagattcctaaagaggaagttaagccatttataactgaaagtaaaccttcagttgaacagagaaaacaagatgataagaaaatcaaagcttgtgttgaagaagttacaacaactctggaagaaactaagttcctcacagaaaacttgttactttatattgacattaatggcaatcttcatccagattctgccactcttgttagtgacattgacatcactttcttaaagaaagatgctccatatatagtgggtgatgttgttcaagagggtgttttaactgctgtggttatacctactaaaaaggctggtggcactactgaaatgctagcgaaagctttgagaaaagtgccaacagacaattatataaccacttacccgggtcagggtttaaatggttacactgtagaggaggcaaagacagtgcttaaaaagtgtaaaagtgccttttacattctaccatctattatctctaatgagaagcaagaaattcttggaactgtttcttggaatttgcgagaaatgcttgcacatgcagaagaaacacgcaaattaatgcctgtctgtgtggaaactaaagccatagtttcaactatacagcgtaaatataagggtattaaaatacaagagggtgtggttgattatggtgctagattttacttttacaccagtaaaacaactgtagcgtcacttatcaacacacttaacgatctaaatgaaactcttgttacaatgccacttggctatgtaacacatggcttaaatttggaagaagctgctcggtatatgagatctctcaaagtgccagctacagtttctgtttcttcacctgatgctgttacagcgtataatggttatcttacttcttcttctaaaacacctgaagaacattttattgaaaccatctcacttgctggttcctataaagattggtcctattctggacaatctacacaactaggtatagaatttcttaagagaggtgataaaagtgtatattacactagtaatcctaccacattccacctagatggtgaagttatcacctttgacaatcttaagacacttctttctttgagagaagtgaggactattaaggtgtttacaacagtagacaacattaacctccacacgcaagttgtggacatgtcaatgacatatggacaacagtttggtccaacttatttggatggagctgatgttactaaaataaaacctcataattcacatgaaggtaaaacattttatgttttacctaatgatgacactctacgtgttgaggcttttgagtactaccacacaactgatcctagttttctgggtaggtacatgtcagcattaaatcacactaaaaagtggaaatacccacaagttaatggtttaacttctattaaatgggcagataacaactgttatcttgccactgcattgttaacactccaacaaatagagttgaagtttaatccacctgctctacaagatgcttattacagagcaagggctggtgaagctgctaacttttgtgcacttatcttagcctactgtaataagacagtaggtgagttaggtgatgttagagaaacaatgagttacttgtttcaacatgccaatttagattcttgcaaaagagtcttgaacgtggtgtgtaaaacttgtggacaacagcagacaacccttaagggtgtagaagctgttatgtacatgggcacactttcttatgaacaatttaagaaaggtgttcagataccttgtacgtgtggtaaacaagctacaaaatatctagtacaacaggagtcaccttttgttatgatgtcagcaccacctgctcagtatgaacttaagcatggtacatttacttgtgctagtgagtacactggtaattaccagtgtggtcactataaacatataacttctaaagaaactttgtattgcatagacggtgctttacttacaaagtcctcagaatacaaaggtcctattacggatgttttctacaaagaaaacagttacacaacaaccataaaaccagttacttataaattggatggtgttgtttgtacagaaattgaccctaagttggacaattattataagaaagacaattcttatttcacagagcaaccaattgatcttgtaccaaaccaaccatatccaaacgcaagcttcgataattttaagtttgtatgtgataatatcaaatttgctgatgatttaaaccagttaactggttataagaaacctgcttcaagagagcttaaagttacatttttccctgacttaaatggtgatgtggtggctattgattataaacactacacaccctcttttaagaaaggagctaaattgttacataaacctattgtttggcatgttaacaatgcaactaataaagccacgtataaaccaaatacctggtgtatacgttgtctttggagcacaaaaccagttgaaacatcaaattcgtttgatgtactgaagtcagaggacgcgcagggaatggataatcttgcctgcgaagatctaaaaccagtctctgaagaagtagtggaaaatcctaccatacagaaagacgttcttgagtgtaatgtgaaaactaccgaagttgtaggagacattatacttaaaccagcaaataatagtttaaaaattacagaagaggttggccacacagatctaatggctgcttatgtagacaattctagtcttactattaagaaacctaatgaattatctagagtattaggtttgaaaacccttgctactcatggtttagctgctgttaatagtgtcccttgggatactatagctaattatgctaagccttttcttaacaaagttgttagtacaactactaacatagttacacggtgtttaaaccgtgtttgtactaattatatgccttatttctttactttattgctacaattgtgtacttttactagaagtacaaattctagaattaaagcatctatgccgactactatagcaaagaatactgttaagagtgtcggtaaattttgtctagaggcttcatttaattatttgaagtcacctaatttttctaaactgataaatattataatttggtttttactattaagtgtttgcctaggttctttaatctactcaaccgctgctttaggtgttttaatgtctaatttaggcatgccttcttactgtactggttacagagaaggctatttgaactctactaatgtcactattgcaacctactgtactggttctataccttgtagtgtttgtcttagtggtttagattctttagacacctatccttctttagaaactatacaaattaccatttcatcttttaaatgggatttaactgcttttggcttagttgcagagtggtttttggcatatattcttttcactaggtttttctatgtacttggattggctgcaatcatgcaattgtttttcagctattttgcagtacattttattagtaattcttggcttatgtggttaataattaatcttgtacaaatggccccgatttcagctatggttagaatgtacatcttctttgcatcattttattatgtatggaaaagttatgtgcatgttgtagacggttgtaattcatcaacttgtatgatgtgttacaaacgtaatagagcaacaagagtcgaatgtacaactattgttaatggtgttagaaggtccttttatgtctatgctaatggaggtaaaggcttttgcaaactacacaattggaattgtgttaattgtgatacattctgtgctggtagtacatttattagtgatgaagttgcgagagacttgtcactacagtttaaaagaccaataaatcctactgaccagtcttcttacatcgttgatagtgttacagtgaagaatggttccatccatctttactttgataaagctggtcaaaagacttatgaaagacattctctctctcattttgttaacttagacaacctgagagctaataacactaaaggttcattgcctattaatgttatagtttttgatggtaaatcaaaatgtgaagaatcatctgcaaaatcagcgtctgtttactacagtcagcttatgtgtcaacctatactgttactagatcaggcattagtgtctgatgttggtgatagtgcggaagttgcagttaaaatgtttgatgcttacgttaatacgttttcatcaacttttaacgtaccaatggaaaaactcaaaacactagttgcaactgcagaagctgaacttgcaaagaatgtgtccttagacaatgtcttatctacttttatttcagcagctcggcaagggtttgttgattcagatgtagaaactaaagatgttgttgaatgtcttaaattgtcacatcaatctgacatagaagttactggcgatagttgtaataactatatgctcacctataacaaagttgaaaacatgacaccccgtgaccttggtgcttgtattgactgtagtgcgcgtcatattaatgcgcaggtagcaaaaagtcacaacattgctttgatatggaacgttaaagatttcatgtcattgtctgaacaactacgaaaacaaatacgtagtgctgctaaaaagaataacttaccttttaagttgacatgtgcaactactagacaagttgttaatgttgtaacaacaaagatagcacttaagggtggtaaaattgttaataattggttgaagcagttaattaaagttacacttgtgttcctttttgttgctgctattttctatttaataacacctgttcatgtcatgtctaaacatactgacttttcaagtgaaatcataggatacaaggctattgatggtggtgtcactcgtgacatagcatctacagatacttgttttgctaacaaacatgctgattttgacacatggtttagccagcgtggtggtagttatactaatgacaaagcttgcccattgattgctgcagtcataacaagagaagtgggttttgtcgtgcctggtttgcctggcacgatattacgcacaactaatggtgactttttgcatttcttacctagagtttttagtgcagttggtaacatctgttacacaccatcaaaacttatagagtacactgactttgcaacatcagcttgtgttttggctgctgaatgtacaatttttaaagatgcttctggtaagccagtaccatattgttatgataccaatgtactagaaggttctgttgcttatgaaagtttacgccctgacacacgttatgtgctcatggatggctctattattcaatttcctaacacctaccttgaaggttctgttagagtggtaacaacttttgattctgagtactgtaggcacggcacttgtgaaagatcagaagctggtgtttgtgtatctactagtggtagatgggtacttaacaatgattattacagatctttaccaggagttttctgtggtgtagatgctgtaaatttacttactaatatgtttacaccactaattcaacctattggtgctttggacatatcagcatctatagtagctggtggtattgtagctatcgtagtaacatgccttgcctactattttatgaggtttagaagagcttttggtgaatacagtcatgtagttgcctttaatactttactattccttatgtcattcactgtactctgtttaacaccagtttactcattcttacctggtgtttattctgttatttacttgtacttgacattttatcttactaatgatgtttcttttttagcacatattcagtggatggttatgttcacacctttagtacctttctggataacaattgcttatatcatttgtatttccacaaagcatttctattggttctttagtaattacctaaagagacgtgtagtctttaatggtgtttcctttagtacttttgaagaagctgcgctgtgcacctttttgttaaataaagaaatgtatctaaagttgcgtagtgatgtgctattacctcttacgcaatataatagatacttagctctttataataagtacaagtattttagtggagcaatggatacaactagctacagagaagctgcttgttgtcatctcgcaaaggctctcaatgacttcagtaactcaggttctgatgttctttaccaaccaccacaaacctctatcacctcagctgttttgcagagtggttttagaaaaatggcattcccatctggtaaagttgagggttgtatggtacaagtaacttgtggtacaactacacttaacggtctttggcttgatgacgtagtttactgtccaagacatgtgatctgcacctctgaagacatgcttaaccctaattatgaagatttactcattcgtaagtctaatcataatttcttggtacaggctggtaatgttcaactcagggttattggacattctatgcaaaattgtgtacttaagcttaaggttgatacagccaatcctaagacacctaagtataagtttgttcgcattcaaccaggacagactttttcagtgttagcttgttacaatggttcaccatctggtgtttaccaatgtgctatgaggcccaatttcactattaagggttcattccttaatggttcatgtggtagtgttggttttaacatagattatgactgtgtctctttttgttacatgcaccatatggaattaccaactggagttcatgctggcacagacttagaaggtaacttttatggaccttttgttgacaggcaaacagcacaagcagctggtacggacacaactattacagttaatgttttagcttggttgtacgctgctgttataaatggagacaggtggtttctcaatcgatttaccacaactcttaatgactttaaccttgtggctatgaagtacaattatgaacctctaacacaagaccatgttgacatactaggacctctttctgctcaaactggaattgccgttttagatatgtgtgcttcattaaaagaattactgcaaaatggtatgaatggacgtaccatattgggtagtgctttattagaagatgaatttacaccttttgatgttgttagacaatgctcaggtgttactttccaaagtgcagtgaaaagaacaatcaagggtacacaccactggttgttactcacaattttgacttcacttttagttttagtccagagtactcaatggtctttgttcttttttttgtatgaaaatgcctttttaccttttgctatgggtattattgctatgtctgcttttgcaatgatgtttgtcaaacataagcatgcatttctctgtttgtttttgttaccttctcttgccactgtagcttattttaatatggtctatatgcctgctagttgggtgatgcgtattatgacatggttggatatggttgatactagtttgtctggttttaagctaaaagactgtgttatgtatgcatcagctgtagtgttactaatccttatgacagcaagaactgtgtatgatgatggtgctaggagagtgtggacacttatgaatgtcttgacactcgtttataaagtttattatggtaatgctttagatcaagccatttccatgtgggctcttataatctctgttacttctaactactcaggtgtagttacaactgtcatgtttttggccagaggtattgtttttatgtgtgttgagtattgccctattttcttcataactggtaatacacttcagtgtataatgctagtttattgtttcttaggctatttttgtacttgttactttggcctcttttgtttactcaaccgctactttagactgactcttggtgtttatgattacttagtttctacacaggagtttagatatatgaattcacagggactactcccacccaagaatagcatagatgccttcaaactcaacattaaattgttgggtgttggtggcaaaccttgtatcaaagtagccactgtacagtctaaaatgtcagatgtaaagtgcacatcagtagtcttactctcagttttgcaacaactcagagtagaatcatcatctaaattgtgggctcaatgtgtccagttacacaatgacattctcttagctaaagatactactgaagcctttgaaaaaatggtttcactactttctgttttgctttccatgcagggtgctgtagacataaacaagctttgtgaagaaatgctggacaacagggcaaccttacaagctatagcctcagagtttagttcccttccatcatatgcagcttttgctactgctcaagaagcttatgagcaggctgttgctaatggtgattctgaagttgttcttaaaaagttgaagaagtctttgaatgtggctaaatctgaatttgaccgtgatgcagccatgcaacgtaagttggaaaagatggctgatcaagctatgacccaaatgtataaacaggctagatctgaggacaagagggcaaaagttactagtgctatgcagacaatgcttttcactatgcttagaaagttggataatgatgcactcaacaacattatcaacaatgcaagagatggttgtgttcccttgaacataatacctcttacaacagcagccaaactaatggttgtcataccagactataacacatataaaaatacgtgtgatggtacaacatttacttatgcatcagcattgtgggaaatccaacaggttgtagatgcagatagtaaaattgttcaacttagtgaaattagtatggacaattcacctaatttagcatggcctcttattgtaacagctttaagggccaattctgctgtcaaattacagaataatgagcttagtcctgttgcactacgacagatgtcttgtgctgccggtactacacaaactgcttgcactgatgacaatgcgttagcttactacaacacaacaaagggaggtaggtttgtacttgcactgttatccgatttacaggatttgaaatgggctagattccctaagagtgatggaactggtactatctatacagaactggaaccaccttgtaggtttgttacagacacacctaaaggtcctaaagtgaagtatttatactttattaaaggattaaacaacctaaatagaggtatggtacttggtagtttagctgccacagtacgtctacaagctggtaatgcaacagaagtgcctgccaattcaactgtattatctttctgtgcttttgctgtagatgctgctaaagcttacaaagattatctagctagtgggggacaaccaatcactaattgtgttaagatgttgtgtacacacactggtactggtcaggcaataacagttacaccggaagccaatatggatcaagaatcctttggtggtgcatcgtgttgtctgtactgccgttgccacatagatcatccaaatcctaaaggattttgtgacttaaaaggtaagtatgtacaaatacctacaacttgtgctaatgaccctgtgggttttacacttaaaaacacagtctgtaccgtctgcggtatgtggaaaggttatggctgtagttgtgatcaactccgcgaacccatgcttcagtcagctgatgcacaatcgtttttaaacgggtttgcggtgtaagtgcagcccgtcttacaccgtgcggcacaggcactagtactgatgtcgtatacagggcttttgacatctacaatgataaagtagctggttttgctaaattcctaaaaactaattgttgtcgcttccaagaaaaggacgaagatgacaatttaattgattcttactttgtagttaagagacacactttctctaactaccaacatgaagaaacaatttataatttacttaaggattgtccagctgttgctaaacatgacttctttaagtttagaatagacggtgacatggtaccacatatatcacgtcaacgtcttactaaatacacaatggcagacctcgtctatgctttaaggcattttgatgaaggtaattgtgacacattaaaagaaatacttgtcacatacaattgttgtgatgatgattatttcaataaaaaggactggtatgattttgtagaaaacccagatatattacgcgtatacgccaacttaggtgaacgtgtacgccaagctttgttaaaaacagtacaattctgtgatgccatgcgaaatgctggtattgttggtgtactgacattagataatcaagatctcaatggtaactggtatgatttcggtgatttcatacaaaccacgccaggtagtggagttcctgttgtagattcttattattcattgttaatgcctatattaaccttgaccagggctttaactgcagagtcacatgttgacactgacttaacaaagccttacattaagtgggatttgttaaaatatgacttcacggaagagaggttaaaactctttgaccgttattttaaatattgggatcagacataccacccaaattgtgttaactgtttggatgacagatgcattctgcattgtgcaaactttaatgttttattctctacagtgttcccacctacaagttttggaccactagtgagaaaaatatttgttgatggtgttccatttgtagtttcaactggataccacttcagagagctaggtgttgtacataatcaggatgtaaacttacatagctctagacttagttttaaggaattacttgtgtatgctgctgaccctgctatgcacgctgcttctggtaatctattactagataaacgcactacgtgcttttcagtagctgcacttactaacaatgttgcttttcaaactgtcaaacccggtaattttaacaaagacttctatgactttgctgtgtctaagggtttctttaaggaaggaagttctgttgaattaaaacacttcttctttgctcaggatggtaatgctgctatcagcgattatgactactatcgttataatctaccaacaatgtgtgatatcagacaactactatttgtagttgaagttgttgataagtactttgattgttacgatggtggctgtattaatgctaaccaagtcatcgtcaacaacctagacaaatcagctggttttccatttaataaatggggtaaggctagactttattatgattcaatgagttatgaggatcaagatgcacttttcgcatatacaaaacgtaatgtcatccctactataactcaaatgaatcttaagtatgccattagtgcaaagaatagagctcgcaccgtagctggtgtctctatctgtagtactatgaccaatagacagtttcatcaaaaattattgaaatcaatagccgccactagaggagctactgtagtaattggaacaagcaaattctatggtggttggcacaacatgttaaaaactgtttatagtgatgtagaaaaccctcaccttatgggttgggattatcctaaatgtgatagagccatgcctaacatgcttagaattatggcctcacttgttcttgctcgcaaacatacaacgtgttgtagcttgtcacaccgtttctatagattagctaatgagtgtgctcaagtattgagtgaaatggtcatgtgtggcggttcactatatgttaaaccaggtggaacctcatcaggagatgccacaactgcttatgctaatagtgtttttaacatttgtcaagctgtcacggccaatgttaatgcacttttatctactgatggtaacaaaattgccgataagtatgtccgcaatttacaacacagactttatgagtgtctctatagaaatagagatgttgacacagactttgtgaatgagttttacgcatatttgcgtaaacatttctcaatgatgatactctctgacgatgctgttgtgtgtttcaatagcacttatgcatctcaaggtctagtggctagcataaagaactttaagtcagttctttattatcaaaacaatgtttttatgtctgaagcaaaatgttggactgagactgaccttactaaaggacctcatgaattttgctctcaacatacaatgctagttaaacagggtgatgattatgtgtaccttccttacccagatccatcaagaatcctaggggccggctgttttgtagatgatatcgtaaaaacagatggtacacttatgattgaacggttcgtgtctttagctatagatgcttacccacttactaaacatcctaatcaggagtatgctgatgtctttcatttgtacttacaatacataagaaagctacatgatgagttaacaggacacatgttagacatgtattctgttatgcttactaatgataacacttcaaggtattgggaacctgagttttatgaggctatgtacacaccgcatacagtcttacaggctgttggggcttgtgttctttgcaattcacagacttcattaagatgtggtgcttgcatacgtagaccattcttatgttgtaaatgctgttacgaccatgtcatatcaacatcacataaattagtcttgtctgttaatccgtatgtttgcaatgctccaggttgtgatgtcacagatgtgactcaactttacttaggaggtatgagctattattgtaaatcacataaaccacccattagttttccattgtgtgctaatggacaagtttttggtttatataaaaatacatgtgttggtagcgataatgttactgactttaatgcaattgcaacatgtgactggacaaatgctggtgattacattttagctaacacctgtactgaaagactcaagctttttgcagcagaaacgctcaaagctactgaggagacatttaaactgtcttatggtattgctactgtacgtgaagtgctgtctgacagagaattacatctttcatgggaagttggtaaacctagaccaccacttaaccgaaattatgtctttactggttatcgtgtaactaaaaacagtaaagtacaaataggagagtacacctttgaaaaaggtgactatggtgatgctgttgtttaccgaggtacaacaacttacaaattaaatgttggtgattattttgtgctgacatcacatacagtaatgccattaagtgcacctacactagtgccacaagagcactatgttagaattactggcttatacccaacactcaatatctcagatgagttttctagcaatgttgcaaattatcaaaaggttggtatgcaaaagtattctacactccagggaccacctggtactggtaagagtcattttgctattggcctagctctctactacccttctgctcgcatagtgtatacagcttgctctcatgccgctgttgatgcactatgtgagaaggcattaaaatatttgcctatagataaatgtagtagaattatacctgcacgtgctcgtgtagagtgttttgataaattcaaagtgaattcaacattagaacagtatgtcttttgtactgtaaatgcattgcctgagacgacagcagatatagttgtctttgatgaaatttcaatggccacaaattatgatttgagtgttgtcaatgccagattacgtgctaagcactatgtgtacattggcgaccctgctcaattacctgcaccacgcacattgctaactaagggcacactagaaccagaatatttcaattcagtgtgtagacttatgaaaactataggtccagacatgttcctcggaacttgtcggcgttgtcctgctgaaattgttgacactgtgagtgctttggtttatgataataagcttaaagcacataaagacaaatcagctcaatgctttaaaatgttttataagggtgttatcacgcatgatgtttcatctgcaattaacaggccacaaataggcgtggtaagagaattccttacacgtaaccctgcttggagaaaagctgtctttatttcaccttataattcacagaatgctgtagcctcaaagattttgggactaccaactcaaactgttgattcatcacagggctcagaatatgactatgtcatattcactcaaaccactgaaacagctcactcttgtaatgtaaacagatttaatgttgctattaccagagcaaaagtaggcatactttgcataatgtctgatagagacctttatgacaagttgcaatttacaagtcttgaaattccacgtaggaatgtggcaactttacaagctgaaaatgtaacaggactctttaaagattgtagtaaggtaatcactgggttacatcctacacaggcacctacacacctcagtgttgacactaaattcaaaactgaaggtttatgtgttgacatacctggcatacctaaggacatgacctatagaagactcatctctatgatgggttttaaaatgaattatcaagttaatggttaccctaacatgtttatcacccgcgaagaagctataagacatgtacgtgcatggattggcttcgatgtcgaggggtgtcatgctactagagaagctgttggtaccaatttacctttacagctaggtttttctacaggtgttaacctagttgctgtacctacaggttatgttgatacacctaataatacagatttttccagagttagtgctaaaccaccgcctggagatcaatttaaacacctcataccacttatgtacaaaggacttccttggaatgtagtgcgtataaagattgtacaaatgttaagtgacacacttaaaaatctctctgacagagtcgtatttgtcttatgggcacatggctttgagttgacatctatgaagtattttgtgaaaataggacctgagcgcacctgttgtctatgtgatagacgtgccacatgcttttccactgcttcagacacttatgcctgttggcatcattctattggatttgattacgtctataatccgtttatgattgatgttcaacaatggggttttacaggtaacctacaaagcaaccatgatctgtattgtcaagtccatggtaatgcacatgtagctagttgtgatgcaatcatgactaggtgtctagctgtccacgagtgctttgttaagcgtgttgactggactattgaatatcctataattggtgatgaactgaagattaatgcggcttgtagaaaggttcaacacatggttgttaaagctgcattattagcagacaaattcccagttcttcacgacattggtaaccctaaagctattaagtgtgtacctcaagctgatgtagaatggaagttctatgatgcacagccttgtagtgacaaagcttataaaatagaagaattattctattcttatgccacacattctgacaaattcacagatggtgtatgcctattttggaattgcaatgtcgatagatatcctgctaattccattgtttgtagatttgacactagagtgctatctaaccttaacttgcctggttgtgatggtggcagtttgtatgtaaataaacatgcattccacacaccagcttttgataaaagtgcttttgttaatttaaaacaattaccatttttctattactctgacagtccatgtgagtctcatggaaaacaagtagtgtcagatatagattatgtaccactaaagtctgctacgtgtataacacgttgcaatttaggtggtgctgtctgtagacatcatgctaatgagtacagattgtatctcgatgcttataacatgatgatctcagctggctttagcttgtgggtttacaaacaatttgatacttataacctctggaacacttttacaagacttcagagtttagaaaatgtggcttttaatgttgtaaataagggacactttgatggacaacagggtgaagtaccagtttctatcattaataacactgtttacacaaaagttgatggtgttgatgtagaattgtttgaaaataaaacaacattacctgttaatgtagcatttgagctttgggctaagcgcaacattaaaccagtaccagaggtgaaaatactcaataatttgggtgtggacattgctgctaatactgtgatctgggactacaaaagagatgctccagcacatatatctactattggtgtttgttctatgactgacatagccaagaaaccaactgaaacgatttgtgcaccactcactgtcttttttgatggtagagttgatggtcaagtagacttatttagaaatgcccgtaatggtgttcttattacagaaggtagtgttaaaggtttacaaccatctgtgggtcccaaacaagctagtcttaatggagtcacattaattggagaagccgtaaaaacacagttcaattattataagaaagttgatggtgttgtccaacaattacctgaaacttactttactcagagtagaaatttacaagaatttaaacccaggagtcaaatggaaattgatttcttagaattagctatggatgaattcattgaacggtataaattagaaggctatgccttcgaacatatcgtttatggagattttagtcatagtcagttaggtggtttacatctactgattggactagctaaacgttttaaggaatcaccttttgaattagaagattttattcctatggacagtacagttaaaaactatttcataacagatgcgcaaacaggttcatctaagtgtgtgtgttctgttattgatttattacttgatgattttgttgaaataataaaatcccaagatttatctgtagtttctaaggttgtcaaagtgactattgactatacagaaatttcatttatgctttggtgtaaagatggccatgtagaaacattttacccaaaattacaatctagtcaagcgtggcaaccgggtgttgctatgcctaatctttacaaaatgcaaagaatgctattagaaaagtgtgaccttcaaaattatggtgatagtgcaacattacctaaaggcataatgatgaatgtcgcaaaatatactcaactgtgtcaatatttaaacacattaacattagctgtaccctataatatgagagttatacattttggtgctggttctgataaaggagttgcaccaggtacagctgttttaagacagtggttgcctacgggtacgctgcttgtcgattcagatcttaatgactttgtctctgatgcagattcaactttgattggtgattgtgcaactgtacatacagctaataaatgggatctcattattagtgatatgtacgaccctaagactaaaaatgttacaaaagaaaatgactctaaagagggttttttcacttacatttgtgggtttatacaacaaaagctagctcttggaggttccgtggctataaagataacagaacattcttggaatgctgatctttataagctcatgggacacttcgcatggtggacagcctttgttactaatgtgaatgcgtcatcatctgaagcatttttaattggatgtaattatcttggcaaaccacgcgaacaaatagatggttatgtcatgcatgcaaattacatattttggaggaatacaaatccaattcagttgtcttcctattctttatttgacatgagtaaatttccccttaaattaaggggtactgctgttatgtctttaaaagaaggtcaaatcaatgatatgattttatctcttcttagtaaaggtagacttataattagagaaaacaacagagttgttatttctagtgatgttcttgttaacaactaaacgaacaatgtttgtttttcttgttttattgccactagtctctagtcagtgtgttaatcttacaaccagaactcaattaccccctgcatacactaattctttcacacgtggtgtttattaccctgacaaagttttcagatcctcagttttacattcaactcaggacttgttcttacctttcttttccaatgttacttggttccatgctatacatgtctctgggaccaatggtactaagaggtttgataaccctgtcctaccatttaatgatggtgtttattttgcttccactgagaagtctaacataataagaggctggatttttggtactactttagattcgaagacccagtccctacttattgttaataacgctactaatgttgttattaaagtctgtgaatttcaattttgtaatgatccatttttgggtgtttattaccacaaaaacaacaaaagttggatggaaagtgagttcagagtttattctagtgcgaataattgcacttttgaatatgtctctcagccttttcttatggaccttgaaggaaaacagggtaatttcaaaaatcttagggaatttgtgtttaagaatattgatggttattttaaaatatattctaagcacacgcctattaatttagtgcgtgatctccctcagggtttttcggctttagaaccattggtagatttgccaataggtattaacatcactaggtttcaaactttacttgctttacatagaagttatttgactcctggtgattcttcttcaggttggacagctggtgctgcagcttattatgtgggttatcttcaacctaggacttttctattaaaatataatgaaaatggaaccattacagatgctgtagactgtgcacttgaccctctctcagaaacaaagtgtacgttgaaatccttcactgtagaaaaaggaatctatcaaacttctaactttagagtccaaccaacagaatctattgttagatttcctaatattacaaacttgtgcccttttggtgaagtttttaacgccaccagatttgcatctgtttatgcttggaacaggaagagaatcagcaactgtgttgctgattattctgtcctatataattccgcatcattttccacttttaagtgttatggagtgtctcctactaaattaaatgatctctgctttactaatgtctatgcagattcatttgtaattagaggtgatgaagtcagacaaatcgctccagggcaaactggaaagattgctgattataattataaattaccagatgattttacaggctgcgttatagcttggaattctaacaatcttgattctaaggttggtggtaattataattacctgtatagattgtttaggaagtctaatctcaaaccttttgagagagatatttcaactgaaatctatcaggccggtagcacaccttgtaatggtgttgaaggttttaattgttactttcctttacaatcatatggtttccaacccactaatggtgttggttaccaaccatacagagtagtagtactttcttttgaacttctacatgcaccagcaactgtttgtggacctaaaaagtctactaatttggttaaaaacaaatgtgtcaatttcaacttcaatggtttaacaggcacaggtgttcttactgagtctaacaaaaagtttctgcctttccaacaatttggcagagacattgctgacactactgatgctgtccgtgatccacagacacttgagattcttgacattacaccatgttcttttggtggtgtcagtgttataacaccaggaacaaatacttctaaccaggttgctgttctttatcaggatgttaactgcacagaagtccctgttgctattcatgcagatcaacttactcctacttggcgtgtttattctacaggttctaatgtttttcaaacacgtgcaggctgtttaataggggctgaacatgtcaacaactcatatgagtgtgacatacccattggtgcaggtatatgcgctagttatcagactcagactaattctcctcggcgggcacgtagtgtagctagtcaatccatcattgcctacactatgtcacttggtgcagaaaattcagttgcttactctaataactctattgccatacccacaaattttactattagtgttaccacagaaattctaccagtgtctatgaccaagacatcagtagattgtacaatgtacatttgtggtgattcaactgaatgcagcaatcttttgttgcaatatggcagtttttgtacacaattaaaccgtgctttaactggaatagctgttgaacaagacaaaaacacccaagaagtttttgcacaagtcaaacaaatttacaaaacaccaccaattaaagattttggtggttttaatttttcacaaatattaccagatccatcaaaaccaagcaagaggtcatttattgaagatctacttttcaacaaagtgacacttgcagatgctggcttcatcaaacaatatggtgattgccttggtgatattgctgctagagacctcatttgtgcacaaaagtttaacggccttactgttttgccacctttgctcacagatgaaatgattgctcaatacacttctgcactgttagcgggtacaatcacttctggttggacctttggtgcaggtgctgcattacaaataccatttgctatgcaaatggcttataggtttaatggtattggagttacacagaatgttctctatgagaaccaaaaattgattgccaaccaatttaatagtgctattggcaaaattcaagactcactttcttccacagcaagtgcacttggaaaacttcaagatgtggtcaaccaaaatgcacaagctttaaacacgcttgttaaacaacttagctccaattttggtgcaatttcaagtgttttaaatgatatcctttcacgtcttgacaaagttgaggctgaagtgcaaattgataggttgatcacaggcagacttcaaagtttgcagacatatgtgactcaacaattaattagagctgcagaaatcagagcttctgctaatcttgctgctactaaaatgtcagagtgtgtacttggacaatcaaaaagagttgatttttgtggaaagggctatcatcttatgtccttccctcagtcagcacctcatggtgtagtcttcttgcatgtgacttatgtccctgcacaagaaaagaacttcacaactgctcctgccatttgtcatgatggaaaagcacactttcctcgtgaaggtgtctttgtttcaaatggcacacactggtttgtaacacaaaggaatttttatgaaccacaaatcattactacagacaacacatttgtgtctggtaactgtgatgttgtaataggaattgtcaacaacacagtttatgatcctttgcaacctgaattagactcattcaaggaggagttagataaatattttaagaatcatacatcaccagatgttgatttaggtgacatctctggcattaatgcttcagttgtaaacattcaaaaagaaattgaccgcctcaatgaggttgccaagaatttaaatgaatctctcatcgatctccaagaacttggaaagtatgagcagtatataaaatggccatggtacatttggctaggttttatagctggcttgattgccatagtaatggtgacaattatgctttgctgtatgaccagttgctgtagttgtctcaagggctgttgttcttgtggatcctgctgcaaatttgatgaagacgactctgagccagtgctcaaaggagtcaaattacattacacataattcctgatcttctggtctaaacgaactaaatattatattagtttttctgtttggaactttaattttagccatggcagattccaacggtactattaccgttgaagagcttaaaaagctccttgaacaatggaacctagtaataggtttcctattccttacatggatttgtcttctacaatttgcctatgccaacaggaataggtttttgtatataattaagttaattttcctctggctgttatggccagtaactttagcttgttttgtgcttgctgctgtttacagaataaattggatcaccggtggaattgctatcgcaatggcttgtcttgtaggcttgatgtggctcagctacttcattgcttctttcagactgtttgcgcgtacccgttccatgtggtcattcaatccagaaactaacattcttctcaacgtgccactccatggcactattctgaccagaccgcttctagaaagtgaactcgtaatcggagctgtgatccttcgtggacatcttcgtattgctggacaccatctaggacgctgtgacatcaaggacctgcctaaagaaatcactgttgctacatcccgcacgctttcttattacaaattgggagcttcgcagcgtgtagcaggtgactcaggttttgctgcatacagtcgctacaggattggcaactataaattaaacacagaccattccagtagcagtgacaatattgctttgcttgtacagtaagtgacaacagttgttttagatttcatctaaacgaacaaactaaaatgtctgataatggaccccaaaatcagcgaaatgcaccccgcattacgtttggtggaccctcagattcaactggcagtaaccagaatggagaacgcagtggggcgcgatcaaaacaacgtcggccccaaggtttacccaataatactgcgtcttggttcaccgctctcactcaacatggcaaggaagaccttaaattccctcgaggacaaggcgttccaattaacaccaatagcagtccagatgaccaaattggctactaccgaagagctaccagacgaattcgtggtggtgacggtaaaatgaaagatctcagtccaagatggtatttctactacctaggaactgggccagaagctggacttccctatggtgctaacaaagacggcatcatatgggttgcaactgagggagccttgaatacaccaaaagatcacattggcacccgcaatcctgctaacaatgctgcaatcgtgctacaacttcctcaaggaacaacattgccaaaaggcttctacgcagaagggagcagaggcggcagtcaagcctcttctcgttcctcatcacgtagtcgcaacagttcaagaaattcaactccaggcagcagtaggggaacttctcctgctagaatggctggcaatggcggtgatgctgctcttgctttgctgctgcttgacagattgaaccagcttgagagcaaaatgtctggtaaaggccaacaacaacaaggccaaactgtcactaagaaatctgctgctgaggcttctaagaagcctcggcaaaaacgtactgccactaaagcatacaatgtaacacaagctttcggcagacgtggtccagaacaaacccaaggaaattttggggaccaggaactaatcagacaaggaactgattacaaacattggccgcaaattgcacaatttgcccccagcgcttcagcgttcttcggaatgtcgcgcattggcatggaagtcacaccttcgggaacgtggttgacctacacaggtgccatcaaattggatgacaaagatccaaatttcaaagatcaagtcattttgctgaataagcatattgacgcatacaaaacattcccaccaacagagcctaaaaaggacaaaaagaagaaggctgatgaaactcaagccttaccgcagagacagaagaaacagcaaactgtgactcttcttcctgctgcagatttggatgatttctccaaacaattgcaacaatccatgagcagtgctgactcaactcaggcctaaactcatgcagaccacacaaggcagatgggctatataaacgttttcgcttttccgtttacgatatatagtctactcttgtgcagaatgaattctcgtaactacatagcacaagtagatgtagttaactttaatctcacatagcaatctttaatcagtgtgtaacattagggaggacttgaaagagccaccacattttcaccgaggccacgcggagtacgatcgagtgtacagtgaacaatgctagggagagctgcctatatggaagagccctaatgtgtaaaattaattttagtagtgctatccccatgtgattttaatagcttcttaggagaatgacaaaaaaaaaaaaaaaaaaaaaaaaa

SEQ ID NO: 3 - DNA, 27753 bp, Coronaviridae
  misc_feature 1..27753: note = SARS-CoV-2- nsp1D-[3,E,6,7,8]
  source 1..27753: mol_type = other DNA
attaaaggtttataccttcccaggtaacaaaccaaccaactttcgatctcttgtagatctgttctctaaacgaactttaaaatctgtgtggctgtcactcggctgcatgcttagtgcactcacgcagtataattaataactaattactgtcgttgacaggacacgagtaactcgtctatcttctgcaggctgcttacggtttcgtccgtgttgcagccgatcatcagcacatctaggtttcgtccgggtgtgaccgaaaggtaagatggagagccttgtccctggtttcaacgagaaaacacacgtccaactcagtttgcctgttttacaggttcgcgacgtgctcgtacgtggctttggagactccgtggaggaggtcttatcagaggcacgtcaacatcttaaagatggcacttgtggcttagtagaagttgaaaaaggcgttttgcctcaacttgaacagccctatgtgttcatcaaacgttcggatgctcgaactgcacctcatggtcatgttatggttgagctggtagcagaactcgaaggcattcagtacggtcgtagtggtgagacacttggtgtccttgtccctcatgtgggcgaaataccagtggcttaccgcaaggttcttcttcgtaagaacggtaataaaggagctggtggccatagttacggcgccgatctaaagtcatttgacttaggcgacgagcttggcactgatccttatagtggtgttacccgtgaactcatgcgtgagcttaacggaggggcatacactcgctatgtcgataacaacttctgtggccctgatggctaccctcttgagtgcattaaagaccttctagcacgtgctggtaaagcttcatgcactttgtccgaacaactggactttattgacactaagaggggtgtatactgctgccgtgaacatgagcatgaaattgcttggtacacggaacgttctgaaaagagctatgaattgcagacaccttttgaaattaaattggcaaagaaatttgacaccttcaatggggaatgtccaaattttgtatttcccttaaattccataatcaagactattcaaccaagggttgaaaagaaaaagcttgatggctttatgggtagaattcgatctgtctatccagttgcgtcaccaaatgaatgcaaccaaatgtgcctttcaactctcatgaagtgtgatcattgtggtgaaacttcatggcagacgggcgattttgttaaagccacttgcgaattttgtggcactgagaatttgactaaagaaggtgccactacttgtggttacttaccccaaaatgctgttgttaaaatttattgtccagcatgtcacaattcagaagtaggacctgagcatagtcttgccgaataccataatgaatctggcttgaaaaccattcttcgtaagggtggtcgcactattgcctttggaggctgtgtgttctcttatgttggttgccataacaagtgtgcctattgggttccacgtgctagcgctaacataggttgtaaccatacaggtgttgttggagaaggttccgaaggtcttaatgacaaccttcttgaaatactccaaaaagagaaagtcaacatcaatattgttggtgactttaaacttaatgaagagatcgccattattttggcatctttttctgcttccacaagtgcttttgtggaaactgtgaaaggtttggattataaagcattcaaacaaattgttgaatcctgtggtaattttaaagttacaaaaggaaaagctaaaaaaggtgcctggaatattggtgaacagaaatcaatactgagtcctctttatgcatttgcatcagaggctgctcgtgttgtacgatcaattttctcccgcactcttgaaactgctcaaaattctgtgcgtgttttacagaaggccgctataacaatactagatggaatttcacagtattcactgagactcattgatgctatgatgttcacatctgatttggctactaacaatctagttgtaatggcctacattacaggtggtgttgttcagttgacttcgcagtggctaactaacatctttggcactgtttatgaaaaactcaaacccgtccttgattggcttgaagagaagtttaaggaaggtgtagagtttcttagagacggttgggaaattgttaaatttatctcaacctgtgcttgtgaaattgtcggtggacaaattgtcacctgtgcaaaggaaattaaggagagtgttcagacattctttaagcttgtaaataaatttttggctttgtgtgctgactctatcattattggtggagctaaacttaaagccttgaatttaggtgaaacatttgtcacgcactcaaagggattgtacagaaagtgtgttaaatccagagaagaaactggcctactcatgcctctaaaagccccaaaagaaattatcttcttagagggagaaacacttcccacagaagtgttaacagaggaagttgtcttgaaaactggtgatttacaaccattagaacaacctactagtgaagctgttgaagctccattggttggtacaccagtttgtattaacgggcttatgttgctcgaaatcaaagacacagaaaagtactgtgcccttgcacctaatatgatggtaacaaacaataccttcacactcaaaggcggtgcaccaacaaaggttacttttggtgatgacactgtgatagaagtgcaaggttacaagagtgtgaatatcacttttgaacttgatgaaaggattgataaagtacttaatgagaagtgctctgcctatacagttgaactcggtacagaagtaaatgagttcgcctgtgttgtggcagatgctgtcataaaaactttgcaaccagtatctgaattacttacaccactgggcattgatttagatgagtggagtatggctacatactacttatttgatgagtctggtgagtttaaattggcttcacatatgtattgttctttctaccctccagatgaggatgaagaagaaggtgattgtgaagaagaagagtttgagccatcaactcaatatgagtatggtactgaagatgattaccaaggtaaacctttggaatttggtgccacttctgctgctcttcaacctgaagaagagcaagaagaagattggttagatgatgatagtcaacaaactgttggtcaacaagacggcagtgaggacaatcagacaactactattcaaacaattgttgaggttcaacctcaattagagatggaacttacaccagttgttcagactattgaagtgaatagttttagtggttatttaaaacttactgacaatgtatacattaaaaatgcagacattgtggaagaagctaaaaaggtaaaaccaacagtggttgttaatgcagccaatgtttaccttaaacatggaggaggtgttgcaggagccttaaataaggctactaacaatgccatgcaagttgaatctgatgattacatagctactaatggaccacttaaagtgggtggtagttgtgttttaagcggacacaatcttgctaaacactgtcttcatgttgtcggcccaaatgttaacaaaggtgaagacattcaacttcttaagagtgcttatgaaaattttaatcagcacgaagttctacttgcaccattattatcagctggtatttttggtgctgaccctatacattctttaagagtttgtgtagatactgttcgcacaaatgtctacttagctgtctttgataaaaatctctatgacaaacttgtttcaagctttttggaaatgaagagtgaaaagcaagttgaacaaaagatcgctgagattcctaaagaggaagttaagccatttataactgaaagtaaaccttcagttgaacagagaaaacaagatgataagaaaatcaaagcttgtgttgaagaagttacaacaactctggaagaaactaagttcctcacagaaaacttgttactttatattgacattaatggcaatcttcatccagattctgccactcttgttagtgacattgacatcactttcttaaagaaagatgctccatatatagtgggtgatgttgttcaagagggtgttttaactgctgtggttatacctactaaaaaggctggtggcactactgaaatgctagcgaaagctttgagaaaagtgccaacagacaattatataaccacttacccgggtcagggtttaaatggttacactgtagaggaggcaaagacagtgcttaaaaagtgtaaaagtgccttttacattctaccatctattatctctaatgagaagcaagaaattcttggaactgtttcttggaatttgcgagaaatgcttgcacatgcagaagaaacacgcaaattaatgcctgtctgtgtggaaactaaagccatagtttcaactatacagcgtaaatataagggtattaaaatacaagagggtgtggttgattatggtgctagattttacttttacaccagtaaaacaactgtagcgtcacttatcaacacacttaacgatctaaatgaaactcttgttacaatgccacttggctatgtaacacatggcttaaatttggaagaagctgctcggtatatgagatctctcaaagtgccagctacagtttctgtttcttcacctgatgctgttacagcgtataatggttatcttacttcttcttctaaaacacctgaagaacattttattgaaaccatctcacttgctggttcctataaagattggtcctattctggacaatctacacaactaggtatagaatttcttaagagaggtgataaaagtgtatattacactagtaatcctaccacattccacctagatggtgaagttatcacctttgacaatcttaagacacttctttctttgagagaagtgaggactattaaggtgtttacaacagtagacaacattaacctccacacgcaagttgtggacatgtcaatgacatatggacaacagtttggtccaacttatttggatggagctgatgttactaaaataaaacctcataattcacatgaaggtaaaacattttatgttttacctaatgatgacactctacgtgttgaggcttttgagtactaccacacaactgatcctagttttctgggtaggtacatgtcagcattaaatcacactaaaaagtggaaatacccacaagttaatggtttaacttctattaaatgggcagataacaactgttatcttgccactgcattgttaacactccaacaaatagagttgaagtttaatccacctgctctacaagatgcttattacagagcaagggctggtgaagctgctaacttttgtgcacttatcttagcctactgtaataagacagtaggtgagttaggtgatgttagagaaacaatgagttacttgtttcaacatgccaatttagattcttgcaaaagagtcttgaacgtggtgtgtaaaacttgtggacaacagcagacaacccttaagggtgtagaagctgttatgtacatgggcacactttcttatgaacaatttaagaaaggtgttcagataccttgtacgtgtggtaaacaagctacaaaatatctagtacaacaggagtcaccttttgttatgatgtcagcaccacctgctcagtatgaacttaagcatggtacatttacttgtgctagtgagtacactggtaattaccagtgtggtcactataaacatataacttctaaagaaactttgtattgcatagacggtgctttacttacaaagtcctcagaatacaaaggtcctattacggatgttttctacaaagaaaacagttacacaacaaccataaaaccagttacttataaattggatggtgttgtttgtacagaaattgaccctaagttggacaattattataagaaagacaattcttatttcacagagcaaccaattgatcttgtaccaaaccaaccatatccaaacgcaagcttcgataattttaagtttgtatgtgataatatcaaatttgctgatgatttaaaccagttaactggttataagaaacctgcttcaagagagcttaaagttacatttttccctgacttaaatggtgatgtggtggctattgattataaacactacacaccctcttttaagaaaggagctaaattgttacataaacctattgtttggcatgttaacaatgcaactaataaagccacgtataaaccaaatacctggtgtatacgttgtctttggagcacaaaaccagttgaaacatcaaattcgtttgatgtactgaagtcagaggacgcgcagggaatggataatcttgcctgcgaagatctaaaaccagtctctgaagaagtagtggaaaatcctaccatacagaaagacgttcttgagtgtaatgtgaaaactaccgaagttgtaggagacattatacttaaaccagcaaataatagtttaaaaattacagaagaggttggccacacagatctaatggctgcttatgtagacaattctagtcttactattaagaaacctaatgaattatctagagtattaggtttgaaaacccttgctactcatggtttagctgctgttaatagtgtcccttgggatactatagctaattatgctaagccttttcttaacaaagttgttagtacaactactaacatagttacacggtgtttaaaccgtgtttgtactaattatatgccttatttctttactttattgctacaattgtgtacttttactagaagtacaaattctagaattaaagcatctatgccgactactatagcaaagaatactgttaagagtgtcggtaaattttgtctagaggcttcatttaattatttgaagtcacctaatttttctaaactgataaatattataatttggtttttactattaagtgtttgcctaggttctttaatctactcaaccgctgctttaggtgttttaatgtctaatttaggcatgccttcttactgtactggttacagagaaggctatttgaactctactaatgtcactattgcaacctactgtactggttctataccttgtagtgtttgtcttagtggtttagattctttagacacctatccttctttagaaactatacaaattaccatttcatcttttaaatgggatttaactgcttttggcttagttgcagagtggtttttggcatatattcttttcactaggtttttctatgtacttggattggctgcaatcatgcaattgtttttcagctattttgcagtacattttattagtaattcttggcttatgtggttaataattaatcttgtacaaatggccccgatttcagctatggttagaatgtacatcttctttgcatcattttattatgtatggaaaagttatgtgcatgttgtagacggttgtaattcatcaacttgtatgatgtgttacaaacgtaatagagcaacaagagtcgaatgtacaactattgttaatggtgttagaaggtccttttatgtctatgctaatggaggtaaaggcttttgcaaactacacaattggaattgtgttaattgtgatacattctgtgctggtagtacatttattagtgatgaagttgcgagagacttgtcactacagtttaaaagaccaataaatcctactgaccagtcttcttacatcgttgatagtgttacagtgaagaatggttccatccatctttactttgataaagctggtcaaaagacttatgaaagacattctctctctcattttgttaacttagacaacctgagagctaataacactaaaggttcattgcctattaatgttatagtttttgatggtaaatcaaaatgtgaagaatcatctgcaaaatcagcgtctgtttactacagtcagcttatgtgtcaacctatactgttactagatcaggcattagtgtctgatgttggtgatagtgcggaagttgcagttaaaatgtttgatgcttacgttaatacgttttcatcaacttttaacgtaccaatggaaaaactcaaaacactagttgcaactgcagaagctgaacttgcaaagaatgtgtccttagacaatgtcttatctacttttatttcagcagctcggcaagggtttgttgattcagatgtagaaactaaagatgttgttgaatgtcttaaattgtcacatcaatctgacatagaagttactggcgatagttgtaataactatatgctcacctataacaaagttgaaaacatgacaccccgtgaccttggtgcttgtattgactgtagtgcgcgtcatattaatgcgcaggtagcaaaaagtcacaacattgctttgatatggaacgttaaagatttcatgtcattgtctgaacaactacgaaaacaaatacgtagtgctgctaaaaagaataacttaccttttaagttgacatgtgcaactactagacaagttgttaatgttgtaacaacaaagatagcacttaagggtggtaaaattgttaataattggttgaagcagttaattaaagttacacttgtgttcctttttgttgctgctattttctatttaataacacctgttcatgtcatgtctaaacatactgacttttcaagtgaaatcataggatacaaggctattgatggtggtgtcactcgtgacatagcatctacagatacttgttttgctaacaaacatgctgattttgacacatggtttagccagcgtggtggtagttatactaatgacaaagcttgcccattgattgctgcagtcataacaagagaagtgggttttgtcgtgcctggtttgcctggcacgatattacgcacaactaatggtgactttttgcatttcttacctagagtttttagtgcagttggtaacatctgttacacaccatcaaaacttatagagtacactgactttgcaacatcagcttgtgttttggctgctgaatgtacaatttttaaagatgcttctggtaagccagtaccatattgttatgataccaatgtactagaaggttctgttgcttatgaaagtttacgccctgacacacgttatgtgctcatggatggctctattattcaatttcctaacacctaccttgaaggttctgttagagtggtaacaacttttgattctgagtactgtaggcacggcacttgtgaaagatcagaagctggtgtttgtgtatctactagtggtagatgggtacttaacaatgattattacagatctttaccaggagttttctgtggtgtagatgctgtaaatttacttactaatatgtttacaccactaattcaacctattggtgctttggacatatcagcatctatagtagctggtggtattgtagctatcgtagtaacatgccttgcctactattttatgaggtttagaagagcttttggtgaatacagtcatgtagttgcctttaatactttactattccttatgtcattcactgtactctgtttaacaccagtttactcattcttacctggtgtttattctgttatttacttgtacttgacattttatcttactaatgatgtttcttttttagcacatattcagtggatggttatgttcacacctttagtacctttctggataacaattgcttatatcatttgtatttccacaaagcatttctattggttctttagtaattacctaaagagacgtgtagtctttaatggtgtttcctttagtacttttgaagaagctgcgctgtgcacctttttgttaaataaagaaatgtatctaaagttgcgtagtgatgtgctattacctcttacgcaatataatagatacttagctctttataataagtacaagtattttagtggagcaatggatacaactagctacagagaagctgcttgttgtcatctcgcaaaggctctcaatgacttcagtaactcaggttctgatgttctttaccaaccaccacaaacctctatcacctcagctgttttgcagagtggttttagaaaaatggcattcccatctggtaaagttgagggttgtatggtacaagtaacttgtggtacaactacacttaacggtctttggcttgatgacgtagtttactgtccaagacatgtgatctgcacctctgaagacatgcttaaccctaattatgaagatttactcattcgtaagtctaatcataatttcttggtacaggctggtaatgttcaactcagggttattggacattctatgcaaaattgtgtacttaagcttaaggttgatacagccaatcctaagacacctaagtataagtttgttcgcattcaaccaggacagactttttcagtgttagcttgttacaatggttcaccatctggtgtttaccaatgtgctatgaggcccaatttcactattaagggttcattccttaatggttcatgtggtagtgttggttttaacatagattatgactgtgtctctttttgttacatgcaccatatggaattaccaactggagttcatgctggcacagacttagaaggtaacttttatggaccttttgttgacaggcaaacagcacaagcagctggtacggacacaactattacagttaatgttttagcttggttgtacgctgctgttataaatggagacaggtggtttctcaatcgatttaccacaactcttaatgactttaaccttgtggctatgaagtacaattatgaacctctaacacaagaccatgttgacatactaggacctctttctgctcaaactggaattgccgttttagatatgtgtgcttcattaaaagaattactgcaaaatggtatgaatggacgtaccatattgggtagtgctttattagaagatgaatttacaccttttgatgttgttagacaatgctcaggtgttactttccaaagtgcagtgaaaagaacaatcaagggtacacaccactggttgttactcacaattttgacttcacttttagttttagtccagagtactcaatggtctttgttcttttttttgtatgaaaatgcctttttaccttttgctatgggtattattgctatgtctgcttttgcaatgatgtttgtcaaacataagcatgcatttctctgtttgtttttgttaccttctcttgccactgtagcttattttaatatggtctatatgcctgctagttgggtgatgcgtattatgacatggttggatatggttgatactagtttgtctggttttaagctaaaagactgtgttatgtatgcatcagctgtagtgttactaatccttatgacagcaagaactgtgtatgatgatggtgctaggagagtgtggacacttatgaatgtcttgacactcgtttataaagtttattatggtaatgctttagatcaagccatttccatgtgggctcttataatctctgttacttctaactactcaggtgtagttacaactgtcatgtttttggccagaggtattgtttttatgtgtgttgagtattgccctattttcttcataactggtaatacacttcagtgtataatgctagtttattgtttcttaggctatttttgtacttgttactttggcctcttttgtttactcaaccgctactttagactgactcttggtgtttatgattacttagtttctacacaggagtttagatatatgaattcacagggactactcccacccaagaatagcatagatgccttcaaactcaacattaaattgttgggtgttggtggcaaaccttgtatcaaagtagccactgtacagtctaaaatgtcagatgtaaagtgcacatcagtagtcttactctcagttttgcaacaactcagagtagaatcatcatctaaattgtgggctcaatgtgtccagttacacaatgacattctcttagctaaagatactactgaagcctttgaaaaaatggtttcactactttctgttttgctttccatgcagggtgctgtagacataaacaagctttgtgaagaaatgctggacaacagggcaaccttacaagctatagcctcagagtttagttcccttccatcatatgcagcttttgctactgctcaagaagcttatgagcaggctgttgctaatggtgattctgaagttgttcttaaaaagttgaagaagtctttgaatgtggctaaatctgaatttgaccgtgatgcagccatgcaacgtaagttggaaaagatggctgatcaagctatgacccaaatgtataaacaggctagatctgaggacaagagggcaaaagttactagtgctatgcagacaatgcttttcactatgcttagaaagttggataatgatgcactcaacaacattatcaacaatgcaagagatggttgtgttcccttgaacataatacctcttacaacagcagccaaactaatggttgtcataccagactataacacatataaaaatacgtgtgatggtacaacatttacttatgcatcagcattgtgggaaatccaacaggttgtagatgcagatagtaaaattgttcaacttagtgaaattagtatggacaattcacctaatttagcatggcctcttattgtaacagctttaagggccaattctgctgtcaaattacagaataatgagcttagtcctgttgcactacgacagatgtcttgtgctgccggtactacacaaactgcttgcactgatgacaatgcgttagcttactacaacacaacaaagggaggtaggtttgtacttgcactgttatccgatttacaggatttgaaatgggctagattccctaagagtgatggaactggtactatctatacagaactggaaccaccttgtaggtttgttacagacacacctaaaggtcctaaagtgaagtatttatactttattaaaggattaaacaacctaaatagaggtatggtacttggtagtttagctgccacagtacgtctacaagctggtaatgcaacagaagtgcctgccaattcaactgtattatctttctgtgcttttgctgtagatgctgctaaagcttacaaagattatctagctagtgggggacaaccaatcactaattgtgttaagatgttgtgtacacacactggtactggtcaggcaataacagttacaccggaagccaatatggatcaagaatcctttggtggtgcatcgtgttgtctgtactgccgttgccacatagatcatccaaatcctaaaggattttgtgacttaaaaggtaagtatgtacaaatacctacaacttgtgctaatgaccctgtgggttttacacttaaaaacacagtctgtaccgtctgcggtatgtggaaaggttatggctgtagttgtgatcaactccgcgaacccatgcttcagtcagctgatgcacaatcgtttttaaacgggtttgcggtgtaagtgcagcccgtcttacaccgtgcggcacaggcactagtactgatgtcgtatacagggcttttgacatctacaatgataaagtagctggttttgctaaattcctaaaaactaattgttgtcgcttccaagaaaaggacgaagatgacaatttaattgattcttactttgtagttaagagacacactttctctaactaccaacatgaagaaacaatttataatttacttaaggattgtccagctgttgctaaacatgacttctttaagtttagaatagacggtgacatggtaccacatatatcacgtcaacgtcttactaaatacacaatggcagacctcgtctatgctttaaggcattttgatgaaggtaattgtgacacattaaaagaaatacttgtcacatacaattgttgtgatgatgattatttcaataaaaaggactggtatgattttgtagaaaacccagatatattacgcgtatacgccaacttaggtgaacgtgtacgccaagctttgttaaaaacagtacaattctgtgatgccatgcgaaatgctggtattgttggtgtactgacattagataatcaagatctcaatggtaactggtatgatttcggtgatttcatacaaaccacgccaggtagtggagttcctgttgtagattcttattattcattgttaatgcctatattaaccttgaccagggctttaactgcagagtcacatgttgacactgacttaacaaagccttacattaagtgggatttgttaaaatatgacttcacggaagagaggttaaaactctttgaccgttattttaaatattgggatcagacataccacccaaattgtgttaactgtttggatgacagatgcattctgcattgtgcaaactttaatgttttattctctacagtgttcccacctacaagttttggaccactagtgagaaaaatatttgttgatggtgttccatttgtagtttcaactggataccacttcagagagctaggtgttgtacataatcaggatgtaaacttacatagctctagacttagttttaaggaattacttgtgtatgctgctgaccctgctatgcacgctgcttctggtaatctattactagataaacgcactacgtgcttttcagtagctgcacttactaacaatgttgcttttcaaactgtcaaacccggtaattttaacaaagacttctatgactttgctgtgtctaagggtttctttaaggaaggaagttctgttgaattaaaacacttcttctttgctcaggatggtaatgctgctatcagcgattatgactactatcgttataatctaccaacaatgtgtgatatcagacaactactatttgtagttgaagttgttgataagtactttgattgttacgatggtggctgtattaatgctaaccaagtcatcgtcaacaacctagacaaatcagctggttttccatttaataaatggggtaaggctagactttattatgattcaatgagttatgaggatcaagatgcacttttcgcatatacaaaacgtaatgtcatccctactataactcaaatgaatcttaagtatgccattagtgcaaagaatagagctcgcaccgtagctggtgtctctatctgtagtactatgaccaatagacagtttcatcaaaaattattgaaatcaatagccgccactagaggagctactgtagtaattggaacaagcaaattctatggtggttggcacaacatgttaaaaactgtttatagtgatgtagaaaaccctcaccttatgggttgggattatcctaaatgtgatagagccatgcctaacatgcttagaattatggcctcacttgttcttgctcgcaaacatacaacgtgttgtagcttgtcacaccgtttctatagattagctaatgagtgtgctcaagtattgagtgaaatggtcatgtgtggcggttcactatatgttaaaccaggtggaacctcatcaggagatgccacaactgcttatgctaatagtgtttttaacatttgtcaagctgtcacggccaatgttaatgcacttttatctactgatggtaacaaaattgccgataagtatgtccgcaatttacaacacagactttatgagtgtctctatagaaatagagatgttgacacagactttgtgaatgagttttacgcatatttgcgtaaacatttctcaatgatgatactctctgacgatgctgttgtgtgtttcaatagcacttatgcatctcaaggtctagtggctagcataaagaactttaagtcagttctttattatcaaaacaatgtttttatgtctgaagcaaaatgttggactgagactgaccttactaaaggacctcatgaattttgctctcaacatacaatgctagttaaacagggtgatgattatgtgtaccttccttacccagatccatcaagaatcctaggggccggctgttttgtagatgatatcgtaaaaacagatggtacacttatgattgaacggttcgtgtctttagctatagatgcttacccacttactaaacatcctaatcaggagtatgctgatgtctttcatttgtacttacaatacataagaaagctacatgatgagttaacaggacacatgttagacatgtattctgttatgcttactaatgataacacttcaaggtattgggaacctgagttttatgaggctatgtacacaccgcatacagtcttacaggctgttggggcttgtgttctttgcaattcacagacttcattaagatgtggtgcttgcatacgtagaccattcttatgttgtaaatgctgttacgaccatgtcatatcaacatcacataaattagtcttgtctgttaatccgtatgtttgcaatgctccaggttgtgatgtcacagatgtgactcaactttacttaggaggtatgagctattattgtaaatcacataaaccacccattagttttccattgtgtgctaatggacaagtttttggtttatataaaaatacatgtgttggtagcgataatgttactgactttaatgcaattgcaacatgtgactggacaaatgctggtgattacattttagctaacacctgtactgaaagactcaagctttttgcagcagaaacgctcaaagctactgaggagacatttaaactgtcttatggtattgctactgtacgtgaagtgctgtctgacagagaattacatctttcatgggaagttggtaaacctagaccaccacttaaccgaaattatgtctttactggttatcgtgtaactaaaaacagtaaagtacaaataggagagtacacctttgaaaaaggtgactatggtgatgctgttgtttaccgaggtacaacaacttacaaattaaatgttggtgattattttgtgctgacatcacatacagtaatgccattaagtgcacctacactagtgccacaagagcactatgttagaattactggcttatacccaacactcaatatctcagatgagttttctagcaatgttgcaaattatcaaaaggttggtatgcaaaagtattctacactccagggaccacctggtactggtaagagtcattttgctattggcctagctctctactacccttctgctcgcatagtgtatacagcttgctctcatgccgctgttgatgcactatgtgagaaggcattaaaatatttgcctatagataaatgtagtagaattatacctgcacgtgctcgtgtagagtgttttgataaattcaaagtgaattcaacattagaacagtatgtcttttgtactgtaaatgcattgcctgagacgacagcagatatagttgtctttgatgaaatttcaatggccacaaattatgatttgagtgttgtcaatgccagattacgtgctaagcactatgtgtacattggcgaccctgctcaattacctgcaccacgcacattgctaactaagggcacactagaaccagaatatttcaattcagtgtgtagacttatgaaaactataggtccagacatgttcctcggaacttgtcggcgttgtcctgctgaaattgttgacactgtgagtgctttggtttatgataataagcttaaagcacataaagacaaatcagctcaatgctttaaaatgttttataagggtgttatcacgcatgatgtttcatctgcaattaacaggccacaaataggcgtggtaagagaattccttacacgtaaccctgcttggagaaaagctgtctttatttcaccttataattcacagaatgctgtagcctcaaagattttgggactaccaactcaaactgttgattcatcacagggctcagaatatgactatgtcatattcactcaaaccactgaaacagctcactcttgtaatgtaaacagatttaatgttgctattaccagagcaaaagtaggcatactttgcataatgtctgatagagacctttatgacaagttgcaatttacaagtcttgaaattccacgtaggaatgtggcaactttacaagctgaaaatgtaacaggactctttaaagattgtagtaaggtaatcactgggttacatcctacacaggcacctacacacctcagtgttgacactaaattcaaaactgaaggtttatgtgttgacatacctggcatacctaaggacatgacctatagaagactcatctctatgatgggttttaaaatgaattatcaagttaatggttaccctaacatgtttatcacccgcgaagaagctataagacatgtacgtgcatggattggcttcgatgtcgaggggtgtcatgctactagagaagctgttggtaccaatttacctttacagctaggtttttctacaggtgttaacctagttgctgtacctacaggttatgttgatacacctaataatacagatttttccagagttagtgctaaaccaccgcctggagatcaatttaaacacctcataccacttatgtacaaaggacttccttggaatgtagtgcgtataaagattgtacaaatgttaagtgacacacttaaaaatctctctgacagagtcgtatttgtcttatgggcacatggctttgagttgacatctatgaagtattttgtgaaaataggacctgagcgcacctgttgtctatgtgatagacgtgccacatgcttttccactgcttcagacacttatgcctgttggcatcattctattggatttgattacgtctataatccgtttatgattgatgttcaacaatggggttttacaggtaacctacaaagcaaccatgatctgtattgtcaagtccatggtaatgcacatgtagctagttgtgatgcaatcatgactaggtgtctagctgtccacgagtgctttgttaagcgtgttgactggactattgaatatcctataattggtgatgaactgaagattaatgcggcttgtagaaaggttcaacacatggttgttaaagctgcattattagcagacaaattcccagttcttcacgacattggtaaccctaaagctattaagtgtgtacctcaagctgatgtagaatggaagttctatgatgcacagccttgtagtgacaaagcttataaaatagaagaattattctattcttatgccacacattctgacaaattcacagatggtgtatgcctattttggaattgcaatgtcgatagatatcctgctaattccattgtttgtagatttgacactagagtgctatctaaccttaacttgcctggttgtgatggtggcagtttgtatgtaaataaacatgcattccacacaccagcttttgataaaagtgcttttgttaatttaaaacaattaccatttttctattactctgacagtccatgtgagtctcatggaaaacaagtagtgtcagatatagattatgtaccactaaagtctgctacgtgtataacacgttgcaatttaggtggtgctgtctgtagacatcatgctaatgagtacagattgtatctcgatgcttataacatgatgatctcagctggctttagcttgtgggtttacaaacaatttgatacttataacctctggaacacttttacaagacttcagagtttagaaaatgtggcttttaatgttgtaaataagggacactttgatggacaacagggtgaagtaccagtttctatcattaataacactgtttacacaaaagttgatggtgttgatgtagaattgtttgaaaataaaacaacattacctgttaatgtagcatttgagctttgggctaagcgcaacattaaaccagtaccagaggtgaaaatactcaataatttgggtgtggacattgctgctaatactgtgatctgggactacaaaagagatgctccagcacatatatctactattggtgtttgttctatgactgacatagccaagaaaccaactgaaacgatttgtgcaccactcactgtcttttttgatggtagagttgatggtcaagtagacttatttagaaatgcccgtaatggtgttcttattacagaaggtagtgttaaaggtttacaaccatctgtgggtcccaaacaagctagtcttaatggagtcacattaattggagaagccgtaaaaacacagttcaattattataagaaagttgatggtgttgtccaacaattacctgaaacttactttactcagagtagaaatttacaagaatttaaacccaggagtcaaatggaaattgatttcttagaattagctatggatgaattcattgaacggtataaattagaaggctatgccttcgaacatatcgtttatggagattttagtcatagtcagttaggtggtttacatctactgattggactagctaaacgttttaaggaatcaccttttgaattagaagattttattcctatggacagtacagttaaaaactatttcataacagatgcgcaaacaggttcatctaagtgtgtgtgttctgttattgatttattacttgatgattttgttgaaataataaaatcccaagatttatctgtagtttctaaggttgtcaaagtgactattgactatacagaaatttcatttatgctttggtgtaaagatggccatgtagaaacattttacccaaaattacaatctagtcaagcgtggcaaccgggtgttgctatgcctaatctttacaaaatgcaaagaatgctattagaaaagtgtgaccttcaaaattatggtgatagtgcaacattacctaaaggcataatgatgaatgtcgcaaaatatactcaactgtgtcaatatttaaacacattaacattagctgtaccctataatatgagagttatacattttggtgctggttctgataaaggagttgcaccaggtacagctgttttaagacagtggttgcctacgggtacgctgcttgtcgattcagatcttaatgactttgtctctgatgcagattcaactttgattggtgattgtgcaactgtacatacagctaataaatgggatctcattattagtgatatgtacgaccctaagactaaaaatgttacaaaagaaaatgactctaaagagggttttttcacttacatttgtgggtttatacaacaaaagctagctcttggaggttccgtggctataaagataacagaacattcttggaatgctgatctttataagctcatgggacacttcgcatggtggacagcctttgttactaatgtgaatgcgtcatcatctgaagcatttttaattggatgtaattatcttggcaaaccacgcgaacaaatagatggttatgtcatgcatgcaaattacatattttggaggaatacaaatccaattcagttgtcttcctattctttatttgacatgagtaaatttccccttaaattaaggggtactgctgttatgtctttaaaagaaggtcaaatcaatgatatgattttatctcttcttagtaaaggtagacttataattagagaaaacaacagagttgttatttctagtgatgttcttgttaacaactaaacgaacaatgtttgtttttcttgttttattgccactagtctctagtcagtgtgttaatcttacaaccagaactcaattaccccctgcatacactaattctttcacacgtggtgtttattaccctgacaaagttttcagatcctcagttttacattcaactcaggacttgttcttacctttcttttccaatgttacttggttccatgctatacatgtctctgggaccaatggtactaagaggtttgataaccctgtcctaccatttaatgatggtgtttattttgcttccactgagaagtctaacataataagaggctggatttttggtactactttagattcgaagacccagtccctacttattgttaataacgctactaatgttgttattaaagtctgtgaatttcaattttgtaatgatccatttttgggtgtttattaccacaaaaacaacaaaagttggatggaaagtgagttcagagtttattctagtgcgaataattgcacttttgaatatgtctctcagccttttcttatggaccttgaaggaaaacagggtaatttcaaaaatcttagggaatttgtgtttaagaatattgatggttattttaaaatatattctaagcacacgcctattaatttagtgcgtgatctccctcagggtttttcggctttagaaccattggtagatttgccaataggtattaacatcactaggtttcaaactttacttgctttacatagaagttatttgactcctggtgattcttcttcaggttggacagctggtgctgcagcttattatgtgggttatcttcaacctaggacttttctattaaaatataatgaaaatggaaccattacagatgctgtagactgtgcacttgaccctctctcagaaacaaagtgtacgttgaaatccttcactgtagaaaaaggaatctatcaaacttctaactttagagtccaaccaacagaatctattgttagatttcctaatattacaaacttgtgcccttttggtgaagtttttaacgccaccagatttgcatctgtttatgcttggaacaggaagagaatcagcaactgtgttgctgattattctgtcctatataattccgcatcattttccacttttaagtgttatggagtgtctcctactaaattaaatgatctctgctttactaatgtctatgcagattcatttgtaattagaggtgatgaagtcagacaaatcgctccagggcaaactggaaagattgctgattataattataaattaccagatgattttacaggctgcgttatagcttggaattctaacaatcttgattctaaggttggtggtaattataattacctgtatagattgtttaggaagtctaatctcaaaccttttgagagagatatttcaactgaaatctatcaggccggtagcacaccttgtaatggtgttgaaggttttaattgttactttcctttacaatcatatggtttccaacccactaatggtgttggttaccaaccatacagagtagtagtactttcttttgaacttctacatgcaccagcaactgtttgtggacctaaaaagtctactaatttggttaaaaacaaatgtgtcaatttcaacttcaatggtttaacaggcacaggtgttcttactgagtctaacaaaaagtttctgcctttccaacaatttggcagagacattgctgacactactgatgctgtccgtgatccacagacacttgagattcttgacattacaccatgttcttttggtggtgtcagtgttataacaccaggaacaaatacttctaaccaggttgctgttctttatcaggatgttaactgcacagaagtccctgttgctattcatgcagatcaacttactcctacttggcgtgtttattctacaggttctaatgtttttcaaacacgtgcaggctgtttaataggggctgaacatgtcaacaactcatatgagtgtgacatacccattggtgcaggtatatgcgctagttatcagactcagactaattctcctcggcgggcacgtagtgtagctagtcaatccatcattgcctacactatgtcacttggtgcagaaaattcagttgcttactctaataactctattgccatacccacaaattttactattagtgttaccacagaaattctaccagtgtctatgaccaagacatcagtagattgtacaatgtacatttgtggtgattcaactgaatgcagcaatcttttgttgcaatatggcagtttttgtacacaattaaaccgtgctttaactggaatagctgttgaacaagacaaaaacacccaagaagtttttgcacaagtcaaacaaatttacaaaacaccaccaattaaagattttggtggttttaatttttcacaaatattaccagatccatcaaaaccaagcaagaggtcatttattgaagatctacttttcaacaaagtgacacttgcagatgctggcttcatcaaacaatatggtgattgccttggtgatattgctgctagagacctcatttgtgcacaaaagtttaacggccttactgttttgccacctttgctcacagatgaaatgattgctcaatacacttctgcactgttagcgggtacaatcacttctggttggacctttggtgcaggtgctgcattacaaataccatttgctatgcaaatggcttataggtttaatggtattggagttacacagaatgttctctatgagaaccaaaaattgattgccaaccaatttaatagtgctattggcaaaattcaagactcactttcttccacagcaagtgcacttggaaaacttcaagatgtggtcaaccaaaatgcacaagctttaaacacgcttgttaaacaacttagctccaattttggtgcaatttcaagtgttttaaatgatatcctttcacgtcttgacaaagttgaggctgaagtgcaaattgataggttgatcacaggcagacttcaaagtttgcagacatatgtgactcaacaattaattagagctgcagaaatcagagcttctgctaatcttgctgctactaaaatgtcagagtgtgtacttggacaatcaaaaagagttgatttttgtggaaagggctatcatcttatgtccttccctcagtcagcacctcatggtgtagtcttcttgcatgtgacttatgtccctgcacaagaaaagaacttcacaactgctcctgccatttgtcatgatggaaaagcacactttcctcgtgaaggtgtctttgtttcaaatggcacacactggtttgtaacacaaaggaatttttatgaaccacaaatcattactacagacaacacatttgtgtctggtaactgtgatgttgtaataggaattgtcaacaacacagtttatgatcctttgcaacctgaattagactcattcaaggaggagttagataaatattttaagaatcatacatcaccagatgttgatttaggtgacatctctggcattaatgcttcagttgtaaacattcaaaaagaaattgaccgcctcaatgaggttgccaagaatttaaatgaatctctcatcgatctccaagaacttggaaagtatgagcagtatataaaatggccatggtacatttggctaggttttatagctggcttgattgccatagtaatggtgacaattatgctttgctgtatgaccagttgctgtagttgtctcaagggctgttgttcttgtggatcctgctgcaaatttgatgaagacgactctgagccagtgctcaaaggagtcaaattacattacacataattcctgatcttctggtctaaacgaactaaatattatattagtttttctgtttggaactttaattttagccatggcagattccaacggtactattaccgttgaagagcttaaaaagctccttgaacaatggaacctagtaataggtttcctattccttacatggatttgtcttctacaatttgcctatgccaacaggaataggtttttgtatataattaagttaattttcctctggctgttatggccagtaactttagcttgttttgtgcttgctgctgtttacagaataaattggatcaccggtggaattgctatcgcaatggcttgtcttgtaggcttgatgtggctcagctacttcattgcttctttcagactgtttgcgcgtacccgttccatgtggtcattcaatccagaaactaacattcttctcaacgtgccactccatggcactattctgaccagaccgcttctagaaagtgaactcgtaatcggagctgtgatccttcgtggacatcttcgtattgctggacaccatctaggacgctgtgacatcaaggacctgcctaaagaaatcactgttgctacatcccgcacgctttcttattacaaattgggagcttcgcagcgtgtagcaggtgactcaggttttgctgcatacagtcgctacaggattggcaactataaattaaacacagaccattccagtagcagtgacaatattgctttgcttgtacagtaagtgacaacagttgttttagatttcatctaaacgaacaaactaaaatgtctgataatggaccccaaaatcagcgaaatgcaccccgcattacgtttggtggaccctcagattcaactggcagtaaccagaatggagaacgcagtggggcgcgatcaaaacaacgtcggccccaaggtttacccaataatactgcgtcttggttcaccgctctcactcaacatggcaaggaagaccttaaattccctcgaggacaaggcgttccaattaacaccaatagcagtccagatgaccaaattggctactaccgaagagctaccagacgaattcgtggtggtgacggtaaaatgaaagatctcagtccaagatggtatttctactacctaggaactgggccagaagctggacttccctatggtgctaacaaagacggcatcatatgggttgcaactgagggagccttgaatacaccaaaagatcacattggcacccgcaatcctgctaacaatgctgcaatcgtgctacaacttcctcaaggaacaacattgccaaaaggcttctacgcagaagggagcagaggcggcagtcaagcctcttctcgttcctcatcacgtagtcgcaacagttcaagaaattcaactccaggcagcagtaggggaacttctcctgctagaatggctggcaatggcggtgatgctgctcttgctttgctgctgcttgacagattgaaccagcttgagagcaaaatgtctggtaaaggccaacaacaacaaggccaaactgtcactaagaaatctgctgctgaggcttctaagaagcctcggcaaaaacgtactgccactaaagcatacaatgtaacacaagctttcggcagacgtggtccagaacaaacccaaggaaattttggggaccaggaactaatcagacaaggaactgattacaaacattggccgcaaattgcacaatttgcccccagcgcttcagcgttcttcggaatgtcgcgcattggcatggaagtcacaccttcgggaacgtggttgacctacacaggtgccatcaaattggatgacaaagatccaaatttcaaagatcaagtcattttgctgaataagcatattgacgcatacaaaacattcccaccaacagagcctaaaaaggacaaaaagaagaaggctgatgaaactcaagccttaccgcagagacagaagaaacagcaaactgtgactcttcttcctgctgcagatttggatgatttctccaaacaattgcaacaatccatgagcagtgctgactcaactcaggcctaaactcatgcagaccacacaaggcagatgggctatataaacgttttcgcttttccgtttacgatatatagtctactcttgtgcagaatgaattctcgtaactacatagcacaagtagatgtagttaactttaatctcacatagcaatctttaatcagtgtgtaacattagggaggacttgaaagagccaccacattttcaccgaggccacgcggagtacgatcgagtgtacagtgaacaatgctagggagagctgcctatatggaagagccctaatgtgtaaaattaattttagtagtgctatccccatgtgattttaatagcttcttaggagaatgacaaaaaaaaaaaaaaaaaaaaaaaaa

SEQ ID NO: 4 - DNA, 3822 bp, Coronaviridae
  source 1..3822: mol_type = genomic DNA
  CDS 1..3822: note = Gene S polynucleotide sequence
atgtttgtttttcttgttttattgccactagtctctagtcagtgtgttaatcttacaaccagaactcaattaccccctgcatacactaattctttcacacgtggtgtttattaccctgacaaagttttcagatcctcagttttacattcaactcaggacttgttcttacctttcttttccaatgttacttggttccatgctatacatgtctctgggaccaatggtactaagaggtttgataaccctgtcctaccatttaatgatggtgtttattttgcttccactgagaagtctaacataataagaggctggatttttggtactactttagattcgaagacccagtccctacttattgttaataacgctactaatgttgttattaaagtctgtgaatttcaattttgtaatgatccatttttgggtgtttattaccacaaaaacaacaaaagttggatggaaagtgagttcagagtttattctagtgcgaataattgcacttttgaatatgtctctcagccttttcttatggaccttgaaggaaaacagggtaatttcaaaaatcttagggaatttgtgtttaagaatattgatggttattttaaaatatattctaagcacacgcctattaatttagtgcgtgatctccctcagggtttttcggctttagaaccattggtagatttgccaataggtattaacatcactaggtttcaaactttacttgctttacatagaagttatttgactcctggtgattcttcttcaggttggacagctggtgctgcagcttattatgtgggttatcttcaacctaggacttttctattaaaatataatgaaaatggaaccattacagatgctgtagactgtgcacttgaccctctctcagaaacaaagtgtacgttgaaatccttcactgtagaaaaaggaatctatcaaacttctaactttagagtccaaccaacagaatctattgttagatttcctaatattacaaacttgtgcccttttggtgaagtttttaacgccaccagatttgcatctgtttatgcttggaacaggaagagaatcagcaactgtgttgctgattattctgtcctatataattccgcatcattttccacttttaagtgttatggagtgtctcctactaaattaaatgatctctgctttactaatgtctatgcagattcatttgtaattagaggtgatgaagtcagacaaatcgctccagggcaaactggaaagattgctgattataattataaattaccagatgattttacaggctgcgttatagcttggaattctaacaatcttgattctaaggttggtggtaattataattacctgtatagattgtttaggaagtctaatctcaaaccttttgagagagatatttcaactgaaatctatcaggccggtagcacaccttgtaatggtgttgaaggttttaattgttactttcctttacaatcatatggtttccaacccactaatggtgttggttaccaaccatacagagtagtagtactttcttttgaacttctacatgcaccagcaactgtttgtggacctaaaaagtctactaatttggttaaaaacaaatgtgtcaatttcaacttcaatggtttaacaggcacaggtgttcttactgagtctaacaaaaagtttctgcctttccaacaatttggcagagacattgctgacactactgatgctgtccgtgatccacagacacttgagattcttgacattacaccatgttcttttggtggtgtcagtgttataacaccaggaacaaatacttctaaccaggttgctgttctttatcaggatgttaactgcacagaagtccctgttgctattcatgcagatcaacttactcctacttggcgtgtttattctacaggttctaatgtttttcaaacacgtgcaggctgtttaataggggctgaacatgtcaacaactcatatgagtgtgacatacccattggtgcaggtatatgcgctagttatcagactcagactaattctcctcggcgggcacgtagtgtagctagtcaatccatcattgcctacactatgtcacttggtgcagaaaattcagttgcttactctaataactctattgccatacccacaaattttactattagtgttaccacagaaattctaccagtgtctatgaccaagacatcagtagattgtacaatgtacatttgtggtgattcaactgaatgcagcaatcttttgttgcaatatggcagtttttgtacacaattaaaccgtgctttaactggaatagctgttgaacaagacaaaaacacccaagaagtttttgcacaagtcaaacaaatttacaaaacaccaccaattaaagattttggtggttttaatttttcacaaatattaccagatccatcaaaaccaagcaagaggtcatttattgaagatctacttttcaacaaagtgacacttgcagatgctggcttcatcaaacaatatggtgattgccttggtgatattgctgctagagacctcatttgtgcacaaaagtttaacggccttactgttttgccacctttgctcacagatgaaatgattgctcaatacacttctgcactgttagcgggtacaatcacttctggttggacctttggtgcaggtgctgcattacaaataccatttgctatgcaaatggcttataggtttaatggtattggagttacacagaatgttctctatgagaaccaaaaattgattgccaaccaatttaatagtgctattggcaaaattcaagactcactttcttccacagcaagtgcacttggaaaacttcaagatgtggtcaaccaaaatgcacaagctttaaacacgcttgttaaacaacttagctccaattttggtgcaatttcaagtgttttaaatgatatcctttcacgtcttgacaaagttgaggctgaagtgcaaattgataggttgatcacaggcagacttcaaagtttgcagacatatgtgactcaacaattaattagagctgcagaaatcagagcttctgctaatcttgctgctactaaaatgtcagagtgtgtacttggacaatcaaaaagagttgatttttgtggaaagggctatcatcttatgtccttccctcagtcagcacctcatggtgtagtcttcttgcatgtgacttatgtccctgcacaagaaaagaacttcacaactgctcctgccatttgtcatgatggaaaagcacactttcctcgtgaaggtgtctttgtttcaaatggcacacactggtttgtaacacaaaggaatttttatgaaccacaaatcattactacagacaacacatttgtgtctggtaactgtgatgttgtaataggaattgtcaacaacacagtttatgatcctttgcaacctgaattagactcattcaaggaggagttagataaatattttaagaatcatacatcaccagatgttgatttaggtgacatctctggcattaatgcttcagttgtaaacattcaaaaagaaattgaccgcctcaatgaggttgccaagaatttaaatgaatctctcatcgatctccaagaacttggaaagtatgagcagtatataaaatggccatggtacatttggctaggttttatagctggcttgattgccatagtaatggtgacaattatgctttgctgtatgaccagttgctgtagttgtctcaagggctgttgttcttgtggatcctgctgcaaatttgatgaagacgactctgagccagtgctcaaaggagtcaaattacattacacataa

SEQ ID NO: 5 - DNA, 3822 bp, Coronaviridae
  source 1..3822: mol_type = other DNA
  CDS 1..3822: note = codon-optimized gene S polynucleotide sequence
atgttcgtgttcctggtcctgctgccactagtgtcttctcaatgtgtgaacctgaccacaagaacacaactgcctcctgcctataccaacagcttcaccagaggcgtgtactaccccgataaggtgtttagaagcagcgtgctgcacagcacacaggacctgtttctgccatttttctctaatgtgacctggttccacgccatccacgtgagcgggacaaatggcaccaagaggttcgacaaccccgtgctccctttcaacgacggcgtttacttcgccagcaccgagaagtccaacatcatccgcggctggatcttcggcaccaccctggacagcaagacccaaagtctgctgatcgtgaataacgccacaaacgtggttatcaaggtgtgcgagttccagttttgcaacgacccttttctgggcgtgtactaccacaagaacaacaagagctggatggaatctgaattcagagtgtacagcagcgccaacaactgcacattcgagtacgttagccagcctttcctgatggacctggagggcaagcagggaaacttcaagaatctgcgggagttcgtgtttaagaacatcgacggctacttcaaaatctatagcaagcacacccctatcaacctggttagagatctgccccagggcttcagcgctctcgagcctctggtggacctgcctatcggaatcaacattacccggtttcaaaccctgctcgccctccacagaagctacctgacccctggcgacagtagcagcggctggacagccggagcggctgcctactacgtgggctacctgcaacctaggaccttcctgctgaagtacaacgaaaacggcaccatcaccgatgccgtggattgtgctctggaccctctgagcgagacaaagtgcaccctgaagtcctttaccgtggaaaaaggcatctaccagacatccaacttcagggtacagcccaccgaaagcatcgtgcgattccccaacatcacaaacctgtgtcctttcggcgaggtgttcaatgccaccagattcgccagcgtgtacgcctggaaccggaagcggatcagcaattgcgtcgccgattactcagtgctttataacagcgccagctttagcaccttcaagtgctatggcgtgtcccctaccaagctcaatgacctctgcttcaccaacgtgtacgccgacagcttcgtgatcagaggcgatgaggtgagacagatcgcccctggacagaccggcaagatcgccgattacaactacaagctgcctgatgacttcaccggctgcgtgattgcctggaacagcaacaacctggacagcaaggtgggcggcaattacaactacctgtatcggctgttcagaaagagcaacctgaagccattcgagcgggacatcagcactgagatctaccaggccggaagcaccccatgcaacggcgtagaaggcttcaattgctactttccactgcagagctatggttttcagcctaccaatggcgtgggttaccagccttacagagttgtggtgctgagcttcgaactgctgcacgccccagccaccgtctgtggccctaagaaaagcacaaacctagtgaagaacaagtgcgtgaacttcaatttcaacggactgaccggcaccggcgtgctgaccgagagcaacaagaagttcctacctttccaacagttcggcagagacatcgccgacaccacagacgccgtgagagaccctcagaccctggaaatcctggacatcaccccctgttccttcggaggcgtgtctgttatcactcccggcaccaacacgagcaaccaggtggccgtgctgtaccaggatgtcaactgcaccgaggtgcctgtcgccatccacgccgatcagctgacacctacttggcgggtgtattctaccggcagcaacgtgttccagaccagagccggttgcctgattggcgccgaacacgtgaacaacagctatgaatgcgacatccccattggcgctggaatctgcgccagctaccaaacccagactaacagccctcggcgggctcggtctgtggccagccagagcatcatcgcttacaccatgagcctgggcgccgaaaatagcgtagcctacagcaacaattctatcgcgatccccacaaacttcaccatcagcgtcacaacagagatcctgcctgtgtctatgacgaaaacaagcgtggactgcaccatgtacatttgcggcgatagcacagaatgcagcaatctgctgctgcagtacggctctttctgcacccagctgaacagagccctgaccggaattgctgttgagcaggataagaatacccaagaggtgttcgcccaggtgaagcagatctacaagacaccccccatcaaggacttcggcggcttcaacttcagccagatcctgccagacccctccaagccctctaagcggtctttcatcgaggacctgctgttcaacaaggtgacactggctgatgccggcttcatcaaacagtacggcgactgcctgggcgacatcgccgccagagatctgatctgcgcccagaaattcaacggcctgaccgtgcttccacctttgctgacagacgagatgatcgcccagtacaccagcgccctgctggccggcacaatcaccagcggatggacctttggcgccggagccgccctgcaaatcccctttgctatgcagatggcctatagattcaacggaatcggcgtgactcagaatgttctgtatgaaaaccaaaagctgatcgccaatcagtttaactcggccatcggaaagatccaggactctctcagcagcaccgccagtgcactgggcaaactgcaagatgtggtgaaccagaatgcccaagctctgaacaccctggtgaaacagctgtcttccaacttcggcgccatcagctcagtgctgaacgatatcctgtcacgtctggacaaagtggaagccgaggtgcagatcgacagactgatcacagggagactgcagagcctgcagacctacgtgacacagcaactgatcagagccgccgagatccgggcctctgctaatctggccgctaccaaaatgtccgagtgtgtgctgggccagagcaagagagtggacttctgtggaaagggctaccatctgatgtcctttcctcagagcgcccctcacggcgtggtgttccttcatgtgacatacgtgcccgcccaggagaagaactttaccaccgcccctgccatctgccacgatggcaaagcccacttccctagagagggcgtgtttgtgtccaacggcacccactggttcgtgacacagcggaacttctacgaacctcagatcatcacaaccgacaacaccttcgtctccggcaactgtgatgtggtgatcggcatcgtgaacaacacggtgtacgaccctctgcagcccgagctggattctttcaaggaagagctggacaagtacttcaagaaccatacaagccctgatgtggacctgggcgacattagcggcatcaacgcaagtgtggtgaatatccagaaggaaatcgacagactgaacgaggtggccaagaacctgaacgaaagcctgatcgatctgcaggagctgggcaagtacgagcagtacatcaagtggccatggtacatctggctgggattcatcgccggcctgatcgctatcgtgatggtcactatcatgctgtgctgcatgaccagctgctgctcatgtctgaaaggctgttgcagttgtggatcctgctgcaaatttgatgaagacgactctgagccagtgctcaaaggagtcaaattacattacacataa

SEQ ID NO: 6 - protein, 275 aa, Coronaviridae
  REGION 1..275: note = MISC_FEATURE - protein 3a amino acid sequence GenBank YP_009724391
MDLFMRIFTIGTVTLKQGEIKDATPSDFVRATATIPIQASLPFGWLIVGVALLAVFQSASKIITLKKRWQLALSKGVHFVCNLLLLFVTVYSHLLLVAAGLEAPFLYLYALVYFLQSINFVRIIMRLWLCWKCRSKNPLLYDANYFLCWHTNCYDYCIPYNSVTSSIVITSGDGTTSPISEHDYQIGGYTEKWESGVKDCVVLHSYFTSDYYQLYSTQLSTDTGVEHVTFFIYNKIVDEPEEHVQIHTIDGSSGVVNPVMEPIYDEPTTTTSVPL

SEQ ID NO: 7 - protein, 75 aa, Coronaviridae
  REGION 1..75: note = MISC_FEATURE - protein E amino acid sequence GenBank YP_009724392
MYSFVSEETGTLIVNSVLLFLAFVVFLLVTLAILTALRLCAYCCNIVNVSLVKPSFYVYSRVKNLNSSRVPDLLV

SEQ ID NO: 8 - DNA, 38125 bp, Coronaviridae
  misc_feature 1..38125: note = pBAC-SARS-CoV-2-FL: pBAC sequence (nucleotides 1 to 7889), SARS-CoV-2 genome sequence (nucleotides 7890 to 37784) and pBAC sequence (nucleotides 37785 to 38125).
  source 1..38125: mol_type = other DNA
agcttgagtattctatagtgtcacctaaatagcttggcgtaatcatggtcatagctgtttcctgtgtgaaattgttatccgctcacaattccacacaacatacgagccggaagcataaagtgtaaagcctggggtgcctaatgagtgagctaactcacattaattgcgttgcgctcactgcccgctttccagtcgggaaacctgtcgtgccagctgcattaatgaatcggccaacgcgaaccccttgcggccgcccgggccgtcgaccaattctcatgtttgacagcttatcatcgaatttctgccattcatccgcttattatcacttattcaggcgtagcaaccaggcgtttaagggcaccaataactgccttaaaaaaattacgccccgccctgccactcatcgcagtactgttgtaattcattaagcattctgccgacatggaagccatcacaaacggcatgatgaacctgaatcgccagcggcatcagcaccttgtcgccttgcgtataatatttgcccatggtgaaaacgggggcgaagaagttgtccatattggccacgtttaaatcaaaactggtgaaactcacccagggattggctgagacgaaaaacatattctcaataaaccctttagggaaataggccaggttttcaccgtaacacgccacatcttgcgaatatatgtgtagaaactgccggaaatcgtcgtggtattcactccagagcgatgaaaacgtttcagtttgctcatggaaaacggtgtaacaagggtgaacactatcccatatcaccagctcaccgtctttcattgccatacggaattccggatgagcattcatcaggcgggcaagaatgtgaataaaggccggataaaacttgtgcttatttttctttacggtctttaaaaaggccgtaatatccagctgaacggtctggttataggtacattgagcaactgactgaaatgcctcaaaatgttctttacgatgccattgggatatatcaacggtggtatatccagtgatttttttctccattttagcttccttagctcctgaaaatctcgataactcaaaaaatacgcccggtagtgatcttatttcattatggtgaaagttggaacctcttacgtgccgatcaacgtctcattttcgccaaaagttggcccagggcttcccggtatcaacagggacaccaggatttatttattctgcgaagtgatcttccgtcacaggtatttattcgcgataagctcatggagcggcgtaaccgtcgcacaggaaggacagagaaagcgcggatctgggaagtgacggacagaacggtcaggacctggattggggaggcggttgccgccgctgctgctgacggtgtgacgttctctgttccggtcacaccacatacgttccgccattcctatgcgatgcacatgctgtatgccggtataccgctgaaagttctgcaaagcctgatgggacataagtccatcagttcaacggaagtctacacgaaggtttttgcgctggatgtggctgcccggcaccgggtgcagtttgcgatgccggagtctgatgcggttgcgatgctgaaacaattatcctgagaataaatgccttggcctttatatggaaatgtggaactgagtggatatgctgtttttgtctgttaaacagagaagctggctgttatccactgagaagcgaacgaaacagtcgggaaaatctcccattatcgtagagatccgcattattaatctcaggagcctgtgtagcgtttataggaagtagtgttctgtcatgatgcctgcaagcggtaacgaaaacgatttgaatatgccttcaggaacaatagaaatcttcgtgcggtgttacgttgaagtggagcggattatgtcagcaatggacagaacaacctaatgaacacagaaccatgatgtggtctgtccttttacagccagtagtgctcgccgcagtcgagcgacagggcgaagccctcgagtgagcgaggaagcaccagggaacagcacttatatattctgcttacacacgatgcctgaaaaaacttcccttggggttatccacttatccacggggatatttttataattattttttttatagtttttagatcttcttttttagagcgccttgtagacctttatccatgctggttctagagaaggtgttgtgacaaattgccctttcagtgtgacaaatcaccctcaaatgacagtcctgtctgtgacaaattgcccttaaccctgtgacaaattgccctcagaagaagctgttttttcacaaagttatccctgcttattgactcttttttatttagtgtgacaatctaaaaacttgtcacacttcacatggatctgtcatggcggaaacagcggttatcaatcacaagaaacgtaaaaatagcccgcgaatcgtccagtcaaacgacctcactgaggcggcatatagtctctcccgggatcaaaaacgtatgctgtatctgttcgttgaccagatcagaaaatctgatggcaccctacaggaacatgacggtatctgcgagatccatgttgctaaatatgctgaaatattcggattgacctctgcggaagccagtaaggatatacggcaggcattgaagagtttcgcggggaaggaagtggttttttatcgccctgaagaggatgccggcgatgaaaaaggctatgaatcttttccttggtttatcaaacgtgcgcacagtccatccagagggctttacagtgtacatatcaacccatatctcattcccttctttatcgggttacagaaccggtttacgcagtttcggcttagtgaaacaaaagaaatcaccaatccgtatgccatgcgtttatacgaatccctgtgtcagtatcgtaagccggatggctcaggcatcgtctctctgaaaatcgactggatcatagagcgttaccagctgcctcaaagttaccagcgtatgcctgacttccgccgccgcttcctgcaggtctgtgttaatgagatcaacagcagaactccaatgcgcctctcatacattgagaaaaagaaaggccgccagacgactcatatcgtattttccttccgcgatatcacttccatgacgacaggatagtctgagggttatctgtcacagatttgagggtggttcgtcacatttgttctgacctactgagggtaatttgtcacagttttgctgtttccttcagcctgcatggattttctcatactttttgaactgtaatttttaaggaagccaaatttgagggcagtttgtcacagttgatttccttctctttcccttcgtcatgtgacctgatatcgggggttagttcgtcatcattgatgagggttgattatcacagtttattactctgaattggctatccgcgtgtgtacctctacctggagtttttcccacggtggatatttcttcttgcgctgagcgtaagagctatctgacagaacagttcttctttgcttcctcgccagttcgctcgctatgctcggttacacggctgcggcgagcgctagtgataataagtgactgaggtatgtgctcttcttatctccttttgtagtgttgctcttattttaaacaactttgcggttttttgatgactttgcgattttgttgttgctttgcagtaaattgcaagatttaataaaaaaacgcaaagcaatgattaaaggatgttcagaatgaaactcatggaaacacttaaccagtgcataaacgctggtcatgaaatgacgaaggctatcgccattgcacagtttaatgatgacagcccggaagcgaggaaaataacccggcgctggagaataggtgaagcagcggatttagttggggtttcttctcaggctatcagagatgccgagaaagcagggcgactaccgcacccggatatggaaattcgaggacgggttgagcaacgtgttggttatacaattgaacaaattaatcatatgcgtgatgtgtttggtacgcgattgcgacgtgctgaagacgtatttccaccggtgatcggggttgctgcccataaaggtggcgtttacaaaacctcagtttctgttcatcttgctcaggatctggctctgaaggggctacgtgttttgctcgtggaaggtaacgacccccagggaacagcctcaatgtatcacggatgggtaccagatcttcatattcatgcagaagacactctcctgcctttctatcttggggaaaaggacgatgtcacttatgcaataaagcccacttgctggccggggcttgacattattccttcctgtctggctctgcaccgtattgaaactgagttaatgggcaaatttgatgaaggtaaactgcccaccgatccacacctgatgctccgactggccattgaaactgttgctcatgactatgatgtcatagttattgacagcgcgcctaacctgggtatcggcacgattaatgtcgtatgtgctgctgatgtgctgattgttcccacgcctgctgagttgtttgactacacctccgcactgcagtttttcgatatgcttcgtgatctgctcaagaacgttgatcttaaagggttcgagcctgatgtacgtattttgcttaccaaatacagcaatagtaatggctctcagtccccgtggatggaggagcaaattcgggatgcctggggaagcatggttctaaaaaatgttgtacgtgaaacggatgaagttggtaaaggtcagatccggatgagaactgtttttgaacaggccattgatcaacgctcttcaactggtgcctggagaaatgctctttctatttgggaacctgtctgcaatgaaattttcgatcgtctgattaaaccacgctgggagattagataatgaagcgtgcgcctgttattccaaaacatacgctcaatactcaaccggttgaagatacttcgttatcgacaccagctgccccgatggtggattcgttaattgcgcgcgtaggagtaatggctcgcggtaatgccattactttgcctgtatgtggtcgggatgtgaagtttactcttgaagtgctccggggtgatagtgttgagaagacctctcgggtatggtcaggtaatgaacgtgaccaggagctgcttactgaggacgcactggatgatctcatcccttcttttctactgactggtcaacagacaccggcgttcggtcgaagagtatctggtgtcatagaaattgccgatgggagtcgccgtcgtaaagctgctgcacttaccgaaagtgattatcgtgttctggttggcgagctggatgatgagcagatggctgcattatccagattgggtaacgattatcgcccaacaagtgcttatgaacgtggtcagcgttatgcaagccgattgcagaatgaatttgctggaaatatttctgcgctggctgatgcggaaaatatttcacgtaagattattacccgctgtatcaacaccgccaaattgcctaaatcagttgttgctcttttttctcaccccggtgaactatctgcccggtcaggtgatgcacttcaaaaagcctttacagataaagaggaattacttaagcagcaggcatctaaccttcatgagcagaaaaaagctggggtgatatttgaagctgaagaagttatcactcttttaacttctgtgcttaaaacgtcatctgcatcaagaactagtttaagctcacgacatcagtttgctcctggagcgacagtattgtataagggcgataaaatggtgcttaacctggacaggtctcgtgttccaactgagtgtatagagaaaattgaggccattcttaaggaacttgaaaagccagcaccctgatgcgaccacgttttagtctacgtttatctgtctttacttaatgtcctttgttacaggccagaaagcataactggcctgaatattctctctgggcccactgttccacttgtatcgtcggtctgataatcagactgggaccacggtcccactcgtatcgtcggtctgattattagtctgggaccacggtcccactcgtatcgtcggtctgattattagtctgggaccacggtcccactcgtatcgtcggtctgataatcagactgggaccacggtcccactcgtatcgtcggtctgattattagtctgggaccatggtcccactcgtatcgtcggtctgattattagtctgggaccacggtcccactcgtatcgtcggtctgattattagtctggaaccacggtcccactcgtatcgtcggtctgattattagtctgggaccacggtcccactcgtatcgtcggtctgattattagtctgggaccacgatcccactcgtgttgtcggtctgattatcggtctgggaccacggtcccacttgtattgtcgatcagactatcagcgtgagactacgattccatcaatgcctgtcaagggcaagtattgacatgtcgtcgtaacctgtagaacggagtaacctcggtgtgcggttgtatgcctgctgtggattgctgctgtgtcctgcttatccacaacattttgcgcacggttatgtggacaaaatacctggttacccaggccgtgccggcacgttaaccgggctgcatccgatgcaagtgtgtcgctgtcgacgagctcgcgagctcggacatgaggttgccccgtattcagtgtcgctgatttgtattgtctgaagttgtttttacgttaagttgatgcagatcaattaatacgatacctgcgtcataattgattatttgacgtggtttgatggcctccacgcacgttgtgatatgtagatgataatcattatcactttacgggtcctttccggtgatccgacaggttacggggcggcgacctcgcgggttttcgctatttatgaaaattttccggtttaaggcgtttccgttcttcttcgtcataacttaatgtttttatttaaaataccctctgaaaagaaaggaaacgacaggtgctgaaagcgagctttttggcctctgtcgtttcctttctctgtttttgtccgtggaatgaacaatggaagtccgagctcatcgctaataacttcgtatagcatacattatacgaagttatattcgatgcggccgcaaggggttcgcgtcagcgggtgttggcgggtgtcggggctggcttaactatgcggcatcagagcagattgtactgagagtgcaccatatgcggtgtgaaataccgcacagatgcgtaaggagaaaataccgcatcaggcgcctatggcgcgcctaagttgacattgattattgactagttattaatagtaatcaattacggggtcattagttcatagcccatatatggagttccgcgttacataacttacggtaaatggcccgcctggctgaccgcccaacgacccccgcccattgacgtcaataatgacgtatgttcccatagtaacgccaatagggactttccattgacgtcaatgggtggagtatttacggtaaactgcccacttggcagtacatcaagtgtatcatatgccaagtacgccccctattgacgtcaatgacggtaaatggcccgcctggcattatgcccagtacatgaccttatgggactttcctacttggcagtacatctacgtattagtcatcgctattaccatggtgatgcggttttggcagtacatcaatgggcgtggatagcggtttgactcacggggatttccaagtctccaccccattgacgtcaatgggagtttgttttggcaccaaaatcaacgggactttccaaaatgtcgtaacaactccgccccattgacgcaaatgggcggtaggcgtgtacggtgggaggtctatataagcagagctcgtttagtgaaccgtattaaaggtttataccttcccaggtaacaaaccaaccaactttcgatctcttgtagatctgttctctaaacgaactttaaaatctgtgtggctgtcactcggctgcatgcttagtgcactcacgcagtataattaataactaattactgtcgttgacaggacacgagtaactcgtctatcttctgcaggctgcttacggtttcgtccgtgttgcagccgatcatcagcacatctaggtttcgtccgggtgtgaccgaaaggtaagatggagagccttgtccctggtttcaacgagaaaacacacgtccaactcagtttgcctgttttacaggttcgcgacgtgctcgtacgtggctttggagactccgtggaggaggtcttatcagaggcacgtcaacatcttaaagatggcacttgtggcttagtagaagttgaaaaaggcgttttgcctcaacttgaacagccctatgtgttcatcaaacgttcggatgctcgaactgcacctcatggtcatgttatggttgagctggtagcagaactcgaaggcattcagtacggtcgtagtggtgagacacttggtgtccttgtccctcatgtgggcgaaataccagtggcttaccgcaaggttcttcttcgtaagaacggtaataaaggagctggtggccatagttacggcgccgatctaaagtcatttgacttaggcgacgagcttggcactgatccttatgaagattttcaagaaaactggaacactaaacatagcagtggtgttacccgtgaactcatgcgtgagcttaacggaggggcatacactcgctatgtcgataacaacttctgtggccctgatggctaccctcttgagtgcattaaagaccttctagcacgtgctggtaaagcttcatgcactttgtccgaacaactggactttattgacactaagaggggtgtatactgctgccgtgaacatgagcatgaaattgcttggtacacggaacgttctgaaaagagctatgaattgcagacaccttttgaaattaaattggcaaagaaatttgacaccttcaatggggaatgtccaaattttgtatttcccttaaattccataatcaagactattcaaccaagggttgaaaagaaaaagcttgatggctttatgggtagaattcgatctgtctatccagttgcgtcaccaaatgaatgcaaccaaatgtgcctttcaactctcatgaagtgtgatcattgtggtgaaacttcatggcagacgggcgattttgttaaagccacttgcgaattttgtggcactgagaatttgactaaagaaggtgccactacttgtggttacttaccccaaaatgctgttgttaaaatttattgtccagcatgtcacaattcagaagtaggacctgagcatagtcttgccgaataccataatgaatctggcttgaaaaccattcttcgtaagggtggtcgcactattgcctttggaggctgtgtgttctcttatgttggttgccataacaagtgtgcctattgggttccacgtgctagcgctaacataggttgtaaccatacaggtgttgttggagaaggttccgaaggtcttaatgacaaccttcttgaaatactccaaaaagagaaagtcaacatcaatattgttggtgactttaaacttaatgaagagatcgccattattttggcatctttttctgcttccacaagtgcttttgtggaaactgtgaaaggtttggattataaagcattcaaacaaattgttgaatcctgtggtaattttaaagttacaaaaggaaaagctaaaaaaggtgcctggaatattggtgaacagaaatcaatactgagtcctctttatgcatttgcatcagaggctgctcgtgttgtacgatcaattttctcccgcactcttgaaactgctcaaaattctgtgcgtgttttacagaaggccgctataacaatactagatggaatttcacagtattcactgagactcattgatgctatgatgttcacatctgatttggctactaacaatctagttgtaatggcctacattacaggtggtgttgttcagttgacttcgcagtggctaactaacatctttggcactgtttatgaaaaactcaaacccgtccttgattggcttgaagagaagtttaaggaaggtgtagagtttcttagagacggttgggaaattgttaaatttatctcaacctgtgcttgtgaaattgtcggtggacaaattgtcacctgtgcaaaggaaattaaggagagtgttcagacattctttaagcttgtaaataaatttttggctttgtgtgctgactctatcattattggtggagctaaacttaaagccttgaatttaggtgaaacatttgtcacgcactcaaagggattgtacagaaagtgtgttaaatccagagaagaaactggcctactcatgcctctaaaagccccaaaagaaattatcttcttagagggagaaacacttcccacagaagtgttaacagaggaagttgtcttgaaaactggtgatttacaaccattagaacaacctactagtgaagctgttgaagctccattggttggtacaccagtttgtattaacgggcttatgttgctcgaaatcaaagacacagaaaagtactgtgcccttgcacctaatatgatggtaacaaacaataccttcacactcaaaggcggtgcaccaacaaaggttacttttggtgatgacactgtgatagaagtgcaaggttacaagagtgtgaatatcacttttgaacttgatgaaaggattgataaagtacttaatgagaagtgctctgcctatacagttgaactcggtacagaagtaaatgagttcgcctgtgttgtggcagatgctgtcataaaaactttgcaaccagtatctgaattacttacaccactgggcattgatttagatgagtggagtatggctacatactacttatttgatgagtctggtgagtttaaattggcttcacatatgtattgttctttctaccctccagatgaggatgaagaagaaggtgattgtgaagaagaagagtttgagccatcaactcaatatgagtatggtactgaagatgattaccaaggtaaacctttggaatttggtgccacttctgctgctcttcaacctgaagaagagcaagaagaagattggttagatgatgatagtcaacaaactgttggtcaacaagacggcagtgaggacaatcagacaactactattcaaacaattgttgaggttcaacctcaattagagatggaacttacaccagttgttcagactattgaagtgaatagttttagtggttatttaaaacttactgacaatgtatacattaaaaatgcagacattgtggaagaagctaaaaaggtaaaaccaacagtggttgttaatgcagccaatgtttaccttaaacatggaggaggtgttgcaggagccttaaataaggctactaacaatgccatgcaagttgaatctgatgattacatagctactaatggaccacttaaagtgggtggtagttgtgttttaagcggacacaatcttgctaaacactgtcttcatgttgtcggcccaaatgttaacaaaggtgaagacattcaacttcttaagagtgcttatgaaaattttaatcagcacgaagttctacttgcaccattattatcagctggtatttttggtgctgaccctatacattctttaagagtttgtgtagatactgttcgcacaaatgtctacttagctgtctttgataaaaatctctatgacaaacttgtttcaagctttttggaaatgaagagtgaaaagcaagttgaacaaaagatcgctgagattcctaaagaggaagttaagccatttataactgaaagtaaaccttcagttgaacagagaaaacaagatgataagaaaatcaaagcttgtgttgaagaagttacaacaactctggaagaaactaagttcctcacagaaaacttgttactttatattgacattaatggcaatcttcatccagattctgccactcttgttagtgacattgacatcactttcttaaagaaagatgctccatatatagtgggtgatgttgttcaagagggtgttttaactgctgtggttatacctactaaaaaggctggtggcactactgaaatgctagcgaaagctttgagaaaagtgccaacagacaattatataaccacttacccgggtcagggtttaaatggttacactgtagaggaggcaaagacagtgcttaaaaagtgtaaaagtgccttttacattctaccatctattatctctaatgagaagcaagaaattcttggaactgtttcttggaatttgcgagaaatgcttgcacatgcagaagaaacacgcaaattaatgcctgtctgtgtggaaactaaagccatagtttcaactatacagcgtaaatataagggtattaaaatacaagagggtgtggttgattatggtgctagattttacttttacaccagtaaaacaactgtagcgtcacttatcaacacacttaacgatctaaatgaaactcttgttacaatgccacttggctatgtaacacatggcttaaatttggaagaagctgctcggtatatgagatctctcaaagtgccagctacagtttctgtttcttcacctgatgctgttacagcgtataatggttatcttacttcttcttctaaaacacctgaagaacattttattgaaaccatctcacttgctggttcctataaagattggtcctattctggacaatctacacaactaggtatagaatttcttaagagaggtgataaaagtgtatattacactagtaatcctaccacattccacctagatggtgaagttatcacctttgacaatcttaagacacttctttctttgagagaagtgaggactattaaggtgtttacaacagtagacaacattaacctccacacgcaagttgtggacatgtcaatgacatatggacaacagtttggtccaacttatttggatggagctgatgttactaaaataaaacctcataattcacatgaaggtaaaacattttatgttttacctaatgatgacactctacgtgttgaggcttttgagtactaccacacaactgatcctagttttctgggtaggtacatgtcagcattaaatcacactaaaaagtggaaatacccacaagttaatggtttaacttctattaaatgggcagataacaactgttatcttgccactgcattgttaacactccaacaaatagagttgaagtttaatccacctgctctacaagatgcttattacagagcaagggctggtgaagctgctaacttttgtgcacttatcttagcctactgtaataagacagtaggtgagttaggtgatgttagagaaacaatgagttacttgtttcaacatgccaatttagattcttgcaaaagagtcttgaacgtggtgtgtaaaacttgtggacaacagcagacaacccttaagggtgtagaagctgttatgtacatgggcacactttcttatgaacaatttaagaaaggtgttcagataccttgtacgtgtggtaaacaagctacaaaatatctagtacaacaggagtcaccttttgttatgatgtcagcaccacctgctcagtatgaacttaagcatggtacatttacttgtgctagtgagtacactggtaattaccagtgtggtcactataaacatataacttctaaagaaactttgtattgcatagacggtgctttacttacaaagtcctcagaatacaaaggtcctattacggatgttttctacaaagaaaacagttacacaacaaccataaaaccagttacttataaattggatggtgttgtttgtacagaaattgaccctaagttggacaattattataagaaagacaattcttatttcacagagcaaccaattgatcttgtaccaaaccaaccatatccaaacgcaagcttcgataattttaagtttgtatgtgataatatcaaatttgctgatgatttaaaccagttaactggttataagaaacctgcttcaagagagcttaaagttacatttttccctgacttaaatggtgatgtggtggctattgattataaacactacacaccctcttttaagaaaggagctaaattgttacataaacctattgtttggcatgttaacaatgcaactaataaagccacgtataaaccaaatacctggtgtatacgttgtctttggagcacaaaaccagttgaaacatcaaattcgtttgatgtactgaagtcagaggacgcgcagggaatggataatcttgcctgcgaagatctaaaaccagtctctgaagaagtagtggaaaatcctaccatacagaaagacgttcttgagtgtaatgtgaaaactaccgaagttgtaggagacattatacttaaaccagcaaataatagtttaaaaattacagaagaggttggccacacagatctaatggctgcttatgtagacaattctagtcttactattaagaaacctaatgaattatctagagtattaggtttgaaaacccttgctactcatggtttagctgctgttaatagtgtcccttgggatactatagctaattatgctaagccttttcttaacaaagttgttagtacaactactaacatagttacacggtgtttaaaccgtgtttgtactaattatatgccttatttctttactttattgctacaattgtgtacttttactagaagtacaaattctagaattaaagcatctatgccgactactatagcaaagaatactgttaagagtgtcggtaaattttgtctagaggcttcatttaattatttgaagtcacctaatttttctaaactgataaatattataatttggtttttactattaagtgtttgcctaggttctttaatctactcaaccgctgctttaggtgttttaatgtctaatttaggcatgccttcttactgtactggttacagagaaggctatttgaactctactaatgtcactattgcaacctactgtactggttctataccttgtagtgtttgtcttagtggtttagattctttagacacctatccttctttagaaactatacaaattaccatttcatcttttaaatgggatttaactgcttttggcttagttgcagagtggtttttggcatatattcttttcactaggtttttctatgtacttggattggctgcaatcatgcaattgtttttcagctattttgcagtacattttattagtaattcttggcttatgtggttaataattaatcttgtacaaatggccccgatttcagctatggttagaatgtacatcttctttgcatcattttattatgtatggaaaagttatgtgcatgttgtagacggttgtaattcatcaacttgtatgatgtgttacaaacgtaatagagcaacaagagtcgaatgtacaactattgttaatggtgttagaaggtccttttatgtctatgctaatggaggtaaaggcttttgcaaactacacaattggaattgtgttaattgtgatacattctgtgctggtagtacatttattagtgatgaagttgcgagagacttgtcactacagtttaaaagaccaataaatcctactgaccagtcttcttacatcgttgatagtgttacagtgaagaatggttccatccatctttactttgataaagctggtcaaaagacttatgaaagacattctctctctcattttgttaacttagacaacctgagagctaataacactaaaggttcattgcctattaatgttatagtttttgatggtaaatcaaaatgtgaagaatcatctgcaaaatcagcgtctgtttactacagtcagcttatgtgtcaacctatactgttactagatcaggcattagtgtctgatgttggtgatagtgcggaagttgcagttaaaatgtttgatgcttacgttaatacgttttcatcaacttttaacgtaccaatggaaaaactcaaaacactagttgcaactgcagaagctgaacttgcaaagaatgtgtccttagacaatgtcttatctacttttatttcagcagctcggcaagggtttgttgattcagatgtagaaactaaagatgttgttgaatgtcttaaattgtcacatcaatctgacatagaagttactggcgatagttgtaataactatatgctcacctataacaaagttgaaaacatgacaccccgtgaccttggtgcttgtattgactgtagtgcgcgtcatattaatgcgcaggtagcaaaaagtcacaacattgctttgatatggaacgttaaagatttcatgtcattgtctgaacaactacgaaaacaaatacgtagtgctgctaaaaagaataacttaccttttaagttgacatgtgcaactactagacaagttgttaatgttgtaacaacaaagatagcacttaagggtggtaaaattgttaataattggttgaagcagttaattaaagttacacttgtgttcctttttgttgctgctattttctatttaataacacctgttcatgtcatgtctaaacatactgacttttcaagtgaaatcataggatacaaggctattgatggtggtgtcactcgtgacatagcatctacagatacttgttttgctaacaaacatgctgattttgacacatggtttagccagcgtggtggtagttatactaatgacaaagcttgcccattgattgctgcagtcataacaagagaagtgggttttgtcgtgcctggtttgcctggcacgatattacgcacaactaatggtgactttttgcatttcttacctagagtttttagtgcagttggtaacatctgttacacaccatcaaaacttatagagtacactgactttgcaacatcagcttgtgttttggctgctgaatgtacaatttttaaagatgcttctggtaagccagtaccatattgttatgataccaatgtactagaaggttctgttgcttatgaaagtttacgccctgacacacgttatgtgctcatggatggctctattattcaatttcctaacacctaccttgaaggttctgttagagtggtaacaacttttgattctgagtactgtaggcacggcacttgtgaaagatcagaagctggtgtttgtgtatctactagtggtagatgggtacttaacaatgattattacagatctttaccaggagttttctgtggtgtagatgctgtaaatttacttactaatatgtttacaccactaattcaacctattggtgctttggacatatcagcatctatagtagctggtggtattgtagctatcgtagtaacatgccttgcctactattttatgaggtttagaagagcttttggtgaatacagtcatgtagttgcctttaatactttactattccttatgtcattcactgtactctgtttaacaccagtttactcattcttacctggtgtttattctgttatttacttgtacttgacattttatcttactaatgatgtttcttttttagcacatattcagtggatggttatgttcacacctttagtacctttctggataacaattgcttatatcatttgtatttccacaaagcatttctattggttctttagtaattacctaaagagacgtgtagtctttaatggtgtttcctttagtacttttgaagaagctgcgctgtgcacctttttgttaaataaagaaatgtatctaaagttgcgtagtgatgtgctattacctcttacgcaatataatagatacttagctctttataataagtacaagtattttagtggagcaatggatacaactagctacagagaagctgcttgttgtcatctcgcaaaggctctcaatgacttcagtaactcaggttctgatgttctttaccaaccaccacaaacctctatcacctcagctgttttgcagagtggttttagaaaaatggcattcccatctggtaaagttgagggttgtatggtacaagtaacttgtggtacaactacacttaacggtctttggcttgatgacgtagtttactgtccaagacatgtgatctgcacctctgaagacatgcttaaccctaattatgaagatttactcattcgtaagtctaatcataatttcttggtacaggctggtaatgttcaactcagggttattggacattctatgcaaaattgtgtacttaagcttaaggttgatacagccaatcctaagacacctaagtataagtttgttcgcattcaaccaggacagactttttcagtgttagcttgttacaatggttcaccatctggtgtttaccaatgtgctatgaggcccaatttcactattaagggttcattccttaatggttcatgtggtagtgttggttttaacatagattatgactgtgtctctttttgttacatgcaccatatggaattaccaactggagttcatgctggcacagacttagaaggtaacttttatggaccttttgttgacaggcaaacagcacaagcagctggtacggacacaactattacagttaatgttttagcttggttgtacgctgctgttataaatggagacaggtggtttctcaatcgatttaccacaactcttaatgactttaaccttgtggctatgaagtacaattatgaacctctaacacaagaccatgttgacatactaggacctctttctgctcaaactggaattgccgttttagatatgtgtgcttcattaaaagaattactgcaaaatggtatgaatggacgtaccatattgggtagtgctttattagaagatgaatttacaccttttgatgttgttagacaatgctcaggtgttactttccaaagtgcagtgaaaagaacaatcaagggtacacaccactggttgttactcacaattttgacttcacttttagttttagtccagagtactcaatggtctttgttcttttttttgtatgaaaatgcctttttaccttttgctatgggtattattgctatgtctgcttttgcaatgatgtttgtcaaacataagcatgcatttctctgtttgtttttgttaccttctcttgccactgtagcttattttaatatggtctatatgcctgctagttgggtgatgcgtattatgacatggttggatatggttgatactagtttgtctggttttaagctaaaagactgtgttatgtatgcatcagctgtagtgttactaatccttatgacagcaagaactgtgtatgatgatggtgctaggagagtgtggacacttatgaatgtcttgacactcgtttataaagtttattatggtaatgctttagatcaagccatttccatgtgggctcttataatctctgttacttctaactactcaggtgtagttacaactgtcatgtttttggccagaggtattgtttttatgtgtgttgagtattgccctattttcttcataactggtaatacacttcagtgtataatgctagtttattgtttcttaggctatttttgtacttgttactttggcctcttttgtttactcaaccgctactttagactgactcttggtgtttatgattacttagtttctacacaggagtttagatatatgaattcacagggactactcccacccaagaatagcatagatgccttcaaactcaacattaaattgttgggtgttggtggcaaaccttgtatcaaagtagccactgtacagtctaaaatgtcagatgtaaagtgcacatcagtagtcttactctcagttttgcaacaactcagagtagaatcatcatctaaattgtgggctcaatgtgtccagttacacaatgacattctcttagctaaagatactactgaagcctttgaaaaaatggtttcactactttctgttttgctttccatgcagggtgctgtagacataaacaagctttgtgaagaaatgctggacaacagggcaaccttacaagctatagcctcagagtttagttcccttccatcatatgcagcttttgctactgctcaagaagcttatgagcaggctgttgctaatggtgattctgaagttgttcttaaaaagttgaagaagtctttgaatgtggctaaatctgaatttgaccgtgatgcagccatgcaacgtaagttggaaaagatggctgatcaagctatgacccaaatgtataaacaggctagatctgaggacaagagggcaaaagttactagtgctatgcagacaatgcttttcactatgcttagaaagttggataatgatgcactcaacaacattatcaacaatgcaagagatggttgtgttcccttgaacataatacctcttacaacagcagccaaactaatggttgtcataccagactataacacatataaaaatacgtgtgatggtacaacatttacttatgcatcagcattgtgggaaatccaacaggttgtagatgcagatagtaaaattgttcaacttagtgaaattagtatggacaattcacctaatttagcatggcctcttattgtaacagctttaagggccaattctgctgtcaaattacagaataatgagcttagtcctgttgcactacgacagatgtcttgtgctgccggtactacacaaactgcttgcactgatgacaatgcgttagcttactacaacacaacaaagggaggtaggtttgtacttgcactgttatccgatttacaggatttgaaatgggctagattccctaagagtgatggaactggtactatctatacagaactggaaccaccttgtaggtttgttacagacacacctaaaggtcctaaagtgaagtatttatactttattaaaggattaaacaacctaaatagaggtatggtacttggtagtttagctgccacagtacgtctacaagctggtaatgcaacagaagtgcctgccaattcaactgtattatctttctgtgcttttgctgtagatgctgctaaagcttacaaagattatctagctagtgggggacaaccaatcactaattgtgttaagatgttgtgtacacacactggtactggtcaggcaataacagttacaccggaagccaatatggatcaagaatcctttggtggtgcatcgtgttgtctgtactgccgttgccacatagatcatccaaatcctaaaggattttgtgacttaaaaggtaagtatgtacaaatacctacaacttgtgctaatgaccctgtgggttttacacttaaaaacacagtctgtaccgtctgcggtatgtggaaaggttatggctgtagttgtgatcaactccgcgaacccatgcttcagtcagctgatgcacaatcgtttttaaacgggtttgcggtgtaagtgcagcccgtcttacaccgtgcggcacaggcactagtactgatgtcgtatacagggcttttgacatctacaatgataaagtagctggttttgctaaattcctaaaaactaattgttgtcgcttccaagaaaaggacgaagatgacaatttaattgattcttactttgtagttaagagacacactttctctaactaccaacatgaagaaacaatttataatttacttaaggattgtccagctgttgctaaacatgacttctttaagtttagaatagacggtgacatggtaccacatatatcacgtcaacgtcttactaaatacacaatggcagacctcgtctatgctttaaggcattttgatgaaggtaattgtgacacattaaaagaaatacttgtcacatacaattgttgtgatgatgattatttcaataaaaaggactggtatgattttgtagaaaacccagatatattacgcgtatacgccaacttaggtgaacgtgtacgccaagctttgttaaaaacagtacaattctgtgatgccatgcgaaatgctggtattgttggtgtactgacattagataatcaagatctcaatggtaactggtatgatttcggtgatttcatacaaaccacgccaggtagtggagttcctgttgtagattcttattattcattgttaatgcctatattaaccttgaccagggctttaactgcagagtcacatgttgacactgacttaacaaagccttacattaagtgggatttgttaaaatatgacttcacggaagagaggttaaaactctttgaccgttattttaaatattgggatcagacataccacccaaattgtgttaactgtttggatgacagatgcattctgcattgtgcaaactttaatgttttattctctacagtgttcccacctacaagttttggaccactagtgagaaaaatatttgttgatggtgttccatttgtagtttcaactggataccacttcagagagctaggtgttgtacataatcaggatgtaaacttacatagctctagacttagttttaaggaattacttgtgtatgctgctgaccctgctatgcacgctgcttctggtaatctattactagataaacgcactacgtgcttttcagtagctgcacttactaacaatgttgcttttcaaactgtcaaacccggtaattttaacaaagacttctatgactttgctgtgtctaagggtttctttaaggaaggaagttctgttgaattaaaacacttcttctttgctcaggatggtaatgctgctatcagcgattatgactactatcgttataatctaccaacaatgtgtgatatcagacaactactatttgtagttgaagttgttgataagtactttgattgttacgatggtggctgtattaatgctaaccaagtcatcgtcaacaacctagacaaatcagctggttttccatttaataaatggggtaaggctagactttattatgattcaatgagttatgaggatcaagatgcacttttcgcatatacaaaacgtaatgtcatccctactataactcaaatgaatcttaagtatgccattagtgcaaagaatagagctcgcaccgtagctggtgtctctatctgtagtactatgaccaatagacagtttcatcaaaaattattgaaatcaatagccgccactagaggagctactgtagtaattggaacaagcaaattctatggtggttggcacaacatgttaaaaactgtttatagtgatgtagaaaaccctcaccttatgggttgggattatcctaaatgtgatagagccatgcctaacatgcttagaattatggcctcacttgttcttgctcgcaaacatacaacgtgttgtagcttgtcacaccgtttctatagattagctaatgagtgtgctcaagtattgagtgaaatggtcatgtgtggcggttcactatatgttaaaccaggtggaacctcatcaggagatgccacaactgcttatgctaatagtgtttttaacatttgtcaagctgtcacggccaatgttaatgcacttttatctactgatggtaacaaaattgccgataagtatgtccgcaatttacaacacagactttatgagtgtctctatagaaatagagatgttgacacagactttgtgaatgagttttacgcatatttgcgtaaacatttctcaatgatgatactctctgacgatgctgttgtgtgtttcaatagcacttatgcatctcaaggtctagtggctagcataaagaactttaagtcagttctttattatcaaaacaatgtttttatgtctgaagcaaaatgttggactgagactgaccttactaaaggacctcatgaattttgctctcaacatacaatgctagttaaacagggtgatgattatgtgtaccttccttacccagatccatcaagaatcctaggggccggctgttttgtagatgatatcgtaaaaacagatggtacacttatgattgaacggttcgtgtctttagctatagatgcttacccacttactaaacatcctaatcaggagtatgctgatgtctttcatttgtacttacaatacataagaaagctacatgatgagttaacaggacacatgttagacatgtattctgttatgcttactaatgataacacttcaaggtattgggaacctgagttttatgaggctatgtacacaccgcatacagtcttacaggctgttggggcttgtgttctttgcaattcacagacttcattaagatgtggtgcttgcatacgtagaccattcttatgttgtaaatgctgttacgaccatgtcatatcaacatcacataaattagtcttgtctgttaatccgtatgtttgcaatgctccaggttgtgatgtcacagatgtgactcaactttacttaggaggtatgagctattattgtaaatcacataaaccacccattagttttccattgtgtgctaatggacaagtttttggtttatataaaaatacatgtgttggtagcgataatgttactgactttaatgcaattgcaacatgtgactggacaaatgctggtgattacattttagctaacacctgtactgaaagactcaagctttttgcagcagaaacgctcaaagctactgaggagacatttaaactgtcttatggtattgctactgtacgtgaagtgctgtctgacagagaattacatctttcatgggaagttggtaaacctagaccaccacttaaccgaaattatgtctttactggttatcgtgtaactaaaaacagtaaagtacaaataggagagtacacctttgaaaaaggtgactatggtgatgctgttgtttaccgaggtacaacaacttacaaattaaatgttggtgattattttgtgctgacatcacatacagtaatgccattaagtgcacctacactagtgccacaagagcactatgttagaattactggcttatacccaacactcaatatctcagatgagttttctagcaatgttgcaaattatcaaaaggttggtatgcaaaagtattctacactccagggaccacctggtactggtaagagtcattttgctattggcctagctctctactacccttctgctcgcatagtgtatacagcttgctctcatgccgctgttgatgcactatgtgagaaggcattaaaatatttgcctatagataaatgtagtagaattatacctgcacgtgctcgtgtagagtgttttgataaattcaaagtgaattcaacattagaacagtatgtcttttgtactgtaaatgcattgcctgagacgacagcagatatagttgtctttgatgaaatttcaatggccacaaattatgatttgagtgttgtcaatgccagattacgtgctaagcactatgtgtacattggcgaccctgctcaattacctgcaccacgcacattgctaactaagggcacactagaaccagaatatttcaattcagtgtgtagacttatgaaaactataggtccagacatgttcctcggaacttgtcggcgttgtcctgctgaaattgttgacactgtgagtgctttggtttatgataataagcttaaagcacataaagacaaatcagctcaatgctttaaaatgttttataagggtgttatcacgcatgatgtttcatctgcaattaacaggccacaaataggcgtggtaagagaattccttacacgtaaccctgcttggagaaaagctgtctttatttcaccttataattcacagaatgctgtagcctcaaagattttgggactaccaactcaaactgttgattcatcacagggctcagaatatgactatgtcatattcactcaaaccactgaaacagctcactcttgtaatgtaaacagatttaatgttgctattaccagagcaaaagtaggcatactttgcataatgtctgatagagacctttatgacaagttgcaatttacaagtcttgaaattccacgtaggaatgtggcaactttacaagctgaaaatgtaacaggactctttaaagattgtagtaaggtaatcactgggttacatcctacacaggcacctacacacctcagtgttgacactaaattcaaaactgaaggtttatgtgttgacatacctggcatacctaaggacatgacctatagaagactcatctctatgatgggttttaaaatgaattatcaagttaatggttaccctaacatgtttatcacccgcgaagaagctataagacatgtacgtgcatggattggcttcgatgtcgaggggtgtcatgctactagagaagctgttggtaccaatttacctttacagctaggtttttctacaggtgttaacctagttgctgtacctacaggttatgttgatacacctaataatacagatttttccagagttagtgctaaaccaccgcctggagatcaatttaaacacctcataccacttatgtacaaaggacttccttggaatgtagtgcgtataaagattgtacaaatgttaagtgacacacttaaaaatctctctgacagagtcgtatttgtcttatgggcacatggctttgagttgacatctatgaagtattttgtgaaaataggacctgagcgcacctgttgtctatgtgatagacgtgccacatgcttttccactgcttcagacacttatgcctgttggcatcattctattggatttgattacgtctataatccgtttatgattgatgttcaacaatggggttttacaggtaacctacaaagcaaccatgatctgtattgtcaagtccatggtaatgcacatgtagctagttgtgatgcaatcatgactaggtgtctagctgtccacgagtgctttgttaagcgtgttgactggactattgaatatcctataattggtgatgaactgaagattaatgcggcttgtagaaaggttcaacacatggttgttaaagctgcattattagcagacaaattcccagttcttcacgacattggtaaccctaaagctattaagtgtgtacctcaagctgatgtagaatggaagttctatgatgcacagccttgtagtgacaaagcttataaaatagaagaattattctattcttatgccacacattctgacaaattcacagatggtgtatgcctattttggaattgcaatgtcgatagatatcctgctaattccattgtttgtagatttgacactagagtgctatctaaccttaacttgcctggttgtgatggtggcagtttgtatgtaaataaacatgcattccacacaccagcttttgataaaagtgcttttgttaatttaaaacaattaccatttttctattactctgacagtccatgtgagtctcatggaaaacaagtagtgtcagatatagattatgtaccactaaagtctgctacgtgtataacacgttgcaatttaggtggtgctgtctgtagacatcatgctaatgagtacagattgtatctcgatgcttataacatgatgatctcagctggctttagcttgtgggtttacaaacaatttgatacttataacctctggaacacttttacaagacttcagagtttagaaaatgtggcttttaatgttgtaaataagggacactttgatggacaacagggtgaagtaccagtttctatcattaataacactgtttacacaaaagttgatggtgttgatgtagaattgtttgaaaataaaacaacattacctgttaatgtagcatttgagctttgggctaagcgcaacattaaaccagtaccagaggtgaaaatactcaataatttgggtgtggacattgctgctaatactgtgatctgggactacaaaagagatgctccagcacatatatctactattggtgtttgttctatgactgacatagccaagaaaccaactgaaacgatttgtgcaccactcactgtcttttttgatggtagagttgatggtcaagtagacttatttagaaatgcccgtaatggtgttcttattacagaaggtagtgttaaaggtttacaaccatctgtgggtcccaaacaagctagtcttaatggagtcacattaattggagaagccgtaaaaacacagttcaattattataagaaagttgatggtgttgtccaacaattacctgaaacttactttactcagagtagaaatttacaagaatttaaacccaggagtcaaatggaaattgatttcttagaattagctatggatgaattcattgaacggtataaattagaaggctatgccttcgaacatatcgtttatggagattttagtcatagtcagttaggtggtttacatctactgattggactagctaaacgttttaaggaatcaccttttgaattagaagattttattcctatggacagtacagttaaaaactatttcataacagatgcgcaaacaggttcatctaagtgtgtgtgttctgttattgatttattacttgatgattttgttgaaataataaaatcccaagatttatctgtagtttctaaggttgtcaaagtgactattgactatacagaaatttcatttatgctttggtgtaaagatggccatgtagaaacattttacccaaaattacaatctagtcaagcgtggcaaccgggtgttgctatgcctaatctttacaaaatgcaaagaatgctattagaaaagtgtgaccttcaaaattatggtgatagtgcaacattacctaaaggcataatgatgaatgtcgcaaaatatactcaactgtgtcaatatttaaacacattaacattagctgtaccctataatatgagagttatacattttggtgctggttctgataaaggagttgcaccaggtacagctgttttaagacagtggttgcctacgggtacgctgcttgtcgattcagatcttaatgactttgtctctgatgcagattcaactttgattggtgattgtgcaactgtacatacagctaataaatgggatctcattattagtgatatgtacgaccctaagactaaaaatgttacaaaagaaaatgactctaaagagggttttttcacttacatttgtgggtttatacaacaaaagctagctcttggaggttccgtggctataaagataacagaacattcttggaatgctgatctttataagctcatgggacacttcgcatggtggacagcctttgttactaatgtgaatgcgtcatcatctgaagcatttttaattggatgtaattatcttggcaaaccacgcgaacaaatagatggttatgtcatgcatgcaaattacatattttggaggaatacaaatccaattcagttgtcttcctattctttatttgacatgagtaaatttccccttaaattaaggggtactgctgttatgtctttaaaagaaggtcaaatcaatgatatgattttatctcttcttagtaaaggtagacttataattagagaaaacaacagagttgttatttctagtgatgttcttgttaacaactaaacgaacaatgtttgtttttcttgttttattgccactagtctctagtcagtgtgttaatcttacaaccagaactcaattaccccctgcatacactaattctttcacacgtggtgtttattaccctgacaaagttttcagatcctcagttttacattcaactcaggacttgttcttacctttcttttccaatgttacttggttccatgctatacatgtctctgggaccaatggtactaagaggtttgataaccctgtcctaccatttaatgatggtgtttattttgcttccactgagaagtctaacataataagaggctggatttttggtactactttagattcgaagacccagtccctacttattgttaataacgctactaatgttgttattaaagtctgtgaatttcaattttgtaatgatccatttttgggtgtttattaccacaaaaacaacaaaagttggatggaaagtgagttcagagtttattctagtgcgaataattgcacttttgaatatgtctctcagccttttcttatggaccttgaaggaaaacagggtaatttcaaaaatcttagggaatttgtgtttaagaatattgatggttattttaaaatatattctaagcacacgcctattaatttagtgcgtgatctccctcagggtttttcggctttagaaccattggtagatttgccaataggtattaacatcactaggtttcaaactttacttgctttacatagaagttatttgactcctggtgattcttcttcaggttggacagctggtgctgcagcttattatgtgggttatcttcaacctaggacttttctattaaaatataatgaaaatggaaccattacagatgctgtagactgtgcacttgaccctctctcagaaacaaagtgtacgttgaaatccttcactgtagaaaaaggaatctatcaaacttctaactttagagtccaaccaacagaatctattgttagatttcctaatattacaaacttgtgcccttttggtgaagtttttaacgccaccagatttgcatctgtttatgcttggaacaggaagagaatcagcaactgtgttgctgattattctgtcctatataattccgcatcattttccacttttaagtgttatggagtgtctcctactaaattaaatgatctctgctttactaatgtctatgcagattcatttgtaattagaggtgatgaagtcagacaaatcgctccagggcaaactggaaagattgctgattataattataaattaccagatgattttacaggctgcgttatagcttggaattctaacaatcttgattctaaggttggtggtaattataattacctgtatagattgtttaggaagtctaatctcaaaccttttgagagagatatttcaactgaaatctatcaggccggtagcacaccttgtaatggtgttgaaggttttaattgttactttcctttacaatcatatggtttccaacccactaatggtgttggttaccaaccatacagagtagtagtactttcttttgaacttctacatgcaccagcaactgtttgtggacctaaaaagtctactaatttggttaaaaacaaatgtgtcaatttcaacttcaatggtttaacaggcacaggtgttcttactgagtctaacaaaaagtttctgcctttccaacaatttggcagagacattgctgacactactgatgctgtccgtgatccacagacacttgagattcttgacattacaccatgttcttttggtggtgtcagtgttataacaccaggaacaaatacttctaaccaggttgctgttctttatcaggatgttaactgcacagaagtccctgttgctattcatgcagatcaacttactcctacttggcgtgtttattctacaggttctaatgtttttcaaacacgtgcaggctgtttaataggggctgaacatgtcaacaactcatatgagtgtgacatacccattggtgcaggtatatgcgctagttatcagactcagactaattctcctcggcgggcacgtagtgtagctagtcaatccatcattgcctacactatgtcacttggtgcagaaaattcagttgcttactctaataactctattgccatacccacaaattttactattagtgttaccacagaaattctaccagtgtctatgaccaagacatcagtagattgtacaatgtacatttgtggtgattcaactgaatgcagcaatcttttgttgcaatatggcagtttttgtacacaattaaaccgtgctttaactggaatagctgttgaacaagacaaaaacacccaagaagtttttgcacaagtcaaacaaatttacaaaacaccaccaattaaagattttggtggttttaatttttcacaaatattaccagatccatcaaaaccaagcaagaggtcatttattgaagatctacttttcaacaaagtgacacttgcagatgctggcttcatcaaacaatatggtgattgccttggtgatattgctgctagagacctcatttgtgcacaaaagtttaacggccttactgttttgccacctttgctcacagatgaaatgattgctcaatacacttctgcactgttagcgggtacaatcacttctggttggacctttggtgcaggtgctgcattacaaataccatttgctatgcaaatggcttataggtttaatggtattggagttacacagaatgttctctatgagaaccaaaaattgattgccaaccaatttaatagtgctattggcaaaattcaagactcactttcttccacagcaagtgcacttggaaaacttcaagatgtggtcaaccaaaatgcacaagctttaaacacgcttgttaaacaacttagctccaattttggtgcaatttcaagtgttttaaatgatatcctttcacgtcttgacaaagttgaggctgaagtgcaaattgataggttgatcacaggcagacttcaaagtttgcagacatatgtgactcaacaattaattagagctgcagaaatcagagcttctgctaatcttgctgctactaaaatgtcagagtgtgtacttggacaatcaaaaagagttgatttttgtggaaagggctatcatcttatgtccttccctcagtcagcacctcatggtgtagtcttcttgcatgtgacttatgtccctgcacaagaaaagaacttcacaactgctcctgccatttgtcatgatggaaaagcacactttcctcgtgaaggtgtctttgtttcaaatggcacacactggtttgtaacacaaaggaatttttatgaaccacaaatcattactacagacaacacatttgtgtctggtaactgtgatgttgtaataggaattgtcaacaacacagtttatgatcctttgcaacctgaattagactcattcaaggaggagttagataaatattttaagaatcatacatcaccagatgttgatttaggtgacatctctggcattaatgcttcagttgtaaacattcaaaaagaaattgaccgcctcaatgaggttgccaagaatttaaatgaatctctcatcgatctccaagaacttggaaagtatgagcagtatataaaatggccatggtacatttggctaggttttatagctggcttgattgccatagtaatggtgacaattatgctttgctgtatgaccagttgctgtagttgtctcaagggctgttgttcttgtggatcctgctgcaaatttgatgaagacgactctgagccagtgctcaaaggagtcaaattacattacacataaacgaacttatggatttgtttatgagaatcttcacaattggaactgtaactttgaagcaaggtgaaatcaaggatgctactccttcagattttgttcgcgctactgcaacgataccgatacaagcctcactccctttcggatggcttattgttggcgttgcacttcttgctgtttttcagagcgcttccaaaatcataaccctcaaaaagagatggcaactagcactctccaagggtgttcactttgtttgcaacttgctgttgttgtttgtaacagtttactcacaccttttgctcgttgctgctggccttgaagccccttttctctatctttatgctttagtctacttcttgcagagtataaactttgtaagaataataatgaggctttggctttgctggaaatgccgttccaaaaacccattactttatgatgccaactattttctttgctggcatactaattgttacgactattgtataccttacaatagtgtaacttcttcaattgtcattacttcaggtgatggcacaacaagtcctatttctgaacatgactaccagattggtggttatactgaaaaatgggaatctggagtaaaagactgtgttgtattacacagttacttcacttcagactattaccagctgtactcaactcaattgagtacagacactggtgttgaacatgttaccttcttcatctacaataaaattgttgatgagcctgaagaacatgtccaaattcacacaatcgacggttcatccggagttgttaatccagtaatggaaccaatttatgatgaaccgacgacgactactagcgtgcctttgtaagcacaagctgatgagtacgaacttatgtactcattcgtttcggaagagacaggtacgttaatagttaatagcgtacttctttttcttgctttcgtggtattcttgctagttacactagccatccttactgcgcttcgattgtgtgcgtactgctgcaatattgttaacgtgagtcttgtaaaaccttctttttacgtttactctcgtgttaaaaatctgaattcttctagagttcctgatcttctggtctaaacgaactaaatattatattagtttttctgtttggaactttaattttagccatggcagattccaacggtactattaccgttgaagagcttaaaaagctccttgaacaatggaacctagtaataggtttcctattccttacatggatttgtcttctacaatttgcctatgccaacaggaataggtttttgtatataattaagttaattttcctctggctgttatggccagtaactttagcttgttttgtgcttgctgctgtttacagaataaattggatcaccggtggaattgctatcgcaatggcttgtcttgtaggcttgatgtggctcagctacttcattgcttctttcagactgtttgcgcgtacccgttccatgtggtcattcaatccagaaactaacattcttctcaacgtgccactccatggcactattctgaccagaccgcttctagaaagtgaactcgtaatcggagctgtgatccttcgtggacatcttcgtattgctggacaccatctaggacgctgtgacatcaaggacctgcctaaagaaatcactgttgctacatcacgaacgctttcttattacaaattgggagcttcgcagcgtgtagcaggtgactcaggttttgctgcatacagtcgctacaggattggcaactataaattaaacacagaccattccagtagcagtgacaatattgctttgcttgtacagtaagtgacaacagatgtttcatctcgttgactttcaggttactatagcagagatattactaattattatgaggacttttaaagtttccatttggaatcttgattacatcataaacctcataattaaaaatttatctaagtcactaactgagaataaatattctcaattagatgaagagcaaccaatggagattgattaaacgaacatgaaaattattcttttcttggcactgataacactcgctacttgtgagctttatcactaccaagagtgtgttagaggtacaacagtacttttaaaagaaccttgctcttctggaacatacgagggcaattcaccatttcatcctctagctgataacaaatttgcactgacttgctttagcactcaatttgcttttgcttgtcctgacggcgtaaaacacgtctatcagttacgtgccagatcagtttcacctaaactgttcatcagacaagaggaagttcaagaactttactctccaatttttcttattgttgcggcaatagtgtttataacactttgcttcacactcaaaagaaagacagaatgattgaactttcattaattgacttctatttgtgctttttagcctttctgctattccttgttttaattatgcttattatcttttggttctcacttgaactgcaagatcataatgaaacttgtcacgcctaaacgaacatgaaatttcttgttttcttaggaatcatcacaactgtagctgcatttcaccaagaatgtagtttacagtcatgtactcaacatcaaccatatgtagttgatgacccgtgtcctattcacttctattctaaatggtatattagagtaggagctagaaaatcagcacctttaattgaattgtgcgtggatgaggctggttctaaatcacccattcagtacatcgatatcggtaattatacagtttcctgtttaccttttacaattaattgccaggaacctaaattgggtagtcttgtagtgcgttgttcgttctatgaagactttttagagtatcatgacgttcgtgttgttttagatttcatctaaacgaacaaactaaaatgtctgataatggaccccaaaatcagcgaaatgcaccccgcattacgtttggtggaccctcagattcaactggcagtaaccagaatggagaacgcagtggggcgcgatcaaaacaacgtcggccccaaggtttacccaataatactgcgtcttggttcaccgctctcactcaacatggcaaggaagaccttaaattccctcgaggacaaggcgttccaattaacaccaatagcagtccagatgaccaaattggctactaccgaagagctaccagacgaattcgtggtggtgacggtaaaatgaaagatctcagtccaagatggtatttctactacctaggaactgggccagaagctggacttccctatggtgctaacaaagacggcatcatatgggttgcaactgagggagccttgaatacaccaaaagatcacattggcacccgcaatcctgctaacaatgctgcaatcgtgctacaacttcctcaaggaacaacattgccaaaaggcttctacgcagaagggagcagaggcggcagtcaagcctcttctcgttcctcatcacgtagtcgcaacagttcaagaaattcaactccaggcagcagtaggggaacttctcctgctagaatggctggcaatggcggtgatgctgctcttgctttgctgctgcttgacagattgaaccagcttgagagcaaaatgtctggtaaaggccaacaacaacaaggccaaactgtcactaagaaatctgctgctgaggcttctaagaagcctcggcaaaaacgtactgccactaaagcatacaatgtaacacaagctttcggcagacgtggtccagaacaaacccaaggaaattttggggaccaggaactaatcagacaaggaactgattacaaacattggccgcaaattgcacaatttgcccccagcgcttcagcgttcttcggaatgtcgcgcattggcatggaagtcacaccttcgggaacgtggttgacctacacaggtgccatcaaattggatgacaaagatccaaatttcaaagatcaagtcattttgctgaataagcatattgacgcatacaaaacattcccaccaacagagcctaaaaaggacaaaaagaagaaggctgatgaaactcaagccttaccgcagagacagaagaaacagcaaactgtgactcttcttcctgctgcagatttggatgatttctccaaacaattgcaacaatccatgagcagtgctgactcaactcaggcctaaactcatgcagaccacacaaggcagatgggctatataaacgttttcgcttttccgtttacgatatatagtctactcttgtgcagaatgaattctcgtaactacatagcacaagtagatgtagttaactttaatctcacatagcaatctttaatcagtgtgtaacattagggaggacttgaaagagccaccacattttcaccgaggccacgcggagtacgatcgagtgtacagtgaacaatgctagggagagctgcctatatggaagagccctaatgtgtaaaattaattttagtagtgctatccccatgtgattttaatagcttcttaggagaatgacaaaaaaaaaaaaaaaaaaaaaaaaagggtcggcatggcatctccacctcctcgcggtccgacctgggcatccgaaggaggacgtcgtccactcggatggctaagggagagctcggatcgatccgcctcgactgtgccttctagttgccagccatctgttgtttgcccctcccccgtgccttccttgaccctggaaggtgccactcccactgtcctttcctaataaaatgaggaaattgcatcgcattgtctgagtaggtgtcattctattctggggggtggggtggggcaggacagcaagggggaggattgggaagacaatagcaggcatgctggggagagctcgagctctgtacatgtccgcgga

SEQ ID NO: 9 - DNA, 964 bp, Coronaviridae
  misc_feature 1..964: note = F1 fragment polynucleotide sequence
  source 1..964: mol_type = other DNA
ggcgcgcctaagttgacattgattattgactagttattaatagtaatcaattacggggtcattagttcatagcccatatatggagttccgcgttacataacttacggtaaatggcccgcctggctgaccgcccaacgacccccgcccattgacgtcaataatgacgtatgttcccatagtaacgccaatagggactttccattgacgtcaatgggtggagtatttacggtaaactgcccacttggcagtacatcaagtgtatcatatgccaagtacgccccctattgacgtcaatgacggtaaatggcccgcctggcattatgcccagtacatgaccttatgggactttcctacttggcagtacatctacgtattagtcatcgctattaccatggtgatgcggttttggcagtacatcaatgggcgtggatagcggtttgactcacggggatttccaagtctccaccccattgacgtcaatgggagtttgttttggcaccaaaatcaacgggactttccaaaatgtcgtaacaactccgccccattgacgcaaatgggcggtaggcgtgtacggtgggaggtctatataagcagagctcgtttagtgaaccgtattaaaggtttataccttcccaggtaacaaaccaaccaactttcgatctcttgtagatctgttctctaaacgaactttaaaatctgtgtggctgtcactcggctgcatgcttagtgcactcacgcagtataattaataactaattactgtcgttgacaggacacgagtaactcgtctatcttctgcaggctgcttacggtttcgtccgtgttgcagccgatcatcagcacatctaggtttcgtccgggtgtgaccgaaaggtaagatggagagccttgtccctggtttcaacgagaaaacacacgtccaactcagtttgcctgttttacaggttcgcgacgtgctcgtacg

SEQ ID NO: 10 - DNA, 6406 bp, Coronaviridae
  misc_feature 1..6406: note = F2 fragment polynucleotide sequence
  source 1..6406: mol_type = other DNA
cgtacgtggctttggagactccgtggaggaggtcttatcagaggcacgtcaacatcttaaagatggcacttgtggcttagtagaagttgaaaaaggcgttttgcctcaacttgaacagccctatgtgttcatcaaacgttcggatgctcgaactgcacctcatggtcatgttatggttgagctggtagcagaactcgaaggcattcagtacggtcgtagtggtgagacacttggtgtccttgtccctcatgtgggcgaaataccagtggcttaccgcaaggttcttcttcgtaagaacggtaataaaggagctggtggccatagttacggcgccgatctaaagtcatttgacttaggcgacgagcttggcactgatccttatgaagattttcaagaaaactggaacactaaacatagcagtggtgttacccgtgaactcatgcgtgagcttaacggaggggcatacactcgctatgtcgataacaacttctgtggccctgatggctaccctcttgagtgcattaaagaccttctagcacgtgctggtaaagcttcatgcactttgtccgaacaactggactttattgacactaagaggggtgtatactgctgccgtgaacatgagcatgaaattgcttggtacacggaacgttctgaaaagagctatgaattgcagacaccttttgaaattaaattggcaaagaaatttgacaccttcaatggggaatgtccaaattttgtatttcccttaaattccataatcaagactattcaaccaagggttgaaaagaaaaagcttgatggctttatgggtagaattcgatctgtctatccagttgcgtcaccaaatgaatgcaaccaaatgtgcctttcaactctcatgaagtgtgatcattgtggtgaaacttcatggcagacgggcgattttgttaaagccacttgcgaattttgtggcactgagaatttgactaaagaaggtgccactacttgtggttacttaccccaaaatgctgttgttaaaatttattgtccagcatgtcacaattcagaagtaggacctgagcatagtcttgccgaataccataatgaatctggcttgaaaaccattcttcgtaagggtggtcgcactattgcctttggaggctgtgtgttctcttatgttggttgccataacaagtgtgcctattgggttccacgtgctagcgctaacataggttgtaaccatacaggtgttgttggagaaggttccgaaggtcttaatgacaaccttcttgaaatactccaaaaagagaaagtcaacatcaatattgttggtgactttaaacttaatgaagagatcgccattattttggcatctttttctgcttccacaagtgcttttgtggaaactgtgaaaggtttggattataaagcattcaaacaaattgttgaatcctgtggtaattttaaagttacaaaaggaaaagctaaaaaaggtgcctggaatattggtgaacagaaatcaatactgagtcctctttatgcatttgcatcagaggctgctcgtgttgtacgatcaattttctcccgcactcttgaaactgctcaaaattctgtgcgtgttttacagaaggccgctataacaatactagatggaatttcacagtattcactgagactcattgatgctatgatgttcacatctgatttggctactaacaatctagttgtaatggcctacattacaggtggtgttgttcagttgacttcgcagtggctaactaacatctttggcactgtttatgaaaaactcaaacccgtccttgattggcttgaagagaagtttaaggaaggtgtagagtttcttagagacggttgggaaattgttaaatttatctcaacctgtgcttgtgaaattgtcggtggacaaattgtcacctgtgcaaaggaaattaaggagagtgttcagacattctttaagcttgtaaataaatttttggctttgtgtgctgactctatcattattggtggagctaaacttaaagccttgaatttaggtgaaacatttgtcacgcactcaaagggattgtacagaaagtgtgttaaatccagagaagaaactggcctactcatgcctctaaaagccccaaaagaaattatcttcttagagggagaaacacttcccacagaagtgttaacagaggaagttgtcttgaaaactggtgatttacaaccattagaacaacctactagtgaagctgttgaagctccattggttggtacaccagtttgtattaacgggcttatgttgctcgaaatcaaagacacagaaaagtactgtgcccttgcacctaatatgatggtaacaaacaataccttcacactcaaaggcggtgcaccaacaaaggttacttttggtgatgacactgtgatagaagtgcaaggttacaagagtgtgaatatcacttttgaacttgatgaaaggattgataaagtacttaatgagaagtgctctgcctatacagttgaactcggtacagaagtaaatgagttcgcctgtgttgtggcagatgctgtcataaaaactttgcaaccagtatctgaattacttacaccactgggcattgatttagatgagtggagtatggctacatactacttatttgatgagtctggtgagtttaaattggcttcacatatgtattgttctttctaccctccagatgaggatgaagaagaaggtgattgtgaagaagaagagtttgagccatcaactcaatatgagtatggtactgaagatgattaccaaggtaaacctttggaatttggtgccacttctgctgctcttcaacctgaagaagagcaagaagaagattggttagatgatgatagtcaacaaactgttggtcaacaagacggcagtgaggacaatcagacaactactattcaaacaattgttgaggttcaacctcaattagagatggaacttacaccagttgttcagactattgaagtgaatagttttagtggttatttaaaacttactgacaatgtatacattaaaaatgcagacattgtggaagaagctaaaaaggtaaaaccaacagtggttgttaatgcagccaatgtttaccttaaacatggaggaggtgttgcaggagccttaaataaggctactaacaatgccatgcaagttgaatctgatgattacatagctactaatggaccacttaaagtgggtggtagttgtgttttaagcggacacaatcttgctaaacactgtcttcatgttgtcggcccaaatgttaacaaaggtgaagacattcaacttcttaagagtgcttatgaaaattttaatcagcacgaagttctacttgcaccattattatcagctggtatttttggtgctgaccctatacattctttaagagtttgtgtagatactgttcgcacaaatgtctacttagctgtctttgataaaaatctctatgacaaacttgtttcaagctttttggaaatgaagagtgaaaagcaagttgaacaaaagatcgctgagattcctaaagaggaagttaagccatttataactgaaagtaaaccttcagttgaacagagaaaacaagatgataagaaaatcaaagcttgtgttgaagaagttacaacaactctggaagaaactaagttcctcacagaaaacttgttactttatattgacattaatggcaatcttcatccagattctgccactcttgttagtgacattgacatcactttcttaaagaaagatgctccatatatagtgggtgatgttgttcaagagggtgttttaactgctgtggttatacctactaaaaaggctggtggcactactgaaatgctagcgaaagctttgagaaaagtgccaacagacaattatataaccacttacccgggtcagggtttaaatggttacactgtagaggaggcaaagacagtgcttaaaaagtgtaaaagtgccttttacattctaccatctattatctctaatgagaagcaagaaattcttggaactgtttcttggaatttgcgagaaatgcttgcacatgcagaagaaacacgcaaattaatgcctgtctgtgtggaaactaaagccatagtttcaactatacagcgtaaatataagggtattaaaatacaagagggtgtggttgattatggtgctagattttacttttacaccagtaaaacaactgtagcgtcacttatcaacacacttaacgatctaaatgaaactcttgttacaatgccacttggctatgtaacacatggcttaaatttggaagaagctgctcggtatatgagatctctcaaagtgccagctacagtttctgtttcttcacctgatgctgttacagcgtataatggttatcttacttcttcttctaaaacacctgaagaacattttattgaaaccatctcacttgctggttcctataaagattggtcctattctggacaatctacacaactaggtatagaatttcttaagagaggtgataaaagtgtatattacactagtaatcctaccacattccacctagatggtgaagttatcacctttgacaatcttaagacacttctttctttgagagaagtgaggactattaaggtgtttacaacagtagacaacattaacctccacacgcaagttgtggacatgtcaatgacatatggacaacagtttggtccaacttatttggatggagctgatgttactaaaataaaacctcataattcacatgaaggtaaaacattttatgttttacctaatgatgacactctacgtgttgaggcttttgagtactaccacacaactgatcctagttttctgggtaggtacatgtcagcattaaatcacactaaaaagtggaaatacccacaagttaatggtttaacttctattaaatgggcagataacaactgttatcttgccactgcattgttaacactccaacaaatagagttgaagtttaatccacctgctctacaagatgcttattacagagcaagggctggtgaagctgctaacttttgtgcacttatcttagcctactgtaataagacagtaggtgagttaggtgatgttagagaaacaatgagttacttgtttcaacatgccaatttagattcttgcaaaagagtcttgaacgtggtgtgtaaaacttgtggacaacagcagacaacccttaagggtgtagaagctgttatgtacatgggcacactttcttatgaacaatttaagaaaggtgttcagataccttgtacgtgtggtaaacaagctacaaaatatctagtacaacaggagtcaccttttgttatgatgtcagcaccacctgctcagtatgaacttaagcatggtacatttacttgtgctagtgagtacactggtaattaccagtgtggtcactataaacatataacttctaaagaaactttgtattgcatagacggtgctttacttacaaagtcctcagaatacaaaggtcctattacggatgttttctacaaagaaaacagttacacaacaaccataaaaccagttacttataaattggatggtgttgtttgtacagaaattgaccctaagttggacaattattataagaaagacaattcttatttcacagagcaaccaattgatcttgtaccaaaccaaccatatccaaacgcaagcttcgataattttaagtttgtatgtgataatatcaaatttgctgatgatttaaaccagttaactggttataagaaacctgcttcaagagagcttaaagttacatttttccctgacttaaatggtgatgtggtggctattgattataaacactacacaccctcttttaagaaaggagctaaattgttacataaacctattgtttggcatgttaacaatgcaactaataaagccacgtataaaccaaatacctggtgtatacgttgtctttggagcacaaaaccagttgaaacatcaaattcgtttgatgtactgaagtcagaggacgcgcagggaatggataatcttgcctgcgaagatctaaaaccagtctctgaagaagtagtggaaaatcctaccatacagaaagacgttcttgagtgtaatgtgaaaactaccgaagttgtaggagacattatacttaaaccagcaaataatagtttaaaaattacagaagaggttggccacacagatctaatggctgcttatgtagacaattctagtcttactattaagaaacctaatgaattatctagagtattaggtttgaaaacccttgctactcatggtttagctgctgttaatagtgtcccttgggatactatagctaattatgctaagccttttcttaacaaagttgttagtacaactactaacatagttacacggtgtttaaac

SEQ ID NO: 11 - DNA, 7218 bp, Coronaviridae
  misc_feature 1..7218: note = F3 fragment polynucleotide sequence
  source 1..7218: mol_type = other DNA
gtttaaaccgtgtttgtactaattatatgccttatttctttactttattgctacaattgtgtacttttactagaagtacaaattctagaattaaagcatctatgccgactactatagcaaagaatactgttaagagtgtcggtaaattttgtctagaggcttcatttaattatttgaagtcacctaatttttctaaactgataaatattataatttggtttttactattaagtgtttgcctaggttctttaatctactcaaccgctgctttaggtgttttaatgtctaatttaggcatgccttcttactgtactggttacagagaaggctatttgaactctactaatgtcactattgcaacctactgtactggttctataccttgtagtgtttgtcttagtggtttagattctttagacacctatccttctttagaaactatacaaattaccatttcatcttttaaatgggatttaactgcttttggcttagttgcagagtggtttttggcatatattcttttcactaggtttttctatgtacttggattggctgcaatcatgcaattgtttttcagctattttgcagtacattttattagtaattcttggcttatgtggttaataattaatcttgtacaaatggccccgatttcagctatggttagaatgtacatcttctttgcatcattttattatgtatggaaaagttatgtgcatgttgtagacggttgtaattcatcaacttgtatgatgtgttacaaacgtaatagagcaacaagagtcgaatgtacaactattgttaatggtgttagaaggtccttttatgtctatgctaatggaggtaaaggcttttgcaaactacacaattggaattgtgttaattgtgatacattctgtgctggtagtacatttattagtgatgaagttgcgagagacttgtcactacagtttaaaagaccaataaatcctactgaccagtcttcttacatcgttgatagtgttacagtgaagaatggttccatccatctttactttgataaagctggtcaaaagacttatgaaagacattctctctctcattttgttaacttagacaacctgagagctaataacactaaaggttcattgcctattaatgttatagtttttgatggtaaatcaaaatgtgaagaatcatctgcaaaatcagcgtctgtttactacagtcagcttatgtgtcaacctatactgttactagatcaggcattagtgtctgatgttggtgatagtgcggaagttgcagttaaaatgtttgatgcttacgttaatacgttttcatcaacttttaacgtaccaatggaaaaactcaaaacactagttgcaactgcagaagctgaacttgcaaagaatgtgtccttagacaatgtcttatctacttttatttcagcagctcggcaagggtttgttgattcagatgtagaaactaaagatgttgttgaatgtcttaaattgtcacatcaatctgacatagaagttactggcgatagttgtaataactatatgctcacctataacaaagttgaaaacatgacaccccgtgaccttggtgcttgtattgactgtagtgcgcgtcatattaatgcgcaggtagcaaaaagtcacaacattgctttgatatggaacgttaaagatttcatgtcattgtctgaacaactacgaaaacaaatacgtagtgctgctaaaaagaataacttaccttttaagttgacatgtgcaactactagacaagttgttaatgttgtaacaacaaagatagcacttaagggtggtaaaattgttaataattggttgaagcagttaattaaagttacacttgtgttcctttttgttgctgctattttctatttaataacacctgttcatgtcatgtctaaacatactgacttttcaagtgaaatcataggatacaaggctattgatggtggtgtcactcgtgacatagcatctacagatacttgttttgctaacaaacatgctgattttgacacatggtttagccagcgtggtggtagttatactaatgacaaagcttgcccattgattgctgcagtcataacaagagaagtgggttttgtcgtgcctggtttgcctggcacgatattacgcacaactaatggtgactttttgcatttcttacctagagtttttagtgcagttggtaacatctgttacacaccatcaaaacttatagagtacactgactttgcaacatcagcttgtgttttggctgctgaatgtacaatttttaaagatgcttctggtaagccagtaccatattgttatgataccaatgtactagaaggttctgttgcttatgaaagtttacgccctgacacacgttatgtgctcatggatggctctattattcaatttcctaacacctaccttgaaggttctgttagagtggtaacaacttttgattctgagtactgtaggcacggcacttgtgaaagatcagaagctggtgtttgtgtatctactagtggtagatgggtacttaacaatgattattacagatctttaccaggagttttctgtggtgtagatgctgtaaatttacttactaatatgtttacaccactaattcaacctattggtgctttggacatatcagcatctatagtagctggtggtattgtagctatcgtagtaacatgccttgcctactattttatgaggtttagaagagcttttggtgaatacagtcatgtagttgcctttaatactttactattccttatgtcattcactgtactctgtttaacaccagtttactcattcttacctggtgtttattctgttatttacttgtacttgacattttatcttactaatgatgtttcttttttagcacatattcagtggatggttatgttcacacctttagtacctttctggataacaattgcttatatcatttgtatttccacaaagcatttctattggttctttagtaattacctaaagagacgtgtagtctttaatggtgtttcctttagtacttttgaagaagctgcgctgtgcacctttttgttaaataaagaaatgtatctaaagttgcgtagtgatgtgctattacctcttacgcaatataatagatacttagctctttataataagtacaagtattttagtggagcaatggatacaactagctacagagaagctgcttgttgtcatctcgcaaaggctctcaatgacttcagtaactcaggttctgatgttctttaccaaccaccacaaacctctatcacctcagctgttttgcagagtggttttagaaaaatggcattcccatctggtaaagttgagggttgtatggtacaagtaacttgtggtacaactacacttaacggtctttggcttgatgacgtagtttactgtccaagacatgtgatctgcacctctgaagacatgcttaaccctaattatgaagatttactcattcgtaagtctaatcataatttcttggtacaggctggtaatgttcaactcagggttattggacattctatgcaaaattgtgtacttaagcttaaggttgatacagccaatcctaagacacctaagtataagtttgttcgcattcaaccaggacagactttttcagtgttagcttgttacaatggttcaccatctggtgtttaccaatgtgctatgaggcccaatttcactattaagggttcattccttaatggttcatgtggtagtgttggttttaacatagattatgactgtgtctctttttgttacatgcaccatatggaattaccaactggagttcatgctggcacagacttagaaggtaacttttatggaccttttgttgacaggcaaacagcacaagcagctggtacggacacaactattacagttaatgttttagcttggttgtacgctgctgttataaatggagacaggtggtttctcaatcgatttaccacaactcttaatgactttaaccttgtggctatgaagtacaattatgaacctctaacacaagaccatgttgacatactaggacctctttctgctcaaactggaattgccgttttagatatgtgtgcttcattaaaagaattactgcaaaatggtatgaatggacgtaccatattgggtagtgctttattagaagatgaatttacaccttttgatgttgttagacaatgctcaggtgttactttccaaagtgcagtgaaaagaacaatcaagggtacacaccactggttgttactcacaattttgacttcacttttagttttagtccagagtactcaatggtctttgttcttttttttgtatgaaaatgcctttttaccttttgctatgggtattattgctatgtctgcttttgcaatgatgtttgtcaaacataagcatgcatttctctgtttgtttttgttaccttctcttgccactgtagcttattttaatatggtctatatgcctgctagttgggtgatgcgtattatgacatggttggatatggttgatactagtttgtctggttttaagctaaaagactgtgttatgtatgcatcagctgtagtgttactaatccttatgacagcaagaactgtgtatgatgatggtgctaggagagtgtggacacttatgaatgtcttgacactcgtttataaagtttattatggtaatgctttagatcaagccatttccatgtgggctcttataatctctgttacttctaactactcaggtgtagttacaactgtcatgtttttggccagaggtattgtttttatgtgtgttgagtattgccctattttcttcataactggtaatacacttcagtgtataatgctagtttattgtttcttaggctatttttgtacttgttactttggcctcttttgtttactcaaccgctactttagactgactcttggtgtttatgattacttagtttctacacaggagtttagatatatgaattcacagggactactcccacccaagaatagcatagatgccttcaaactcaacattaaattgttgggtgttggtggcaaaccttgtatcaaagtagccactgtacagtctaaaatgtcagatgtaaagtgcacatcagtagtcttactctcagttttgcaacaactcagagtagaatcatcatctaaattgtgggctcaatgtgtccagttacacaatgacattctcttagctaaagatactactgaagcctttgaaaaaatggtttcactactttctgttttgctttccatgcagggtgctgtagacataaacaagctttgtgaagaaatgctggacaacagggcaaccttacaagctatagcctcagagtttagttcccttccatcatatgcagcttttgctactgctcaagaagcttatgagcaggctgttgctaatggtgattctgaagttgttcttaaaaagttgaagaagtctttgaatgtggctaaatctgaatttgaccgtgatgcagccatgcaacgtaagttggaaaagatggctgatcaagctatgacccaaatgtataaacaggctagatctgaggacaagagggcaaaagttactagtgctatgcagacaatgcttttcactatgcttagaaagttggataatgatgcactcaacaacattatcaacaatgcaagagatggttgtgttcccttgaacataatacctcttacaacagcagccaaactaatggttgtcataccagactataacacatataaaaatacgtgtgatggtacaacatttacttatgcatcagcattgtgggaaatccaacaggttgtagatgcagatagtaaaattgttcaacttagtgaaattagtatggacaattcacctaatttagcatggcctcttattgtaacagctttaagggccaattctgctgtcaaattacagaataatgagcttagtcctgttgcactacgacagatgtcttgtgctgccggtactacacaaactgcttgcactgatgacaatgcgttagcttactacaacacaacaaagggaggtaggtttgtacttgcactgttatccgatttacaggatttgaaatgggctagattccctaagagtgatggaactggtactatctatacagaactggaaccaccttgtaggtttgttacagacacacctaaaggtcctaaagtgaagtatttatactttattaaaggattaaacaacctaaatagaggtatggtacttggtagtttagctgccacagtacgtctacaagctggtaatgcaacagaagtgcctgccaattcaactgtattatctttctgtgcttttgctgtagatgctgctaaagcttacaaagattatctagctagtgggggacaaccaatcactaattgtgttaagatgttgtgtacacacactggtactggtcaggcaataacagttacaccggaagccaatatggatcaagaatcctttggtggtgcatcgtgttgtctgtactgccgttgccacatagatcatccaaatcctaaaggattttgtgacttaaaaggtaagtatgtacaaatacctacaacttgtgctaatgaccctgtgggttttacacttaaaaacacagtctgtaccgtctgcggtatgtggaaaggttatggctgtagttgtgatcaactccgcgaacccatgcttcagtcagctgatgcacaatcgtttttaaacgggtttgcggtgtaagtgcagcccgtcttacaccgtgcggcacaggcactagtactgatgtcgtatacagggcttttgacatctacaatgataaagtagctggttttgctaaattcctaaaaactaattgttgtcgcttccaagaaaaggacgaagatgacaatttaattgattcttactttgtagttaagagacacactttctctaactaccaacatgaagaaacaatttataatttacttaaggattgtccagctgttgctaaacatgacttctttaagtttagaatagacggtgacatggtaccacatatatcacgtcaacgtcttactaaatacacaatggcagacctcgtctatgctttaaggcattttgatgaaggtaattgtgacacattaaaagaaatacttgtcacatacaattgttgtgatgatgattatttcaataaaaaggactggtatgattttgtagaaaacccagatatattacgcgt

SEQ ID NO: 12 - DNA, 6136 bp, Coronaviridae
  misc_feature 1..6136: note = F4 fragment polynucleotide sequence
  source 1..6136: mol_type = other DNA
acgcgtatacgccaacttaggtgaacgtgtacgccaagctttgttaaaaacagtacaattctgtgatgccatgcgaaatgctggtattgttggtgtactgacattagataatcaagatctcaatggtaactggtatgatttcggtgatttcatacaaaccacgccaggtagtggagttcctgttgtagattcttattattcattgttaatgcctatattaaccttgaccagggctttaactgcagagtcacatgttgacactgacttaacaaagccttacattaagtgggatttgttaaaatatgacttcacggaagagaggttaaaactctttgaccgttattttaaatattgggatcagacataccacccaaattgtgttaactgtttggatgacagatgcattctgcattgtgcaaactttaatgttttattctctacagtgttcccacctacaagttttggaccactagtgagaaaaatatttgttgatggtgttccatttgtagtttcaactggataccacttcagagagctaggtgttgtacataatcaggatgtaaacttacatagctctagacttagttttaaggaattacttgtgtatgctgctgaccctgctatgcacgctgcttctggtaatctattactagataaacgcactacgtgcttttcagtagctgcacttactaacaatgttgcttttcaaactgtcaaacccggtaattttaacaaagacttctatgactttgctgtgtctaagggtttctttaaggaaggaagttctgttgaattaaaacacttcttctttgctcaggatggtaatgctgctatcagcgattatgactactatcgttataatctaccaacaatgtgtgatatcagacaactactatttgtagttgaagttgttgataagtactttgattgttacgatggtggctgtattaatgctaaccaagtcatcgtcaacaacctagacaaatcagctggttttccatttaataaatggggtaaggctagactttattatgattcaatgagttatgaggatcaagatgcacttttcgcatatacaaaacgtaatgtcatccctactataactcaaatgaatcttaagtatgccattagtgcaaagaatagagctcgcaccgtagctggtgtctctatctgtagtactatgaccaatagacagtttcatcaaaaattattgaaatcaatagccgccactagaggagctactgtagtaattggaacaagcaaattctatggtggttggcacaacatgttaaaaactgtttatagtgatgtagaaaaccctcaccttatgggttgggattatcctaaatgtgatagagccatgcctaacatgcttagaattatggcctcacttgttcttgctcgcaaacatacaacgtgttgtagcttgtcacaccgtttctatagattagctaatgagtgtgctcaagtattgagtgaaatggtcatgtgtggcggttcactatatgttaaaccaggtggaacctcatcaggagatgccacaactgcttatgctaatagtgtttttaacatttgtcaagctgtcacggccaatgttaatgcacttttatctactgatggtaacaaaattgccgataagtatgtccgcaatttacaacacagactttatgagtgtctctatagaaatagagatgttgacacagactttgtgaatgagttttacgcatatttgcgtaaacatttctcaatgatgatactctctgacgatgctgttgtgtgtttcaatagcacttatgcatctcaaggtctagtggctagcataaagaactttaagtcagttctttattatcaaaacaatgtttttatgtctgaagcaaaatgttggactgagactgaccttactaaaggacctcatgaattttgctctcaacatacaatgctagttaaacagggtgatgattatgtgtaccttccttacccagatccatcaagaatcctaggggccggctgttttgtagatgatatcgtaaaaacagatggtacacttatgattgaacggttcgtgtctttagctatagatgcttacccacttactaaacatcctaatcaggagtatgctgatgtctttcatttgtacttacaatacataagaaagctacatgatgagttaacaggacacatgttagacatgtattctgttatgcttactaatgataacacttcaaggtattgggaacctgagttttatgaggctatgtacacaccgcatacagtcttacaggctgttggggcttgtgttctttgcaattcacagacttcattaagatgtggtgcttgcatacgtagaccattcttatgttgtaaatgctgttacgaccatgtcatatcaacatcacataaattagtcttgtctgttaatccgtatgtttgcaatgctccaggttgtgatgtcacagatgtgactcaactttacttaggaggtatgagctattattgtaaatcacataaaccacccattagttttccattgtgtgctaatggacaagtttttggtttatataaaaatacatgtgttggtagcgataatgttactgactttaatgcaattgcaacatgtgactggacaaatgctggtgattacattttagctaacacctgtactgaaagactcaagctttttgcagcagaaacgctcaaagctactgaggagacatttaaactgtcttatggtattgctactgtacgtgaagtgctgtctgacagagaattacatctttcatgggaagttggtaaacctagaccaccacttaaccgaaattatgtctttactggttatcgtgtaactaaaaacagtaaagtacaaataggagagtacacctttgaaaaaggtgactatggtgatgctgttgtttaccgaggtacaacaacttacaaattaaatgttggtgattattttgtgctgacatcacatacagtaatgccattaagtgcacctacactagtgccacaagagcactatgttagaattactggcttatacccaacactcaatatctcagatgagttttctagcaatgttgcaaattatcaaaaggttggtatgcaaaagtattctacactccagggaccacctggtactggtaagagtcattttgctattggcctagctctctactacccttctgctcgcatagtgtatacagcttgctctcatgccgctgttgatgcactatgtgagaaggcattaaaatatttgcctatagataaatgtagtagaattatacctgcacgtgctcgtgtagagtgttttgataaattcaaagtgaattcaacattagaacagtatgtcttttgtactgtaaatgcattgcctgagacgacagcagatatagttgtctttgatgaaatttcaatggccacaaattatgatttgagtgttgtcaatgccagattacgtgctaagcactatgtgtacattggcgaccctgctcaattacctgcaccacgcacattgctaactaagggcacactagaaccagaatatttcaattcagtgtgtagacttatgaaaactataggtccagacatgttcctcggaacttgtcggcgttgtcctgctgaaattgttgacactgtgagtgctttggtttatgataataagcttaaagcacataaagacaaatcagctcaatgctttaaaatgttttataagggtgttatcacgcatgatgtttcatctgcaattaacaggccacaaataggcgtggtaagagaattccttacacgtaaccctgcttggagaaaagctgtctttatttcaccttataattcacagaatgctgtagcctcaaagattttgggactaccaactcaaactgttgattcatcacagggctcagaatatgactatgtcatattcactcaaaccactgaaacagctcactcttgtaatgtaaacagatttaatgttgctattaccagagcaaaagtaggcatactttgcataatgtctgatagagacctttatgacaagttgcaatttacaagtcttgaaattccacgtaggaatgtggcaactttacaagctgaaaatgtaacaggactctttaaagattgtagtaaggtaatcactgggttacatcctacacaggcacctacacacctcagtgttgacactaaattcaaaactgaaggtttatgtgttgacatacctggcatacctaaggacatgacctatagaagactcatctctatgatgggttttaaaatgaattatcaagttaatggttaccctaacatgtttatcacccgcgaagaagctataagacatgtacgtgcatggattggcttcgatgtcgaggggtgtcatgctactagagaagctgttggtaccaatttacctttacagctaggtttttctacaggtgttaacctagttgctgtacctacaggttatgttgatacacctaataatacagatttttccagagttagtgctaaaccaccgcctggagatcaatttaaacacctcataccacttatgtacaaaggacttccttggaatgtagtgcgtataaagattgtacaaatgttaagtgacacacttaaaaatctctctgacagagtcgtatttgtcttatgggcacatggctttgagttgacatctatgaagtattttgtgaaaataggacctgagcgcacctgttgtctatgtgatagacgtgccacatgcttttccactgcttcagacacttatgcctgttggcatcattctattggatttgattacgtctataatccgtttatgattgatgttcaacaatggggttttacaggtaacctacaaagcaaccatgatctgtattgtcaagtccatggtaatgcacatgtagctagttgtgatgcaatcatgactaggtgtctagctgtccacgagtgctttgttaagcgtgttgactggactattgaatatcctataattggtgatgaactgaagattaatgcggcttgtagaaaggttcaacacatggttgttaaagctgcattattagcagacaaattcccagttcttcacgacattggtaaccctaaagctattaagtgtgtacctcaagctgatgtagaatggaagttctatgatgcacagccttgtagtgacaaagcttataaaatagaagaattattctattcttatgccacacattctgacaaattcacagatggtgtatgcctattttggaattgcaatgtcgatagatatcctgctaattccattgtttgtagatttgacactagagtgctatctaaccttaacttgcctggttgtgatggtggcagtttgtatgtaaataaacatgcattccacacaccagcttttgataaaagtgcttttgttaatttaaaacaattaccatttttctattactctgacagtccatgtgagtctcatggaaaacaagtagtgtcagatatagattatgtaccactaaagtctgctacgtgtataacacgttgcaatttaggtggtgctgtctgtagacatcatgctaatgagtacagattgtatctcgatgcttataacatgatgatctcagctggctttagcttgtgggtttacaaacaatttgatacttataacctctggaacacttttacaagacttcagagtttagaaaatgtggcttttaatgttgtaaataagggacactttgatggacaacagggtgaagtaccagtttctatcattaataacactgtttacacaaaagttgatggtgttgatgtagaattgtttgaaaataaaacaacattacctgttaatgtagcatttgagctttgggctaagcgcaacattaaaccagtaccagaggtgaaaatactcaataatttgggtgtggacattgctgctaatactgtgatctgggactacaaaagagatgctccagcacatatatctactattggtgtttgttctatgactgacatagccaagaaaccaactgaaacgatttgtgcaccactcactgtcttttttgatggtagagttgatggtcaagtagacttatttagaaatgcccgtaatggtgttcttattacagaaggtagtgttaaaggtttacaaccatctgtgggtccc

SEQ ID NO: 13 - DNA, 5234 bp, Coronaviridae
  misc_feature 1..5234: note = F5 fragment polynucleotide sequence
  source 1..5234: mol_type = other DNA
gggtcccaaacaagctagtcttaatggagtcacattaattggagaagccgtaaaaacacagttcaattattataagaaagttgatggtgttgtccaacaattacctgaaacttactttactcagagtagaaatttacaagaatttaaacccaggagtcaaatggaaattgatttcttagaattagctatggatgaattcattgaacggtataaattagaaggctatgccttcgaacatatcgtttatggagattttagtcatagtcagttaggtggtttacatctactgattggactagctaaacgttttaaggaatcaccttttgaattagaagattttattcctatggacagtacagttaaaaactatttcataacagatgcgcaaacaggttcatctaagtgtgtgtgttctgttattgatttattacttgatgattttgttgaaataataaaatcccaagatttatctgtagtttctaaggttgtcaaagtgactattgactatacagaaatttcatttatgctttggtgtaaagatggccatgtagaaacattttacccaaaattacaatctagtcaagcgtggcaaccgggtgttgctatgcctaatctttacaaaatgcaaagaatgctattagaaaagtgtgaccttcaaaattatggtgatagtgcaacattacctaaaggcataatgatgaatgtcgcaaaatatactcaactgtgtcaatatttaaacacattaacattagctgtaccctataatatgagagttatacattttggtgctggttctgataaaggagttgcaccaggtacagctgttttaagacagtggttgcctacgggtacgctgcttgtcgattcagatcttaatgactttgtctctgatgcagattcaactttgattggtgattgtgcaactgtacatacagctaataaatgggatctcattattagtgatatgtacgaccctaagactaaaaatgttacaaaagaaaatgactctaaagagggttttttcacttacatttgtgggtttatacaacaaaagctagctcttggaggttccgtggctataaagataacagaacattcttggaatgctgatctttataagctcatgggacacttcgcatggtggacagcctttgttactaatgtgaatgcgtcatcatctgaagcatttttaattggatgtaattatcttggcaaaccacgcgaacaaatagatggttatgtcatgcatgcaaattacatattttggaggaatacaaatccaattcagttgtcttcctattctttatttgacatgagtaaatttccccttaaattaaggggtactgctgttatgtctttaaaagaaggtcaaatcaatgatatgattttatctcttcttagtaaaggtagacttataattagagaaaacaacagagttgttatttctagtgatgttcttgttaacaactaaacgaacaatgtttgtttttcttgttttattgccactagtctctagtcagtgtgttaatcttacaaccagaactcaattaccccctgcatacactaattctttcacacgtggtgtttattaccctgacaaagttttcagatcctcagttttacattcaactcaggacttgttcttacctttcttttccaatgttacttggttccatgctatacatgtctctgggaccaatggtactaagaggtttgataaccctgtcctaccatttaatgatggtgtttattttgcttccactgagaagtctaacataataagaggctggatttttggtactactttagattcgaagacccagtccctacttattgttaataacgctactaatgttgttattaaagtctgtgaatttcaattttgtaatgatccatttttgggtgtttattaccacaaaaacaacaaaagttggatggaaagtgagttcagagtttattctagtgcgaataattgcacttttgaatatgtctctcagccttttcttatggaccttgaaggaaaacagggtaatttcaaaaatcttagggaatttgtgtttaagaatattgatggttattttaaaatatattctaagcacacgcctattaatttagtgcgtgatctccctcagggtttttcggctttagaaccattggtagatttgccaataggtattaacatcactaggtttcaaactttacttgctttacatagaagttatttgactcctggtgattcttcttcaggttggacagctggtgctgcagcttattatgtgggttatcttcaacctaggacttttctattaaaatataatgaaaatggaaccattacagatgctgtagactgtgcacttgaccctctctcagaaacaaagtgtacgttgaaatccttcactgtagaaaaaggaatctatcaaacttctaactttagagtccaaccaacagaatctattgttagatttcctaatattacaaacttgtgcccttttggtgaagtttttaacgccaccagatttgcatctgtttatgcttggaacaggaagagaatcagcaactgtgttgctgattattctgtcctatataattccgcatcattttccacttttaagtgttatggagtgtctcctactaaattaaatgatctctgctttactaatgtctatgcagattcatttgtaattagaggtgatgaagtcagacaaatcgctccagggcaaactggaaagattgctgattataattataaattaccagatgattttacaggctgcgttatagcttggaattctaacaatcttgattctaaggttggtggtaattataattacctgtatagattgtttaggaagtctaatctcaaaccttttgagagagatatttcaactgaaatctatcaggccggtagcacaccttgtaatggtgttgaaggttttaattgttactttcctttacaatcatatggtttccaacccactaatggtgttggttaccaaccatacagagtagtagtactttcttttgaacttctacatgcaccagcaactgtttgtggacctaaaaagtctactaatttggttaaaaacaaatgtgtcaatttcaacttcaatggtttaacaggcacaggtgttcttactgagtctaacaaaaagtttctgcctttccaacaatttggcagagacattgctgacactactgatgctgtccgtgatccacagacacttgagattcttgacattacaccatgttcttttggtggtgtcagtgttataacaccaggaacaaatacttctaaccaggttgctgttctttatcaggatgttaactgcacagaagtccctgttgctattcatgcagatcaacttactcctacttggcgtgtttattctacaggttctaatgtttttcaaacacgtgcaggctgtttaataggggctgaacatgtcaacaactcatatgagtgtgacatacccattggtgcaggtatatgcgctagttatcagactcagactaattctcctcggcgggcacgtagtgtagctagtcaatccatcattgcctacactatgtcacttggtgcagaaaattcagttgcttactctaataactctattgccatacccacaaattttactattagtgttaccacagaaattctaccagtgtctatgaccaagacatcagtagattgtacaatgtacatttgtggtgattcaactgaatgcagcaatcttttgttgcaatatggcagtttttgtacacaattaaaccgtgctttaactggaatagctgttgaacaagacaaaaacacccaagaagtttttgcacaagtcaaacaaatttacaaaacaccaccaattaaagattttggtggttttaatttttcacaaatattaccagatccatcaaaaccaagcaagaggtcatttattgaagatctacttttcaacaaagtgacacttgcagatgctggcttcatcaaacaatatggtgattgccttggtgatattgctgctagagacctcatttgtgcacaaaagtttaacggccttactgttttgccacctttgctcacagatgaaatgattgctcaatacacttctgcactgttagcgggtacaatcacttctggttggacctttggtgcaggtgctgcattacaaataccatttgctatgcaaatggcttataggtttaatggtattggagttacacagaatgttctctatgagaaccaaaaattgattgccaaccaatttaatagtgctattggcaaaattcaagactcactttcttccacagcaagtgcacttggaaaacttcaagatgtggtcaaccaaaatgcacaagctttaaacacgcttgttaaacaacttagctccaattttggtgcaatttcaagtgttttaaatgatatcctttcacgtcttgacaaagttgaggctgaagtgcaaattgataggttgatcacaggcagacttcaaagtttgcagacatatgtgactcaacaattaattagagctgcagaaatcagagcttctgctaatcttgctgctactaaaatgtcagagtgtgtacttggacaatcaaaaagagttgatttttgtggaaagggctatcatcttatgtccttccctcagtcagcacctcatggtgtagtcttcttgcatgtgacttatgtccctgcacaagaaaagaacttcacaactgctcctgccatttgtcatgatggaaaagcacactttcctcgtgaaggtgtctttgtttcaaatggcacacactggtttgtaacacaaaggaatttttatgaaccacaaatcattactacagacaacacatttgtgtctggtaactgtgatgttgtaataggaattgtcaacaacacagtttatgatcctttgcaacctgaattagactcattcaaggaggagttagataaatattttaagaatcatacatcaccagatgttgatttaggtgacatctctggcattaatgcttcagttgtaaacattcaaaaagaaattgaccgcctcaatgaggttgccaagaatttaaatgaatctctcatcgatctccaagaacttggaaagtatgagcagtatataaaatggccatggtacatttggctaggttttatagctggcttgattgccatagtaatggtgacaattatgctttgctgtatgaccagttgctgtagttgtctcaagggctgttgttcttgtggatcc

SEQ ID NO: 14 - DNA, 4618 bp, Coronaviridae
  misc_feature 1..4618: note = F6 fragment polynucleotide sequence
  source 1..4618: mol_type = other DNA
ggatcctgctgcaaatttgatgaagacgactctgagccagtgctcaaaggagtcaaattacattacacataaacgaacttatggatttgtttatgagaatcttcacaattggaactgtaactttgaagcaaggtgaaatcaaggatgctactccttcagattttgttcgcgctactgcaacgataccgatacaagcctcactccctttcggatggcttattgttggcgttgcacttcttgctgtttttcagagcgcttccaaaatcataaccctcaaaaagagatggcaactagcactctccaagggtgttcactttgtttgcaacttgctgttgttgtttgtaacagtttactcacaccttttgctcgttgctgctggccttgaagccccttttctctatctttatgctttagtctacttcttgcagagtataaactttgtaagaataataatgaggctttggctttgctggaaatgccgttccaaaaacccattactttatgatgccaactattttctttgctggcatactaattgttacgactattgtataccttacaatagtgtaacttcttcaattgtcattacttcaggtgatggcacaacaagtcctatttctgaacatgactaccagattggtggttatactgaaaaatgggaatctggagtaaaagactgtgttgtattacacagttacttcacttcagactattaccagctgtactcaactcaattgagtacagacactggtgttgaacatgttaccttcttcatctacaataaaattgttgatgagcctgaagaacatgtccaaattcacacaatcgacggttcatccggagttgttaatccagtaatggaaccaatttatgatgaaccgacgacgactactagcgtgcctttgtaagcacaagctgatgagtacgaacttatgtactcattcgtttcggaagagacaggtacgttaatagttaatagcgtacttctttttcttgctttcgtggtattcttgctagttacactagccatccttactgcgcttcgattgtgtgcgtactgctgcaatattgttaacgtgagtcttgtaaaaccttctttttacgtttactctcgtgttaaaaatctgaattcttctagagttcctgatcttctggtctaaacgaactaaatattatattagtttttctgtttggaactttaattttagccatggcagattccaacggtactattaccgttgaagagcttaaaaagctccttgaacaatggaacctagtaataggtttcctattccttacatggatttgtcttctacaatttgcctatgccaacaggaataggtttttgtatataattaagttaattttcctctggctgttatggccagtaactttagcttgttttgtgcttgctgctgtttacagaataaattggatcaccggtggaattgctatcgcaatggcttgtcttgtaggcttgatgtggctcagctacttcattgcttctttcagactgtttgcgcgtacccgttccatgtggtcattcaatccagaaactaacattcttctcaacgtgccactccatggcactattctgaccagaccgcttctagaaagtgaactcgtaatcggagctgtgatccttcgtggacatcttcgtattgctggacaccatctaggacgctgtgacatcaaggacctgcctaaagaaatcactgttgctacatcacgaacgctttcttattacaaattgggagcttcgcagcgtgtagcaggtgactcaggttttgctgcatacagtcgctacaggattggcaactataaattaaacacagaccattccagtagcagtgacaatattgctttgcttgtacagtaagtgacaacagatgtttcatctcgttgactttcaggttactatagcagagatattactaattattatgaggacttttaaagtttccatttggaatcttgattacatcataaacctcataattaaaaatttatctaagtcactaactgagaataaatattctcaattagatgaagagcaaccaatggagattgattaaacgaacatgaaaattattcttttcttggcactgataacactcgctacttgtgagctttatcactaccaagagtgtgttagaggtacaacagtacttttaaaagaaccttgctcttctggaacatacgagggcaattcaccatttcatcctctagctgataacaaatttgcactgacttgctttagcactcaatttgcttttgcttgtcctgacggcgtaaaacacgtctatcagttacgtgccagatcagtttcacctaaactgttcatcagacaagaggaagttcaagaactttactctccaatttttcttattgttgcggcaatagtgtttataacactttgcttcacactcaaaagaaagacagaatgattgaactttcattaattgacttctatttgtgctttttagcctttctgctattccttgttttaattatgcttattatcttttggttctcacttgaactgcaagatcataatgaaacttgtcacgcctaaacgaacatgaaatttcttgttttcttaggaatcatcacaactgtagctgcatttcaccaagaatgtagtttacagtcatgtactcaacatcaaccatatgtagttgatgacccgtgtcctattcacttctattctaaatggtatattagagtaggagctagaaaatcagcacctttaattgaattgtgcgtggatgaggctggttctaaatcacccattcagtacatcgatatcggtaattatacagtttcctgtttaccttttacaattaattgccaggaacctaaattgggtagtcttgtagtgcgttgttcgttctatgaagactttttagagtatcatgacgttcgtgttgttttagatttcatctaaacgaacaaactaaaatgtctgataatggaccccaaaatcagcgaaatgcaccccgcattacgtttggtggaccctcagattcaactggcagtaaccagaatggagaacgcagtggggcgcgatcaaaacaacgtcggccccaaggtttacccaataatactgcgtcttggttcaccgctctcactcaacatggcaaggaagaccttaaattccctcgaggacaaggcgttccaattaacaccaatagcagtccagatgaccaaattggctactaccgaagagctaccagacgaattcgtggtggtgacggtaaaatgaaagatctcagtccaagatggtatttctactacctaggaactgggccagaagctggacttccctatggtgctaacaaagacggcatcatatgggttgcaactgagggagccttgaatacaccaaaagatcacattggcacccgcaatcctgctaacaatgctgcaatcgtgctacaacttcctcaaggaacaacattgccaaaaggcttctacgcagaagggagcagaggcggcagtcaagcctcttctcgttcctcatcacgtagtcgcaacagttcaagaaattcaactccaggcagcagtaggggaacttctcctgctagaatggctggcaatggcggtgatgctgctcttgctttgctgctgcttgacagattgaaccagcttgagagcaaaatgtctggtaaaggccaacaacaacaaggccaaactgtcactaagaaatctgctgctgaggcttctaagaagcctcggcaaaaacgtactgccactaaagcatacaatgtaacacaagctttcggcagacgtggtccagaacaaacccaaggaaattttggggaccaggaactaatcagacaaggaactgattacaaacattggccgcaaattgcacaatttgcccccagcgcttcagcgttcttcggaatgtcgcgcattggcatggaagtcacaccttcgggaacgtggttgacctacacaggtgccatcaaattggatgacaaagatccaaatttcaaagatcaagtcattttgctgaataagcatattgacgcatacaaaacattcccaccaacagagcctaaaaaggacaaaaagaagaaggctgatgaaactcaagccttaccgcagagacagaagaaacagcaaactgtgactcttcttcctgctgcagatttggatgatttctccaaacaattgcaacaatccatgagcagtgctgactcaactcaggcctaaactcatgcagaccacacaaggcagatgggctatataaacgttttcgcttttccgtttacgatatatagtctactcttgtgcagaatgaattctcgtaactacatagcacaagtagatgtagttaactttaatctcacatagcaatctttaatcagtgtgtaacattagggaggacttgaaagagccaccacattttcaccgaggccacgcggagtacgatcgagtgtacagtgaacaatgctagggagagctgcctatatggaagagccctaatgtgtaaaattaattttagtagtgctatccccatgtgattttaatagcttcttaggagaatgacaaaaaaaaaaaaaaaaaaaaaaaaagggtcggcatggcatctccacctcctcgcggtccg

SEQ ID NO: 15 - DNA, 29062 bp, Coronaviridae
  misc_feature 1..29062: note = SARS-CoV-2-3
  source 1..29062: mol_type = other DNA
attaaaggtttataccttcccaggtaacaaaccaaccaactttcgatctcttgtagatctgttctctaaacgaactttaaaatctgtgtggctgtcactcggctgcatgcttagtgcactcacgcagtataattaataactaattactgtcgttgacaggacacgagtaactcgtctatcttctgcaggctgcttacggtttcgtccgtgttgcagccgatcatcagcacatctaggtttcgtccgggtgtgaccgaaaggtaagatggagagccttgtccctggtttcaacgagaaaacacacgtccaactcagtttgcctgttttacaggttcgcgacgtgctcgtacgtggctttggagactccgtggaggaggtcttatcagaggcacgtcaacatcttaaagatggcacttgtggcttagtagaagttgaaaaaggcgttttgcctcaacttgaacagccctatgtgttcatcaaacgttcggatgctcgaactgcacctcatggtcatgttatggttgagctggtagcagaactcgaaggcattcagtacggtcgtagtggtgagacacttggtgtccttgtccctcatgtgggcgaaataccagtggcttaccgcaaggttcttcttcgtaagaacggtaataaaggagctggtggccatagttacggcgccgatctaaagtcatttgacttaggcgacgagcttggcactgatccttatgaagattttcaagaaaactggaacactaaacatagcagtggtgttacccgtgaactcatgcgtgagcttaacggaggggcatacactcgctatgtcgataacaacttctgtggccctgatggctaccctcttgagtgcattaaagaccttctagcacgtgctggtaaagcttcatgcactttgtccgaacaactggactttattgacactaagaggggtgtatactgctgccgtgaacatgagcatgaaattgcttggtacacggaacgttctgaaaagagctatgaattgcagacaccttttgaaattaaattggcaaagaaatttgacaccttcaatggggaatgtccaaattttgtatttcccttaaattccataatcaagactattcaaccaagggttgaaaagaaaaagcttgatggctttatgggtagaattcgatctgtctatccagttgcgtcaccaaatgaatgcaaccaaatgtgcctttcaactctcatgaagtgtgatcattgtggtgaaacttcatggcagacgggcgattttgttaaagccacttgcgaattttgtggcactgagaatttgactaaagaaggtgccactacttgtggttacttaccccaaaatgctgttgttaaaatttattgtccagcatgtcacaattcagaagtaggacctgagcatagtcttgccgaataccataatgaatctggcttgaaaaccattcttcgtaagggtggtcgcactattgcctttggaggctgtgtgttctcttatgttggttgccataacaagtgtgcctattgggttccacgtgctagcgctaacataggttgtaaccatacaggtgttgttggagaaggttccgaaggtcttaatgacaaccttcttgaaatactccaaaaagagaaagtcaacatcaatattgttggtgactttaaacttaatgaagagatcgccattattttggcatctttttctgcttccacaagtgcttttgtggaaactgtgaaaggtttggattataaagcattcaaacaaattgttgaatcctgtggtaattttaaagttacaaaaggaaaagctaaaaaaggtgcctggaatattggtgaacagaaatcaatactgagtcctctttatgcatttgcatcagaggctgctcgtgttgtacgatcaattttctcccgcactcttgaaactgctcaaaattctgtgcgtgttttacagaaggccgctataacaatactagatggaatttcacagtattcactgagactcattgatgctatgatgttcacatctgatttggctactaacaatctagttgtaatggcctacattacaggtggtgttgttcagttgacttcgcagtggctaactaacatctttggcactgtttatgaaaaactcaaacccgtccttgattggcttgaagagaagtttaaggaaggtgtagagtttcttagagacggttgggaaattgttaaatttatctcaacctgtgcttgtgaaattgtcggtggacaaattgtcacctgtgcaaaggaaattaaggagagtgttcagacattctttaagcttgtaaataaatttttggctttgtgtgctgactctatcattattggtggagctaaacttaaagccttgaatttaggtgaaacatttgtcacgcactcaaagggattgtacagaaagtgtgttaaatccagagaagaaactggcctactcatgcctctaaaagccccaaaagaaattatcttcttagagggagaaacacttcccacagaagtgttaacagaggaagttgtcttgaaaactggtgatttacaaccattagaacaacctactagtgaagctgttgaagctccattggttggtacaccagtttgtattaacgggcttatgttgctcgaaatcaaagacacagaaaagtactgtgcccttgcacctaatatgatggtaacaaacaataccttcacactcaaaggcggtgcaccaacaaaggttacttttggtgatgacactgtgatagaagtgcaaggttacaagagtgtgaatatcacttttgaacttgatgaaaggattgataaagtacttaatgagaagtgctctgcctatacagttgaactcggtacagaagtaaatgagttcgcctgtgttgtggcagatgctgtcataaaaactttgcaaccagtatctgaattacttacaccactgggcattgatttagatgagtggagtatggctacatactacttatttgatgagtctggtgagtttaaattggcttcacatatgtattgttctttctaccctccagatgaggatgaagaagaaggtgattgtgaagaagaagagtttgagccatcaactcaatatgagtatggtactgaagatgattaccaaggtaaacctttggaatttggtgccacttctgctgctcttcaacctgaagaagagcaagaagaagattggttagatgatgatagtcaacaaactgttggtcaacaagacggcagtgaggacaatcagacaactactattcaaacaattgttgaggttcaacctcaattagagatggaacttacaccagttgttcagactattgaagtgaatagttttagtggttatttaaaacttactgacaatgtatacattaaaaatgcagacattgtggaagaagctaaaaaggtaaaaccaacagtggttgttaatgcagccaatgtttaccttaaacatggaggaggtgttgcaggagccttaaataaggctactaacaatgccatgcaagttgaatctgatgattacatagctactaatggaccacttaaagtgggtggtagttgtgttttaagcggacacaatcttgctaaacactgtcttcatgttgtcggcccaaatgttaacaaaggtgaagacattcaacttcttaagagtgcttatgaaaattttaatcagcacgaagttctacttgcaccattattatcagctggtatttttggtgctgaccctatacattctttaagagtttgtgtagatactgttcgcacaaatgtctacttagctgtctttgataaaaatctctatgacaaacttgtttcaagctttttggaaatgaagagtgaaaagcaagttgaacaaaagatcgctgagattcctaaagaggaagttaagccatttataactgaaagtaaaccttcagttgaacagagaaaacaagatgataagaaaatcaaagcttgtgttgaagaagttacaacaactctggaagaaactaagttcctcacagaaaacttgttactttatattgacattaatggcaatcttcatccagattctgccactcttgttagtgacattgacatcactttcttaaagaaagatgctccatatatagtgggtgatgttgttcaagagggtgttttaactgctgtggttatacctactaaaaaggctggtggcactactgaaatgctagcgaaagctttgagaaaagtgccaacagacaattatataaccacttacccgggtcagggtttaaatggttacactgtagaggaggcaaagacagtgcttaaaaagtgtaaaagtgccttttacattctaccatctattatctctaatgagaagcaagaaattcttggaactgtttcttggaatttgcgagaaatgcttgcacatgcagaagaaacacgcaaattaatgcctgtctgtgtggaaactaaagccatagtttcaactatacagcgtaaatataagggtattaaaatacaagagggtgtggttgattatggtgctagattttacttttacaccagtaaaacaactgtagcgtcacttatcaacacacttaacgatctaaatgaaactcttgttacaatgccacttggctatgtaacacatggcttaaatttggaagaagctgctcggtatatgagatctctcaaagtgccagctacagtttctgtttcttcacctgatgctgttacagcgtataatggttatcttacttcttcttctaaaacacctgaagaacattttattgaaaccatctcacttgctggttcctataaagattggtcctattctggacaatctacacaactaggtatagaatttcttaagagaggtgataaaagtgtatattacactagtaatcctaccacattccacctagatggtgaagttatcacctttgacaatcttaagacacttctttctttgagagaagtgaggactattaaggtgtttacaacagtagacaacattaacctccacacgcaagttgtggacatgtcaatgacatatggacaacagtttggtccaacttatttggatggagctgatgttactaaaataaaacctcataattcacatgaaggtaaaacattttatgttttacctaatgatgacactctacgtgttgaggcttttgagtactaccacacaactgatcctagttttctgggtaggtacatgtcagcattaaatcacactaaaaagtggaaatacccacaagttaatggtttaacttctattaaatgggcagataacaactgttatcttgccactgcattgttaacactccaacaaatagagttgaagtttaatccacctgctctacaagatgcttattacagagcaagggctggtgaagctgctaacttttgtgcacttatcttagcctactgtaataagacagtaggtgagttaggtgatgttagagaaacaatgagttacttgtttcaacatgccaatttagattcttgcaaaagagtcttgaacgtggtgtgtaaaacttgtggacaacagcagacaacccttaagggtgtagaagctgttatgtacatgggcacactttcttatgaacaatttaagaaaggtgttcagataccttgtacgtgtggtaaacaagctacaaaatatctagtacaacaggagtcaccttttgttatgatgtcagcaccacctgctcagtatgaacttaagcatggtacatttacttgtgctagtgagtacactggtaattaccagtgtggtcactataaacatataacttctaaagaaactttgtattgcatagacggtgctttacttacaaagtcctcagaatacaaaggtcctattacggatgttttctacaaagaaaacagttacacaacaaccataaaaccagttacttataaattggatggtgttgtttgtacagaaattgaccctaagttggacaattattataagaaagacaattcttatttcacagagcaaccaattgatcttgtaccaaaccaaccatatccaaacgcaagcttcgataattttaagtttgtatgtgataatatcaaatttgctgatgatttaaaccagttaactggttataagaaacctgcttcaagagagcttaaagttacatttttccctgacttaaatggtgatgtggtggctattgattataaacactacacaccctcttttaagaaaggagctaaattgttacataaacctattgtttggcatgttaacaatgcaactaataaagccacgtataaaccaaatacctggtgtatacgttgtctttggagcacaaaaccagttgaaacatcaaattcgtttgatgtactgaagtcagaggacgcgcagggaatggataatcttgcctgcgaagatctaaaaccagtctctgaagaagtagtggaaaatcctaccatacagaaagacgttcttgagtgtaatgtgaaaactaccgaagttgtaggagacattatacttaaaccagcaaataatagtttaaaaattacagaagaggttggccacacagatctaatggctgcttatgtagacaattctagtcttactattaagaaacctaatgaattatctagagtattaggtttgaaaacccttgctactcatggtttagctgctgttaatagtgtcccttgggatactatagctaattatgctaagccttttcttaacaaagttgttagtacaactactaacatagttacacggtgtttaaaccgtgtttgtactaattatatgccttatttctttactttattgctacaattgtgtacttttactagaagtacaaattctagaattaaagcatctatgccgactactatagcaaagaatactgttaagagtgtcggtaaattttgtctagaggcttcatttaattatttgaagtcacctaatttttctaaactgataaatattataatttggtttttactattaagtgtttgcctaggttctttaatctactcaaccgctgctttaggtgttttaatgtctaatttaggcatgccttcttactgtactggttacagagaaggctatttgaactctactaatgtcactattgcaacctactgtactggttctataccttgtagtgtttgtcttagtggtttagattctttagacacctatccttctttagaaactatacaaattaccatttcatcttttaaatgggatttaactgcttttggcttagttgcagagtggtttttggcatatattcttttcactaggtttttctatgtacttggattggctgcaatcatgcaattgtttttcagctattttgcagtacattttattagtaattcttggcttatgtggttaataattaatcttgtacaaatggccccgatttcagctatggttagaatgtacatcttctttgcatcattttattatgtatggaaaagttatgtgcatgttgtagacggttgtaattcatcaacttgtatgatgtgttacaaacgtaatagagcaacaagagtcgaatgtacaactattgttaatggtgttagaaggtccttttatgtctatgctaatggaggtaaaggcttttgcaaactacacaattggaattgtgttaattgtgatacattctgtgctggtagtacatttattagtgatgaagttgcgagagacttgtcactacagtttaaaagaccaataaatcctactgaccagtcttcttacatcgttgatagtgttacagtgaagaatggttccatccatctttactttgataaagctggtcaaaagacttatgaaagacattctctctctcattttgttaacttagacaacctgagagctaataacactaaaggttcattgcctattaatgttatagtttttgatggtaaatcaaaatgtgaagaatcatctgcaaaatcagcgtctgtttactacagtcagcttatgtgtcaacctatactgttactagatcaggcattagtgtctgatgttggtgatagtgcggaagttgcagttaaaatgtttgatgcttacgttaatacgttttcatcaacttttaacgtaccaatggaaaaactcaaaacactagttgcaactgcagaagctgaacttgcaaagaatgtgtccttagacaatgtcttatctacttttatttcagcagctcggcaagggtttgttgattcagatgtagaaactaaagatgttgttgaatgtcttaaattgtcacatcaatctgacatagaagttactggcgatagttgtaataactatatgctcacctataacaaagttgaaaacatgacaccccgtgaccttggtgcttgtattgactgtagtgcgcgtcatattaatgcgcaggtagcaaaaagtcacaacattgctttgatatggaacgttaaagatttcatgtcattgtctgaacaactacgaaaacaaatacgtagtgctgctaaaaagaataacttaccttttaagttgacatgtgcaactactagacaagttgttaatgttgtaacaacaaagatagcacttaagggtggtaaaattgttaataattggttgaagcagttaattaaagttacacttgtgttcctttttgttgctgctattttctatttaataacacctgttcatgtcatgtctaaacatactgacttttcaagtgaaatcataggatacaaggctattgatggtggtgtcactcgtgacatagcatctacagatacttgttttgctaacaaacatgctgattttgacacatggtttagccagcgtggtggtagttatactaatgacaaagcttgcccattgattgctgcagtcataacaagagaagtgggttttgtcgtgcctggtttgcctggcacgatattacgcacaactaatggtgactttttgcatttcttacctagagtttttagtgcagttggtaacatctgttacacaccatcaaaacttatagagtacactgactttgcaacatcagcttgtgttttggctgctgaatgtacaatttttaaagatgcttctggtaagccagtaccatattgttatgataccaatgtactagaaggttctgttgcttatgaaagtttacgccctgacacacgttatgtgctcatggatggctctattattcaatttcctaacacctaccttgaaggttctgttagagtggtaacaacttttgattctgagtactgtaggcacggcacttgtgaaagatcagaagctggtgtttgtgtatctactagtggtagatgggtacttaacaatgattattacagatctttaccaggagttttctgtggtgtagatgctgtaaatttacttactaatatgtttacaccactaattcaacctattggtgctttggacatatcagcatctatagtagctggtggtattgtagctatcgtagtaacatgccttgcctactattttatgaggtttagaagagcttttggtgaatacagtcatgtagttgcctttaatactttactattccttatgtcattcactgtactctgtttaacaccagtttactcattcttacctggtgtttattctgttatttacttgtacttgacattttatcttactaatgatgtttcttttttagcacatattcagtggatggttatgttcacacctttagtacctttctggataacaattgcttatatcatttgtatttccacaaagcatttctattggttctttagtaattacctaaagagacgtgtagtctttaatggtgtttcctttagtacttttgaagaagctgcgctgtgcacctttttgttaaataaagaaatgtatctaaagttgcgtagtgatgtgctattacctcttacgcaatataatagatacttagctctttataataagtacaagtattttagtggagcaatggatacaactagctacagagaagctgcttgttgtcatctcgcaaaggctctcaatgacttcagtaactcaggttctgatgttctttaccaaccaccacaaacctctatcacctcagctgttttgcagagtggttttagaaaaatggcattcccatctggtaaagttgagggttgtatggtacaagtaacttgtggtacaactacacttaacggtctttggcttgatgacgtagtttactgtccaagacatgtgatctgcacctctgaagacatgcttaaccctaattatgaagatttactcattcgtaagtctaatcataatttcttggtacaggctggtaatgttcaactcagggttattggacattctatgcaaaattgtgtacttaagcttaaggttgatacagccaatcctaagacacctaagtataagtttgttcgcattcaaccaggacagactttttcagtgttagcttgttacaatggttcaccatctggtgtttaccaatgtgctatgaggcccaatttcactattaagggttcattccttaatggttcatgtggtagtgttggttttaacatagattatgactgtgtctctttttgttacatgcaccatatggaattaccaactggagttcatgctggcacagacttagaaggtaacttttatggaccttttgttgacaggcaaacagcacaagcagctggtacggacacaactattacagttaatgttttagcttggttgtacgctgctgttataaatggagacaggtggtttctcaatcgatttaccacaactcttaatgactttaaccttgtggctatgaagtacaattatgaacctctaacacaagaccatgttgacatactaggacctctttctgctcaaactggaattgccgttttagatatgtgtgcttcattaaaagaattactgcaaaatggtatgaatggacgtaccatattgggtagtgctttattagaagatgaatttacaccttttgatgttgttagacaatgctcaggtgttactttccaaagtgcagtgaaaagaacaatcaagggtacacaccactggttgttactcacaattttgacttcacttttagttttagtccagagtactcaatggtctttgttcttttttttgtatgaaaatgcctttttaccttttgctatgggtattattgctatgtctgcttttgcaatgatgtttgtcaaacataagcatgcatttctctgtttgtttttgttaccttctcttgccactgtagcttattttaatatggtctatatgcctgctagttgggtgatgcgtattatgacatggttggatatggttgatactagtttgtctggttttaagctaaaagactgtgttatgtatgcatcagctgtagtgttactaatccttatgacagcaagaactgtgtatgatgatggtgctaggagagtgtggacacttatgaatgtcttgacactcgtttataaagtttattatggtaatgctttagatcaagccatttccatgtgggctcttataatctctgttacttctaactactcaggtgtagttacaactgtcatgtttttggccagaggtattgtttttatgtgtgttgagtattgccctattttcttcataactggtaatacacttcagtgtataatgctagtttattgtttcttaggctatttttgtacttgttactttggcctcttttgtttactcaaccgctactttagactgactcttggtgtttatgattacttagtttctacacaggagtttagatatatgaattcacagggactactcccacccaagaatagcatagatgccttcaaactcaacattaaattgttgggtgttggtggcaaaccttgtatcaaagtagccactgtacagtctaaaatgtcagatgtaaagtgcacatcagtagtcttactctcagttttgcaacaactcagagtagaatcatcatctaaattgtgggctcaatgtgtccagttacacaatgacattctcttagctaaagatactactgaagcctttgaaaaaatggtttcactactttctgttttgctttccatgcagggtgctgtagacataaacaagctttgtgaagaaatgctggacaacagggcaaccttacaagctatagcctcagagtttagttcccttccatcatatgcagcttttgctactgctcaagaagcttatgagcaggctgttgctaatggtgattctgaagttgttcttaaaaagttgaagaagtctttgaatgtggctaaatctgaatttgaccgtgatgcagccatgcaacgtaagttggaaaagatggctgatcaagctatgacccaaatgtataaacaggctagatctgaggacaagagggcaaaagttactagtgctatgcagacaatgcttttcactatgcttagaaagttggataatgatgcactcaacaacattatcaacaatgcaagagatggttgtgttcccttgaacataatacctcttacaacagcagccaaactaatggttgtcataccagactataacacatataaaaatacgtgtgatggtacaacatttacttatgcatcagcattgtgggaaatccaacaggttgtagatgcagatagtaaaattgttcaacttagtgaaattagtatggacaattcacctaatttagcatggcctcttattgtaacagctttaagggccaattctgctgtcaaattacagaataatgagcttagtcctgttgcactacgacagatgtcttgtgctgccggtactacacaaactgcttgcactgatgacaatgcgttagcttactacaacacaacaaagggaggtaggtttgtacttgcactgttatccgatttacaggatttgaaatgggctagattccctaagagtgatggaactggtactatctatacagaactggaaccaccttgtaggtttgttacagacacacctaaaggtcctaaagtgaagtatttatactttattaaaggattaaacaacctaaatagaggtatggtacttggtagtttagctgccacagtacgtctacaagctggtaatgcaacagaagtgcctgccaattcaactgtattatctttctgtgcttttgctgtagatgctgctaaagcttacaaagattatctagctagtgggggacaaccaatcactaattgtgttaagatgttgtgtacacacactggtactggtcaggcaataacagttacaccggaagccaatatggatcaagaatcctttggtggtgcatcgtgttgtctgtactgccgttgccacatagatcatccaaatcctaaaggattttgtgacttaaaaggtaagtatgtacaaatacctacaacttgtgctaatgaccctgtgggttttacacttaaaaacacagtctgtaccgtctgcggtatgtggaaaggttatggctgtagttgtgatcaactccgcgaacccatgcttcagtcagctgatgcacaatcgtttttaaacgggtttgcggtgtaagtgcagcccgtcttacaccgtgcggcacaggcactagtactgatgtcgtatacagggcttttgacatctacaatgataaagtagctggttttgctaaattcctaaaaactaattgttgtcgcttccaagaaaaggacgaagatgacaatttaattgattcttactttgtagttaagagacacactttctctaactaccaacatgaagaaacaatttataatttacttaaggattgtccagctgttgctaaacatgacttctttaagtttagaatagacggtgacatggtaccacatatatcacgtcaacgtcttactaaatacacaatggcagacctcgtctatgctttaaggcattttgatgaaggtaattgtgacacattaaaagaaatacttgtcacatacaattgttgtgatgatgattatttcaataaaaaggactggtatgattttgtagaaaacccagatatattacgcgtatacgccaacttaggtgaacgtgtacgccaagctttgttaaaaacagtacaattctgtgatgccatgcgaaatgctggtattgttggtgtactgacattagataatcaagatctcaatggtaactggtatgatttcggtgatttcatacaaaccacgccaggtagtggagttcctgttgtagattcttattattcattgttaatgcctatattaaccttgaccagggctttaactgcagagtcacatgttgacactgacttaacaaagccttacattaagtgggatttgttaaaatatgacttcacggaagagaggttaaaactctttgaccgttattttaaatattgggatcagacataccacccaaattgtgttaactgtttggatgacagatgcattctgcattgtgcaaactttaatgttttattctctacagtgttcccacctacaagttttggaccactagtgagaaaaatatttgttgatggtgttccatttgtagtttcaactggataccacttcagagagctaggtgttgtacataatcaggatgtaaacttacatagctctagacttagttttaaggaattacttgtgtatgctgctgaccctgctatgcacgctgcttctggtaatctattactagataaacgcactacgtgcttttcagtagctgcacttactaacaatgttgcttttcaaactgtcaaacccggtaattttaacaaagacttctatgactttgctgtgtctaagggtttctttaaggaaggaagttctgttgaattaaaacacttcttctttgctcaggatggtaatgctgctatcagcgattatgactactatcgttataatctaccaacaatgtgtgatatcagacaactactatttgtagttgaagttgttgataagtactttgattgttacgatggtggctgtattaatgctaaccaagtcatcgtcaacaacctagacaaatcagctggttttccatttaataaatggggtaaggctagactttattatgattcaatgagttatgaggatcaagatgcacttttcgcatatacaaaacgtaatgtcatccctactataactcaaatgaatcttaagtatgccattagtgcaaagaatagagctcgcaccgtagctggtgtctctatctgtagtactatgaccaatagacagtttcatcaaaaattattgaaatcaatagccgccactagaggagctactgtagtaattggaacaagcaaattctatggtggttggcacaacatgttaaaaactgtttatagtgatgtagaaaaccctcaccttatgggttgggattatcctaaatgtgatagagccatgcctaacatgcttagaattatggcctcacttgttcttgctcgcaaacatacaacgtgttgtagcttgtcacaccgtttctatagattagctaatgagtgtgctcaagtattgagtgaaatggtcatgtgtggcggttcactatatgttaaaccaggtggaacctcatcaggagatgccacaactgcttatgctaatagtgtttttaacatttgtcaagctgtcacggccaatgttaatgcacttttatctactgatggtaacaaaattgccgataagtatgtccgcaatttacaacacagactttatgagtgtctctatagaaatagagatgttgacacagactttgtgaatgagttttacgcatatttgcgtaaacatttctcaatgatgatactctctgacgatgctgttgtgtgtttcaatagcacttatgcatctcaaggtctagtggctagcataaagaactttaagtcagttctttattatcaaaacaatgtttttatgtctgaagcaaaatgttggactgagactgaccttactaaaggacctcatgaattttgctctcaacatacaatgctagttaaacagggtgatgattatgtgtaccttccttacccagatccatcaagaatcctaggggccggctgttttgtagatgatatcgtaaaaacagatggtacacttatgattgaacggttcgtgtctttagctatagatgcttacccacttactaaacatcctaatcaggagtatgctgatgtctttcatttgtacttacaatacataagaaagctacatgatgagttaacaggacacatgttagacatgtattctgttatgcttactaatgataacacttcaaggtattgggaacctgagttttatgaggctatgtacacaccgcatacagtcttacaggctgttggggcttgtgttctttgcaattcacagacttcattaagatgtggtgcttgcatacgtagaccattcttatgttgtaaatgctgttacgaccatgtcatatcaacatcacataaattagtcttgtctgttaatccgtatgtttgcaatgctccaggttgtgatgtcacagatgtgactcaactttacttaggaggtatgagctattattgtaaatcacataaaccacccattagttttccattgtgtgctaatggacaagtttttggtttatataaaaatacatgtgttggtagcgataatgttactgactttaatgcaattgcaacatgtgactggacaaatgctggtgattacattttagctaacacctgtactgaaagactcaagctttttgcagcagaaacgctcaaagctactgaggagacatttaaactgtcttatggtattgctactgtacgtgaagtgctgtctgacagagaattacatctttcatgggaagttggtaaacctagaccaccacttaaccgaaattatgtctttactggttatcgtgtaactaaaaacagtaaagtacaaataggagagtacacctttgaaaaaggtgactatggtgatgctgttgtttaccgaggtacaacaacttacaaattaaatgttggtgattattttgtgctgacatcacatacagtaatgccattaagtgcacctacactagtgccacaagagcactatgttagaattactggcttatacccaacactcaatatctcagatgagttttctagcaatgttgcaaattatcaaaaggttggtatgcaaaagtattctacactccagggaccacctggtactggtaagagtcattttgctattggcctagctctctactacccttctgctcgcatagtgtatacagcttgctctcatgccgctgttgatgcactatgtgagaaggcattaaaatatttgcctatagataaatgtagtagaattatacctgcacgtgctcgtgtagagtgttttgataaattcaaagtgaattcaacattagaacagtatgtcttttgtactgtaaatgcattgcctgagacgacagcagatatagttgtctttgatgaaatttcaatggccacaaattatgatttgagtgttgtcaatgccagattacgtgctaagcactatgtgtacattggcgaccctgctcaattacctgcaccacgcacattgctaactaagggcacactagaaccagaatatttcaattcagtgtgtagacttatgaaaactataggtccagacatgttcctcggaacttgtcggcgttgtcctgctgaaattgttgacactgtgagtgctttggtttatgataataagcttaaagcacataaagacaaatcagctcaatgctttaaaatgttttataagggtgttatcacgcatgatgtttcatctgcaattaacaggccacaaataggcgtggtaagagaattccttacacgtaaccctgcttggagaaaagctgtctttatttcaccttataattcacagaatgctgtagcctcaaagattttgggactaccaactcaaactgttgattcatcacagggctcagaatatgactatgtcatattcactcaaaccactgaaacagctcactcttgtaatgtaaacagatttaatgttgctattaccagagcaaaagtaggcatactttgcataatgtctgatagagacctttatgacaagttgcaatttacaagtcttgaaattccacgtaggaatgtggcaactttacaagctgaaaatgtaacaggactctttaaagattgtagtaaggtaatcactgggttacatcctacacaggcacctacacacctcagtgttgacactaaattcaaaactgaaggtttatgtgttgacatacctggcatacctaaggacatgacctatagaagactcatctctatgatgggttttaaaatgaattatcaagttaatggttaccctaacatgtttatcacccgcgaagaagctataagacatgtacgtgcatggattggcttcgatgtcgaggggtgtcatgctactagagaagctgttggtaccaatttacctttacagctaggtttttctacaggtgttaacctagttgctgtacctacaggttatgttgatacacctaataatacagatttttccagagttagtgctaaaccaccgcctggagatcaatttaaacacctcataccacttatgtacaaaggacttccttggaatgtagtgcgtataaagattgtacaaatgttaagtgacacacttaaaaatctctctgacagagtcgtatttgtcttatgggcacatggctttgagttgacatctatgaagtattttgtgaaaataggacctgagcgcacctgttgtctatgtgatagacgtgccacatgcttttccactgcttcagacacttatgcctgttggcatcattctattggatttgattacgtctataatccgtttatgattgatgttcaacaatggggttttacaggtaacctacaaagcaaccatgatctgtattgtcaagtccatggtaatgcacatgtagctagttgtgatgcaatcatgactaggtgtctagctgtccacgagtgctttgttaagcgtgttgactggactattgaatatcctataattggtgatgaactgaagattaatgcggcttgtagaaaggttcaacacatggttgttaaagctgcattattagcagacaaattcccagttcttcacgacattggtaaccctaaagctattaagtgtgtacctcaagctgatgtagaatggaagttctatgatgcacagccttgtagtgacaaagcttataaaatagaagaattattctattcttatgccacacattctgacaaattcacagatggtgtatgcctattttggaattgcaatgtcgatagatatcctgctaattccattgtttgtagatttgacactagagtgctatctaaccttaacttgcctggttgtgatggtggcagtttgtatgtaaataaacatgcattccacacaccagcttttgataaaagtgcttttgttaatttaaaacaattaccatttttctattactctgacagtccatgtgagtctcatggaaaacaagtagtgtcagatatagattatgtaccactaaagtctgctacgtgtataacacgttgcaatttaggtggtgctgtctgtagacatcatgctaatgagtacagattgtatctcgatgcttataacatgatgatctcagctggctttagcttgtgggtttacaaacaatttgatacttataacctctggaacacttttacaagacttcagagtttagaaaatgtggcttttaatgttgtaaataagggacactttgatggacaacagggtgaagtaccagtttctatcattaataacactgtttacacaaaagttgatggtgttgatgtagaattgtttgaaaataaaacaacattacctgttaatgtagcatttgagctttgggctaagcgcaacattaaaccagtaccagaggtgaaaatactcaataatttgggtgtggacattgctgctaatactgtgatctgggactacaaaagagatgctccagcacatatatctactattggtgtttgttctatgactgacatagccaagaaaccaactgaaacgatttgtgcaccactcactgtcttttttgatggtagagttgatggtcaagtagacttatttagaaatgcccgtaatggtgttcttattacagaaggtagtgttaaaggtttacaaccatctgtgggtcccaaacaagctagtcttaatggagtcacattaattggagaagccgtaaaaacacagttcaattattataagaaagttgatggtgttgtccaacaattacctgaaacttactttactcagagtagaaatttacaagaatttaaacccaggagtcaaatggaaattgatttcttagaattagctatggatgaattcattgaacggtataaattagaaggctatgccttcgaacatatcgtttatggagattttagtcatagtcagttaggtggtttacatctactgattggactagctaaacgttttaaggaatcaccttttgaattagaagattttattcctatggacagtacagttaaaaactatttcataacagatgcgcaaacaggttcatctaagtgtgtgtgttctgttattgatttattacttgatgattttgttgaaataataaaatcccaagatttatctgtagtttctaaggttgtcaaagtgactattgactatacagaaatttcatttatgctttggtgtaaagatggccatgtagaaacattttacccaaaattacaatctagtcaagcgtggcaaccgggtgttgctatgcctaatctttacaaaatgcaaagaatgctattagaaaagtgtgaccttcaaaattatggtgatagtgcaacattacctaaaggcataatgatgaatgtcgcaaaatatactcaactgtgtcaatatttaaacacattaacattagctgtaccctataatatgagagttatacattttggtgctggttctgataaaggagttgcaccaggtacagctgttttaagacagtggttgcctacgggtacgctgcttgtcgattcagatcttaatgactttgtctctgatgcagattcaactttgattggtgattgtgcaactgtacatacagctaataaatgggatctcattattagtgatatgtacgaccctaagactaaaaatgttacaaaagaaaatgactctaaagagggttttttcacttacatttgtgggtttatacaacaaaagctagctcttggaggttccgtggctataaagataacagaacattcttggaatgctgatctttataagctcatgggacacttcgcatggtggacagcctttgttactaatgtgaatgcgtcatcatctgaagcatttttaattggatgtaattatcttggcaaaccacgcgaacaaatagatggttatgtcatgcatgcaaattacatattttggaggaatacaaatccaattcagttgtcttcctattctttatttgacatgagtaaatttccccttaaattaaggggtactgctgttatgtctttaaaagaaggtcaaatcaatgatatgattttatctcttcttagtaaaggtagacttataattagagaaaacaacagagttgttatttctagtgatgttcttgttaacaactaaacgaacaatgtttgtttttcttgttttattgccactagtctctagtcagtgtgttaatcttacaaccagaactcaattaccccctgcatacactaattctttcacacgtggtgtttattaccctgacaaagttttcagatcctcagttttacattcaactcaggacttgttcttacctttcttttccaatgttacttggttccatgctatacatgtctctgggaccaatggtactaagaggtttgataaccctgtcctaccatttaatgatggtgtttattttgcttccactgagaagtctaacataataagaggctggatttttggtactactttagattcgaagacccagtccctacttattgttaataacgctactaatgttgttattaaagtctgtgaatttcaattttgtaatgatccatttttgggtgtttattaccacaaaaacaacaaaagttggatggaaagtgagttcagagtttattctagtgcgaataattgcacttttgaatatgtctctcagccttttcttatggaccttgaaggaaaacagggtaatttcaaaaatcttagggaatttgtgtttaagaatattgatggttattttaaaatatattctaagcacacgcctattaatttagtgcgtgatctccctcagggtttttcggctttagaaccattggtagatttgccaataggtattaacatcactaggtttcaaactttacttgctttacatagaagttatttgactcctggtgattcttcttcaggttggacagctggtgctgcagcttattatgtgggttatcttcaacctaggacttttctattaaaatataatgaaaatggaaccattacagatgctgtagactgtgcacttgaccctctctcagaaacaaagtgtacgttgaaatccttcactgtagaaaaaggaatctatcaaacttctaactttagagtccaaccaacagaatctattgttagatttcctaatattacaaacttgtgcccttttggtgaagtttttaacgccaccagatttgcatctgtttatgcttggaacaggaagagaatcagcaactgtgttgctgattattctgtcctatataattccgcatcattttccacttttaagtgttatggagtgtctcctactaaattaaatgatctctgctttactaatgtctatgcagattcatttgtaattagaggtgatgaagtcagacaaatcgctccagggcaaactggaaagattgctgattataattataaattaccagatgattttacaggctgcgttatagcttggaattctaacaatcttgattctaaggttggtggtaattataattacctgtatagattgtttaggaagtctaatctcaaaccttttgagagagatatttcaactgaaatctatcaggccggtagcacaccttgtaatggtgttgaaggttttaattgttactttcctttacaatcatatggtttccaacccactaatggtgttggttaccaaccatacagagtagtagtactttcttttgaacttctacatgcaccagcaactgtttgtggacctaaaaagtctactaatttggttaaaaacaaatgtgtcaatttcaacttcaatggtttaacaggcacaggtgttcttactgagtctaacaaaaagtttctgcctttccaacaatttggcagagacattgctgacactactgatgctgtccgtgatccacagacacttgagattcttgacattacaccatgttcttttggtggtgtcagtgttataacaccaggaacaaatacttctaaccaggttgctgttctttatcaggatgttaactgcacagaagtccctgttgctattcatgcagatcaacttactcctacttggcgtgtttattctacaggttctaatgtttttcaaacacgtgcaggctgtttaataggggctgaacatgtcaacaactcatatgagtgtgacatacccattggtgcaggtatatgcgctagttatcagactcagactaattctcctcggcgggcacgtagtgtagctagtcaatccatcattgcctacactatgtcacttggtgcagaaaattcagttgcttactctaataactctattgccatacccacaaattttactattagtgttaccacagaaattctaccagtgtctatgaccaagacatcagtagattgtacaatgtacatttgtggtgattcaactgaatgcagcaatcttttgttgcaatatggcagtttttgtacacaattaaaccgtgctttaactggaatagctgttgaacaagacaaaaacacccaagaagtttttgcacaagtcaaacaaatttacaaaacaccaccaattaaagattttggtggttttaatttttcacaaatattaccagatccatcaaaaccaagcaagaggtcatttattgaagatctacttttcaacaaagtgacacttgcagatgctggcttcatcaaacaatatggtgattgccttggtgatattgctgctagagacctcatttgtgcacaaaagtttaacggccttactgttttgccacctttgctcacagatgaaatgattgctcaatacacttctgcactgttagcgggtacaatcacttctggttggacctttggtgcaggtgctgcattacaaataccatttgctatgcaaatggcttataggtttaatggtattggagttacacagaatgttctctatgagaaccaaaaattgattgccaaccaatttaatagtgctattggcaaaattcaagactcactttcttccacagcaagtgcacttggaaaacttcaagatgtggtcaaccaaaatgcacaagctttaaacacgcttgttaaacaacttagctccaattttggtgcaatttcaagtgttttaaatgatatcctttcacgtcttgacaaagttgaggctgaagtgcaaattgataggttgatcacaggcagacttcaaagtttgcagacatatgtgactcaacaattaattagagctgcagaaatcagagcttctgctaatcttgctgctactaaaatgtcagagtgtgtacttggacaatcaaaaagagttgatttttgtggaaagggctatcatcttatgtccttccctcagtcagcacctcatggtgtagtcttcttgcatgtgacttatgtccctgcacaagaaaagaacttcacaactgctcctgccatttgtcatgatggaaaagcacactttcctcgtgaaggtgtctttgtttcaaatggcacacactggtttgtaacacaaaggaatttttatgaaccacaaatcattactacagacaacacatttgtgtctggtaactgtgatgttgtaataggaattgtcaacaacacagtttatgatcctttgcaacctgaattagactcattcaaggaggagttagataaatattttaagaatcatacatcaccagatgttgatttaggtgacatctctggcattaatgcttcagttgtaaacattcaaaaagaaattgaccgcctcaatgaggttgccaagaatttaaatgaatctctcatcgatctccaagaacttggaaagtatgagcagtatataaaatggccatggtacatttggctaggttttatagctggcttgattgccatagtaatggtgacaattatgctttgctgtatgaccagttgctgtagttgtctcaagggctgttgttcttgtggatcctgctgcaaatttgatgaagacgactctgagccagtgctcaaaggagtcaaattacattacacataagcgtgcctttgtaagcacaagctgatgagtacgaacttatgtactcattcgtttcggaagagacaggtacgttaatagttaatagcgtacttctttttcttgctttcgtggtattcttgctagttacactagccatccttactgcgcttcgattgtgtgcgtactgctgcaatattgttaacgtgagtcttgtaaaaccttctttttacgtttactctcgtgttaaaaatctgaattcttctagagttcctgatcttctggtctaaacgaactaaatattatattagtttttctgtttggaactttaattttagccatggcagattccaacggtactattaccgttgaagagcttaaaaagctccttgaacaatggaacctagtaataggtttcctattccttacatggatttgtcttctacaatttgcctatgccaacaggaataggtttttgtatataattaagttaattttcctctggctgttatggccagtaactttagcttgttttgtgcttgctgctgtttacagaataaattggatcaccggtggaattgctatcgcaatggcttgtcttgtaggcttgatgtggctcagctacttcattgcttctttcagactgtttgcgcgtacccgttccatgtggtcattcaatccagaaactaacattcttctcaacgtgccactccatggcactattctgaccagaccgcttctagaaagtgaactcgtaatcggagctgtgatccttcgtggacatcttcgtattgctggacaccatctaggacgctgtgacatcaaggacctgcctaaagaaatcactgttgctacatcacgaacgctttcttattacaaattgggagcttcgcagcgtgtagcaggtgactcaggttttgctgcatacagtcgctacaggattggcaactataaattaaacacagaccattccagtagcagtgacaatattgctttgcttgtacagtaagtgacaacagatgtttcatctcgttgactttcaggttactatagcagagatattactaattattatgaggacttttaaagtttccatttggaatcttgattacatcataaacctcataattaaaaatttatctaagtcactaactgagaataaatattctcaattagatgaagagcaaccaatggagattgattaaacgaacatgaaaattattcttttcttggcactgataacactcgctacttgtgagctttatcactaccaagagtgtgttagaggtacaacagtacttttaaaagaaccttgctcttctggaacatacgagggcaattcaccatttcatcctctagctgataacaaatttgcactgacttgctttagcactcaatttgcttttgcttgtcctgacggcgtaaaacacgtctatcagttacgtgccagatcagtttcacctaaactgttcatcagacaagaggaagttcaagaactttactctccaatttttcttattgttgcggcaatagtgtttataacactttgcttcacactcaaaagaaagacagaatgattgaactttcattaattgacttctatttgtgctttttagcctttctgctattccttgttttaattatgcttattatcttttggttctcacttgaactgcaagatcataatgaaacttgtcacgcctaaacgaacatgaaatttcttgttttcttaggaatcatcacaactgtagctgcatttcaccaagaatgtagtttacagtcatgtactcaacatcaaccatatgtagttgatgacccgtgtcctattcacttctattctaaatggtatattagagtaggagctagaaaatcagcacctttaattgaattgtgcgtggatgaggctggttctaaatcacccattcagtacatcgatatcggtaattatacagtttcctgtttaccttttacaattaattgccaggaacctaaattgggtagtcttgtagtgcgttgttcgttctatgaagactttttagagtatcatgacgttcgtgttgttttagatttcatctaaacgaacaaactaaaatgtctgataatggaccccaaaatcagcgaaatgcaccccgcattacgtttggtggaccctcagattcaactggcagtaaccagaatggagaacgcagtggggcgcgatcaaaacaacgtcggccccaaggtttacccaataatactgcgtcttggttcaccgctctcactcaacatggcaaggaagaccttaaattccctcgaggacaaggcgttccaattaacaccaatagcagtccagatgaccaaattggctactaccgaagagctaccagacgaattcgtggtggtgacggtaaaatgaaagatctcagtccaagatggtatttctactacctaggaactgggccagaagctggacttccctatggtgctaacaaagacggcatcatatgggttgcaactgagggagccttgaatacaccaaaagatcacattggcacccgcaatcctgctaacaatgctgcaatcgtgctacaacttcctcaaggaacaacattgccaaaaggcttctacgcagaagggagcagaggcggcagtcaagcctcttctcgttcctcatcacgtagtcgcaacagttcaagaaattcaactccaggcagcagtaggggaacttctcctgctagaatggctggcaatggcggtgatgctgctcttgctttgctgctgcttgacagattgaaccagcttgagagcaaaatgtctggtaaaggccaacaacaacaaggccaaactgtcactaagaaatctgctgctgaggcttctaagaagcctcggcaaaaacgtactgccactaaagcatacaatgtaacacaagctttcggcagacgtggtccagaacaaacccaaggaaattttggggaccaggaactaatcagacaaggaactgattacaaacattggccgcaaattgcacaatttgcccccagcgcttcagcgttcttcggaatgtcgcgcattggcatggaagtcacaccttcgggaacgtggttgacctacacagctgccatcaaattggatgacaaagatccaaatttcaaagatcaagtcattttgctgaataagcatattgacgcatacaaaacattcccaccaacagagcctaaaaaggacaaaaagaagaaggctgatgaaactcaagccttaccgcagagacagaagaaacagcaaactgtgactcttcttcctgctgcagatttggatgatttctccaaacaattgcaacaatccatgagcagtgctgactcaactcaggcctaaactcatgcagaccacacaaggcagatgggctatataaacgttttcgcttttccgtttacgatatatagtctactcttgtgcagaatgaattctcgtaactacatagcacaagtagatgtagttaactttaatctcacatagcaatctttaatcagtgtgtaacattagggaggacttgaaagagccaccacattttcaccgaggccacgcggagtacgatcgagtgtacagtgaacaatgctagggagagctgcctatatggaagagccctaatgtgtaaaattaattttagtagtgctatccccatgtgattttaatagcttcttaaaaaaaaaaaaaaaaaaaaaaaaa

SEQ ID NO: 16 - DNA, 29668 bp, Coronaviridae
  misc_feature 1..29668: note = SARS-CoV-2-E
  source 1..29668: mol_type = other DNA
attaaaggtttataccttcccaggtaacaaaccaaccaactttcgatctcttgtagatctgttctctaaacgaactttaaaatctgtgtggctgtcactcggctgcatgcttagtgcactcacgcagtataattaataactaattactgtcgttgacaggacacgagtaactcgtctatcttctgcaggctgcttacggtttcgtccgtgttgcagccgatcatcagcacatctaggtttcgtccgggtgtgaccgaaaggtaagatggagagccttgtccctggtttcaacgagaaaacacacgtccaactcagtttgcctgttttacaggttcgcgacgtgctcgtacgtggctttggagactccgtggaggaggtcttatcagaggcacgtcaacatcttaaagatggcacttgtggcttagtagaagttgaaaaaggcgttttgcctcaacttgaacagccctatgtgttcatcaaacgttcggatgctcgaactgcacctcatggtcatgttatggttgagctggtagcagaactcgaaggcattcagtacggtcgtagtggtgagacacttggtgtccttgtccctcatgtgggcgaaataccagtggcttaccgcaaggttcttcttcgtaagaacggtaataaaggagctggtggccatagttacggcgccgatctaaagtcatttgacttaggcgacgagcttggcactgatccttatgaagattttcaagaaaactggaacactaaacatagcagtggtgttacccgtgaactcatgcgtgagcttaacggaggggcatacactcgctatgtcgataacaacttctgtggccctgatggctaccctcttgagtgcattaaagaccttctagcacgtgctggtaaagcttcatgcactttgtccgaacaactggactttattgacactaagaggggtgtatactgctgccgtgaacatgagcatgaaattgcttggtacacggaacgttctgaaaagagctatgaattgcagacaccttttgaaattaaattggcaaagaaatttgacaccttcaatggggaatgtccaaattttgtatttcccttaaattccataatcaagactattcaaccaagggttgaaaagaaaaagcttgatggctttatgggtagaattcgatctgtctatccagttgcgtcaccaaatgaatgcaaccaaatgtgcctttcaactctcatgaagtgtgatcattgtggtgaaacttcatggcagacgggcgattttgttaaagccacttgcgaattttgtggcactgagaatttgactaaagaaggtgccactacttgtggttacttaccccaaaatgctgttgttaaaatttattgtccagcatgtcacaattcagaagtaggacctgagcatagtcttgccgaataccataatgaatctggcttgaaaaccattcttcgtaagggtggtcgcactattgcctttggaggctgtgtgttctcttatgttggttgccataacaagtgtgcctattgggttccacgtgctagcgctaacataggttgtaaccatacaggtgttgttggagaaggttccgaaggtcttaatgacaaccttcttgaaatactccaaaaagagaaagtcaacatcaatattgttggtgactttaaacttaatgaagagatcgccattattttggcatctttttctgcttccacaagtgcttttgtggaaactgtgaaaggtttggattataaagcattcaaacaaattgttgaatcctgtggtaattttaaagttacaaaaggaaaagctaaaaaaggtgcctggaatattggtgaacagaaatcaatactgagtcctctttatgcatttgcatcagaggctgctcgtgttgtacgatcaattttctcccgcactcttgaaactgctcaaaattctgtgcgtgttttacagaaggccgctataacaatactagatggaatttcacagtattcactgagactcattgatgctatgatgttcacatctgatttggctactaacaatctagttgtaatggcctacattacaggtggtgttgttcagttgacttcgcagtggctaactaacatctttggcactgtttatgaaaaactcaaacccgtccttgattggcttgaagagaagtttaaggaaggtgtagagtttcttagagacggttgggaaattgttaaatttatctcaacctgtgcttgtgaaattgtcggtggacaaattgtcacctgtgcaaaggaaattaaggagagtgttcagacattctttaagcttgtaaataaatttttggctttgtgtgctgactctatcattattggtggagctaaacttaaagccttgaatttaggtgaaacatttgtcacgcactcaaagggattgtacagaaagtgtgttaaatccagagaagaaactggcctactcatgcctctaaaagccccaaaagaaattatcttcttagagggagaaacacttcccacagaagtgttaacagaggaagttgtcttgaaaactggtgatttacaaccattagaacaacctactagtgaagctgttgaagctccattggttggtacaccagtttgtattaacgggcttatgttgctcgaaatcaaagacacagaaaagtactgtgcccttgcacctaatatgatggtaacaaacaataccttcacactcaaaggcggtgcaccaacaaaggttacttttggtgatgacactgtgatagaagtgcaaggttacaagagtgtgaatatcacttttgaacttgatgaaaggattgataaagtacttaatgagaagtgctctgcctatacagttgaactcggtacagaagtaaatgagttcgcctgtgttgtggcagatgctgtcataaaaactttgcaaccagtatctgaattacttacaccactgggcattgatttagatgagtggagtatggctacatactacttatttgatgagtctggtgagtttaaattggcttcacatatgtattgttctttctaccctccagatgaggatgaagaagaaggtgattgtgaagaagaagagtttgagccatcaactcaatatgagtatggtactgaagatgattaccaaggtaaacctttggaatttggtgccacttctgctgctcttcaacctgaagaagagcaagaagaagattggttagatgatgatagtcaacaaactgttggtcaacaagacggcagtgaggacaatcagacaactactattcaaacaattgttgaggttcaacctcaattagagatggaacttacaccagttgttcagactattgaagtgaatagttttagtggttatttaaaacttactgacaatgtatacattaaaaatgcagacattgtggaagaagctaaaaaggtaaaaccaacagtggttgttaatgcagccaatgtttaccttaaacatggaggaggtgttgcaggagccttaaataaggctactaacaatgccatgcaagttgaatctgatgattacatagctactaatggaccacttaaagtgggtggtagttgtgttttaagcggacacaatcttgctaaacactgtcttcatgttgtcggcccaaatgttaacaaaggtgaagacattcaacttcttaagagtgcttatgaaaattttaatcagcacgaagttctacttgcaccattattatcagctggtatttttggtgctgaccctatacattctttaagagtttgtgtagatactgttcgcacaaatgtctacttagctgtctttgataaaaatctctatgacaaacttgtttcaagctttttggaaatgaagagtgaaaagcaagttgaacaaaagatcgctgagattcctaaagaggaagttaagccatttataactgaaagtaaaccttcagttgaacagagaaaacaagatgataagaaaatcaaagcttgtgttgaagaagttacaacaactctggaagaaactaagttcctcacagaaaacttgttactttatattgacattaatggcaatcttcatccagattctgccactcttgttagtgacattgacatcactttcttaaagaaagatgctccatatatagtgggtgatgttgttcaagagggtgttttaactgctgtggttatacctactaaaaaggctggtggcactactgaaatgctagcgaaagctttgagaaaagtgccaacagacaattatataaccacttacccgggtcagggtttaaatggttacactgtagaggaggcaaagacagtgcttaaaaagtgtaaaagtgccttttacattctaccatctattatctctaatgagaagcaagaaattcttggaactgtttcttggaatttgcgagaaatgcttgcacatgcagaagaaacacgcaaattaatgcctgtctgtgtggaaactaaagccatagtttcaactatacagcgtaaatataagggtattaaaatacaagagggtgtggttgattatggtgctagattttacttttacaccagtaaaacaactgtagcgtcacttatcaacacacttaacgatctaaatgaaactcttgttacaatgccacttggctatgtaacacatggcttaaatttggaagaagctgctcggtatatgagatctctcaaagtgccagctacagtttctgtttcttcacctgatgctgttacagcgtataatggttatcttacttcttcttctaaaacacctgaagaacattttattgaaaccatctcacttgctggttcctataaagattggtcctattctggacaatctacacaactaggtatagaatttcttaagagaggtgataaaagtgtatattacactagtaatcctaccacattccacctagatggtgaagttatcacctttgacaatcttaagacacttctttctttgagagaagtgaggactattaaggtgtttacaacagtagacaacattaacctccacacgcaagttgtggacatgtcaatgacatatggacaacagtttggtccaacttatttggatggagctgatgttactaaaataaaacctcataattcacatgaaggtaaaacattttatgttttacctaatgatgacactctacgtgttgaggcttttgagtactaccacacaactgatcctagttttctgggtaggtacatgtcagcattaaatcacactaaaaagtggaaatacccacaagttaatggtttaacttctattaaatgggcagataacaactgttatcttgccactgcattgttaacactccaacaaatagagttgaagtttaatccacctgctctacaagatgcttattacagagcaagggctggtgaagctgctaacttttgtgcacttatcttagcctactgtaataagacagtaggtgagttaggtgatgttagagaaacaatgagttacttgtttcaacatgccaatttagattcttgcaaaagagtcttgaacgtggtgtgtaaaacttgtggacaacagcagacaacccttaagggtgtagaagctgttatgtacatgggcacactttcttatgaacaatttaagaaaggtgttcagataccttgtacgtgtggtaaacaagctacaaaatatctagtacaacaggagtcaccttttgttatgatgtcagcaccacctgctcagtatgaacttaagcatggtacatttacttgtgctagtgagtacactggtaattaccagtgtggtcactataaacatataacttctaaagaaactttgtattgcatagacggtgctttacttacaaagtcctcagaatacaaaggtcctattacggatgttttctacaaagaaaacagttacacaacaaccataaaaccagttacttataaattggatggtgttgtttgtacagaaattgaccctaagttggacaattattataagaaagacaattcttatttcacagagcaaccaattgatcttgtaccaaaccaaccatatccaaacgcaagcttcgataattttaagtttgtatgtgataatatcaaatttgctgatgatttaaaccagttaactggttataagaaacctgcttcaagagagcttaaagttacatttttccctgacttaaatggtgatgtggtggctattgattataaacactacacaccctcttttaagaaaggagctaaattgttacataaacctattgtttggcatgttaacaatgcaactaataaagccacgtataaaccaaatacctggtgtatacgttgtctttggagcacaaaaccagttgaaacatcaaattcgtttgatgtactgaagtcagaggacgcgcagggaatggataatcttgcctgcgaagatctaaaaccagtctctgaagaagtagtggaaaatcctaccatacagaaagacgttcttgagtgtaatgtgaaaactaccgaagttgtaggagacattatacttaaaccagcaaataatagtttaaaaattacagaagaggttggccacacagatctaatggctgcttatgtagacaattctagtcttactattaagaaacctaatgaattatctagagtattaggtttgaaaacccttgctactcatggtttagctgctgttaatagtgtcccttgggatactatagctaattatgctaagccttttcttaacaaagttgttagtacaactactaacatagttacacggtgtttaaaccgtgtttgtactaattatatgccttatttctttactttattgctacaattgtgtacttttactagaagtacaaattctagaattaaagcatctatgccgactactatagcaaagaatactgttaagagtgtcggtaaattttgtctagaggcttcatttaattatttgaagtcacctaatttttctaaactgataaatattataatttggtttttactattaagtgtttgcctaggttctttaatctactcaaccgctgctttaggtgttttaatgtctaatttaggcatgccttcttactgtactggttacagagaaggctatttgaactctactaatgtcactattgcaacctactgtactggttctataccttgtagtgtttgtcttagtggtttagattctttagacacctatccttctttagaaactatacaaattaccatttcatcttttaaatgggatttaactgcttttggcttagttgcagagtggtttttggcatatattcttttcactaggtttttctatgtacttggattggctgcaatcatgcaattgtttttcagctattttgcagtacattttattagtaattcttggcttatgtggttaataattaatcttgtacaaatggccccgatttcagctatggttagaatgtacatcttctttgcatcattttattatgtatggaaaagttatgtgcatgttgtagacggttgtaattcatcaacttgtatgatgtgttacaaacgtaatagagcaacaagagtcgaatgtacaactattgttaatggtgttagaaggtccttttatgtctatgctaatggaggtaaaggcttttgcaaactacacaattggaattgtgttaattgtgatacattctgtgctggtagtacatttattagtgatgaagttgcgagagacttgtcactacagtttaaaagaccaataaatcctactgaccagtcttcttacatcgttgatagtgttacagtgaagaatggttccatccatctttactttgataaagctggtcaaaagacttatgaaagacattctctctctcattttgttaacttagacaacctgagagctaataacactaaaggttcattgcctattaatgttatagtttttgatggtaaatcaaaatgtgaagaatcatctgcaaaatcagcgtctgtttactacagtcagcttatgtgtcaacctatactgttactagatcaggcattagtgtctgatgttggtgatagtgcggaagttgcagttaaaatgtttgatgcttacgttaatacgttttcatcaacttttaacgtaccaatggaaaaactcaaaacactagttgcaactgcagaagctgaacttgcaaagaatgtgtccttagacaatgtcttatctacttttatttcagcagctcggcaagggtttgttgattcagatgtagaaactaaagatgttgttgaatgtcttaaattgtcacatcaatctgacatagaagttactggcgatagttgtaataactatatgctcacctataacaaagttgaaaacatgacaccccgtgaccttggtgcttgtattgactgtagtgcgcgtcatattaatgcgcaggtagcaaaaagtcacaacattgctttgatatggaacgttaaagatttcatgtcattgtctgaacaactacgaaaacaaatacgtagtgctgctaaaaagaataacttaccttttaagttgacatgtgcaactactagacaagttgttaatgttgtaacaacaaagatagcacttaagggtggtaaaattgttaataattggttgaagcagttaattaaagttacacttgtgttcctttttgttgctgctattttctatttaataacacctgttcatgtcatgtctaaacatactgacttttcaagtgaaatcataggatacaaggctattgatggtggtgtcactcgtgacatagcatctacagatacttgttttgctaacaaacatgctgattttgacacatggtttagccagcgtggtggtagttatactaatgacaaagcttgcccattgattgctgcagtcataacaagagaagtgggttttgtcgtgcctggtttgcctggcacgatattacgcacaactaatggtgactttttgcatttcttacctagagtttttagtgcagttggtaacatctgttacacaccatcaaaacttatagagtacactgactttgcaacatcagcttgtgttttggctgctgaatgtacaatttttaaagatgcttctggtaagccagtaccatattgttatgataccaatgtactagaaggttctgttgcttatgaaagtttacgccctgacacacgttatgtgctcatggatggctctattattcaatttcctaacacctaccttgaaggttctgttagagtggtaacaacttttgattctgagtactgtaggcacggcacttgtgaaagatcagaagctggtgtttgtgtatctactagtggtagatgggtacttaacaatgattattacagatctttaccaggagttttctgtggtgtagatgctgtaaatttacttactaatatgtttacaccactaattcaacctattggtgctttggacatatcagcatctatagtagctggtggtattgtagctatcgtagtaacatgccttgcctactattttatgaggtttagaagagcttttggtgaatacagtcatgtagttgcctttaatactttactattccttatgtcattcactgtactctgtttaacaccagtttactcattcttacctggtgtttattctgttatttacttgtacttgacattttatcttactaatgatgtttcttttttagcacatattcagtggatggttatgttcacacctttagtacctttctggataacaattgcttatatcatttgtatttccacaaagcatttctattggttctttagtaattacctaaagagacgtgtagtctttaatggtgtttcctttagtacttttgaagaagctgcgctgtgcacctttttgttaaataaagaaatgtatctaaagttgcgtagtgatgtgctattacctcttacgcaatataatagatacttagctctttataataagtacaagtattttagtggagcaatggatacaactagctacagagaagctgcttgttgtcatctcgcaaaggctctcaatgacttcagtaactcaggttctgatgttctttaccaaccaccacaaacctctatcacctcagctgttttgcagagtggttttagaaaaatggcattcccatctggtaaagttgagggttgtatggtacaagtaacttgtggtacaactacacttaacggtctttggcttgatgacgtagtttactgtccaagacatgtgatctgcacctctgaagacatgcttaaccctaattatgaagatttactcattcgtaagtctaatcataatttcttggtacaggctggtaatgttcaactcagggttattggacattctatgcaaaattgtgtacttaagcttaaggttgatacagccaatcctaagacacctaagtataagtttgttcgcattcaaccaggacagactttttcagtgttagcttgttacaatggttcaccatctggtgtttaccaatgtgctatgaggcccaatttcactattaagggttcattccttaatggttcatgtggtagtgttggttttaacatagattatgactgtgtctctttttgttacatgcaccatatggaattaccaactggagttcatgctggcacagacttagaaggtaacttttatggaccttttgttgacaggcaaacagcacaagcagctggtacggacacaactattacagttaatgttttagcttggttgtacgctgctgttataaatggagacaggtggtttctcaatcgatttaccacaactcttaatgactttaaccttgtggctatgaagtacaattatgaacctctaacacaagaccatgttgacatactaggacctctttctgctcaaactggaattgccgttttagatatgtgtgcttcattaaaagaattactgcaaaatggtatgaatggacgtaccatattgggtagtgctttattagaagatgaatttacaccttttgatgttgttagacaatgctcaggtgttactttccaaagtgcagtgaaaagaacaatcaagggtacacaccactggttgttactcacaattttgacttcacttttagttttagtccagagtactcaatggtctttgttcttttttttgtatgaaaatgcctttttaccttttgctatgggtattattgctatgtctgcttttgcaatgatgtttgtcaaacataagcatgcatttctctgtttgtttttgttaccttctcttgccactgtagcttattttaatatggtctatatgcctgctagttgggtgatgcgtattatgacatggttggatatggttgatactagtttgtctggttttaagctaaaagactgtgttatgtatgcatcagctgtagtgttactaatccttatgacagcaagaactgtgtatgatgatggtgctaggagagtgtggacacttatgaatgtcttgacactcgtttataaagtttattatggtaatgctttagatcaagccatttccatgtgggctcttataatctctgttacttctaactactcaggtgtagttacaactgtcatgtttttggccagaggtattgtttttatgtgtgttgagtattgccctattttcttcataactggtaatacacttcagtgtataatgctagtttattgtttcttaggctatttttgtacttgttactttggcctcttttgtttactcaaccgctactttagactgactcttggtgtttatgattacttagtttctacacaggagtttagatatatgaattcacagggactactcccacccaagaatagcatagatgccttcaaactcaacattaaattgttgggtgttggtggcaaaccttgtatcaaagtagccactgtacagtctaaaatgtcagatgtaaagtgcacatcagtagtcttactctcagttttgcaacaactcagagtagaatcatcatctaaattgtgggctcaatgtgtccagttacacaatgacattctcttagctaaagatactactgaagcctttgaaaaaatggtttcactactttctgttttgctttccatgcagggtgctgtagacataaacaagctttgtgaagaaatgctggacaacagggcaaccttacaagctatagcctcagagtttagttcccttccatcatatgcagcttttgctactgctcaagaagcttatgagcaggctgttgctaatggtgattctgaagttgttcttaaaaagttgaagaagtctttgaatgtggctaaatctgaatttgaccgtgatgcagccatgcaacgtaagttggaaaagatggctgatcaagctatgacccaaatgtataaacaggctagatctgaggacaagagggcaaaagttactagtgctatgcagacaatgcttttcactatgcttagaaagttggataatgatgcactcaacaacattatcaacaatgcaagagatggttgtgttcccttgaacataatacctcttacaacagcagccaaactaatggttgtcataccagactataacacatataaaaatacgtgtgatggtacaacatttacttatgcatcagcattgtgggaaatccaacaggttgtagatgcagatagtaaaattgttcaacttagtgaaattagtatggacaattcacctaatttagcatggcctcttattgtaacagctttaagggccaattctgctgtcaaattacagaataatgagcttagtcctgttgcactacgacagatgtcttgtgctgccggtactacacaaactgcttgcactgatgacaatgcgttagcttactacaacacaacaaagggaggtaggtttgtacttgcactgttatccgatttacaggatttgaaatgggctagattccctaagagtgatggaactggtactatctatacagaactggaaccaccttgtaggtttgttacagacacacctaaaggtcctaaagtgaagtatttatactttattaaaggattaaacaacctaaatagaggtatggtacttggtagtttagctgccacagtacgtctacaagctggtaatgcaacagaagtgcctgccaattcaactgtattatctttctgtgcttttgctgtagatgctgctaaagcttacaaagattatctagctagtgggggacaaccaatcactaattgtgttaagatgttgtgtacacacactggtactggtcaggcaataacagttacaccggaagccaatatggatcaagaatcctttggtggtgcatcgtgttgtctgtactgccgttgccacatagatcatccaaatcctaaaggattttgtgacttaaaaggtaagtatgtacaaatacctacaacttgtgctaatgaccctgtgggttttacacttaaaaacacagtctgtaccgtctgcggtatgtggaaaggttatggctgtagttgtgatcaactccgcgaacccatgcttcagtcagctgatgcacaatcgtttttaaacgggtttgcggtgtaagtgcagcccgtcttacaccgtgcggcacaggcactagtactgatgtcgtatacagggcttttgacatctacaatgataaagtagctggttttgctaaattcctaaaaactaattgttgtcgcttccaagaaaaggacgaagatgacaatttaattgattcttactttgtagttaagagacacactttctctaactaccaacatgaagaaacaatttataatttacttaaggattgtccagctgttgctaaacatgacttctttaagtttagaatagacggtgacatggtaccacatatatcacgtcaacgtcttactaaatacacaatggcagacctcgtctatgctttaaggcattttgatgaaggtaattgtgacacattaaaagaaatacttgtcacatacaattgttgtgatgatgattatttcaataaaaaggactggtatgattttgtagaaaacccagatatattacgcgtatacgccaacttaggtgaacgtgtacgccaagctttgttaaaaacagtacaattctgtgatgccatgcgaaatgctggtattgttggtgtactgacattagataatcaagatctcaatggtaactggtatgatttcggtgatttcatacaaaccacgccaggtagtggagttcctgttgtagattcttattattcattgttaatgcctatattaaccttgaccagggctttaactgcagagtcacatgttgacactgacttaacaaagccttacattaagtgggatttgttaaaatatgacttcacggaagagaggttaaaactctttgaccgttattttaaatattgggatcagacataccacccaaattgtgttaactgtttggatgacagatgcattctgcattgtgcaaactttaatgttttattctctacagtgttcccacctacaagttttggaccactagtgagaaaaatatttgttgatggtgttccatttgtagtttcaactggataccacttcagagagctaggtgttgtacataatcaggatgtaaacttacatagctctagacttagttttaaggaattacttgtgtatgctgctgaccctgctatgcacgctgcttctggtaatctattactagataaacgcactacgtgcttttcagtagctgcacttactaacaatgttgcttttcaaactgtcaaacccggtaattttaacaaagacttctatgactttgctgtgtctaagggtttctttaaggaaggaagttctgttgaattaaaacacttcttctttgctcaggatggtaatgctgctatcagcgattatgactactatcgttataatctaccaacaatgtgtgatatcagacaactactatttgtagttgaagttgttgataagtactttgattgttacgatggtggctgtattaatgctaaccaagtcatcgtcaacaacctagacaaatcagctggttttccatttaataaatggggtaaggctagactttattatgattcaatgagttatgaggatcaagatgcacttttcgcatatacaaaacgtaatgtcatccctactataactcaaatgaatcttaagtatgccattagtgcaaagaatagagctcgcaccgtagctggtgtctctatctgtagtactatgaccaatagacagtttcatcaaaaattattgaaatcaatagccgccactagaggagctactgtagtaattggaacaagcaaattctatggtggttggcacaacatgttaaaaactgtttatagtgatgtagaaaaccctcaccttatgggttgggattatcctaaatgtgatagagccatgcctaacatgcttagaattatggcctcacttgttcttgctcgcaaacatacaacgtgttgtagcttgtcacaccgtttctatagattagctaatgagtgtgctcaagtattgagtgaaatggtcatgtgtggcggttcactatatgttaaaccaggtggaacctcatcaggagatgccacaactgcttatgctaatagtgtttttaacatttgtcaagctgtcacggccaatgttaatgcacttttatctactgatggtaacaaaattgccgataagtatgtccgcaatttacaacacagactttatgagtgtctctatagaaatagagatgttgacacagactttgtgaatgagttttacgcatatttgcgtaaacatttctcaatgatgatactctctgacgatgctgttgtgtgtttcaatagcacttatgcatctcaaggtctagtggctagcataaagaactttaagtcagttctttattatcaaaacaatgtttttatgtctgaagcaaaatgttggactgagactgaccttactaaaggacctcatgaattttgctctcaacatacaatgctagttaaacagggtgatgattatgtgtaccttccttacccagatccatcaagaatcctaggggccggctgttttgtagatgatatcgtaaaaacagatggtacacttatgattgaacggttcgtgtctttagctatagatgcttacccacttactaaacatcctaatcaggagtatgctgatgtctttcatttgtacttacaatacataagaaagctacatgatgagttaacaggacacatgttagacatgtattctgttatgcttactaatgataacacttcaaggtattgggaacctgagttttatgaggctatgtacacaccgcatacagtcttacaggctgttggggcttgtgttctttgcaattcacagacttcattaagatgtggtgcttgcatacgtagaccattcttatgttgtaaatgctgttacgaccatgtcatatcaacatcacataaattagtcttgtctgttaatccgtatgtttgcaatgctccaggttgtgatgtcacagatgtgactcaactttacttaggaggtatgagctattattgtaaatcacataaaccacccattagttttccattgtgtgctaatggacaagtttttggtttatataaaaatacatgtgttggtagcgataatgttactgactttaatgcaattgcaacatgtgactggacaaatgctggtgattacattttagctaacacctgtactgaaagactcaagctttttgcagcagaaacgctcaaagctactgaggagacatttaaactgtcttatggtattgctactgtacgtgaagtgctgtctgacagagaattacatctttcatgggaagttggtaaacctagaccaccacttaaccgaaattatgtctttactggttatcgtgtaactaaaaacagtaaagtacaaataggagagtacacctttgaaaaaggtgactatggtgatgctgttgtttaccgaggtacaacaacttacaaattaaatgttggtgattattttgtgctgacatcacatacagtaatgccattaagtgcacctacactagtgccacaagagcactatgttagaattactggcttatacccaacactcaatatctcagatgagttttctagcaatgttgcaaattatcaaaaggttggtatgcaaaagtattctacactccagggaccacctggtactggtaagagtcattttgctattggcctagctctctactacccttctgctcgcatagtgtatacagcttgctctcatgccgctgttgatgcactatgtgagaaggcattaaaatatttgcctatagataaatgtagtagaattatacctgcacgtgctcgtgtagagtgttttgataaattcaaagtgaattcaacattagaacagtatgtcttttgtactgtaaatgcattgcctgagacgacagcagatatagttgtctttgatgaaatttcaatggccacaaattatgatttgagtgttgtcaatgccagattacgtgctaagcactatgtgtacattggcgaccctgctcaattacctgcaccacgcacattgctaactaagggcacactagaaccagaatatttcaattcagtgtgtagacttatgaaaactataggtccagacatgttcctcggaacttgtcggcgttgtcctgctgaaattgttgacactgtgagtgctttggtttatgataataagcttaaagcacataaagacaaatcagctcaatgctttaaaatgttttataagggtgttatcacgcatgatgtttcatctgcaattaacaggccacaaataggcgtggtaagagaattccttacacgtaaccctgcttggagaaaagctgtctttatttcaccttataattcacagaatgctgtagcctcaaagattttgggactaccaactcaaactgttgattcatcacagggctcagaatatgactatgtcatattcactcaaaccactgaaacagctcactcttgtaatgtaaacagatttaatgttgctattaccagagcaaaagtaggcatactttgcataatgtctgatagagacctttatgacaagttgcaatttacaagtcttgaaattccacgtaggaatgtggcaactttacaagctgaaaatgtaacaggactctttaaagattgtagtaaggtaatcactgggttacatcctacacaggcacctacacacctcagtgttgacactaaattcaaaactgaaggtttatgtgttgacatacctggcatacctaaggacatgacctatagaagactcatctctatgatgggttttaaaatgaattatcaagttaatggttaccctaacatgtttatcacccgcgaagaagctataagacatgtacgtgcatggattggcttcgatgtcgaggggtgtcatgctactagagaagctgttggtaccaatttacctttacagctaggtttttctacaggtgttaacctagttgctgtacctacaggttatgttgatacacctaataatacagatttttccagagttagtgctaaaccaccgcctggagatcaatttaaacacctcataccacttatgtacaaaggacttccttggaatgtagtgcgtataaagattgtacaaatgttaagtgacacacttaaaaatctctctgacagagtcgtatttgtcttatgggcacatggctttgagttgacatctatgaagtattttgtgaaaataggacctgagcgcacctgttgtctatgtgatagacgtgccacatgcttttccactgcttcagacacttatgcctgttggcatcattctattggatttgattacgtctataatccgtttatgattgatgttcaacaatggggttttacaggtaacctacaaagcaaccatgatctgtattgtcaagtccatggtaatgcacatgtagctagttgtgatgcaatcatgactaggtgtctagctgtccacgagtgctttgttaagcgtgttgactggactattgaatatcctataattggtgatgaactgaagattaatgcggcttgtagaaaggttcaacacatggttgttaaagctgcattattagcagacaaattcccagttcttcacgacattggtaaccctaaagctattaagtgtgtacctcaagctgatgtagaatggaagttctatgatgcacagccttgtagtgacaaagcttataaaatagaagaattattctattcttatgccacacattctgacaaattcacagatggtgtatgcctattttggaattgcaatgtcgatagatatcctgctaattccattgtttgtagatttgacactagagtgctatctaaccttaacttgcctggttgtgatggtggcagtttgtatgtaaataaacatgcattccacacaccagcttttgataaaagtgcttttgttaatttaaaacaattaccatttttctattactctgacagtccatgtgagtctcatggaaaacaagtagtgtcagatatagattatgtaccactaaagtctgctacgtgtataacacgttgcaatttaggtggtgctgtctgtagacatcatgctaatgagtacagattgtatctcgatgcttataacatgatgatctcagctggctttagcttgtgggtttacaaacaatttgatacttataacctctggaacacttttacaagacttcagagtttagaaaatgtggcttttaatgttgtaaataagggacactttgatggacaacagggtgaagtaccagtttctatcattaataacactgtttacacaaaagttgatggtgttgatgtagaattgtttgaaaataaaacaacattacctgttaatgtagcatttgagctttgggctaagcgcaacattaaaccagtaccagaggtgaaaatactcaataatttgggtgtggacattgctgctaatactgtgatctgggactacaaaagagatgctccagcacatatatctactattggtgtttgttctatgactgacatagccaagaaaccaactgaaacgatttgtgcaccactcactgtcttttttgatggtagagttgatggtcaagtagacttatttagaaatgcccgtaatggtgttcttattacagaaggtagtgttaaaggtttacaaccatctgtgggtcccaaacaagctagtcttaatggagtcacattaattggagaagccgtaaaaacacagttcaattattataagaaagttgatggtgttgtccaacaattacctgaaacttactttactcagagtagaaatttacaagaatttaaacccaggagtcaaatggaaattgatttcttagaattagctatggatgaattcattgaacggtataaattagaaggctatgccttcgaacatatcgtttatggagattttagtcatagtcagttaggtggtttacatctactgattggactagctaaacgttttaaggaatcaccttttgaattagaagattttattcctatggacagtacagttaaaaactatttcataacagatgcgcaaacaggttcatctaagtgtgtgtgttctgttattgatttattacttgatgattttgttgaaataataaaatcccaagatttatctgtagtttctaaggttgtcaaagtgactattgactatacagaaatttcatttatgctttggtgtaaagatggccatgtagaaacattttacccaaaattacaatctagtcaagcgtggcaaccgggtgttgctatgcctaatctttacaaaatgcaaagaatgctattagaaaagtgtgaccttcaaaattatggtgatagtgcaacattacctaaaggcataatgatgaatgtcgcaaaatatactcaactgtgtcaatatttaaacacattaacattagctgtaccctataatatgagagttatacattttggtgctggttctgataaaggagttgcaccaggtacagctgttttaagacagtggttgcctacgggtacgctgcttgtcgattcagatcttaatgactttgtctctgatgcagattcaactttgattggtgattgtgcaactgtacatacagctaataaatgggatctcattattagtgatatgtacgaccctaagactaaaaatgttacaaaagaaaatgactctaaagagggttttttcacttacatttgtgggtttatacaacaaaagctagctcttggaggttccgtggctataaagataacagaacattcttggaatgctgatctttataagctcatgggacacttcgcatggtggacagcctttgttactaatgtgaatgcgtcatcatctgaagcatttttaattggatgtaattatcttggcaaaccacgcgaacaaatagatggttatgtcatgcatgcaaattacatattttggaggaatacaaatccaattcagttgtcttcctattctttatttgacatgagtaaatttccccttaaattaaggggtactgctgttatgtctttaaaagaaggtcaaatcaatgatatgattttatctcttcttagtaaaggtagacttataattagagaaaacaacagagttgttatttctagtgatgttcttgttaacaactaaacgaacaatgtttgtttttcttgttttattgccactagtctctagtcagtgtgttaatcttacaaccagaactcaattaccccctgcatacactaattctttcacacgtggtgtttattaccctgacaaagttttcagatcctcagttttacattcaactcaggacttgttcttacctttcttttccaatgttacttggttccatgctatacatgtctctgggaccaatggtactaagaggtttgataaccctgtcctaccatttaatgatggtgtttattttgcttccactgagaagtctaacataataagaggctggatttttggtactactttagattcgaagacccagtccctacttattgttaataacgctactaatgttgttattaaagtctgtgaatttcaattttgtaatgatccatttttgggtgtttattaccacaaaaacaacaaaagttggatggaaagtgagttcagagtttattctagtgcgaataattgcacttttgaatatgtctctcagccttttcttatggaccttgaaggaaaacagggtaatttcaaaaatcttagggaatttgtgtttaagaatattgatggttattttaaaatatattctaagcacacgcctattaatttagtgcgtgatctccctcagggtttttcggctttagaaccattggtagatttgccaataggtattaacatcactaggtttcaaactttacttgctttacatagaagttatttgactcctggtgattcttcttcaggttggacagctggtgctgcagcttattatgtgggttatcttcaacctaggacttttctattaaaatataatgaaaatggaaccattacagatgctgtagactgtgcacttgaccctctctcagaaacaaagtgtacgttgaaatccttcactgtagaaaaaggaatctatcaaacttctaactttagagtccaaccaacagaatctattgttagatttcctaatattacaaacttgtgcccttttggtgaagtttttaacgccaccagatttgcatctgtttatgcttggaacaggaagagaatcagcaactgtgttgctgattattctgtcctatataattccgcatcattttccacttttaagtgttatggagtgtctcctactaaattaaatgatctctgctttactaatgtctatgcagattcatttgtaattagaggtgatgaagtcagacaaatcgctccagggcaaactggaaagattgctgattataattataaattaccagatgattttacaggctgcgttatagcttggaattctaacaatcttgattctaaggttggtggtaattataattacctgtatagattgtttaggaagtctaatctcaaaccttttgagagagatatttcaactgaaatctatcaggccggtagcacaccttgtaatggtgttgaaggttttaattgttactttcctttacaatcatatggtttccaacccactaatggtgttggttaccaaccatacagagtagtagtactttcttttgaacttctacatgcaccagcaactgtttgtggacctaaaaagtctactaatttggttaaaaacaaatgtgtcaatttcaacttcaatggtttaacaggcacaggtgttcttactgagtctaacaaaaagtttctgcctttccaacaatttggcagagacattgctgacactactgatgctgtccgtgatccacagacacttgagattcttgacattacaccatgttcttttggtggtgtcagtgttataacaccaggaacaaatacttctaaccaggttgctgttctttatcaggatgttaactgcacagaagtccctgttgctattcatgcagatcaacttactcctacttggcgtgtttattctacaggttctaatgtttttcaaacacgtgcaggctgtttaataggggctgaacatgtcaacaactcatatgagtgtgacatacccattggtgcaggtatatgcgctagttatcagactcagactaattctcctcggcgggcacgtagtgtagctagtcaatccatcattgcctacactatgtcacttggtgcagaaaattcagttgcttactctaataactctattgccatacccacaaattttactattagtgttaccacagaaattctaccagtgtctatgaccaagacatcagtagattgtacaatgtacatttgtggtgattcaactgaatgcagcaatcttttgttgcaatatggcagtttttgtacacaattaaaccgtgctttaactggaatagctgttgaacaagacaaaaacacccaagaagtttttgcacaagtcaaacaaatttacaaaacaccaccaattaaagattttggtggttttaatttttcacaaatattaccagatccatcaaaaccaagcaagaggtcatttattgaagatctacttttcaacaaagtgacacttgcagatgctggcttcatcaaacaatatggtgattgccttggtgatattgctgctagagacctcatttgtgcacaaaagtttaacggccttactgttttgccacctttgctcacagatgaaatgattgctcaatacacttctgcactgttagcgggtacaatcacttctggttggacctttggtgcaggtgctgcattacaaataccatttgctatgcaaatggcttataggtttaatggtattggagttacacagaatgttctctatgagaaccaaaaattgattgccaaccaatttaatagtgctattggcaaaattcaagactcactttcttccacagcaagtgcacttggaaaacttcaagatgtggtcaaccaaaatgcacaagctttaaacacgcttgttaaacaacttagctccaattttggtgcaatttcaagtgttttaaatgatatcctttcacgtcttgacaaagttgaggctgaagtgcaaattgataggttgatcacaggcagacttcaaagtttgcagacatatgtgactcaacaattaattagagctgcagaaatcagagcttctgctaatcttgctgctactaaaatgtcagagtgtgtacttggacaatcaaaaagagttgatttttgtggaaagggctatcatcttatgtccttccctcagtcagcacctcatggtgtagtcttcttgcatgtgacttatgtccctgcacaagaaaagaacttcacaactgctcctgccatttgtcatgatggaaaagcacactttcctcgtgaaggtgtctttgtttcaaatggcacacactggtttgtaacacaaaggaatttttatgaaccacaaatcattactacagacaacacatttgtgtctggtaactgtgatgttgtaataggaattgtcaacaacacagtttatgatcctttgcaacctgaattagactcattcaaggaggagttagataaatattttaagaatcatacatcaccagatgttgatttaggtgacatctctggcattaatgcttcagttgtaaacattcaaaaagaaattgaccgcctcaatgaggttgccaagaatttaaatgaatctctcatcgatctccaagaacttggaaagtatgagcagtatataaaatggccatggtacatttggctaggttttatagctggcttgattgccatagtaatggtgacaattatgctttgctgtatgaccagttgctgtagttgtctcaagggctgttgttcttgtggatcctgctgcaaatttgatgaagacgactctgagccagtgctcaaaggagtcaaattacattacacataaacgaacttatggatttgtttatgagaatcttcacaattggaactgtaactttgaagcaaggtgaaatcaaggatgctactccttcagattttgttcgcgctactgcaacgataccgatacaagcctcactccctttcggatggcttattgttggcgttgcacttcttgctgtttttcagagcgcttccaaaatcataaccctcaaaaagagatggcaactagcactctccaagggtgttcactttgtttgcaacttgctgttgttgtttgtaacagtttactcacaccttttgctcgttgctgctggccttgaagccccttttctctatctttatgctttagtctacttcttgcagagtataaactttgtaagaataataatgaggctttggctttgctggaaatgccgttccaaaaacccattactttatgatgccaactattttctttgctggcatactaattgttacgactattgtataccttacaatagtgtaacttcttcaattgtcattacttcaggtgatggcacaacaagtcctatttctgaacatgactaccagattggtggttatactgaaaaatgggaatctggagtaaaagactgtgttgtattacacagttacttcacttcagactattaccagctgtactcaactcaattgagtacagacactggtgttgaacatgttaccttcttcatctacaataaaattgttgatgagcctgaagaacatgtccaaattcacacaatcgacggttcatccggagttgttaatccagtaatggaaccaatttatgatgaaccgacgacgactactagcgtgcctttgtaagcacaagctgatgagtttcctgatcttctggtctaaacgaactaaatattatattagtttttctgtttggaactttaattttagccatggcagattccaacggtactattaccgttgaagagcttaaaaagctccttgaacaatggaacctagtaataggtttcctattccttacatggatttgtcttctacaatttgcctatgccaacaggaataggtttttgtatataattaagttaattttcctctggctgttatggccagtaactttagcttgttttgtgcttgctgctgtttacagaataaattggatcaccggtggaattgctatcgcaatggcttgtcttgtaggcttgatgtggctcagctacttcattgcttctttcagactgtttgcgcgtacccgttccatgtggtcattcaatccagaaactaacattcttctcaacgtgccactccatggcactattctgaccagaccgcttctagaaagtgaactcgtaatcggagctgtgatccttcgtggacatcttcgtattgctggacaccatctaggacgctgtgacatcaaggacctgcctaaagaaatcactgttgctacatcacgaacgctttcttattacaaattgggagcttcgcagcgtgtagcaggtgactcaggttttgctgcatacagtcgctacaggattggcaactataaattaaacacagaccattccagtagcagtgacaatattgctttgcttgtacagtaagtgacaacagatgtttcatctcgttgactttcaggttactatagcagagatattactaattattatgaggacttttaaagtttccatttggaatcttgattacatcataaacctcataattaaaaatttatctaagtcactaactgagaataaatattctcaattagatgaagagcaaccaatggagattgattaaacgaacatgaaaattattcttttcttggcactgataacactcgctacttgtgagctttatcactaccaagagtgtgttagaggtacaacagtacttttaaaagaaccttgctcttctggaacatacgagggcaattcaccatttcatcctctagctgataacaaatttgcactgacttgctttagcactcaatttgcttttgcttgtcctgacggcgtaaaacacgtctatcagttacgtgccagatcagtttcacctaaactgttcatcagacaagaggaagttcaagaactttactctccaatttttcttattgttgcggcaatagtgtttataacactttgcttcacactcaaaagaaagacagaatgattgaactttcattaattgacttctatttgtgctttttagcctttctgctattccttgttttaattatgcttattatcttttggttctcacttgaactgcaagatcataatgaaacttgtcacgcctaaacgaacatgaaatttcttgttttcttaggaatcatcacaactgtagctgcatttcaccaagaatgtagtttacagtcatgtactcaacatcaaccatatgtagttgatgacccgtgtcctattcacttctattctaaatggtatattagagtaggagctagaaaatcagcacctttaattgaattgtgcgtggatgaggctggttctaaatcacccattcagtacatcgatatcggtaattatacagtttcctgtttaccttttacaattaattgccaggaacctaaattgggtagtcttgtagtgcgttgttcgttctatgaagactttttagagtatcatgacgttcgtgttgttttagatttcatctaaacgaacaaactaaaatgtctgataatggaccccaaaatcagcgaaatgcaccccgcattacgtttggtggaccctcagattcaactggcagtaaccagaatggagaacgcagtggggcgcgatcaaaacaacgtcggccccaaggtttacccaataatactgcgtcttggttcaccgctctcactcaacatggcaaggaagaccttaaattccctcgaggacaaggcgttccaattaacaccaatagcagtccagatgaccaaattggctactaccgaagagctaccagacgaattcgtggtggtgacggtaaaatgaaagatctcagtccaagatggtatttctactacctaggaactgggccagaagctggacttccctatggtgctaacaaagacggcatcatatgggttgcaactgagggagccttgaatacaccaaaagatcacattggcacccgcaatcctgctaacaatgctgcaatcgtgctacaacttcctcaaggaacaacattgccaaaaggcttctacgcagaagggagcagaggcggcagtcaagcctcttctcgttcctcatcacgtagtcgcaacagttcaagaaattcaactccaggcagcagtaggggaacttctcctgctagaatggctggcaatggcggtgatgctgctcttgctttgctgctgcttgacagattgaaccagcttgagagcaaaatgtctggtaaaggccaacaacaacaaggccaaactgtcactaagaaatctgctgctgaggcttctaagaagcctcggcaaaaacgtactgccactaaagcatacaatgtaacacaagctttcggcagacgtggtccagaacaaacccaaggaaattttggggaccaggaactaatcagacaaggaactgattacaaacattggccgcaaattgcacaatttgcccccagcgcttcagcgttcttcggaatgtcgcgcattggcatggaagtcacaccttcgggaacgtggttgacctacacagctgccatcaaattggatgacaaagatccaaatttcaaagatcaagtcattttgctgaataagcatattgacgcatacaaaacattcccaccaacagagcctaaaaaggacaaaaagaagaaggctgatgaaactcaagccttaccgcagagacagaagaaacagcaaactgtgactcttcttcctgctgcagatttggatgatttctccaaacaattgcaacaatccatgagcagtgctgactcaactcaggcctaaactcatgcagaccacacaaggcagatgggctatataaacgttttcgcttttccgtttacgatatatagtctactcttgtgcagaatgaattctcgtaactacatagcacaagtagatgtagttaactttaatctcacatagcaatctttaatcagtgtgtaacattagggaggacttgaaagagccaccacattttcaccgaggccacgcggagtacgatcgagtgtacagtgaacaatgctagggagagctgcctatatggaagagccctaatgtgtaaaattaattttagtagtgctatccccatgtgattttaatagcttcttaaaaaaaaaaaaaaaaaaaaaaaaa

SEQ ID NO: 17 - DNA, 28816 bp, Coronaviridae
  misc_feature 1..28816: note = SARS-CoV-2-[3,E]
  source 1..28816: mol_type = other DNA
attaaaggtttataccttcccaggtaacaaaccaaccaactttcgatctcttgtagatctgttctctaaacgaactttaaaatctgtgtggctgtcactcggctgcatgcttagtgcactcacgcagtataattaataactaattactgtcgttgacaggacacgagtaactcgtctatcttctgcaggctgcttacggtttcgtccgtgttgcagccgatcatcagcacatctaggtttcgtccgggtgtgaccgaaaggtaagatggagagccttgtccctggtttcaacgagaaaacacacgtccaactcagtttgcctgttttacaggttcgcgacgtgctcgtacgtggctttggagactccgtggaggaggtcttatcagaggcacgtcaacatcttaaagatggcacttgtggcttagtagaagttgaaaaaggcgttttgcctcaacttgaacagccctatgtgttcatcaaacgttcggatgctcgaactgcacctcatggtcatgttatggttgagctggtagcagaactcgaaggcattcagtacggtcgtagtggtgagacacttggtgtccttgtccctcatgtgggcgaaataccagtggcttaccgcaaggttcttcttcgtaagaacggtaataaaggagctggtggccatagttacggcgccgatctaaagtcatttgacttaggcgacgagcttggcactgatccttatgaagattttcaagaaaactggaacactaaacatagcagtggtgttacccgtgaactcatgcgtgagcttaacggaggggcatacactcgctatgtcgataacaacttctgtggccctgatggctaccctcttgagtgcattaaagaccttctagcacgtgctggtaaagcttcatgcactttgtccgaacaactggactttattgacactaagaggggtgtatactgctgccgtgaacatgagcatgaaattgcttggtacacggaacgttctgaaaagagctatgaattgcagacaccttttgaaattaaattggcaaagaaatttgacaccttcaatggggaatgtccaaattttgtatttcccttaaattccataatcaagactattcaaccaagggttgaaaagaaaaagcttgatggctttatgggtagaattcgatctgtctatccagttgcgtcaccaaatgaatgcaaccaaatgtgcctttcaactctcatgaagtgtgatcattgtggtgaaacttcatggcagacgggcgattttgttaaagccacttgcgaattttgtggcactgagaatttgactaaagaaggtgccactacttgtggttacttaccccaaaatgctgttgttaaaatttattgtccagcatgtcacaattcagaagtaggacctgagcatagtcttgccgaataccataatgaatctggcttgaaaaccattcttcgtaagggtggtcgcactattgcctttggaggctgtgtgttctcttatgttggttgccataacaagtgtgcctattgggttccacgtgctagcgctaacataggttgtaaccatacaggtgttgttggagaaggttccgaaggtcttaatgacaaccttcttgaaatactccaaaaagagaaagtcaacatcaatattgttggtgactttaaacttaatgaagagatcgccattattttggcatctttttctgcttccacaagtgcttttgtggaaactgtgaaaggtttggattataaagcattcaaacaaattgttgaatcctgtggtaattttaaagttacaaaaggaaaagctaaaaaaggtgcctggaatattggtgaacagaaatcaatactgagtcctctttatgcatttgcatcagaggctgctcgtgttgtacgatcaattttctcccgcactcttgaaactgctcaaaattctgtgcgtgttttacagaaggccgctataacaatactagatggaatttcacagtattcactgagactcattgatgctatgatgttcacatctgatttggctactaacaatctagttgtaatggcctacattacaggtggtgttgttcagttgacttcgcagtggctaactaacatctttggcactgtttatgaaaaactcaaacccgtccttgattggcttgaagagaagtttaaggaaggtgtagagtttcttagagacggttgggaaattgttaaatttatctcaacctgtgcttgtgaaattgtcggtggacaaattgtcacctgtgcaaaggaaattaaggagagtgttcagacattctttaagcttgtaaataaatttttggctttgtgtgctgactctatcattattggtggagctaaacttaaagccttgaatttaggtgaaacatttgtcacgcactcaaagggattgtacagaaagtgtgttaaatccagagaagaaactggcctactcatgcctctaaaagccccaaaagaaattatcttcttagagggagaaacacttcccacagaagtgttaacagaggaagttgtcttgaaaactggtgatttacaaccattagaacaacctactagtgaagctgttgaagctccattggttggtacaccagtttgtattaacgggcttatgttgctcgaaatcaaagacacagaaaagtactgtgcccttgcacctaatatgatggtaacaaacaataccttcacactcaaaggcggtgcaccaacaaaggttacttttggtgatgacactgtgatagaagtgcaaggttacaagagtgtgaatatcacttttgaacttgatgaaaggattgataaagtacttaatgagaagtgctctgcctatacagttgaactcggtacagaagtaaatgagttcgcctgtgttgtggcagatgctgtcataaaaactttgcaaccagtatctgaattacttacaccactgggcattgatttagatgagtggagtatggctacatactacttatttgatgagtctggtgagtttaaattggcttcacatatgtattgttctttctaccctccagatgaggatgaagaagaaggtgattgtgaagaagaagagtttgagccatcaactcaatatgagtatggtactgaagatgattaccaaggtaaacctttggaatttggtgccacttctgctgctcttcaacctgaagaagagcaagaagaagattggttagatgatgatagtcaacaaactgttggtcaacaagacggcagtgaggacaatcagacaactactattcaaacaattgttgaggttcaacctcaattagagatggaacttacaccagttgttcagactattgaagtgaatagttttagtggttatttaaaacttactgacaatgtatacattaaaaatgcagacattgtggaagaagctaaaaaggtaaaaccaacagtggttgttaatgcagccaatgtttaccttaaacatggaggaggtgttgcaggagccttaaataaggctactaacaatgccatgcaagttgaatctgatgattacatagctactaatggaccacttaaagtgggtggtagttgtgttttaagcggacacaatcttgctaaacactgtcttcatgttgtcggcccaaatgttaacaaaggtgaagacattcaacttcttaagagtgcttatgaaaattttaatcagcacgaagttctacttgcaccattattatcagctggtatttttggtgctgaccctatacattctttaagagtttgtgtagatactgttcgcacaaatgtctacttagctgtctttgataaaaatctctatgacaaacttgtttcaagctttttggaaatgaagagtgaaaagcaagttgaacaaaagatcgctgagattcctaaagaggaagttaagccatttataactgaaagtaaaccttcagttgaacagagaaaacaagatgataagaaaatcaaagcttgtgttgaagaagttacaacaactctggaagaaactaagttcctcacagaaaacttgttactttatattgacattaatggcaatcttcatccagattctgccactcttgttagtgacattgacatcactttcttaaagaaagatgctccatatatagtgggtgatgttgttcaagagggtgttttaactgctgtggttatacctactaaaaaggctggtggcactactgaaatgctagcgaaagctttgagaaaagtgccaacagacaattatataaccacttacccgggtcagggtttaaatggttacactgtagaggaggcaaagacagtgcttaaaaagtgtaaaagtgccttttacattctaccatctattatctctaatgagaagcaagaaattcttggaactgtttcttggaatttgcgagaaatgcttgcacatgcagaagaaacacgcaaattaatgcctgtctgtgtggaaactaaagccatagtttcaactatacagcgtaaatataagggtattaaaatacaagagggtgtggttgattatggtgctagattttacttttacaccagtaaaacaactgtagcgtcacttatcaacacacttaacgatctaaatgaaactcttgttacaatgccacttggctatgtaacacatggcttaaatttggaagaagctgctcggtatatgagatctctcaaagtgccagctacagtttctgtttcttcacctgatgctgttacagcgtataatggttatcttacttcttcttctaaaacacctgaagaacattttattgaaaccatctcacttgctggttcctataaagattggtcctattctggacaatctacacaactaggtatagaatttcttaagagaggtgataaaagtgtatattacactagtaatcctaccacattccacctagatggtgaagttatcacctttgacaatcttaagacacttctttctttgagagaagtgaggactattaaggtgtttacaacagtagacaacattaacctccacacgcaagttgtggacatgtcaatgacatatggacaacagtttggtccaacttatttggatggagctgatgttactaaaataaaacctcataattcacatgaaggtaaaacattttatgttttacctaatgatgacactctacgtgttgaggcttttgagtactaccacacaactgatcctagttttctgggtaggtacatgtcagcattaaatcacactaaaaagtggaaatacccacaagttaatggtttaacttctattaaatgggcagataacaactgttatcttgccactgcattgttaacactccaacaaatagagttgaagtttaatccacctgctctacaagatgcttattacagagcaagggctggtgaagctgctaacttttgtgcacttatcttagcctactgtaataagacagtaggtgagttaggtgatgttagagaaacaatgagttacttgtttcaacatgccaatttagattcttgcaaaagagtcttgaacgtggtgtgtaaaacttgtggacaacagcagacaacccttaagggtgtagaagctgttatgtacatgggcacactttcttatgaacaatttaagaaaggtgttcagataccttgtacgtgtggtaaacaagctacaaaatatctagtacaacaggagtcaccttttgttatgatgtcagcaccacctgctcagtatgaacttaagcatggtacatttacttgtgctagtgagtacactggtaattaccagtgtggtcactataaacatataacttctaaagaaactttgtattgcatagacggtgctttacttacaaagtcctcagaatacaaaggtcctattacggatgttttctacaaagaaaacagttacacaacaaccataaaaccagttacttataaattggatggtgttgtttgtacagaaattgaccctaagttggacaattattataagaaagacaattcttatttcacagagcaaccaattgatcttgtaccaaaccaaccatatccaaacgcaagcttcgataattttaagtttgtatgtgataatatcaaatttgctgatgatttaaaccagttaactggttataagaaacctgcttcaagagagcttaaagttacatttttccctgacttaaatggtgatgtggtggctattgattataaacactacacaccctcttttaagaaaggagctaaattgttacataaacctattgtttggcatgttaacaatgcaactaataaagccacgtataaaccaaatacctggtgtatacgttgtctttggagcacaaaaccagttgaaacatcaaattcgtttgatgtactgaagtcagaggacgcgcagggaatggataatcttgcctgcgaagatctaaaaccagtctctgaagaagtagtggaaaatcctaccatacagaaagacgttcttgagtgtaatgtgaaaactaccgaagttgtaggagacattatacttaaaccagcaaataatagtttaaaaattacagaagaggttggccacacagatctaatggctgcttatgtagacaattctagtcttactattaagaaacctaatgaattatctagagtattaggtttgaaaacccttgctactcatggtttagctgctgttaatagtgtcccttgggatactatagctaattatgctaagccttttcttaacaaagttgttagtacaactactaacatagttacacggtgtttaaaccgtgtttgtactaattatatgccttatttctttactttattgctacaattgtgtacttttactagaagtacaaattctagaattaaagcatctatgccgactactatagcaaagaatactgttaagagtgtcggtaaattttgtctagaggcttcatttaattatttgaagtcacctaatttttctaaactgataaatattataatttggtttttactattaagtgtttgcctaggttctttaatctactcaaccgctgctttaggtgttttaatgtctaatttaggcatgccttcttactgtactggttacagagaaggctatttgaactctactaatgtcactattgcaacctactgtactggttctataccttgtagtgtttgtcttagtggtttagattctttagacacctatccttctttagaaactatacaaattaccatttcatcttttaaatgggatttaactgcttttggcttagttgcagagtggtttttggcatatattcttttcactaggtttttctatgtacttggattggctgcaatcatgcaattgtttttcagctattttgcagtacattttattagtaattcttggcttatgtggttaataattaatcttgtacaaatggccccgatttcagctatggttagaatgtacatcttctttgcatcattttattatgtatggaaaagttatgtgcatgttgtagacggttgtaattcatcaacttgtatgatgtgttacaaacgtaatagagcaacaagagtcgaatgtacaactattgttaatggtgttagaaggtccttttatgtctatgctaatggaggtaaaggcttttgcaaactacacaattggaattgtgttaattgtgatacattctgtgctggtagtacatttattagtgatgaagttgcgagagacttgtcactacagtttaaaagaccaataaatcctactgaccagtcttcttacatcgttgatagtgttacagtgaagaatggttccatccatctttactttgataaagctggtcaaaagacttatgaaagacattctctctctcattttgttaacttagacaacctgagagctaataacactaaaggttcattgcctattaatgttatagtttttgatggtaaatcaaaatgtgaagaatcatctgcaaaatcagcgtctgtttactacagtcagcttatgtgtcaacctatactgttactagatcaggcattagtgtctgatgttggtgatagtgcggaagttgcagttaaaatgtttgatgcttacgttaatacgttttcatcaacttttaacgtaccaatggaaaaactcaaaacactagttgcaactgcagaagctgaacttgcaaagaatgtgtccttagacaatgtcttatctacttttatttcagcagctcggcaagggtttgttgattcagatgtagaaactaaagatgttgttgaatgtcttaaattgtcacatcaatctgacatagaagttactggcgatagttgtaataactatatgctcacctataacaaagttgaaaacatgacaccccgtgaccttggtgcttgtattgactgtagtgcgcgtcatattaatgcgcaggtagcaaaaagtcacaacattgctttgatatggaacgttaaagatttcatgtcattgtctgaacaactacgaaaacaaatacgtagtgctgctaaaaagaataacttaccttttaagttgacatgtgcaactactagacaagttgttaatgttgtaacaacaaagatagcacttaagggtggtaaaattgttaataattggttgaagcagttaattaaagttacacttgtgttcctttttgttgctgctattttctatttaataacacctgttcatgtcatgtctaaacatactgacttttcaagtgaaatcataggatacaaggctattgatggtggtgtcactcgtgacatagcatctacagatacttgttttgctaacaaacatgctgattttgacacatggtttagccagcgtggtggtagttatactaatgacaaagcttgcccattgattgctgcagtcataacaagagaagtgggttttgtcgtgcctggtttgcctggcacgatattacgcacaactaatggtgactttttgcatttcttacctagagtttttagtgcagttggtaacatctgttacacaccatcaaaacttatagagtacactgactttgcaacatcagcttgtgttttggctgctgaatgtacaatttttaaagatgcttctggtaagccagtaccatattgttatgataccaatgtactagaaggttctgttgcttatgaaagtttacgccctgacacacgttatgtgctcatggatggctctattattcaatttcctaacacctaccttgaaggttctgttagagtggtaacaacttttgattctgagtactgtaggcacggcacttgtgaaagatcagaagctggtgtttgtgtatctactagtggtagatgggtacttaacaatgattattacagatctttaccaggagttttctgtggtgtagatgctgtaaatttacttactaatatgtttacaccactaattcaacctattggtgctttggacatatcagcatctatagtagctggtggtattgtagctatcgtagtaacatgccttgcctactattttatgaggtttagaagagcttttggtgaatacagtcatgtagttgcctttaatactttactattccttatgtcattcactgtactctgtttaacaccagtttactcattcttacctggtgtttattctgttatttacttgtacttgacattttatcttactaatgatgtttcttttttagcacatattcagtggatggttatgttcacacctttagtacctttctggataacaattgcttatatcatttgtatttccacaaagcatttctattggttctttagtaattacctaaagagacgtgtagtctttaatggtgtttcctttagtacttttgaagaagctgcgctgtgcacctttttgttaaataaagaaatgtatctaaagttgcgtagtgatgtgctattacctcttacgcaatataatagatacttagctctttataataagtacaagtattttagtggagcaatggatacaactagctacagagaagctgcttgttgtcatctcgcaaaggctctcaatgacttcagtaactcaggttctgatgttctttaccaaccaccacaaacctctatcacctcagctgttttgcagagtggttttagaaaaatggcattcccatctggtaaagttgagggttgtatggtacaagtaacttgtggtacaactacacttaacggtctttggcttgatgacgtagtttactgtccaagacatgtgatctgcacctctgaagacatgcttaaccctaattatgaagatttactcattcgtaagtctaatcataatttcttggtacaggctggtaatgttcaactcagggttattggacattctatgcaaaattgtgtacttaagcttaaggttgatacagccaatcctaagacacctaagtataagtttgttcgcattcaaccaggacagactttttcagtgttagcttgttacaatggttcaccatctggtgtttaccaatgtgctatgaggcccaatttcactattaagggttcattccttaatggttcatgtggtagtgttggttttaacatagattatgactgtgtctctttttgttacatgcaccatatggaattaccaactggagttcatgctggcacagacttagaaggtaacttttatggaccttttgttgacaggcaaacagcacaagcagctggtacggacacaactattacagttaatgttttagcttggttgtacgctgctgttataaatggagacaggtggtttctcaatcgatttaccacaactcttaatgactttaaccttgtggctatgaagtacaattatgaacctctaacacaagaccatgttgacatactaggacctctttctgctcaaactggaattgccgttttagatatgtgtgcttcattaaaagaattactgcaaaatggtatgaatggacgtaccatattgggtagtgctttattagaagatgaatttacaccttttgatgttgttagacaatgctcaggtgttactttccaaagtgcagtgaaaagaacaatcaagggtacacaccactggttgttactcacaattttgacttcacttttagttttagtccagagtactcaatggtctttgttcttttttttgtatgaaaatgcctttttaccttttgctatgggtattattgctatgtctgcttttgcaatgatgtttgtcaaacataagcatgcatttctctgtttgtttttgttaccttctcttgccactgtagcttattttaatatggtctatatgcctgctagttgggtgatgcgtattatgacatggttggatatggttgatactagtttgtctggttttaagctaaaagactgtgttatgtatgcatcagctgtagtgttactaatccttatgacagcaagaactgtgtatgatgatggtgctaggagagtgtggacacttatgaatgtcttgacactcgtttataaagtttattatggtaatgctttagatcaagccatttccatgtgggctcttataatctctgttacttctaactactcaggtgtagttacaactgtcatgtttttggccagaggtattgtttttatgtgtgttgagtattgccctattttcttcataactggtaatacacttcagtgtataatgctagtttattgtttcttaggctatttttgtacttgttactttggcctcttttgtttactcaaccgctactttagactgactcttggtgtttatgattacttagtttctacacaggagtttagatatatgaattcacagggactactcccacccaagaatagcatagatgccttcaaactcaacattaaattgttgggtgttggtggcaaaccttgtatcaaagtagccactgtacagtctaaaatgtcagatgtaaagtgcacatcagtagtcttactctcagttttgcaacaactcagagtagaatcatcatctaaattgtgggctcaatgtgtccagttacacaatgacattctcttagctaaagatactactgaagcctttgaaaaaatggtttcactactttctgttttgctttccatgcagggtgctgtagacataaacaagctttgtgaagaaatgctggacaacagggcaaccttacaagctatagcctcagagtttagttcccttccatcatatgcagcttttgctactgctcaagaagcttatgagcaggctgttgctaatggtgattctgaagttgttcttaaaaagttgaagaagtctttgaatgtggctaaatctgaatttgaccgtgatgcagccatgcaacgtaagttggaaaagatggctgatcaagctatgacccaaatgtataaacaggctagatctgaggacaagagggcaaaagttactagtgctatgcagacaatgcttttcactatgcttagaaagttggataatgatgcactcaacaacattatcaacaatgcaagagatggttgtgttcccttgaacataatacctcttacaacagcagccaaactaatggttgtcataccagactataacacatataaaaatacgtgtgatggtacaacatttacttatgcatcagcattgtgggaaatccaacaggttgtagatgcagatagtaaaattgttcaacttagtgaaattagtatggacaattcacctaatttagcatggcctcttattgtaacagctttaagggccaattctgctgtcaaattacagaataatgagcttagtcctgttgcactacgacagatgtcttgtgctgccggtactacacaaactgcttgcactgatgacaatgcgttagcttactacaacacaacaaagggaggtaggtttgtacttgcactgttatccgatttacaggatttgaaatgggctagattccctaagagtgatggaactggtactatctatacagaactggaaccaccttgtaggtttgttacagacacacctaaaggtcctaaagtgaagtatttatactttattaaaggattaaacaacctaaatagaggtatggtacttggtagtttagctgccacagtacgtctacaagctggtaatgcaacagaagtgcctgccaattcaactgtattatctttctgtgcttttgctgtagatgctgctaaagcttacaaagattatctagctagtgggggacaaccaatcactaattgtgttaagatgttgtgtacacacactggtactggtcaggcaataacagttacaccggaagccaatatggatcaagaatcctttggtggtgcatcgtgttgtctgtactgccgttgccacatagatcatccaaatcctaaaggattttgtgacttaaaaggtaagtatgtacaaatacctacaacttgtgctaatgaccctgtgggttttacacttaaaaacacagtctgtaccgtctgcggtatgtggaaaggttatggctgtagttgtgatcaactccgcgaacccatgcttcagtcagctgatgcacaatcgtttttaaacgggtttgcggtgtaagtgcagcccgtcttacaccgtgcggcacaggcactagtactgatgtcgtatacagggcttttgacatctacaatgataaagtagctggttttgctaaattcctaaaaactaattgttgtcgcttccaagaaaaggacgaagatgacaatttaattgattcttactttgtagttaagagacacactttctctaactaccaacatgaagaaacaatttataatttacttaaggattgtccagctgttgctaaacatgacttctttaagtttagaatagacggtgacatggtaccacatatatcacgtcaacgtcttactaaatacacaatggcagacctcgtctatgctttaaggcattttgatgaaggtaattgtgacacattaaaagaaatacttgtcacatacaattgttgtgatgatgattatttcaataaaaaggactggtatgattttgtagaaaacccagatatattacgcgtatacgccaacttaggtgaacgtgtacgccaagctttgttaaaaacagtacaattctgtgatgccatgcgaaatgctggtattgttggtgtactgacattagataatcaagatctcaatggtaactggtatgatttcggtgatttcatacaaaccacgccaggtagtggagttcctgttgtagattcttattattcattgttaatgcctatattaaccttgaccagggctttaactgcagagtcacatgttgacactgacttaacaaagccttacattaagtgggatttgttaaaatatgacttcacggaagagaggttaaaactctttgaccgttattttaaatattgggatcagacataccacccaaattgtgttaactgtttggatgacagatgcattctgcattgtgcaaactttaatgttttattctctacagtgttcccacctacaagttttggaccactagtgagaaaaatatttgttgatggtgttccatttgtagtttcaactggataccacttcagagagctaggtgttgtacataatcaggatgtaaacttacatagctctagacttagttttaaggaattacttgtgtatgctgctgaccctgctatgcacgctgcttctggtaatctattactagataaacgcactacgtgcttttcagtagctgcacttactaacaatgttgcttttcaaactgtcaaacccggtaattttaacaaagacttctatgactttgctgtgtctaagggtttctttaaggaaggaagttctgttgaattaaaacacttcttctttgctcaggatggtaatgctgctatcagcgattatgactactatcgttataatctaccaacaatgtgtgatatcagacaactactatttgtagttgaagttgttgataagtactttgattgttacgatggtggctgtattaatgctaaccaagtcatcgtcaacaacctagacaaatcagctggttttccatttaataaatggggtaaggctagactttattatgattcaatgagttatgaggatcaagatgcacttttcgcatatacaaaacgtaatgtcatccctactataactcaaatgaatcttaagtatgccattagtgcaaagaatagagctcgcaccgtagctggtgtctctatctgtagtactatgaccaatagacagtttcatcaaaaattattgaaatcaatagccgccactagaggagctactgtagtaattggaacaagcaaattctatggtggttggcacaacatgttaaaaactgtttatagtgatgtagaaaaccctcaccttatgggttgggattatcctaaatgtgatagagccatgcctaacatgcttagaattatggcctcacttgttcttgctcgcaaacatacaacgtgttgtagcttgtcacaccgtttctatagattagctaatgagtgtgctcaagtattgagtgaaatggtcatgtgtggcggttcactatatgttaaaccaggtggaacctcatcaggagatgccacaactgcttatgctaatagtgtttttaacatttgtcaagctgtcacggccaatgttaatgcacttttatctactgatggtaacaaaattgccgataagtatgtccgcaatttacaacacagactttatgagtgtctctatagaaatagagatgttgacacagactttgtgaatgagttttacgcatatttgcgtaaacatttctcaatgatgatactctctgacgatgctgttgtgtgtttcaatagcacttatgcatctcaaggtctagtggctagcataaagaactttaagtcagttctttattatcaaaacaatgtttttatgtctgaagcaaaatgttggactgagactgaccttactaaaggacctcatgaattttgctctcaacatacaatgctagttaaacagggtgatgattatgtgtaccttccttacccagatccatcaagaatcctaggggccggctgttttgtagatgatatcgtaaaaacagatggtacacttatgattgaacggttcgtgtctttagctatagatgcttacccacttactaaacatcctaatcaggagtatgctgatgtctttcatttgtacttacaatacataagaaagctacatgatgagttaacaggacacatgttagacatgtattctgttatgcttactaatgataacacttcaaggtattgggaacctgagttttatgaggctatgtacacaccgcatacagtcttacaggctgttggggcttgtgttctttgcaattcacagacttcattaagatgtggtgcttgcatacgtagaccattcttatgttgtaaatgctgttacgaccatgtcatatcaacatcacataaattagtcttgtctgttaatccgtatgtttgcaatgctccaggttgtgatgtcacagatgtgactcaactttacttaggaggtatgagctattattgtaaatcacataaaccacccattagttttccattgtgtgctaatggacaagtttttggtttatataaaaatacatgtgttggtagcgataatgttactgactttaatgcaattgcaacatgtgactggacaaatgctggtgattacattttagctaacacctgtactgaaagactcaagctttttgcagcagaaacgctcaaagctactgaggagacatttaaactgtcttatggtattgctactgtacgtgaagtgctgtctgacagagaattacatctttcatgggaagttggtaaacctagaccaccacttaaccgaaattatgtctttactggttatcgtgtaactaaaaacagtaaagtacaaataggagagtacacctttgaaaaaggtgactatggtgatgctgttgtttaccgaggtacaacaacttacaaattaaatgttggtgattattttgtgctgacatcacatacagtaatgccattaagtgcacctacactagtgccacaagagcactatgttagaattactggcttatacccaacactcaatatctcagatgagttttctagcaatgttgcaaattatcaaaaggttggtatgcaaaagtattctacactccagggaccacctggtactggtaagagtcattttgctattggcctagctctctactacccttctgctcgcatagtgtatacagcttgctctcatgccgctgttgatgcactatgtgagaaggcattaaaatatttgcctatagataaatgtagtagaattatacctgcacgtgctcgtgtagagtgttttgataaattcaaagtgaattcaacattagaacagtatgtcttttgtactgtaaatgcattgcctgagacgacagcagatatagttgtctttgatgaaatttcaatggccacaaattatgatttgagtgttgtcaatgccagattacgtgctaagcactatgtgtacattggcgaccctgctcaattacctgcaccacgcacattgctaactaagggcacactagaaccagaatatttcaattcagtgtgtagacttatgaaaactataggtccagacatgttcctcggaacttgtcggcgttgtcctgctgaaattgttgacactgtgagtgctttggtttatgataataagcttaaagcacataaagacaaatcagctcaatgctttaaaatgttttataagggtgttatcacgcatgatgtttcatctgcaattaacaggccacaaataggcgtggtaagagaattccttacacgtaaccctgcttggagaaaagctgtctttatttcaccttataattcacagaatgctgtagcctcaaagattttgggactaccaactcaaactgttgattcatcacagggctcagaatatgactatgtcatattcactcaaaccactgaaacagctcactcttgtaatgtaaacagatttaatgttgctattaccagagcaaaagtaggcatactttgcataatgtctgatagagacctttatgacaagttgcaatttacaagtcttgaaattccacgtaggaatgtggcaactttacaagctgaaaatgtaacaggactctttaaagattgtagtaaggtaatcactgggttacatcctacacaggcacctacacacctcagtgttgacactaaattcaaaactgaaggtttatgtgttgacatacctggcatacctaaggacatgacctatagaagactcatctctatgatgggttttaaaatgaattatcaagttaatggttaccctaacatgtttatcacccgcgaagaagctataagacatgtacgtgcatggattggcttcgatgtcgaggggtgtcatgctactagagaagctgttggtaccaatttacctttacagctaggtttttctacaggtgttaacctagttgctgtacctacaggttatgttgatacacctaataatacagatttttccagagttagtgctaaaccaccgcctggagatcaatttaaacacctcataccacttatgtacaaaggacttccttggaatgtagtgcgtataaagattgtacaaatgttaagtgacacacttaaaaatctctctgacagagtcgtatttgtcttatgggcacatggctttgagttgacatctatgaagtattttgtgaaaataggacctgagcgcacctgttgtctatgtgatagacgtgccacatgcttttccactgcttcagacacttatgcctgttggcatcattctattggatttgattacgtctataatccgtttatgattgatgttcaacaatggggttttacaggtaacctacaaagcaaccatgatctgtattgtcaagtccatggtaatgcacatgtagctagttgtgatgcaatcatgactaggtgtctagctgtccacgagtgctttgttaagcgtgttgactggactattgaatatcctataattggtgatgaactgaagattaatgcggcttgtagaaaggttcaacacatggttgttaaagctgcattattagcagacaaattcccagttcttcacgacattggtaaccctaaagctattaagtgtgtacctcaagctgatgtagaatggaagttctatgatgcacagccttgtagtgacaaagcttataaaatagaagaattattctattcttatgccacacattctgacaaattcacagatggtgtatgcctattttggaattgcaatgtcgatagatatcctgctaattccattgtttgtagatttgacactagagtgctatctaaccttaacttgcctggttgtgatggtggcagtttgtatgtaaataaacatgcattccacacaccagcttttgataaaagtgcttttgttaatttaaaacaattaccatttttctattactctgacagtccatgtgagtctcatggaaaacaagtagtgtcagatatagattatgtaccactaaagtctgctacgtgtataacacgttgcaatttaggtggtgctgtctgtagacatcatgctaatgagtacagattgtatctcgatgcttataacatgatgatctcagctggctttagcttgtgggtttacaaacaatttgatacttataacctctggaacacttttacaagacttcagagtttagaaaatgtggcttttaatgttgtaaataagggacactttgatggacaacagggtgaagtaccagtttctatcattaataacactgtttacacaaaagttgatggtgttgatgtagaattgtttgaaaataaaacaacattacctgttaatgtagcatttgagctttgggctaagcgcaacattaaaccagtaccagaggtgaaaatactcaataatttgggtgtggacattgctgctaatactgtgatctgggactacaaaagagatgctccagcacatatatctactattggtgtttgttctatgactgacatagccaagaaaccaactgaaacgatttgtgcaccactcactgtcttttttgatggtagagttgatggtcaagtagacttatttagaaatgcccgtaatggtgttcttattacagaaggtagtgttaaaggtttacaaccatctgtgggtcccaaacaagctagtcttaatggagtcacattaattggagaagccgtaaaaacacagttcaattattataagaaagttgatggtgttgtccaacaattacctgaaacttactttactcagagtagaaatttacaagaatttaaacccaggagtcaaatggaaattgatttcttagaattagctatggatgaattcattgaacggtataaattagaaggctatgccttcgaacatatcgtttatggagattttagtcatagtcagttaggtggtttacatctactgattggactagctaaacgttttaaggaatcaccttttgaattagaagattttattcctatggacagtacagttaaaaactatttcataacagatgcgcaaacaggttcatctaagtgtgtgtgttctgttattgatttattacttgatgattttgttgaaataataaaatcccaagatttatctgtagtttctaaggttgtcaaagtgactattgactatacagaaatttcatttatgctttggtgtaaagatggccatgtagaaacattttacccaaaattacaatctagtcaagcgtggcaaccgggtgttgctatgcctaatctttacaaaatgcaaagaatgctattagaaaagtgtgaccttcaaaattatggtgatagtgcaacattacctaaaggcataatgatgaatgtcgcaaaatatactcaactgtgtcaatatttaaacacattaacattagctgtaccctataatatgagagttatacattttggtgctggttctgataaaggagttgcaccaggtacagctgttttaagacagtggttgcctacgggtacgctgcttgtcgattcagatcttaatgactttgtctctgatgcagattcaactttgattggtgattgtgcaactgtacatacagctaataaatgggatctcattattagtgatatgtacgaccctaagactaaaaatgttacaaaagaaaatgactctaaagagggttttttcacttacatttgtgggtttatacaacaaaagctagctcttggaggttccgtggctataaagataacagaacattcttggaatgctgatctttataagctcatgggacacttcgcatggtggacagcctttgttactaatgtgaatgcgtcatcatctgaagcatttttaattggatgtaattatcttggcaaaccacgcgaacaaatagatggttatgtcatgcatgcaaattacatattttggaggaatacaaatccaattcagttgtcttcctattctttatttgacatgagtaaatttccccttaaattaaggggtactgctgttatgtctttaaaagaaggtcaaatcaatgatatgattttatctcttcttagtaaaggtagacttataattagagaaaacaacagagttgttatttctagtgatgttcttgttaacaactaaacgaacaatgtttgtttttcttgttttattgccactagtctctagtcagtgtgttaatcttacaaccagaactcaattaccccctgcatacactaattctttcacacgtggtgtttattaccctgacaaagttttcagatcctcagttttacattcaactcaggacttgttcttacctttcttttccaatgttacttggttccatgctatacatgtctctgggaccaatggtactaagaggtttgataaccctgtcctaccatttaatgatggtgtttattttgcttccactgagaagtctaacataataagaggctggatttttggtactactttagattcgaagacccagtccctacttattgttaataacgctactaatgttgttattaaagtctgtgaatttcaattttgtaatgatccatttttgggtgtttattaccacaaaaacaacaaaagttggatggaaagtgagttcagagtttattctagtgcgaataattgcacttttgaatatgtctctcagccttttcttatggaccttgaaggaaaacagggtaatttcaaaaatcttagggaatttgtgtttaagaatattgatggttattttaaaatatattctaagcacacgcctattaatttagtgcgtgatctccctcagggtttttcggctttagaaccattggtagatttgccaataggtattaacatcactaggtttcaaactttacttgctttacatagaagttatttgactcctggtgattcttcttcaggttggacagctggtgctgcagcttattatgtgggttatcttcaacctaggacttttctattaaaatataatgaaaatggaaccattacagatgctgtagactgtgcacttgaccctctctcagaaacaaagtgtacgttgaaatccttcactgtagaaaaaggaatctatcaaacttctaactttagagtccaaccaacagaatctattgttagatttcctaatattacaaacttgtgcccttttggtgaagtttttaacgccaccagatttgcatctgtttatgcttggaacaggaagagaatcagcaactgtgttgctgattattctgtcctatataattccgcatcattttccacttttaagtgttatggagtgtctcctactaaattaaatgatctctgctttactaatgtctatgcagattcatttgtaattagaggtgatgaagtcagacaaatcgctccagggcaaactggaaagattgctgattataattataaattaccagatgattttacaggctgcgttatagcttggaattctaacaatcttgattctaaggttggtggtaattataattacctgtatagattgtttaggaagtctaatctcaaaccttttgagagagatatttcaactgaaatctatcaggccggtagcacaccttgtaatggtgttgaaggttttaattgttactttcctttacaatcatatggtttccaacccactaatggtgttggttaccaaccatacagagtagtagtactttcttttgaacttctacatgcaccagcaactgtttgtggacctaaaaagtctactaatttggttaaaaacaaatgtgtcaatttcaacttcaatggtttaacaggcacaggtgttcttactgagtctaacaaaaagtttctgcctttccaacaatttggcagagacattgctgacactactgatgctgtccgtgatccacagacacttgagattcttgacattacaccatgttcttttggtggtgtcagtgttataacaccaggaacaaatacttctaaccaggttgctgttctttatcaggatgttaactgcacagaagtccctgttgctattcatgcagatcaacttactcctacttggcgtgtttattctacaggttctaatgtttttcaaacacgtgcaggctgtttaataggggctgaacatgtcaacaactcatatgagtgtgacatacccattggtgcaggtatatgcgctagttatcagactcagactaattctcctcggcgggcacgtagtgtagctagtcaatccatcattgcctacactatgtcacttggtgcagaaaattcagttgcttactctaataactctattgccatacccacaaattttactattagtgttaccacagaaattctaccagtgtctatgaccaagacatcagtagattgtacaatgtacatttgtggtgattcaactgaatgcagcaatcttttgttgcaatatggcagtttttgtacacaattaaaccgtgctttaactggaatagctgttgaacaagacaaaaacacccaagaagtttttgcacaagtcaaacaaatttacaaaacaccaccaattaaagattttggtggttttaatttttcacaaatattaccagatccatcaaaaccaagcaagaggtcatttattgaagatctacttttcaacaaagtgacacttgcagatgctggcttcatcaaacaatatggtgattgccttggtgatattgctgctagagacctcatttgtgcacaaaagtttaacggccttactgttttgccacctttgctcacagatgaaatgattgctcaatacacttctgcactgttagcgggtacaatcacttctggttggacctttggtgcaggtgctgcattacaaataccatttgctatgcaaatggcttataggtttaatggtattggagttacacagaatgttctctatgagaaccaaaaattgattgccaaccaatttaatagtgctattggcaaaattcaagactcactttcttccacagcaagtgcacttggaaaacttcaagatgtggtcaaccaaaatgcacaagctttaaacacgcttgttaaacaacttagctccaattttggtgcaatttcaagtgttttaaatgatatcctttcacgtcttgacaaagttgaggctgaagtgcaaattgataggttgatcacaggcagacttcaaagtttgcagacatatgtgactcaacaattaattagagctgcagaaatcagagcttctgctaatcttgctgctactaaaatgtcagagtgtgtacttggacaatcaaaaagagttgatttttgtggaaagggctatcatcttatgtccttccctcagtcagcacctcatggtgtagtcttcttgcatgtgacttatgtccctgcacaagaaaagaacttcacaactgctcctgccatttgtcatgatggaaaagcacactttcctcgtgaaggtgtctttgtttcaaatggcacacactggtttgtaacacaaaggaatttttatgaaccacaaatcattactacagacaacacatttgtgtctggtaactgtgatgttgtaataggaattgtcaacaacacagtttatgatcctttgcaacctgaattagactcattcaaggaggagttagataaatattttaagaatcatacatcaccagatgttgatttaggtgacatctctggcattaatgcttcagttgtaaacattcaaaaagaaattgaccgcctcaatgaggttgccaagaatttaaatgaatctctcatcgatctccaagaacttggaaagtatgagcagtatataaaatggccatggtacatttggctaggttttatagctggcttgattgccatagtaatggtgacaattatgctttgctgtatgaccagttgctgtagttgtctcaagggctgttgttcttgtggatcctgctgcaaatttgatgaagacgactctgagccagtgctcaaaggagtcaaattacattacacataattcctgatcttctggtctaaacgaactaaatattatattagtttttctgtttggaactttaattttagccatggcagattccaacggtactattaccgttgaagagcttaaaaagctccttgaacaatggaacctagtaataggtttcctattccttacatggatttgtcttctacaatttgcctatgccaacaggaataggtttttgtatataattaagttaattttcctctggctgttatggccagtaactttagcttgttttgtgcttgctgctgtttacagaataaattggatcaccggtggaattgctatcgcaatggcttgtcttgtaggcttgatgtggctcagctacttcattgcttctttcagactgtttgcgcgtacccgttccatgtggtcattcaatccagaaactaacattcttctcaacgtgccactccatggcactattctgaccagaccgcttctagaaagtgaactcgtaatcggagctgtgatccttcgtggacatcttcgtattgctggacaccatctaggacgctgtgacatcaaggacctgcctaaagaaatcactgttgctacatcacgaacgctttcttattacaaattgggagcttcgcagcgtgtagcaggtgactcaggttttgctgcatacagtcgctacaggattggcaactataaattaaacacagaccattccagtagcagtgacaatattgctttgcttgtacagtaagtgacaacagatgtttcatctcgttgactttcaggttactatagcagagatattactaattattatgaggacttttaaagtttccatttggaatcttgattacatcataaacctcataattaaaaatttatctaagtcactaactgagaataaatattctcaattagatgaagagcaaccaatggagattgattaaacgaacatgaaaattattcttttcttggcactgataacactcgctacttgtgagctttatcactaccaagagtgtgttagaggtacaacagtacttttaaaagaaccttgctcttctggaacatacgagggcaattcaccatttcatcctctagctgataacaaatttgcactgacttgctttagcactcaatttgcttttgcttgtcctgacggcgtaaaacacgtctatcagttacgtgccagatcagtttcacctaaactgttcatcagacaagaggaagttcaagaactttactctccaatttttcttattgttgcggcaatagtgtttataacactttgcttcacactcaaaagaaagacagaatgattgaactttcattaattgacttctatttgtgctttttagcctttctgctattccttgttttaattatgcttattatcttttggttctcacttgaactgcaagatcataatgaaacttgtcacgcctaaacgaacatgaaatttcttgttttcttaggaatcatcacaactgtagctgcatttcaccaagaatgtagtttacagtcatgtactcaacatcaaccatatgtagttgatgacccgtgtcctattcacttctattctaaatggtatattagagtaggagctagaaaatcagcacctttaattgaattgtgcgtggatgaggctggttctaaatcacccattcagtacatcgatatcggtaattatacagtttcctgtttaccttttacaattaattgccaggaacctaaattgggtagtcttgtagtgcgttgttcgttctatgaagactttttagagtatcatgacgttcgtgttgttttagatttcatctaaacgaacaaactaaaatgtctgataatggaccccaaaatcagcgaaatgcaccccgcattacgtttggtggaccctcagattcaactggcagtaaccagaatggagaacgcagtggggcgcgatcaaaacaacgtcggccccaaggtttacccaataatactgcgtcttggttcaccgctctcactcaacatggcaaggaagaccttaaattccctcgaggacaaggcgttccaattaacaccaatagcagtccagatgaccaaattggctactaccgaagagctaccagacgaattcgtggtggtgacggtaaaatgaaagatctcagtccaagatggtatttctactacctaggaactgggccagaagctggacttccctatggtgctaacaaagacggcatcatatgggttgcaactgagggagccttgaatacaccaaaagatcacattggcacccgcaatcctgctaacaatgctgcaatcgtgctacaacttcctcaaggaacaacattgccaaaaggcttctacgcagaagggagcagaggcggcagtcaagcctcttctcgttcctcatcacgtagtcgcaacagttcaagaaattcaactccaggcagcagtaggggaacttctcctgctagaatggctggcaatggcggtgatgctgctcttgctttgctgctgcttgacagattgaaccagcttgagagcaaaatgtctggtaaaggccaacaacaacaaggccaaactgtcactaagaaatctgctgctgaggcttctaagaagcctcggcaaaaacgtactgccactaaagcatacaatgtaacacaagctttcggcagacgtggtccagaacaaacccaaggaaattttggggaccaggaactaatcagacaaggaactgattacaaacattggccgcaaattgcacaatttgcccccagcgcttcagcgttcttcggaatgtcgcgcattggcatggaagtcacaccttcgggaacgtggttgacctacacagctgccatcaaattggatgacaaagatccaaatttcaaagatcaagtcattttgctgaataagcatattgacgcatacaaaacattcccaccaacagagcctaaaaaggacaaaaagaagaaggctgatgaaactcaagccttaccgcagagacagaagaaacagcaaactgtgactcttcttcctgctgcagatttggatgatttctccaaacaattgcaacaatccatgagcagtgctgactcaactcaggcctaaactcatgcagaccacacaaggcagatgggctatataaacgttttcgcttttccgtttacgatatatagtctactcttgtgcagaatgaattctcgtaactacatagcacaagtagatgtagttaactttaatctcacatagcaatctttaatcagtgtgtaacattagggaggacttgaaagagccaccacattttcaccgaggccacgcggagtacgatcgagtgtacagtgaacaatgctagggagagctgcctatatggaagagccctaatgtgtaaaattaattttagtagtgctatccccatgtgattttaatagcttcttaaaaaaaaaaaaaaaaaaaaaaaaa

SEQ ID NO: 18 - DNA, 29729 bp, Coronaviridae
  misc_feature 1..29729: note = SARS-CoV-2-6, it contains two punctual substitutions (c.27041A'C and c.27044A'C) and a deletion (Nucleotides 27202 - 27367) comparing to the reference rSARS-CoV-2-WT sequence.
  source 1..29729: mol_type = other DNA
attaaaggtttataccttcccaggtaacaaaccaaccaactttcgatctcttgtagatctgttctctaaacgaactttaaaatctgtgtggctgtcactcggctgcatgcttagtgcactcacgcagtataattaataactaattactgtcgttgacaggacacgagtaactcgtctatcttctgcaggctgcttacggtttcgtccgtgttgcagccgatcatcagcacatctaggtttcgtccgggtgtgaccgaaaggtaagatggagagccttgtccctggtttcaacgagaaaacacacgtccaactcagtttgcctgttttacaggttcgcgacgtgctcgtacgtggctttggagactccgtggaggaggtcttatcagaggcacgtcaacatcttaaagatggcacttgtggcttagtagaagttgaaaaaggcgttttgcctcaacttgaacagccctatgtgttcatcaaacgttcggatgctcgaactgcacctcatggtcatgttatggttgagctggtagcagaactcgaaggcattcagtacggtcgtagtggtgagacacttggtgtccttgtccctcatgtgggcgaaataccagtggcttaccgcaaggttcttcttcgtaagaacggtaataaaggagctggtggccatagttacggcgccgatctaaagtcatttgacttaggcgacgagcttggcactgatccttatgaagattttcaagaaaactggaacactaaacatagcagtggtgttacccgtgaactcatgcgtgagcttaacggaggggcatacactcgctatgtcgataacaacttctgtggccctgatggctaccctcttgagtgcattaaagaccttctagcacgtgctggtaaagcttcatgcactttgtccgaacaactggactttattgacactaagaggggtgtatactgctgccgtgaacatgagcatgaaattgcttggtacacggaacgttctgaaaagagctatgaattgcagacaccttttgaaattaaattggcaaagaaatttgacaccttcaatggggaatgtccaaattttgtatttcccttaaattccataatcaagactattcaaccaagggttgaaaagaaaaagcttgatggctttatgggtagaattcgatctgtctatccagttgcgtcaccaaatgaatgcaaccaaatgtgcctttcaactctcatgaagtgtgatcattgtggtgaaacttcatggcagacgggcgattttgttaaagccacttgcgaattttgtggcactgagaatttgactaaagaaggtgccactacttgtggttacttaccccaaaatgctgttgttaaaatttattgtccagcatgtcacaattcagaagtaggacctgagcatagtcttgccgaataccataatgaatctggcttgaaaaccattcttcgtaagggtggtcgcactattgcctttggaggctgtgtgttctcttatgttggttgccataacaagtgtgcctattgggttccacgtgctagcgctaacataggttgtaaccatacaggtgttgttggagaaggttccgaaggtcttaatgacaaccttcttgaaatactccaaaaagagaaagtcaacatcaatattgttggtgactttaaacttaatgaagagatcgccattattttggcatctttttctgcttccacaagtgcttttgtggaaactgtgaaaggtttggattataaagcattcaaacaaattgttgaatcctgtggtaattttaaagttacaaaaggaaaagctaaaaaaggtgcctggaatattggtgaacagaaatcaatactgagtcctctttatgcatttgcatcagaggctgctcgtgttgtacgatcaattttctcccgcactcttgaaactgctcaaaattctgtgcgtgttttacagaaggccgctataacaatactagatggaatttcacagtattcactgagactcattgatgctatgatgttcacatctgatttggctactaacaatctagttgtaatggcctacattacaggtggtgttgttcagttgacttcgcagtggctaactaacatctttggcactgtttatgaaaaactcaaacccgtccttgattggcttgaagagaagtttaaggaaggtgtagagtttcttagagacggttgggaaattgttaaatttatctcaacctgtgcttgtgaaattgtcggtggacaaattgtcacctgtgcaaaggaaattaaggagagtgttcagacattctttaagcttgtaaataaatttttggctttgtgtgctgactctatcattattggtggagctaaacttaaagccttgaatttaggtgaaacatttgtcacgcactcaaagggattgtacagaaagtgtgttaaatccagagaagaaactggcctactcatgcctctaaaagccccaaaagaaattatcttcttagagggagaaacacttcccacagaagtgttaacagaggaagttgtcttgaaaactggtgatttacaaccattagaacaacctactagtgaagctgttgaagctccattggttggtacaccagtttgtattaacgggcttatgttgctcgaaatcaaagacacagaaaagtactgtgcccttgcacctaatatgatggtaacaaacaataccttcacactcaaaggcggtgcaccaacaaaggttacttttggtgatgacactgtgatagaagtgcaaggttacaagagtgtgaatatcacttttgaacttgatgaaaggattgataaagtacttaatgagaagtgctctgcctatacagttgaactcggtacagaagtaaatgagttcgcctgtgttgtggcagatgctgtcataaaaactttgcaaccagtatctgaattacttacaccactgggcattgatttagatgagtggagtatggctacatactacttatttgatgagtctggtgagtttaaattggcttcacatatgtattgttctttctaccctccagatgaggatgaagaagaaggtgattgtgaagaagaagagtttgagccatcaactcaatatgagtatggtactgaagatgattaccaaggtaaacctttggaatttggtgccacttctgctgctcttcaacctgaagaagagcaagaagaagattggttagatgatgatagtcaacaaactgttggtcaacaagacggcagtgaggacaatcagacaactactattcaaacaattgttgaggttcaacctcaattagagatggaacttacaccagttgttcagactattgaagtgaatagttttagtggttatttaaaacttactgacaatgtatacattaaaaatgcagacattgtggaagaagctaaaaaggtaaaaccaacagtggttgttaatgcagccaatgtttaccttaaacatggaggaggtgttgcaggagccttaaataaggctactaacaatgccatgcaagttgaatctgatgattacatagctactaatggaccacttaaagtgggtggtagttgtgttttaagcggacacaatcttgctaaacactgtcttcatgttgtcggcccaaatgttaacaaaggtgaagacattcaacttcttaagagtgcttatgaaaattttaatcagcacgaagttctacttgcaccattattatcagctggtatttttggtgctgaccctatacattctttaagagtttgtgtagatactgttcgcacaaatgtctacttagctgtctttgataaaaatctctatgacaaacttgtttcaagctttttggaaatgaagagtgaaaagcaagttgaacaaaagatcgctgagattcctaaagaggaagttaagccatttataactgaaagtaaaccttcagttgaacagagaaaacaagatgataagaaaatcaaagcttgtgttgaagaagttacaacaactctggaagaaactaagttcctcacagaaaacttgttactttatattgacattaatggcaatcttcatccagattctgccactcttgttagtgacattgacatcactttcttaaagaaagatgctccatatatagtgggtgatgttgttcaagagggtgttttaactgctgtggttatacctactaaaaaggctggtggcactactgaaatgctagcgaaagctttgagaaaagtgccaacagacaattatataaccacttacccgggtcagggtttaaatggttacactgtagaggaggcaaagacagtgcttaaaaagtgtaaaagtgccttttacattctaccatctattatctctaatgagaagcaagaaattcttggaactgtttcttggaatttgcgagaaatgcttgcacatgcagaagaaacacgcaaattaatgcctgtctgtgtggaaactaaagccatagtttcaactatacagcgtaaatataagggtattaaaatacaagagggtgtggttgattatggtgctagattttacttttacaccagtaaaacaactgtagcgtcacttatcaacacacttaacgatctaaatgaaactcttgttacaatgccacttggctatgtaacacatggcttaaatttggaagaagctgctcggtatatgagatctctcaaagtgccagctacagtttctgtttcttcacctgatgctgttacagcgtataatggttatcttacttcttcttctaaaacacctgaagaacattttattgaaaccatctcacttgctggttcctataaagattggtcctattctggacaatctacacaactaggtatagaatttcttaagagaggtgataaaagtgtatattacactagtaatcctaccacattccacctagatggtgaagttatcacctttgacaatcttaagacacttctttctttgagagaagtgaggactattaaggtgtttacaacagtagacaacattaacctccacacgcaagttgtggacatgtcaatgacatatggacaacagtttggtccaacttatttggatggagctgatgttactaaaataaaacctcataattcacatgaaggtaaaacattttatgttttacctaatgatgacactctacgtgttgaggcttttgagtactaccacacaactgatcctagttttctgggtaggtacatgtcagcattaaatcacactaaaaagtggaaatacccacaagttaatggtttaacttctattaaatgggcagataacaactgttatcttgccactgcattgttaacactccaacaaatagagttgaagtttaatccacctgctctacaagatgcttattacagagcaagggctggtgaagctgctaacttttgtgcacttatcttagcctactgtaataagacagtaggtgagttaggtgatgttagagaaacaatgagttacttgtttcaacatgccaatttagattcttgcaaaagagtcttgaacgtggtgtgtaaaacttgtggacaacagcagacaacccttaagggtgtagaagctgttatgtacatgggcacactttcttatgaacaatttaagaaaggtgttcagataccttgtacgtgtggtaaacaagctacaaaatatctagtacaacaggagtcaccttttgttatgatgtcagcaccacctgctcagtatgaacttaagcatggtacatttacttgtgctagtgagtacactggtaattaccagtgtggtcactataaacatataacttctaaagaaactttgtattgcatagacggtgctttacttacaaagtcctcagaatacaaaggtcctattacggatgttttctacaaagaaaacagttacacaacaaccataaaaccagttacttataaattggatggtgttgtttgtacagaaattgaccctaagttggacaattattataagaaagacaattcttatttcacagagcaaccaattgatcttgtaccaaaccaaccatatccaaacgcaagcttcgataattttaagtttgtatgtgataatatcaaatttgctgatgatttaaaccagttaactggttataagaaacctgcttcaagagagcttaaagttacatttttccctgacttaaatggtgatgtggtggctattgattataaacactacacaccctcttttaagaaaggagctaaattgttacataaacctattgtttggcatgttaacaatgcaactaataaagccacgtataaaccaaatacctggtgtatacgttgtctttggagcacaaaaccagttgaaacatcaaattcgtttgatgtactgaagtcagaggacgcgcagggaatggataatcttgcctgcgaagatctaaaaccagtctctgaagaagtagtggaaaatcctaccatacagaaagacgttcttgagtgtaatgtgaaaactaccgaagttgtaggagacattatacttaaaccagcaaataatagtttaaaaattacagaagaggttggccacacagatctaatggctgcttatgtagacaattctagtcttactattaagaaacctaatgaattatctagagtattaggtttgaaaacccttgctactcatggtttagctgctgttaatagtgtcccttgggatactatagctaattatgctaagccttttcttaacaaagttgttagtacaactactaacatagttacacggtgtttaaaccgtgtttgtactaattatatgccttatttctttactttattgctacaattgtgtacttttactagaagtacaaattctagaattaaagcatctatgccgactactatagcaaagaatactgttaagagtgtcggtaaattttgtctagaggcttcatttaattatttgaagtcacctaatttttctaaactgataaatattataatttggtttttactattaagtgtttgcctaggttctttaatctactcaaccgctgctttaggtgttttaatgtctaatttaggcatgccttcttactgtactggttacagagaaggctatttgaactctactaatgtcactattgcaacctactgtactggttctataccttgtagtgtttgtcttagtggtttagattctttagacacctatccttctttagaaactatacaaattaccatttcatcttttaaatgggatttaactgcttttggcttagttgcagagtggtttttggcatatattcttttcactaggtttttctatgtacttggattggctgcaatcatgcaattgtttttcagctattttgcagtacattttattagtaattcttggcttatgtggttaataattaatcttgtacaaatggccccgatttcagctatggttagaatgtacatcttctttgcatcattttattatgtatggaaaagttatgtgcatgttgtagacggttgtaattcatcaacttgtatgatgtgttacaaacgtaatagagcaacaagagtcgaatgtacaactattgttaatggtgttagaaggtccttttatgtctatgctaatggaggtaaaggcttttgcaaactacacaattggaattgtgttaattgtgatacattctgtgctggtagtacatttattagtgatgaagttgcgagagacttgtcactacagtttaaaagaccaataaatcctactgaccagtcttcttacatcgttgatagtgttacagtgaagaatggttccatccatctttactttgataaagctggtcaaaagacttatgaaagacattctctctctcattttgttaacttagacaacctgagagctaataacactaaaggttcattgcctattaatgttatagtttttgatggtaaatcaaaatgtgaagaatcatctgcaaaatcagcgtctgtttactacagtcagcttatgtgtcaacctatactgttactagatcaggcattagtgtctgatgttggtgatagtgcggaagttgcagttaaaatgtttgatgcttacgttaatacgttttcatcaacttttaacgtaccaatggaaaaactcaaaacactagttgcaactgcagaagctgaacttgcaaagaatgtgtccttagacaatgtcttatctacttttatttcagcagctcggcaagggtttgttgattcagatgtagaaactaaagatgttgttgaatgtcttaaattgtcacatcaatctgacatagaagttactggcgatagttgtaataactatatgctcacctataacaaagttgaaaacatgacaccccgtgaccttggtgcttgtattgactgtagtgcgcgtcatattaatgcgcaggtagcaaaaagtcacaacattgctttgatatggaacgttaaagatttcatgtcattgtctgaacaactacgaaaacaaatacgtagtgctgctaaaaagaataacttaccttttaagttgacatgtgcaactactagacaagttgttaatgttgtaacaacaaagatagcacttaagggtggtaaaattgttaataattggttgaagcagttaattaaagttacacttgtgttcctttttgttgctgctattttctatttaataacacctgttcatgtcatgtctaaacatactgacttttcaagtgaaatcataggatacaaggctattgatggtggtgtcactcgtgacatagcatctacagatacttgttttgctaacaaacatgctgattttgacacatggtttagccagcgtggtggtagttatactaatgacaaagcttgcccattgattgctgcagtcataacaagagaagtgggttttgtcgtgcctggtttgcctggcacgatattacgcacaactaatggtgactttttgcatttcttacctagagtttttagtgcagttggtaacatctgttacacaccatcaaaacttatagagtacactgactttgcaacatcagcttgtgttttggctgctgaatgtacaatttttaaagatgcttctggtaagccagtaccatattgttatgataccaatgtactagaaggttctgttgcttatgaaagtttacgccctgacacacgttatgtgctcatggatggctctattattcaatttcctaacacctaccttgaaggttctgttagagtggtaacaacttttgattctgagtactgtaggcacggcacttgtgaaagatcagaagctggtgtttgtgtatctactagtggtagatgggtacttaacaatgattattacagatctttaccaggagttttctgtggtgtagatgctgtaaatttacttactaatatgtttacaccactaattcaacctattggtgctttggacatatcagcatctatagtagctggtggtattgtagctatcgtagtaacatgccttgcctactattttatgaggtttagaagagcttttggtgaatacagtcatgtagttgcctttaatactttactattccttatgtcattcactgtactctgtttaacaccagtttactcattcttacctggtgtttattctgttatttacttgtacttgacattttatcttactaatgatgtttcttttttagcacatattcagtggatggttatgttcacacctttagtacctttctggataacaattgcttatatcatttgtatttccacaaagcatttctattggttctttagtaattacctaaagagacgtgtagtctttaatggtgtttcctttagtacttttgaagaagctgcgctgtgcacctttttgttaaataaagaaatgtatctaaagttgcgtagtgatgtgctattacctcttacgcaatataatagatacttagctctttataataagtacaagtattttagtggagcaatggatacaactagctacagagaagctgcttgttgtcatctcgcaaaggctctcaatgacttcagtaactcaggttctgatgttctttaccaaccaccacaaacctctatcacctcagctgttttgcagagtggttttagaaaaatggcattcccatctggtaaagttgagggttgtatggtacaagtaacttgtggtacaactacacttaacggtctttggcttgatgacgtagtttactgtccaagacatgtgatctgcacctctgaagacatgcttaaccctaattatgaagatttactcattcgtaagtctaatcataatttcttggtacaggctggtaatgttcaactcagggttattggacattctatgcaaaattgtgtacttaagcttaaggttgatacagccaatcctaagacacctaagtataagtttgttcgcattcaaccaggacagactttttcagtgttagcttgttacaatggttcaccatctggtgtttaccaatgtgctatgaggcccaatttcactattaagggttcattccttaatggttcatgtggtagtgttggttttaacatagattatgactgtgtctctttttgttacatgcaccatatggaattaccaactggagttcatgctggcacagacttagaaggtaacttttatggaccttttgttgacaggcaaacagcacaagcagctggtacggacacaactattacagttaatgttttagcttggttgtacgctgctgttataaatggagacaggtggtttctcaatcgatttaccacaactcttaatgactttaaccttgtggctatgaagtacaattatgaacctctaacacaagaccatgttgacatactaggacctctttctgctcaaactggaattgccgttttagatatgtgtgcttcattaaaagaattactgcaaaatggtatgaatggacgtaccatattgggtagtgctttattagaagatgaatttacaccttttgatgttgttagacaatgctcaggtgttactttccaaagtgcagtgaaaagaacaatcaagggtacacaccactggttgttactcacaattttgacttcacttttagttttagtccagagtactcaatggtctttgttcttttttttgtatgaaaatgcctttttaccttttgctatgggtattattgctatgtctgcttttgcaatgatgtttgtcaaacataagcatgcatttctctgtttgtttttgttaccttctcttgccactgtagcttattttaatatggtctatatgcctgctagttgggtgatgcgtattatgacatggttggatatggttgatactagtttgtctggttttaagctaaaagactgtgttatgtatgcatcagctgtagtgttactaatccttatgacagcaagaactgtgtatgatgatggtgctaggagagtgtggacacttatgaatgtcttgacactcgtttataaagtttattatggtaatgctttagatcaagccatttccatgtgggctcttataatctctgttacttctaactactcaggtgtagttacaactgtcatgtttttggccagaggtattgtttttatgtgtgttgagtattgccctattttcttcataactggtaatacacttcagtgtataatgctagtttattgtttcttaggctatttttgtacttgttactttggcctcttttgtttactcaaccgctactttagactgactcttggtgtttatgattacttagtttctacacaggagtttagatatatgaattcacagggactactcccacccaagaatagcatagatgccttcaaactcaacattaaattgttgggtgttggtggcaaaccttgtatcaaagtagccactgtacagtctaaaatgtcagatgtaaagtgcacatcagtagtcttactctcagttttgcaacaactcagagtagaatcatcatctaaattgtgggctcaatgtgtccagttacacaatgacattctcttagctaaagatactactgaagcctttgaaaaaatggtttcactactttctgttttgctttccatgcagggtgctgtagacataaacaagctttgtgaagaaatgctggacaacagggcaaccttacaagctatagcctcagagtttagttcccttccatcatatgcagcttttgctactgctcaagaagcttatgagcaggctgttgctaatggtgattctgaagttgttcttaaaaagttgaagaagtctttgaatgtggctaaatctgaatttgaccgtgatgcagccatgcaacgtaagttggaaaagatggctgatcaagctatgacccaaatgtataaacaggctagatctgaggacaagagggcaaaagttactagtgctatgcagacaatgcttttcactatgcttagaaagttggataatgatgcactcaacaacattatcaacaatgcaagagatggttgtgttcccttgaacataatacctcttacaacagcagccaaactaatggttgtcataccagactataacacatataaaaatacgtgtgatggtacaacatttacttatgcatcagcattgtgggaaatccaacaggttgtagatgcagatagtaaaattgttcaacttagtgaaattagtatggacaattcacctaatttagcatggcctcttattgtaacagctttaagggccaattctgctgtcaaattacagaataatgagcttagtcctgttgcactacgacagatgtcttgtgctgccggtactacacaaactgcttgcactgatgacaatgcgttagcttactacaacacaacaaagggaggtaggtttgtacttgcactgttatccgatttacaggatttgaaatgggctagattccctaagagtgatggaactggtactatctatacagaactggaaccaccttgtaggtttgttacagacacacctaaaggtcctaaagtgaagtatttatactttattaaaggattaaacaacctaaatagaggtatggtacttggtagtttagctgccacagtacgtctacaagctggtaatgcaacagaagtgcctgccaattcaactgtattatctttctgtgcttttgctgtagatgctgctaaagcttacaaagattatctagctagtgggggacaaccaatcactaattgtgttaagatgttgtgtacacacactggtactggtcaggcaataacagttacaccggaagccaatatggatcaagaatcctttggtggtgcatcgtgttgtctgtactgccgttgccacatagatcatccaaatcctaaaggattttgtgacttaaaaggtaagtatgtacaaatacctacaacttgtgctaatgaccctgtgggttttacacttaaaaacacagtctgtaccgtctgcggtatgtggaaaggttatggctgtagttgtgatcaactccgcgaacccatgcttcagtcagctgatgcacaatcgtttttaaacgggtttgcggtgtaagtgcagcccgtcttacaccgtgcggcacaggcactagtactgatgtcgtatacagggcttttgacatctacaatgataaagtagctggttttgctaaattcctaaaaactaattgttgtcgcttccaagaaaaggacgaagatgacaatttaattgattcttactttgtagttaagagacacactttctctaactaccaacatgaagaaacaatttataatttacttaaggattgtccagctgttgctaaacatgacttctttaagtttagaatagacggtgacatggtaccacatatatcacgtcaacgtcttactaaatacacaatggcagacctcgtctatgctttaaggcattttgatgaaggtaattgtgacacattaaaagaaatacttgtcacatacaattgttgtgatgatgattatttcaataaaaaggactggtatgattttgtagaaaacccagatatattacgcgtatacgccaacttaggtgaacgtgtacgccaagctttgttaaaaacagtacaattctgtgatgccatgcgaaatgctggtattgttggtgtactgacattagataatcaagatctcaatggtaactggtatgatttcggtgatttcatacaaaccacgccaggtagtggagttcctgttgtagattcttattattcattgttaatgcctatattaaccttgaccagggctttaactgcagagtcacatgttgacactgacttaacaaagccttacattaagtgggatttgttaaaatatgacttcacggaagagaggttaaaactctttgaccgttattttaaatattgggatcagacataccacccaaattgtgttaactgtttggatgacagatgcattctgcattgtgcaaactttaatgttttattctctacagtgttcccacctacaagttttggaccactagtgagaaaaatatttgttgatggtgttccatttgtagtttcaactggataccacttcagagagctaggtgttgtacataatcaggatgtaaacttacatagctctagacttagttttaaggaattacttgtgtatgctgctgaccctgctatgcacgctgcttctggtaatctattactagataaacgcactacgtgcttttcagtagctgcacttactaacaatgttgcttttcaaactgtcaaacccggtaattttaacaaagacttctatgactttgctgtgtctaagggtttctttaaggaaggaagttctgttgaattaaaacacttcttctttgctcaggatggtaatgctgctatcagcgattatgactactatcgttataatctaccaacaatgtgtgatatcagacaactactatttgtagttgaagttgttgataagtactttgattgttacgatggtggctgtattaatgctaaccaagtcatcgtcaacaacctagacaaatcagctggttttccatttaataaatggggtaaggctagactttattatgattcaatgagttatgaggatcaagatgcacttttcgcatatacaaaacgtaatgtcatccctactataactcaaatgaatcttaagtatgccattagtgcaaagaatagagctcgcaccgtagctggtgtctctatctgtagtactatgaccaatagacagtttcatcaaaaattattgaaatcaatagccgccactagaggagctactgtagtaattggaacaagcaaattctatggtggttggcacaacatgttaaaaactgtttatagtgatgtagaaaaccctcaccttatgggttgggattatcctaaatgtgatagagccatgcctaacatgcttagaattatggcctcacttgttcttgctcgcaaacatacaacgtgttgtagcttgtcacaccgtttctatagattagctaatgagtgtgctcaagtattgagtgaaatggtcatgtgtggcggttcactatatgttaaaccaggtggaacctcatcaggagatgccacaactgcttatgctaatagtgtttttaacatttgtcaagctgtcacggccaatgttaatgcacttttatctactgatggtaacaaaattgccgataagtatgtccgcaatttacaacacagactttatgagtgtctctatagaaatagagatgttgacacagactttgtgaatgagttttacgcatatttgcgtaaacatttctcaatgatgatactctctgacgatgctgttgtgtgtttcaatagcacttatgcatctcaaggtctagtggctagcataaagaactttaagtcagttctttattatcaaaacaatgtttttatgtctgaagcaaaatgttggactgagactgaccttactaaaggacctcatgaattttgctctcaacatacaatgctagttaaacagggtgatgattatgtgtaccttccttacccagatccatcaagaatcctaggggccggctgttttgtagatgatatcgtaaaaacagatggtacacttatgattgaacggttcgtgtctttagctatagatgcttacccacttactaaacatcctaatcaggagtatgctgatgtctttcatttgtacttacaatacataagaaagctacatgatgagttaacaggacacatgttagacatgtattctgttatgcttactaatgataacacttcaaggtattgggaacctgagttttatgaggctatgtacacaccgcatacagtcttacaggctgttggggcttgtgttctttgcaattcacagacttcattaagatgtggtgcttgcatacgtagaccattcttatgttgtaaatgctgttacgaccatgtcatatcaacatcacataaattagtcttgtctgttaatccgtatgtttgcaatgctccaggttgtgatgtcacagatgtgactcaactttacttaggaggtatgagctattattgtaaatcacataaaccacccattagttttccattgtgtgctaatggacaagtttttggtttatataaaaatacatgtgttggtagcgataatgttactgactttaatgcaattgcaacatgtgactggacaaatgctggtgattacattttagctaacacctgtactgaaagactcaagctttttgcagcagaaacgctcaaagctactgaggagacatttaaactgtcttatggtattgctactgtacgtgaagtgctgtctgacagagaattacatctttcatgggaagttggtaaacctagaccaccacttaaccgaaattatgtctttactggttatcgtgtaactaaaaacagtaaagtacaaataggagagtacacctttgaaaaaggtgactatggtgatgctgttgtttaccgaggtacaacaacttacaaattaaatgttggtgattattttgtgctgacatcacatacagtaatgccattaagtgcacctacactagtgccacaagagcactatgttagaattactggcttatacccaacactcaatatctcagatgagttttctagcaatgttgcaaattatcaaaaggttggtatgcaaaagtattctacactccagggaccacctggtactggtaagagtcattttgctattggcctagctctctactacccttctgctcgcatagtgtatacagcttgctctcatgccgctgttgatgcactatgtgagaaggcattaaaatatttgcctatagataaatgtagtagaattatacctgcacgtgctcgtgtagagtgttttgataaattcaaagtgaattcaacattagaacagtatgtcttttgtactgtaaatgcattgcctgagacgacagcagatatagttgtctttgatgaaatttcaatggccacaaattatgatttgagtgttgtcaatgccagattacgtgctaagcactatgtgtacattggcgaccctgctcaattacctgcaccacgcacattgctaactaagggcacactagaaccagaatatttcaattcagtgtgtagacttatgaaaactataggtccagacatgttcctcggaacttgtcggcgttgtcctgctgaaattgttgacactgtgagtgctttggtttatgataataagcttaaagcacataaagacaaatcagctcaatgctttaaaatgttttataagggtgttatcacgcatgatgtttcatctgcaattaacaggccacaaataggcgtggtaagagaattccttacacgtaaccctgcttggagaaaagctgtctttatttcaccttataattcacagaatgctgtagcctcaaagattttgggactaccaactcaaactgttgattcatcacagggctcagaatatgactatgtcatattcactcaaaccactgaaacagctcactcttgtaatgtaaacagatttaatgttgctattaccagagcaaaagtaggcatactttgcataatgtctgatagagacctttatgacaagttgcaatttacaagtcttgaaattccacgtaggaatgtggcaactttacaagctgaaaatgtaacaggactctttaaagattgtagtaaggtaatcactgggttacatcctacacaggcacctacacacctcagtgttgacactaaattcaaaactgaaggtttatgtgttgacatacctggcatacctaaggacatgacctatagaagactcatctctatgatgggttttaaaatgaattatcaagttaatggttaccctaacatgtttatcacccgcgaagaagctataagacatgtacgtgcatggattggcttcgatgtcgaggggtgtcatgctactagagaagctgttggtaccaatttacctttacagctaggtttttctacaggtgttaacctagttgctgtacctacaggttatgttgatacacctaataatacagatttttccagagttagtgctaaaccaccgcctggagatcaatttaaacacctcataccacttatgtacaaaggacttccttggaatgtagtgcgtataaagattgtacaaatgttaagtgacacacttaaaaatctctctgacagagtcgtatttgtcttatgggcacatggctttgagttgacatctatgaagtattttgtgaaaataggacctgagcgcacctgttgtctatgtgatagacgtgccacatgcttttccactgcttcagacacttatgcctgttggcatcattctattggatttgattacgtctataatccgtttatgattgatgttcaacaatggggttttacaggtaacctacaaagcaaccatgatctgtattgtcaagtccatggtaatgcacatgtagctagttgtgatgcaatcatgactaggtgtctagctgtccacgagtgctttgttaagcgtgttgactggactattgaatatcctataattggtgatgaactgaagattaatgcggcttgtagaaaggttcaacacatggttgttaaagctgcattattagcagacaaattcccagttcttcacgacattggtaaccctaaagctattaagtgtgtacctcaagctgatgtagaatggaagttctatgatgcacagccttgtagtgacaaagcttataaaatagaagaattattctattcttatgccacacattctgacaaattcacagatggtgtatgcctattttggaattgcaatgtcgatagatatcctgctaattccattgtttgtagatttgacactagagtgctatctaaccttaacttgcctggttgtgatggtggcagtttgtatgtaaataaacatgcattccacacaccagcttttgataaaagtgcttttgttaatttaaaacaattaccatttttctattactctgacagtccatgtgagtctcatggaaaacaagtagtgtcagatatagattatgtaccactaaagtctgctacgtgtataacacgttgcaatttaggtggtgctgtctgtagacatcatgctaatgagtacagattgtatctcgatgcttataacatgatgatctcagctggctttagcttgtgggtttacaaacaatttgatacttataacctctggaacacttttacaagacttcagagtttagaaaatgtggcttttaatgttgtaaataagggacactttgatggacaacagggtgaagtaccagtttctatcattaataacactgtttacacaaaagttgatggtgttgatgtagaattgtttgaaaataaaacaacattacctgttaatgtagcatttgagctttgggctaagcgcaacattaaaccagtaccagaggtgaaaatactcaataatttgggtgtggacattgctgctaatactgtgatctgggactacaaaagagatgctccagcacatatatctactattggtgtttgttctatgactgacatagccaagaaaccaactgaaacgatttgtgcaccactcactgtcttttttgatggtagagttgatggtcaagtagacttatttagaaatgcccgtaatggtgttcttattacagaaggtagtgttaaaggtttacaaccatctgtgggtcccaaacaagctagtcttaatggagtcacattaattggagaagccgtaaaaacacagttcaattattataagaaagttgatggtgttgtccaacaattacctgaaacttactttactcagagtagaaatttacaagaatttaaacccaggagtcaaatggaaattgatttcttagaattagctatggatgaattcattgaacggtataaattagaaggctatgccttcgaacatatcgtttatggagattttagtcatagtcagttaggtggtttacatctactgattggactagctaaacgttttaaggaatcaccttttgaattagaagattttattcctatggacagtacagttaaaaactatttcataacagatgcgcaaacaggttcatctaagtgtgtgtgttctgttattgatttattacttgatgattttgttgaaataataaaatcccaagatttatctgtagtttctaaggttgtcaaagtgactattgactatacagaaatttcatttatgctttggtgtaaagatggccatgtagaaacattttacccaaaattacaatctagtcaagcgtggcaaccgggtgttgctatgcctaatctttacaaaatgcaaagaatgctattagaaaagtgtgaccttcaaaattatggtgatagtgcaacattacctaaaggcataatgatgaatgtcgcaaaatatactcaactgtgtcaatatttaaacacattaacattagctgtaccctataatatgagagttatacattttggtgctggttctgataaaggagttgcaccaggtacagctgttttaagacagtggttgcctacgggtacgctgcttgtcgattcagatcttaatgactttgtctctgatgcagattcaactttgattggtgattgtgcaactgtacatacagctaataaatgggatctcattattagtgatatgtacgaccctaagactaaaaatgttacaaaagaaaatgactctaaagagggttttttcacttacatttgtgggtttatacaacaaaagctagctcttggaggttccgtggctataaagataacagaacattcttggaatgctgatctttataagctcatgggacacttcgcatggtggacagcctttgttactaatgtgaatgcgtcatcatctgaagcatttttaattggatgtaattatcttggcaaaccacgcgaacaaatagatggttatgtcatgcatgcaaattacatattttggaggaatacaaatccaattcagttgtcttcctattctttatttgacatgagtaaatttccccttaaattaaggggtactgctgttatgtctttaaaagaaggtcaaatcaatgatatgattttatctcttcttagtaaaggtagacttataattagagaaaacaacagagttgttatttctagtgatgttcttgttaacaactaaacgaacaatgtttgtttttcttgttttattgccactagtctctagtcagtgtgttaatcttacaaccagaactcaattaccccctgcatacactaattctttcacacgtggtgtttattaccctgacaaagttttcagatcctcagttttacattcaactcaggacttgttcttacctttcttttccaatgttacttggttccatgctatacatgtctctgggaccaatggtactaagaggtttgataaccctgtcctaccatttaatgatggtgtttattttgcttccactgagaagtctaacataataagaggctggatttttggtactactttagattcgaagacccagtccctacttattgttaataacgctactaatgttgttattaaagtctgtgaatttcaattttgtaatgatccatttttgggtgtttattaccacaaaaacaacaaaagttggatggaaagtgagttcagagtttattctagtgcgaataattgcacttttgaatatgtctctcagccttttcttatggaccttgaaggaaaacagggtaatttcaaaaatcttagggaatttgtgtttaagaatattgatggttattttaaaatatattctaagcacacgcctattaatttagtgcgtgatctccctcagggtttttcggctttagaaccattggtagatttgccaataggtattaacatcactaggtttcaaactttacttgctttacatagaagttatttgactcctggtgattcttcttcaggttggacagctggtgctgcagcttattatgtgggttatcttcaacctaggacttttctattaaaatataatgaaaatggaaccattacagatgctgtagactgtgcacttgaccctctctcagaaacaaagtgtacgttgaaatccttcactgtagaaaaaggaatctatcaaacttctaactttagagtccaaccaacagaatctattgttagatttcctaatattacaaacttgtgcccttttggtgaagtttttaacgccaccagatttgcatctgtttatgcttggaacaggaagagaatcagcaactgtgttgctgattattctgtcctatataattccgcatcattttccacttttaagtgttatggagtgtctcctactaaattaaatgatctctgctttactaatgtctatgcagattcatttgtaattagaggtgatgaagtcagacaaatcgctccagggcaaactggaaagattgctgattataattataaattaccagatgattttacaggctgcgttatagcttggaattctaacaatcttgattctaaggttggtggtaattataattacctgtatagattgtttaggaagtctaatctcaaaccttttgagagagatatttcaactgaaatctatcaggccggtagcacaccttgtaatggtgttgaaggttttaattgttactttcctttacaatcatatggtttccaacccactaatggtgttggttaccaaccatacagagtagtagtactttcttttgaacttctacatgcaccagcaactgtttgtggacctaaaaagtctactaatttggttaaaaacaaatgtgtcaatttcaacttcaatggtttaacaggcacaggtgttcttactgagtctaacaaaaagtttctgcctttccaacaatttggcagagacattgctgacactactgatgctgtccgtgatccacagacacttgagattcttgacattacaccatgttcttttggtggtgtcagtgttataacaccaggaacaaatacttctaaccaggttgctgttctttatcaggatgttaactgcacagaagtccctgttgctattcatgcagatcaacttactcctacttggcgtgtttattctacaggttctaatgtttttcaaacacgtgcaggctgtttaataggggctgaacatgtcaacaactcatatgagtgtgacatacccattggtgcaggtatatgcgctagttatcagactcagactaattctcctcggcgggcacgtagtgtagctagtcaatccatcattgcctacactatgtcacttggtgcagaaaattcagttgcttactctaataactctattgccatacccacaaattttactattagtgttaccacagaaattctaccagtgtctatgaccaagacatcagtagattgtacaatgtacatttgtggtgattcaactgaatgcagcaatcttttgttgcaatatggcagtttttgtacacaattaaaccgtgctttaactggaatagctgttgaacaagacaaaaacacccaagaagtttttgcacaagtcaaacaaatttacaaaacaccaccaattaaagattttggtggttttaatttttcacaaatattaccagatccatcaaaaccaagcaagaggtcatttattgaagatctacttttcaacaaagtgacacttgcagatgctggcttcatcaaacaatatggtgattgccttggtgatattgctgctagagacctcatttgtgcacaaaagtttaacggccttactgttttgccacctttgctcacagatgaaatgattgctcaatacacttctgcactgttagcgggtacaatcacttctggttggacctttggtgcaggtgctgcattacaaataccatttgctatgcaaatggcttataggtttaatggtattggagttacacagaatgttctctatgagaaccaaaaattgattgccaaccaatttaatagtgctattggcaaaattcaagactcactttcttccacagcaagtgcacttggaaaacttcaagatgtggtcaaccaaaatgcacaagctttaaacacgcttgttaaacaacttagctccaattttggtgcaatttcaagtgttttaaatgatatcctttcacgtcttgacaaagttgaggctgaagtgcaaattgataggttgatcacaggcagacttcaaagtttgcagacatatgtgactcaacaattaattagagctgcagaaatcagagcttctgctaatcttgctgctactaaaatgtcagagtgtgtacttggacaatcaaaaagagttgatttttgtggaaagggctatcatcttatgtccttccctcagtcagcacctcatggtgtagtcttcttgcatgtgacttatgtccctgcacaagaaaagaacttcacaactgctcctgccatttgtcatgatggaaaagcacactttcctcgtgaaggtgtctttgtttcaaatggcacacactggtttgtaacacaaaggaatttttatgaaccacaaatcattactacagacaacacatttgtgtctggtaactgtgatgttgtaataggaattgtcaacaacacagtttatgatcctttgcaacctgaattagactcattcaaggaggagttagataaatattttaagaatcatacatcaccagatgttgatttaggtgacatctctggcattaatgcttcagttgtaaacattcaaaaagaaattgaccgcctcaatgaggttgccaagaatttaaatgaatctctcatcgatctccaagaacttggaaagtatgagcagtatataaaatggccatggtacatttggctaggttttatagctggcttgattgccatagtaatggtgacaattatgctttgctgtatgaccagttgctgtagttgtctcaagggctgttgttcttgtggatcctgctgcaaatttgatgaagacgactctgagccagtgctcaaaggagtcaaattacattacacataaacgaacttatggatttgtttatgagaatcttcacaattggaactgtaactttgaagcaaggtgaaatcaaggatgctactccttcagattttgttcgcgctactgcaacgataccgatacaagcctcactccctttcggatggcttattgttggcgttgcacttcttgctgtttttcagagcgcttccaaaatcataaccctcaaaaagagatggcaactagcactctccaagggtgttcactttgtttgcaacttgctgttgttgtttgtaacagtttactcacaccttttgctcgttgctgctggccttgaagccccttttctctatctttatgctttagtctacttcttgcagagtataaactttgtaagaataataatgaggctttggctttgctggaaatgccgttccaaaaacccattactttatgatgccaactattttctttgctggcatactaattgttacgactattgtataccttacaatagtgtaacttcttcaattgtcattacttcaggtgatggcacaacaagtcctatttctgaacatgactaccagattggtggttatactgaaaaatgggaatctggagtaaaagactgtgttgtattacacagttacttcacttcagactattaccagctgtactcaactcaattgagtacagacactggtgttgaacatgttaccttcttcatctacaataaaattgttgatgagcctgaagaacatgtccaaattcacacaatcgacggttcatccggagttgttaatccagtaatggaaccaatttatgatgaaccgacgacgactactagcgtgcctttgtaagcacaagctgatgagtacgaacttatgtactcattcgtttcggaagagacaggtacgttaatagttaatagcgtacttctttttcttgctttcgtggtattcttgctagttacactagccatccttactgcgcttcgattgtgtgcgtactgctgcaatattgttaacgtgagtcttgtaaaaccttctttttacgtttactctcgtgttaaaaatctgaattcttctagagttcctgatcttctggtctaaacgaactaaatattatattagtttttctgtttggaactttaattttagccatggcagattccaacggtactattaccgttgaagagcttaaaaagctccttgaacaatggaacctagtaataggtttcctattccttacatggatttgtcttctacaatttgcctatgccaacaggaataggtttttgtatataattaagttaattttcctctggctgttatggccagtaactttagcttgttttgtgcttgctgctgtttacagaataaattggatcaccggtggaattgctatcgcaatggcttgtcttgtaggcttgatgtggctcagctacttcattgcttctttcagactgtttgcgcgtacccgttccatgtggtcattcaatccagaaactaacattcttctcaacgtgccactccatggcactattctgaccagaccgcttctagaaagtgaactcgtaatcggagctgtgatccttcgtggacatcttcgtattgctggacaccatctaggacgctgtgacatcaaggacctgcctaaagaaatcactgttgctacatcccgcacgctttcttattacaaattgggagcttcgcagcgtgtagcaggtgactcaggttttgctgcatacagtcgctacaggattggcaactataaattaaacacagaccattccagtagcagtgacaatattgctttgcttgtacagtaagtgacaacagaaccaatggagattgattaaacgaacatgaaaattattcttttcttggcactgataacactcgctacttgtgagctttatcactaccaagagtgtgttagaggtacaacagtacttttaaaagaaccttgctcttctggaacatacgagggcaattcaccatttcatcctctagctgataacaaatttgcactgacttgctttagcactcaatttgcttttgcttgtcctgacggcgtaaaacacgtctatcagttacgtgccagatcagtttcacctaaactgttcatcagacaagaggaagttcaagaactttactctccaatttttcttattgttgcggcaatagtgtttataacactttgcttcacactcaaaagaaagacagaatgattgaactttcattaattgacttctatttgtgctttttagcctttctgctattccttgttttaattatgcttattatcttttggttctcacttgaactgcaagatcataatgaaacttgtcacgcctaaacgaacatgaaatttcttgttttcttaggaatcatcacaactgtagctgcatttcaccaagaatgtagtttacagtcatgtactcaacatcaaccatatgtagttgatgacccgtgtcctattcacttctattctaaatggtatattagagtaggagctagaaaatcagcacctttaattgaattgtgcgtggatgaggctggttctaaatcacccattcagtacatcgatatcggtaattatacagtttcctgtttaccttttacaattaattgccaggaacctaaattgggtagtcttgtagtgcgttgttcgttctatgaagactttttagagtatcatgacgttcgtgttgttttagatttcatctaaacgaacaaactaaaatgtctgataatggaccccaaaatcagcgaaatgcaccccgcattacgtttggtggaccctcagattcaactggcagtaaccagaatggagaacgcagtggggcgcgatcaaaacaacgtcggccccaaggtttacccaataatactgcgtcttggttcaccgctctcactcaacatggcaaggaagaccttaaattccctcgaggacaaggcgttccaattaacaccaatagcagtccagatgaccaaattggctactaccgaagagctaccagacgaattcgtggtggtgacggtaaaatgaaagatctcagtccaagatggtatttctactacctaggaactgggccagaagctggacttccctatggtgctaacaaagacggcatcatatgggttgcaactgagggagccttgaatacaccaaaagatcacattggcacccgcaatcctgctaacaatgctgcaatcgtgctacaacttcctcaaggaacaacattgccaaaaggcttctacgcagaagggagcagaggcggcagtcaagcctcttctcgttcctcatcacgtagtcgcaacagttcaagaaattcaactccaggcagcagtaggggaacttctcctgctagaatggctggcaatggcggtgatgctgctcttgctttgctgctgcttgacagattgaaccagcttgagagcaaaatgtctggtaaaggccaacaacaacaaggccaaactgtcactaagaaatctgctgctgaggcttctaagaagcctcggcaaaaacgtactgccactaaagcatacaatgtaacacaagctttcggcagacgtggtccagaacaaacccaaggaaattttggggaccaggaactaatcagacaaggaactgattacaaacattggccgcaaattgcacaatttgcccccagcgcttcagcgttcttcggaatgtcgcgcattggcatggaagtcacaccttcgggaacgtggttgacctacacaggtgccatcaaattggatgacaaagatccaaatttcaaagatcaagtcattttgctgaataagcatattgacgcatacaaaacattcccaccaacagagcctaaaaaggacaaaaagaagaaggctgatgaaactcaagccttaccgcagagacagaagaaacagcaaactgtgactcttcttcctgctgcagatttggatgatttctccaaacaattgcaacaatccatgagcagtgctgactcaactcaggcctaaactcatgcagaccacacaaggcagatgggctatataaacgttttcgcttttccgtttacgatatatagtctactcttgtgcagaatgaattctcgtaactacatagcacaagtagatgtagttaactttaatctcacatagcaatctttaatcagtgtgtaacattagggaggacttgaaagagccaccacattttcaccgaggccacgcggagtacgatcgagtgtacagtgaacaatgctagggagagctgcctatatggaagagccctaatgtgtaaaattaattttagtagtgctatccccatgtgattttaatagcttcttaggagaatgacaaaaaaaaaaaaaaaaaaaaaaaaa

SEQ ID NO: 19 - DNA, 29523 bp, Coronaviridae
  misc_feature 1..29523: note = SARS-CoV-2-7, includes the deletion of both 7a and 7b genes
  source 1..29523: mol_type = other DNA
attaaaggtttataccttcccaggtaacaaaccaaccaactttcgatctcttgtagatctgttctctaaacgaactttaaaatctgtgtggctgtcactcggctgcatgcttagtgcactcacgcagtataattaataactaattactgtcgttgacaggacacgagtaactcgtctatcttctgcaggctgcttacggtttcgtccgtgttgcagccgatcatcagcacatctaggtttcgtccgggtgtgaccgaaaggtaagatggagagccttgtccctggtttcaacgagaaaacacacgtccaactcagtttgcctgttttacaggttcgcgacgtgctcgtacgtggctttggagactccgtggaggaggtcttatcagaggcacgtcaacatcttaaagatggcacttgtggcttagtagaagttgaaaaaggcgttttgcctcaacttgaacagccctatgtgttcatcaaacgttcggatgctcgaactgcacctcatggtcatgttatggttgagctggtagcagaactcgaaggcattcagtacggtcgtagtggtgagacacttggtgtccttgtccctcatgtgggcgaaataccagtggcttaccgcaaggttcttcttcgtaagaacggtaataaaggagctggtggccatagttacggcgccgatctaaagtcatttgacttaggcgacgagcttggcactgatccttatgaagattttcaagaaaactggaacactaaacatagcagtggtgttacccgtgaactcatgcgtgagcttaacggaggggcatacactcgctatgtcgataacaacttctgtggccctgatggctaccctcttgagtgcattaaagaccttctagcacgtgctggtaaagcttcatgcactttgtccgaacaactggactttattgacactaagaggggtgtatactgctgccgtgaacatgagcatgaaattgcttggtacacggaacgttctgaaaagagctatgaattgcagacaccttttgaaattaaattggcaaagaaatttgacaccttcaatggggaatgtccaaattttgtatttcccttaaattccataatcaagactattcaaccaagggttgaaaagaaaaagcttgatggctttatgggtagaattcgatctgtctatccagttgcgtcaccaaatgaatgcaaccaaatgtgcctttcaactctcatgaagtgtgatcattgtggtgaaacttcatggcagacgggcgattttgttaaagccacttgcgaattttgtggcactgagaatttgactaaagaaggtgccactacttgtggttacttaccccaaaatgctgttgttaaaatttattgtccagcatgtcacaattcagaagtaggacctgagcatagtcttgccgaataccataatgaatctggcttgaaaaccattcttcgtaagggtggtcgcactattgcctttggaggctgtgtgttctcttatgttggttgccataacaagtgtgcctattgggttccacgtgctagcgctaacataggttgtaaccatacaggtgttgttggagaaggttccgaaggtcttaatgacaaccttcttgaaatactccaaaaagagaaagtcaacatcaatattgttggtgactttaaacttaatgaagagatcgccattattttggcatctttttctgcttccacaagtgcttttgtggaaactgtgaaaggtttggattataaagcattcaaacaaattgttgaatcctgtggtaattttaaagttacaaaaggaaaagctaaaaaaggtgcctggaatattggtgaacagaaatcaatactgagtcctctttatgcatttgcatcagaggctgctcgtgttgtacgatcaattttctcccgcactcttgaaactgctcaaaattctgtgcgtgttttacagaaggccgctataacaatactagatggaatttcacagtattcactgagactcattgatgctatgatgttcacatctgatttggctactaacaatctagttgtaatggcctacattacaggtggtgttgttcagttgacttcgcagtggctaactaacatctttggcactgtttatgaaaaactcaaacccgtccttgattggcttgaagagaagtttaaggaaggtgtagagtttcttagagacggttgggaaattgttaaatttatctcaacctgtgcttgtgaaattgtcggtggacaaattgtcacctgtgcaaaggaaattaaggagagtgttcagacattctttaagcttgtaaataaatttttggctttgtgtgctgactctatcattattggtggagctaaacttaaagccttgaatttaggtgaaacatttgtcacgcactcaaagggattgtacagaaagtgtgttaaatccagagaagaaactggcctactcatgcctctaaaagccccaaaagaaattatcttcttagagggagaaacacttcccacagaagtgttaacagaggaagttgtcttgaaaactggtgatttacaaccattagaacaacctactagtgaagctgttgaagctccattggttggtacaccagtttgtattaacgggcttatgttgctcgaaatcaaagacacagaaaagtactgtgcccttgcacctaatatgatggtaacaaacaataccttcacactcaaaggcggtgcaccaacaaaggttacttttggtgatgacactgtgatagaagtgcaaggttacaagagtgtgaatatcacttttgaacttgatgaaaggattgataaagtacttaatgagaagtgctctgcctatacagttgaactcggtacagaagtaaatgagttcgcctgtgttgtggcagatgctgtcataaaaactttgcaaccagtatctgaattacttacaccactgggcattgatttagatgagtggagtatggctacatactacttatttgatgagtctggtgagtttaaattggcttcacatatgtattgttctttctaccctccagatgaggatgaagaagaaggtgattgtgaagaagaagagtttgagccatcaactcaatatgagtatggtactgaagatgattaccaaggtaaacctttggaatttggtgccacttctgctgctcttcaacctgaagaagagcaagaagaagattggttagatgatgatagtcaacaaactgttggtcaacaagacggcagtgaggacaatcagacaactactattcaaacaattgttgaggttcaacctcaattagagatggaacttacaccagttgttcagactattgaagtgaatagttttagtggttatttaaaacttactgacaatgtatacattaaaaatgcagacattgtggaagaagctaaaaaggtaaaaccaacagtggttgttaatgcagccaatgtttaccttaaacatggaggaggtgttgcaggagccttaaataaggctactaacaatgccatgcaagttgaatctgatgattacatagctactaatggaccacttaaagtgggtggtagttgtgttttaagcggacacaatcttgctaaacactgtcttcatgttgtcggcccaaatgttaacaaaggtgaagacattcaacttcttaagagtgcttatgaaaattttaatcagcacgaagttctacttgcaccattattatcagctggtatttttggtgctgaccctatacattctttaagagtttgtgtagatactgttcgcacaaatgtctacttagctgtctttgataaaaatctctatgacaaacttgtttcaagctttttggaaatgaagagtgaaaagcaagttgaacaaaagatcgctgagattcctaaagaggaagttaagccatttataactgaaagtaaaccttcagttgaacagagaaaacaagatgataagaaaatcaaagcttgtgttgaagaagttacaacaactctggaagaaactaagttcctcacagaaaacttgttactttatattgacattaatggcaatcttcatccagattctgccactcttgttagtgacattgacatcactttcttaaagaaagatgctccatatatagtgggtgatgttgttcaagagggtgttttaactgctgtggttatacctactaaaaaggctggtggcactactgaaatgctagcgaaagctttgagaaaagtgccaacagacaattatataaccacttacccgggtcagggtttaaatggttacactgtagaggaggcaaagacagtgcttaaaaagtgtaaaagtgccttttacattctaccatctattatctctaatgagaagcaagaaattcttggaactgtttcttggaatttgcgagaaatgcttgcacatgcagaagaaacacgcaaattaatgcctgtctgtgtggaaactaaagccatagtttcaactatacagcgtaaatataagggtattaaaatacaagagggtgtggttgattatggtgctagattttacttttacaccagtaaaacaactgtagcgtcacttatcaacacacttaacgatctaaatgaaactcttgttacaatgccacttggctatgtaacacatggcttaaatttggaagaagctgctcggtatatgagatctctcaaagtgccagctacagtttctgtttcttcacctgatgctgttacagcgtataatggttatcttacttcttcttctaaaacacctgaagaacattttattgaaaccatctcacttgctggttcctataaagattggtcctattctggacaatctacacaactaggtatagaatttcttaagagaggtgataaaagtgtatattacactagtaatcctaccacattccacctagatggtgaagttatcacctttgacaatcttaagacacttctttctttgagagaagtgaggactattaaggtgtttacaacagtagacaacattaacctccacacgcaagttgtggacatgtcaatgacatatggacaacagtttggtccaacttatttggatggagctgatgttactaaaataaaacctcataattcacatgaaggtaaaacattttatgttttacctaatgatgacactctacgtgttgaggcttttgagtactaccacacaactgatcctagttttctgggtaggtacatgtcagcattaaatcacactaaaaagtggaaatacccacaagttaatggtttaacttctattaaatgggcagataacaactgttatcttgccactgcattgttaacactccaacaaatagagttgaagtttaatccacctgctctacaagatgcttattacagagcaagggctggtgaagctgctaacttttgtgcacttatcttagcctactgtaataagacagtaggtgagttaggtgatgttagagaaacaatgagttacttgtttcaacatgccaatttagattcttgcaaaagagtcttgaacgtggtgtgtaaaacttgtggacaacagcagacaacccttaagggtgtagaagctgttatgtacatgggcacactttcttatgaacaatttaagaaaggtgttcagataccttgtacgtgtggtaaacaagctacaaaatatctagtacaacaggagtcaccttttgttatgatgtcagcaccacctgctcagtatgaacttaagcatggtacatttacttgtgctagtgagtacactggtaattaccagtgtggtcactataaacatataacttctaaagaaactttgtattgcatagacggtgctttacttacaaagtcctcagaatacaaaggtcctattacggatgttttctacaaagaaaacagttacacaacaaccataaaaccagttacttataaattggatggtgttgtttgtacagaaattgaccctaagttggacaattattataagaaagacaattcttatttcacagagcaaccaattgatcttgtaccaaaccaaccatatccaaacgcaagcttcgataattttaagtttgtatgtgataatatcaaatttgctgatgatttaaaccagttaactggttataagaaacctgcttcaagagagcttaaagttacatttttccctgacttaaatggtgatgtggtggctattgattataaacactacacaccctcttttaagaaaggagctaaattgttacataaacctattgtttggcatgttaacaatgcaactaataaagccacgtataaaccaaatacctggtgtatacgttgtctttggagcacaaaaccagttgaaacatcaaattcgtttgatgtactgaagtcagaggacgcgcagggaatggataatcttgcctgcgaagatctaaaaccagtctctgaagaagtagtggaaaatcctaccatacagaaagacgttcttgagtgtaatgtgaaaactaccgaagttgtaggagacattatacttaaaccagcaaataatagtttaaaaattacagaagaggttggccacacagatctaatggctgcttatgtagacaattctagtcttactattaagaaacctaatgaattatctagagtattaggtttgaaaacccttgctactcatggtttagctgctgttaatagtgtcccttgggatactatagctaattatgctaagccttttcttaacaaagttgttagtacaactactaacatagttacacggtgtttaaaccgtgtttgtactaattatatgccttatttctttactttattgctacaattgtgtacttttactagaagtacaaattctagaattaaagcatctatgccgactactatagcaaagaatactgttaagagtgtcggtaaattttgtctagaggcttcatttaattatttgaagtcacctaatttttctaaactgataaatattataatttggtttttactattaagtgtttgcctaggttctttaatctactcaaccgctgctttaggtgttttaatgtctaatttaggcatgccttcttactgtactggttacagagaaggctatttgaactctactaatgtcactattgcaacctactgtactggttctataccttgtagtgtttgtcttagtggtttagattctttagacacctatccttctttagaaactatacaaattaccatttcatcttttaaatgggatttaactgcttttggcttagttgcagagtggtttttggcatatattcttttcactaggtttttctatgtacttggattggctgcaatcatgcaattgtttttcagctattttgcagtacattttattagtaattcttggcttatgtggttaataattaatcttgtacaaatggccccgatttcagctatggttagaatgtacatcttctttgcatcattttattatgtatggaaaagttatgtgcatgttgtagacggttgtaattcatcaacttgtatgatgtgttacaaacgtaatagagcaacaagagtcgaatgtacaactattgttaatggtgttagaaggtccttttatgtctatgctaatggaggtaaaggcttttgcaaactacacaattggaattgtgttaattgtgatacattctgtgctggtagtacatttattagtgatgaagttgcgagagacttgtcactacagtttaaaagaccaataaatcctactgaccagtcttcttacatcgttgatagtgttacagtgaagaatggttccatccatctttactttgataaagctggtcaaaagacttatgaaagacattctctctctcattttgttaacttagacaacctgagagctaataacactaaaggttcattgcctattaatgttatagtttttgatggtaaatcaaaatgtgaagaatcatctgcaaaatcagcgtctgtttactacagtcagcttatgtgtcaacctatactgttactagatcaggcattagtgtctgatgttggtgatagtgcggaagttgcagttaaaatgtttgatgcttacgttaatacgttttcatcaacttttaacgtaccaatggaaaaactcaaaacactagttgcaactgcagaagctgaacttgcaaagaatgtgtccttagacaatgtcttatctacttttatttcagcagctcggcaagggtttgttgattcagatgtagaaactaaagatgttgttgaatgtcttaaattgtcacatcaatctgacatagaagttactggcgatagttgtaataactatatgctcacctataacaaagttgaaaacatgacaccccgtgaccttggtgcttgtattgactgtagtgcgcgtcatattaatgcgcaggtagcaaaaagtcacaacattgctttgatatggaacgttaaagatttcatgtcattgtctgaacaactacgaaaacaaatacgtagtgctgctaaaaagaataacttaccttttaagttgacatgtgcaactactagacaagttgttaatgttgtaacaacaaagatagcacttaagggtggtaaaattgttaataattggttgaagcagttaattaaagttacacttgtgttcctttttgttgctgctattttctatttaataacacctgttcatgtcatgtctaaacatactgacttttcaagtgaaatcataggatacaaggctattgatggtggtgtcactcgtgacatagcatctacagatacttgttttgctaacaaacatgctgattttgacacatggtttagccagcgtggtggtagttatactaatgacaaagcttgcccattgattgctgcagtcataacaagagaagtgggttttgtcgtgcctggtttgcctggcacgatattacgcacaactaatggtgactttttgcatttcttacctagagtttttagtgcagttggtaacatctgttacacaccatcaaaacttatagagtacactgactttgcaacatcagcttgtgttttggctgctgaatgtacaatttttaaagatgcttctggtaagccagtaccatattgttatgataccaatgtactagaaggttctgttgcttatgaaagtttacgccctgacacacgttatgtgctcatggatggctctattattcaatttcctaacacctaccttgaaggttctgttagagtggtaacaacttttgattctgagtactgtaggcacggcacttgtgaaagatcagaagctggtgtttgtgtatctactagtggtagatgggtacttaacaatgattattacagatctttaccaggagttttctgtggtgtagatgctgtaaatttacttactaatatgtttacaccactaattcaacctattggtgctttggacatatcagcatctatagtagctggtggtattgtagctatcgtagtaacatgccttgcctactattttatgaggtttagaagagcttttggtgaatacagtcatgtagttgcctttaatactttactattccttatgtcattcactgtactctgtttaacaccagtttactcattcttacctggtgtttattctgttatttacttgtacttgacattttatcttactaatgatgtttcttttttagcacatattcagtggatggttatgttcacacctttagtacctttctggataacaattgcttatatcatttgtatttccacaaagcatttctattggttctttagtaattacctaaagagacgtgtagtctttaatggtgtttcctttagtacttttgaagaagctgcgctgtgcacctttttgttaaataaagaaatgtatctaaagttgcgtagtgatgtgctattacctcttacgcaatataatagatacttagctctttataataagtacaagtattttagtggagcaatggatacaactagctacagagaagctgcttgttgtcatctcgcaaaggctctcaatgacttcagtaactcaggttctgatgttctttaccaaccaccacaaacctctatcacctcagctgttttgcagagtggttttagaaaaatggcattcccatctggtaaagttgagggttgtatggtacaagtaacttgtggtacaactacacttaacggtctttggcttgatgacgtagtttactgtccaagacatgtgatctgcacctctgaagacatgcttaaccctaattatgaagatttactcattcgtaagtctaatcataatttcttggtacaggctggtaatgttcaactcagggttattggacattctatgcaaaattgtgtacttaagcttaaggttgatacagccaatcctaagacacctaagtataagtttgttcgcattcaaccaggacagactttttcagtgttagcttgttacaatggttcaccatctggtgtttaccaatgtgctatgaggcccaatttcactattaagggttcattccttaatggttcatgtggtagtgttggttttaacatagattatgactgtgtctctttttgttacatgcaccatatggaattaccaactggagttcatgctggcacagacttagaaggtaacttttatggaccttttgttgacaggcaaacagcacaagcagctggtacggacacaactattacagttaatgttttagcttggttgtacgctgctgttataaatggagacaggtggtttctcaatcgatttaccacaactcttaatgactttaaccttgtggctatgaagtacaattatgaacctctaacacaagaccatgttgacatactaggacctctttctgctcaaactggaattgccgttttagatatgtgtgcttcattaaaagaattactgcaaaatggtatgaatggacgtaccatattgggtagtgctttattagaagatgaatttacaccttttgatgttgttagacaatgctcaggtgttactttccaaagtgcagtgaaaagaacaatcaagggtacacaccactggttgttactcacaattttgacttcacttttagttttagtccagagtactcaatggtctttgttcttttttttgtatgaaaatgcctttttaccttttgctatgggtattattgctatgtctgcttttgcaatgatgtttgtcaaacataagcatgcatttctctgtttgtttttgttaccttctcttgccactgtagcttattttaatatggtctatatgcctgctagttgggtgatgcgtattatgacatggttggatatggttgatactagtttgtctggttttaagctaaaagactgtgttatgtatgcatcagctgtagtgttactaatccttatgacagcaagaactgtgtatgatgatggtgctaggagagtgtggacacttatgaatgtcttgacactcgtttataaagtttattatggtaatgctttagatcaagccatttccatgtgggctcttataatctctgttacttctaactactcaggtgtagttacaactgtcatgtttttggccagaggtattgtttttatgtgtgttgagtattgccctattttcttcataactggtaatacacttcagtgtataatgctagtttattgtttcttaggctatttttgtacttgttactttggcctcttttgtttactcaaccgctactttagactgactcttggtgtttatgattacttagtttctacacaggagtttagatatatgaattcacagggactactcccacccaagaatagcatagatgccttcaaactcaacattaaattgttgggtgttggtggcaaaccttgtatcaaagtagccactgtacagtctaaaatgtcagatgtaaagtgcacatcagtagtcttactctcagttttgcaacaactcagagtagaatcatcatctaaattgtgggctcaatgtgtccagttacacaatgacattctcttagctaaagatactactgaagcctttgaaaaaatggtttcactactttctgttttgctttccatgcagggtgctgtagacataaacaagctttgtgaagaaatgctggacaacagggcaaccttacaagctatagcctcagagtttagttcccttccatcatatgcagcttttgctactgctcaagaagcttatgagcaggctgttgctaatggtgattctgaagttgttcttaaaaagttgaagaagtctttgaatgtggctaaatctgaatttgaccgtgatgcagccatgcaacgtaagttggaaaagatggctgatcaagctatgacccaaatgtataaacaggctagatctgaggacaagagggcaaaagttactagtgctatgcagacaatgcttttcactatgcttagaaagttggataatgatgcactcaacaacattatcaacaatgcaagagatggttgtgttcccttgaacataatacctcttacaacagcagccaaactaatggttgtcataccagactataacacatataaaaatacgtgtgatggtacaacatttacttatgcatcagcattgtgggaaatccaacaggttgtagatgcagatagtaaaattgttcaacttagtgaaattagtatggacaattcacctaatttagcatggcctcttattgtaacagctttaagggccaattctgctgtcaaattacagaataatgagcttagtcctgttgcactacgacagatgtcttgtgctgccggtactacacaaactgcttgcactgatgacaatgcgttagcttactacaacacaacaaagggaggtaggtttgtacttgcactgttatccgatttacaggatttgaaatgggctagattccctaagagtgatggaactggtactatctatacagaactggaaccaccttgtaggtttgttacagacacacctaaaggtcctaaagtgaagtatttatactttattaaaggattaaacaacctaaatagaggtatggtacttggtagtttagctgccacagtacgtctacaagctggtaatgcaacagaagtgcctgccaattcaactgtattatctttctgtgcttttgctgtagatgctgctaaagcttacaaagattatctagctagtgggggacaaccaatcactaattgtgttaagatgttgtgtacacacactggtactggtcaggcaataacagttacaccggaagccaatatggatcaagaatcctttggtggtgcatcgtgttgtctgtactgccgttgccacatagatcatccaaatcctaaaggattttgtgacttaaaaggtaagtatgtacaaatacctacaacttgtgctaatgaccctgtgggttttacacttaaaaacacagtctgtaccgtctgcggtatgtggaaaggttatggctgtagttgtgatcaactccgcgaacccatgcttcagtcagctgatgcacaatcgtttttaaacgggtttgcggtgtaagtgcagcccgtcttacaccgtgcggcacaggcactagtactgatgtcgtatacagggcttttgacatctacaatgataaagtagctggttttgctaaattcctaaaaactaattgttgtcgcttccaagaaaaggacgaagatgacaatttaattgattcttactttgtagttaagagacacactttctctaactaccaacatgaagaaacaatttataatttacttaaggattgtccagctgttgctaaacatgacttctttaagtttagaatagacggtgacatggtaccacatatatcacgtcaacgtcttactaaatacacaatggcagacctcgtctatgctttaaggcattttgatgaaggtaattgtgacacattaaaagaaatacttgtcacatacaattgttgtgatgatgattatttcaataaaaaggactggtatgattttgtagaaaacccagatatattacgcgtatacgccaacttaggtgaacgtgtacgccaagctttgttaaaaacagtacaattctgtgatgccatgcgaaatgctggtattgttggtgtactgacattagataatcaagatctcaatggtaactggtatgatttcggtgatttcatacaaaccacgccaggtagtggagttcctgttgtagattcttattattcattgttaatgcctatattaaccttgaccagggctttaactgcagagtcacatgttgacactgacttaacaaagccttacattaagtgggatttgttaaaatatgacttcacggaagagaggttaaaactctttgaccgttattttaaatattgggatcagacataccacccaaattgtgttaactgtttggatgacagatgcattctgcattgtgcaaactttaatgttttattctctacagtgttcccacctacaagttttggaccactagtgagaaaaatatttgttgatggtgttccatttgtagtttcaactggataccacttcagagagctaggtgttgtacataatcaggatgtaaacttacatagctctagacttagttttaaggaattacttgtgtatgctgctgaccctgctatgcacgctgcttctggtaatctattactagataaacgcactacgtgcttttcagtagctgcacttactaacaatgttgcttttcaaactgtcaaacccggtaattttaacaaagacttctatgactttgctgtgtctaagggtttctttaaggaaggaagttctgttgaattaaaacacttcttctttgctcaggatggtaatgctgctatcagcgattatgactactatcgttataatctaccaacaatgtgtgatatcagacaactactatttgtagttgaagttgttgataagtactttgattgttacgatggtggctgtattaatgctaaccaagtcatcgtcaacaacctagacaaatcagctggttttccatttaataaatggggtaaggctagactttattatgattcaatgagttatgaggatcaagatgcacttttcgcatatacaaaacgtaatgtcatccctactataactcaaatgaatcttaagtatgccattagtgcaaagaatagagctcgcaccgtagctggtgtctctatctgtagtactatgaccaatagacagtttcatcaaaaattattgaaatcaatagccgccactagaggagctactgtagtaattggaacaagcaaattctatggtggttggcacaacatgttaaaaactgtttatagtgatgtagaaaaccctcaccttatgggttgggattatcctaaatgtgatagagccatgcctaacatgcttagaattatggcctcacttgttcttgctcgcaaacatacaacgtgttgtagcttgtcacaccgtttctatagattagctaatgagtgtgctcaagtattgagtgaaatggtcatgtgtggcggttcactatatgttaaaccaggtggaacctcatcaggagatgccacaactgcttatgctaatagtgtttttaacatttgtcaagctgtcacggccaatgttaatgcacttttatctactgatggtaacaaaattgccgataagtatgtccgcaatttacaacacagactttatgagtgtctctatagaaatagagatgttgacacagactttgtgaatgagttttacgcatatttgcgtaaacatttctcaatgatgatactctctgacgatgctgttgtgtgtttcaatagcacttatgcatctcaaggtctagtggctagcataaagaactttaagtcagttctttattatcaaaacaatgtttttatgtctgaagcaaaatgttggactgagactgaccttactaaaggacctcatgaattttgctctcaacatacaatgctagttaaacagggtgatgattatgtgtaccttccttacccagatccatcaagaatcctaggggccggctgttttgtagatgatatcgtaaaaacagatggtacacttatgattgaacggttcgtgtctttagctatagatgcttacccacttactaaacatcctaatcaggagtatgctgatgtctttcatttgtacttacaatacataagaaagctacatgatgagttaacaggacacatgttagacatgtattctgttatgcttactaatgataacacttcaaggtattgggaacctgagttttatgaggctatgtacacaccgcatacagtcttacaggctgttggggcttgtgttctttgcaattcacagacttcattaagatgtggtgcttgcatacgtagaccattcttatgttgtaaatgctgttacgaccatgtcatatcaacatcacataaattagtcttgtctgttaatccgtatgtttgcaatgctccaggttgtgatgtcacagatgtgactcaactttacttaggaggtatgagctattattgtaaatcacataaaccacccattagttttccattgtgtgctaatggacaagtttttggtttatataaaaatacatgtgttggtagcgataatgttactgactttaatgcaattgcaacatgtgactggacaaatgctggtgattacattttagctaacacctgtactgaaagactcaagctttttgcagcagaaacgctcaaagctactgaggagacatttaaactgtcttatggtattgctactgtacgtgaagtgctgtctgacagagaattacatctttcatgggaagttggtaaacctagaccaccacttaaccgaaattatgtctttactggttatcgtgtaactaaaaacagtaaagtacaaataggagagtacacctttgaaaaaggtgactatggtgatgctgttgtttaccgaggtacaacaacttacaaattaaatgttggtgattattttgtgctgacatcacatacagtaatgccattaagtgcacctacactagtgccacaagagcactatgttagaattactggcttatacccaacactcaatatctcagatgagttttctagcaatgttgcaaattatcaaaaggttggtatgcaaaagtattctacactccagggaccacctggtactggtaagagtcattttgctattggcctagctctctactacccttctgctcgcatagtgtatacagcttgctctcatgccgctgttgatgcactatgtgagaaggcattaaaatatttgcctatagataaatgtagtagaattatacctgcacgtgctcgtgtagagtgttttgataaattcaaagtgaattcaacattagaacagtatgtcttttgtactgtaaatgcattgcctgagacgacagcagatatagttgtctttgatgaaatttcaatggccacaaattatgatttgagtgttgtcaatgccagattacgtgctaagcactatgtgtacattggcgaccctgctcaattacctgcaccacgcacattgctaactaagggcacactagaaccagaatatttcaattcagtgtgtagacttatgaaaactataggtccagacatgttcctcggaacttgtcggcgttgtcctgctgaaattgttgacactgtgagtgctttggtttatgataataagcttaaagcacataaagacaaatcagctcaatgctttaaaatgttttataagggtgttatcacgcatgatgtttcatctgcaattaacaggccacaaataggcgtggtaagagaattccttacacgtaaccctgcttggagaaaagctgtctttatttcaccttataattcacagaatgctgtagcctcaaagattttgggactaccaactcaaactgttgattcatcacagggctcagaatatgactatgtcatattcactcaaaccactgaaacagctcactcttgtaatgtaaacagatttaatgttgctattaccagagcaaaagtaggcatactttgcataatgtctgatagagacctttatgacaagttgcaatttacaagtcttgaaattccacgtaggaatgtggcaactttacaagctgaaaatgtaacaggactctttaaagattgtagtaaggtaatcactgggttacatcctacacaggcacctacacacctcagtgttgacactaaattcaaaactgaaggtttatgtgttgacatacctggcatacctaaggacatgacctatagaagactcatctctatgatgggttttaaaatgaattatcaagttaatggttaccctaacatgtttatcacccgcgaagaagctataagacatgtacgtgcatggattggcttcgatgtcgaggggtgtcatgctactagagaagctgttggtaccaatttacctttacagctaggtttttctacaggtgttaacctagttgctgtacctacaggttatgttgatacacctaataatacagatttttccagagttagtgctaaaccaccgcctggagatcaatttaaacacctcataccacttatgtacaaaggacttccttggaatgtagtgcgtataaagattgtacaaatgttaagtgacacacttaaaaatctctctgacagagtcgtatttgtcttatgggcacatggctttgagttgacatctatgaagtattttgtgaaaataggacctgagcgcacctgttgtctatgtgatagacgtgccacatgcttttccactgcttcagacacttatgcctgttggcatcattctattggatttgattacgtctataatccgtttatgattgatgttcaacaatggggttttacaggtaacctacaaagcaaccatgatctgtattgtcaagtccatggtaatgcacatgtagctagttgtgatgcaatcatgactaggtgtctagctgtccacgagtgctttgttaagcgtgttgactggactattgaatatcctataattggtgatgaactgaagattaatgcggcttgtagaaaggttcaacacatggttgttaaagctgcattattagcagacaaattcccagttcttcacgacattggtaaccctaaagctattaagtgtgtacctcaagctgatgtagaatggaagttctatgatgcacagccttgtagtgacaaagcttataaaatagaagaattattctattcttatgccacacattctgacaaattcacagatggtgtatgcctattttggaattgcaatgtcgatagatatcctgctaattccattgtttgtagatttgacactagagtgctatctaaccttaacttgcctggttgtgatggtggcagtttgtatgtaaataaacatgcattccacacaccagcttttgataaaagtgcttttgttaatttaaaacaattaccatttttctattactctgacagtccatgtgagtctcatggaaaacaagtagtgtcagatatagattatgtaccactaaagtctgctacgtgtataacacgttgcaatttaggtggtgctgtctgtagacatcatgctaatgagtacagattgtatctcgatgcttataacatgatgatctcagctggctttagcttgtgggtttacaaacaatttgatacttataacctctggaacacttttacaagacttcagagtttagaaaatgtggcttttaatgttgtaaataagggacactttgatggacaacagggtgaagtaccagtttctatcattaataacactgtttacacaaaagttgatggtgttgatgtagaattgtttgaaaataaaacaacattacctgttaatgtagcatttgagctttgggctaagcgcaacattaaaccagtaccagaggtgaaaatactcaataatttgggtgtggacattgctgctaatactgtgatctgggactacaaaagagatgctccagcacatatatctactattggtgtttgttctatgactgacatagccaagaaaccaactgaaacgatttgtgcaccactcactgtcttttttgatggtagagttgatggtcaagtagacttatttagaaatgcccgtaatggtgttcttattacagaaggtagtgttaaaggtttacaaccatctgtgggtcccaaacaagctagtcttaatggagtcacattaattggagaagccgtaaaaacacagttcaattattataagaaagttgatggtgttgtccaacaattacctgaaacttactttactcagagtagaaatttacaagaatttaaacccaggagtcaaatggaaattgatttcttagaattagctatggatgaattcattgaacggtataaattagaaggctatgccttcgaacatatcgtttatggagattttagtcatagtcagttaggtggtttacatctactgattggactagctaaacgttttaaggaatcaccttttgaattagaagattttattcctatggacagtacagttaaaaactatttcataacagatgcgcaaacaggttcatctaagtgtgtgtgttctgttattgatttattacttgatgattttgttgaaataataaaatcccaagatttatctgtagtttctaaggttgtcaaagtgactattgactatacagaaatttcatttatgctttggtgtaaagatggccatgtagaaacattttacccaaaattacaatctagtcaagcgtggcaaccgggtgttgctatgcctaatctttacaaaatgcaaagaatgctattagaaaagtgtgaccttcaaaattatggtgatagtgcaacattacctaaaggcataatgatgaatgtcgcaaaatatactcaactgtgtcaatatttaaacacattaacattagctgtaccctataatatgagagttatacattttggtgctggttctgataaaggagttgcaccaggtacagctgttttaagacagtggttgcctacgggtacgctgcttgtcgattcagatcttaatgactttgtctctgatgcagattcaactttgattggtgattgtgcaactgtacatacagctaataaatgggatctcattattagtgatatgtacgaccctaagactaaaaatgttacaaaagaaaatgactctaaagagggttttttcacttacatttgtgggtttatacaacaaaagctagctcttggaggttccgtggctataaagataacagaacattcttggaatgctgatctttataagctcatgggacacttcgcatggtggacagcctttgttactaatgtgaatgcgtcatcatctgaagcatttttaattggatgtaattatcttggcaaaccacgcgaacaaatagatggttatgtcatgcatgcaaattacatattttggaggaatacaaatccaattcagttgtcttcctattctttatttgacatgagtaaatttccccttaaattaaggggtactgctgttatgtctttaaaagaaggtcaaatcaatgatatgattttatctcttcttagtaaaggtagacttataattagagaaaacaacagagttgttatttctagtgatgttcttgttaacaactaaacgaacaatgtttgtttttcttgttttattgccactagtctctagtcagtgtgttaatcttacaaccagaactcaattaccccctgcatacactaattctttcacacgtggtgtttattaccctgacaaagttttcagatcctcagttttacattcaactcaggacttgttcttacctttcttttccaatgttacttggttccatgctatacatgtctctgggaccaatggtactaagaggtttgataaccctgtcctaccatttaatgatggtgtttattttgcttccactgagaagtctaacataataagaggctggatttttggtactactttagattcgaagacccagtccctacttattgttaataacgctactaatgttgttattaaagtctgtgaatttcaattttgtaatgatccatttttgggtgtttattaccacaaaaacaacaaaagttggatggaaagtgagttcagagtttattctagtgcgaataattgcacttttgaatatgtctctcagccttttcttatggaccttgaaggaaaacagggtaatttcaaaaatcttagggaatttgtgtttaagaatattgatggttattttaaaatatattctaagcacacgcctattaatttagtgcgtgatctccctcagggtttttcggctttagaaccattggtagatttgccaataggtattaacatcactaggtttcaaactttacttgctttacatagaagttatttgactcctggtgattcttcttcaggttggacagctggtgctgcagcttattatgtgggttatcttcaacctaggacttttctattaaaatataatgaaaatggaaccattacagatgctgtagactgtgcacttgaccctctctcagaaacaaagtgtacgttgaaatccttcactgtagaaaaaggaatctatcaaacttctaactttagagtccaaccaacagaatctattgttagatttcctaatattacaaacttgtgcccttttggtgaagtttttaacgccaccagatttgcatctgtttatgcttggaacaggaagagaatcagcaactgtgttgctgattattctgtcctatataattccgcatcattttccacttttaagtgttatggagtgtctcctactaaattaaatgatctctgctttactaatgtctatgcagattcatttgtaattagaggtgatgaagtcagacaaatcgctccagggcaaactggaaagattgctgattataattataaattaccagatgattttacaggctgcgttatagcttggaattctaacaatcttgattctaaggttggtggtaattataattacctgtatagattgtttaggaagtctaatctcaaaccttttgagagagatatttcaactgaaatctatcaggccggtagcacaccttgtaatggtgttgaaggttttaattgttactttcctttacaatcatatggtttccaacccactaatggtgttggttaccaaccatacagagtagtagtactttcttttgaacttctacatgcaccagcaactgtttgtggacctaaaaagtctactaatttggttaaaaacaaatgtgtcaatttcaacttcaatggtttaacaggcacaggtgttcttactgagtctaacaaaaagtttctgcctttccaacaatttggcagagacattgctgacactactgatgctgtccgtgatccacagacacttgagattcttgacattacaccatgttcttttggtggtgtcagtgttataacaccaggaacaaatacttctaaccaggttgctgttctttatcaggatgttaactgcacagaagtccctgttgctattcatgcagatcaacttactcctacttggcgtgtttattctacaggttctaatgtttttcaaacacgtgcaggctgtttaataggggctgaacatgtcaacaactcatatgagtgtgacatacccattggtgcaggtatatgcgctagttatcagactcagactaattctcctcggcgggcacgtagtgtagctagtcaatccatcattgcctacactatgtcacttggtgcagaaaattcagttgcttactctaataactctattgccatacccacaaattttactattagtgttaccacagaaattctaccagtgtctatgaccaagacatcagtagattgtacaatgtacatttgtggtgattcaactgaatgcagcaatcttttgttgcaatatggcagtttttgtacacaattaaaccgtgctttaactggaatagctgttgaacaagacaaaaacacccaagaagtttttgcacaagtcaaacaaatttacaaaacaccaccaattaaagattttggtggttttaatttttcacaaatattaccagatccatcaaaaccaagcaagaggtcatttattgaagatctacttttcaacaaagtgacacttgcagatgctggcttcatcaaacaatatggtgattgccttggtgatattgctgctagagacctcatttgtgcacaaaagtttaacggccttactgttttgccacctttgctcacagatgaaatgattgctcaatacacttctgcactgttagcgggtacaatcacttctggttggacctttggtgcaggtgctgcattacaaataccatttgctatgcaaatggcttataggtttaatggtattggagttacacagaatgttctctatgagaaccaaaaattgattgccaaccaatttaatagtgctattggcaaaattcaagactcactttcttccacagcaagtgcacttggaaaacttcaagatgtggtcaaccaaaatgcacaagctttaaacacgcttgttaaacaacttagctccaattttggtgcaatttcaagtgttttaaatgatatcctttcacgtcttgacaaagttgaggctgaagtgcaaattgataggttgatcacaggcagacttcaaagtttgcagacatatgtgactcaacaattaattagagctgcagaaatcagagcttctgctaatcttgctgctactaaaatgtcagagtgtgtacttggacaatcaaaaagagttgatttttgtggaaagggctatcatcttatgtccttccctcagtcagcacctcatggtgtagtcttcttgcatgtgacttatgtccctgcacaagaaaagaacttcacaactgctcctgccatttgtcatgatggaaaagcacactttcctcgtgaaggtgtctttgtttcaaatggcacacactggtttgtaacacaaaggaatttttatgaaccacaaatcattactacagacaacacatttgtgtctggtaactgtgatgttgtaataggaattgtcaacaacacagtttatgatcctttgcaacctgaattagactcattcaaggaggagttagataaatattttaagaatcatacatcaccagatgttgatttaggtgacatctctggcattaatgcttcagttgtaaacattcaaaaagaaattgaccgcctcaatgaggttgccaagaatttaaatgaatctctcatcgatctccaagaacttggaaagtatgagcagtatataaaatggccatggtacatttggctaggttttatagctggcttgattgccatagtaatggtgacaattatgctttgctgtatgaccagttgctgtagttgtctcaagggctgttgttcttgtggatcctgctgcaaatttgatgaagacgactctgagccagtgctcaaaggagtcaaattacattacacataaacgaacttatggatttgtttatgagaatcttcacaattggaactgtaactttgaagcaaggtgaaatcaaggatgctactccttcagattttgttcgcgctactgcaacgataccgatacaagcctcactccctttcggatggcttattgttggcgttgcacttcttgctgtttttcagagcgcttccaaaatcataaccctcaaaaagagatggcaactagcactctccaagggtgttcactttgtttgcaacttgctgttgttgtttgtaacagtttactcacaccttttgctcgttgctgctggccttgaagccccttttctctatctttatgctttagtctacttcttgcagagtataaactttgtaagaataataatgaggctttggctttgctggaaatgccgttccaaaaacccattactttatgatgccaactattttctttgctggcatactaattgttacgactattgtataccttacaatagtgtaacttcttcaattgtcattacttcaggtgatggcacaacaagtcctatttctgaacatgactaccagattggtggttatactgaaaaatgggaatctggagtaaaagactgtgttgtattacacagttacttcacttcagactattaccagctgtactcaactcaattgagtacagacactggtgttgaacatgttaccttcttcatctacaataaaattgttgatgagcctgaagaacatgtccaaattcacacaatcgacggttcatccggagttgttaatccagtaatggaaccaatttatgatgaaccgacgacgactactagcgtgcctttgtaagcacaagctgatgagtacgaacttatgtactcattcgtttcggaagagacaggtacgttaatagttaatagcgtacttctttttcttgctttcgtggtattcttgctagttacactagccatccttactgcgcttcgattgtgtgcgtactgctgcaatattgttaacgtgagtcttgtaaaaccttctttttacgtttactctcgtgttaaaaatctgaattcttctagagttcctgatcttctggtctaaacgaactaaatattatattagtttttctgtttggaactttaattttagccatggcagattccaacggtactattaccgttgaagagcttaaaaagctccttgaacaatggaacctagtaataggtttcctattccttacatggatttgtcttctacaatttgcctatgccaacaggaataggtttttgtatataattaagttaattttcctctggctgttatggccagtaactttagcttgttttgtgcttgctgctgtttacagaataaattggatcaccggtggaattgctatcgcaatggcttgtcttgtaggcttgatgtggctcagctacttcattgcttctttcagactgtttgcgcgtacccgttccatgtggtcattcaatccagaaactaacattcttctcaacgtgccactccatggcactattctgaccagaccgcttctagaaagtgaactcgtaatcggagctgtgatccttcgtggacatcttcgtattgctggacaccatctaggacgctgtgacatcaaggacctgcctaaagaaatcactgttgctacatcacgaacgctttcttattacaaattgggagcttcgcagcgtgtagcaggtgactcaggttttgctgcatacagtcgctacaggattggcaactataaattaaacacagaccattccagtagcagtgacaatattgctttgcttgtacagtaagtgacaacagatgtttcatctcgttgactttcaggttactatagcagagatattactaattattatgaggacttttaaagtttccatttggaatcttgattacatcataaacctcataattaaaaatttatctaagtcactaactgagaataaatattctcaattagatgaagagcaaccaatggagattgattaattgaactttcattaattgacttctatttgtgctttttagcctttctgctattccttgttttaattatgcttattatcttttggttctcacttgaactgcaagatcataatgaaacttgtcacgcctaaacgaacatgaaatttcttgttttcttaggaatcatcacaactgtagctgcatttcaccaagaatgtagtttacagtcatgtactcaacatcaaccatatgtagttgatgacccgtgtcctattcacttctattctaaatggtatattagagtaggagctagaaaatcagcacctttaattgaattgtgcgtggatgaggctggttctaaatcacccattcagtacatcgatatcggtaattatacagtttcctgtttaccttttacaattaattgccaggaacctaaattgggtagtcttgtagtgcgttgttcgttctatgaagactttttagagtatcatgacgttcgtgttgttttagatttcatctaaacgaacaaactaaaatgtctgataatggaccccaaaatcagcgaaatgcaccccgcattacgtttggtggaccctcagattcaactggcagtaaccagaatggagaacgcagtggggcgcgatcaaaacaacgtcggccccaaggtttacccaataatactgcgtcttggttcaccgctctcactcaacatggcaaggaagaccttaaattccctcgaggacaaggcgttccaattaacaccaatagcagtccagatgaccaaattggctactaccgaagagctaccagacgaattcgtggtggtgacggtaaaatgaaagatctcagtccaagatggtatttctactacctaggaactgggccagaagctggacttccctatggtgctaacaaagacggcatcatatgggttgcaactgagggagccttgaatacaccaaaagatcacattggcacccgcaatcctgctaacaatgctgcaatcgtgctacaacttcctcaaggaacaacattgccaaaaggcttctacgcagaagggagcagaggcggcagtcaagcctcttctcgttcctcatcacgtagtcgcaacagttcaagaaattcaactccaggcagcagtaggggaacttctcctgctagaatggctggcaatggcggtgatgctgctcttgctttgctgctgcttgacagattgaaccagcttgagagcaaaatgtctggtaaaggccaacaacaacaaggccaaactgtcactaagaaatctgctgctgaggcttctaagaagcctcggcaaaaacgtactgccactaaagcatacaatgtaacacaagctttcggcagacgtggtccagaacaaacccaaggaaattttggggaccaggaactaatcagacaaggaactgattacaaacattggccgcaaattgcacaatttgcccccagcgcttcagcgttcttcggaatgtcgcgcattggcatggaagtcacaccttcgggaacgtggttgacctacacaggtgccatcaaattggatgacaaagatccaaatttcaaagatcaagtcattttgctgaataagcatattgacgcatacaaaacattcccaccaacagagcctaaaaaggacaaaaagaagaaggctgatgaaactcaagccttaccgcagagacagaagaaacagcaaactgtgactcttcttcctgctgcagatttggatgatttctccaaacaattgcaacaatccatgagcagtgctgactcaactcaggcctaaactcatgcagaccacacaaggcagatgggctatataaacgttttcgcttttccgtttacgatatatagtctactcttgtgcagaatgaattctcgtaactacatagcacaagtagatgtagttaactttaatctcacatagcaatctttaatcagtgtgtaacattagggaggacttgaaagagccaccacattttcaccgaggccacgcggagtacgatcgagtgtacagtgaacaatgctagggagagctgcctatatggaagagccctaatgtgtaaaattaattttagtagtgctatccccatgtgattttaatagcttcttaggagaatgacaaaaaaaaaaaaaaaaaaaaaaaaa

SEQ ID NO: 20 - DNA, 29604 bp, Coronaviridae
  misc_feature 1..29604: note = SARS-CoV-2-7a
  source 1..29604: mol_type = other DNA
attaaaggtttataccttcccaggtaacaaaccaaccaactttcgatctcttgtagatctgttctctaaacgaactttaaaatctgtgtggctgtcactcggctgcatgcttagtgcactcacgcagtataattaataactaattactgtcgttgacaggacacgagtaactcgtctatcttctgcaggctgcttacggtttcgtccgtgttgcagccgatcatcagcacatctaggtttcgtccgggtgtgaccgaaaggtaagatggagagccttgtccctggtttcaacgagaaaacacacgtccaactcagtttgcctgttttacaggttcgcgacgtgctcgtacgtggctttggagactccgtggaggaggtcttatcagaggcacgtcaacatcttaaagatggcacttgtggcttagtagaagttgaaaaaggcgttttgcctcaacttgaacagccctatgtgttcatcaaacgttcggatgctcgaactgcacctcatggtcatgttatggttgagctggtagcagaactcgaaggcattcagtacggtcgtagtggtgagacacttggtgtccttgtccctcatgtgggcgaaataccagtggcttaccgcaaggttcttcttcgtaagaacggtaataaaggagctggtggccatagttacggcgccgatctaaagtcatttgacttaggcgacgagcttggcactgatccttatgaagattttcaagaaaactggaacactaaacatagcagtggtgttacccgtgaactcatgcgtgagcttaacggaggggcatacactcgctatgtcgataacaacttctgtggccctgatggctaccctcttgagtgcattaaagaccttctagcacgtgctggtaaagcttcatgcactttgtccgaacaactggactttattgacactaagaggggtgtatactgctgccgtgaacatgagcatgaaattgcttggtacacggaacgttctgaaaagagctatgaattgcagacaccttttgaaattaaattggcaaagaaatttgacaccttcaatggggaatgtccaaattttgtatttcccttaaattccataatcaagactattcaaccaagggttgaaaagaaaaagcttgatggctttatgggtagaattcgatctgtctatccagttgcgtcaccaaatgaatgcaaccaaatgtgcctttcaactctcatgaagtgtgatcattgtggtgaaacttcatggcagacgggcgattttgttaaagccacttgcgaattttgtggcactgagaatttgactaaagaaggtgccactacttgtggttacttaccccaaaatgctgttgttaaaatttattgtccagcatgtcacaattcagaagtaggacctgagcatagtcttgccgaataccataatgaatctggcttgaaaaccattcttcgtaagggtggtcgcactattgcctttggaggctgtgtgttctcttatgttggttgccataacaagtgtgcctattgggttccacgtgctagcgctaacataggttgtaaccatacaggtgttgttggagaaggttccgaaggtcttaatgacaaccttcttgaaatactccaaaaagagaaagtcaacatcaatattgttggtgactttaaacttaatgaagagatcgccattattttggcatctttttctgcttccacaagtgcttttgtggaaactgtgaaaggtttggattataaagcattcaaacaaattgttgaatcctgtggtaattttaaagttacaaaaggaaaagctaaaaaaggtgcctggaatattggtgaacagaaatcaatactgagtcctctttatgcatttgcatcagaggctgctcgtgttgtacgatcaattttctcccgcactcttgaaactgctcaaaattctgtgcgtgttttacagaaggccgctataacaatactagatggaatttcacagtattcactgagactcattgatgctatgatgttcacatctgatttggctactaacaatctagttgtaatggcctacattacaggtggtgttgttcagttgacttcgcagtggctaactaacatctttggcactgtttatgaaaaactcaaacccgtccttgattggcttgaagagaagtttaaggaaggtgtagagtttcttagagacggttgggaaattgttaaatttatctcaacctgtgcttgtgaaattgtcggtggacaaattgtcacctgtgcaaaggaaattaaggagagtgttcagacattctttaagcttgtaaataaatttttggctttgtgtgctgactctatcattattggtggagctaaacttaaagccttgaatttaggtgaaacatttgtcacgcactcaaagggattgtacagaaagtgtgttaaatccagagaagaaactggcctactcatgcctctaaaagccccaaaagaaattatcttcttagagggagaaacacttcccacagaagtgttaacagaggaagttgtcttgaaaactggtgatttacaaccattagaacaacctactagtgaagctgttgaagctccattggttggtacaccagtttgtattaacgggcttatgttgctcgaaatcaaagacacagaaaagtactgtgcccttgcacctaatatgatggtaacaaacaataccttcacactcaaaggcggtgcaccaacaaaggttacttttggtgatgacactgtgatagaagtgcaaggttacaagagtgtgaatatcacttttgaacttgatgaaaggattgataaagtacttaatgagaagtgctctgcctatacagttgaactcggtacagaagtaaatgagttcgcctgtgttgtggcagatgctgtcataaaaactttgcaaccagtatctgaattacttacaccactgggcattgatttagatgagtggagtatggctacatactacttatttgatgagtctggtgagtttaaattggcttcacatatgtattgttctttctaccctccagatgaggatgaagaagaaggtgattgtgaagaagaagagtttgagccatcaactcaatatgagtatggtactgaagatgattaccaaggtaaacctttggaatttggtgccacttctgctgctcttcaacctgaagaagagcaagaagaagattggttagatgatgatagtcaacaaactgttggtcaacaagacggcagtgaggacaatcagacaactactattcaaacaattgttgaggttcaacctcaattagagatggaacttacaccagttgttcagactattgaagtgaatagttttagtggttatttaaaacttactgacaatgtatacattaaaaatgcagacattgtggaagaagctaaaaaggtaaaaccaacagtggttgttaatgcagccaatgtttaccttaaacatggaggaggtgttgcaggagccttaaataaggctactaacaatgccatgcaagttgaatctgatgattacatagctactaatggaccacttaaagtgggtggtagttgtgttttaagcggacacaatcttgctaaacactgtcttcatgttgtcggcccaaatgttaacaaaggtgaagacattcaacttcttaagagtgcttatgaaaattttaatcagcacgaagttctacttgcaccattattatcagctggtatttttggtgctgaccctatacattctttaagagtttgtgtagatactgttcgcacaaatgtctacttagctgtctttgataaaaatctctatgacaaacttgtttcaagctttttggaaatgaagagtgaaaagcaagttgaacaaaagatcgctgagattcctaaagaggaagttaagccatttataactgaaagtaaaccttcagttgaacagagaaaacaagatgataagaaaatcaaagcttgtgttgaagaagttacaacaactctggaagaaactaagttcctcacagaaaacttgttactttatattgacattaatggcaatcttcatccagattctgccactcttgttagtgacattgacatcactttcttaaagaaagatgctccatatatagtgggtgatgttgttcaagagggtgttttaactgctgtggttatacctactaaaaaggctggtggcactactgaaatgctagcgaaagctttgagaaaagtgccaacagacaattatataaccacttacccgggtcagggtttaaatggttacactgtagaggaggcaaagacagtgcttaaaaagtgtaaaagtgccttttacattctaccatctattatctctaatgagaagcaagaaattcttggaactgtttcttggaatttgcgagaaatgcttgcacatgcagaagaaacacgcaaattaatgcctgtctgtgtggaaactaaagccatagtttcaactatacagcgtaaatataagggtattaaaatacaagagggtgtggttgattatggtgctagattttacttttacaccagtaaaacaactgtagcgtcacttatcaacacacttaacgatctaaatgaaactcttgttacaatgccacttggctatgtaacacatggcttaaatttggaagaagctgctcggtatatgagatctctcaaagtgccagctacagtttctgtttcttcacctgatgctgttacagcgtataatggttatcttacttcttcttctaaaacacctgaagaacattttattgaaaccatctcacttgctggttcctataaagattggtcctattctggacaatctacacaactaggtatagaatttcttaagagaggtgataaaagtgtatattacactagtaatcctaccacattccacctagatggtgaagttatcacctttgacaatcttaagacacttctttctttgagagaagtgaggactattaaggtgtttacaacagtagacaacattaacctccacacgcaagttgtggacatgtcaatgacatatggacaacagtttggtccaacttatttggatggagctgatgttactaaaataaaacctcataattcacatgaaggtaaaacattttatgttttacctaatgatgacactctacgtgttgaggcttttgagtactaccacacaactgatcctagttttctgggtaggtacatgtcagcattaaatcacactaaaaagtggaaatacccacaagttaatggtttaacttctattaaatgggcagataacaactgttatcttgccactgcattgttaacactccaacaaatagagttgaagtttaatccacctgctctacaagatgcttattacagagcaagggctggtgaagctgctaacttttgtgcacttatcttagcctactgtaataagacagtaggtgagttaggtgatgttagagaaacaatgagttacttgtttcaacatgccaatttagattcttgcaaaagagtcttgaacgtggtgtgtaaaacttgtggacaacagcagacaacccttaagggtgtagaagctgttatgtacatgggcacactttcttatgaacaatttaagaaaggtgttcagataccttgtacgtgtggtaaacaagctacaaaatatctagtacaacaggagtcaccttttgttatgatgtcagcaccacctgctcagtatgaacttaagcatggtacatttacttgtgctagtgagtacactggtaattaccagtgtggtcactataaacatataacttctaaagaaactttgtattgcatagacggtgctttacttacaaagtcctcagaatacaaaggtcctattacggatgttttctacaaagaaaacagttacacaacaaccataaaaccagttacttataaattggatggtgttgtttgtacagaaattgaccctaagttggacaattattataagaaagacaattcttatttcacagagcaaccaattgatcttgtaccaaaccaaccatatccaaacgcaagcttcgataattttaagtttgtatgtgataatatcaaatttgctgatgatttaaaccagttaactggttataagaaacctgcttcaagagagcttaaagttacatttttccctgacttaaatggtgatgtggtggctattgattataaacactacacaccctcttttaagaaaggagctaaattgttacataaacctattgtttggcatgttaacaatgcaactaataaagccacgtataaaccaaatacctggtgtatacgttgtctttggagcacaaaaccagttgaaacatcaaattcgtttgatgtactgaagtcagaggacgcgcagggaatggataatcttgcctgcgaagatctaaaaccagtctctgaagaagtagtggaaaatcctaccatacagaaagacgttcttgagtgtaatgtgaaaactaccgaagttgtaggagacattatacttaaaccagcaaataatagtttaaaaattacagaagaggttggccacacagatctaatggctgcttatgtagacaattctagtcttactattaagaaacctaatgaattatctagagtattaggtttgaaaacccttgctactcatggtttagctgctgttaatagtgtcccttgggatactatagctaattatgctaagccttttcttaacaaagttgttagtacaactactaacatagttacacggtgtttaaaccgtgtttgtactaattatatgccttatttctttactttattgctacaattgtgtacttttactagaagtacaaattctagaattaaagcatctatgccgactactatagcaaagaatactgttaagagtgtcggtaaattttgtctagaggcttcatttaattatttgaagtcacctaatttttctaaactgataaatattataatttggtttttactattaagtgtttgcctaggttctttaatctactcaaccgctgctttaggtgttttaatgtctaatttaggcatgccttcttactgtactggttacagagaaggctatttgaactctactaatgtcactattgcaacctactgtactggttctataccttgtagtgtttgtcttagtggtttagattctttagacacctatccttctttagaaactatacaaattaccatttcatcttttaaatgggatttaactgcttttggcttagttgcagagtggtttttggcatatattcttttcactaggtttttctatgtacttggattggctgcaatcatgcaattgtttttcagctattttgcagtacattttattagtaattcttggcttatgtggttaataattaatcttgtacaaatggccccgatttcagctatggttagaatgtacatcttctttgcatcattttattatgtatggaaaagttatgtgcatgttgtagacggttgtaattcatcaacttgtatgatgtgttacaaacgtaatagagcaacaagagtcgaatgtacaactattgttaatggtgttagaaggtccttttatgtctatgctaatggaggtaaaggcttttgcaaactacacaattggaattgtgttaattgtgatacattctgtgctggtagtacatttattagtgatgaagttgcgagagacttgtcactacagtttaaaagaccaataaatcctactgaccagtcttcttacatcgttgatagtgttacagtgaagaatggttccatccatctttactttgataaagctggtcaaaagacttatgaaagacattctctctctcattttgttaacttagacaacctgagagctaataacactaaaggttcattgcctattaatgttatagtttttgatggtaaatcaaaatgtgaagaatcatctgcaaaatcagcgtctgtttactacagtcagcttatgtgtcaacctatactgttactagatcaggcattagtgtctgatgttggtgatagtgcggaagttgcagttaaaatgtttgatgcttacgttaatacgttttcatcaacttttaacgtaccaatggaaaaactcaaaacactagttgcaactgcagaagctgaacttgcaaagaatgtgtccttagacaatgtcttatctacttttatttcagcagctcggcaagggtttgttgattcagatgtagaaactaaagatgttgttgaatgtcttaaattgtcacatcaatctgacatagaagttactggcgatagttgtaataactatatgctcacctataacaaagttgaaaacatgacaccccgtgaccttggtgcttgtattgactgtagtgcgcgtcatattaatgcgcaggtagcaaaaagtcacaacattgctttgatatggaacgttaaagatttcatgtcattgtctgaacaactacgaaaacaaatacgtagtgctgctaaaaagaataacttaccttttaagttgacatgtgcaactactagacaagttgttaatgttgtaacaacaaagatagcacttaagggtggtaaaattgttaataattggttgaagcagttaattaaagttacacttgtgttcctttttgttgctgctattttctatttaataacacctgttcatgtcatgtctaaacatactgacttttcaagtgaaatcataggatacaaggctattgatggtggtgtcactcgtgacatagcatctacagatacttgttttgctaacaaacatgctgattttgacacatggtttagccagcgtggtggtagttatactaatgacaaagcttgcccattgattgctgcagtcataacaagagaagtgggttttgtcgtgcctggtttgcctggcacgatattacgcacaactaatggtgactttttgcatttcttacctagagtttttagtgcagttggtaacatctgttacacaccatcaaaacttatagagtacactgactttgcaacatcagcttgtgttttggctgctgaatgtacaatttttaaagatgcttctggtaagccagtaccatattgttatgataccaatgtactagaaggttctgttgcttatgaaagtttacgccctgacacacgttatgtgctcatggatggctctattattcaatttcctaacacctaccttgaaggttctgttagagtggtaacaacttttgattctgagtactgtaggcacggcacttgtgaaagatcagaagctggtgtttgtgtatctactagtggtagatgggtacttaacaatgattattacagatctttaccaggagttttctgtggtgtagatgctgtaaatttacttactaatatgtttacaccactaattcaacctattggtgctttggacatatcagcatctatagtagctggtggtattgtagctatcgtagtaacatgccttgcctactattttatgaggtttagaagagcttttggtgaatacagtcatgtagttgcctttaatactttactattccttatgtcattcactgtactctgtttaacaccagtttactcattcttacctggtgtttattctgttatttacttgtacttgacattttatcttactaatgatgtttcttttttagcacatattcagtggatggttatgttcacacctttagtacctttctggataacaattgcttatatcatttgtatttccacaaagcatttctattggttctttagtaattacctaaagagacgtgtagtctttaatggtgtttcctttagtacttttgaagaagctgcgctgtgcacctttttgttaaataaagaaatgtatctaaagttgcgtagtgatgtgctattacctcttacgcaatataatagatacttagctctttataataagtacaagtattttagtggagcaatggatacaactagctacagagaagctgcttgttgtcatctcgcaaaggctctcaatgacttcagtaactcaggttctgatgttctttaccaaccaccacaaacctctatcacctcagctgttttgcagagtggttttagaaaaatggcattcccatctggtaaagttgagggttgtatggtacaagtaacttgtggtacaactacacttaacggtctttggcttgatgacgtagtttactgtccaagacatgtgatctgcacctctgaagacatgcttaaccctaattatgaagatttactcattcgtaagtctaatcataatttcttggtacaggctggtaatgttcaactcagggttattggacattctatgcaaaattgtgtacttaagcttaaggttgatacagccaatcctaagacacctaagtataagtttgttcgcattcaaccaggacagactttttcagtgttagcttgttacaatggttcaccatctggtgtttaccaatgtgctatgaggcccaatttcactattaagggttcattccttaatggttcatgtggtagtgttggttttaacatagattatgactgtgtctctttttgttacatgcaccatatggaattaccaactggagttcatgctggcacagacttagaaggtaacttttatggaccttttgttgacaggcaaacagcacaagcagctggtacggacacaactattacagttaatgttttagcttggttgtacgctgctgttataaatggagacaggtggtttctcaatcgatttaccacaactcttaatgactttaaccttgtggctatgaagtacaattatgaacctctaacacaagaccatgttgacatactaggacctctttctgctcaaactggaattgccgttttagatatgtgtgcttcattaaaagaattactgcaaaatggtatgaatggacgtaccatattgggtagtgctttattagaagatgaatttacaccttttgatgttgttagacaatgctcaggtgttactttccaaagtgcagtgaaaagaacaatcaagggtacacaccactggttgttactcacaattttgacttcacttttagttttagtccagagtactcaatggtctttgttcttttttttgtatgaaaatgcctttttaccttttgctatgggtattattgctatgtctgcttttgcaatgatgtttgtcaaacataagcatgcatttctctgtttgtttttgttaccttctcttgccactgtagcttattttaatatggtctatatgcctgctagttgggtgatgcgtattatgacatggttggatatggttgatactagtttgtctggttttaagctaaaagactgtgttatgtatgcatcagctgtagtgttactaatccttatgacagcaagaactgtgtatgatgatggtgctaggagagtgtggacacttatgaatgtcttgacactcgtttataaagtttattatggtaatgctttagatcaagccatttccatgtgggctcttataatctctgttacttctaactactcaggtgtagttacaactgtcatgtttttggccagaggtattgtttttatgtgtgttgagtattgccctattttcttcataactggtaatacacttcagtgtataatgctagtttattgtttcttaggctatttttgtacttgttactttggcctcttttgtttactcaaccgctactttagactgactcttggtgtttatgattacttagtttctacacaggagtttagatatatgaattcacagggactactcccacccaagaatagcatagatgccttcaaactcaacattaaattgttgggtgttggtggcaaaccttgtatcaaagtagccactgtacagtctaaaatgtcagatgtaaagtgcacatcagtagtcttactctcagttttgcaacaactcagagtagaatcatcatctaaattgtgggctcaatgtgtccagttacacaatgacattctcttagctaaagatactactgaagcctttgaaaaaatggtttcactactttctgttttgctttccatgcagggtgctgtagacataaacaagctttgtgaagaaatgctggacaacagggcaaccttacaagctatagcctcagagtttagttcccttccatcatatgcagcttttgctactgctcaagaagcttatgagcaggctgttgctaatggtgattctgaagttgttcttaaaaagttgaagaagtctttgaatgtggctaaatctgaatttgaccgtgatgcagccatgcaacgtaagttggaaaagatggctgatcaagctatgacccaaatgtataaacaggctagatctgaggacaagagggcaaaagttactagtgctatgcagacaatgcttttcactatgcttagaaagttggataatgatgcactcaacaacattatcaacaatgcaagagatggttgtgttcccttgaacataatacctcttacaacagcagccaaactaatggttgtcataccagactataacacatataaaaatacgtgtgatggtacaacatttacttatgcatcagcattgtgggaaatccaacaggttgtagatgcagatagtaaaattgttcaacttagtgaaattagtatggacaattcacctaatttagcatggcctcttattgtaacagctttaagggccaattctgctgtcaaattacagaataatgagcttagtcctgttgcactacgacagatgtcttgtgctgccggtactacacaaactgcttgcactgatgacaatgcgttagcttactacaacacaacaaagggaggtaggtttgtacttgcactgttatccgatttacaggatttgaaatgggctagattccctaagagtgatggaactggtactatctatacagaactggaaccaccttgtaggtttgttacagacacacctaaaggtcctaaagtgaagtatttatactttattaaaggattaaacaacctaaatagaggtatggtacttggtagtttagctgccacagtacgtctacaagctggtaatgcaacagaagtgcctgccaattcaactgtattatctttctgtgcttttgctgtagatgctgctaaagcttacaaagattatctagctagtgggggacaaccaatcactaattgtgttaagatgttgtgtacacacactggtactggtcaggcaataacagttacaccggaagccaatatggatcaagaatcctttggtggtgcatcgtgttgtctgtactgccgttgccacatagatcatccaaatcctaaaggattttgtgacttaaaaggtaagtatgtacaaatacctacaacttgtgctaatgaccctgtgggttttacacttaaaaacacagtctgtaccgtctgcggtatgtggaaaggttatggctgtagttgtgatcaactccgcgaacccatgcttcagtcagctgatgcacaatcgtttttaaacgggtttgcggtgtaagtgcagcccgtcttacaccgtgcggcacaggcactagtactgatgtcgtatacagggcttttgacatctacaatgataaagtagctggttttgctaaattcctaaaaactaattgttgtcgcttccaagaaaaggacgaagatgacaatttaattgattcttactttgtagttaagagacacactttctctaactaccaacatgaagaaacaatttataatttacttaaggattgtccagctgttgctaaacatgacttctttaagtttagaatagacggtgacatggtaccacatatatcacgtcaacgtcttactaaatacacaatggcagacctcgtctatgctttaaggcattttgatgaaggtaattgtgacacattaaaagaaatacttgtcacatacaattgttgtgatgatgattatttcaataaaaaggactggtatgattttgtagaaaacccagatatattacgcgtatacgccaacttaggtgaacgtgtacgccaagctttgttaaaaacagtacaattctgtgatgccatgcgaaatgctggtattgttggtgtactgacattagataatcaagatctcaatggtaactggtatgatttcggtgatttcatacaaaccacgccaggtagtggagttcctgttgtagattcttattattcattgttaatgcctatattaaccttgaccagggctttaactgcagagtcacatgttgacactgacttaacaaagccttacattaagtgggatttgttaaaatatgacttcacggaagagaggttaaaactctttgaccgttattttaaatattgggatcagacataccacccaaattgtgttaactgtttggatgacagatgcattctgcattgtgcaaactttaatgttttattctctacagtgttcccacctacaagttttggaccactagtgagaaaaatatttgttgatggtgttccatttgtagtttcaactggataccacttcagagagctaggtgttgtacataatcaggatgtaaacttacatagctctagacttagttttaaggaattacttgtgtatgctgctgaccctgctatgcacgctgcttctggtaatctattactagataaacgcactacgtgcttttcagtagctgcacttactaacaatgttgcttttcaaactgtcaaacccggtaattttaacaaagacttctatgactttgctgtgtctaagggtttctttaaggaaggaagttctgttgaattaaaacacttcttctttgctcaggatggtaatgctgctatcagcgattatgactactatcgttataatctaccaacaatgtgtgatatcagacaactactatttgtagttgaagttgttgataagtactttgattgttacgatggtggctgtattaatgctaaccaagtcatcgtcaacaacctagacaaatcagctggttttccatttaataaatggggtaaggctagactttattatgattcaatgagttatgaggatcaagatgcacttttcgcatatacaaaacgtaatgtcatccctactataactcaaatgaatcttaagtatgccattagtgcaaagaatagagctcgcaccgtagctggtgtctctatctgtagtactatgaccaatagacagtttcatcaaaaattattgaaatcaatagccgccactagaggagctactgtagtaattggaacaagcaaattctatggtggttggcacaacatgttaaaaactgtttatagtgatgtagaaaaccctcaccttatgggttgggattatcctaaatgtgatagagccatgcctaacatgcttagaattatggcctcacttgttcttgctcgcaaacatacaacgtgttgtagcttgtcacaccgtttctatagattagctaatgagtgtgctcaagtattgagtgaaatggtcatgtgtggcggttcactatatgttaaaccaggtggaacctcatcaggagatgccacaactgcttatgctaatagtgtttttaacatttgtcaagctgtcacggccaatgttaatgcacttttatctactgatggtaacaaaattgccgataagtatgtccgcaatttacaacacagactttatgagtgtctctatagaaatagagatgttgacacagactttgtgaatgagttttacgcatatttgcgtaaacatttctcaatgatgatactctctgacgatgctgttgtgtgtttcaatagcacttatgcatctcaaggtctagtggctagcataaagaactttaagtcagttctttattatcaaaacaatgtttttatgtctgaagcaaaatgttggactgagactgaccttactaaaggacctcatgaattttgctctcaacatacaatgctagttaaacagggtgatgattatgtgtaccttccttacccagatccatcaagaatcctaggggccggctgttttgtagatgatatcgtaaaaacagatggtacacttatgattgaacggttcgtgtctttagctatagatgcttacccacttactaaacatcctaatcaggagtatgctgatgtctttcatttgtacttacaatacataagaaagctacatgatgagttaacaggacacatgttagacatgtattctgttatgcttactaatgataacacttcaaggtattgggaacctgagttttatgaggctatgtacacaccgcatacagtcttacaggctgttggggcttgtgttctttgcaattcacagacttcattaagatgtggtgcttgcatacgtagaccattcttatgttgtaaatgctgttacgaccatgtcatatcaacatcacataaattagtcttgtctgttaatccgtatgtttgcaatgctccaggttgtgatgtcacagatgtgactcaactttacttaggaggtatgagctattattgtaaatcacataaaccacccattagttttccattgtgtgctaatggacaagtttttggtttatataaaaatacatgtgttggtagcgataatgttactgactttaatgcaattgcaacatgtgactggacaaatgctggtgattacattttagctaacacctgtactgaaagactcaagctttttgcagcagaaacgctcaaagctactgaggagacatttaaactgtcttatggtattgctactgtacgtgaagtgctgtctgacagagaattacatctttcatgggaagttggtaaacctagaccaccacttaaccgaaattatgtctttactggttatcgtgtaactaaaaacagtaaagtacaaataggagagtacacctttgaaaaaggtgactatggtgatgctgttgtttaccgaggtacaacaacttacaaattaaatgttggtgattattttgtgctgacatcacatacagtaatgccattaagtgcacctacactagtgccacaagagcactatgttagaattactggcttatacccaacactcaatatctcagatgagttttctagcaatgttgcaaattatcaaaaggttggtatgcaaaagtattctacactccagggaccacctggtactggtaagagtcattttgctattggcctagctctctactacccttctgctcgcatagtgtatacagcttgctctcatgccgctgttgatgcactatgtgagaaggcattaaaatatttgcctatagataaatgtagtagaattatacctgcacgtgctcgtgtagagtgttttgataaattcaaagtgaattcaacattagaacagtatgtcttttgtactgtaaatgcattgcctgagacgacagcagatatagttgtctttgatgaaatttcaatggccacaaattatgatttgagtgttgtcaatgccagattacgtgctaagcactatgtgtacattggcgaccctgctcaattacctgcaccacgcacattgctaactaagggcacactagaaccagaatatttcaattcagtgtgtagacttatgaaaactataggtccagacatgttcctcggaacttgtcggcgttgtcctgctgaaattgttgacactgtgagtgctttggtttatgataataagcttaaagcacataaagacaaatcagctcaatgctttaaaatgttttataagggtgttatcacgcatgatgtttcatctgcaattaacaggccacaaataggcgtggtaagagaattccttacacgtaaccctgcttggagaaaagctgtctttatttcaccttataattcacagaatgctgtagcctcaaagattttgggactaccaactcaaactgttgattcatcacagggctcagaatatgactatgtcatattcactcaaaccactgaaacagctcactcttgtaatgtaaacagatttaatgttgctattaccagagcaaaagtaggcatactttgcataatgtctgatagagacctttatgacaagttgcaatttacaagtcttgaaattccacgtaggaatgtggcaactttacaagctgaaaatgtaacaggactctttaaagattgtagtaaggtaatcactgggttacatcctacacaggcacctacacacctcagtgttgacactaaattcaaaactgaaggtttatgtgttgacatacctggcatacctaaggacatgacctatagaagactcatctctatgatgggttttaaaatgaattatcaagttaatggttaccctaacatgtttatcacccgcgaagaagctataagacatgtacgtgcatggattggcttcgatgtcgaggggtgtcatgctactagagaagctgttggtaccaatttacctttacagctaggtttttctacaggtgttaacctagttgctgtacctacaggttatgttgatacacctaataatacagatttttccagagttagtgctaaaccaccgcctggagatcaatttaaacacctcataccacttatgtacaaaggacttccttggaatgtagtgcgtataaagattgtacaaatgttaagtgacacacttaaaaatctctctgacagagtcgtatttgtcttatgggcacatggctttgagttgacatctatgaagtattttgtgaaaataggacctgagcgcacctgttgtctatgtgatagacgtgccacatgcttttccactgcttcagacacttatgcctgttggcatcattctattggatttgattacgtctataatccgtttatgattgatgttcaacaatggggttttacaggtaacctacaaagcaaccatgatctgtattgtcaagtccatggtaatgcacatgtagctagttgtgatgcaatcatgactaggtgtctagctgtccacgagtgctttgttaagcgtgttgactggactattgaatatcctataattggtgatgaactgaagattaatgcggcttgtagaaaggttcaacacatggttgttaaagctgcattattagcagacaaattcccagttcttcacgacattggtaaccctaaagctattaagtgtgtacctcaagctgatgtagaatggaagttctatgatgcacagccttgtagtgacaaagcttataaaatagaagaattattctattcttatgccacacattctgacaaattcacagatggtgtatgcctattttggaattgcaatgtcgatagatatcctgctaattccattgtttgtagatttgacactagagtgctatctaaccttaacttgcctggttgtgatggtggcagtttgtatgtaaataaacatgcattccacacaccagcttttgataaaagtgcttttgttaatttaaaacaattaccatttttctattactctgacagtccatgtgagtctcatggaaaacaagtagtgtcagatatagattatgtaccactaaagtctgctacgtgtataacacgttgcaatttaggtggtgctgtctgtagacatcatgctaatgagtacagattgtatctcgatgcttataacatgatgatctcagctggctttagcttgtgggtttacaaacaatttgatacttataacctctggaacacttttacaagacttcagagtttagaaaatgtggcttttaatgttgtaaataagggacactttgatggacaacagggtgaagtaccagtttctatcattaataacactgtttacacaaaagttgatggtgttgatgtagaattgtttgaaaataaaacaacattacctgttaatgtagcatttgagctttgggctaagcgcaacattaaaccagtaccagaggtgaaaatactcaataatttgggtgtggacattgctgctaatactgtgatctgggactacaaaagagatgctccagcacatatatctactattggtgtttgttctatgactgacatagccaagaaaccaactgaaacgatttgtgcaccactcactgtcttttttgatggtagagttgatggtcaagtagacttatttagaaatgcccgtaatggtgttcttattacagaaggtagtgttaaaggtttacaaccatctgtgggtcccaaacaagctagtcttaatggagtcacattaattggagaagccgtaaaaacacagttcaattattataagaaagttgatggtgttgtccaacaattacctgaaacttactttactcagagtagaaatttacaagaatttaaacccaggagtcaaatggaaattgatttcttagaattagctatggatgaattcattgaacggtataaattagaaggctatgccttcgaacatatcgtttatggagattttagtcatagtcagttaggtggtttacatctactgattggactagctaaacgttttaaggaatcaccttttgaattagaagattttattcctatggacagtacagttaaaaactatttcataacagatgcgcaaacaggttcatctaagtgtgtgtgttctgttattgatttattacttgatgattttgttgaaataataaaatcccaagatttatctgtagtttctaaggttgtcaaagtgactattgactatacagaaatttcatttatgctttggtgtaaagatggccatgtagaaacattttacccaaaattacaatctagtcaagcgtggcaaccgggtgttgctatgcctaatctttacaaaatgcaaagaatgctattagaaaagtgtgaccttcaaaattatggtgatagtgcaacattacctaaaggcataatgatgaatgtcgcaaaatatactcaactgtgtcaatatttaaacacattaacattagctgtaccctataatatgagagttatacattttggtgctggttctgataaaggagttgcaccaggtacagctgttttaagacagtggttgcctacgggtacgctgcttgtcgattcagatcttaatgactttgtctctgatgcagattcaactttgattggtgattgtgcaactgtacatacagctaataaatgggatctcattattagtgatatgtacgaccctaagactaaaaatgttacaaaagaaaatgactctaaagagggttttttcacttacatttgtgggtttatacaacaaaagctagctcttggaggttccgtggctataaagataacagaacattcttggaatgctgatctttataagctcatgggacacttcgcatggtggacagcctttgttactaatgtgaatgcgtcatcatctgaagcatttttaattggatgtaattatcttggcaaaccacgcgaacaaatagatggttatgtcatgcatgcaaattacatattttggaggaatacaaatccaattcagttgtcttcctattctttatttgacatgagtaaatttccccttaaattaaggggtactgctgttatgtctttaaaagaaggtcaaatcaatgatatgattttatctcttcttagtaaaggtagacttataattagagaaaacaacagagttgttatttctagtgatgttcttgttaacaactaaacgaacaatgtttgtttttcttgttttattgccactagtctctagtcagtgtgttaatcttacaaccagaactcaattaccccctgcatacactaattctttcacacgtggtgtttattaccctgacaaagttttcagatcctcagttttacattcaactcaggacttgttcttacctttcttttccaatgttacttggttccatgctatacatgtctctgggaccaatggtactaagaggtttgataaccctgtcctaccatttaatgatggtgtttattttgcttccactgagaagtctaacataataagaggctggatttttggtactactttagattcgaagacccagtccctacttattgttaataacgctactaatgttgttattaaagtctgtgaatttcaattttgtaatgatccatttttgggtgtttattaccacaaaaacaacaaaagttggatggaaagtgagttcagagtttattctagtgcgaataattgcacttttgaatatgtctctcagccttttcttatggaccttgaaggaaaacagggtaatttcaaaaatcttagggaatttgtgtttaagaatattgatggttattttaaaatatattctaagcacacgcctattaatttagtgcgtgatctccctcagggtttttcggctttagaaccattggtagatttgccaataggtattaacatcactaggtttcaaactttacttgctttacatagaagttatttgactcctggtgattcttcttcaggttggacagctggtgctgcagcttattatgtgggttatcttcaacctaggacttttctattaaaatataatgaaaatggaaccattacagatgctgtagactgtgcacttgaccctctctcagaaacaaagtgtacgttgaaatccttcactgtagaaaaaggaatctatcaaacttctaactttagagtccaaccaacagaatctattgttagatttcctaatattacaaacttgtgcccttttggtgaagtttttaacgccaccagatttgcatctgtttatgcttggaacaggaagagaatcagcaactgtgttgctgattattctgtcctatataattccgcatcattttccacttttaagtgttatggagtgtctcctactaaattaaatgatctctgctttactaatgtctatgcagattcatttgtaattagaggtgatgaagtcagacaaatcgctccagggcaaactggaaagattgctgattataattataaattaccagatgattttacaggctgcgttatagcttggaattctaacaatcttgattctaaggttggtggtaattataattacctgtatagattgtttaggaagtctaatctcaaaccttttgagagagatatttcaactgaaatctatcaggccggtagcacaccttgtaatggtgttgaaggttttaattgttactttcctttacaatcatatggtttccaacccactaatggtgttggttaccaaccatacagagtagtagtactttcttttgaacttctacatgcaccagcaactgtttgtggacctaaaaagtctactaatttggttaaaaacaaatgtgtcaatttcaacttcaatggtttaacaggcacaggtgttcttactgagtctaacaaaaagtttctgcctttccaacaatttggcagagacattgctgacactactgatgctgtccgtgatccacagacacttgagattcttgacattacaccatgttcttttggtggtgtcagtgttataacaccaggaacaaatacttctaaccaggttgctgttctttatcaggatgttaactgcacagaagtccctgttgctattcatgcagatcaacttactcctacttggcgtgtttattctacaggttctaatgtttttcaaacacgtgcaggctgtttaataggggctgaacatgtcaacaactcatatgagtgtgacatacccattggtgcaggtatatgcgctagttatcagactcagactaattctcctcggcgggcacgtagtgtagctagtcaatccatcattgcctacactatgtcacttggtgcagaaaattcagttgcttactctaataactctattgccatacccacaaattttactattagtgttaccacagaaattctaccagtgtctatgaccaagacatcagtagattgtacaatgtacatttgtggtgattcaactgaatgcagcaatcttttgttgcaatatggcagtttttgtacacaattaaaccgtgctttaactggaatagctgttgaacaagacaaaaacacccaagaagtttttgcacaagtcaaacaaatttacaaaacaccaccaattaaagattttggtggttttaatttttcacaaatattaccagatccatcaaaaccaagcaagaggtcatttattgaagatctacttttcaacaaagtgacacttgcagatgctggcttcatcaaacaatatggtgattgccttggtgatattgctgctagagacctcatttgtgcacaaaagtttaacggccttactgttttgccacctttgctcacagatgaaatgattgctcaatacacttctgcactgttagcgggtacaatcacttctggttggacctttggtgcaggtgctgcattacaaataccatttgctatgcaaatggcttataggtttaatggtattggagttacacagaatgttctctatgagaaccaaaaattgattgccaaccaatttaatagtgctattggcaaaattcaagactcactttcttccacagcaagtgcacttggaaaacttcaagatgtggtcaaccaaaatgcacaagctttaaacacgcttgttaaacaacttagctccaattttggtgcaatttcaagtgttttaaatgatatcctttcacgtcttgacaaagttgaggctgaagtgcaaattgataggttgatcacaggcagacttcaaagtttgcagacatatgtgactcaacaattaattagagctgcagaaatcagagcttctgctaatcttgctgctactaaaatgtcagagtgtgtacttggacaatcaaaaagagttgatttttgtggaaagggctatcatcttatgtccttccctcagtcagcacctcatggtgtagtcttcttgcatgtgacttatgtccctgcacaagaaaagaacttcacaactgctcctgccatttgtcatgatggaaaagcacactttcctcgtgaaggtgtctttgtttcaaatggcacacactggtttgtaacacaaaggaatttttatgaaccacaaatcattactacagacaacacatttgtgtctggtaactgtgatgttgtaataggaattgtcaacaacacagtttatgatcctttgcaacctgaattagactcattcaaggaggagttagataaatattttaagaatcatacatcaccagatgttgatttaggtgacatctctggcattaatgcttcagttgtaaacattcaaaaagaaattgaccgcctcaatgaggttgccaagaatttaaatgaatctctcatcgatctccaagaacttggaaagtatgagcagtatataaaatggccatggtacatttggctaggttttatagctggcttgattgccatagtaatggtgacaattatgctttgctgtatgaccagttgctgtagttgtctcaagggctgttgttcttgtggatcctgctgcaaatttgatgaagacgactctgagccagtgctcaaaggagtcaaattacattacacataaacgaacttatggatttgtttatgagaatcttcacaattggaactgtaactttgaagcaaggtgaaatcaaggatgctactccttcagattttgttcgcgctactgcaacgataccgatacaagcctcactccctttcggatggcttattgttggcgttgcacttcttgctgtttttcagagcgcttccaaaatcataaccctcaaaaagagatggcaactagcactctccaagggtgttcactttgtttgcaacttgctgttgttgtttgtaacagtttactcacaccttttgctcgttgctgctggccttgaagccccttttctctatctttatgctttagtctacttcttgcagagtataaactttgtaagaataataatgaggctttggctttgctggaaatgccgttccaaaaacccattactttatgatgccaactattttctttgctggcatactaattgttacgactattgtataccttacaatagtgtaacttcttcaattgtcattacttcaggtgatggcacaacaagtcctatttctgaacatgactaccagattggtggttatactgaaaaatgggaatctggagtaaaagactgtgttgtattacacagttacttcacttcagactattaccagctgtactcaactcaattgagtacagacactggtgttgaacatgttaccttcttcatctacaataaaattgttgatgagcctgaagaacatgtccaaattcacacaatcgacggttcatccggagttgttaatccagtaatggaaccaatttatgatgaaccgacgacgactactagcgtgcctttgtaagcacaagctgatgagtacgaacttatgtactcattcgtttcggaagagacaggtacgttaatagttaatagcgtacttctttttcttgctttcgtggtattcttgctagttacactagccatccttactgcgcttcgattgtgtgcgtactgctgcaatattgttaacgtgagtcttgtaaaaccttctttttacgtttactctcgtgttaaaaatctgaattcttctagagttcctgatcttctggtctaaacgaactaaatattatattagtttttctgtttggaactttaattttagccatggcagattccaacggtactattaccgttgaagagcttaaaaagctccttgaacaatggaacctagtaataggtttcctattccttacatggatttgtcttctacaatttgcctatgccaacaggaataggtttttgtatataattaagttaattttcctctggctgttatggccagtaactttagcttgttttgtgcttgctgctgtttacagaataaattggatcaccggtggaattgctatcgcaatggcttgtcttgtaggcttgatgtggctcagctacttcattgcttctttcagactgtttgcgcgtacccgttccatgtggtcattcaatccagaaactaacattcttctcaacgtgccactccatggcactattctgaccagaccgcttctagaaagtgaactcgtaatcggagctgtgatccttcgtggacatcttcgtattgctggacaccatctaggacgctgtgacatcaaggacctgcctaaagaaatcactgttgctacatcacgaacgctttcttattacaaattgggagcttcgcagcgtgtagcaggtgactcaggttttgctgcatacagtcgctacaggattggcaactataaattaaacacagaccattccagtagcagtgacaatattgctttgcttgtacagtaagtgacaacagatgtttcatctcgttgactttcaggttactatagcagagatattactaattattatgaggacttttaaagtttccatttggaatcttgattacatcataaacctcataattaaaaatttatctaagtcactaactgagaataaatattctcaattagatgaagagcaaccaatggagattgattaaacgaacatgaaaattattcttttcttggcaccaatagtgtttataacactttgcttcacactcaaaagaaagacagaatgattgaactttcattaattgacttctatttgtgctttttagcctttctgctattccttgttttaattatgcttattatcttttggttctcacttgaactgcaagatcataatgaaacttgtcacgcctaaacgaacatgaaatttcttgttttcttaggaatcatcacaactgtagctgcatttcaccaagaatgtagtttacagtcatgtactcaacatcaaccatatgtagttgatgacccgtgtcctattcacttctattctaaatggtatattagagtaggagctagaaaatcagcacctttaattgaattgtgcgtggatgaggctggttctaaatcacccattcagtacatcgatatcggtaattatacagtttcctgtttaccttttacaattaattgccaggaacctaaattgggtagtcttgtagtgcgttgttcgttctatgaagactttttagagtatcatgacgttcgtgttgttttagatttcatctaaacgaacaaactaaaatgtctgataatggaccccaaaatcagcgaaatgcaccccgcattacgtttggtggaccctcagattcaactggcagtaaccagaatggagaacgcagtggggcgcgatcaaaacaacgtcggccccaaggtttacccaataatactgcgtcttggttcaccgctctcactcaacatggcaaggaagaccttaaattccctcgaggacaaggcgttccaattaacaccaatagcagtccagatgaccaaattggctactaccgaagagctaccagacgaattcgtggtggtgacggtaaaatgaaagatctcagtccaagatggtatttctactacctaggaactgggccagaagctggacttccctatggtgctaacaaagacggcatcatatgggttgcaactgagggagccttgaatacaccaaaagatcacattggcacccgcaatcctgctaacaatgctgcaatcgtgctacaacttcctcaaggaacaacattgccaaaaggcttctacgcagaagggagcagaggcggcagtcaagcctcttctcgttcctcatcacgtagtcgcaacagttcaagaaattcaactccaggcagcagtaggggaacttctcctgctagaatggctggcaatggcggtgatgctgctcttgctttgctgctgcttgacagattgaaccagcttgagagcaaaatgtctggtaaaggccaacaacaacaaggccaaactgtcactaagaaatctgctgctgaggcttctaagaagcctcggcaaaaacgtactgccactaaagcatacaatgtaacacaagctttcggcagacgtggtccagaacaaacccaaggaaattttggggaccaggaactaatcagacaaggaactgattacaaacattggccgcaaattgcacaatttgcccccagcgcttcagcgttcttcggaatgtcgcgcattggcatggaagtcacaccttcgggaacgtggttgacctacacaggtgccatcaaattggatgacaaagatccaaatttcaaagatcaagtcattttgctgaataagcatattgacgcatacaaaacattcccaccaacagagcctaaaaaggacaaaaagaagaaggctgatgaaactcaagccttaccgcagagacagaagaaacagcaaactgtgactcttcttcctgctgcagatttggatgatttctccaaacaattgcaacaatccatgagcagtgctgactcaactcaggcctaaactcatgcagaccacacaaggcagatgggctatataaacgttttcgcttttccgtttacgatatatagtctactcttgtgcagaatgaattctcgtaactacatagcacaagtagatgtagttaactttaatctcacatagcaatctttaatcagtgtgtaacattagggaggacttgaaagagccaccacattttcaccgaggccacgcggagtacgatcgagtgtacagtgaacaatgctagggagagctgcctatatggaagagccctaatgtgtaaaattaattttagtagtgctatccccatgtgattttaatagcttcttaggagaatgacaaaaaaaaaaaaaaaaaaaaaaaaa

SEQ ID NO: 21 - DNA, 29786 bp, Coronaviridae
  misc_feature 1..29786: note = SARS-CoV-2-7b nucleotide sequence
  source 1..29786: mol_type = other DNA
attaaaggtttataccttcccaggtaacaaaccaaccaactttcgatctcttgtagatctgttctctaaacgaactttaaaatctgtgtggctgtcactcggctgcatgcttagtgcactcacgcagtataattaataactaattactgtcgttgacaggacacgagtaactcgtctatcttctgcaggctgcttacggtttcgtccgtgttgcagccgatcatcagcacatctaggtttcgtccgggtgtgaccgaaaggtaagatggagagccttgtccctggtttcaacgagaaaacacacgtccaactcagtttgcctgttttacaggttcgcgacgtgctcgtacgtggctttggagactccgtggaggaggtcttatcagaggcacgtcaacatcttaaagatggcacttgtggcttagtagaagttgaaaaaggcgttttgcctcaacttgaacagccctatgtgttcatcaaacgttcggatgctcgaactgcacctcatggtcatgttatggttgagctggtagcagaactcgaaggcattcagtacggtcgtagtggtgagacacttggtgtccttgtccctcatgtgggcgaaataccagtggcttaccgcaaggttcttcttcgtaagaacggtaataaaggagctggtggccatagttacggcgccgatctaaagtcatttgacttaggcgacgagcttggcactgatccttatgaagattttcaagaaaactggaacactaaacatagcagtggtgttacccgtgaactcatgcgtgagcttaacggaggggcatacactcgctatgtcgataacaacttctgtggccctgatggctaccctcttgagtgcattaaagaccttctagcacgtgctggtaaagcttcatgcactttgtccgaacaactggactttattgacactaagaggggtgtatactgctgccgtgaacatgagcatgaaattgcttggtacacggaacgttctgaaaagagctatgaattgcagacaccttttgaaattaaattggcaaagaaatttgacaccttcaatggggaatgtccaaattttgtatttcccttaaattccataatcaagactattcaaccaagggttgaaaagaaaaagcttgatggctttatgggtagaattcgatctgtctatccagttgcgtcaccaaatgaatgcaaccaaatgtgcctttcaactctcatgaagtgtgatcattgtggtgaaacttcatggcagacgggcgattttgttaaagccacttgcgaattttgtggcactgagaatttgactaaagaaggtgccactacttgtggttacttaccccaaaatgctgttgttaaaatttattgtccagcatgtcacaattcagaagtaggacctgagcatagtcttgccgaataccataatgaatctggcttgaaaaccattcttcgtaagggtggtcgcactattgcctttggaggctgtgtgttctcttatgttggttgccataacaagtgtgcctattgggttccacgtgctagcgctaacataggttgtaaccatacaggtgttgttggagaaggttccgaaggtcttaatgacaaccttcttgaaatactccaaaaagagaaagtcaacatcaatattgttggtgactttaaacttaatgaagagatcgccattattttggcatctttttctgcttccacaagtgcttttgtggaaactgtgaaaggtttggattataaagcattcaaacaaattgttgaatcctgtggtaattttaaagttacaaaaggaaaagctaaaaaaggtgcctggaatattggtgaacagaaatcaatactgagtcctctttatgcatttgcatcagaggctgctcgtgttgtacgatcaattttctcccgcactcttgaaactgctcaaaattctgtgcgtgttttacagaaggccgctataacaatactagatggaatttcacagtattcactgagactcattgatgctatgatgttcacatctgatttggctactaacaatctagttgtaatggcctacattacaggtggtgttgttcagttgacttcgcagtggctaactaacatctttggcactgtttatgaaaaactcaaacccgtccttgattggcttgaagagaagtttaaggaaggtgtagagtttcttagagacggttgggaaattgttaaatttatctcaacctgtgcttgtgaaattgtcggtggacaaattgtcacctgtgcaaaggaaattaaggagagtgttcagacattctttaagcttgtaaataaatttttggctttgtgtgctgactctatcattattggtggagctaaacttaaagccttgaatttaggtgaaacatttgtcacgcactcaaagggattgtacagaaagtgtgttaaatccagagaagaaactggcctactcatgcctctaaaagccccaaaagaaattatcttcttagagggagaaacacttcccacagaagtgttaacagaggaagttgtcttgaaaactggtgatttacaaccattagaacaacctactagtgaagctgttgaagctccattggttggtacaccagtttgtattaacgggcttatgttgctcgaaatcaaagacacagaaaagtactgtgcccttgcacctaatatgatggtaacaaacaataccttcacactcaaaggcggtgcaccaacaaaggttacttttggtgatgacactgtgatagaagtgcaaggttacaagagtgtgaatatcacttttgaacttgatgaaaggattgataaagtacttaatgagaagtgctctgcctatacagttgaactcggtacagaagtaaatgagttcgcctgtgttgtggcagatgctgtcataaaaactttgcaaccagtatctgaattacttacaccactgggcattgatttagatgagtggagtatggctacatactacttatttgatgagtctggtgagtttaaattggcttcacatatgtattgttctttctaccctccagatgaggatgaagaagaaggtgattgtgaagaagaagagtttgagccatcaactcaatatgagtatggtactgaagatgattaccaaggtaaacctttggaatttggtgccacttctgctgctcttcaacctgaagaagagcaagaagaagattggttagatgatgatagtcaacaaactgttggtcaacaagacggcagtgaggacaatcagacaactactattcaaacaattgttgaggttcaacctcaattagagatggaacttacaccagttgttcagactattgaagtgaatagttttagtggttatttaaaacttactgacaatgtatacattaaaaatgcagacattgtggaagaagctaaaaaggtaaaaccaacagtggttgttaatgcagccaatgtttaccttaaacatggaggaggtgttgcaggagccttaaataaggctactaacaatgccatgcaagttgaatctgatgattacatagctactaatggaccacttaaagtgggtggtagttgtgttttaagcggacacaatcttgctaaacactgtcttcatgttgtcggcccaaatgttaacaaaggtgaagacattcaacttcttaagagtgcttatgaaaattttaatcagcacgaagttctacttgcaccattattatcagctggtatttttggtgctgaccctatacattctttaagagtttgtgtagatactgttcgcacaaatgtctacttagctgtctttgataaaaatctctatgacaaacttgtttcaagctttttggaaatgaagagtgaaaagcaagttgaacaaaagatcgctgagattcctaaagaggaagttaagccatttataactgaaagtaaaccttcagttgaacagagaaaacaagatgataagaaaatcaaagcttgtgttgaagaagttacaacaactctggaagaaactaagttcctcacagaaaacttgttactttatattgacattaatggcaatcttcatccagattctgccactcttgttagtgacattgacatcactttcttaaagaaagatgctccatatatagtgggtgatgttgttcaagagggtgttttaactgctgtggttatacctactaaaaaggctggtggcactactgaaatgctagcgaaagctttgagaaaagtgccaacagacaattatataaccacttacccgggtcagggtttaaatggttacactgtagaggaggcaaagacagtgcttaaaaagtgtaaaagtgccttttacattctaccatctattatctctaatgagaagcaagaaattcttggaactgtttcttggaatttgcgagaaatgcttgcacatgcagaagaaacacgcaaattaatgcctgtctgtgtggaaactaaagccatagtttcaactatacagcgtaaatataagggtattaaaatacaagagggtgtggttgattatggtgctagattttacttttacaccagtaaaacaactgtagcgtcacttatcaacacacttaacgatctaaatgaaactcttgttacaatgccacttggctatgtaacacatggcttaaatttggaagaagctgctcggtatatgagatctctcaaagtgccagctacagtttctgtttcttcacctgatgctgttacagcgtataatggttatcttacttcttcttctaaaacacctgaagaacattttattgaaaccatctcacttgctggttcctataaagattggtcctattctggacaatctacacaactaggtatagaatttcttaagagaggtgataaaagtgtatattacactagtaatcctaccacattccacctagatggtgaagttatcacctttgacaatcttaagacacttctttctttgagagaagtgaggactattaaggtgtttacaacagtagacaacattaacctccacacgcaagttgtggacatgtcaatgacatatggacaacagtttggtccaacttatttggatggagctgatgttactaaaataaaacctcataattcacatgaaggtaaaacattttatgttttacctaatgatgacactctacgtgttgaggcttttgagtactaccacacaactgatcctagttttctgggtaggtacatgtcagcattaaatcacactaaaaagtggaaatacccacaagttaatggtttaacttctattaaatgggcagataacaactgttatcttgccactgcattgttaacactccaacaaatagagttgaagtttaatccacctgctctacaagatgcttattacagagcaagggctggtgaagctgctaacttttgtgcacttatcttagcctactgtaataagacagtaggtgagttaggtgatgttagagaaacaatgagttacttgtttcaacatgccaatttagattcttgcaaaagagtcttgaacgtggtgtgtaaaacttgtggacaacagcagacaacccttaagggtgtagaagctgttatgtacatgggcacactttcttatgaacaatttaagaaaggtgttcagataccttgtacgtgtggtaaacaagctacaaaatatctagtacaacaggagtcaccttttgttatgatgtcagcaccacctgctcagtatgaacttaagcatggtacatttacttgtgctagtgagtacactggtaattaccagtgtggtcactataaacatataacttctaaagaaactttgtattgcatagacggtgctttacttacaaagtcctcagaatacaaaggtcctattacggatgttttctacaaagaaaacagttacacaacaaccataaaaccagttacttataaattggatggtgttgtttgtacagaaattgaccctaagttggacaattattataagaaagacaattcttatttcacagagcaaccaattgatcttgtaccaaaccaaccatatccaaacgcaagcttcgataattttaagtttgtatgtgataatatcaaatttgctgatgatttaaaccagttaactggttataagaaacctgcttcaagagagcttaaagttacatttttccctgacttaaatggtgatgtggtggctattgattataaacactacacaccctcttttaagaaaggagctaaattgttacataaacctattgtttggcatgttaacaatgcaactaataaagccacgtataaaccaaatacctggtgtatacgttgtctttggagcacaaaaccagttgaaacatcaaattcgtttgatgtactgaagtcagaggacgcgcagggaatggataatcttgcctgcgaagatctaaaaccagtctctgaagaagtagtggaaaatcctaccatacagaaagacgttcttgagtgtaatgtgaaaactaccgaagttgtaggagacattatacttaaaccagcaaataatagtttaaaaattacagaagaggttggccacacagatctaatggctgcttatgtagacaattctagtcttactattaagaaacctaatgaattatctagagtattaggtttgaaaacccttgctactcatggtttagctgctgttaatagtgtcccttgggatactatagctaattatgctaagccttttcttaacaaagttgttagtacaactactaacatagttacacggtgtttaaaccgtgtttgtactaattatatgccttatttctttactttattgctacaattgtgtacttttactagaagtacaaattctagaattaaagcatctatgccgactactatagcaaagaatactgttaagagtgtcggtaaattttgtctagaggcttcatttaattatttgaagtcacctaatttttctaaactgataaatattataatttggtttttactattaagtgtttgcctaggttctttaatctactcaaccgctgctttaggtgttttaatgtctaatttaggcatgccttcttactgtactggttacagagaaggctatttgaactctactaatgtcactattgcaacctactgtactggttctataccttgtagtgtttgtcttagtggtttagattctttagacacctatccttctttagaaactatacaaattaccatttcatcttttaaatgggatttaactgcttttggcttagttgcagagtggtttttggcatatattcttttcactaggtttttctatgtacttggattggctgcaatcatgcaattgtttttcagctattttgcagtacattttattagtaattcttggcttatgtggttaataattaatcttgtacaaatggccccgatttcagctatggttagaatgtacatcttctttgcatcattttattatgtatggaaaagttatgtgcatgttgtagacggttgtaattcatcaacttgtatgatgtgttacaaacgtaatagagcaacaagagtcgaatgtacaactattgttaatggtgttagaaggtccttttatgtctatgctaatggaggtaaaggcttttgcaaactacacaattggaattgtgttaattgtgatacattctgtgctggtagtacatttattagtgatgaagttgcgagagacttgtcactacagtttaaaagaccaataaatcctactgaccagtcttcttacatcgttgatagtgttacagtgaagaatggttccatccatctttactttgataaagctggtcaaaagacttatgaaagacattctctctctcattttgttaacttagacaacctgagagctaataacactaaaggttcattgcctattaatgttatagtttttgatggtaaatcaaaatgtgaagaatcatctgcaaaatcagcgtctgtttactacagtcagcttatgtgtcaacctatactgttactagatcaggcattagtgtctgatgttggtgatagtgcggaagttgcagttaaaatgtttgatgcttacgttaatacgttttcatcaacttttaacgtaccaatggaaaaactcaaaacactagttgcaactgcagaagctgaacttgcaaagaatgtgtccttagacaatgtcttatctacttttatttcagcagctcggcaagggtttgttgattcagatgtagaaactaaagatgttgttgaatgtcttaaattgtcacatcaatctgacatagaagttactggcgatagttgtaataactatatgctcacctataacaaagttgaaaacatgacaccccgtgaccttggtgcttgtattgactgtagtgcgcgtcatattaatgcgcaggtagcaaaaagtcacaacattgctttgatatggaacgttaaagatttcatgtcattgtctgaacaactacgaaaacaaatacgtagtgctgctaaaaagaataacttaccttttaagttgacatgtgcaactactagacaagttgttaatgttgtaacaacaaagatagcacttaagggtggtaaaattgttaataattggttgaagcagttaattaaagttacacttgtgttcctttttgttgctgctattttctatttaataacacctgttcatgtcatgtctaaacatactgacttttcaagtgaaatcataggatacaaggctattgatggtggtgtcactcgtgacatagcatctacagatacttgttttgctaacaaacatgctgattttgacacatggtttagccagcgtggtggtagttatactaatgacaaagcttgcccattgattgctgcagtcataacaagagaagtgggttttgtcgtgcctggtttgcctggcacgatattacgcacaactaatggtgactttttgcatttcttacctagagtttttagtgcagttggtaacatctgttacacaccatcaaaacttatagagtacactgactttgcaacatcagcttgtgttttggctgctgaatgtacaatttttaaagatgcttctggtaagccagtaccatattgttatgataccaatgtactagaaggttctgttgcttatgaaagtttacgccctgacacacgttatgtgctcatggatggctctattattcaatttcctaacacctaccttgaaggttctgttagagtggtaacaacttttgattctgagtactgtaggcacggcacttgtgaaagatcagaagctggtgtttgtgtatctactagtggtagatgggtacttaacaatgattattacagatctttaccaggagttttctgtggtgtagatgctgtaaatttacttactaatatgtttacaccactaattcaacctattggtgctttggacatatcagcatctatagtagctggtggtattgtagctatcgtagtaacatgccttgcctactattttatgaggtttagaagagcttttggtgaatacagtcatgtagttgcctttaatactttactattccttatgtcattcactgtactctgtttaacaccagtttactcattcttacctggtgtttattctgttatttacttgtacttgacattttatcttactaatgatgtttcttttttagcacatattcagtggatggttatgttcacacctttagtacctttctggataacaattgcttatatcatttgtatttccacaaagcatttctattggttctttagtaattacctaaagagacgtgtagtctttaatggtgtttcctttagtacttttgaagaagctgcgctgtgcacctttttgttaaataaagaaatgtatctaaagttgcgtagtgatgtgctattacctcttacgcaatataatagatacttagctctttataataagtacaagtattttagtggagcaatggatacaactagctacagagaagctgcttgttgtcatctcgcaaaggctctcaatgacttcagtaactcaggttctgatgttctttaccaaccaccacaaacctctatcacctcagctgttttgcagagtggttttagaaaaatggcattcccatctggtaaagttgagggttgtatggtacaagtaacttgtggtacaactacacttaacggtctttggcttgatgacgtagtttactgtccaagacatgtgatctgcacctctgaagacatgcttaaccctaattatgaagatttactcattcgtaagtctaatcataatttcttggtacaggctggtaatgttcaactcagggttattggacattctatgcaaaattgtgtacttaagcttaaggttgatacagccaatcctaagacacctaagtataagtttgttcgcattcaaccaggacagactttttcagtgttagcttgttacaatggttcaccatctggtgtttaccaatgtgctatgaggcccaatttcactattaagggttcattccttaatggttcatgtggtagtgttggttttaacatagattatgactgtgtctctttttgttacatgcaccatatggaattaccaactggagttcatgctggcacagacttagaaggtaacttttatggaccttttgttgacaggcaaacagcacaagcagctggtacggacacaactattacagttaatgttttagcttggttgtacgctgctgttataaatggagacaggtggtttctcaatcgatttaccacaactcttaatgactttaaccttgtggctatgaagtacaattatgaacctctaacacaagaccatgttgacatactaggacctctttctgctcaaactggaattgccgttttagatatgtgtgcttcattaaaagaattactgcaaaatggtatgaatggacgtaccatattgggtagtgctttattagaagatgaatttacaccttttgatgttgttagacaatgctcaggtgttactttccaaagtgcagtgaaaagaacaatcaagggtacacaccactggttgttactcacaattttgacttcacttttagttttagtccagagtactcaatggtctttgttcttttttttgtatgaaaatgcctttttaccttttgctatgggtattattgctatgtctgcttttgcaatgatgtttgtcaaacataagcatgcatttctctgtttgtttttgttaccttctcttgccactgtagcttattttaatatggtctatatgcctgctagttgggtgatgcgtattatgacatggttggatatggttgatactagtttgtctggttttaagctaaaagactgtgttatgtatgcatcagctgtagtgttactaatccttatgacagcaagaactgtgtatgatgatggtgctaggagagtgtggacacttatgaatgtcttgacactcgtttataaagtttattatggtaatgctttagatcaagccatttccatgtgggctcttataatctctgttacttctaactactcaggtgtagttacaactgtcatgtttttggccagaggtattgtttttatgtgtgttgagtattgccctattttcttcataactggtaatacacttcagtgtataatgctagtttattgtttcttaggctatttttgtacttgttactttggcctcttttgtttactcaaccgctactttagactgactcttggtgtttatgattacttagtttctacacaggagtttagatatatgaattcacagggactactcccacccaagaatagcatagatgccttcaaactcaacattaaattgttgggtgttggtggcaaaccttgtatcaaagtagccactgtacagtctaaaatgtcagatgtaaagtgcacatcagtagtcttactctcagttttgcaacaactcagagtagaatcatcatctaaattgtgggctcaatgtgtccagttacacaatgacattctcttagctaaagatactactgaagcctttgaaaaaatggtttcactactttctgttttgctttccatgcagggtgctgtagacataaacaagctttgtgaagaaatgctggacaacagggcaaccttacaagctatagcctcagagtttagttcccttccatcatatgcagcttttgctactgctcaagaagcttatgagcaggctgttgctaatggtgattctgaagttgttcttaaaaagttgaagaagtctttgaatgtggctaaatctgaatttgaccgtgatgcagccatgcaacgtaagttggaaaagatggctgatcaagctatgacccaaatgtataaacaggctagatctgaggacaagagggcaaaagttactagtgctatgcagacaatgcttttcactatgcttagaaagttggataatgatgcactcaacaacattatcaacaatgcaagagatggttgtgttcccttgaacataatacctcttacaacagcagccaaactaatggttgtcataccagactataacacatataaaaatacgtgtgatggtacaacatttacttatgcatcagcattgtgggaaatccaacaggttgtagatgcagatagtaaaattgttcaacttagtgaaattagtatggacaattcacctaatttagcatggcctcttattgtaacagctttaagggccaattctgctgtcaaattacagaataatgagcttagtcctgttgcactacgacagatgtcttgtgctgccggtactacacaaactgcttgcactgatgacaatgcgttagcttactacaacacaacaaagggaggtaggtttgtacttgcactgttatccgatttacaggatttgaaatgggctagattccctaagagtgatggaactggtactatctatacagaactggaaccaccttgtaggtttgttacagacacacctaaaggtcctaaagtgaagtatttatactttattaaaggattaaacaacctaaatagaggtatggtacttggtagtttagctgccacagtacgtctacaagctggtaatgcaacagaagtgcctgccaattcaactgtattatctttctgtgcttttgctgtagatgctgctaaagcttacaaagattatctagctagtgggggacaaccaatcactaattgtgttaagatgttgtgtacacacactggtactggtcaggcaataacagttacaccggaagccaatatggatcaagaatcctttggtggtgcatcgtgttgtctgtactgccgttgccacatagatcatccaaatcctaaaggattttgtgacttaaaaggtaagtatgtacaaatacctacaacttgtgctaatgaccctgtgggttttacacttaaaaacacagtctgtaccgtctgcggtatgtggaaaggttatggctgtagttgtgatcaactccgcgaacccatgcttcagtcagctgatgcacaatcgtttttaaacgggtttgcggtgtaagtgcagcccgtcttacaccgtgcggcacaggcactagtactgatgtcgtatacagggcttttgacatctacaatgataaagtagctggttttgctaaattcctaaaaactaattgttgtcgcttccaagaaaaggacgaagatgacaatttaattgattcttactttgtagttaagagacacactttctctaactaccaacatgaagaaacaatttataatttacttaaggattgtccagctgttgctaaacatgacttctttaagtttagaatagacggtgacatggtaccacatatatcacgtcaacgtcttactaaatacacaatggcagacctcgtctatgctttaaggcattttgatgaaggtaattgtgacacattaaaagaaatacttgtcacatacaattgttgtgatgatgattatttcaataaaaaggactggtatgattttgtagaaaacccagatatattacgcgtatacgccaacttaggtgaacgtgtacgccaagctttgttaaaaacagtacaattctgtgatgccatgcgaaatgctggtattgttggtgtactgacattagataatcaagatctcaatggtaactggtatgatttcggtgatttcatacaaaccacgccaggtagtggagttcctgttgtagattcttattattcattgttaatgcctatattaaccttgaccagggctttaactgcagagtcacatgttgacactgacttaacaaagccttacattaagtgggatttgttaaaatatgacttcacggaagagaggttaaaactctttgaccgttattttaaatattgggatcagacataccacccaaattgtgttaactgtttggatgacagatgcattctgcattgtgcaaactttaatgttttattctctacagtgttcccacctacaagttttggaccactagtgagaaaaatatttgttgatggtgttccatttgtagtttcaactggataccacttcagagagctaggtgttgtacataatcaggatgtaaacttacatagctctagacttagttttaaggaattacttgtgtatgctgctgaccctgctatgcacgctgcttctggtaatctattactagataaacgcactacgtgcttttcagtagctgcacttactaacaatgttgcttttcaaactgtcaaacccggtaattttaacaaagacttctatgactttgctgtgtctaagggtttctttaaggaaggaagttctgttgaattaaaacacttcttctttgctcaggatggtaatgctgctatcagcgattatgactactatcgttataatctaccaacaatgtgtgatatcagacaactactatttgtagttgaagttgttgataagtactttgattgttacgatggtggctgtattaatgctaaccaagtcatcgtcaacaacctagacaaatcagctggttttccatttaataaatggggtaaggctagactttattatgattcaatgagttatgaggatcaagatgcacttttcgcatatacaaaacgtaatgtcatccctactataactcaaatgaatcttaagtatgccattagtgcaaagaatagagctcgcaccgtagctggtgtctctatctgtagtactatgaccaatagacagtttcatcaaaaattattgaaatcaatagccgccactagaggagctactgtagtaattggaacaagcaaattctatggtggttggcacaacatgttaaaaactgtttatagtgatgtagaaaaccctcaccttatgggttgggattatcctaaatgtgatagagccatgcctaacatgcttagaattatggcctcacttgttcttgctcgcaaacatacaacgtgttgtagcttgtcacaccgtttctatagattagctaatgagtgtgctcaagtattgagtgaaatggtcatgtgtggcggttcactatatgttaaaccaggtggaacctcatcaggagatgccacaactgcttatgctaatagtgtttttaacatttgtcaagctgtcacggccaatgttaatgcacttttatctactgatggtaacaaaattgccgataagtatgtccgcaatttacaacacagactttatgagtgtctctatagaaatagagatgttgacacagactttgtgaatgagttttacgcatatttgcgtaaacatttctcaatgatgatactctctgacgatgctgttgtgtgtttcaatagcacttatgcatctcaaggtctagtggctagcataaagaactttaagtcagttctttattatcaaaacaatgtttttatgtctgaagcaaaatgttggactgagactgaccttactaaaggacctcatgaattttgctctcaacatacaatgctagttaaacagggtgatgattatgtgtaccttccttacccagatccatcaagaatcctaggggccggctgttttgtagatgatatcgtaaaaacagatggtacacttatgattgaacggttcgtgtctttagctatagatgcttacccacttactaaacatcctaatcaggagtatgctgatgtctttcatttgtacttacaatacataagaaagctacatgatgagttaacaggacacatgttagacatgtattctgttatgcttactaatgataacacttcaaggtattgggaacctgagttttatgaggctatgtacacaccgcatacagtcttacaggctgttggggcttgtgttctttgcaattcacagacttcattaagatgtggtgcttgcatacgtagaccattcttatgttgtaaatgctgttacgaccatgtcatatcaacatcacataaattagtcttgtctgttaatccgtatgtttgcaatgctccaggttgtgatgtcacagatgtgactcaactttacttaggaggtatgagctattattgtaaatcacataaaccacccattagttttccattgtgtgctaatggacaagtttttggtttatataaaaatacatgtgttggtagcgataatgttactgactttaatgcaattgcaacatgtgactggacaaatgctggtgattacattttagctaacacctgtactgaaagactcaagctttttgcagcagaaacgctcaaagctactgaggagacatttaaactgtcttatggtattgctactgtacgtgaagtgctgtctgacagagaattacatctttcatgggaagttggtaaacctagaccaccacttaaccgaaattatgtctttactggttatcgtgtaactaaaaacagtaaagtacaaataggagagtacacctttgaaaaaggtgactatggtgatgctgttgtttaccgaggtacaacaacttacaaattaaatgttggtgattattttgtgctgacatcacatacagtaatgccattaagtgcacctacactagtgccacaagagcactatgttagaattactggcttatacccaacactcaatatctcagatgagttttctagcaatgttgcaaattatcaaaaggttggtatgcaaaagtattctacactccagggaccacctggtactggtaagagtcattttgctattggcctagctctctactacccttctgctcgcatagtgtatacagcttgctctcatgccgctgttgatgcactatgtgagaaggcattaaaatatttgcctatagataaatgtagtagaattatacctgcacgtgctcgtgtagagtgttttgataaattcaaagtgaattcaacattagaacagtatgtcttttgtactgtaaatgcattgcctgagacgacagcagatatagttgtctttgatgaaatttcaatggccacaaattatgatttgagtgttgtcaatgccagattacgtgctaagcactatgtgtacattggcgaccctgctcaattacctgcaccacgcacattgctaactaagggcacactagaaccagaatatttcaattcagtgtgtagacttatgaaaactataggtccagacatgttcctcggaacttgtcggcgttgtcctgctgaaattgttgacactgtgagtgctttggtttatgataataagcttaaagcacataaagacaaatcagctcaatgctttaaaatgttttataagggtgttatcacgcatgatgtttcatctgcaattaacaggccacaaataggcgtggtaagagaattccttacacgtaaccctgcttggagaaaagctgtctttatttcaccttataattcacagaatgctgtagcctcaaagattttgggactaccaactcaaactgttgattcatcacagggctcagaatatgactatgtcatattcactcaaaccactgaaacagctcactcttgtaatgtaaacagatttaatgttgctattaccagagcaaaagtaggcatactttgcataatgtctgatagagacctttatgacaagttgcaatttacaagtcttgaaattccacgtaggaatgtggcaactttacaagctgaaaatgtaacaggactctttaaagattgtagtaaggtaatcactgggttacatcctacacaggcacctacacacctcagtgttgacactaaattcaaaactgaaggtttatgtgttgacatacctggcatacctaaggacatgacctatagaagactcatctctatgatgggttttaaaatgaattatcaagttaatggttaccctaacatgtttatcacccgcgaagaagctataagacatgtacgtgcatggattggcttcgatgtcgaggggtgtcatgctactagagaagctgttggtaccaatttacctttacagctaggtttttctacaggtgttaacctagttgctgtacctacaggttatgttgatacacctaataatacagatttttccagagttagtgctaaaccaccgcctggagatcaatttaaacacctcataccacttatgtacaaaggacttccttggaatgtagtgcgtataaagattgtacaaatgttaagtgacacacttaaaaatctctctgacagagtcgtatttgtcttatgggcacatggctttgagttgacatctatgaagtattttgtgaaaataggacctgagcgcacctgttgtctatgtgatagacgtgccacatgcttttccactgcttcagacacttatgcctgttggcatcattctattggatttgattacgtctataatccgtttatgattgatgttcaacaatggggttttacaggtaacctacaaagcaaccatgatctgtattgtcaagtccatggtaatgcacatgtagctagttgtgatgcaatcatgactaggtgtctagctgtccacgagtgctttgttaagcgtgttgactggactattgaatatcctataattggtgatgaactgaagattaatgcggcttgtagaaaggttcaacacatggttgttaaagctgcattattagcagacaaattcccagttcttcacgacattggtaaccctaaagctattaagtgtgtacctcaagctgatgtagaatggaagttctatgatgcacagccttgtagtgacaaagcttataaaatagaagaattattctattcttatgccacacattctgacaaattcacagatggtgtatgcctattttggaattgcaatgtcgatagatatcctgctaattccattgtttgtagatttgacactagagtgctatctaaccttaacttgcctggttgtgatggtggcagtttgtatgtaaataaacatgcattccacacaccagcttttgataaaagtgcttttgttaatttaaaacaattaccatttttctattactctgacagtccatgtgagtctcatggaaaacaagtagtgtcagatatagattatgtaccactaaagtctgctacgtgtataacacgttgcaatttaggtggtgctgtctgtagacatcatgctaatgagtacagattgtatctcgatgcttataacatgatgatctcagctggctttagcttgtgggtttacaaacaatttgatacttataacctctggaacacttttacaagacttcagagtttagaaaatgtggcttttaatgttgtaaataagggacactttgatggacaacagggtgaagtaccagtttctatcattaataacactgtttacacaaaagttgatggtgttgatgtagaattgtttgaaaataaaacaacattacctgttaatgtagcatttgagctttgggctaagcgcaacattaaaccagtaccagaggtgaaaatactcaataatttgggtgtggacattgctgctaatactgtgatctgggactacaaaagagatgctccagcacatatatctactattggtgtttgttctatgactgacatagccaagaaaccaactgaaacgatttgtgcaccactcactgtcttttttgatggtagagttgatggtcaagtagacttatttagaaatgcccgtaatggtgttcttattacagaaggtagtgttaaaggtttacaaccatctgtgggtcccaaacaagctagtcttaatggagtcacattaattggagaagccgtaaaaacacagttcaattattataagaaagttgatggtgttgtccaacaattacctgaaacttactttactcagagtagaaatttacaagaatttaaacccaggagtcaaatggaaattgatttcttagaattagctatggatgaattcattgaacggtataaattagaaggctatgccttcgaacatatcgtttatggagattttagtcatagtcagttaggtggtttacatctactgattggactagctaaacgttttaaggaatcaccttttgaattagaagattttattcctatggacagtacagttaaaaactatttcataacagatgcgcaaacaggttcatctaagtgtgtgtgttctgttattgatttattacttgatgattttgttgaaataataaaatcccaagatttatctgtagtttctaaggttgtcaaagtgactattgactatacagaaatttcatttatgctttggtgtaaagatggccatgtagaaacattttacccaaaattacaatctagtcaagcgtggcaaccgggtgttgctatgcctaatctttacaaaatgcaaagaatgctattagaaaagtgtgaccttcaaaattatggtgatagtgcaacattacctaaaggcataatgatgaatgtcgcaaaatatactcaactgtgtcaatatttaaacacattaacattagctgtaccctataatatgagagttatacattttggtgctggttctgataaaggagttgcaccaggtacagctgttttaagacagtggttgcctacgggtacgctgcttgtcgattcagatcttaatgactttgtctctgatgcagattcaactttgattggtgattgtgcaactgtacatacagctaataaatgggatctcattattagtgatatgtacgaccctaagactaaaaatgttacaaaagaaaatgactctaaagagggttttttcacttacatttgtgggtttatacaacaaaagctagctcttggaggttccgtggctataaagataacagaacattcttggaatgctgatctttataagctcatgggacacttcgcatggtggacagcctttgttactaatgtgaatgcgtcatcatctgaagcatttttaattggatgtaattatcttggcaaaccacgcgaacaaatagatggttatgtcatgcatgcaaattacatattttggaggaatacaaatccaattcagttgtcttcctattctttatttgacatgagtaaatttccccttaaattaaggggtactgctgttatgtctttaaaagaaggtcaaatcaatgatatgattttatctcttcttagtaaaggtagacttataattagagaaaacaacagagttgttatttctagtgatgttcttgttaacaactaaacgaacaatgtttgtttttcttgttttattgccactagtctctagtcagtgtgttaatcttacaaccagaactcaattaccccctgcatacactaattctttcacacgtggtgtttattaccctgacaaagttttcagatcctcagttttacattcaactcaggacttgttcttacctttcttttccaatgttacttggttccatgctatacatgtctctgggaccaatggtactaagaggtttgataaccctgtcctaccatttaatgatggtgtttattttgcttccactgagaagtctaacataataagaggctggatttttggtactactttagattcgaagacccagtccctacttattgttaataacgctactaatgttgttattaaagtctgtgaatttcaattttgtaatgatccatttttgggtgtttattaccacaaaaacaacaaaagttggatggaaagtgagttcagagtttattctagtgcgaataattgcacttttgaatatgtctctcagccttttcttatggaccttgaaggaaaacagggtaatttcaaaaatcttagggaatttgtgtttaagaatattgatggttattttaaaatatattctaagcacacgcctattaatttagtgcgtgatctccctcagggtttttcggctttagaaccattggtagatttgccaataggtattaacatcactaggtttcaaactttacttgctttacatagaagttatttgactcctggtgattcttcttcaggttggacagctggtgctgcagcttattatgtgggttatcttcaacctaggacttttctattaaaatataatgaaaatggaaccattacagatgctgtagactgtgcacttgaccctctctcagaaacaaagtgtacgttgaaatccttcactgtagaaaaaggaatctatcaaacttctaactttagagtccaaccaacagaatctattgttagatttcctaatattacaaacttgtgcccttttggtgaagtttttaacgccaccagatttgcatctgtttatgcttggaacaggaagagaatcagcaactgtgttgctgattattctgtcctatataattccgcatcattttccacttttaagtgttatggagtgtctcctactaaattaaatgatctctgctttactaatgtctatgcagattcatttgtaattagaggtgatgaagtcagacaaatcgctccagggcaaactggaaagattgctgattataattataaattaccagatgattttacaggctgcgttatagcttggaattctaacaatcttgattctaaggttggtggtaattataattacctgtatagattgtttaggaagtctaatctcaaaccttttgagagagatatttcaactgaaatctatcaggccggtagcacaccttgtaatggtgttgaaggttttaattgttactttcctttacaatcatatggtttccaacccactaatggtgttggttaccaaccatacagagtagtagtactttcttttgaacttctacatgcaccagcaactgtttgtggacctaaaaagtctactaatttggttaaaaacaaatgtgtcaatttcaacttcaatggtttaacaggcacaggtgttcttactgagtctaacaaaaagtttctgcctttccaacaatttggcagagacattgctgacactactgatgctgtccgtgatccacagacacttgagattcttgacattacaccatgttcttttggtggtgtcagtgttataacaccaggaacaaatacttctaaccaggttgctgttctttatcaggatgttaactgcacagaagtccctgttgctattcatgcagatcaacttactcctacttggcgtgtttattctacaggttctaatgtttttcaaacacgtgcaggctgtttaataggggctgaacatgtcaacaactcatatgagtgtgacatacccattggtgcaggtatatgcgctagttatcagactcagactaattctcctcggcgggcacgtagtgtagctagtcaatccatcattgcctacactatgtcacttggtgcagaaaattcagttgcttactctaataactctattgccatacccacaaattttactattagtgttaccacagaaattctaccagtgtctatgaccaagacatcagtagattgtacaatgtacatttgtggtgattcaactgaatgcagcaatcttttgttgcaatatggcagtttttgtacacaattaaaccgtgctttaactggaatagctgttgaacaagacaaaaacacccaagaagtttttgcacaagtcaaacaaatttacaaaacaccaccaattaaagattttggtggttttaatttttcacaaatattaccagatccatcaaaaccaagcaagaggtcatttattgaagatctacttttcaacaaagtgacacttgcagatgctggcttcatcaaacaatatggtgattgccttggtgatattgctgctagagacctcatttgtgcacaaaagtttaacggccttactgttttgccacctttgctcacagatgaaatgattgctcaatacacttctgcactgttagcgggtacaatcacttctggttggacctttggtgcaggtgctgcattacaaataccatttgctatgcaaatggcttataggtttaatggtattggagttacacagaatgttctctatgagaaccaaaaattgattgccaaccaatttaatagtgctattggcaaaattcaagactcactttcttccacagcaagtgcacttggaaaacttcaagatgtggtcaaccaaaatgcacaagctttaaacacgcttgttaaacaacttagctccaattttggtgcaatttcaagtgttttaaatgatatcctttcacgtcttgacaaagttgaggctgaagtgcaaattgataggttgatcacaggcagacttcaaagtttgcagacatatgtgactcaacaattaattagagctgcagaaatcagagcttctgctaatcttgctgctactaaaatgtcagagtgtgtacttggacaatcaaaaagagttgatttttgtggaaagggctatcatcttatgtccttccctcagtcagcacctcatggtgtagtcttcttgcatgtgacttatgtccctgcacaagaaaagaacttcacaactgctcctgccatttgtcatgatggaaaagcacactttcctcgtgaaggtgtctttgtttcaaatggcacacactggtttgtaacacaaaggaatttttatgaaccacaaatcattactacagacaacacatttgtgtctggtaactgtgatgttgtaataggaattgtcaacaacacagtttatgatcctttgcaacctgaattagactcattcaaggaggagttagataaatattttaagaatcatacatcaccagatgttgatttaggtgacatctctggcattaatgcttcagttgtaaacattcaaaaagaaattgaccgcctcaatgaggttgccaagaatttaaatgaatctctcatcgatctccaagaacttggaaagtatgagcagtatataaaatggccatggtacatttggctaggttttatagctggcttgattgccatagtaatggtgacaattatgctttgctgtatgaccagttgctgtagttgtctcaagggctgttgttcttgtggatcctgctgcaaatttgatgaagacgactctgagccagtgctcaaaggagtcaaattacattacacataaacgaacttatggatttgtttatgagaatcttcacaattggaactgtaactttgaagcaaggtgaaatcaaggatgctactccttcagattttgttcgcgctactgcaacgataccgatacaagcctcactccctttcggatggcttattgttggcgttgcacttcttgctgtttttcagagcgcttccaaaatcataaccctcaaaaagagatggcaactagcactctccaagggtgttcactttgtttgcaacttgctgttgttgtttgtaacagtttactcacaccttttgctcgttgctgctggccttgaagccccttttctctatctttatgctttagtctacttcttgcagagtataaactttgtaagaataataatgaggctttggctttgctggaaatgccgttccaaaaacccattactttatgatgccaactattttctttgctggcatactaattgttacgactattgtataccttacaatagtgtaacttcttcaattgtcattacttcaggtgatggcacaacaagtcctatttctgaacatgactaccagattggtggttatactgaaaaatgggaatctggagtaaaagactgtgttgtattacacagttacttcacttcagactattaccagctgtactcaactcaattgagtacagacactggtgttgaacatgttaccttcttcatctacaataaaattgttgatgagcctgaagaacatgtccaaattcacacaatcgacggttcatccggagttgttaatccagtaatggaaccaatttatgatgaaccgacgacgactactagcgtgcctttgtaagcacaagctgatgagtacgaacttatgtactcattcgtttcggaagagacaggtacgttaatagttaatagcgtacttctttttcttgctttcgtggtattcttgctagttacactagccatccttactgcgcttcgattgtgtgcgtactgctgcaatattgttaacgtgagtcttgtaaaaccttctttttacgtttactctcgtgttaaaaatctgaattcttctagagttcctgatcttctggtctaaacgaactaaatattatattagtttttctgtttggaactttaattttagccatggcagattccaacggtactattaccgttgaagagcttaaaaagctccttgaacaatggaacctagtaataggtttcctattccttacatggatttgtcttctacaatttgcctatgccaacaggaataggtttttgtatataattaagttaattttcctctggctgttatggccagtaactttagcttgttttgtgcttgctgctgtttacagaataaattggatcaccggtggaattgctatcgcaatggcttgtcttgtaggcttgatgtggctcagctacttcattgcttctttcagactgtttgcgcgtacccgttccatgtggtcattcaatccagaaactaacattcttctcaacgtgccactccatggcactattctgaccagaccgcttctagaaagtgaactcgtaatcggagctgtgatccttcgtggacatcttcgtattgctggacaccatctaggacgctgtgacatcaaggacctgcctaaagaaatcactgttgctacatcacgaacgctttcttattacaaattgggagcttcgcagcgtgtagcaggtgactcaggttttgctgcatacagtcgctacaggattggcaactataaattaaacacagaccattccagtagcagtgacaatattgctttgcttgtacagtaagtgacaacagatgtttcatctcgttgactttcaggttactatagcagagatattactaattattatgaggacttttaaagtttccatttggaatcttgattacatcataaacctcataattaaaaatttatctaagtcactaactgagaataaatattctcaattagatgaagagcaaccaatggagattgattaaacgaacatgaaaattattcttttcttggcactgataacactcgctacttgtgagctttatcactaccaagagtgtgttagaggtacaacagtacttttaaaagaaccttgctcttctggaacatacgagggcaattcaccatttcatcctctagctgataacaaatttgcactgacttgctttagcactcaatttgcttttgcttgtcctgacggcgtaaaacacgtctatcagttacgtgccagatcagtttcacctaaactgttcatcagacaagaggaagttcaagaactttactctccaatttttcttattgttgcggcaatagtgtttataacactttgcttcacactcaaaagaaagacagaatgattgaacttgtcacgcctaaacgaacatgaaatttcttgttttcttaggaatcatcacaactgtagctgcatttcaccaagaatgtagtttacagtcatgtactcaacatcaaccatatgtagttgatgacccgtgtcctattcacttctattctaaatggtatattagagtaggagctagaaaatcagcacctttaattgaattgtgcgtggatgaggctggttctaaatcacccattcagtacatcgatatcggtaattatacagtttcctgtttaccttttacaattaattgccaggaacctaaattgggtagtcttgtagtgcgttgttcgttctatgaagactttttagagtatcatgacgttcgtgttgttttagatttcatctaaacgaacaaactaaaatgtctgataatggaccccaaaatcagcgaaatgcaccccgcattacgtttggtggaccctcagattcaactggcagtaaccagaatggagaacgcagtggggcgcgatcaaaacaacgtcggccccaaggtttacccaataatactgcgtcttggttcaccgctctcactcaacatggcaaggaagaccttaaattccctcgaggacaaggcgttccaattaacaccaatagcagtccagatgaccaaattggctactaccgaagagctaccagacgaattcgtggtggtgacggtaaaatgaaagatctcagtccaagatggtatttctactacctaggaactgggccagaagctggacttccctatggtgctaacaaagacggcatcatatgggttgcaactgagggagccttgaatacaccaaaagatcacattggcacccgcaatcctgctaacaatgctgcaatcgtgctacaacttcctcaaggaacaacattgccaaaaggcttctacgcagaagggagcagaggcggcagtcaagcctcttctcgttcctcatcacgtagtcgcaacagttcaagaaattcaactccaggcagcagtaggggaacttctcctgctagaatggctggcaatggcggtgatgctgctcttgctttgctgctgcttgacagattgaaccagcttgagagcaaaatgtctggtaaaggccaacaacaacaaggccaaactgtcactaagaaatctgctgctgaggcttctaagaagcctcggcaaaaacgtactgccactaaagcatacaatgtaacacaagctttcggcagacgtggtccagaacaaacccaaggaaattttggggaccaggaactaatcagacaaggaactgattacaaacattggccgcaaattgcacaatttgcccccagcgcttcagcgttcttcggaatgtcgcgcattggcatggaagtcacaccttcgggaacgtggttgacctacacaggtgccatcaaattggatgacaaagatccaaatttcaaagatcaagtcattttgctgaataagcatattgacgcatacaaaacattcccaccaacagagcctaaaaaggacaaaaagaagaaggctgatgaaactcaagccttaccgcagagacagaagaaacagcaaactgtgactcttcttcctgctgcagatttggatgatttctccaaacaattgcaacaatccatgagcagtgctgactcaactcaggcctaaactcatgcagaccacacaaggcagatgggctatataaacgttttcgcttttccgtttacgatatatagtctactcttgtgcagaatgaattctcgtaactacatagcacaagtagatgtagttaactttaatctcacatagcaatctttaatcagtgtgtaacattagggaggacttgaaagagccaccacattttcaccgaggccacgcggagtacgatcgagtgtacagtgaacaatgctagggagagctgcctatatggaagagccctaatgtgtaaaattaattttagtagtgctatccccatgtgattttaatagcttcttaggagaatgacaaaaaaaaaaaaaaaaaaaaaaaaa

SEQ ID NO: 22 - DNA, 29542 bp, Coronaviridae
  misc_feature 1..29542: note = SARS-CoV-2-8 nucleotide sequence
  source 1..29542: mol_type = other DNA
attaaaggtttataccttcccaggtaacaaaccaaccaactttcgatctcttgtagatctgttctctaaacgaactttaaaatctgtgtggctgtcactcggctgcatgcttagtgcactcacgcagtataattaataactaattactgtcgttgacaggacacgagtaactcgtctatcttctgcaggctgcttacggtttcgtccgtgttgcagccgatcatcagcacatctaggtttcgtccgggtgtgaccgaaaggtaagatggagagccttgtccctggtttcaacgagaaaacacacgtccaactcagtttgcctgttttacaggttcgcgacgtgctcgtacgtggctttggagactccgtggaggaggtcttatcagaggcacgtcaacatcttaaagatggcacttgtggcttagtagaagttgaaaaaggcgttttgcctcaacttgaacagccctatgtgttcatcaaacgttcggatgctcgaactgcacctcatggtcatgttatggttgagctggtagcagaactcgaaggcattcagtacggtcgtagtggtgagacacttggtgtccttgtccctcatgtgggcgaaataccagtggcttaccgcaaggttcttcttcgtaagaacggtaataaaggagctggtggccatagttacggcgccgatctaaagtcatttgacttaggcgacgagcttggcactgatccttatgaagattttcaagaaaactggaacactaaacatagcagtggtgttacccgtgaactcatgcgtgagcttaacggaggggcatacactcgctatgtcgataacaacttctgtggccctgatggctaccctcttgagtgcattaaagaccttctagcacgtgctggtaaagcttcatgcactttgtccgaacaactggactttattgacactaagaggggtgtatactgctgccgtgaacatgagcatgaaattgcttggtacacggaacgttctgaaaagagctatgaattgcagacaccttttgaaattaaattggcaaagaaatttgacaccttcaatggggaatgtccaaattttgtatttcccttaaattccataatcaagactattcaaccaagggttgaaaagaaaaagcttgatggctttatgggtagaattcgatctgtctatccagttgcgtcaccaaatgaatgcaaccaaatgtgcctttcaactctcatgaagtgtgatcattgtggtgaaacttcatggcagacgggcgattttgttaaagccacttgcgaattttgtggcactgagaatttgactaaagaaggtgccactacttgtggttacttaccccaaaatgctgttgttaaaatttattgtccagcatgtcacaattcagaagtaggacctgagcatagtcttgccgaataccataatgaatctggcttgaaaaccattcttcgtaagggtggtcgcactattgcctttggaggctgtgtgttctcttatgttggttgccataacaagtgtgcctattgggttccacgtgctagcgctaacataggttgtaaccatacaggtgttgttggagaaggttccgaaggtcttaatgacaaccttcttgaaatactccaaaaagagaaagtcaacatcaatattgttggtgactttaaacttaatgaagagatcgccattattttggcatctttttctgcttccacaagtgcttttgtggaaactgtgaaaggtttggattataaagcattcaaacaaattgttgaatcctgtggtaattttaaagttacaaaaggaaaagctaaaaaaggtgcctggaatattggtgaacagaaatcaatactgagtcctctttatgcatttgcatcagaggctgctcgtgttgtacgatcaattttctcccgcactcttgaaactgctcaaaattctgtgcgtgttttacagaaggccgctataacaatactagatggaatttcacagtattcactgagactcattgatgctatgatgttcacatctgatttggctactaacaatctagttgtaatggcctacattacaggtggtgttgttcagttgacttcgcagtggctaactaacatctttggcactgtttatgaaaaactcaaacccgtccttgattggcttgaagagaagtttaaggaaggtgtagagtttcttagagacggttgggaaattgttaaatttatctcaacctgtgcttgtgaaattgtcggtggacaaattgtcacctgtgcaaaggaaattaaggagagtgttcagacattctttaagcttgtaaataaatttttggctttgtgtgctgactctatcattattggtggagctaaacttaaagccttgaatttaggtgaaacatttgtcacgcactcaaagggattgtacagaaagtgtgttaaatccagagaagaaactggcctactcatgcctctaaaagccccaaaagaaattatcttcttagagggagaaacacttcccacagaagtgttaacagaggaagttgtcttgaaaactggtgatttacaaccattagaacaacctactagtgaagctgttgaagctccattggttggtacaccagtttgtattaacgggcttatgttgctcgaaatcaaagacacagaaaagtactgtgcccttgcacctaatatgatggtaacaaacaataccttcacactcaaaggcggtgcaccaacaaaggttacttttggtgatgacactgtgatagaagtgcaaggttacaagagtgtgaatatcacttttgaacttgatgaaaggattgataaagtacttaatgagaagtgctctgcctatacagttgaactcggtacagaagtaaatgagttcgcctgtgttgtggcagatgctgtcataaaaactttgcaaccagtatctgaattacttacaccactgggcattgatttagatgagtggagtatggctacatactacttatttgatgagtctggtgagtttaaattggcttcacatatgtattgttctttctaccctccagatgaggatgaagaagaaggtgattgtgaagaagaagagtttgagccatcaactcaatatgagtatggtactgaagatgattaccaaggtaaacctttggaatttggtgccacttctgctgctcttcaacctgaagaagagcaagaagaagattggttagatgatgatagtcaacaaactgttggtcaacaagacggcagtgaggacaatcagacaactactattcaaacaattgttgaggttcaacctcaattagagatggaacttacaccagttgttcagactattgaagtgaatagttttagtggttatttaaaacttactgacaatgtatacattaaaaatgcagacattgtggaagaagctaaaaaggtaaaaccaacagtggttgttaatgcagccaatgtttaccttaaacatggaggaggtgttgcaggagccttaaataaggctactaacaatgccatgcaagttgaatctgatgattacatagctactaatggaccacttaaagtgggtggtagttgtgttttaagcggacacaatcttgctaaacactgtcttcatgttgtcggcccaaatgttaacaaaggtgaagacattcaacttcttaagagtgcttatgaaaattttaatcagcacgaagttctacttgcaccattattatcagctggtatttttggtgctgaccctatacattctttaagagtttgtgtagatactgttcgcacaaatgtctacttagctgtctttgataaaaatctctatgacaaacttgtttcaagctttttggaaatgaagagtgaaaagcaagttgaacaaaagatcgctgagattcctaaagaggaagttaagccatttataactgaaagtaaaccttcagttgaacagagaaaacaagatgataagaaaatcaaagcttgtgttgaagaagttacaacaactctggaagaaactaagttcctcacagaaaacttgttactttatattgacattaatggcaatcttcatccagattctgccactcttgttagtgacattgacatcactttcttaaagaaagatgctccatatatagtgggtgatgttgttcaagagggtgttttaactgctgtggttatacctactaaaaaggctggtggcactactgaaatgctagcgaaagctttgagaaaagtgccaacagacaattatataaccacttacccgggtcagggtttaaatggttacactgtagaggaggcaaagacagtgcttaaaaagtgtaaaagtgccttttacattctaccatctattatctctaatgagaagcaagaaattcttggaactgtttcttggaatttgcgagaaatgcttgcacatgcagaagaaacacgcaaattaatgcctgtctgtgtggaaactaaagccatagtttcaactatacagcgtaaatataagggtattaaaatacaagagggtgtggttgattatggtgctagattttacttttacaccagtaaaacaactgtagcgtcacttatcaacacacttaacgatctaaatgaaactcttgttacaatgccacttggctatgtaacacatggcttaaatttggaagaagctgctcggtatatgagatctctcaaagtgccagctacagtttctgtttcttcacctgatgctgttacagcgtataatggttatcttacttcttcttctaaaacacctgaagaacattttattgaaaccatctcacttgctggttcctataaagattggtcctattctggacaatctacacaactaggtatagaatttcttaagagaggtgataaaagtgtatattacactagtaatcctaccacattccacctagatggtgaagttatcacctttgacaatcttaagacacttctttctttgagagaagtgaggactattaaggtgtttacaacagtagacaacattaacctccacacgcaagttgtggacatgtcaatgacatatggacaacagtttggtccaacttatttggatggagctgatgttactaaaataaaacctcataattcacatgaaggtaaaacattttatgttttacctaatgatgacactctacgtgttgaggcttttgagtactaccacacaactgatcctagttttctgggtaggtacatgtcagcattaaatcacactaaaaagtggaaatacccacaagttaatggtttaacttctattaaatgggcagataacaactgttatcttgccactgcattgttaacactccaacaaatagagttgaagtttaatccacctgctctacaagatgcttattacagagcaagggctggtgaagctgctaacttttgtgcacttatcttagcctactgtaataagacagtaggtgagttaggtgatgttagagaaacaatgagttacttgtttcaacatgccaatttagattcttgcaaaagagtcttgaacgtggtgtgtaaaacttgtggacaacagcagacaacccttaagggtgtagaagctgttatgtacatgggcacactttcttatgaacaatttaagaaaggtgttcagataccttgtacgtgtggtaaacaagctacaaaatatctagtacaacaggagtcaccttttgttatgatgtcagcaccacctgctcagtatgaacttaagcatggtacatttacttgtgctagtgagtacactggtaattaccagtgtggtcactataaacatataacttctaaagaaactttgtattgcatagacggtgctttacttacaaagtcctcagaatacaaaggtcctattacggatgttttctacaaagaaaacagttacacaacaaccataaaaccagttacttataaattggatggtgttgtttgtacagaaattgaccctaagttggacaattattataagaaagacaattcttatttcacagagcaaccaattgatcttgtaccaaaccaaccatatccaaacgcaagcttcgataattttaagtttgtatgtgataatatcaaatttgctgatgatttaaaccagttaactggttataagaaacctgcttcaagagagcttaaagttacatttttccctgacttaaatggtgatgtggtggctattgattataaacactacacaccctcttttaagaaaggagctaaattgttacataaacctattgtttggcatgttaacaatgcaactaataaagccacgtataaaccaaatacctggtgtatacgttgtctttggagcacaaaaccagttgaaacatcaaattcgtttgatgtactgaagtcagaggacgcgcagggaatggataatcttgcctgcgaagatctaaaaccagtctctgaagaagtagtggaaaatcctaccatacagaaagacgttcttgagtgtaatgtgaaaactaccgaagttgtaggagacattatacttaaaccagcaaataatagtttaaaaattacagaagaggttggccacacagatctaatggctgcttatgtagacaattctagtcttactattaagaaacctaatgaattatctagagtattaggtttgaaaacccttgctactcatggtttagctgctgttaatagtgtcccttgggatactatagctaattatgctaagccttttcttaacaaagttgttagtacaactactaacatagttacacggtgtttaaaccgtgtttgtactaattatatgccttatttctttactttattgctacaattgtgtacttttactagaagtacaaattctagaattaaagcatctatgccgactactatagcaaagaatactgttaagagtgtcggtaaattttgtctagaggcttcatttaattatttgaagtcacctaatttttctaaactgataaatattataatttggtttttactattaagtgtttgcctaggttctttaatctactcaaccgctgctttaggtgttttaatgtctaatttaggcatgccttcttactgtactggttacagagaaggctatttgaactctactaatgtcactattgcaacctactgtactggttctataccttgtagtgtttgtcttagtggtttagattctttagacacctatccttctttagaaactatacaaattaccatttcatcttttaaatgggatttaactgcttttggcttagttgcagagtggtttttggcatatattcttttcactaggtttttctatgtacttggattggctgcaatcatgcaattgtttttcagctattttgcagtacattttattagtaattcttggcttatgtggttaataattaatcttgtacaaatggccccgatttcagctatggttagaatgtacatcttctttgcatcattttattatgtatggaaaagttatgtgcatgttgtagacggttgtaattcatcaacttgtatgatgtgttacaaacgtaatagagcaacaagagtcgaatgtacaactattgttaatggtgttagaaggtccttttatgtctatgctaatggaggtaaaggcttttgcaaactacacaattggaattgtgttaattgtgatacattctgtgctggtagtacatttattagtgatgaagttgcgagagacttgtcactacagtttaaaagaccaataaatcctactgaccagtcttcttacatcgttgatagtgttacagtgaagaatggttccatccatctttactttgataaagctggtcaaaagacttatgaaagacattctctctctcattttgttaacttagacaacctgagagctaataacactaaaggttcattgcctattaatgttatagtttttgatggtaaatcaaaatgtgaagaatcatctgcaaaatcagcgtctgtttactacagtcagcttatgtgtcaacctatactgttactagatcaggcattagtgtctgatgttggtgatagtgcggaagttgcagttaaaatgtttgatgcttacgttaatacgttttcatcaacttttaacgtaccaatggaaaaactcaaaacactagttgcaactgcagaagctgaacttgcaaagaatgtgtccttagacaatgtcttatctacttttatttcagcagctcggcaagggtttgttgattcagatgtagaaactaaagatgttgttgaatgtcttaaattgtcacatcaatctgacatagaagttactggcgatagttgtaataactatatgctcacctataacaaagttgaaaacatgacaccccgtgaccttggtgcttgtattgactgtagtgcgcgtcatattaatgcgcaggtagcaaaaagtcacaacattgctttgatatggaacgttaaagatttcatgtcattgtctgaacaactacgaaaacaaatacgtagtgctgctaaaaagaataacttaccttttaagttgacatgtgcaactactagacaagttgttaatgttgtaacaacaaagatagcacttaagggtggtaaaattgttaataattggttgaagcagttaattaaagttacacttgtgttcctttttgttgctgctattttctatttaataacacctgttcatgtcatgtctaaacatactgacttttcaagtgaaatcataggatacaaggctattgatggtggtgtcactcgtgacatagcatctacagatacttgttttgctaacaaacatgctgattttgacacatggtttagccagcgtggtggtagttatactaatgacaaagcttgcccattgattgctgcagtcataacaagagaagtgggttttgtcgtgcctggtttgcctggcacgatattacgcacaactaatggtgactttttgcatttcttacctagagtttttagtgcagttggtaacatctgttacacaccatcaaaacttatagagtacactgactttgcaacatcagcttgtgttttggctgctgaatgtacaatttttaaagatgcttctggtaagccagtaccatattgttatgataccaatgtactagaaggttctgttgcttatgaaagtttacgccctgacacacgttatgtgctcatggatggctctattattcaatttcctaacacctaccttgaaggttctgttagagtggtaacaacttttgattctgagtactgtaggcacggcacttgtgaaagatcagaagctggtgtttgtgtatctactagtggtagatgggtacttaacaatgattattacagatctttaccaggagttttctgtggtgtagatgctgtaaatttacttactaatatgtttacaccactaattcaacctattggtgctttggacatatcagcatctatagtagctggtggtattgtagctatcgtagtaacatgccttgcctactattttatgaggtttagaagagcttttggtgaatacagtcatgtagttgcctttaatactttactattccttatgtcattcactgtactctgtttaacaccagtttactcattcttacctggtgtttattctgttatttacttgtacttgacattttatcttactaatgatgtttcttttttagcacatattcagtggatggttatgttcacacctttagtacctttctggataacaattgcttatatcatttgtatttccacaaagcatttctattggttctttagtaattacctaaagagacgtgtagtctttaatggtgtttcctttagtacttttgaagaagctgcgctgtgcacctttttgttaaataaagaaatgtatctaaagttgcgtagtgatgtgctattacctcttacgcaatataatagatacttagctctttataataagtacaagtattttagtggagcaatggatacaactagctacagagaagctgcttgttgtcatctcgcaaaggctctcaatgacttcagtaactcaggttctgatgttctttaccaaccaccacaaacctctatcacctcagctgttttgcagagtggttttagaaaaatggcattcccatctggtaaagttgagggttgtatggtacaagtaacttgtggtacaactacacttaacggtctttggcttgatgacgtagtttactgtccaagacatgtgatctgcacctctgaagacatgcttaaccctaattatgaagatttactcattcgtaagtctaatcataatttcttggtacaggctggtaatgttcaactcagggttattggacattctatgcaaaattgtgtacttaagcttaaggttgatacagccaatcctaagacacctaagtataagtttgttcgcattcaaccaggacagactttttcagtgttagcttgttacaatggttcaccatctggtgtttaccaatgtgctatgaggcccaatttcactattaagggttcattccttaatggttcatgtggtagtgttggttttaacatagattatgactgtgtctctttttgttacatgcaccatatggaattaccaactggagttcatgctggcacagacttagaaggtaacttttatggaccttttgttgacaggcaaacagcacaagcagctggtacggacacaactattacagttaatgttttagcttggttgtacgctgctgttataaatggagacaggtggtttctcaatcgatttaccacaactcttaatgactttaaccttgtggctatgaagtacaattatgaacctctaacacaagaccatgttgacatactaggacctctttctgctcaaactggaattgccgttttagatatgtgtgcttcattaaaagaattactgcaaaatggtatgaatggacgtaccatattgggtagtgctttattagaagatgaatttacaccttttgatgttgttagacaatgctcaggtgttactttccaaagtgcagtgaaaagaacaatcaagggtacacaccactggttgttactcacaattttgacttcacttttagttttagtccagagtactcaatggtctttgttcttttttttgtatgaaaatgcctttttaccttttgctatgggtattattgctatgtctgcttttgcaatgatgtttgtcaaacataagcatgcatttctctgtttgtttttgttaccttctcttgccactgtagcttattttaatatggtctatatgcctgctagttgggtgatgcgtattatgacatggttggatatggttgatactagtttgtctggttttaagctaaaagactgtgttatgtatgcatcagctgtagtgttactaatccttatgacagcaagaactgtgtatgatgatggtgctaggagagtgtggacacttatgaatgtcttgacactcgtttataaagtttattatggtaatgctttagatcaagccatttccatgtgggctcttataatctctgttacttctaactactcaggtgtagttacaactgtcatgtttttggccagaggtattgtttttatgtgtgttgagtattgccctattttcttcataactggtaatacacttcagtgtataatgctagtttattgtttcttaggctatttttgtacttgttactttggcctcttttgtttactcaaccgctactttagactgactcttggtgtttatgattacttagtttctacacaggagtttagatatatgaattcacagggactactcccacccaagaatagcatagatgccttcaaactcaacattaaattgttgggtgttggtggcaaaccttgtatcaaagtagccactgtacagtctaaaatgtcagatgtaaagtgcacatcagtagtcttactctcagttttgcaacaactcagagtagaatcatcatctaaattgtgggctcaatgtgtccagttacacaatgacattctcttagctaaagatactactgaagcctttgaaaaaatggtttcactactttctgttttgctttccatgcagggtgctgtagacataaacaagctttgtgaagaaatgctggacaacagggcaaccttacaagctatagcctcagagtttagttcccttccatcatatgcagcttttgctactgctcaagaagcttatgagcaggctgttgctaatggtgattctgaagttgttcttaaaaagttgaagaagtctttgaatgtggctaaatctgaatttgaccgtgatgcagccatgcaacgtaagttggaaaagatggctgatcaagctatgacccaaatgtataaacaggctagatctgaggacaagagggcaaaagttactagtgctatgcagacaatgcttttcactatgcttagaaagttggataatgatgcactcaacaacattatcaacaatgcaagagatggttgtgttcccttgaacataatacctcttacaacagcagccaaactaatggttgtcataccagactataacacatataaaaatacgtgtgatggtacaacatttacttatgcatcagcattgtgggaaatccaacaggttgtagatgcagatagtaaaattgttcaacttagtgaaattagtatggacaattcacctaatttagcatggcctcttattgtaacagctttaagggccaattctgctgtcaaattacagaataatgagcttagtcctgttgcactacgacagatgtcttgtgctgccggtactacacaaactgcttgcactgatgacaatgcgttagcttactacaacacaacaaagggaggtaggtttgtacttgcactgttatccgatttacaggatttgaaatgggctagattccctaagagtgatggaactggtactatctatacagaactggaaccaccttgtaggtttgttacagacacacctaaaggtcctaaagtgaagtatttatactttattaaaggattaaacaacctaaatagaggtatggtacttggtagtttagctgccacagtacgtctacaagctggtaatgcaacagaagtgcctgccaattcaactgtattatctttctgtgcttttgctgtagatgctgctaaagcttacaaagattatctagctagtgggggacaaccaatcactaattgtgttaagatgttgtgtacacacactggtactggtcaggcaataacagttacaccggaagccaatatggatcaagaatcctttggtggtgcatcgtgttgtctgtactgccgttgccacatagatcatccaaatcctaaaggattttgtgacttaaaaggtaagtatgtacaaatacctacaacttgtgctaatgaccctgtgggttttacacttaaaaacacagtctgtaccgtctgcggtatgtggaaaggttatggctgtagttgtgatcaactccgcgaacccatgcttcagtcagctgatgcacaatcgtttttaaacgggtttgcggtgtaagtgcagcccgtcttacaccgtgcggcacaggcactagtactgatgtcgtatacagggcttttgacatctacaatgataaagtagctggttttgctaaattcctaaaaactaattgttgtcgcttccaagaaaaggacgaagatgacaatttaattgattcttactttgtagttaagagacacactttctctaactaccaacatgaagaaacaatttataatttacttaaggattgtccagctgttgctaaacatgacttctttaagtttagaatagacggtgacatggtaccacatatatcacgtcaacgtcttactaaatacacaatggcagacctcgtctatgctttaaggcattttgatgaaggtaattgtgacacattaaaagaaatacttgtcacatacaattgttgtgatgatgattatttcaataaaaaggactggtatgattttgtagaaaacccagatatattacgcgtatacgccaacttaggtgaacgtgtacgccaagctttgttaaaaacagtacaattctgtgatgccatgcgaaatgctggtattgttggtgtactgacattagataatcaagatctcaatggtaactggtatgatttcggtgatttcatacaaaccacgccaggtagtggagttcctgttgtagattcttattattcattgttaatgcctatattaaccttgaccagggctttaactgcagagtcacatgttgacactgacttaacaaagccttacattaagtgggatttgttaaaatatgacttcacggaagagaggttaaaactctttgaccgttattttaaatattgggatcagacataccacccaaattgtgttaactgtttggatgacagatgcattctgcattgtgcaaactttaatgttttattctctacagtgttcccacctacaagttttggaccactagtgagaaaaatatttgttgatggtgttccatttgtagtttcaactggataccacttcagagagctaggtgttgtacataatcaggatgtaaacttacatagctctagacttagttttaaggaattacttgtgtatgctgctgaccctgctatgcacgctgcttctggtaatctattactagataaacgcactacgtgcttttcagtagctgcacttactaacaatgttgcttttcaaactgtcaaacccggtaattttaacaaagacttctatgactttgctgtgtctaagggtttctttaaggaaggaagttctgttgaattaaaacacttcttctttgctcaggatggtaatgctgctatcagcgattatgactactatcgttataatctaccaacaatgtgtgatatcagacaactactatttgtagttgaagttgttgataagtactttgattgttacgatggtggctgtattaatgctaaccaagtcatcgtcaacaacctagacaaatcagctggttttccatttaataaatggggtaaggctagactttattatgattcaatgagttatgaggatcaagatgcacttttcgcatatacaaaacgtaatgtcatccctactataactcaaatgaatcttaagtatgccattagtgcaaagaatagagctcgcaccgtagctggtgtctctatctgtagtactatgaccaatagacagtttcatcaaaaattattgaaatcaatagccgccactagaggagctactgtagtaattggaacaagcaaattctatggtggttggcacaacatgttaaaaactgtttatagtgatgtagaaaaccctcaccttatgggttgggattatcctaaatgtgatagagccatgcctaacatgcttagaattatggcctcacttgttcttgctcgcaaacatacaacgtgttgtagcttgtcacaccgtttctatagattagctaatgagtgtgctcaagtattgagtgaaatggtcatgtgtggcggttcactatatgttaaaccaggtggaacctcatcaggagatgccacaactgcttatgctaatagtgtttttaacatttgtcaagctgtcacggccaatgttaatgcacttttatctactgatggtaacaaaattgccgataagtatgtccgcaatttacaacacagactttatgagtgtctctatagaaatagagatgttgacacagactttgtgaatgagttttacgcatatttgcgtaaacatttctcaatgatgatactctctgacgatgctgttgtgtgtttcaatagcacttatgcatctcaaggtctagtggctagcataaagaactttaagtcagttctttattatcaaaacaatgtttttatgtctgaagcaaaatgttggactgagactgaccttactaaaggacctcatgaattttgctctcaacatacaatgctagttaaacagggtgatgattatgtgtaccttccttacccagatccatcaagaatcctaggggccggctgttttgtagatgatatcgtaaaaacagatggtacacttatgattgaacggttcgtgtctttagctatagatgcttacccacttactaaacatcctaatcaggagtatgctgatgtctttcatttgtacttacaatacataagaaagctacatgatgagttaacaggacacatgttagacatgtattctgttatgcttactaatgataacacttcaaggtattgggaacctgagttttatgaggctatgtacacaccgcatacagtcttacaggctgttggggcttgtgttctttgcaattcacagacttcattaagatgtggtgcttgcatacgtagaccattcttatgttgtaaatgctgttacgaccatgtcatatcaacatcacataaattagtcttgtctgttaatccgtatgtttgcaatgctccaggttgtgatgtcacagatgtgactcaactttacttaggaggtatgagctattattgtaaatcacataaaccacccattagttttccattgtgtgctaatggacaagtttttggtttatataaaaatacatgtgttggtagcgataatgttactgactttaatgcaattgcaacatgtgactggacaaatgctggtgattacattttagctaacacctgtactgaaagactcaagctttttgcagcagaaacgctcaaagctactgaggagacatttaaactgtcttatggtattgctactgtacgtgaagtgctgtctgacagagaattacatctttcatgggaagttggtaaacctagaccaccacttaaccgaaattatgtctttactggttatcgtgtaactaaaaacagtaaagtacaaataggagagtacacctttgaaaaaggtgactatggtgatgctgttgtttaccgaggtacaacaacttacaaattaaatgttggtgattattttgtgctgacatcacatacagtaatgccattaagtgcacctacactagtgccacaagagcactatgttagaattactggcttatacccaacactcaatatctcagatgagttttctagcaatgttgcaaattatcaaaaggttggtatgcaaaagtattctacactccagggaccacctggtactggtaagagtcattttgctattggcctagctctctactacccttctgctcgcatagtgtatacagcttgctctcatgccgctgttgatgcactatgtgagaaggcattaaaatatttgcctatagataaatgtagtagaattatacctgcacgtgctcgtgtagagtgttttgataaattcaaagtgaattcaacattagaacagtatgtcttttgtactgtaaatgcattgcctgagacgacagcagatatagttgtctttgatgaaatttcaatggccacaaattatgatttgagtgttgtcaatgccagattacgtgctaagcactatgtgtacattggcgaccctgctcaattacctgcaccacgcacattgctaactaagggcacactagaaccagaatatttcaattcagtgtgtagacttatgaaaactataggtccagacatgttcctcggaacttgtcggcgttgtcctgctgaaattgttgacactgtgagtgctttggtttatgataataagcttaaagcacataaagacaaatcagctcaatgctttaaaatgttttataagggtgttatcacgcatgatgtttcatctgcaattaacaggccacaaataggcgtggtaagagaattccttacacgtaaccctgcttggagaaaagctgtctttatttcaccttataattcacagaatgctgtagcctcaaagattttgggactaccaactcaaactgttgattcatcacagggctcagaatatgactatgtcatattcactcaaaccactgaaacagctcactcttgtaatgtaaacagatttaatgttgctattaccagagcaaaagtaggcatactttgcataatgtctgatagagacctttatgacaagttgcaatttacaagtcttgaaattccacgtaggaatgtggcaactttacaagctgaaaatgtaacaggactctttaaagattgtagtaaggtaatcactgggttacatcctacacaggcacctacacacctcagtgttgacactaaattcaaaactgaaggtttatgtgttgacatacctggcatacctaaggacatgacctatagaagactcatctctatgatgggttttaaaatgaattatcaagttaatggttaccctaacatgtttatcacccgcgaagaagctataagacatgtacgtgcatggattggcttcgatgtcgaggggtgtcatgctactagagaagctgttggtaccaatttacctttacagctaggtttttctacaggtgttaacctagttgctgtacctacaggttatgttgatacacctaataatacagatttttccagagttagtgctaaaccaccgcctggagatcaatttaaacacctcataccacttatgtacaaaggacttccttggaatgtagtgcgtataaagattgtacaaatgttaagtgacacacttaaaaatctctctgacagagtcgtatttgtcttatgggcacatggctttgagttgacatctatgaagtattttgtgaaaataggacctgagcgcacctgttgtctatgtgatagacgtgccacatgcttttccactgcttcagacacttatgcctgttggcatcattctattggatttgattacgtctataatccgtttatgattgatgttcaacaatggggttttacaggtaacctacaaagcaaccatgatctgtattgtcaagtccatggtaatgcacatgtagctagttgtgatgcaatcatgactaggtgtctagctgtccacgagtgctttgttaagcgtgttgactggactattgaatatcctataattggtgatgaactgaagattaatgcggcttgtagaaaggttcaacacatggttgttaaagctgcattattagcagacaaattcccagttcttcacgacattggtaaccctaaagctattaagtgtgtacctcaagctgatgtagaatggaagttctatgatgcacagccttgtagtgacaaagcttataaaatagaagaattattctattcttatgccacacattctgacaaattcacagatggtgtatgcctattttggaattgcaatgtcgatagatatcctgctaattccattgtttgtagatttgacactagagtgctatctaaccttaacttgcctggttgtgatggtggcagtttgtatgtaaataaacatgcattccacacaccagcttttgataaaagtgcttttgttaatttaaaacaattaccatttttctattactctgacagtccatgtgagtctcatggaaaacaagtagtgtcagatatagattatgtaccactaaagtctgctacgtgtataacacgttgcaatttaggtggtgctgtctgtagacatcatgctaatgagtacagattgtatctcgatgcttataacatgatgatctcagctggctttagcttgtgggtttacaaacaatttgatacttataacctctggaacacttttacaagacttcagagtttagaaaatgtggcttttaatgttgtaaataagggacactttgatggacaacagggtgaagtaccagtttctatcattaataacactgtttacacaaaagttgatggtgttgatgtagaattgtttgaaaataaaacaacattacctgttaatgtagcatttgagctttgggctaagcgcaacattaaaccagtaccagaggtgaaaatactcaataatttgggtgtggacattgctgctaatactgtgatctgggactacaaaagagatgctccagcacatatatctactattggtgtttgttctatgactgacatagccaagaaaccaactgaaacgatttgtgcaccactcactgtcttttttgatggtagagttgatggtcaagtagacttatttagaaatgcccgtaatggtgttcttattacagaaggtagtgttaaaggtttacaaccatctgtgggtcccaaacaagctagtcttaatggagtcacattaattggagaagccgtaaaaacacagttcaattattataagaaagttgatggtgttgtccaacaattacctgaaacttactttactcagagtagaaatttacaagaatttaaacccaggagtcaaatggaaattgatttcttagaattagctatggatgaattcattgaacggtataaattagaaggctatgccttcgaacatatcgtttatggagattttagtcatagtcagttaggtggtttacatctactgattggactagctaaacgttttaaggaatcaccttttgaattagaagattttattcctatggacagtacagttaaaaactatttcataacagatgcgcaaacaggttcatctaagtgtgtgtgttctgttattgatttattacttgatgattttgttgaaataataaaatcccaagatttatctgtagtttctaaggttgtcaaagtgactattgactatacagaaatttcatttatgctttggtgtaaagatggccatgtagaaacattttacccaaaattacaatctagtcaagcgtggcaaccgggtgttgctatgcctaatctttacaaaatgcaaagaatgctattagaaaagtgtgaccttcaaaattatggtgatagtgcaacattacctaaaggcataatgatgaatgtcgcaaaatatactcaactgtgtcaatatttaaacacattaacattagctgtaccctataatatgagagttatacattttggtgctggttctgataaaggagttgcaccaggtacagctgttttaagacagtggttgcctacgggtacgctgcttgtcgattcagatcttaatgactttgtctctgatgcagattcaactttgattggtgattgtgcaactgtacatacagctaataaatgggatctcattattagtgatatgtacgaccctaagactaaaaatgttacaaaagaaaatgactctaaagagggttttttcacttacatttgtgggtttatacaacaaaagctagctcttggaggttccgtggctataaagataacagaacattcttggaatgctgatctttataagctcatgggacacttcgcatggtggacagcctttgttactaatgtgaatgcgtcatcatctgaagcatttttaattggatgtaattatcttggcaaaccacgcgaacaaatagatggttatgtcatgcatgcaaattacatattttggaggaatacaaatccaattcagttgtcttcctattctttatttgacatgagtaaatttccccttaaattaaggggtactgctgttatgtctttaaaagaaggtcaaatcaatgatatgattttatctcttcttagtaaaggtagacttataattagagaaaacaacagagttgttatttctagtgatgttcttgttaacaactaaacgaacaatgtttgtttttcttgttttattgccactagtctctagtcagtgtgttaatcttacaaccagaactcaattaccccctgcatacactaattctttcacacgtggtgtttattaccctgacaaagttttcagatcctcagttttacattcaactcaggacttgttcttacctttcttttccaatgttacttggttccatgctatacatgtctctgggaccaatggtactaagaggtttgataaccctgtcctaccatttaatgatggtgtttattttgcttccactgagaagtctaacataataagaggctggatttttggtactactttagattcgaagacccagtccctacttattgttaataacgctactaatgttgttattaaagtctgtgaatttcaattttgtaatgatccatttttgggtgtttattaccacaaaaacaacaaaagttggatggaaagtgagttcagagtttattctagtgcgaataattgcacttttgaatatgtctctcagccttttcttatggaccttgaaggaaaacagggtaatttcaaaaatcttagggaatttgtgtttaagaatattgatggttattttaaaatatattctaagcacacgcctattaatttagtgcgtgatctccctcagggtttttcggctttagaaccattggtagatttgccaataggtattaacatcactaggtttcaaactttacttgctttacatagaagttatttgactcctggtgattcttcttcaggttggacagctggtgctgcagcttattatgtgggttatcttcaacctaggacttttctattaaaatataatgaaaatggaaccattacagatgctgtagactgtgcacttgaccctctctcagaaacaaagtgtacgttgaaatccttcactgtagaaaaaggaatctatcaaacttctaactttagagtccaaccaacagaatctattgttagatttcctaatattacaaacttgtgcccttttggtgaagtttttaacgccaccagatttgcatctgtttatgcttggaacaggaagagaatcagcaactgtgttgctgattattctgtcctatataattccgcatcattttccacttttaagtgttatggagtgtctcctactaaattaaatgatctctgctttactaatgtctatgcagattcatttgtaattagaggtgatgaagtcagacaaatcgctccagggcaaactggaaagattgctgattataattataaattaccagatgattttacaggctgcgttatagcttggaattctaacaatcttgattctaaggttggtggtaattataattacctgtatagattgtttaggaagtctaatctcaaaccttttgagagagatatttcaactgaaatctatcaggccggtagcacaccttgtaatggtgttgaaggttttaattgttactttcctttacaatcatatggtttccaacccactaatggtgttggttaccaaccatacagagtagtagtactttcttttgaacttctacatgcaccagcaactgtttgtggacctaaaaagtctactaatttggttaaaaacaaatgtgtcaatttcaacttcaatggtttaacaggcacaggtgttcttactgagtctaacaaaaagtttctgcctttccaacaatttggcagagacattgctgacactactgatgctgtccgtgatccacagacacttgagattcttgacattacaccatgttcttttggtggtgtcagtgttataacaccaggaacaaatacttctaaccaggttgctgttctttatcaggatgttaactgcacagaagtccctgttgctattcatgcagatcaacttactcctacttggcgtgtttattctacaggttctaatgtttttcaaacacgtgcaggctgtttaataggggctgaacatgtcaacaactcatatgagtgtgacatacccattggtgcaggtatatgcgctagttatcagactcagactaattctcctcggcgggcacgtagtgtagctagtcaatccatcattgcctacactatgtcacttggtgcagaaaattcagttgcttactctaataactctattgccatacccacaaattttactattagtgttaccacagaaattctaccagtgtctatgaccaagacatcagtagattgtacaatgtacatttgtggtgattcaactgaatgcagcaatcttttgttgcaatatggcagtttttgtacacaattaaaccgtgctttaactggaatagctgttgaacaagacaaaaacacccaagaagtttttgcacaagtcaaacaaatttacaaaacaccaccaattaaagattttggtggttttaatttttcacaaatattaccagatccatcaaaaccaagcaagaggtcatttattgaagatctacttttcaacaaagtgacacttgcagatgctggcttcatcaaacaatatggtgattgccttggtgatattgctgctagagacctcatttgtgcacaaaagtttaacggccttactgttttgccacctttgctcacagatgaaatgattgctcaatacacttctgcactgttagcgggtacaatcacttctggttggacctttggtgcaggtgctgcattacaaataccatttgctatgcaaatggcttataggtttaatggtattggagttacacagaatgttctctatgagaaccaaaaattgattgccaaccaatttaatagtgctattggcaaaattcaagactcactttcttccacagcaagtgcacttggaaaacttcaagatgtggtcaaccaaaatgcacaagctttaaacacgcttgttaaacaacttagctccaattttggtgcaatttcaagtgttttaaatgatatcctttcacgtcttgacaaagttgaggctgaagtgcaaattgataggttgatcacaggcagacttcaaagtttgcagacatatgtgactcaacaattaattagagctgcagaaatcagagcttctgctaatcttgctgctactaaaatgtcagagtgtgtacttggacaatcaaaaagagttgatttttgtggaaagggctatcatcttatgtccttccctcagtcagcacctcatggtgtagtcttcttgcatgtgacttatgtccctgcacaagaaaagaacttcacaactgctcctgccatttgtcatgatggaaaagcacactttcctcgtgaaggtgtctttgtttcaaatggcacacactggtttgtaacacaaaggaatttttatgaaccacaaatcattactacagacaacacatttgtgtctggtaactgtgatgttgtaataggaattgtcaacaacacagtttatgatcctttgcaacctgaattagactcattcaaggaggagttagataaatattttaagaatcatacatcaccagatgttgatttaggtgacatctctggcattaatgcttcagttgtaaacattcaaaaagaaattgaccgcctcaatgaggttgccaagaatttaaatgaatctctcatcgatctccaagaacttggaaagtatgagcagtatataaaatggccatggtacatttggctaggttttatagctggcttgattgccatagtaatggtgacaattatgctttgctgtatgaccagttgctgtagttgtctcaagggctgttgttcttgtggatcctgctgcaaatttgatgaagacgactctgagccagtgctcaaaggagtcaaattacattacacataaacgaacttatggatttgtttatgagaatcttcacaattggaactgtaactttgaagcaaggtgaaatcaaggatgctactccttcagattttgttcgcgctactgcaacgataccgatacaagcctcactccctttcggatggcttattgttggcgttgcacttcttgctgtttttcagagcgcttccaaaatcataaccctcaaaaagagatggcaactagcactctccaagggtgttcactttgtttgcaacttgctgttgttgtttgtaacagtttactcacaccttttgctcgttgctgctggccttgaagccccttttctctatctttatgctttagtctacttcttgcagagtataaactttgtaagaataataatgaggctttggctttgctggaaatgccgttccaaaaacccattactttatgatgccaactattttctttgctggcatactaattgttacgactattgtataccttacaatagtgtaacttcttcaattgtcattacttcaggtgatggcacaacaagtcctatttctgaacatgactaccagattggtggttatactgaaaaatgggaatctggagtaaaagactgtgttgtattacacagttacttcacttcagactattaccagctgtactcaactcaattgagtacagacactggtgttgaacatgttaccttcttcatctacaataaaattgttgatgagcctgaagaacatgtccaaattcacacaatcgacggttcatccggagttgttaatccagtaatggaaccaatttatgatgaaccgacgacgactactagcgtgcctttgtaagcacaagctgatgagtacgaacttatgtactcattcgtttcggaagagacaggtacgttaatagttaatagcgtacttctttttcttgctttcgtggtattcttgctagttacactagccatccttactgcgcttcgattgtgtgcgtactgctgcaatattgttaacgtgagtcttgtaaaaccttctttttacgtttactctcgtgttaaaaatctgaattcttctagagttcctgatcttctggtctaaacgaactaaatattatattagtttttctgtttggaactttaattttagccatggcagattccaacggtactattaccgttgaagagcttaaaaagctccttgaacaatggaacctagtaataggtttcctattccttacatggatttgtcttctacaatttgcctatgccaacaggaataggtttttgtatataattaagttaattttcctctggctgttatggccagtaactttagcttgttttgtgcttgctgctgtttacagaataaattggatcaccggtggaattgctatcgcaatggcttgtcttgtaggcttgatgtggctcagctacttcattgcttctttcagactgtttgcgcgtacccgttccatgtggtcattcaatccagaaactaacattcttctcaacgtgccactccatggcactattctgaccagaccgcttctagaaagtgaactcgtaatcggagctgtgatccttcgtggacatcttcgtattgctggacaccatctaggacgctgtgacatcaaggacctgcctaaagaaatcactgttgctacatcacgaacgctttcttattacaaattgggagcttcgcagcgtgtagcaggtgactcaggttttgctgcatacagtcgctacaggattggcaactataaattaaacacagaccattccagtagcagtgacaatattgctttgcttgtacagtaagtgacaacagatgtttcatctcgttgactttcaggttactatagcagagatattactaattattatgaggacttttaaagtttccatttggaatcttgattacatcataaacctcataattaaaaatttatctaagtcactaactgagaataaatattctcaattagatgaagagcaaccaatggagattgattaaacgaacatgaaaattattcttttcttggcactgataacactcgctacttgtgagctttatcactaccaagagtgtgttagaggtacaacagtacttttaaaagaaccttgctcttctggaacatacgagggcaattcaccatttcatcctctagctgataacaaatttgcactgacttgctttagcactcaatttgcttttgcttgtcctgacggcgtaaaacacgtctatcagttacgtgccagatcagtttcacctaaactgttcatcagacaagaggaagttcaagaactttactctccaatttttcttattgttgcggcaatagtgtttataacactttgcttcacactcaaaagaaagacagaatgattgaactttcattaattgacttctatttgtgctttttagcctttctgctattccttgttttaattatgcttattatcttttggttctcacttgaactgcaagatcataatgaaacttgtcacgcctaatgttttagatttcatctaaacgaacaaactaaaatgtctgataatggaccccaaaatcagcgaaatgcaccccgcattacgtttggtggaccctcagattcaactggcagtaaccagaatggagaacgcagtggggcgcgatcaaaacaacgtcggccccaaggtttacccaataatactgcgtcttggttcaccgctctcactcaacatggcaaggaagaccttaaattccctcgaggacaaggcgttccaattaacaccaatagcagtccagatgaccaaattggctactaccgaagagctaccagacgaattcgtggtggtgacggtaaaatgaaagatctcagtccaagatggtatttctactacctaggaactgggccagaagctggacttccctatggtgctaacaaagacggcatcatatgggttgcaactgagggagccttgaatacaccaaaagatcacattggcacccgcaatcctgctaacaatgctgcaatcgtgctacaacttcctcaaggaacaacattgccaaaaggcttctacgcagaagggagcagaggcggcagtcaagcctcttctcgttcctcatcacgtagtcgcaacagttcaagaaattcaactccaggcagcagtaggggaacttctcctgctagaatggctggcaatggcggtgatgctgctcttgctttgctgctgcttgacagattgaaccagcttgagagcaaaatgtctggtaaaggccaacaacaacaaggccaaactgtcactaagaaatctgctgctgaggcttctaagaagcctcggcaaaaacgtactgccactaaagcatacaatgtaacacaagctttcggcagacgtggtccagaacaaacccaaggaaattttggggaccaggaactaatcagacaaggaactgattacaaacattggccgcaaattgcacaatttgcccccagcgcttcagcgttcttcggaatgtcgcgcattggcatggaagtcacaccttcgggaacgtggttgacctacacaggtgccatcaaattggatgacaaagatccaaatttcaaagatcaagtcattttgctgaataagcatattgacgcatacaaaacattcccaccaacagagcctaaaaaggacaaaaagaagaaggctgatgaaactcaagccttaccgcagagacagaagaaacagcaaactgtgactcttcttcctgctgcagatttggatgatttctccaaacaattgcaacaatccatgagcagtgctgactcaactcaggcctaaactcatgcagaccacacaaggcagatgggctatataaacgttttcgcttttccgtttacgatatatagtctactcttgtgcagaatgaattctcgtaactacatagcacaagtagatgtagttaactttaatctcacatagcaatctttaatcagtgtgtaacattagggaggacttgaaagagccaccacattttcaccgaggccacgcggagtacgatcgagtgtacagtgaacaatgctagggagagctgcctatatggaagagccctaatgtgtaaaattaattttagtagtgctatccccatgtgattttaatagcttcttaggagaatgacaaaaaaaaaaaaaaaaaaaaaaaaa

SEQ ID NO: 23 - DNA, 29376 bp, Coronaviridae
  misc_feature 1..29376: note = SARS-CoV-2-[6,8] nucleotide sequence, it contains two punctual substitutions (c.27041A-C and c.27044A-C)
  source 1..29376: mol_type = other DNA
attaaaggtttataccttcccaggtaacaaaccaaccaactttcgatctcttgtagatctgttctctaaacgaactttaaaatctgtgtggctgtcactcggctgcatgcttagtgcactcacgcagtataattaataactaattactgtcgttgacaggacacgagtaactcgtctatcttctgcaggctgcttacggtttcgtccgtgttgcagccgatcatcagcacatctaggtttcgtccgggtgtgaccgaaaggtaagatggagagccttgtccctggtttcaacgagaaaacacacgtccaactcagtttgcctgttttacaggttcgcgacgtgctcgtacgtggctttggagactccgtggaggaggtcttatcagaggcacgtcaacatcttaaagatggcacttgtggcttagtagaagttgaaaaaggcgttttgcctcaacttgaacagccctatgtgttcatcaaacgttcggatgctcgaactgcacctcatggtcatgttatggttgagctggtagcagaactcgaaggcattcagtacggtcgtagtggtgagacacttggtgtccttgtccctcatgtgggcgaaataccagtggcttaccgcaaggttcttcttcgtaagaacggtaataaaggagctggtggccatagttacggcgccgatctaaagtcatttgacttaggcgacgagcttggcactgatccttatgaagattttcaagaaaactggaacactaaacatagcagtggtgttacccgtgaactcatgcgtgagcttaacggaggggcatacactcgctatgtcgataacaacttctgtggccctgatggctaccctcttgagtgcattaaagaccttctagcacgtgctggtaaagcttcatgcactttgtccgaacaactggactttattgacactaagaggggtgtatactgctgccgtgaacatgagcatgaaattgcttggtacacggaacgttctgaaaagagctatgaattgcagacaccttttgaaattaaattggcaaagaaatttgacaccttcaatggggaatgtccaaattttgtatttcccttaaattccataatcaagactattcaaccaagggttgaaaagaaaaagcttgatggctttatgggtagaattcgatctgtctatccagttgcgtcaccaaatgaatgcaaccaaatgtgcctttcaactctcatgaagtgtgatcattgtggtgaaacttcatggcagacgggcgattttgttaaagccacttgcgaattttgtggcactgagaatttgactaaagaaggtgccactacttgtggttacttaccccaaaatgctgttgttaaaatttattgtccagcatgtcacaattcagaagtaggacctgagcatagtcttgccgaataccataatgaatctggcttgaaaaccattcttcgtaagggtggtcgcactattgcctttggaggctgtgtgttctcttatgttggttgccataacaagtgtgcctattgggttccacgtgctagcgctaacataggttgtaaccatacaggtgttgttggagaaggttccgaaggtcttaatgacaaccttcttgaaatactccaaaaagagaaagtcaacatcaatattgttggtgactttaaacttaatgaagagatcgccattattttggcatctttttctgcttccacaagtgcttttgtggaaactgtgaaaggtttggattataaagcattcaaacaaattgttgaatcctgtggtaattttaaagttacaaaaggaaaagctaaaaaaggtgcctggaatattggtgaacagaaatcaatactgagtcctctttatgcatttgcatcagaggctgctcgtgttgtacgatcaattttctcccgcactcttgaaactgctcaaaattctgtgcgtgttttacagaaggccgctataacaatactagatggaatttcacagtattcactgagactcattgatgctatgatgttcacatctgatttggctactaacaatctagttgtaatggcctacattacaggtggtgttgttcagttgacttcgcagtggctaactaacatctttggcactgtttatgaaaaactcaaacccgtccttgattggcttgaagagaagtttaaggaaggtgtagagtttcttagagacggttgggaaattgttaaatttatctcaacctgtgcttgtgaaattgtcggtggacaaattgtcacctgtgcaaaggaaattaaggagagtgttcagacattctttaagcttgtaaataaatttttggctttgtgtgctgactctatcattattggtggagctaaacttaaagccttgaatttaggtgaaacatttgtcacgcactcaaagggattgtacagaaagtgtgttaaatccagagaagaaactggcctactcatgcctctaaaagccccaaaagaaattatcttcttagagggagaaacacttcccacagaagtgttaacagaggaagttgtcttgaaaactggtgatttacaaccattagaacaacctactagtgaagctgttgaagctccattggttggtacaccagtttgtattaacgggcttatgttgctcgaaatcaaagacacagaaaagtactgtgcccttgcacctaatatgatggtaacaaacaataccttcacactcaaaggcggtgcaccaacaaaggttacttttggtgatgacactgtgatagaagtgcaaggttacaagagtgtgaatatcacttttgaacttgatgaaaggattgataaagtacttaatgagaagtgctctgcctatacagttgaactcggtacagaagtaaatgagttcgcctgtgttgtggcagatgctgtcataaaaactttgcaaccagtatctgaattacttacaccactgggcattgatttagatgagtggagtatggctacatactacttatttgatgagtctggtgagtttaaattggcttcacatatgtattgttctttctaccctccagatgaggatgaagaagaaggtgattgtgaagaagaagagtttgagccatcaactcaatatgagtatggtactgaagatgattaccaaggtaaacctttggaatttggtgccacttctgctgctcttcaacctgaagaagagcaagaagaagattggttagatgatgatagtcaacaaactgttggtcaacaagacggcagtgaggacaatcagacaactactattcaaacaattgttgaggttcaacctcaattagagatggaacttacaccagttgttcagactattgaagtgaatagttttagtggttatttaaaacttactgacaatgtatacattaaaaatgcagacattgtggaagaagctaaaaaggtaaaaccaacagtggttgttaatgcagccaatgtttaccttaaacatggaggaggtgttgcaggagccttaaataaggctactaacaatgccatgcaagttgaatctgatgattacatagctactaatggaccacttaaagtgggtggtagttgtgttttaagcggacacaatcttgctaaacactgtcttcatgttgtcggcccaaatgttaacaaaggtgaagacattcaacttcttaagagtgcttatgaaaattttaatcagcacgaagttctacttgcaccattattatcagctggtatttttggtgctgaccctatacattctttaagagtttgtgtagatactgttcgcacaaatgtctacttagctgtctttgataaaaatctctatgacaaacttgtttcaagctttttggaaatgaagagtgaaaagcaagttgaacaaaagatcgctgagattcctaaagaggaagttaagccatttataactgaaagtaaaccttcagttgaacagagaaaacaagatgataagaaaatcaaagcttgtgttgaagaagttacaacaactctggaagaaactaagttcctcacagaaaacttgttactttatattgacattaatggcaatcttcatccagattctgccactcttgttagtgacattgacatcactttcttaaagaaagatgctccatatatagtgggtgatgttgttcaagagggtgttttaactgctgtggttatacctactaaaaaggctggtggcactactgaaatgctagcgaaagctttgagaaaagtgccaacagacaattatataaccacttacccgggtcagggtttaaatggttacactgtagaggaggcaaagacagtgcttaaaaagtgtaaaagtgccttttacattctaccatctattatctctaatgagaagcaagaaattcttggaactgtttcttggaatttgcgagaaatgcttgcacatgcagaagaaacacgcaaattaatgcctgtctgtgtggaaactaaagccatagtttcaactatacagcgtaaatataagggtattaaaatacaagagggtgtggttgattatggtgctagattttacttttacaccagtaaaacaactgtagcgtcacttatcaacacacttaacgatctaaatgaaactcttgttacaatgccacttggctatgtaacacatggcttaaatttggaagaagctgctcggtatatgagatctctcaaagtgccagctacagtttctgtttcttcacctgatgctgttacagcgtataatggttatcttacttcttcttctaaaacacctgaagaacattttattgaaaccatctcacttgctggttcctataaagattggtcctattctggacaatctacacaactaggtatagaatttcttaagagaggtgataaaagtgtatattacactagtaatcctaccacattccacctagatggtgaagttatcacctttgacaatcttaagacacttctttctttgagagaagtgaggactattaaggtgtttacaacagtagacaacattaacctccacacgcaagttgtggacatgtcaatgacatatggacaacagtttggtccaacttatttggatggagctgatgttactaaaataaaacctcataattcacatgaaggtaaaacattttatgttttacctaatgatgacactctacgtgttgaggcttttgagtactaccacacaactgatcctagttttctgggtaggtacatgtcagcattaaatcacactaaaaagtggaaatacccacaagttaatggtttaacttctattaaatgggcagataacaactgttatcttgccactgcattgttaacactccaacaaatagagttgaagtttaatccacctgctctacaagatgcttattacagagcaagggctggtgaagctgctaacttttgtgcacttatcttagcctactgtaataagacagtaggtgagttaggtgatgttagagaaacaatgagttacttgtttcaacatgccaatttagattcttgcaaaagagtcttgaacgtggtgtgtaaaacttgtggacaacagcagacaacccttaagggtgtagaagctgttatgtacatgggcacactttcttatgaacaatttaagaaaggtgttcagataccttgtacgtgtggtaaacaagctacaaaatatctagtacaacaggagtcaccttttgttatgatgtcagcaccacctgctcagtatgaacttaagcatggtacatttacttgtgctagtgagtacactggtaattaccagtgtggtcactataaacatataacttctaaagaaactttgtattgcatagacggtgctttacttacaaagtcctcagaatacaaaggtcctattacggatgttttctacaaagaaaacagttacacaacaaccataaaaccagttacttataaattggatggtgttgtttgtacagaaattgaccctaagttggacaattattataagaaagacaattcttatttcacagagcaaccaattgatcttgtaccaaaccaaccatatccaaacgcaagcttcgataattttaagtttgtatgtgataatatcaaatttgctgatgatttaaaccagttaactggttataagaaacctgcttcaagagagcttaaagttacatttttccctgacttaaatggtgatgtggtggctattgattataaacactacacaccctcttttaagaaaggagctaaattgttacataaacctattgtttggcatgttaacaatgcaactaataaagccacgtataaaccaaatacctggtgtatacgttgtctttggagcacaaaaccagttgaaacatcaaattcgtttgatgtactgaagtcagaggacgcgcagggaatggataatcttgcctgcgaagatctaaaaccagtctctgaagaagtagtggaaaatcctaccatacagaaagacgttcttgagtgtaatgtgaaaactaccgaagttgtaggagacattatacttaaaccagcaaataatagtttaaaaattacagaagaggttggccacacagatctaatggctgcttatgtagacaattctagtcttactattaagaaacctaatgaattatctagagtattaggtttgaaaacccttgctactcatggtttagctgctgttaatagtgtcccttgggatactatagctaattatgctaagccttttcttaacaaagttgttagtacaactactaacatagttacacggtgtttaaaccgtgtttgtactaattatatgccttatttctttactttattgctacaattgtgtacttttactagaagtacaaattctagaattaaagcatctatgccgactactatagcaaagaatactgttaagagtgtcggtaaattttgtctagaggcttcatttaattatttgaagtcacctaatttttctaaactgataaatattataatttggtttttactattaagtgtttgcctaggttctttaatctactcaaccgctgctttaggtgttttaatgtctaatttaggcatgccttcttactgtactggttacagagaaggctatttgaactctactaatgtcactattgcaacctactgtactggttctataccttgtagtgtttgtcttagtggtttagattctttagacacctatccttctttagaaactatacaaattaccatttcatcttttaaatgggatttaactgcttttggcttagttgcagagtggtttttggcatatattcttttcactaggtttttctatgtacttggattggctgcaatcatgcaattgtttttcagctattttgcagtacattttattagtaattcttggcttatgtggttaataattaatcttgtacaaatggccccgatttcagctatggttagaatgtacatcttctttgcatcattttattatgtatggaaaagttatgtgcatgttgtagacggttgtaattcatcaacttgtatgatgtgttacaaacgtaatagagcaacaagagtcgaatgtacaactattgttaatggtgttagaaggtccttttatgtctatgctaatggaggtaaaggcttttgcaaactacacaattggaattgtgttaattgtgatacattctgtgctggtagtacatttattagtgatgaagttgcgagagacttgtcactacagtttaaaagaccaataaatcctactgaccagtcttcttacatcgttgatagtgttacagtgaagaatggttccatccatctttactttgataaagctggtcaaaagacttatgaaagacattctctctctcattttgttaacttagacaacctgagagctaataacactaaaggttcattgcctattaatgttatagtttttgatggtaaatcaaaatgtgaagaatcatctgcaaaatcagcgtctgtttactacagtcagcttatgtgtcaacctatactgttactagatcaggcattagtgtctgatgttggtgatagtgcggaagttgcagttaaaatgtttgatgcttacgttaatacgttttcatcaacttttaacgtaccaatggaaaaactcaaaacactagttgcaactgcagaagctgaacttgcaaagaatgtgtccttagacaatgtcttatctacttttatttcagcagctcggcaagggtttgttgattcagatgtagaaactaaagatgttgttgaatgtcttaaattgtcacatcaatctgacatagaagttactggcgatagttgtaataactatatgctcacctataacaaagttgaaaacatgacaccccgtgaccttggtgcttgtattgactgtagtgcgcgtcatattaatgcgcaggtagcaaaaagtcacaacattgctttgatatggaacgttaaagatttcatgtcattgtctgaacaactacgaaaacaaatacgtagtgctgctaaaaagaataacttaccttttaagttgacatgtgcaactactagacaagttgttaatgttgtaacaacaaagatagcacttaagggtggtaaaattgttaataattggttgaagcagttaattaaagttacacttgtgttcctttttgttgctgctattttctatttaataacacctgttcatgtcatgtctaaacatactgacttttcaagtgaaatcataggatacaaggctattgatggtggtgtcactcgtgacatagcatctacagatacttgttttgctaacaaacatgctgattttgacacatggtttagccagcgtggtggtagttatactaatgacaaagcttgcccattgattgctgcagtcataacaagagaagtgggttttgtcgtgcctggtttgcctggcacgatattacgcacaactaatggtgactttttgcatttcttacctagagtttttagtgcagttggtaacatctgttacacaccatcaaaacttatagagtacactgactttgcaacatcagcttgtgttttggctgctgaatgtacaatttttaaagatgcttctggtaagccagtaccatattgttatgataccaatgtactagaaggttctgttgcttatgaaagtttacgccctgacacacgttatgtgctcatggatggctctattattcaatttcctaacacctaccttgaaggttctgttagagtggtaacaacttttgattctgagtactgtaggcacggcacttgtgaaagatcagaagctggtgtttgtgtatctactagtggtagatgggtacttaacaatgattattacagatctttaccaggagttttctgtggtgtagatgctgtaaatttacttactaatatgtttacaccactaattcaacctattggtgctttggacatatcagcatctatagtagctggtggtattgtagctatcgtagtaacatgccttgcctactattttatgaggtttagaagagcttttggtgaatacagtcatgtagttgcctttaatactttactattccttatgtcattcactgtactctgtttaacaccagtttactcattcttacctggtgtttattctgttatttacttgtacttgacattttatcttactaatgatgtttcttttttagcacatattcagtggatggttatgttcacacctttagtacctttctggataacaattgcttatatcatttgtatttccacaaagcatttctattggttctttagtaattacctaaagagacgtgtagtctttaatggtgtttcctttagtacttttgaagaagctgcgctgtgcacctttttgttaaataaagaaatgtatctaaagttgcgtagtgatgtgctattacctcttacgcaatataatagatacttagctctttataataagtacaagtattttagtggagcaatggatacaactagctacagagaagctgcttgttgtcatctcgcaaaggctctcaatgacttcagtaactcaggttctgatgttctttaccaaccaccacaaacctctatcacctcagctgttttgcagagtggttttagaaaaatggcattcccatctggtaaagttgagggttgtatggtacaagtaacttgtggtacaactacacttaacggtctttggcttgatgacgtagtttactgtccaagacatgtgatctgcacctctgaagacatgcttaaccctaattatgaagatttactcattcgtaagtctaatcataatttcttggtacaggctggtaatgttcaactcagggttattggacattctatgcaaaattgtgtacttaagcttaaggttgatacagccaatcctaagacacctaagtataagtttgttcgcattcaaccaggacagactttttcagtgttagcttgttacaatggttcaccatctggtgtttaccaatgtgctatgaggcccaatttcactattaagggttcattccttaatggttcatgtggtagtgttggttttaacatagattatgactgtgtctctttttgttacatgcaccatatggaattaccaactggagttcatgctggcacagacttagaaggtaacttttatggaccttttgttgacaggcaaacagcacaagcagctggtacggacacaactattacagttaatgttttagcttggttgtacgctgctgttataaatggagacaggtggtttctcaatcgatttaccacaactcttaatgactttaaccttgtggctatgaagtacaattatgaacctctaacacaagaccatgttgacatactaggacctctttctgctcaaactggaattgccgttttagatatgtgtgcttcattaaaagaattactgcaaaatggtatgaatggacgtaccatattgggtagtgctttattagaagatgaatttacaccttttgatgttgttagacaatgctcaggtgttactttccaaagtgcagtgaaaagaacaatcaagggtacacaccactggttgttactcacaattttgacttcacttttagttttagtccagagtactcaatggtctttgttcttttttttgtatgaaaatgcctttttaccttttgctatgggtattattgctatgtctgcttttgcaatgatgtttgtcaaacataagcatgcatttctctgtttgtttttgttaccttctcttgccactgtagcttattttaatatggtctatatgcctgctagttgggtgatgcgtattatgacatggttggatatggttgatactagtttgtctggttttaagctaaaagactgtgttatgtatgcatcagctgtagtgttactaatccttatgacagcaagaactgtgtatgatgatggtgctaggagagtgtggacacttatgaatgtcttgacactcgtttataaagtttattatggtaatgctttagatcaagccatttccatgtgggctcttataatctctgttacttctaactactcaggtgtagttacaactgtcatgtttttggccagaggtattgtttttatgtgtgttgagtattgccctattttcttcataactggtaatacacttcagtgtataatgctagtttattgtttcttaggctatttttgtacttgttactttggcctcttttgtttactcaaccgctactttagactgactcttggtgtttatgattacttagtttctacacaggagtttagatatatgaattcacagggactactcccacccaagaatagcatagatgccttcaaactcaacattaaattgttgggtgttggtggcaaaccttgtatcaaagtagccactgtacagtctaaaatgtcagatgtaaagtgcacatcagtagtcttactctcagttttgcaacaactcagagtagaatcatcatctaaattgtgggctcaatgtgtccagttacacaatgacattctcttagctaaagatactactgaagcctttgaaaaaatggtttcactactttctgttttgctttccatgcagggtgctgtagacataaacaagctttgtgaagaaatgctggacaacagggcaaccttacaagctatagcctcagagtttagttcccttccatcatatgcagcttttgctactgctcaagaagcttatgagcaggctgttgctaatggtgattctgaagttgttcttaaaaagttgaagaagtctttgaatgtggctaaatctgaatttgaccgtgatgcagccatgcaacgtaagttggaaaagatggctgatcaagctatgacccaaatgtataaacaggctagatctgaggacaagagggcaaaagttactagtgctatgcagacaatgcttttcactatgcttagaaagttggataatgatgcactcaacaacattatcaacaatgcaagagatggttgtgttcccttgaacataatacctcttacaacagcagccaaactaatggttgtcataccagactataacacatataaaaatacgtgtgatggtacaacatttacttatgcatcagcattgtgggaaatccaacaggttgtagatgcagatagtaaaattgttcaacttagtgaaattagtatggacaattcacctaatttagcatggcctcttattgtaacagctttaagggccaattctgctgtcaaattacagaataatgagcttagtcctgttgcactacgacagatgtcttgtgctgccggtactacacaaactgcttgcactgatgacaatgcgttagcttactacaacacaacaaagggaggtaggtttgtacttgcactgttatccgatttacaggatttgaaatgggctagattccctaagagtgatggaactggtactatctatacagaactggaaccaccttgtaggtttgttacagacacacctaaaggtcctaaagtgaagtatttatactttattaaaggattaaacaacctaaatagaggtatggtacttggtagtttagctgccacagtacgtctacaagctggtaatgcaacagaagtgcctgccaattcaactgtattatctttctgtgcttttgctgtagatgctgctaaagcttacaaagattatctagctagtgggggacaaccaatcactaattgtgttaagatgttgtgtacacacactggtactggtcaggcaataacagttacaccggaagccaatatggatcaagaatcctttggtggtgcatcgtgttgtctgtactgccgttgccacatagatcatccaaatcctaaaggattttgtgacttaaaaggtaagtatgtacaaatacctacaacttgtgctaatgaccctgtgggttttacacttaaaaacacagtctgtaccgtctgcggtatgtggaaaggttatggctgtagttgtgatcaactccgcgaacccatgcttcagtcagctgatgcacaatcgtttttaaacgggtttgcggtgtaagtgcagcccgtcttacaccgtgcggcacaggcactagtactgatgtcgtatacagggcttttgacatctacaatgataaagtagctggttttgctaaattcctaaaaactaattgttgtcgcttccaagaaaaggacgaagatgacaatttaattgattcttactttgtagttaagagacacactttctctaactaccaacatgaagaaacaatttataatttacttaaggattgtccagctgttgctaaacatgacttctttaagtttagaatagacggtgacatggtaccacatatatcacgtcaacgtcttactaaatacacaatggcagacctcgtctatgctttaaggcattttgatgaaggtaattgtgacacattaaaagaaatacttgtcacatacaattgttgtgatgatgattatttcaataaaaaggactggtatgattttgtagaaaacccagatatattacgcgtatacgccaacttaggtgaacgtgtacgccaagctttgttaaaaacagtacaattctgtgatgccatgcgaaatgctggtattgttggtgtactgacattagataatcaagatctcaatggtaactggtatgatttcggtgatttcatacaaaccacgccaggtagtggagttcctgttgtagattcttattattcattgttaatgcctatattaaccttgaccagggctttaactgcagagtcacatgttgacactgacttaacaaagccttacattaagtgggatttgttaaaatatgacttcacggaagagaggttaaaactctttgaccgttattttaaatattgggatcagacataccacccaaattgtgttaactgtttggatgacagatgcattctgcattgtgcaaactttaatgttttattctctacagtgttcccacctacaagttttggaccactagtgagaaaaatatttgttgatggtgttccatttgtagtttcaactggataccacttcagagagctaggtgttgtacataatcaggatgtaaacttacatagctctagacttagttttaaggaattacttgtgtatgctgctgaccctgctatgcacgctgcttctggtaatctattactagataaacgcactacgtgcttttcagtagctgcacttactaacaatgttgcttttcaaactgtcaaacccggtaattttaacaaagacttctatgactttgctgtgtctaagggtttctttaaggaaggaagttctgttgaattaaaacacttcttctttgctcaggatggtaatgctgctatcagcgattatgactactatcgttataatctaccaacaatgtgtgatatcagacaactactatttgtagttgaagttgttgataagtactttgattgttacgatggtggctgtattaatgctaaccaagtcatcgtcaacaacctagacaaatcagctggttttccatttaataaatggggtaaggctagactttattatgattcaatgagttatgaggatcaagatgcacttttcgcatatacaaaacgtaatgtcatccctactataactcaaatgaatcttaagtatgccattagtgcaaagaatagagctcgcaccgtagctggtgtctctatctgtagtactatgaccaatagacagtttcatcaaaaattattgaaatcaatagccgccactagaggagctactgtagtaattggaacaagcaaattctatggtggttggcacaacatgttaaaaactgtttatagtgatgtagaaaaccctcaccttatgggttgggattatcctaaatgtgatagagccatgcctaacatgcttagaattatggcctcacttgttcttgctcgcaaacatacaacgtgttgtagcttgtcacaccgtttctatagattagctaatgagtgtgctcaagtattgagtgaaatggtcatgtgtggcggttcactatatgttaaaccaggtggaacctcatcaggagatgccacaactgcttatgctaatagtgtttttaacatttgtcaagctgtcacggccaatgttaatgcacttttatctactgatggtaacaaaattgccgataagtatgtccgcaatttacaacacagactttatgagtgtctctatagaaatagagatgttgacacagactttgtgaatgagttttacgcatatttgcgtaaacatttctcaatgatgatactctctgacgatgctgttgtgtgtttcaatagcacttatgcatctcaaggtctagtggctagcataaagaactttaagtcagttctttattatcaaaacaatgtttttatgtctgaagcaaaatgttggactgagactgaccttactaaaggacctcatgaattttgctctcaacatacaatgctagttaaacagggtgatgattatgtgtaccttccttacccagatccatcaagaatcctaggggccggctgttttgtagatgatatcgtaaaaacagatggtacacttatgattgaacggttcgtgtctttagctatagatgcttacccacttactaaacatcctaatcaggagtatgctgatgtctttcatttgtacttacaatacataagaaagctacatgatgagttaacaggacacatgttagacatgtattctgttatgcttactaatgataacacttcaaggtattgggaacctgagttttatgaggctatgtacacaccgcatacagtcttacaggctgttggggcttgtgttctttgcaattcacagacttcattaagatgtggtgcttgcatacgtagaccattcttatgttgtaaatgctgttacgaccatgtcatatcaacatcacataaattagtcttgtctgttaatccgtatgtttgcaatgctccaggttgtgatgtcacagatgtgactcaactttacttaggaggtatgagctattattgtaaatcacataaaccacccattagttttccattgtgtgctaatggacaagtttttggtttatataaaaatacatgtgttggtagcgataatgttactgactttaatgcaattgcaacatgtgactggacaaatgctggtgattacattttagctaacacctgtactgaaagactcaagctttttgcagcagaaacgctcaaagctactgaggagacatttaaactgtcttatggtattgctactgtacgtgaagtgctgtctgacagagaattacatctttcatgggaagttggtaaacctagaccaccacttaaccgaaattatgtctttactggttatcgtgtaactaaaaacagtaaagtacaaataggagagtacacctttgaaaaaggtgactatggtgatgctgttgtttaccgaggtacaacaacttacaaattaaatgttggtgattattttgtgctgacatcacatacagtaatgccattaagtgcacctacactagtgccacaagagcactatgttagaattactggcttatacccaacactcaatatctcagatgagttttctagcaatgttgcaaattatcaaaaggttggtatgcaaaagtattctacactccagggaccacctggtactggtaagagtcattttgctattggcctagctctctactacccttctgctcgcatagtgtatacagcttgctctcatgccgctgttgatgcactatgtgagaaggcattaaaatatttgcctatagataaatgtagtagaattatacctgcacgtgctcgtgtagagtgttttgataaattcaaagtgaattcaacattagaacagtatgtcttttgtactgtaaatgcattgcctgagacgacagcagatatagttgtctttgatgaaatttcaatggccacaaattatgatttgagtgttgtcaatgccagattacgtgctaagcactatgtgtacattggcgaccctgctcaattacctgcaccacgcacattgctaactaagggcacactagaaccagaatatttcaattcagtgtgtagacttatgaaaactataggtccagacatgttcctcggaacttgtcggcgttgtcctgctgaaattgttgacactgtgagtgctttggtttatgataataagcttaaagcacataaagacaaatcagctcaatgctttaaaatgttttataagggtgttatcacgcatgatgtttcatctgcaattaacaggccacaaataggcgtggtaagagaattccttacacgtaaccctgcttggagaaaagctgtctttatttcaccttataattcacagaatgctgtagcctcaaagattttgggactaccaactcaaactgttgattcatcacagggctcagaatatgactatgtcatattcactcaaaccactgaaacagctcactcttgtaatgtaaacagatttaatgttgctattaccagagcaaaagtaggcatactttgcataatgtctgatagagacctttatgacaagttgcaatttacaagtcttgaaattccacgtaggaatgtggcaactttacaagctgaaaatgtaacaggactctttaaagattgtagtaaggtaatcactgggttacatcctacacaggcacctacacacctcagtgttgacactaaattcaaaactgaaggtttatgtgttgacatacctggcatacctaaggacatgacctatagaagactcatctctatgatgggttttaaaatgaattatcaagttaatggttaccctaacatgtttatcacccgcgaagaagctataagacatgtacgtgcatggattggcttcgatgtcgaggggtgtcatgctactagagaagctgttggtaccaatttacctttacagctaggtttttctacaggtgttaacctagttgctgtacctacaggttatgttgatacacctaataatacagatttttccagagttagtgctaaaccaccgcctggagatcaatttaaacacctcataccacttatgtacaaaggacttccttggaatgtagtgcgtataaagattgtacaaatgttaagtgacacacttaaaaatctctctgacagagtcgtatttgtcttatgggcacatggctttgagttgacatctatgaagtattttgtgaaaataggacctgagcgcacctgttgtctatgtgatagacgtgccacatgcttttccactgcttcagacacttatgcctgttggcatcattctattggatttgattacgtctataatccgtttatgattgatgttcaacaatggggttttacaggtaacctacaaagcaaccatgatctgtattgtcaagtccatggtaatgcacatgtagctagttgtgatgcaatcatgactaggtgtctagctgtccacgagtgctttgttaagcgtgttgactggactattgaatatcctataattggtgatgaactgaagattaatgcggcttgtagaaaggttcaacacatggttgttaaagctgcattattagcagacaaattcccagttcttcacgacattggtaaccctaaagctattaagtgtgtacctcaagctgatgtagaatggaagttctatgatgcacagccttgtagtgacaaagcttataaaatagaagaattattctattcttatgccacacattctgacaaattcacagatggtgtatgcctattttggaattgcaatgtcgatagatatcctgctaattccattgtttgtagatttgacactagagtgctatctaaccttaacttgcctggttgtgatggtggcagtttgtatgtaaataaacatgcattccacacaccagcttttgataaaagtgcttttgttaatttaaaacaattaccatttttctattactctgacagtccatgtgagtctcatggaaaacaagtagtgtcagatatagattatgtaccactaaagtctgctacgtgtataacacgttgcaatttaggtggtgctgtctgtagacatcatgctaatgagtacagattgtatctcgatgcttataacatgatgatctcagctggctttagcttgtgggtttacaaacaatttgatacttataacctctggaacacttttacaagacttcagagtttagaaaatgtggcttttaatgttgtaaataagggacactttgatggacaacagggtgaagtaccagtttctatcattaataacactgtttacacaaaagttgatggtgttgatgtagaattgtttgaaaataaaacaacattacctgttaatgtagcatttgagctttgggctaagcgcaacattaaaccagtaccagaggtgaaaatactcaataatttgggtgtggacattgctgctaatactgtgatctgggactacaaaagagatgctccagcacatatatctactattggtgtttgttctatgactgacatagccaagaaaccaactgaaacgatttgtgcaccactcactgtcttttttgatggtagagttgatggtcaagtagacttatttagaaatgcccgtaatggtgttcttattacagaaggtagtgttaaaggtttacaaccatctgtgggtcccaaacaagctagtcttaatggagtcacattaattggagaagccgtaaaaacacagttcaattattataagaaagttgatggtgttgtccaacaattacctgaaacttactttactcagagtagaaatttacaagaatttaaacccaggagtcaaatggaaattgatttcttagaattagctatggatgaattcattgaacggtataaattagaaggctatgccttcgaacatatcgtttatggagattttagtcatagtcagttaggtggtttacatctactgattggactagctaaacgttttaaggaatcaccttttgaattagaagattttattcctatggacagtacagttaaaaactatttcataacagatgcgcaaacaggttcatctaagtgtgtgtgttctgttattgatttattacttgatgattttgttgaaataataaaatcccaagatttatctgtagtttctaaggttgtcaaagtgactattgactatacagaaatttcatttatgctttggtgtaaagatggccatgtagaaacattttacccaaaattacaatctagtcaagcgtggcaaccgggtgttgctatgcctaatctttacaaaatgcaaagaatgctattagaaaagtgtgaccttcaaaattatggtgatagtgcaacattacctaaaggcataatgatgaatgtcgcaaaatatactcaactgtgtcaatatttaaacacattaacattagctgtaccctataatatgagagttatacattttggtgctggttctgataaaggagttgcaccaggtacagctgttttaagacagtggttgcctacgggtacgctgcttgtcgattcagatcttaatgactttgtctctgatgcagattcaactttgattggtgattgtgcaactgtacatacagctaataaatgggatctcattattagtgatatgtacgaccctaagactaaaaatgttacaaaagaaaatgactctaaagagggttttttcacttacatttgtgggtttatacaacaaaagctagctcttggaggttccgtggctataaagataacagaacattcttggaatgctgatctttataagctcatgggacacttcgcatggtggacagcctttgttactaatgtgaatgcgtcatcatctgaagcatttttaattggatgtaattatcttggcaaaccacgcgaacaaatagatggttatgtcatgcatgcaaattacatattttggaggaatacaaatccaattcagttgtcttcctattctttatttgacatgagtaaatttccccttaaattaaggggtactgctgttatgtctttaaaagaaggtcaaatcaatgatatgattttatctcttcttagtaaaggtagacttataattagagaaaacaacagagttgttatttctagtgatgttcttgttaacaactaaacgaacaatgtttgtttttcttgttttattgccactagtctctagtcagtgtgttaatcttacaaccagaactcaattaccccctgcatacactaattctttcacacgtggtgtttattaccctgacaaagttttcagatcctcagttttacattcaactcaggacttgttcttacctttcttttccaatgttacttggttccatgctatacatgtctctgggaccaatggtactaagaggtttgataaccctgtcctaccatttaatgatggtgtttattttgcttccactgagaagtctaacataataagaggctggatttttggtactactttagattcgaagacccagtccctacttattgttaataacgctactaatgttgttattaaagtctgtgaatttcaattttgtaatgatccatttttgggtgtttattaccacaaaaacaacaaaagttggatggaaagtgagttcagagtttattctagtgcgaataattgcacttttgaatatgtctctcagccttttcttatggaccttgaaggaaaacagggtaatttcaaaaatcttagggaatttgtgtttaagaatattgatggttattttaaaatatattctaagcacacgcctattaatttagtgcgtgatctccctcagggtttttcggctttagaaccattggtagatttgccaataggtattaacatcactaggtttcaaactttacttgctttacatagaagttatttgactcctggtgattcttcttcaggttggacagctggtgctgcagcttattatgtgggttatcttcaacctaggacttttctattaaaatataatgaaaatggaaccattacagatgctgtagactgtgcacttgaccctctctcagaaacaaagtgtacgttgaaatccttcactgtagaaaaaggaatctatcaaacttctaactttagagtccaaccaacagaatctattgttagatttcctaatattacaaacttgtgcccttttggtgaagtttttaacgccaccagatttgcatctgtttatgcttggaacaggaagagaatcagcaactgtgttgctgattattctgtcctatataattccgcatcattttccacttttaagtgttatggagtgtctcctactaaattaaatgatctctgctttactaatgtctatgcagattcatttgtaattagaggtgatgaagtcagacaaatcgctccagggcaaactggaaagattgctgattataattataaattaccagatgattttacaggctgcgttatagcttggaattctaacaatcttgattctaaggttggtggtaattataattacctgtatagattgtttaggaagtctaatctcaaaccttttgagagagatatttcaactgaaatctatcaggccggtagcacaccttgtaatggtgttgaaggttttaattgttactttcctttacaatcatatggtttccaacccactaatggtgttggttaccaaccatacagagtagtagtactttcttttgaacttctacatgcaccagcaactgtttgtggacctaaaaagtctactaatttggttaaaaacaaatgtgtcaatttcaacttcaatggtttaacaggcacaggtgttcttactgagtctaacaaaaagtttctgcctttccaacaatttggcagagacattgctgacactactgatgctgtccgtgatccacagacacttgagattcttgacattacaccatgttcttttggtggtgtcagtgttataacaccaggaacaaatacttctaaccaggttgctgttctttatcaggatgttaactgcacagaagtccctgttgctattcatgcagatcaacttactcctacttggcgtgtttattctacaggttctaatgtttttcaaacacgtgcaggctgtttaataggggctgaacatgtcaacaactcatatgagtgtgacatacccattggtgcaggtatatgcgctagttatcagactcagactaattctcctcggcgggcacgtagtgtagctagtcaatccatcattgcctacactatgtcacttggtgcagaaaattcagttgcttactctaataactctattgccatacccacaaattttactattagtgttaccacagaaattctaccagtgtctatgaccaagacatcagtagattgtacaatgtacatttgtggtgattcaactgaatgcagcaatcttttgttgcaatatggcagtttttgtacacaattaaaccgtgctttaactggaatagctgttgaacaagacaaaaacacccaagaagtttttgcacaagtcaaacaaatttacaaaacaccaccaattaaagattttggtggttttaatttttcacaaatattaccagatccatcaaaaccaagcaagaggtcatttattgaagatctacttttcaacaaagtgacacttgcagatgctggcttcatcaaacaatatggtgattgccttggtgatattgctgctagagacctcatttgtgcacaaaagtttaacggccttactgttttgccacctttgctcacagatgaaatgattgctcaatacacttctgcactgttagcgggtacaatcacttctggttggacctttggtgcaggtgctgcattacaaataccatttgctatgcaaatggcttataggtttaatggtattggagttacacagaatgttctctatgagaaccaaaaattgattgccaaccaatttaatagtgctattggcaaaattcaagactcactttcttccacagcaagtgcacttggaaaacttcaagatgtggtcaaccaaaatgcacaagctttaaacacgcttgttaaacaacttagctccaattttggtgcaatttcaagtgttttaaatgatatcctttcacgtcttgacaaagttgaggctgaagtgcaaattgataggttgatcacaggcagacttcaaagtttgcagacatatgtgactcaacaattaattagagctgcagaaatcagagcttctgctaatcttgctgctactaaaatgtcagagtgtgtacttggacaatcaaaaagagttgatttttgtggaaagggctatcatcttatgtccttccctcagtcagcacctcatggtgtagtcttcttgcatgtgacttatgtccctgcacaagaaaagaacttcacaactgctcctgccatttgtcatgatggaaaagcacactttcctcgtgaaggtgtctttgtttcaaatggcacacactggtttgtaacacaaaggaatttttatgaaccacaaatcattactacagacaacacatttgtgtctggtaactgtgatgttgtaataggaattgtcaacaacacagtttatgatcctttgcaacctgaattagactcattcaaggaggagttagataaatattttaagaatcatacatcaccagatgttgatttaggtgacatctctggcattaatgcttcagttgtaaacattcaaaaagaaattgaccgcctcaatgaggttgccaagaatttaaatgaatctctcatcgatctccaagaacttggaaagtatgagcagtatataaaatggccatggtacatttggctaggttttatagctggcttgattgccatagtaatggtgacaattatgctttgctgtatgaccagttgctgtagttgtctcaagggctgttgttcttgtggatcctgctgcaaatttgatgaagacgactctgagccagtgctcaaaggagtcaaattacattacacataaacgaacttatggatttgtttatgagaatcttcacaattggaactgtaactttgaagcaaggtgaaatcaaggatgctactccttcagattttgttcgcgctactgcaacgataccgatacaagcctcactccctttcggatggcttattgttggcgttgcacttcttgctgtttttcagagcgcttccaaaatcataaccctcaaaaagagatggcaactagcactctccaagggtgttcactttgtttgcaacttgctgttgttgtttgtaacagtttactcacaccttttgctcgttgctgctggccttgaagccccttttctctatctttatgctttagtctacttcttgcagagtataaactttgtaagaataataatgaggctttggctttgctggaaatgccgttccaaaaacccattactttatgatgccaactattttctttgctggcatactaattgttacgactattgtataccttacaatagtgtaacttcttcaattgtcattacttcaggtgatggcacaacaagtcctatttctgaacatgactaccagattggtggttatactgaaaaatgggaatctggagtaaaagactgtgttgtattacacagttacttcacttcagactattaccagctgtactcaactcaattgagtacagacactggtgttgaacatgttaccttcttcatctacaataaaattgttgatgagcctgaagaacatgtccaaattcacacaatcgacggttcatccggagttgttaatccagtaatggaaccaatttatgatgaaccgacgacgactactagcgtgcctttgtaagcacaagctgatgagtacgaacttatgtactcattcgtttcggaagagacaggtacgttaatagttaatagcgtacttctttttcttgctttcgtggtattcttgctagttacactagccatccttactgcgcttcgattgtgtgcgtactgctgcaatattgttaacgtgagtcttgtaaaaccttctttttacgtttactctcgtgttaaaaatctgaattcttctagagttcctgatcttctggtctaaacgaactaaatattatattagtttttctgtttggaactttaattttagccatggcagattccaacggtactattaccgttgaagagcttaaaaagctccttgaacaatggaacctagtaataggtttcctattccttacatggatttgtcttctacaatttgcctatgccaacaggaataggtttttgtatataattaagttaattttcctctggctgttatggccagtaactttagcttgttttgtgcttgctgctgtttacagaataaattggatcaccggtggaattgctatcgcaatggcttgtcttgtaggcttgatgtggctcagctacttcattgcttctttcagactgtttgcgcgtacccgttccatgtggtcattcaatccagaaactaacattcttctcaacgtgccactccatggcactattctgaccagaccgcttctagaaagtgaactcgtaatcggagctgtgatccttcgtggacatcttcgtattgctggacaccatctaggacgctgtgacatcaaggacctgcctaaagaaatcactgttgctacatcccgcacgctttcttattacaaattgggagcttcgcagcgtgtagcaggtgactcaggttttgctgcatacagtcgctacaggattggcaactataaattaaacacagaccattccagtagcagtgacaatattgctttgcttgtacagtaagtgacaacagaaccaatggagattgattaaacgaacatgaaaattattcttttcttggcactgataacactcgctacttgtgagctttatcactaccaagagtgtgttagaggtacaacagtacttttaaaagaaccttgctcttctggaacatacgagggcaattcaccatttcatcctctagctgataacaaatttgcactgacttgctttagcactcaatttgcttttgcttgtcctgacggcgtaaaacacgtctatcagttacgtgccagatcagtttcacctaaactgttcatcagacaagaggaagttcaagaactttactctccaatttttcttattgttgcggcaatagtgtttataacactttgcttcacactcaaaagaaagacagaatgattgaactttcattaattgacttctatttgtgctttttagcctttctgctattccttgttttaattatgcttattatcttttggttctcacttgaactgcaagatcataatgaaacttgtcacgcctaatgttttagatttcatctaaacgaacaaactaaaatgtctgataatggaccccaaaatcagcgaaatgcaccccgcattacgtttggtggaccctcagattcaactggcagtaaccagaatggagaacgcagtggggcgcgatcaaaacaacgtcggccccaaggtttacccaataatactgcgtcttggttcaccgctctcactcaacatggcaaggaagaccttaaattccctcgaggacaaggcgttccaattaacaccaatagcagtccagatgaccaaattggctactaccgaagagctaccagacgaattcgtggtggtgacggtaaaatgaaagatctcagtccaagatggtatttctactacctaggaactgggccagaagctggacttccctatggtgctaacaaagacggcatcatatgggttgcaactgagggagccttgaatacaccaaaagatcacattggcacccgcaatcctgctaacaatgctgcaatcgtgctacaacttcctcaaggaacaacattgccaaaaggcttctacgcagaagggagcagaggcggcagtcaagcctcttctcgttcctcatcacgtagtcgcaacagttcaagaaattcaactccaggcagcagtaggggaacttctcctgctagaatggctggcaatggcggtgatgctgctcttgctttgctgctgcttgacagattgaaccagcttgagagcaaaatgtctggtaaaggccaacaacaacaaggccaaactgtcactaagaaatctgctgctgaggcttctaagaagcctcggcaaaaacgtactgccactaaagcatacaatgtaacacaagctttcggcagacgtggtccagaacaaacccaaggaaattttggggaccaggaactaatcagacaaggaactgattacaaacattggccgcaaattgcacaatttgcccccagcgcttcagcgttcttcggaatgtcgcgcattggcatggaagtcacaccttcgggaacgtggttgacctacacaggtgccatcaaattggatgacaaagatccaaatttcaaagatcaagtcattttgctgaataagcatattgacgcatacaaaacattcccaccaacagagcctaaaaaggacaaaaagaagaaggctgatgaaactcaagccttaccgcagagacagaagaaacagcaaactgtgactcttcttcctgctgcagatttggatgatttctccaaacaattgcaacaatccatgagcagtgctgactcaactcaggcctaaactcatgcagaccacacaaggcagatgggctatataaacgttttcgcttttccgtttacgatatatagtctactcttgtgcagaatgaattctcgtaactacatagcacaagtagatgtagttaactttaatctcacatagcaatctttaatcagtgtgtaacattagggaggacttgaaagagccaccacattttcaccgaggccacgcggagtacgatcgagtgtacagtgaacaatgctagggagagctgcctatatggaagagccctaatgtgtaaaattaattttagtagtgctatccccatgtgattttaatagcttcttaggagaatgacaaaaaaaaaaaaaaaaaaaaaaaaa

SEQ ID NO: 24 - DNA, 28857 bp, Coronaviridae
  misc_feature 1..28857: note = SARS-CoV-2-[6,7,8] nucleotide sequence, it contains two punctual substitutions (c.27041A-C and c.27044A-C)
  source 1..28857: mol_type = other DNA
attaaaggtttataccttcccaggtaacaaaccaaccaactttcgatctcttgtagatctgttctctaaacgaactttaaaatctgtgtggctgtcactcggctgcatgcttagtgcactcacgcagtataattaataactaattactgtcgttgacaggacacgagtaactcgtctatcttctgcaggctgcttacggtttcgtccgtgttgcagccgatcatcagcacatctaggtttcgtccgggtgtgaccgaaaggtaagatggagagccttgtccctggtttcaacgagaaaacacacgtccaactcagtttgcctgttttacaggttcgcgacgtgctcgtacgtggctttggagactccgtggaggaggtcttatcagaggcacgtcaacatcttaaagatggcacttgtggcttagtagaagttgaaaaaggcgttttgcctcaacttgaacagccctatgtgttcatcaaacgttcggatgctcgaactgcacctcatggtcatgttatggttgagctggtagcagaactcgaaggcattcagtacggtcgtagtggtgagacacttggtgtccttgtccctcatgtgggcgaaataccagtggcttaccgcaaggttcttcttcgtaagaacggtaataaaggagctggtggccatagttacggcgccgatctaaagtcatttgacttaggcgacgagcttggcactgatccttatgaagattttcaagaaaactggaacactaaacatagcagtggtgttacccgtgaactcatgcgtgagcttaacggaggggcatacactcgctatgtcgataacaacttctgtggccctgatggctaccctcttgagtgcattaaagaccttctagcacgtgctggtaaagcttcatgcactttgtccgaacaactggactttattgacactaagaggggtgtatactgctgccgtgaacatgagcatgaaattgcttggtacacggaacgttctgaaaagagctatgaattgcagacaccttttgaaattaaattggcaaagaaatttgacaccttcaatggggaatgtccaaattttgtatttcccttaaattccataatcaagactattcaaccaagggttgaaaagaaaaagcttgatggctttatgggtagaattcgatctgtctatccagttgcgtcaccaaatgaatgcaaccaaatgtgcctttcaactctcatgaagtgtgatcattgtggtgaaacttcatggcagacgggcgattttgttaaagccacttgcgaattttgtggcactgagaatttgactaaagaaggtgccactacttgtggttacttaccccaaaatgctgttgttaaaatttattgtccagcatgtcacaattcagaagtaggacctgagcatagtcttgccgaataccataatgaatctggcttgaaaaccattcttcgtaagggtggtcgcactattgcctttggaggctgtgtgttctcttatgttggttgccataacaagtgtgcctattgggttccacgtgctagcgctaacataggttgtaaccatacaggtgttgttggagaaggttccgaaggtcttaatgacaaccttcttgaaatactccaaaaagagaaagtcaacatcaatattgttggtgactttaaacttaatgaagagatcgccattattttggcatctttttctgcttccacaagtgcttttgtggaaactgtgaaaggtttggattataaagcattcaaacaaattgttgaatcctgtggtaattttaaagttacaaaaggaaaagctaaaaaaggtgcctggaatattggtgaacagaaatcaatactgagtcctctttatgcatttgcatcagaggctgctcgtgttgtacgatcaattttctcccgcactcttgaaactgctcaaaattctgtgcgtgttttacagaaggccgctataacaatactagatggaatttcacagtattcactgagactcattgatgctatgatgttcacatctgatttggctactaacaatctagttgtaatggcctacattacaggtggtgttgttcagttgacttcgcagtggctaactaacatctttggcactgtttatgaaaaactcaaacccgtccttgattggcttgaagagaagtttaaggaaggtgtagagtttcttagagacggttgggaaattgttaaatttatctcaacctgtgcttgtgaaattgtcggtggacaaattgtcacctgtgcaaaggaaattaaggagagtgttcagacattctttaagcttgtaaataaatttttggctttgtgtgctgactctatcattattggtggagctaaacttaaagccttgaatttaggtgaaacatttgtcacgcactcaaagggattgtacagaaagtgtgttaaatccagagaagaaactggcctactcatgcctctaaaagccccaaaagaaattatcttcttagagggagaaacacttcccacagaagtgttaacagaggaagttgtcttgaaaactggtgatttacaaccattagaacaacctactagtgaagctgttgaagctccattggttggtacaccagtttgtattaacgggcttatgttgctcgaaatcaaagacacagaaaagtactgtgcccttgcacctaatatgatggtaacaaacaataccttcacactcaaaggcggtgcaccaacaaaggttacttttggtgatgacactgtgatagaagtgcaaggttacaagagtgtgaatatcacttttgaacttgatgaaaggattgataaagtacttaatgagaagtgctctgcctatacagttgaactcggtacagaagtaaatgagttcgcctgtgttgtggcagatgctgtcataaaaactttgcaaccagtatctgaattacttacaccactgggcattgatttagatgagtggagtatggctacatactacttatttgatgagtctggtgagtttaaattggcttcacatatgtattgttctttctaccctccagatgaggatgaagaagaaggtgattgtgaagaagaagagtttgagccatcaactcaatatgagtatggtactgaagatgattaccaaggtaaacctttggaatttggtgccacttctgctgctcttcaacctgaagaagagcaagaagaagattggttagatgatgatagtcaacaaactgttggtcaacaagacggcagtgaggacaatcagacaactactattcaaacaattgttgaggttcaacctcaattagagatggaacttacaccagttgttcagactattgaagtgaatagttttagtggttatttaaaacttactgacaatgtatacattaaaaatgcagacattgtggaagaagctaaaaaggtaaaaccaacagtggttgttaatgcagccaatgtttaccttaaacatggaggaggtgttgcaggagccttaaataaggctactaacaatgccatgcaagttgaatctgatgattacatagctactaatggaccacttaaagtgggtggtagttgtgttttaagcggacacaatcttgctaaacactgtcttcatgttgtcggcccaaatgttaacaaaggtgaagacattcaacttcttaagagtgcttatgaaaattttaatcagcacgaagttctacttgcaccattattatcagctggtatttttggtgctgaccctatacattctttaagagtttgtgtagatactgttcgcacaaatgtctacttagctgtctttgataaaaatctctatgacaaacttgtttcaagctttttggaaatgaagagtgaaaagcaagttgaacaaaagatcgctgagattcctaaagaggaagttaagccatttataactgaaagtaaaccttcagttgaacagagaaaacaagatgataagaaaatcaaagcttgtgttgaagaagttacaacaactctggaagaaactaagttcctcacagaaaacttgttactttatattgacattaatggcaatcttcatccagattctgccactcttgttagtgacattgacatcactttcttaaagaaagatgctccatatatagtgggtgatgttgttcaagagggtgttttaactgctgtggttatacctactaaaaaggctggtggcactactgaaatgctagcgaaagctttgagaaaagtgccaacagacaattatataaccacttacccgggtcagggtttaaatggttacactgtagaggaggcaaagacagtgcttaaaaagtgtaaaagtgccttttacattctaccatctattatctctaatgagaagcaagaaattcttggaactgtttcttggaatttgcgagaaatgcttgcacatgcagaagaaacacgcaaattaatgcctgtctgtgtggaaactaaagccatagtttcaactatacagcgtaaatataagggtattaaaatacaagagggtgtggttgattatggtgctagattttacttttacaccagtaaaacaactgtagcgtcacttatcaacacacttaacgatctaaatgaaactcttgttacaatgccacttggctatgtaacacatggcttaaatttggaagaagctgctcggtatatgagatctctcaaagtgccagctacagtttctgtttcttcacctgatgctgttacagcgtataatggttatcttacttcttcttctaaaacacctgaagaacattttattgaaaccatctcacttgctggttcctataaagattggtcctattctggacaatctacacaactaggtatagaatttcttaagagaggtgataaaagtgtatattacactagtaatcctaccacattccacctagatggtgaagttatcacctttgacaatcttaagacacttctttctttgagagaagtgaggactattaaggtgtttacaacagtagacaacattaacctccacacgcaagttgtggacatgtcaatgacatatggacaacagtttggtccaacttatttggatggagctgatgttactaaaataaaacctcataattcacatgaaggtaaaacattttatgttttacctaatgatgacactctacgtgttgaggcttttgagtactaccacacaactgatcctagttttctgggtaggtacatgtcagcattaaatcacactaaaaagtggaaatacccacaagttaatggtttaacttctattaaatgggcagataacaactgttatcttgccactgcattgttaacactccaacaaatagagttgaagtttaatccacctgctctacaagatgcttattacagagcaagggctggtgaagctgctaacttttgtgcacttatcttagcctactgtaataagacagtaggtgagttaggtgatgttagagaaacaatgagttacttgtttcaacatgccaatttagattcttgcaaaagagtcttgaacgtggtgtgtaaaacttgtggacaacagcagacaacccttaagggtgtagaagctgttatgtacatgggcacactttcttatgaacaatttaagaaaggtgttcagataccttgtacgtgtggtaaacaagctacaaaatatctagtacaacaggagtcaccttttgttatgatgtcagcaccacctgctcagtatgaacttaagcatggtacatttacttgtgctagtgagtacactggtaattaccagtgtggtcactataaacatataacttctaaagaaactttgtattgcatagacggtgctttacttacaaagtcctcagaatacaaaggtcctattacggatgttttctacaaagaaaacagttacacaacaaccataaaaccagttacttataaattggatggtgttgtttgtacagaaattgaccctaagttggacaattattataagaaagacaattcttatttcacagagcaaccaattgatcttgtaccaaaccaaccatatccaaacgcaagcttcgataattttaagtttgtatgtgataatatcaaatttgctgatgatttaaaccagttaactggttataagaaacctgcttcaagagagcttaaagttacatttttccctgacttaaatggtgatgtggtggctattgattataaacactacacaccctcttttaagaaaggagctaaattgttacataaacctattgtttggcatgttaacaatgcaactaataaagccacgtataaaccaaatacctggtgtatacgttgtctttggagcacaaaaccagttgaaacatcaaattcgtttgatgtactgaagtcagaggacgcgcagggaatggataatcttgcctgcgaagatctaaaaccagtctctgaagaagtagtggaaaatcctaccatacagaaagacgttcttgagtgtaatgtgaaaactaccgaagttgtaggagacattatacttaaaccagcaaataatagtttaaaaattacagaagaggttggccacacagatctaatggctgcttatgtagacaattctagtcttactattaagaaacctaatgaattatctagagtattaggtttgaaaacccttgctactcatggtttagctgctgttaatagtgtcccttgggatactatagctaattatgctaagccttttcttaacaaagttgttagtacaactactaacatagttacacggtgtttaaaccgtgtttgtactaattatatgccttatttctttactttattgctacaattgtgtacttttactagaagtacaaattctagaattaaagcatctatgccgactactatagcaaagaatactgttaagagtgtcggtaaattttgtctagaggcttcatttaattatttgaagtcacctaatttttctaaactgataaatattataatttggtttttactattaagtgtttgcctaggttctttaatctactcaaccgctgctttaggtgttttaatgtctaatttaggcatgccttcttactgtactggttacagagaaggctatttgaactctactaatgtcactattgcaacctactgtactggttctataccttgtagtgtttgtcttagtggtttagattctttagacacctatccttctttagaaactatacaaattaccatttcatcttttaaatgggatttaactgcttttggcttagttgcagagtggtttttggcatatattcttttcactaggtttttctatgtacttggattggctgcaatcatgcaattgtttttcagctattttgcagtacattttattagtaattcttggcttatgtggttaataattaatcttgtacaaatggccccgatttcagctatggttagaatgtacatcttctttgcatcattttattatgtatggaaaagttatgtgcatgttgtagacggttgtaattcatcaacttgtatgatgtgttacaaacgtaatagagcaacaagagtcgaatgtacaactattgttaatggtgttagaaggtccttttatgtctatgctaatggaggtaaaggcttttgcaaactacacaattggaattgtgttaattgtgatacattctgtgctggtagtacatttattagtgatgaagttgcgagagacttgtcactacagtttaaaagaccaataaatcctactgaccagtcttcttacatcgttgatagtgttacagtgaagaatggttccatccatctttactttgataaagctggtcaaaagacttatgaaagacattctctctctcattttgttaacttagacaacctgagagctaataacactaaaggttcattgcctattaatgttatagtttttgatggtaaatcaaaatgtgaagaatcatctgcaaaatcagcgtctgtttactacagtcagcttatgtgtcaacctatactgttactagatcaggcattagtgtctgatgttggtgatagtgcggaagttgcagttaaaatgtttgatgcttacgttaatacgttttcatcaacttttaacgtaccaatggaaaaactcaaaacactagttgcaactgcagaagctgaacttgcaaagaatgtgtccttagacaatgtcttatctacttttatttcagcagctcggcaagggtttgttgattcagatgtagaaactaaagatgttgttgaatgtcttaaattgtcacatcaatctgacatagaagttactggcgatagttgtaataactatatgctcacctataacaaagttgaaaacatgacaccccgtgaccttggtgcttgtattgactgtagtgcgcgtcatattaatgcgcaggtagcaaaaagtcacaacattgctttgatatggaacgttaaagatttcatgtcattgtctgaacaactacgaaaacaaatacgtagtgctgctaaaaagaataacttaccttttaagttgacatgtgcaactactagacaagttgttaatgttgtaacaacaaagatagcacttaagggtggtaaaattgttaataattggttgaagcagttaattaaagttacacttgtgttcctttttgttgctgctattttctatttaataacacctgttcatgtcatgtctaaacatactgacttttcaagtgaaatcataggatacaaggctattgatggtggtgtcactcgtgacatagcatctacagatacttgttttgctaacaaacatgctgattttgacacatggtttagccagcgtggtggtagttatactaatgacaaagcttgcccattgattgctgcagtcataacaagagaagtgggttttgtcgtgcctggtttgcctggcacgatattacgcacaactaatggtgactttttgcatttcttacctagagtttttagtgcagttggtaacatctgttacacaccatcaaaacttatagagtacactgactttgcaacatcagcttgtgttttggctgctgaatgtacaatttttaaagatgcttctggtaagccagtaccatattgttatgataccaatgtactagaaggttctgttgcttatgaaagtttacgccctgacacacgttatgtgctcatggatggctctattattcaatttcctaacacctaccttgaaggttctgttagagtggtaacaacttttgattctgagtactgtaggcacggcacttgtgaaagatcagaagctggtgtttgtgtatctactagtggtagatgggtacttaacaatgattattacagatctttaccaggagttttctgtggtgtagatgctgtaaatttacttactaatatgtttacaccactaattcaacctattggtgctttggacatatcagcatctatagtagctggtggtattgtagctatcgtagtaacatgccttgcctactattttatgaggtttagaagagcttttggtgaatacagtcatgtagttgcctttaatactttactattccttatgtcattcactgtactctgtttaacaccagtttactcattcttacctggtgtttattctgttatttacttgtacttgacattttatcttactaatgatgtttcttttttagcacatattcagtggatggttatgttcacacctttagtacctttctggataacaattgcttatatcatttgtatttccacaaagcatttctattggttctttagtaattacctaaagagacgtgtagtctttaatggtgtttcctttagtacttttgaagaagctgcgctgtgcacctttttgttaaataaagaaatgtatctaaagttgcgtagtgatgtgctattacctcttacgcaatataatagatacttagctctttataataagtacaagtattttagtggagcaatggatacaactagctacagagaagctgcttgttgtcatctcgcaaaggctctcaatgacttcagtaactcaggttctgatgttctttaccaaccaccacaaacctctatcacctcagctgttttgcagagtggttttagaaaaatggcattcccatctggtaaagttgagggttgtatggtacaagtaacttgtggtacaactacacttaacggtctttggcttgatgacgtagtttactgtccaagacatgtgatctgcacctctgaagacatgcttaaccctaattatgaagatttactcattcgtaagtctaatcataatttcttggtacaggctggtaatgttcaactcagggttattggacattctatgcaaaattgtgtacttaagcttaaggttgatacagccaatcctaagacacctaagtataagtttgttcgcattcaaccaggacagactttttcagtgttagcttgttacaatggttcaccatctggtgtttaccaatgtgctatgaggcccaatttcactattaagggttcattccttaatggttcatgtggtagtgttggttttaacatagattatgactgtgtctctttttgttacatgcaccatatggaattaccaactggagttcatgctggcacagacttagaaggtaacttttatggaccttttgttgacaggcaaacagcacaagcagctggtacggacacaactattacagttaatgttttagcttggttgtacgctgctgttataaatggagacaggtggtttctcaatcgatttaccacaactcttaatgactttaaccttgtggctatgaagtacaattatgaacctctaacacaagaccatgttgacatactaggacctctttctgctcaaactggaattgccgttttagatatgtgtgcttcattaaaagaattactgcaaaatggtatgaatggacgtaccatattgggtagtgctttattagaagatgaatttacaccttttgatgttgttagacaatgctcaggtgttactttccaaagtgcagtgaaaagaacaatcaagggtacacaccactggttgttactcacaattttgacttcacttttagttttagtccagagtactcaatggtctttgttcttttttttgtatgaaaatgcctttttaccttttgctatgggtattattgctatgtctgcttttgcaatgatgtttgtcaaacataagcatgcatttctctgtttgtttttgttaccttctcttgccactgtagcttattttaatatggtctatatgcctgctagttgggtgatgcgtattatgacatggttggatatggttgatactagtttgtctggttttaagctaaaagactgtgttatgtatgcatcagctgtagtgttactaatccttatgacagcaagaactgtgtatgatgatggtgctaggagagtgtggacacttatgaatgtcttgacactcgtttataaagtttattatggtaatgctttagatcaagccatttccatgtgggctcttataatctctgttacttctaactactcaggtgtagttacaactgtcatgtttttggccagaggtattgtttttatgtgtgttgagtattgccctattttcttcataactggtaatacacttcagtgtataatgctagtttattgtttcttaggctatttttgtacttgttactttggcctcttttgtttactcaaccgctactttagactgactcttggtgtttatgattacttagtttctacacaggagtttagatatatgaattcacagggactactcccacccaagaatagcatagatgccttcaaactcaacattaaattgttgggtgttggtggcaaaccttgtatcaaagtagccactgtacagtctaaaatgtcagatgtaaagtgcacatcagtagtcttactctcagttttgcaacaactcagagtagaatcatcatctaaattgtgggctcaatgtgtccagttacacaatgacattctcttagctaaagatactactgaagcctttgaaaaaatggtttcactactttctgttttgctttccatgcagggtgctgtagacataaacaagctttgtgaagaaatgctggacaacagggcaaccttacaagctatagcctcagagtttagttcccttccatcatatgcagcttttgctactgctcaagaagcttatgagcaggctgttgctaatggtgattctgaagttgttcttaaaaagttgaagaagtctttgaatgtggctaaatctgaatttgaccgtgatgcagccatgcaacgtaagttggaaaagatggctgatcaagctatgacccaaatgtataaacaggctagatctgaggacaagagggcaaaagttactagtgctatgcagacaatgcttttcactatgcttagaaagttggataatgatgcactcaacaacattatcaacaatgcaagagatggttgtgttcccttgaacataatacctcttacaacagcagccaaactaatggttgtcataccagactataacacatataaaaatacgtgtgatggtacaacatttacttatgcatcagcattgtgggaaatccaacaggttgtagatgcagatagtaaaattgttcaacttagtgaaattagtatggacaattcacctaatttagcatggcctcttattgtaacagctttaagggccaattctgctgtcaaattacagaataatgagcttagtcctgttgcactacgacagatgtcttgtgctgccggtactacacaaactgcttgcactgatgacaatgcgttagcttactacaacacaacaaagggaggtaggtttgtacttgcactgttatccgatttacaggatttgaaatgggctagattccctaagagtgatggaactggtactatctatacagaactggaaccaccttgtaggtttgttacagacacacctaaaggtcctaaagtgaagtatttatactttattaaaggattaaacaacctaaatagaggtatggtacttggtagtttagctgccacagtacgtctacaagctggtaatgcaacagaagtgcctgccaattcaactgtattatctttctgtgcttttgctgtagatgctgctaaagcttacaaagattatctagctagtgggggacaaccaatcactaattgtgttaagatgttgtgtacacacactggtactggtcaggcaataacagttacaccggaagccaatatggatcaagaatcctttggtggtgcatcgtgttgtctgtactgccgttgccacatagatcatccaaatcctaaaggattttgtgacttaaaaggtaagtatgtacaaatacctacaacttgtgctaatgaccctgtgggttttacacttaaaaacacagtctgtaccgtctgcggtatgtggaaaggttatggctgtagttgtgatcaactccgcgaacccatgcttcagtcagctgatgcacaatcgtttttaaacgggtttgcggtgtaagtgcagcccgtcttacaccgtgcggcacaggcactagtactgatgtcgtatacagggcttttgacatctacaatgataaagtagctggttttgctaaattcctaaaaactaattgttgtcgcttccaagaaaaggacgaagatgacaatttaattgattcttactttgtagttaagagacacactttctctaactaccaacatgaagaaacaatttataatttacttaaggattgtccagctgttgctaaacatgacttctttaagtttagaatagacggtgacatggtaccacatatatcacgtcaacgtcttactaaatacacaatggcagacctcgtctatgctttaaggcattttgatgaaggtaattgtgacacattaaaagaaatacttgtcacatacaattgttgtgatgatgattatttcaataaaaaggactggtatgattttgtagaaaacccagatatattacgcgtatacgccaacttaggtgaacgtgtacgccaagctttgttaaaaacagtacaattctgtgatgccatgcgaaatgctggtattgttggtgtactgacattagataatcaagatctcaatggtaactggtatgatttcggtgatttcatacaaaccacgccaggtagtggagttcctgttgtagattcttattattcattgttaatgcctatattaaccttgaccagggctttaactgcagagtcacatgttgacactgacttaacaaagccttacattaagtgggatttgttaaaatatgacttcacggaagagaggttaaaactctttgaccgttattttaaatattgggatcagacataccacccaaattgtgttaactgtttggatgacagatgcattctgcattgtgcaaactttaatgttttattctctacagtgttcccacctacaagttttggaccactagtgagaaaaatatttgttgatggtgttccatttgtagtttcaactggataccacttcagagagctaggtgttgtacataatcaggatgtaaacttacatagctctagacttagttttaaggaattacttgtgtatgctgctgaccctgctatgcacgctgcttctggtaatctattactagataaacgcactacgtgcttttcagtagctgcacttactaacaatgttgcttttcaaactgtcaaacccggtaattttaacaaagacttctatgactttgctgtgtctaagggtttctttaaggaaggaagttctgttgaattaaaacacttcttctttgctcaggatggtaatgctgctatcagcgattatgactactatcgttataatctaccaacaatgtgtgatatcagacaactactatttgtagttgaagttgttgataagtactttgattgttacgatggtggctgtattaatgctaaccaagtcatcgtcaacaacctagacaaatcagctggttttccatttaataaatggggtaaggctagactttattatgattcaatgagttatgaggatcaagatgcacttttcgcatatacaaaacgtaatgtcatccctactataactcaaatgaatcttaagtatgccattagtgcaaagaatagagctcgcaccgtagctggtgtctctatctgtagtactatgaccaatagacagtttcatcaaaaattattgaaatcaatagccgccactagaggagctactgtagtaattggaacaagcaaattctatggtggttggcacaacatgttaaaaactgtttatagtgatgtagaaaaccctcaccttatgggttgggattatcctaaatgtgatagagccatgcctaacatgcttagaattatggcctcacttgttcttgctcgcaaacatacaacgtgttgtagcttgtcacaccgtttctatagattagctaatgagtgtgctcaagtattgagtgaaatggtcatgtgtggcggttcactatatgttaaaccaggtggaacctcatcaggagatgccacaactgcttatgctaatagtgtttttaacatttgtcaagctgtcacggccaatgttaatgcacttttatctactgatggtaacaaaattgccgataagtatgtccgcaatttacaacacagactttatgagtgtctctatagaaatagagatgttgacacagactttgtgaatgagttttacgcatatttgcgtaaacatttctcaatgatgatactctctgacgatgctgttgtgtgtttcaatagcacttatgcatctcaaggtctagtggctagcataaagaactttaagtcagttctttattatcaaaacaatgtttttatgtctgaagcaaaatgttggactgagactgaccttactaaaggacctcatgaattttgctctcaacatacaatgctagttaaacagggtgatgattatgtgtaccttccttacccagatccatcaagaatcctaggggccggctgttttgtagatgatatcgtaaaaacagatggtacacttatgattgaacggttcgtgtctttagctatagatgcttacccacttactaaacatcctaatcaggagtatgctgatgtctttcatttgtacttacaatacataagaaagctacatgatgagttaacaggacacatgttagacatgtattctgttatgcttactaatgataacacttcaaggtattgggaacctgagttttatgaggctatgtacacaccgcatacagtcttacaggctgttggggcttgtgttctttgcaattcacagacttcattaagatgtggtgcttgcatacgtagaccattcttatgttgtaaatgctgttacgaccatgtcatatcaacatcacataaattagtcttgtctgttaatccgtatgtttgcaatgctccaggttgtgatgtcacagatgtgactcaactttacttaggaggtatgagctattattgtaaatcacataaaccacccattagttttccattgtgtgctaatggacaagtttttggtttatataaaaatacatgtgttggtagcgataatgttactgactttaatgcaattgcaacatgtgactggacaaatgctggtgattacattttagctaacacctgtactgaaagactcaagctttttgcagcagaaacgctcaaagctactgaggagacatttaaactgtcttatggtattgctactgtacgtgaagtgctgtctgacagagaattacatctttcatgggaagttggtaaacctagaccaccacttaaccgaaattatgtctttactggttatcgtgtaactaaaaacagtaaagtacaaataggagagtacacctttgaaaaaggtgactatggtgatgctgttgtttaccgaggtacaacaacttacaaattaaatgttggtgattattttgtgctgacatcacatacagtaatgccattaagtgcacctacactagtgccacaagagcactatgttagaattactggcttatacccaacactcaatatctcagatgagttttctagcaatgttgcaaattatcaaaaggttggtatgcaaaagtattctacactccagggaccacctggtactggtaagagtcattttgctattggcctagctctctactacccttctgctcgcatagtgtatacagcttgctctcatgccgctgttgatgcactatgtgagaaggcattaaaatatttgcctatagataaatgtagtagaattatacctgcacgtgctcgtgtagagtgttttgataaattcaaagtgaattcaacattagaacagtatgtcttttgtactgtaaatgcattgcctgagacgacagcagatatagttgtctttgatgaaatttcaatggccacaaattatgatttgagtgttgtcaatgccagattacgtgctaagcactatgtgtacattggcgaccctgctcaattacctgcaccacgcacattgctaactaagggcacactagaaccagaatatttcaattcagtgtgtagacttatgaaaactataggtccagacatgttcctcggaacttgtcggcgttgtcctgctgaaattgttgacactgtgagtgctttggtttatgataataagcttaaagcacataaagacaaatcagctcaatgctttaaaatgttttataagggtgttatcacgcatgatgtttcatctgcaattaacaggccacaaataggcgtggtaagagaattccttacacgtaaccctgcttggagaaaagctgtctttatttcaccttataattcacagaatgctgtagcctcaaagattttgggactaccaactcaaactgttgattcatcacagggctcagaatatgactatgtcatattcactcaaaccactgaaacagctcactcttgtaatgtaaacagatttaatgttgctattaccagagcaaaagtaggcatactttgcataatgtctgatagagacctttatgacaagttgcaatttacaagtcttgaaattccacgtaggaatgtggcaactttacaagctgaaaatgtaacaggactctttaaagattgtagtaaggtaatcactgggttacatcctacacaggcacctacacacctcagtgttgacactaaattcaaaactgaaggtttatgtgttgacatacctggcatacctaaggacatgacctatagaagactcatctctatgatgggttttaaaatgaattatcaagttaatggttaccctaacatgtttatcacccgcgaagaagctataagacatgtacgtgcatggattggcttcgatgtcgaggggtgtcatgctactagagaagctgttggtaccaatttacctttacagctaggtttttctacaggtgttaacctagttgctgtacctacaggttatgttgatacacctaataatacagatttttccagagttagtgctaaaccaccgcctggagatcaatttaaacacctcataccacttatgtacaaaggacttccttggaatgtagtgcgtataaagattgtacaaatgttaagtgacacacttaaaaatctctctgacagagtcgtatttgtcttatgggcacatggctttgagttgacatctatgaagtattttgtgaaaataggacctgagcgcacctgttgtctatgtgatagacgtgccacatgcttttccactgcttcagacacttatgcctgttggcatcattctattggatttgattacgtctataatccgtttatgattgatgttcaacaatggggttttacaggtaacctacaaagcaaccatgatctgtattgtcaagtccatggtaatgcacatgtagctagttgtgatgcaatcatgactaggtgtctagctgtccacgagtgctttgttaagcgtgttgactggactattgaatatcctataattggtgatgaactgaagattaatgcggcttgtagaaaggttcaacacatggttgttaaagctgcattattagcagacaaattcccagttcttcacgacattggtaaccctaaagctattaagtgtgtacctcaagctgatgtagaatggaagttctatgatgcacagccttgtagtgacaaagcttataaaatagaagaattattctattcttatgccacacattctgacaaattcacagatggtgtatgcctattttggaattgcaatgtcgatagatatcctgctaattccattgtttgtagatttgacactagagtgctatctaaccttaacttgcctggttgtgatggtggcagtttgtatgtaaataaacatgcattccacacaccagcttttgataaaagtgcttttgttaatttaaaacaattaccatttttctattactctgacagtccatgtgagtctcatggaaaacaagtagtgtcagatatagattatgtaccactaaagtctgctacgtgtataacacgttgcaatttaggtggtgctgtctgtagacatcatgctaatgagtacagattgtatctcgatgcttataacatgatgatctcagctggctttagcttgtgggtttacaaacaatttgatacttataacctctggaacacttttacaagacttcagagtttagaaaatgtggcttttaatgttgtaaataagggacactttgatggacaacagggtgaagtaccagtttctatcattaataacactgtttacacaaaagttgatggtgttgatgtagaattgtttgaaaataaaacaacattacctgttaatgtagcatttgagctttgggctaagcgcaacattaaaccagtaccagaggtgaaaatactcaataatttgggtgtggacattgctgctaatactgtgatctgggactacaaaagagatgctccagcacatatatctactattggtgtttgttctatgactgacatagccaagaaaccaactgaaacgatttgtgcaccactcactgtcttttttgatggtagagttgatggtcaagtagacttatttagaaatgcccgtaatggtgttcttattacagaaggtagtgttaaaggtttacaaccatctgtgggtcccaaacaagctagtcttaatggagtcacattaattggagaagccgtaaaaacacagttcaattattataagaaagttgatggtgttgtccaacaattacctgaaacttactttactcagagtagaaatttacaagaatttaaacccaggagtcaaatggaaattgatttcttagaattagctatggatgaattcattgaacggtataaattagaaggctatgccttcgaacatatcgtttatggagattttagtcatagtcagttaggtggtttacatctactgattggactagctaaacgttttaaggaatcaccttttgaattagaagattttattcctatggacagtacagttaaaaactatttcataacagatgcgcaaacaggttcatctaagtgtgtgtgttctgttattgatttattacttgatgattttgttgaaataataaaatcccaagatttatctgtagtttctaaggttgtcaaagtgactattgactatacagaaatttcatttatgctttggtgtaaagatggccatgtagaaacattttacccaaaattacaatctagtcaagcgtggcaaccgggtgttgctatgcctaatctttacaaaatgcaaagaatgctattagaaaagtgtgaccttcaaaattatggtgatagtgcaacattacctaaaggcataatgatgaatgtcgcaaaatatactcaactgtgtcaatatttaaacacattaacattagctgtaccctataatatgagagttatacattttggtgctggttctgataaaggagttgcaccaggtacagctgttttaagacagtggttgcctacgggtacgctgcttgtcgattcagatcttaatgactttgtctctgatgcagattcaactttgattggtgattgtgcaactgtacatacagctaataaatgggatctcattattagtgatatgtacgaccctaagactaaaaatgttacaaaagaaaatgactctaaagagggttttttcacttacatttgtgggtttatacaacaaaagctagctcttggaggttccgtggctataaagataacagaacattcttggaatgctgatctttataagctcatgggacacttcgcatggtggacagcctttgttactaatgtgaatgcgtcatcatctgaagcatttttaattggatgtaattatcttggcaaaccacgcgaacaaatagatggttatgtcatgcatgcaaattacatattttggaggaatacaaatccaattcagttgtcttcctattctttatttgacatgagtaaatttccccttaaattaaggggtactgctgttatgtctttaaaagaaggtcaaatcaatgatatgattttatctcttcttagtaaaggtagacttataattagagaaaacaacagagttgttatttctagtgatgttcttgttaacaactaaacgaacaatgtttgtttttcttgttttattgccactagtctctagtcagtgtgttaatcttacaaccagaactcaattaccccctgcatacactaattctttcacacgtggtgtttattaccctgacaaagttttcagatcctcagttttacattcaactcaggacttgttcttacctttcttttccaatgttacttggttccatgctatacatgtctctgggaccaatggtactaagaggtttgataaccctgtcctaccatttaatgatggtgtttattttgcttccactgagaagtctaacataataagaggctggatttttggtactactttagattcgaagacccagtccctacttattgttaataacgctactaatgttgttattaaagtctgtgaatttcaattttgtaatgatccatttttgggtgtttattaccacaaaaacaacaaaagttggatggaaagtgagttcagagtttattctagtgcgaataattgcacttttgaatatgtctctcagccttttcttatggaccttgaaggaaaacagggtaatttcaaaaatcttagggaatttgtgtttaagaatattgatggttattttaaaatatattctaagcacacgcctattaatttagtgcgtgatctccctcagggtttttcggctttagaaccattggtagatttgccaataggtattaacatcactaggtttcaaactttacttgctttacatagaagttatttgactcctggtgattcttcttcaggttggacagctggtgctgcagcttattatgtgggttatcttcaacctaggacttttctattaaaatataatgaaaatggaaccattacagatgctgtagactgtgcacttgaccctctctcagaaacaaagtgtacgttgaaatccttcactgtagaaaaaggaatctatcaaacttctaactttagagtccaaccaacagaatctattgttagatttcctaatattacaaacttgtgcccttttggtgaagtttttaacgccaccagatttgcatctgtttatgcttggaacaggaagagaatcagcaactgtgttgctgattattctgtcctatataattccgcatcattttccacttttaagtgttatggagtgtctcctactaaattaaatgatctctgctttactaatgtctatgcagattcatttgtaattagaggtgatgaagtcagacaaatcgctccagggcaaactggaaagattgctgattataattataaattaccagatgattttacaggctgcgttatagcttggaattctaacaatcttgattctaaggttggtggtaattataattacctgtatagattgtttaggaagtctaatctcaaaccttttgagagagatatttcaactgaaatctatcaggccggtagcacaccttgtaatggtgttgaaggttttaattgttactttcctttacaatcatatggtttccaacccactaatggtgttggttaccaaccatacagagtagtagtactttcttttgaacttctacatgcaccagcaactgtttgtggacctaaaaagtctactaatttggttaaaaacaaatgtgtcaatttcaacttcaatggtttaacaggcacaggtgttcttactgagtctaacaaaaagtttctgcctttccaacaatttggcagagacattgctgacactactgatgctgtccgtgatccacagacacttgagattcttgacattacaccatgttcttttggtggtgtcagtgttataacaccaggaacaaatacttctaaccaggttgctgttctttatcaggatgttaactgcacagaagtccctgttgctattcatgcagatcaacttactcctacttggcgtgtttattctacaggttctaatgtttttcaaacacgtgcaggctgtttaataggggctgaacatgtcaacaactcatatgagtgtgacatacccattggtgcaggtatatgcgctagttatcagactcagactaattctcctcggcgggcacgtagtgtagctagtcaatccatcattgcctacactatgtcacttggtgcagaaaattcagttgcttactctaataactctattgccatacccacaaattttactattagtgttaccacagaaattctaccagtgtctatgaccaagacatcagtagattgtacaatgtacatttgtggtgattcaactgaatgcagcaatcttttgttgcaatatggcagtttttgtacacaattaaaccgtgctttaactggaatagctgttgaacaagacaaaaacacccaagaagtttttgcacaagtcaaacaaatttacaaaacaccaccaattaaagattttggtggttttaatttttcacaaatattaccagatccatcaaaaccaagcaagaggtcatttattgaagatctacttttcaacaaagtgacacttgcagatgctggcttcatcaaacaatatggtgattgccttggtgatattgctgctagagacctcatttgtgcacaaaagtttaacggccttactgttttgccacctttgctcacagatgaaatgattgctcaatacacttctgcactgttagcgggtacaatcacttctggttggacctttggtgcaggtgctgcattacaaataccatttgctatgcaaatggcttataggtttaatggtattggagttacacagaatgttctctatgagaaccaaaaattgattgccaaccaatttaatagtgctattggcaaaattcaagactcactttcttccacagcaagtgcacttggaaaacttcaagatgtggtcaaccaaaatgcacaagctttaaacacgcttgttaaacaacttagctccaattttggtgcaatttcaagtgttttaaatgatatcctttcacgtcttgacaaagttgaggctgaagtgcaaattgataggttgatcacaggcagacttcaaagtttgcagacatatgtgactcaacaattaattagagctgcagaaatcagagcttctgctaatcttgctgctactaaaatgtcagagtgtgtacttggacaatcaaaaagagttgatttttgtggaaagggctatcatcttatgtccttccctcagtcagcacctcatggtgtagtcttcttgcatgtgacttatgtccctgcacaagaaaagaacttcacaactgctcctgccatttgtcatgatggaaaagcacactttcctcgtgaaggtgtctttgtttcaaatggcacacactggtttgtaacacaaaggaatttttatgaaccacaaatcattactacagacaacacatttgtgtctggtaactgtgatgttgtaataggaattgtcaacaacacagtttatgatcctttgcaacctgaattagactcattcaaggaggagttagataaatattttaagaatcatacatcaccagatgttgatttaggtgacatctctggcattaatgcttcagttgtaaacattcaaaaagaaattgaccgcctcaatgaggttgccaagaatttaaatgaatctctcatcgatctccaagaacttggaaagtatgagcagtatataaaatggccatggtacatttggctaggttttatagctggcttgattgccatagtaatggtgacaattatgctttgctgtatgaccagttgctgtagttgtctcaagggctgttgttcttgtggatcctgctgcaaatttgatgaagacgactctgagccagtgctcaaaggagtcaaattacattacacataaacgaacttatggatttgtttatgagaatcttcacaattggaactgtaactttgaagcaaggtgaaatcaaggatgctactccttcagattttgttcgcgctactgcaacgataccgatacaagcctcactccctttcggatggcttattgttggcgttgcacttcttgctgtttttcagagcgcttccaaaatcataaccctcaaaaagagatggcaactagcactctccaagggtgttcactttgtttgcaacttgctgttgttgtttgtaacagtttactcacaccttttgctcgttgctgctggccttgaagccccttttctctatctttatgctttagtctacttcttgcagagtataaactttgtaagaataataatgaggctttggctttgctggaaatgccgttccaaaaacccattactttatgatgccaactattttctttgctggcatactaattgttacgactattgtataccttacaatagtgtaacttcttcaattgtcattacttcaggtgatggcacaacaagtcctatttctgaacatgactaccagattggtggttatactgaaaaatgggaatctggagtaaaagactgtgttgtattacacagttacttcacttcagactattaccagctgtactcaactcaattgagtacagacactggtgttgaacatgttaccttcttcatctacaataaaattgttgatgagcctgaagaacatgtccaaattcacacaatcgacggttcatccggagttgttaatccagtaatggaaccaatttatgatgaaccgacgacgactactagcgtgcctttgtaagcacaagctgatgagtacgaacttatgtactcattcgtttcggaagagacaggtacgttaatagttaatagcgtacttctttttcttgctttcgtggtattcttgctagttacactagccatccttactgcgcttcgattgtgtgcgtactgctgcaatattgttaacgtgagtcttgtaaaaccttctttttacgtttactctcgtgttaaaaatctgaattcttctagagttcctgatcttctggtctaaacgaactaaatattatattagtttttctgtttggaactttaattttagccatggcagattccaacggtactattaccgttgaagagcttaaaaagctccttgaacaatggaacctagtaataggtttcctattccttacatggatttgtcttctacaatttgcctatgccaacaggaataggtttttgtatataattaagttaattttcctctggctgttatggccagtaactttagcttgttttgtgcttgctgctgtttacagaataaattggatcaccggtggaattgctatcgcaatggcttgtcttgtaggcttgatgtggctcagctacttcattgcttctttcagactgtttgcgcgtacccgttccatgtggtcattcaatccagaaactaacattcttctcaacgtgccactccatggcactattctgaccagaccgcttctagaaagtgaactcgtaatcggagctgtgatccttcgtggacatcttcgtattgctggacaccatctaggacgctgtgacatcaaggacctgcctaaagaaatcactgttgctacatcccgcacgctttcttattacaaattgggagcttcgcagcgtgtagcaggtgactcaggttttgctgcatacagtcgctacaggattggcaactataaattaaacacagaccattccagtagcagtgacaatattgctttgcttgtacagtaagtgacaacagttgttttagatttcatctaaacgaacaaactaaaatgtctgataatggaccccaaaatcagcgaaatgcaccccgcattacgtttggtggaccctcagattcaactggcagtaaccagaatggagaacgcagtggggcgcgatcaaaacaacgtcggccccaaggtttacccaataatactgcgtcttggttcaccgctctcactcaacatggcaaggaagaccttaaattccctcgaggacaaggcgttccaattaacaccaatagcagtccagatgaccaaattggctactaccgaagagctaccagacgaattcgtggtggtgacggtaaaatgaaagatctcagtccaagatggtatttctactacctaggaactgggccagaagctggacttccctatggtgctaacaaagacggcatcatatgggttgcaactgagggagccttgaatacaccaaaagatcacattggcacccgcaatcctgctaacaatgctgcaatcgtgctacaacttcctcaaggaacaacattgccaaaaggcttctacgcagaagggagcagaggcggcagtcaagcctcttctcgttcctcatcacgtagtcgcaacagttcaagaaattcaactccaggcagcagtaggggaacttctcctgctagaatggctggcaatggcggtgatgctgctcttgctttgctgctgcttgacagattgaaccagcttgagagcaaaatgtctggtaaaggccaacaacaacaaggccaaactgtcactaagaaatctgctgctgaggcttctaagaagcctcggcaaaaacgtactgccactaaagcatacaatgtaacacaagctttcggcagacgtggtccagaacaaacccaaggaaattttggggaccaggaactaatcagacaaggaactgattacaaacattggccgcaaattgcacaatttgcccccagcgcttcagcgttcttcggaatgtcgcgcattggcatggaagtcacaccttcgggaacgtggttgacctacacaggtgccatcaaattggatgacaaagatccaaatttcaaagatcaagtcattttgctgaataagcatattgacgcatacaaaacattcccaccaacagagcctaaaaaggacaaaaagaagaaggctgatgaaactcaagccttaccgcagagacagaagaaacagcaaactgtgactcttcttcctgctgcagatttggatgatttctccaaacaattgcaacaatccatgagcagtgctgactcaactcaggcctaaactcatgcagaccacacaaggcagatgggctatataaacgttttcgcttttccgtttacgatatatagtctactcttgtgcagaatgaattctcgtaactacatagcacaagtagatgtagttaactttaatctcacatagcaatctttaatcagtgtgtaacattagggaggacttgaaagagccaccacattttcaccgaggccacgcggagtacgatcgagtgtacagtgaacaatgctagggagagctgcctatatggaagagccctaatgtgtaaaattaattttagtagtgctatccccatgtgattttaatagcttcttaggagaatgacaaaaaaaaaaaaaaaaaaaaaaaaa

SEQ ID NO: 25 - DNA, 836 bp, Coronaviridae
  misc_feature 1..836: note = Fnsp1-D nucleotide sequence: pUC57 sequence (nucleotides 1 to 42) and SARS-CoV-2 nsp1-D sequence (nucleotides 43-836)
  source 1..836: mol_type = other DNA
gaattcgagctcggtacctcgcgaatgcatctagatggatcccgtacgtggctttggagactccgtggaggaggtcttatcagaggcacgtcaacatcttaaagatggcacttgtggcttagtagaagttgaaaaaggcgttttgcctcaacttgaacagccctatgtgttcatcaaacgttcggatgctcgaactgcacctcatggtcatgttatggttgagctggtagcagaactcgaaggcattcagtacggtcgtagtggtgagacacttggtgtccttgtccctcatgtgggcgaaataccagtggcttaccgcaaggttgctggtggccatagttacggcgccgatctaaagtcatttgacttaggcgacgagcttggcactgatccttatgaagattttcaagaaaactggaacactaaacatagcagtggtgttacccgtgaactcatgcgtgagcttaacggaggggcatacactcgctatgtcgataacaacttctgtggccctgatggctaccctcttgagtgcattaaagaccttctagcacgtgctggtaaagcttcatgcactttgtccgaacaactggactttattgacactaagaggggtgtatactgctgccgtgaacatgagcatgaaattgcttggtacacggaacgttctgaaaagagctatgaattgcagacaccttttgaaattaaattggcaaagaaatttgacaccttcaatggggaatgtccaaattttgtatttcccttaaattccataatcaagactattcaaccaagggttgaaaagaaaaagcttgatggctttatgggtagaattc

SEQ ID NO: 26 - DNA, 19 bp, synthetic construct
  misc_feature 1..19: note = Primer
  primer_bind 1..19: note = WH-25155-VS primer
  source 1..19: mol_type = other DNA
tcgatctccaagaacttgg

SEQ ID NO: 27 - DNA, 19 bp, synthetic construct
  misc_feature 1..19: note = Primer
  primer_bind 1..19: note = WH-28957-RS
  source 1..19: mol_type = other DNA
gttcaatctgtcaagcagc

SEQ ID NO: 28 - DNA, 22 bp, synthetic construct
  misc_feature 1..22: note = Primer
  primer_bind 1..22: note = SARS-CoV-2 genomic RNA forward primer
  source 1..22: mol_type = other DNA
gtgaratggtcatgtgtggcgg

SEQ ID NO: 29 - DNA, 26 bp, synthetic construct
  misc_feature 1..26: note = Primer
  primer_bind 1..26: note = SARS-CoV-2 genomic RNA reverse primer
  source 1..26: mol_type = other DNA
caratgttaaasacactattagcata

SEQ ID NO: 30 - DNA, 25 bp, synthetic construct
  misc_feature 1..25: note = Probe
  primer_bind 1..25: note = MGB probe 1
  source 1..25: mol_type = other DNA
caggtggaacctcatcaggagatgc

SEQ ID NO: 31 - DNA, 23 bp, synthetic construct
  misc_feature 1..23: note = Primer
  primer_bind 1..23: note = subgenomic messenger RNA (sgmRNA) N forward primer
  source 1..23: mol_type = other DNA
ccaaccaactttcgatctcttgt

SEQ ID NO: 32 - DNA, 20 bp, synthetic construct
  misc_feature 1..20: note = Primer
  primer_bind 1..20: note = subgenomic messenger RNA (sgmRNA) N reverse primer
  source 1..20: mol_type = other DNA
gggtgcatttcgctgatttt

SEQ ID NO: 33 - DNA, 20 bp, synthetic construct
  misc_feature 1..20: note = Probe
  primer_bind 1..20: note = MGB probe 2
  source 1..20: mol_type = other DNA
ttctctaaacgaacaaacta

SEQ ID NO: 34 - protein, 1273 aa, Coronaviridae
  REGION 1..1273: note = SARS-CoV-2 S protein amino acid sequence, encoded by SEQ ID NO: 4
MFVFLVLLPLVSSQCVNLTTRTQLPPAYTNSFTRGVYYPDKVFRSSVLHSTQDLFLPFFSNVTWFHAIHVSGTNGTKRFDNPVLPFNDGVYFASTEKSNIIRGWIFGTTLDSKTQSLLIVNNATNVVIKVCEFQFCNDPFLGVYYHKNNKSWMESEFRVYSSANNCTFEYVSQPFLMDLEGKQGNFKNLREFVFKNIDGYFKIYSKHTPINLVRDLPQGFSALEPLVDLPIGINITRFQTLLALHRSYLTPGDSSSGWTAGAAAYYVGYLQPRTFLLKYNENGTITDAVDCALDPLSETKCTLKSFTVEKGIYQTSNFRVQPTESIVRFPNITNLCPFGEVFNATRFASVYAWNRKRISNCVADYSVLYNSASFSTFKCYGVSPTKLNDLCFTNVYADSFVIRGDEVRQIAPGQTGKIADYNYKLPDDFTGCVIAWNSNNLDSKVGGNYNYLYRLFRKSNLKPFERDISTEIYQAGSTPCNGVEGFNCYFPLQSYGFQPTNGVGYQPYRVVVLSFELLHAPATVCGPKKSTNLVKNKCVNFNFNGLTGTGVLTESNKKFLPFQQFGRDIADTTDAVRDPQTLEILDITPCSFGGVSVITPGTNTSNQVAVLYQDVNCTEVPVAIHADQLTPTWRVYSTGSNVFQTRAGCLIGAEHVNNSYECDIPIGAGICASYQTQTNSPRRARSVASQSIIAYTMSLGAENSVAYSNNSIAIPTNFTISVTTEILPVSMTKTSVDCTMYICGDSTECSNLLLQYGSFCTQLNRALTGIAVEQDKNTQEVFAQVKQIYKTPPIKDFGGFNFSQILPDPSKPSKRSFIEDLLFNKVTLADAGFIKQYGDCLGDIAARDLICAQKFNGLTVLPPLLTDEMIAQYTSALLAGTITSGWTFGAGAALQIPFAMQMAYRFNGIGVTQNVLYENQKLIANQFNSAIGKIQDSLSSTASALGKLQDVVNQNAQALNTLVKQLSSNFGAISSVLNDILSRLDKVEAEVQIDRLITGRLQSLQTYVTQQLIRAAEIRASANLAATKMSECVLGQSKRVDFCGKGYHLMSFPQSAPHGVVFLHVTYVPAQEKNFTTAPAICHDGKAHFPREGVFVSNGTHWFVTQRNFYEPQIITTDNTFVSGNCDVVIGIVNNTVYDPLQPELDSFKEELDKYFKNHTSPDVDLGDISGINASVVNIQKEIDRLNEVAKNLNESLIDLQELGKYEQYIKWPWYIWLGFIAGLIAIVMVTIMLCCMTSCCSCLKGCCSCGSCCKFDEDDSEPVLKGVKLHYT

SEQ ID NO: 35 - protein, 1273 aa, Coronaviridae; identical to SEQ ID NO: 34
  REGION 1..1273: note = SARS-CoV-2 S protein amino acid sequence, encoded by SEQ ID NO: 5

SEQ ID NO: 36 - DNA, 366 bp, Coronaviridae
  source 1..366: mol_type = genomic DNA
  misc_feature 1..336: note = ORF8 nucleotide sequence
atgaaatttcttgttttcttaggaatcatcacaactgtagctgcatttcaccaagaatgtagtttacagtcatgtactcaacatcaaccatatgtagttgatgacccgtgtcctattcacttctattctaaatggtatattagagtaggagctagaaaatcagcacctttaattgaattgtgcgtggatgaggctggttctaaatcacccattcagtacatcgatatcggtaattatacagtttcctgtttaccttttacaattaattgccaggaacctaaattgggtagtcttgtagtgcgttgttcgttctatgaagactttttagagtatcatgacgttcgtgttgttttagatttcatctaa

SEQ ID NO: 37 - DNA, 186 bp, Coronaviridae
  source 1..186: mol_type = genomic DNA
  misc_feature 1..186: note = ORF 6 nucleotide sequence
atgtttcatctcgttgactttcaggttactatagcagagatattactaattattatgaggacttttaaagtttccatttggaatcttgattacatcataaacctcataattaaaaatttatctaagtcactaactgagaataaatattctcaattagatgaagagcaaccaatggagattgattaa

SEQ ID NO: 38 - DNA, 366 bp, Coronaviridae
  source 1..366: mol_type = genomic DNA
  misc_feature 1..366: note = ORF7a nucleotide sequence
atgaaaattattcttttcttggcactgataacactcgctacttgtgagctttatcactaccaagagtgtgttagaggtacaacagtacttttaaaagaaccttgctcttctggaacatacgagggcaattcaccatttcatcctctagctgataacaaatttgcactgacttgctttagcactcaatttgcttttgcttgtcctgacggcgtaaaacacgtctatcagttacgtgccagatcagtttcacctaaactgttcatcagacaagaggaagttcaagaactttactctccaatttttcttattgttgcggcaatagtgtttataacactttgcttcacactcaaaagaaagacagaatga

SEQ ID NO: 39 - DNA, 132 bp, Coronaviridae
  source 1..132: mol_type = genomic DNA
  misc_feature 1..132: note = ORF7b nucleotide sequence
atgattgaactttcattaattgacttctatttgtgctttttagcctttctgctattccttgttttaattatgcttattatcttttggttctcacttgaactgcaagatcataatgaaacttgtcacgcctaa

SEQ ID NO: 40 - DNA, 5228 bp, Coronaviridae
  source 1..5228: mol_type = genomic DNA
  misc_feature 1..5228: note = F4 with S from Delta VOC
gggtcccaaacaagctagtcttaatggagtcacattaattggagaagccgtaaaaacacagttcaattattataagaaagttgatggtgttgtccaacaattacctgaaacttactttactcagagtagaaatttacaagaatttaaacccaggagtcaaatggaaattgatttcttagaattagctatggatgaattcattgaacggtataaattagaaggctatgccttcgaacatatcgtttatggagattttagtcatagtcagttaggtggtttacatctactgattggactagctaaacgttttaaggaatcaccttttgaattagaagattttattcctatggacagtacagttaaaaactatttcataacagatgcgcaaacaggttcatctaagtgtgtgtgttctgttattgatttattacttgatgattttgttgaaataataaaatcccaagatttatctgtagtttctaaggttgtcaaagtgactattgactatacagaaatttcatttatgctttggtgtaaagatggccatgtagaaacattttacccaaaattacaatctagtcaagcgtggcaaccgggtgttgctatgcctaatctttacaaaatgcaaagaatgctattagaaaagtgtgaccttcaaaattatggtgatagtgcaacattacctaaaggcataatgatgaatgtcgcaaaatatactcaactgtgtcaatatttaaacacattaacattagctgtaccctataatatgagagttatacattttggtgctggttctgataaaggagttgcaccaggtacagctgttttaagacagtggttgcctacgggtacgctgcttgtcgattcagatcttaatgactttgtctctgatgcagattcaactttgattggtgattgtgcaactgtacatacagctaataaatgggatctcattattagtgatatgtacgaccctaagactaaaaatgttacaaaagaaaatgactctaaagagggttttttcacttacatttgtgggtttatacaacaaaagctagctcttggaggttccgtggctataaagataacagaacattcttggaatgctgatctttataagctcatgggacacttcgcatggtggacagcctttgttactaatgtgaatgcgtcatcatctgaagcatttttaattggatgtaattatcttggcaaaccacgcgaacaaatagatggttatgtcatgcatgcaaattacatattttggaggaatacaaatccaattcagttgtcttcctattctttatttgacatgagtaaatttccccttaaattaaggggtactgctgttatgtctttaaaagaaggtcaaatcaatgatatgattttatctcttcttagtaaaggtagacttataattagagaaaacaacagagttgttatttctagtgatgttcttgttaacaactaaacgaacaatgtttgtttttcttgttttattgccactagtctctagtcagtgtgttaatcttagaaccagaactcaattaccccctgcatacactaattctttcacacgtggtgtttattaccctgacaaagttttcagatcctcagttttacattcaactcaggacttgttcttacctttcttttccaatgttacttggttccatgctatacatgtctctgggaccaatggtactaagaggtttgataaccctgtcctaccatttaatgatggtgtttattttgcttccactgagaagtctaacataataagaggctggatttttggtactactttagattcgaagacccagtccctacttattgttaataacgctactaatgttgttattaaagtctgtgaatttcaattttgtaatgatccatttttgggtgtttattaccacaaaaacaacaaaagttggatggaaagtggagtttattctagtgcgaataattgcacttttgaatatgtctctcagccttttcttatggaccttgaaggaaaacagggtaatttcaaaaatcttagggaatttgtgtttaagaatattgatggttattttaaaatatattctaagcacacgcctattaatttagtgcgtgatctccctcagggtttttcggctttagaaccattggtagatttgccaataggtattaacatcactaggtttcaaactttacttgctttacatagaagttatttgactcctggtgattcttcttcaggttggacagctggtgctgcagcttattatgtgggttatcttcaacctaggacttttctattaaaatataatgaaaatggaaccattacagatgctgtagactgtgcacttgaccctctctcagaaacaaagtgtacgttgaaatccttcactgtagaaaaaggaatctatcaaacttctaactttagagtccaaccaacagaatctattgttagatttcctaatattacaaacttgtgcccttttggtgaagtttttaacgccaccagatttgcatctgtttatgcttggaacaggaagagaatcagcaactgtgttgctgattattctgtcctatataattccgcatcattttccacttttaagtgttatggagtgtctcctactaaattaaatgatctctgctttactaatgtctatgcagattcatttgtaattagaggtgatgaagtcagacaaatcgctccagggcaaactggaaagattgctgattataattataaattaccagatgattttacaggctgcgttatagcttggaattctaacaatcttgattctaaggttggtggtaattataattaccggtatagattgtttaggaagtctaatctcaaaccttttgagagagatatttcaactgaaatctatcaggccggtagcaaaccttgtaatggtgttgaaggttttaattgttactttcctttacaatcatatggtttccaacccactaatggtgttggttaccaaccatacagagtagtagtactttcttttgaacttctacatgcaccagcaactgtttgtggacctaaaaagtctactaatttggttaaaaacaaatgtgtcaatttcaacttcaatggtttaacaggcacaggtgttcttactgagtctaacaaaaagtttctgcctttccaacaatttggcagagacattgctgacactactgatgctgtccgtgatccacagacacttgagattcttgacattacaccatgttcttttggtggtgtcagtgttataacaccaggaacaaatacttctaaccaggttgctgttctttatcagggtgttaactgcacagaagtccctgttgctattcatgcagatcaacttactcctacttggcgtgtttattctacaggttctaatgtttttcaaacacgtgcaggctgtttaataggggctgaacatgtcaacaactcatatgagtgtgacatacccattggtgcaggtatatgcgctagttatcagactcagactaattctcgtcggcgggcacgtagtgtagctagtcaatccatcattgcctacactatgtcacttggtgcagaaaattcagttgcttactctaataactctattgccatacccacaaattttactattagtgttaccacagaaattctaccagtgtctatgaccaagacatcagtagattgtacaatgtacatttgtggtgattcaactgaatgcagcaatcttttgttgcaatatggcagtttttgtacacaattaaaccgtgctttaactggaatagctgttgaacaagacaaaaacacccaagaagtttttgcacaagtcaaacaaatttacaaaacaccaccaattaaagattttggtggttttaatttttcacaaatattaccagatccatcaaaaccaagcaagaggtcatttattgaagatctacttttcaacaaagtgacacttgcagatgctggcttcatcaaacaatatggtgattgccttggtgatattgctgctagagacctcatttgtgcacaaaagtttaacggccttactgttttgccacctttgctcacagatgaaatgattgctcaatacacttctgcactgttagcgggtacaatcacttctggttggacctttggtgcaggtgctgcattacaaataccatttgctatgcaaatggcttataggtttaatggtattggagttacacagaatgttctctatgagaaccaaaaattgattgccaaccaatttaatagtgctattggcaaaattcaagactcactttcttccacagcaagtgcacttggaaaacttcaaaatgtggtcaaccaaaatgcacaagctttaaacacgcttgttaaacaacttagctccaattttggtgcaatttcaagtgttttaaatgatatcctttcacgtcttgacaaagttgaggctgaagtgcaaattgataggttgatcacaggcagacttcaaagtttgcagacatatgtgactcaacaattaattagagctgcagaaatcagagcttctgctaatcttgctgctactaaaatgtcagagtgtgtacttggacaatcaaaaagagttgatttttgtggaaagggctatcatcttatgtccttccctcagtcagcacctcatggtgtagtcttcttgcatgtgacttatgtccctgcacaagaaaagaacttcacaactgctcctgccatttgtcatgatggaaaagcacactttcctcgtgaaggtgtctttgtttcaaatggcacacactggtttgtaacacaaaggaatttttatgaaccacaaatcattactacagacaacacatttgtgtctggtaactgtgatgttgtaataggaattgtcaacaacacagtttatgatcctttgcaacctgaattagactcattcaaggaggagttagataaatattttaagaatcatacatcaccagatgttgatttaggtgacatctctggcattaatgcttcagttgtaaacattcaaaaagaaattgaccgcctcaatgaggttgccaagaatttaaatgaatctctcatcgatctccaagaacttggaaagtatgagcagtatataaaatggccatggtacatttggctaggttttatagctggcttgattgccatagtaatggtgacaattatgctttgctgtatgaccagttgctgtagttgtctcaagggctgttgttcttgtggatcc

SEQ ID NO: 41 - DNA, 5216 bp, Coronaviridae
  source 1..5216: mol_type = genomic DNA
  misc_feature 1..5216: note = F4 with S from Omicron VOC
gggtcccaaacaagctagtcttaatggagtcacattaattggagaagccgtaaaaacacagttcaattattataagaaagttgatggtgttgtccaacaattacctgaaacttactttactcagagtagaaatttacaagaatttaaacccaggagtcaaatggaaattgatttcttagaattagctatggatgaattcattgaacggtataaattagaaggctatgccttcgaacatatcgtttatggagattttagtcatagtcagttaggtggtttacatctactgattggactagctaaacgttttaaggaatcaccttttgaattagaagattttattcctatggacagtacagttaaaaactatttcataacagatgcgcaaacaggttcatctaagtgtgtgtgttctgttattgatttattacttgatgattttgttgaaataataaaatcccaagatttatctgtagtttctaaggttgtcaaagtgactattgactatacagaaatttcatttatgctttggtgtaaagatggccatgtagaaacattttacccaaaattacaatctagtcaagcgtggcaaccgggtgttgctatgcctaatctttacaaaatgcaaagaatgctattagaaaagtgtgaccttcaaaattatggtgatagtgcaacattacctaaaggcataatgatgaatgtcgcaaaatatactcaactgtgtcaatatttaaacacattaacattagctgtaccctataatatgagagttatacattttggtgctggttctgataaaggagttgcaccaggtacagctgttttaagacagtggttgcctacgggtacgctgcttgtcgattcagatcttaatgactttgtctctgatgcagattcaactttgattggtgattgtgcaactgtacatacagctaataaatgggatctcattattagtgatatgtacgaccctaagactaaaaatgttacaaaagaaaatgactctaaagagggttttttcacttacatttgtgggtttatacaacaaaagctagctcttggaggttccgtggctataaagataacagaacattcttggaatgctgatctttataagctcatgggacacttcgcatggtggacagcctttgttactaatgtgaatgcgtcatcatctgaagcatttttaattggatgtaattatcttggcaaaccacgcgaacaaatagatggttatgtcatgcatgcaaattacatattttggaggaatacaaatccaattcagttgtcttcctattctttatttgacatgagtaaatttccccttaaattaaggggtactgctgttatgtctttaaaagaaggtcaaatcaatgatatgattttatctcttcttagtaaaggtagacttataattagagaaaacaacagagttgttatttctagtgatgttcttgttaacaactaaacgaacaatgtttgtttttcttgttttattgccactagtctctagtcagtgtgttaatcttacaaccagaactcaattaccccctgcatacactaattctttcacacgtggtgtttattaccctgacaaagttttcagatcctcagttttacattcaactcaggacttgttcttacctttcttttccaatgttacttggttccatgttatatctgggaccaatggtactaagaggtttgataaccctgtcctaccatttaatgatggtgtttattttgcttccatagagaagtctaacataataagaggctggatttttggtactactttagattcgaagacccagtccctacttattgttaataacgctactaatgttgttattaaagtctgtgaatttcaattttgtaatgatccatttttggaccacaaaaacaacaaaagttggatggaaagtgagttcagagtttattctagtgcgaataattgcacttttgaatatgtctctcagccttttcttatggaccttgaaggaaaacagggtaatttcaaaaatcttagggaatttgtgtttaagaatattgatggttattttaaaatatattctaagcacacgcctattatagtgcgtgatctccctcagggtttttcggctttagaaccattggtagatttgccaataggtattaacatcactaggtttcaaactttacttgctttacatagaagttatttgactcctggtgattcttcttcaggttggacagctggtgctgcagcttattatgtgggttatcttcaacctaggacttttctattaaaatataatgaaaatggaaccattacagatgctgtagactgtgcacttgaccctctctcagaaacaaagtgtacgttgaaatccttcactgtagaaaaaggaatctatcaaacttctaactttagagtccaaccaacagaatctattgttagatttcctaatattacaaacttgtgcccttttgatgaagtttttaacgccaccagatttgcatctgtttatgcttggaacaggaagagaatcagcaactgtgttgctgattattctgtcctatataatctcgcaccatttttcacttttaagtgttatggagtgtctcctactaaattaaatgatctctgctttactaatgtctatgcagattcatttgtaattagaggtgatgaagtcagacaaatcgctccagggcaaactggaaatattgctgattataattataaattaccagatgattttacaggctgcgttatagcttggaattctaacaaacttgattctaaggtttctggtaattataattacctgtatagattgtttaggaagtctaatctcaaaccttttgagagagatatttcaactgaaatctatcaggccggtaacaaaccttgtaatggtgttgcaggttttaattgttactttcctttacgatcatattctttccgacccacttatggtgttggtcaccaaccatacagagtagtagtactttcttttgaacttctacatgcaccagcaactgtttgtggacctaaaaagtctactaatttggttaaaaacaaatgtgtcaatttcaacttcaatggtttaaaaggcacaggtgttcttactgagtctaacaaaaagtttctgcctttccaacaatttggcagagacattgctgacactactgatgctgtccgtgatccacagacacttgagattcttgacattacaccatgttcttttggtggtgtcagtgttataacaccaggaacaaatacttctaaccaggttgctgttctttatcagggtgttaactgcacagaagtccctgttgctattcatgcagatcaacttactcctacttggcgtgtttattctacaggttctaatgtttttcaaacacgtgcaggctgtttaataggggctgaatatgtcaacaactcatatgagtgtgacatacccattggtgcaggtatatgcgctagttatcagactcagactaaatctcatcggcgggcacgtagtgtagctagtcaatccatcattgcctacactatgtcacttggtgcagaaaattcagttgcttactctaataactctattgccatacccacaaattttactattagtgttaccacagaaattctaccagtgtctatgaccaagacatcagtagattgtacaatgtacatttgtggtgattcaactgaatgcagcaatcttttgttgcaatatggcagtttttgtacacaattaaaacgtgctttaactggaatagctgttgaacaagacaaaaacacccaagaagtttttgcacaagtcaaacaaatttacaaaacaccaccaattaaatattttggtggttttaatttttcacaaatattaccagatccatcaaaaccaagcaagaggtcatttattgaagatctacttttcaacaaagtgacacttgcagatgctggcttcatcaaacaatatggtgattgccttggtgatattgctgctagagacctcatttgtgcacaaaagtttaaaggccttactgttttgccacctttgctcacagatgaaatgattgctcaatacacttctgcactgttagcgggtacaatcacttctggttggacctttggtgcaggtgctgcattacaaataccatttgctatgcaaatggcttataggtttaatggtattggagttacacagaatgttctctatgagaaccaaaaattgattgccaaccaatttaatagtgctattggcaaaattcaagactcactttcttccacagcaagtgcacttggaaaacttcaagatgtggtcaaccataatgcacaagctttaaacacgcttgttaaacaacttagctccaaatttggtgcaatttcaagtgttttaaatgatatcttttcacgtcttgacaaagttgaggctgaagtgcaaattgataggttgatcacaggcagacttcaaagtttgcagacatatgtgactcaacaattaattagagctgcagaaatcagagcttctgctaatcttgctgctactaaaatgtcagagtgtgtacttggacaatcaaaaagagttgatttttgtggaaagggctatcatcttatgtccttccctcagtcagcacctcatggtgtagtcttcttgcatgtgacttatgtccctgcacaagaaaagaacttcacaactgctcctgccatttgtcatgatggaaaagcacactttcctcgtgaaggtgtctttgtttcaaatggcacacactggtttgtaacacaaaggaatttttatgaaccacaaatcattactacagacaacacatttgtgtctggtaactgtgatgttgtaataggaattgtcaacaacacagtttatgatcctttgcaacctgaattagactcattcaaggaggagttagataaatattttaagaatcatacatcaccagatgttgatttaggtgacatctctggcattaatgcttcagttgtaaacattcaaaaagaaattgaccgcctcaatgaggttgccaagaatttaaatgaatctctcatcgatctccaagaacttggaaagtatgagcagtatataaaatggccatggtacatttggctaggttttatagctggcttgattgccatagtaatggtgacaattatgctttgctgtatgaccagttgctgtagttgtctcaagggctgttgttcttgtggatcc

SEQ ID NO: 42 - DNA, 28173 bp, Coronaviridae
  source 1..28173: mol_type = other DNA
  misc_feature 1..28173: note = SARS-CoV-2-[3,E,6,7] polynucleotide sequence
attaaaggtttataccttcccaggtaacaaaccaaccaactttcgatctcttgtagatctgttctctaaacgaactttaaaatctgtgtggctgtcactcggctgcatgcttagtgcactcacgcagtataattaataactaattactgtcgttgacaggacacgagtaactcgtctatcttctgcaggctgcttacggtttcgtccgtgttgcagccgatcatcagcacatctaggtttcgtccgggtgtgaccgaaaggtaagatggagagccttgtccctggtttcaacgagaaaacacacgtccaactcagtttgcctgttttacaggttcgcgacgtgctcgtacgtggctttggagactccgtggaggaggtcttatcagaggcacgtcaacatcttaaagatggcacttgtggcttagtagaagttgaaaaaggcgttttgcctcaacttgaacagccctatgtgttcatcaaacgttcggatgctcgaactgcacctcatggtcatgttatggttgagctggtagcagaactcgaaggcattcagtacggtcgtagtggtgagacacttggtgtccttgtccctcatgtgggcgaaataccagtggcttaccgcaaggttcttcttcgtaagaacggtaataaaggagctggtggccatagttacggcgccgatctaaagtcatttgacttaggcgacgagcttggcactgatccttatgaagattttcaagaaaactggaacactaaacatagcagtggtgttacccgtgaactcatgcgtgagcttaacggaggggcatacactcgctatgtcgataacaacttctgtggccctgatggctaccctcttgagtgcattaaagaccttctagcacgtgctggtaaagcttcatgcactttgtccgaacaactggactttattgacactaagaggggtgtatactgctgccgtgaacatgagcatgaaattgcttggtacacggaacgttctgaaaagagctatgaattgcagacaccttttgaaattaaattggcaaagaaatttgacaccttcaatggggaatgtccaaattttgtatttcccttaaattccataatcaagactattcaaccaagggttgaaaagaaaaagcttgatggctttatgggtagaattcgatctgtctatccagttgcgtcaccaaatgaatgcaaccaaatgtgcctttcaactctcatgaagtgtgatcattgtggtgaaacttcatggcagacgggcgattttgttaaagccacttgcgaattttgtggcactgagaatttgactaaagaaggtgccactacttgtggttacttaccccaaaatgctgttgttaaaatttattgtccagcatgtcacaattcagaagtaggacctgagcatagtcttgccgaataccataatgaatctggcttgaaaaccattcttcgtaagggtggtcgcactattgcctttggaggctgtgtgttctcttatgttggttgccataacaagtgtgcctattgggttccacgtgctagcgctaacataggttgtaaccatacaggtgttgttggagaaggttccgaaggtcttaatgacaaccttcttgaaatactccaaaaagagaaagtcaacatcaatattgttggtgactttaaacttaatgaagagatcgccattattttggcatctttttctgcttccacaagtgcttttgtggaaactgtgaaaggtttggattataaagcattcaaacaaattgttgaatcctgtggtaattttaaagttacaaaaggaaaagctaaaaaaggtgcctggaatattggtgaacagaaatcaatactgagtcctctttatgcatttgcatcagaggctgctcgtgttgtacgatcaattttctcccgcactcttgaaactgctcaaaattctgtgcgtgttttacagaaggccgctataacaatactagatggaatttcacagtattcactgagactcattgatgctatgatgttcacatctgatttggctactaacaatctagttgtaatggcctacattacaggtggtgttgttcagttgacttcgcagtggctaactaacatctttggcactgtttatgaaaaactcaaacccgtccttgattggcttgaagagaagtttaaggaaggtgtagagtttcttagagacggttgggaaattgttaaatttatctcaacctgtgcttgtgaaattgtcggtggacaaattgtcacctgtgcaaaggaaattaaggagagtgttcagacattctttaagcttgtaaataaatttttggctttgtgtgctgactctatcattattggtggagctaaacttaaagccttgaatttaggtgaaacatttgtcacgcactcaaagggattgtacagaaagtgtgttaaatccagagaagaaactggcctactcatgcctctaaaagccccaaaagaaattatcttcttagagggagaaacacttcccacagaagtgttaacagaggaagttgtcttgaaaactggtgatttacaaccattagaacaacctactagtgaagctgttgaagctccattggttggtacaccagtttgtattaacgggcttatgttgctcgaaatcaaagacacagaaaagtactgtgcccttgcacctaatatgatggtaacaaacaataccttcacactcaaaggcggtgcaccaacaaaggttacttttggtgatgacactgtgatagaagtgcaaggttacaagagtgtgaatatcacttttgaacttgatgaaaggattgataaagtacttaatgagaagtgctctgcctatacagttgaactcggtacagaagtaaatgagttcgcctgtgttgtggcagatgctgtcataaaaactttgcaaccagtatctgaattacttacaccactgggcattgatttagatgagtggagtatggctacatactacttatttgatgagtctggtgagtttaaattggcttcacatatgtattgttctttctaccctccagatgaggatgaagaagaaggtgattgtgaagaagaagagtttgagccatcaactcaatatgagtatggtactgaagatgattaccaaggtaaacctttggaatttggtgccacttctgctgctcttcaacctgaagaagagcaagaagaagattggttagatgatgatagtcaacaaactgttggtcaacaagacggcagtgaggacaatcagacaactactattcaaacaattgttgaggttcaacctcaattagagatggaacttacaccagttgttcagactattgaagtgaatagttttagtggttatttaaaacttactgacaatgtatacattaaaaatgcagacattgtggaagaagctaaaaaggtaaaaccaacagtggttgttaatgcagccaatgtttaccttaaacatggaggaggtgttgcaggagccttaaataaggctactaacaatgccatgcaagttgaatctgatgattacatagctactaatggaccacttaaagtgggtggtagttgtgttttaagcggacacaatcttgctaaacactgtcttcatgttgtcggcccaaatgttaacaaaggtgaagacattcaacttcttaagagtgcttatgaaaattttaatcagcacgaagttctacttgcaccattattatcagctggtatttttggtgctgaccctatacattctttaagagtttgtgtagatactgttcgcacaaatgtctacttagctgtctttgataaaaatctctatgacaaacttgtttcaagctttttggaaatgaagagtgaaaagcaagttgaacaaaagatcgctgagattcctaaagaggaagttaagccatttataactgaaagtaaaccttcagttgaacagagaaaacaagatgataagaaaatcaaagcttgtgttgaagaagttacaacaactctggaagaaactaagttcctcacagaaaacttgttactttatattgacattaatggcaatcttcatccagattctgccactcttgttagtgacattgacatcactttcttaaagaaagatgctccatatatagtgggtgatgttgttcaagagggtgttttaactgctgtggttatacctactaaaaaggctggtggcactactgaaatgctagcgaaagctttgagaaaagtgccaacagacaattatataaccacttacccgggtcagggtttaaatggttacactgtagaggaggcaaagacagtgcttaaaaagtgtaaaagtgccttttacattctaccatctattatctctaatgagaagcaagaaattcttggaactgtttcttggaatttgcgagaaatgcttgcacatgcagaagaaacacgcaaattaatgcctgtctgtgtggaaactaaagccatagtttcaactatacagcgtaaatataagggtattaaaatacaagagggtgtggttgattatggtgctagattttacttttacaccagtaaaacaactgtagcgtcacttatcaacacacttaacgatctaaatgaaactcttgttacaatgccacttggctatgtaacacatggcttaaatttggaagaagctgctcggtatatgagatctctcaaagtgccagctacagtttctgtttcttcacctgatgctgttacagcgtataatggttatcttacttcttcttctaaaacacctgaagaacattttattgaaaccatctcacttgctggttcctataaagattggtcctattctggacaatctacacaactaggtatagaatttcttaagagaggtgataaaagtgtatattacactagtaatcctaccacattccacctagatggtgaagttatcacctttgacaatcttaagacacttctttctttgagagaagtgaggactattaaggtgtttacaacagtagacaacattaacctccacacgcaagttgtggacatgtcaatgacatatggacaacagtttggtccaacttatttggatggagctgatgttactaaaataaaacctcataattcacatgaaggtaaaacattttatgttttacctaatgatgacactctacgtgttgaggcttttgagtactaccacacaactgatcctagttttctgggtaggtacatgtcagcattaaatcacactaaaaagtggaaatacccacaagttaatggtttaacttctattaaatgggcagataacaactgttatcttgccactgcattgttaacactccaacaaatagagttgaagtttaatccacctgctctacaagatgcttattacagagcaagggctggtgaagctgctaacttttgtgcacttatcttagcctactgtaataagacagtaggtgagttaggtgatgttagagaaacaatgagttacttgtttcaacatgccaatttagattcttgcaaaagagtcttgaacgtggtgtgtaaaacttgtggacaacagcagacaacccttaagggtgtagaagctgttatgtacatgggcacactttcttatgaacaatttaagaaaggtgttcagataccttgtacgtgtggtaaacaagctacaaaatatctagtacaacaggagtcaccttttgttatgatgtcagcaccacctgctcagtatgaacttaagcatggtacatttacttgtgctagtgagtacactggtaattaccagtgtggtcactataaacatataacttctaaagaaactttgtattgcatagacggtgctttacttacaaagtcctcagaatacaaaggtcctattacggatgttttctacaaagaaaacagttacacaacaaccataaaaccagttacttataaattggatggtgttgtttgtacagaaattgaccctaagttggacaattattataagaaagacaattcttatttcacagagcaaccaattgatcttgtaccaaaccaaccatatccaaacgcaagcttcgataattttaagtttgtatgtgataatatcaaatttgctgatgatttaaaccagttaactggttataagaaacctgcttcaagagagcttaaagttacatttttccctgacttaaatggtgatgtggtggctattgattataaacactacacaccctcttttaagaaaggagctaaattgttacataaacctattgtttggcatgttaacaatgcaactaataaagccacgtataaaccaaatacctggtgtatacgttgtctttggagcacaaaaccagttgaaacatcaaattcgtttgatgtactgaagtcagaggacgcgcagggaatggataatcttgcctgcgaagatctaaaaccagtctctgaagaagtagtggaaaatcctaccatacagaaagacgttcttgagtgtaatgtgaaaactaccgaagttgtaggagacattatacttaaaccagcaaataatagtttaaaaattacagaagaggttggccacacagatctaatggctgcttatgtagacaattctagtcttactattaagaaacctaatgaattatctagagtattaggtttgaaaacccttgctactcatggtttagctgctgttaatagtgtcccttgggatactatagctaattatgctaagccttttcttaacaaagttgttagtacaactactaacatagttacacggtgtttaaaccgtgtttgtactaattatatgccttatttctttactttattgctacaattgtgtacttttactagaagtacaaattctagaattaaagcatctatgccgactactatagcaaagaatactgttaagagtgtcggtaaattttgtctagaggcttcatttaattatttgaagtcacctaatttttctaaactgataaatattataatttggtttttactattaagtgtttgcctaggttctttaatctactcaaccgctgctttaggtgttttaatgtctaatttaggcatgccttcttactgtactggttacagagaaggctatttgaactctactaatgtcactattgcaacctactgtactggttctataccttgtagtgtttgtcttagtggtttagattctttagacacctatccttctttagaaactatacaaattaccatttcatcttttaaatgggatttaactgcttttggcttagttgcagagtggtttttggcatatattcttttcactaggtttttctatgtacttggattggctgcaatcatgcaattgtttttcagctattttgcagtacattttattagtaattcttggcttatgtggttaataattaatcttgtacaaatggccccgatttcagctatggttagaatgtacatcttctttgcatcattttattatgtatggaaaagttatgtgcatgttgtagacggttgtaattcatcaacttgtatgatgtgttacaaacgtaatagagcaacaagagtcgaatgtacaactattgttaatggtgttagaaggtccttttatgtctatgctaatggaggtaaaggcttttgcaaactacacaattggaattgtgttaattgtgatacattctgtgctggtagtacatttattagtgatgaagttgcgagagacttgtcactacagtttaaaagaccaataaatcctactgaccagtcttcttacatcgttgatagtgttacagtgaagaatggttccatccatctttactttgataaagctggtcaaaagacttatgaaagacattctctctctcattttgttaacttagacaacctgagagctaataacactaaaggttcattgcctattaatgttatagtttttgatggtaaatcaaaatgtgaagaatcatctgcaaaatcagcgtctgtttactacagtcagcttatgtgtcaacctatactgttactagatcaggcattagtgtctgatgttggtgatagtgcggaagttgcagttaaaatgtttgatgcttacgttaatacgttttcatcaacttttaacgtaccaatggaaaaactcaaaacactagttgcaactgcagaagctgaacttgcaaagaatgtgtccttagacaatgtcttatctacttttatttcagcagctcggcaagggtttgttgattcagatgtagaaactaaagatgttgttgaatgtcttaaattgtcacatcaatctgacatagaagttactggcgatagttgtaataactatatgctcacctataacaaagttgaaaacatgacaccccgtgaccttggtgcttgtattgactgtagtgcgcgtcatattaatgcgcaggtagcaaaaagtcacaacattgctttgatatggaacgttaaagatttcatgtcattgtctgaacaactacgaaaacaaatacgtagtgctgctaaaaagaataacttaccttttaagttgacatgtgcaactactagacaagttgttaatgttgtaacaacaaagatagcacttaagggtggtaaaattgttaataattggttgaagcagttaattaaagttacacttgtgttcctttttgttgctgctattttctatttaataacacctgttcatgtcatgtctaaacatactgacttttcaagtgaaatcataggatacaaggctattgatggtggtgtcactcgtgacatagcatctacagatacttgttttgctaacaaacatgctgattttgacacatggtttagccagcgtggtggtagttatactaatgacaaagcttgcccattgattgctgcagtcataacaagagaagtgggttttgtcgtgcctggtttgcctggcacgatattacgcacaactaatggtgactttttgcatttcttacctagagtttttagtgcagttggtaacatctgttacacaccatcaaaacttatagagtacactgactttgcaacatcagcttgtgttttggctgctgaatgtacaatttttaaagatgcttctggtaagccagtaccatattgttatgataccaatgtactagaaggttctgttgcttatgaaagtttacgccctgacacacgttatgtgctcatggatggctctattattcaatttcctaacacctaccttgaaggttctgttagagtggtaacaacttttgattctgagtactgtaggcacggcacttgtgaaagatcagaagctggtgtttgtgtatctactagtggtagatgggtacttaacaatgattattacagatctttaccaggagttttctgtggtgtagatgctgtaaatttacttactaatatgtttacaccactaattcaacctattggtgctttggacatatcagcatctatagtagctggtggtattgtagctatcgtagtaacatgccttgcctactattttatgaggtttagaagagcttttggtgaatacagtcatgtagttgcctttaatactttactattccttatgtcattcactgtactctgtttaacaccagtttactcattcttacctggtgtttattctgttatttacttgtacttgacattttatcttactaatgatgtttcttttttagcacatattcagtggatggttatgttcacacctttagtacctttctggataacaattgcttatatcatttgtatttccacaaagcatttctattggttctttagtaattacctaaagagacgtgtagtctttaatggtgtttcctttagtacttttgaagaagctgcgctgtgcacctttttgttaaataaagaaatgtatctaaagttgcgtagtgatgtgctattacctcttacgcaatataatagatacttagctctttataataagtacaagtattttagtggagcaatggatacaactagctacagagaagctgcttgttgtcatctcgcaaaggctctcaatgacttcagtaactcaggttctgatgttctttaccaaccaccacaaacctctatcacctcagctgttttgcagagtggttttagaaaaatggcattcccatctggtaaagttgagggttgtatggtacaagtaacttgtggtacaactacacttaacggtctttggcttgatgacgtagtttactgtccaagacatgtgatctgcacctctgaagacatgcttaaccctaattatgaagatttactcattcgtaagtctaatcataatttcttggtacaggctggtaatgttcaactcagggttattggacattctatgcaaaattgtgtacttaagcttaaggttgatacagccaatcctaagacacctaagtataagtttgttcgcattcaaccaggacagactttttcagtgttagcttgttacaatggttcaccatctggtgtttaccaatgtgctatgaggcccaatttcactattaagggttcattccttaatggttcatgtggtagtgttggttttaacatagattatgactgtgtctctttttgttacatgcaccatatggaattaccaactggagttcatgctggcacagacttagaaggtaacttttatggaccttttgttgacaggcaaacagcacaagcagctggtacggacacaactattacagttaatgttttagcttggttgtacgctgctgttataaatggagacaggtggtttctcaatcgatttaccacaactcttaatgactttaaccttgtggctatgaagtacaattatgaacctctaacacaagaccatgttgacatactaggacctctttctgctcaaactggaattgccgttttagatatgtgtgcttcattaaaagaattactgcaaaatggtatgaatggacgtaccatattgggtagtgctttattagaagatgaatttacaccttttgatgttgttagacaatgctcaggtgttactttccaaagtgcagtgaaaagaacaatcaagggtacacaccactggttgttactcacaattttgacttcacttttagttttagtccagagtactcaatggtctttgttcttttttttgtatgaaaatgcctttttaccttttgctatgggtattattgctatgtctgcttttgcaatgatgtttgtcaaacataagcatgcatttctctgtttgtttttgttaccttctcttgccactgtagcttattttaatatggtctatatgcctgctagttgggtgatgcgtattatgacatggttggatatggttgatactagtttgtctggttttaagctaaaagactgtgttatgtatgcatcagctgtagtgttactaatccttatgacagcaagaactgtgtatgatgatggtgctaggagagtgtggacacttatgaatgtcttgacactcgtttataaagtttattatggtaatgctttagatcaagccatttccatgtgggctcttataatctctgttacttctaactactcaggtgtagttacaactgtcatgtttttggccagaggtattgtttttatgtgtgttgagtattgccctattttcttcataactggtaatacacttcagtgtataatgctagtttattgtttcttaggctatttttgtacttgttactttggcctcttttgtttactcaaccgctactttagactgactcttggtgtttatgattacttagtttctacacaggagtttagatatatgaattcacagggactactcccacccaagaatagcatagatgccttcaaactcaacattaaattgttgggtgttggtggcaaaccttgtatcaaagtagccactgtacagtctaaaatgtcagatgtaaagtgcacatcagtagtcttactctcagttttgcaacaactcagagtagaatcatcatctaaattgtgggctcaatgtgtccagttacacaatgacattctcttagctaaagatactactgaagcctttgaaaaaatggtttcactactttctgttttgctttccatgcagggtgctgtagacataaacaagctttgtgaagaaatgctggacaacagggcaaccttacaagctatagcctcagagtttagttcccttccatcatatgcagcttttgctactgctcaagaagcttatgagcaggctgttgctaatggtgattctgaagttgttcttaaaaagttgaagaagtctttgaatgtggctaaatctgaatttgaccgtgatgcagccatgcaacgtaagttggaaaagatggctgatcaagctatgacccaaatgtataaacaggctagatctgaggacaagagggcaaaagttactagtgctatgcagacaatgcttttcactatgcttagaaagttggataatgatgcactcaacaacattatcaacaatgcaagagatggttgtgttcccttgaacataatacctcttacaacagcagccaaactaatggttgtcataccagactataacacatataaaaatacgtgtgatggtacaacatttacttatgcatcagcattgtgggaaatccaacaggttgtagatgcagatagtaaaattgttcaacttagtgaaattagtatggacaattcacctaatttagcatggcctcttattgtaacagctttaagggccaattctgctgtcaaattacagaataatgagcttagtcctgttgcactacgacagatgtcttgtgctgccggtactacacaaactgcttgcactgatgacaatgcgttagcttactacaacacaacaaagggaggtaggtttgtacttgcactgttatccgatttacaggatttgaaatgggctagattccctaagagtgatggaactggtactatctatacagaactggaaccaccttgtaggtttgttacagacacacctaaaggtcctaaagtgaagtatttatactttattaaaggattaaacaacctaaatagaggtatggtacttggtagtttagctgccacagtacgtctacaagctggtaatgcaacagaagtgcctgccaattcaactgtattatctttctgtgcttttgctgtagatgctgctaaagcttacaaagattatctagctagtgggggacaaccaatcactaattgtgttaagatgttgtgtacacacactggtactggtcaggcaataacagttacaccggaagccaatatggatcaagaatcctttggtggtgcatcgtgttgtctgtactgccgttgccacatagatcatccaaatcctaaaggattttgtgacttaaaaggtaagtatgtacaaatacctacaacttgtgctaatgaccctgtgggttttacacttaaaaacacagtctgtaccgtctgcggtatgtggaaaggttatggctgtagttgtgatcaactccgcgaacccatgcttcagtcagctgatgcacaatcgtttttaaacgggtttgcggtgtaagtgcagcccgtcttacaccgtgcggcacaggcactagtactgatgtcgtatacagggcttttgacatctacaatgataaagtagctggttttgctaaattcctaaaaactaattgttgtcgcttccaagaaaaggacgaagatgacaatttaattgattcttactttgtagttaagagacacactttctctaactaccaacatgaagaaacaatttataatttacttaaggattgtccagctgttgctaaacatgacttctttaagtttagaatagacggtgacatggtaccacatatatcacgtcaacgtcttactaaatacacaatggcagacctcgtctatgctttaaggcattttgatgaaggtaattgtgacacattaaaagaaatacttgtcacatacaattgttgtgatgatgattatttcaataaaaaggactggtatgattttgtagaaaacccagatatattacgcgtatacgccaacttaggtgaacgtgtacgccaagctttgttaaaaacagtacaattctgtgatgccatgcgaaatgctggtattgttggtgtactgacattagataatcaagatctcaatggtaactggtatgatttcggtgatttcatacaaaccacgccaggtagtggagttcctgttgtagattcttattattcattgttaatgcctatattaaccttgaccagggctttaactgcagagtcacatgttgacactgacttaacaaagccttacattaagtgggatttgttaaaatatgacttcacggaagagaggttaaaactctttgaccgttattttaaatattgggatcagacataccacccaaattgtgttaactgtttggatgacagatgcattctgcattgtgcaaactttaatgttttattctctacagtgttcccacctacaagttttggaccactagtgagaaaaatatttgttgatggtgttccatttgtagtttcaactggataccacttcagagagctaggtgttgtacataatcaggatgtaaacttacatagctctagacttagttttaaggaattacttgtgtatgctgctgaccctgctatgcacgctgcttctggtaatctattactagataaacgcactacgtgcttttcagtagctgcacttactaacaatgttgcttttcaaactgtcaaacccggtaattttaacaaagacttctatgactttgctgtgtctaagggtttctttaaggaaggaagttctgttgaattaaaacacttcttctttgctcaggatggtaatgctgctatcagcgattatgactactatcgttataatctaccaacaatgtgtgatatcagacaactactatttgtagttgaagttgttgataagtactttgattgttacgatggtggctgtattaatgctaaccaagtcatcgtcaacaacctagacaaatcagctggttttccatttaataaatggggtaaggctagactttattatgattcaatgagttatgaggatcaagatgcacttttcgcatatacaaaacgtaatgtcatccctactataactcaaatgaatcttaagtatgccattagtgcaaagaatagagctcgcaccgtagctggtgtctctatctgtagtactatgaccaatagacagtttcatcaaaaattattgaaatcaatagccgccactagaggagctactgtagtaattggaacaagcaaattctatggtggttggcacaacatgttaaaaactgtttatagtgatgtagaaaaccctcaccttatgggttgggattatcctaaatgtgatagagccatgcctaacatgcttagaattatggcctcacttgttcttgctcgcaaacatacaacgtgttgtagcttgtcacaccgtttctatagattagctaatgagtgtgctcaagtattgagtgaaatggtcatgtgtggcggttcactatatgttaaaccaggtggaacctcatcaggagatgccacaactgcttatgctaatagtgtttttaacatttgtcaagctgtcacggccaatgttaatgcacttttatctactgatggtaacaaaattgccgataagtatgtccgcaatttacaacacagactttatgagtgtctctatagaaatagagatgttgacacagactttgtgaatgagttttacgcatatttgcgtaaacatttctcaatgatgatactctctgacgatgctgttgtgtgtttcaatagcacttatgcatctcaaggtctagtggctagcataaagaactttaagtcagttctttattatcaaaacaatgtttttatgtctgaagcaaaatgttggactgagactgaccttactaaaggacctcatgaattttgctctcaacatacaatgctagttaaacagggtgatgattatgtgtaccttccttacccagatccatcaagaatcctaggggccggctgttttgtagatgatatcgtaaaaacagatggtacacttatgattgaacggttcgtgtctttagctatagatgcttacccacttactaaacatcctaatcaggagtatgctgatgtctttcatttgtacttacaatacataagaaagctacatgatgagttaacaggacacatgttagacatgtattctgttatgcttactaatgataacacttcaaggtattgggaacctgagttttatgaggctatgtacacaccgcatacagtcttacaggctgttggggcttgtgttctttgcaattcacagacttcattaagatgtggtgcttgcatacgtagaccattcttatgttgtaaatgctgttacgaccatgtcatatcaacatcacataaattagtcttgtctgttaatccgtatgtttgcaatgctccaggttgtgatgtcacagatgtgactcaactttacttaggaggtatgagctattattgtaaatcacataaaccacccattagttttccattgtgtgctaatggacaagtttttggtttatataaaaatacatgtgttggtagcgataatgttactgactttaatgcaattgcaacatgtgactggacaaatgctggtgattacattttagctaacacctgtactgaaagactcaagctttttgcagcagaaacgctcaaagctactgaggagacatttaaactgtcttatggtattgctactgtacgtgaagtgctgtctgacagagaattacatctttcatgggaagttggtaaacctagaccaccacttaaccgaaattatgtctttactggttatcgtgtaactaaaaacagtaaagtacaaataggagagtacacctttgaaaaaggtgactatggtgatgctgttgtttaccgaggtacaacaacttacaaattaaatgttggtgattattttgtgctgacatcacatacagtaatgccattaagtgcacctacactagtgccacaagagcactatgttagaattactggcttatacccaacactcaatatctcagatgagttttctagcaatgttgcaaattatcaaaaggttggtatgcaaaagtattctacactccagggaccacctggtactggtaagagtcattttgctattggcctagctctctactacccttctgctcgcatagtgtatacagcttgctctcatgccgctgttgatgcactatgtgagaaggcattaaaatatttgcctatagataaatgtagtagaattatacctgcacgtgctcgtgtagagtgttttgataaattcaaagtgaattcaacattagaacagtatgtcttttgtactgtaaatgcattgcctgagacgacagcagatatagttgtctttgatgaaatttcaatggccacaaattatgatttgagtgttgtcaatgccagattacgtgctaagcactatgtgtacattggcgaccctgctcaattacctgcaccacgcacattgctaactaagggcacactagaaccagaatatttcaattcagtgtgtagacttatgaaaactataggtccagacatgttcctcggaacttgtcggcgttgtcctgctgaaattgttgacactgtgagtgctttggtttatgataataagcttaaagcacataaagacaaatcagctcaatgctttaaaatgttttataagggtgttatcacgcatgatgtttcatctgcaattaacaggccacaaataggcgtggtaagagaattccttacacgtaaccctgcttggagaaaagctgtctttatttcaccttataattcacagaatgctgtagcctcaaagattttgggactaccaactcaaactgttgattcatcacagggctcagaatatgactatgtcatattcactcaaaccactgaaacagctcactcttgtaatgtaaacagatttaatgttgctattaccagagcaaaagtaggcatactttgcataatgtctgatagagacctttatgacaagttgcaatttacaagtcttgaaattccacgtaggaatgtggcaactttacaagctgaaaatgtaacaggactctttaaagattgtagtaaggtaatcactgggttacatcctacacaggcacctacacacctcagtgttgacactaaattcaaaactgaaggtttatgtgttgacatacctggcatacctaaggacatgacctatagaagactcatctctatgatgggttttaaaatgaattatcaagttaatggttaccctaacatgtttatcacccgcgaagaagctataagacatgtacgtgcatggattggcttcgatgtcgaggggtgtcatgctactagagaagctgttggtaccaatttacctttacagctaggtttttctacaggtgttaacctagttgctgtacctacaggttatgttgatacacctaataatacagatttttccagagttagtgctaaaccaccgcctggagatcaatttaaacacctcataccacttatgtacaaaggacttccttggaatgtagtgcgtataaagattgtacaaatgttaagtgacacacttaaaaatctctctgacagagtcgtatttgtcttatgggcacatggctttgagttgacatctatgaagtattttgtgaaaataggacctgagcgcacctgttgtctatgtgatagacgtgccacatgcttttccactgcttcagacacttatgcctgttggcatcattctattggatttgattacgtctataatccgtttatgattgatgttcaacaatggggttttacaggtaacctacaaagcaaccatgatctgtattgtcaagtccatggtaatgcacatgtagctagttgtgatgcaatcatgactaggtgtctagctgtccacgagtgctttgttaagcgtgttgactggactattgaatatcctataattggtgatgaactgaagattaatgcggcttgtagaaaggttcaacacatggttgttaaagctgcattattagcagacaaattcccagttcttcacgacattggtaaccctaaagctattaagtgtgtacctcaagctgatgtagaatggaagttctatgatgcacagccttgtagtgacaaagcttataaaatagaagaattattctattcttatgccacacattctgacaaattcacagatggtgtatgcctattttggaattgcaatgtcgatagatatcctgctaattccattgtttgtagatttgacactagagtgctatctaaccttaacttgcctggttgtgatggtggcagtttgtatgtaaataaacatgcattccacacaccagcttttgataaaagtgcttttgttaatttaaaacaattaccatttttctattactctgacagtccatgtgagtctcatggaaaacaagtagtgtcagatatagattatgtaccactaaagtctgctacgtgtataacacgttgcaatttaggtggtgctgtctgtagacatcatgctaatgagtacagattgtatctcgatgcttataacatgatgatctcagctggctttagcttgtgggtttacaaacaatttgatacttataacctctggaacacttttacaagacttcagagtttagaaaatgtggcttttaatgttgtaaataagggacactttgatggacaacagggtgaagtaccagtttctatcattaataacactgtttacacaaaagttgatggtgttgatgtagaattgtttgaaaataaaacaacattacctgttaatgtagcatttgagctttgggctaagcgcaacattaaaccagtaccagaggtgaaaatactcaataatttgggtgtggacattgctgctaatactgtgatctgggactacaaaagagatgctccagcacatatatctactattggtgtttgttctatgactgacatagccaagaaaccaactgaaacgatttgtgcaccactcactgtcttttttgatggtagagttgatggtcaagtagacttatttagaaatgcccgtaatggtgttcttattacagaaggtagtgttaaaggtttacaaccatctgtgggtcccaaacaagctagtcttaatggagtcacattaattggagaagccgtaaaaacacagttcaattattataagaaagttgatggtgttgtccaacaattacctgaaacttactttactcagagtagaaatttacaagaatttaaacccaggagtcaaatggaaattgatttcttagaattagctatggatgaattcattgaacggtataaattagaaggctatgccttcgaacatatcgtttatggagattttagtcatagtcagttaggtggtttacatctactgattggactagctaaacgttttaaggaatcaccttttgaattagaagattttattcctatggacagtacagttaaaaactatttcataacagatgcgcaaacaggttcatctaagtgtgtgtgttctgttattgatttattacttgatgattttgttgaaataataaaatcccaagatttatctgtagtttctaaggttgtcaaagtgactattgactatacagaaatttcatttatgctttggtgtaaagatggccatgtagaaacattttacccaaaattacaatctagtcaagcgtggcaaccgggtgttgctatgcctaatctttacaaaatgcaaagaatgctattagaaaagtgtgaccttcaaaattatggtgatagtgcaacattacctaaaggcataatgatgaatgtcgcaaaatatactcaactgtgtcaatatttaaacacattaacattagctgtaccctataatatgagagttatacattttggtgctggttctgataaaggagttgcaccaggtacagctgttttaagacagtggttgcctacgggtacgctgcttgtcgattcagatcttaatgactttgtctctgatgcagattcaactttgattggtgattgtgcaactgtacatacagctaataaatgggatctcattattagtgatatgtacgaccctaagactaaaaatgttacaaaagaaaatgactctaaagagggttttttcacttacatttgtgggtttatacaacaaaagctagctcttggaggttccgtggctataaagataacagaacattcttggaatgctgatctttataagctcatgggacacttcgcatggtggacagcctttgttactaatgtgaatgcgtcatcatctgaagcatttttaattggatgtaattatcttggcaaaccacgcgaacaaatagatggttatgtcatgcatgcaaattacatattttggaggaatacaaatccaattcagttgtcttcctattctttatttgacatgagtaaatttccccttaaattaaggggtactgctgttatgtctttaaaagaaggtcaaatcaatgatatgattttatctcttcttagtaaaggtagacttataattagagaaaacaacagagttgttatttctagtgatgttcttgttaacaactaaacgaacaatgtttgtttttcttgttttattgccactagtctctagtcagtgtgttaatcttacaaccagaactcaattaccccctgcatacactaattctttcacacgtggtgtttattaccctgacaaagttttcagatcctcagttttacattcaactcaggacttgttcttacctttcttttccaatgttacttggttccatgctatacatgtctctgggaccaatggtactaagaggtttgataaccctgtcctaccatttaatgatggtgtttattttgcttccactgagaagtctaacataataagaggctggatttttggtactactttagattcgaagacccagtccctacttattgttaataacgctactaatgttgttattaaagtctgtgaatttcaattttgtaatgatccatttttgggtgtttattaccacaaaaacaacaaaagttggatggaaagtgagttcagagtttattctagtgcgaataattgcacttttgaatatgtctctcagccttttcttatggaccttgaaggaaaacagggtaatttcaaaaatcttagggaatttgtgtttaagaatattgatggttattttaaaatatattctaagcacacgcctattaatttagtgcgtgatctccctcagggtttttcggctttagaaccattggtagatttgccaataggtattaacatcactaggtttcaaactttacttgctttacatagaagttatttgactcctggtgattcttcttcaggttggacagctggtgctgcagcttattatgtgggttatcttcaacctaggacttttctattaaaatataatgaaaatggaaccattacagatgctgtagactgtgcacttgaccctctctcagaaacaaagtgtacgttgaaatccttcactgtagaaaaaggaatctatcaaacttctaactttagagtccaaccaacagaatctattgttagatttcctaatattacaaacttgtgcccttttggtgaagtttttaacgccaccagatttgcatctgtttatgcttggaacaggaagagaatcagcaactgtgttgctgattattctgtcctatataattccgcatcattttccacttttaagtgttatggagtgtctcctactaaattaaatgatctctgctttactaatgtctatgcagattcatttgtaattagaggtgatgaagtcagacaaatcgctccagggcaaactggaaagattgctgattataattataaattaccagatgattttacaggctgcgttatagcttggaattctaacaatcttgattctaaggttggtggtaattataattacctgtatagattgtttaggaagtctaatctcaaaccttttgagagagatatttcaactgaaatctatcaggccggtagcacaccttgtaatggtgttgaaggttttaattgttactttcctttacaatcatatggtttccaacccactaatggtgttggttaccaaccatacagagtagtagtactttcttttgaacttctacatgcaccagcaactgtttgtggacctaaaaagtctactaatttggttaaaaacaaatgtgtcaatttcaacttcaatggtttaacaggcacaggtgttcttactgagtctaacaaaaagtttctgcctttccaacaatttggcagagacattgctgacactactgatgctgtccgtgatccacagacacttgagattcttgacattacaccatgttcttttggtggtgtcagtgttataacaccaggaacaaatacttctaaccaggttgctgttctttatcaggatgttaactgcacagaagtccctgttgctattcatgcagatcaacttactcctacttggcgtgtttattctacaggttctaatgtttttcaaacacgtgcaggctgtttaataggggctgaacatgtcaacaactcatatgagtgtgacatacccattggtgcaggtatatgcgctagttatcagactcagactaattctcctcggcgggcacgtagtgtagctagtcaatccatcattgcctacactatgtcacttggtgcagaaaattcagttgcttactctaataactctattgccatacccacaaattttactattagtgttaccacagaaattctaccagtgtctatgaccaagacatcagtagattgtacaatgtacatttgtggtgattcaactgaatgcagcaatcttttgttgcaatatggcagtttttgtacacaattaaaccgtgctttaactggaatagctgttgaacaagacaaaaacacccaagaagtttttgcacaagtcaaacaaatttacaaaacaccaccaattaaagattttggtggttttaatttttcacaaatattaccagatccatcaaaaccaagcaagaggtcatttattgaagatctacttttcaacaaagtgacacttgcagatgctggcttcatcaaacaatatggtgattgccttggtgatattgctgctagagacctcatttgtgcacaaaagtttaacggccttactgttttgccacctttgctcacagatgaaatgattgctcaatacacttctgcactgttagcgggtacaatcacttctggttggacctttggtgcaggtgctgcattacaaataccatttgctatgcaaatggcttataggtttaatggtattggagttacacagaatgttctctatgagaaccaaaaattgattgccaaccaatttaatagtgctattggcaaaattcaagactcactttcttccacagcaagtgcacttggaaaacttcaagatgtggtcaaccaaaatgcacaagctttaaacacgcttgttaaacaacttagctccaattttggtgcaatttcaagtgttttaaatgatatcctttcacgtcttgacaaagttgaggctgaagtgcaaattgataggttgatcacaggcagacttcaaagtttgcagacatatgtgactcaacaattaattagagctgcagaaatcagagcttctgctaatcttgctgctactaaaatgtcagagtgtgtacttggacaatcaaaaagagttgatttttgtggaaagggctatcatcttatgtccttccctcagtcagcacctcatggtgtagtcttcttgcatgtgacttatgtccctgcacaagaaaagaacttcacaactgctcctgccatttgtcatgatggaaaagcacactttcctcgtgaaggtgtctttgtttcaaatggcacacactggtttgtaacacaaaggaatttttatgaaccacaaatcattactacagacaacacatttgtgtctggtaactgtgatgttgtaataggaattgtcaacaacacagtttatgatcctttgcaacctgaattagactcattcaaggaggagttagataaatattttaagaatcatacatcaccagatgttgatttaggtgacatctctggcattaatgcttcagttgtaaacattcaaaaagaaattgaccgcctcaatgaggttgccaagaatttaaatgaatctctcatcgatctccaagaacttggaaagtatgagcagtatataaaatggccatggtacatttggctaggttttatagctggcttgattgccatagtaatggtgacaattatgctttgctgtatgaccagttgctgtagttgtctcaagggctgttgttcttgtggatcctgctgcaaatttgatgaagacgactctgagccagtgctcaaaggagtcaaattacattacacataattcctgatcttctggtctaaacgaactaaatattatattagtttttctgtttggaactttaattttagccatggcagattccaacggtactattaccgttgaagagcttaaaaagctccttgaacaatggaacctagtaataggtttcctattccttacatggatttgtcttctacaatttgcctatgccaacaggaataggtttttgtatataattaagttaattttcctctggctgttatggccagtaactttagcttgttttgtgcttgctgctgtttacagaataaattggatcaccggtggaattgctatcgcaatggcttgtcttgtaggcttgatgtggctcagctacttcattgcttctttcagactgtttgcgcgtacccgttccatgtggtcattcaatccagaaactaacattcttctcaacgtgccactccatggcactattctgaccagaccgcttctagaaagtgaactcgtaatcggagctgtgatccttcgtggacatcttcgtattgctggacaccatctaggacgctgtgacatcaaggacctgcctaaagaaatcactgttgctacatcacgaacgctttcttattacaaattgggagcttcgcagcgtgtagcaggtgactcaggttttgctgcatacagtcgctacaggattggcaactataaattaaacacagaccattccagtagcagtgacaatattgctttgcttgtacagtaatcacttgaactgcaagatcataatgaaacttgtcacgcctaaacgaacatgaaatttcttgttttcttaggaatcatcacaactgtagctgcatttcaccaagaatgtagtttacagtcatgtactcaacatcaaccatatgtagttgatgacccgtgtcctattcacttctattctaaatggtatattagagtaggagctagaaaatcagcacctttaattgaattgtgcgtggatgaggctggttctaaatcacccattcagtacatcgatatcggtaattatacagtttcctgtttaccttttacaattaattgccaggaacctaaattgggtagtcttgtagtgcgttgttcgttctatgaagactttttagagtatcatgacgttcgtgttgttttagatttcatctaaacgaacaaactaaaatgtctgataatggaccccaaaatcagcgaaatgcaccccgcattacgtttggtggaccctcagattcaactggcagtaaccagaatggagaacgcagtggggcgcgatcaaaacaacgtcggccccaaggtttacccaataatactgcgtcttggttcaccgctctcactcaacatggcaaggaagaccttaaattccctcgaggacaaggcgttccaattaacaccaatagcagtccagatgaccaaattggctactaccgaagagctaccagacgaattcgtggtggtgacggtaaaatgaaagatctcagtccaagatggtatttctactacctaggaactgggccagaagctggacttccctatggtgctaacaaagacggcatcatatgggttgcaactgagggagccttgaatacaccaaaagatcacattggcacccgcaatcctgctaacaatgctgcaatcgtgctacaacttcctcaaggaacaacattgccaaaaggcttctacgcagaagggagcagaggcggcagtcaagcctcttctcgttcctcatcacgtagtcgcaacagttcaagaaattcaactccaggcagcagtaggggaacttctcctgctagaatggctggcaatggcggtgatgctgctcttgctttgctgctgcttgacagattgaaccagcttgagagcaaaatgtctggtaaaggccaacaacaacaaggccaaactgtcactaagaaatctgctgctgaggcttctaagaagcctcggcaaaaacgtactgccactaaagcatacaatgtaacacaagctttcggcagacgtggtccagaacaaacccaaggaaattttggggaccaggaactaatcagacaaggaactgattacaaacattggccgcaaattgcacaatttgcccccagcgcttcagcgttcttcggaatgtcgcgcattggcatggaagtcacaccttcgggaacgtggttgacctacacaggtgccatcaaattggatgacaaagatccaaatttcaaagatcaagtcattttgctgaataagcatattgacgcatacaaaacattcccaccaacagagcctaaaaaggacaaaaagaagaaggctgatgaaactcaagccttaccgcagagacagaagaaacagcaaactgtgactcttcttcctgctgcagatttggatgatttctccaaacaattgcaacaatccatgagcagtgctgactcaactcaggcctaaactcatgcagaccacacaaggcagatgggctatataaacgttttcgcttttccgtttacgatatatagtctactcttgtgcagaatgaattctcgtaactacatagcacaagtagatgtagttaactttaatctcacatagcaatctttaatcagtgtgtaacattagggaggacttgaaagagccaccacattttcaccgaggccacgcggagtacgatcgagtgtacagtgaacaatgctagggagagctgcctatatggaagagccctaatgtgtaaaattaattttagtagtgctatccccatgtgattttaatagcttcttaggagaatgacaaaaaaaaaaaaaaaaaaaaaaaaa

SEQ ID NO: 43 - DNA, 27975 bp, Coronaviridae
  source 1..27975: mol_type = other DNA
  misc_feature 1..27975: note = SARS-CoV-2-[3,E,7,8] polynucleotide sequence
attaaaggtttataccttcccaggtaacaaaccaaccaactttcgatctcttgtagatctgttctctaaacgaactttaaaatctgtgtggctgtcactcggctgcatgcttagtgcactcacgcagtataattaataactaattactgtcgttgacaggacacgagtaactcgtctatcttctgcaggctgcttacggtttcgtccgtgttgcagccgatcatcagcacatctaggtttcgtccgggtgtgaccgaaaggtaagatggagagccttgtccctggtttcaacgagaaaacacacgtccaactcagtttgcctgttttacaggttcgcgacgtgctcgtacgtggctttggagactccgtggaggaggtcttatcagaggcacgtcaacatcttaaagatggcacttgtggcttagtagaagttgaaaaaggcgttttgcctcaacttgaacagccctatgtgttcatcaaacgttcggatgctcgaactgcacctcatggtcatgttatggttgagctggtagcagaactcgaaggcattcagtacggtcgtagtggtgagacacttggtgtccttgtccctcatgtgggcgaaataccagtggcttaccgcaaggttcttcttcgtaagaacggtaataaaggagctggtggccatagttacggcgccgatctaaagtcatttgacttaggcgacgagcttggcactgatccttatgaagattttcaagaaaactggaacactaaacatagcagtggtgttacccgtgaactcatgcgtgagcttaacggaggggcatacactcgctatgtcgataacaacttctgtggccctgatggctaccctcttgagtgcattaaagaccttctagcacgtgctggtaaagcttcatgcactttgtccgaacaactggactttattgacactaagaggggtgtatactgctgccgtgaacatgagcatgaaattgcttggtacacggaacgttctgaaaagagctatgaattgcagacaccttttgaaattaaattggcaaagaaatttgacaccttcaatggggaatgtccaaattttgtatttcccttaaattccataatcaagactattcaaccaagggttgaaaagaaaaagcttgatggctttatgggtagaattcgatctgtctatccagttgcgtcaccaaatgaatgcaaccaaatgtgcctttcaactctcatgaagtgtgatcattgtggtgaaacttcatggcagacgggcgattttgttaaagccacttgcgaattttgtggcactgagaatttgactaaagaaggtgccactacttgtggttacttaccccaaaatgctgttgttaaaatttattgtccagcatgtcacaattcagaagtaggacctgagcatagtcttgccgaataccataatgaatctggcttgaaaaccattcttcgtaagggtggtcgcactattgcctttggaggctgtgtgttctcttatgttggttgccataacaagtgtgcctattgggttccacgtgctagcgctaacataggttgtaaccatacaggtgttgttggagaaggttccgaaggtcttaatgacaaccttcttgaaatactccaaaaagagaaagtcaacatcaatattgttggtgactttaaacttaatgaagagatcgccattattttggcatctttttctgcttccacaagtgcttttgtggaaactgtgaaaggtttggattataaagcattcaaacaaattgttgaatcctgtggtaattttaaagttacaaaaggaaaagctaaaaaaggtgcctggaatattggtgaacagaaatcaatactgagtcctctttatgcatttgcatcagaggctgctcgtgttgtacgatcaattttctcccgcactcttgaaactgctcaaaattctgtgcgtgttttacagaaggccgctataacaatactagatggaatttcacagtattcactgagactcattgatgctatgatgttcacatctgatttggctactaacaatctagttgtaatggcctacattacaggtggtgttgttcagttgacttcgcagtggctaactaacatctttggcactgtttatgaaaaactcaaacccgtccttgattggcttgaagagaagtttaaggaaggtgtagagtttcttagagacggttgggaaattgttaaatttatctcaacctgtgcttgtgaaattgtcggtggacaaattgtcacctgtgcaaaggaaattaaggagagtgttcagacattctttaagcttgtaaataaatttttggctttgtgtgctgactctatcattattggtggagctaaacttaaagccttgaatttaggtgaaacatttgtcacgcactcaaagggattgtacagaaagtgtgttaaatccagagaagaaactggcctactcatgcctctaaaagccccaaaagaaattatcttcttagagggagaaacacttcccacagaagtgttaacagaggaagttgtcttgaaaactggtgatttacaaccattagaacaacctactagtgaagctgttgaagctccattggttggtacaccagtttgtattaacgggcttatgttgctcgaaatcaaagacacagaaaagtactgtgcccttgcacctaatatgatggtaacaaacaataccttcacactcaaaggcggtgcaccaacaaaggttacttttggtgatgacactgtgatagaagtgcaaggttacaagagtgtgaatatcacttttgaacttgatgaaaggattgataaagtacttaatgagaagtgctctgcctatacagttgaactcggtacagaagtaaatgagttcgcctgtgttgtggcagatgctgtcataaaaactttgcaaccagtatctgaattacttacaccactgggcattgatttagatgagtggagtatggctacatactacttatttgatgagtctggtgagtttaaattggcttcacatatgtattgttctttctaccctccagatgaggatgaagaagaaggtgattgtgaagaagaagagtttgagccatcaactcaatatgagtatggtactgaagatgattaccaaggtaaacctttggaatttggtgccacttctgctgctcttcaacctgaagaagagcaagaagaagattggttagatgatgatagtcaacaaactgttggtcaacaagacggcagtgaggacaatcagacaactactattcaaacaattgttgaggttcaacctcaattagagatggaacttacaccagttgttcagactattgaagtgaatagttttagtggttatttaaaacttactgacaatgtatacattaaaaatgcagacattgtggaagaagctaaaaaggtaaaaccaacagtggttgttaatgcagccaatgtttaccttaaacatggaggaggtgttgcaggagccttaaataaggctactaacaatgccatgcaagttgaatctgatgattacatagctactaatggaccacttaaagtgggtggtagttgtgttttaagcggacacaatcttgctaaacactgtcttcatgttgtcggcccaaatgttaacaaaggtgaagacattcaacttcttaagagtgcttatgaaaattttaatcagcacgaagttctacttgcaccattattatcagctggtatttttggtgctgaccctatacattctttaagagtttgtgtagatactgttcgcacaaatgtctacttagctgtctttgataaaaatctctatgacaaacttgtttcaagctttttggaaatgaagagtgaaaagcaagttgaacaaaagatcgctgagattcctaaagaggaagttaagccatttataactgaaagtaaaccttcagttgaacagagaaaacaagatgataagaaaatcaaagcttgtgttgaagaagttacaacaactctggaagaaactaagttcctcacagaaaacttgttactttatattgacattaatggcaatcttcatccagattctgccactcttgttagtgacattgacatcactttcttaaagaaagatgctccatatatagtgggtgatgttgttcaagagggtgttttaactgctgtggttatacctactaaaaaggctggtggcactactgaaatgctagcgaaagctttgagaaaagtgccaacagacaattatataaccacttacccgggtcagggtttaaatggttacactgtagaggaggcaaagacagtgcttaaaaagtgtaaaagtgccttttacattctaccatctattatctctaatgagaagcaagaaattcttggaactgtttcttggaatttgcgagaaatgcttgcacatgcagaagaaacacgcaaattaatgcctgtctgtgtggaaactaaagccatagtttcaactatacagcgtaaatataagggtattaaaatacaagagggtgtggttgattatggtgctagattttacttttacaccagtaaaacaactgtagcgtcacttatcaacacacttaacgatctaaatgaaactcttgttacaatgccacttggctatgtaacacatggcttaaatttggaagaagctgctcggtatatgagatctctcaaagtgccagctacagtttctgtttcttcacctgatgctgttacagcgtataatggttatcttacttcttcttctaaaacacctgaagaacattttattgaaaccatctcacttgctggttcctataaagattggtcctattctggacaatctacacaactaggtatagaatttcttaagagaggtgataaaagtgtatattacactagtaatcctaccacattccacctagatggtgaagttatcacctttgacaatcttaagacacttctttctttgagagaagtgaggactattaaggtgtttacaacagtagacaacattaacctccacacgcaagttgtggacatgtcaatgacatatggacaacagtttggtccaacttatttggatggagctgatgttactaaaataaaacctcataattcacatgaaggtaaaacattttatgttttacctaatgatgacactctacgtgttgaggcttttgagtactaccacacaactgatcctagttttctgggtaggtacatgtcagcattaaatcacactaaaaagtggaaatacccacaagttaatggtttaacttctattaaatgggcagataacaactgttatcttgccactgcattgttaacactccaacaaatagagttgaagtttaatccacctgctctacaagatgcttattacagagcaagggctggtgaagctgctaacttttgtgcacttatcttagcctactgtaataagacagtaggtgagttaggtgatgttagagaaacaatgagttacttgtttcaacatgccaatttagattcttgcaaaagagtcttgaacgtggtgtgtaaaacttgtggacaacagcagacaacccttaagggtgtagaagctgttatgtacatgggcacactttcttatgaacaatttaagaaaggtgttcagataccttgtacgtgtggtaaacaagctacaaaatatctagtacaacaggagtcaccttttgttatgatgtcagcaccacctgctcagtatgaacttaagcatggtacatttacttgtgctagtgagtacactggtaattaccagtgtggtcactataaacatataacttctaaagaaactttgtattgcatagacggtgctttacttacaaagtcctcagaatacaaaggtcctattacggatgttttctacaaagaaaacagttacacaacaaccataaaaccagttacttataaattggatggtgttgtttgtacagaaattgaccctaagttggacaattattataagaaagacaattcttatttcacagagcaaccaattgatcttgtaccaaaccaaccatatccaaacgcaagcttcgataattttaagtttgtatgtgataatatcaaatttgctgatgatttaaaccagttaactggttataagaaacctgcttcaagagagcttaaagttacatttttccctgacttaaatggtgatgtggtggctattgattataaacactacacaccctcttttaagaaaggagctaaattgttacataaacctattgtttggcatgttaacaatgcaactaataaagccacgtataaaccaaatacctggtgtatacgttgtctttggagcacaaaaccagttgaaacatcaaattcgtttgatgtactgaagtcagaggacgcgcagggaatggataatcttgcctgcgaagatctaaaaccagtctctgaagaagtagtggaaaatcctaccatacagaaagacgttcttgagtgtaatgtgaaaactaccgaagttgtaggagacattatacttaaaccagcaaataatagtttaaaaattacagaagaggttggccacacagatctaatggctgcttatgtagacaattctagtcttactattaagaaacctaatgaattatctagagtattaggtttgaaaacccttgctactcatggtttagctgctgttaatagtgtcccttgggatactatagctaattatgctaagccttttcttaacaaagttgttagtacaactactaacatagttacacggtgtttaaaccgtgtttgtactaattatatgccttatttctttactttattgctacaattgtgtacttttactagaagtacaaattctagaattaaagcatctatgccgactactatagcaaagaatactgttaagagtgtcggtaaattttgtctagaggcttcatttaattatttgaagtcacctaatttttctaaactgataaatattataatttggtttttactattaagtgtttgcctaggttctttaatctactcaaccgctgctttaggtgttttaatgtctaatttaggcatgccttcttactgtactggttacagagaaggctatttgaactctactaatgtcactattgcaacctactgtactggttctataccttgtagtgtttgtcttagtggtttagattctttagacacctatccttctttagaaactatacaaattaccatttcatcttttaaatgggatttaactgcttttggcttagttgcagagtggtttttggcatatattcttttcactaggtttttctatgtacttggattggctgcaatcatgcaattgtttttcagctattttgcagtacattttattagtaattcttggcttatgtggttaataattaatcttgtacaaatggccccgatttcagctatggttagaatgtacatcttctttgcatcattttattatgtatggaaaagttatgtgcatgttgtagacggttgtaattcatcaacttgtatgatgtgttacaaacgtaatagagcaacaagagtcgaatgtacaactattgttaatggtgttagaaggtccttttatgtctatgctaatggaggtaaaggcttttgcaaactacacaattggaattgtgttaattgtgatacattctgtgctggtagtacatttattagtgatgaagttgcgagagacttgtcactacagtttaaaagaccaataaatcctactgaccagtcttcttacatcgttgatagtgttacagtgaagaatggttccatccatctttactttgataaagctggtcaaaagacttatgaaagacattctctctctcattttgttaacttagacaacctgagagctaataacactaaaggttcattgcctattaatgttatagtttttgatggtaaatcaaaatgtgaagaatcatctgcaaaatcagcgtctgtttactacagtcagcttatgtgtcaacctatactgttactagatcaggcattagtgtctgatgttggtgatagtgcggaagttgcagttaaaatgtttgatgcttacgttaatacgttttcatcaacttttaacgtaccaatggaaaaactcaaaacactagttgcaactgcagaagctgaacttgcaaagaatgtgtccttagacaatgtcttatctacttttatttcagcagctcggcaagggtttgttgattcagatgtagaaactaaagatgttgttgaatgtcttaaattgtcacatcaatctgacatagaagttactggcgatagttgtaataactatatgctcacctataacaaagttgaaaacatgacaccccgtgaccttggtgcttgtattgactgtagtgcgcgtcatattaatgcgcaggtagcaaaaagtcacaacattgctttgatatggaacgttaaagatttcatgtcattgtctgaacaactacgaaaacaaatacgtagtgctgctaaaaagaataacttaccttttaagttgacatgtgcaactactagacaagttgttaatgttgtaacaacaaagatagcacttaagggtggtaaaattgttaataattggttgaagcagttaattaaagttacacttgtgttcctttttgttgctgctattttctatttaataacacctgttcatgtcatgtctaaacatactgacttttcaagtgaaatcataggatacaaggctattgatggtggtgtcactcgtgacatagcatctacagatacttgttttgctaacaaacatgctgattttgacacatggtttagccagcgtggtggtagttatactaatgacaaagcttgcccattgattgctgcagtcataacaagagaagtgggttttgtcgtgcctggtttgcctggcacgatattacgcacaactaatggtgactttttgcatttcttacctagagtttttagtgcagttggtaacatctgttacacaccatcaaaacttatagagtacactgactttgcaacatcagcttgtgttttggctgctgaatgtacaatttttaaagatgcttctggtaagccagtaccatattgttatgataccaatgtactagaaggttctgttgcttatgaaagtttacgccctgacacacgttatgtgctcatggatggctctattattcaatttcctaacacctaccttgaaggttctgttagagtggtaacaacttttgattctgagtactgtaggcacggcacttgtgaaagatcagaagctggtgtttgtgtatctactagtggtagatgggtacttaacaatgattattacagatctttaccaggagttttctgtggtgtagatgctgtaaatttacttactaatatgtttacaccactaattcaacctattggtgctttggacatatcagcatctatagtagctggtggtattgtagctatcgtagtaacatgccttgcctactattttatgaggtttagaagagcttttggtgaatacagtcatgtagttgcctttaatactttactattccttatgtcattcactgtactctgtttaacaccagtttactcattcttacctggtgtttattctgttatttacttgtacttgacattttatcttactaatgatgtttcttttttagcacatattcagtggatggttatgttcacacctttagtacctttctggataacaattgcttatatcatttgtatttccacaaagcatttctattggttctttagtaattacctaaagagacgtgtagtctttaatggtgtttcctttagtacttttgaagaagctgcgctgtgcacctttttgttaaataaagaaatgtatctaaagttgcgtagtgatgtgctattacctcttacgcaatataatagatacttagctctttataataagtacaagtattttagtggagcaatggatacaactagctacagagaagctgcttgttgtcatctcgcaaaggctctcaatgacttcagtaactcaggttctgatgttctttaccaaccaccacaaacctctatcacctcagctgttttgcagagtggttttagaaaaatggcattcccatctggtaaagttgagggttgtatggtacaagtaacttgtggtacaactacacttaacggtctttggcttgatgacgtagtttactgtccaagacatgtgatctgcacctctgaagacatgcttaaccctaattatgaagatttactcattcgtaagtctaatcataatttcttggtacaggctggtaatgttcaactcagggttattggacattctatgcaaaattgtgtacttaagcttaaggttgatacagccaatcctaagacacctaagtataagtttgttcgcattcaaccaggacagactttttcagtgttagcttgttacaatggttcaccatctggtgtttaccaatgtgctatgaggcccaatttcactattaagggttcattccttaatggttcatgtggtagtgttggttttaacatagattatgactgtgtctctttttgttacatgcaccatatggaattaccaactggagttcatgctggcacagacttagaaggtaacttttatggaccttttgttgacaggcaaacagcacaagcagctggtacggacacaactattacagttaatgttttagcttggttgtacgctgctgttataaatggagacaggtggtttctcaatcgatttaccacaactcttaatgactttaaccttgtggctatgaagtacaattatgaacctctaacacaagaccatgttgacatactaggacctctttctgctcaaactggaattgccgttttagatatgtgtgcttcattaaaagaattactgcaaaatggtatgaatggacgtaccatattgggtagtgctttattagaagatgaatttacaccttttgatgttgttagacaatgctcaggtgttactttccaaagtgcagtgaaaagaacaatcaagggtacacaccactggttgttactcacaattttgacttcacttttagttttagtccagagtactcaatggtctttgttcttttttttgtatgaaaatgcctttttaccttttgctatgggtattattgctatgtctgcttttgcaatgatgtttgtcaaacataagcatgcatttctctgtttgtttttgttaccttctcttgccactgtagcttattttaatatggtctatatgcctgctagttgggtgatgcgtattatgacatggttggatatggttgatactagtttgtctggttttaagctaaaagactgtgttatgtatgcatcagctgtagtgttactaatccttatgacagcaagaactgtgtatgatgatggtgctaggagagtgtggacacttatgaatgtcttgacactcgtttataaagtttattatggtaatgctttagatcaagccatttccatgtgggctcttataatctctgttacttctaactactcaggtgtagttacaactgtcatgtttttggccagaggtattgtttttatgtgtgttgagtattgccctattttcttcataactggtaatacacttcagtgtataatgctagtttattgtttcttaggctatttttgtacttgttactttggcctcttttgtttactcaaccgctactttagactgactcttggtgtttatgattacttagtttctacacaggagtttagatatatgaattcacagggactactcccacccaagaatagcatagatgccttcaaactcaacattaaattgttgggtgttggtggcaaaccttgtatcaaagtagccactgtacagtctaaaatgtcagatgtaaagtgcacatcagtagtcttactctcagttttgcaacaactcagagtagaatcatcatctaaattgtgggctcaatgtgtccagttacacaatgacattctcttagctaaagatactactgaagcctttgaaaaaatggtttcactactttctgttttgctttccatgcagggtgctgtagacataaacaagctttgtgaagaaatgctggacaacagggcaaccttacaagctatagcctcagagtttagttcccttccatcatatgcagcttttgctactgctcaagaagcttatgagcaggctgttgctaatggtgattctgaagttgttcttaaaaagttgaagaagtctttgaatgtggctaaatctgaatttgaccgtgatgcagccatgcaacgtaagttggaaaagatggctgatcaagctatgacccaaatgtataaacaggctagatctgaggacaagagggcaaaagttactagtgctatgcagacaatgcttttcactatgcttagaaagttggataatgatgcactcaacaacattatcaacaatgcaagagatggttgtgttcccttgaacataatacctcttacaacagcagccaaactaatggttgtcataccagactataacacatataaaaatacgtgtgatggtacaacatttacttatgcatcagcattgtgggaaatccaacaggttgtagatgcagatagtaaaattgttcaacttagtgaaattagtatggacaattcacctaatttagcatggcctcttattgtaacagctttaagggccaattctgctgtcaaattacagaataatgagcttagtcctgttgcactacgacagatgtcttgtgctgccggtactacacaaactgcttgcactgatgacaatgcgttagcttactacaacacaacaaagggaggtaggtttgtacttgcactgttatccgatttacaggatttgaaatgggctagattccctaagagtgatggaactggtactatctatacagaactggaaccaccttgtaggtttgttacagacacacctaaaggtcctaaagtgaagtatttatactttattaaaggattaaacaacctaaatagaggtatggtacttggtagtttagctgccacagtacgtctacaagctggtaatgcaacagaagtgcctgccaattcaactgtattatctttctgtgcttttgctgtagatgctgctaaagcttacaaagattatctagctagtgggggacaaccaatcactaattgtgttaagatgttgtgtacacacactggtactggtcaggcaataacagttacaccggaagccaatatggatcaagaatcctttggtggtgcatcgtgttgtctgtactgccgttgccacatagatcatccaaatcctaaaggattttgtgacttaaaaggtaagtatgtacaaatacctacaacttgtgctaatgaccctgtgggttttacacttaaaaacacagtctgtaccgtctgcggtatgtggaaaggttatggctgtagttgtgatcaactccgcgaacccatgcttcagtcagctgatgcacaatcgtttttaaacgggtttgcggtgtaagtgcagcccgtcttacaccgtgcggcacaggcactagtactgatgtcgtatacagggcttttgacatctacaatgataaagtagctggttttgctaaattcctaaaaactaattgttgtcgcttccaagaaaaggacgaagatgacaatttaattgattcttactttgtagttaagagacacactttctctaactaccaacatgaagaaacaatttataatttacttaaggattgtccagctgttgctaaacatgacttctttaagtttagaatagacggtgacatggtaccacatatatcacgtcaacgtcttactaaatacacaatggcagacctcgtctatgctttaaggcattttgatgaaggtaattgtgacacattaaaagaaatacttgtcacatacaattgttgtgatgatgattatttcaataaaaaggactggtatgattttgtagaaaacccagatatattacgcgtatacgccaacttaggtgaacgtgtacgccaagctttgttaaaaacagtacaattctgtgatgccatgcgaaatgctggtattgttggtgtactgacattagataatcaagatctcaatggtaactggtatgatttcggtgatttcatacaaaccacgccaggtagtggagttcctgttgtagattcttattattcattgttaatgcctatattaaccttgaccagggctttaactgcagagtcacatgttgacactgacttaacaaagccttacattaagtgggatttgttaaaatatgacttcacggaagagaggttaaaactctttgaccgttattttaaatattgggatcagacataccacccaaattgtgttaactgtttggatgacagatgcattctgcattgtgcaaactttaatgttttattctctacagtgttcccacctacaagttttggaccactagtgagaaaaatatttgttgatggtgttccatttgtagtttcaactggataccacttcagagagctaggtgttgtacataatcaggatgtaaacttacatagctctagacttagttttaaggaattacttgtgtatgctgctgaccctgctatgcacgctgcttctggtaatctattactagataaacgcactacgtgcttttcagtagctgcacttactaacaatgttgcttttcaaactgtcaaacccggtaattttaacaaagacttctatgactttgctgtgtctaagggtttctttaaggaaggaagttctgttgaattaaaacacttcttctttgctcaggatggtaatgctgctatcagcgattatgactactatcgttataatctaccaacaatgtgtgatatcagacaactactatttgtagttgaagttgttgataagtactttgattgttacgatggtggctgtattaatgctaaccaagtcatcgtcaacaacctagacaaatcagctggttttccatttaataaatggggtaaggctagactttattatgattcaatgagttatgaggatcaagatgcacttttcgcatatacaaaacgtaatgtcatccctactataactcaaatgaatcttaagtatgccattagtgcaaagaatagagctcgcaccgtagctggtgtctctatctgtagtactatgaccaatagacagtttcatcaaaaattattgaaatcaatagccgccactagaggagctactgtagtaattggaacaagcaaattctatggtggttggcacaacatgttaaaaactgtttatagtgatgtagaaaaccctcaccttatgggttgggattatcctaaatgtgatagagccatgcctaacatgcttagaattatggcctcacttgttcttgctcgcaaacatacaacgtgttgtagcttgtcacaccgtttctatagattagctaatgagtgtgctcaagtattgagtgaaatggtcatgtgtggcggttcactatatgttaaaccaggtggaacctcatcaggagatgccacaactgcttatgctaatagtgtttttaacatttgtcaagctgtcacggccaatgttaatgcacttttatctactgatggtaacaaaattgccgataagtatgtccgcaatttacaacacagactttatgagtgtctctatagaaatagagatgttgacacagactttgtgaatgagttttacgcatatttgcgtaaacatttctcaatgatgatactctctgacgatgctgttgtgtgtttcaatagcacttatgcatctcaaggtctagtggctagcataaagaactttaagtcagttctttattatcaaaacaatgtttttatgtctgaagcaaaatgttggactgagactgaccttactaaaggacctcatgaattttgctctcaacatacaatgctagttaaacagggtgatgattatgtgtaccttccttacccagatccatcaagaatcctaggggccggctgttttgtagatgatatcgtaaaaacagatggtacacttatgattgaacggttcgtgtctttagctatagatgcttacccacttactaaacatcctaatcaggagtatgctgatgtctttcatttgtacttacaatacataagaaagctacatgatgagttaacaggacacatgttagacatgtattctgttatgcttactaatgataacacttcaaggtattgggaacctgagttttatgaggctatgtacacaccgcatacagtcttacaggctgttggggcttgtgttctttgcaattcacagacttcattaagatgtggtgcttgcatacgtagaccattcttatgttgtaaatgctgttacgaccatgtcatatcaacatcacataaattagtcttgtctgttaatccgtatgtttgcaatgctccaggttgtgatgtcacagatgtgactcaactttacttaggaggtatgagctattattgtaaatcacataaaccacccattagttttccattgtgtgctaatggacaagtttttggtttatataaaaatacatgtgttggtagcgataatgttactgactttaatgcaattgcaacatgtgactggacaaatgctggtgattacattttagctaacacctgtactgaaagactcaagctttttgcagcagaaacgctcaaagctactgaggagacatttaaactgtcttatggtattgctactgtacgtgaagtgctgtctgacagagaattacatctttcatgggaagttggtaaacctagaccaccacttaaccgaaattatgtctttactggttatcgtgtaactaaaaacagtaaagtacaaataggagagtacacctttgaaaaaggtgactatggtgatgctgttgtttaccgaggtacaacaacttacaaattaaatgttggtgattattttgtgctgacatcacatacagtaatgccattaagtgcacctacactagtgccacaagagcactatgttagaattactggcttatacccaacactcaatatctcagatgagttttctagcaatgttgcaaattatcaaaaggttggtatgcaaaagtattctacactccagggaccacctggtactggtaagagtcattttgctattggcctagctctctactacccttctgctcgcatagtgtatacagcttgctctcatgccgctgttgatgcactatgtgagaaggcattaaaatatttgcctatagataaatgtagtagaattatacctgcacgtgctcgtgtagagtgttttgataaattcaaagtgaattcaacattagaacagtatgtcttttgtactgtaaatgcattgcctgagacgacagcagatatagttgtctttgatgaaatttcaatggccacaaattatgatttgagtgttgtcaatgccagattacgtgctaagcactatgtgtacattggcgaccctgctcaattacctgcaccacgcacattgctaactaagggcacactagaaccagaatatttcaattcagtgtgtagacttatgaaaactataggtccagacatgttcctcggaacttgtcggcgttgtcctgctgaaattgttgacactgtgagtgctttggtttatgataataagcttaaagcacataaagacaaatcagctcaatgctttaaaatgttttataagggtgttatcacgcatgatgtttcatctgcaattaacaggccacaaataggcgtggtaagagaattccttacacgtaaccctgcttggagaaaagctgtctttatttcaccttataattcacagaatgctgtagcctcaaagattttgggactaccaactcaaactgttgattcatcacagggctcagaatatgactatgtcatattcactcaaaccactgaaacagctcactcttgtaatgtaaacagatttaatgttgctattaccagagcaaaagtaggcatactttgcataatgtctgatagagacctttatgacaagttgcaatttacaagtcttgaaattccacgtaggaatgtggcaactttacaagctgaaaatgtaacaggactctttaaagattgtagtaaggtaatcactgggttacatcctacacaggcacctacacacctcagtgttgacactaaattcaaaactgaaggtttatgtgttgacatacctggcatacctaaggacatgacctatagaagactcatctctatgatgggttttaaaatgaattatcaagttaatggttaccctaacatgtttatcacccgcgaagaagctataagacatgtacgtgcatggattggcttcgatgtcgaggggtgtcatgctactagagaagctgttggtaccaatttacctttacagctaggtttttctacaggtgttaacctagttgctgtacctacaggttatgttgatacacctaataatacagatttttccagagttagtgctaaaccaccgcctggagatcaatttaaacacctcataccacttatgtacaaaggacttccttggaatgtagtgcgtataaagattgtacaaatgttaagtgacacacttaaaaatctctctgacagagtcgtatttgtcttatgggcacatggctttgagttgacatctatgaagtattttgtgaaaataggacctgagcgcacctgttgtctatgtgatagacgtgccacatgcttttccactgcttcagacacttatgcctgttggcatcattctattggatttgattacgtctataatccgtttatgattgatgttcaacaatggggttttacaggtaacctacaaagcaaccatgatctgtattgtcaagtccatggtaatgcacatgtagctagttgtgatgcaatcatgactaggtgtctagctgtccacgagtgctttgttaagcgtgttgactggactattgaatatcctataattggtgatgaactgaagattaatgcggcttgtagaaaggttcaacacatggttgttaaagctgcattattagcagacaaattcccagttcttcacgacattggtaaccctaaagctattaagtgtgtacctcaagctgatgtagaatggaagttctatgatgcacagccttgtagtgacaaagcttataaaatagaagaattattctattcttatgccacacattctgacaaattcacagatggtgtatgcctattttggaattgcaatgtcgatagatatcctgctaattccattgtttgtagatttgacactagagtgctatctaaccttaacttgcctggttgtgatggtggcagtttgtatgtaaataaacatgcattccacacaccagcttttgataaaagtgcttttgttaatttaaaacaattaccatttttctattactctgacagtccatgtgagtctcatggaaaacaagtagtgtcagatatagattatgtaccactaaagtctgctacgtgtataacacgttgcaatttaggtggtgctgtctgtagacatcatgctaatgagtacagattgtatctcgatgcttataacatgatgatctcagctggctttagcttgtgggtttacaaacaatttgatacttataacctctggaacacttttacaagacttcagagtttagaaaatgtggcttttaatgttgtaaataagggacactttgatggacaacagggtgaagtaccagtttctatcattaataacactgtttacacaaaagttgatggtgttgatgtagaattgtttgaaaataaaacaacattacctgttaatgtagcatttgagctttgggctaagcgcaacattaaaccagtaccagaggtgaaaatactcaataatttgggtgtggacattgctgctaatactgtgatctgggactacaaaagagatgctccagcacatatatctactattggtgtttgttctatgactgacatagccaagaaaccaactgaaacgatttgtgcaccactcactgtcttttttgatggtagagttgatggtcaagtagacttatttagaaatgcccgtaatggtgttcttattacagaaggtagtgttaaaggtttacaaccatctgtgggtcccaaacaagctagtcttaatggagtcacattaattggagaagccgtaaaaacacagttcaattattataagaaagttgatggtgttgtccaacaattacctgaaacttactttactcagagtagaaatttacaagaatttaaacccaggagtcaaatggaaattgatttcttagaattagctatggatgaattcattgaacggtataaattagaaggctatgccttcgaacatatcgtttatggagattttagtcatagtcagttaggtggtttacatctactgattggactagctaaacgttttaaggaatcaccttttgaattagaagattttattcctatggacagtacagttaaaaactatttcataacagatgcgcaaacaggttcatctaagtgtgtgtgttctgttattgatttattacttgatgattttgttgaaataataaaatcccaagatttatctgtagtttctaaggttgtcaaagtgactattgactatacagaaatttcatttatgctttggtgtaaagatggccatgtagaaacattttacccaaaattacaatctagtcaagcgtggcaaccgggtgttgctatgcctaatctttacaaaatgcaaagaatgctattagaaaagtgtgaccttcaaaattatggtgatagtgcaacattacctaaaggcataatgatgaatgtcgcaaaatatactcaactgtgtcaatatttaaacacattaacattagctgtaccctataatatgagagttatacattttggtgctggttctgataaaggagttgcaccaggtacagctgttttaagacagtggttgcctacgggtacgctgcttgtcgattcagatcttaatgactttgtctctgatgcagattcaactttgattggtgattgtgcaactgtacatacagctaataaatgggatctcattattagtgatatgtacgaccctaagactaaaaatgttacaaaagaaaatgactctaaagagggttttttcacttacatttgtgggtttatacaacaaaagctagctcttggaggttccgtggctataaagataacagaacattcttggaatgctgatctttataagctcatgggacacttcgcatggtggacagcctttgttactaatgtgaatgcgtcatcatctgaagcatttttaattggatgtaattatcttggcaaaccacgcgaacaaatagatggttatgtcatgcatgcaaattacatattttggaggaatacaaatccaattcagttgtcttcctattctttatttgacatgagtaaatttccccttaaattaaggggtactgctgttatgtctttaaaagaaggtcaaatcaatgatatgattttatctcttcttagtaaaggtagacttataattagagaaaacaacagagttgttatttctagtgatgttcttgttaacaactaaacgaacaatgtttgtttttcttgttttattgccactagtctctagtcagtgtgttaatcttacaaccagaactcaattaccccctgcatacactaattctttcacacgtggtgtttattaccctgacaaagttttcagatcctcagttttacattcaactcaggacttgttcttacctttcttttccaatgttacttggttccatgctatacatgtctctgggaccaatggtactaagaggtttgataaccctgtcctaccatttaatgatggtgtttattttgcttccactgagaagtctaacataataagaggctggatttttggtactactttagattcgaagacccagtccctacttattgttaataacgctactaatgttgttattaaagtctgtgaatttcaattttgtaatgatccatttttgggtgtttattaccacaaaaacaacaaaagttggatggaaagtgagttcagagtttattctagtgcgaataattgcacttttgaatatgtctctcagccttttcttatggaccttgaaggaaaacagggtaatttcaaaaatcttagggaatttgtgtttaagaatattgatggttattttaaaatatattctaagcacacgcctattaatttagtgcgtgatctccctcagggtttttcggctttagaaccattggtagatttgccaataggtattaacatcactaggtttcaaactttacttgctttacatagaagttatttgactcctggtgattcttcttcaggttggacagctggtgctgcagcttattatgtgggttatcttcaacctaggacttttctattaaaatataatgaaaatggaaccattacagatgctgtagactgtgcacttgaccctctctcagaaacaaagtgtacgttgaaatccttcactgtagaaaaaggaatctatcaaacttctaactttagagtccaaccaacagaatctattgttagatttcctaatattacaaacttgtgcccttttggtgaagtttttaacgccaccagatttgcatctgtttatgcttggaacaggaagagaatcagcaactgtgttgctgattattctgtcctatataattccgcatcattttccacttttaagtgttatggagtgtctcctactaaattaaatgatctctgctttactaatgtctatgcagattcatttgtaattagaggtgatgaagtcagacaaatcgctccagggcaaactggaaagattgctgattataattataaattaccagatgattttacaggctgcgttatagcttggaattctaacaatcttgattctaaggttggtggtaattataattacctgtatagattgtttaggaagtctaatctcaaaccttttgagagagatatttcaactgaaatctatcaggccggtagcacaccttgtaatggtgttgaaggttttaattgttactttcctttacaatcatatggtttccaacccactaatggtgttggttaccaaccatacagagtagtagtactttcttttgaacttctacatgcaccagcaactgtttgtggacctaaaaagtctactaatttggttaaaaacaaatgtgtcaatttcaacttcaatggtttaacaggcacaggtgttcttactgagtctaacaaaaagtttctgcctttccaacaatttggcagagacattgctgacactactgatgctgtccgtgatccacagacacttgagattcttgacattacaccatgttcttttggtggtgtcagtgttataacaccaggaacaaatacttctaaccaggttgctgttctttatcaggatgttaactgcacagaagtccctgttgctattcatgcagatcaacttactcctacttggcgtgtttattctacaggttctaatgtttttcaaacacgtgcaggctgtttaataggggctgaacatgtcaacaactcatatgagtgtgacatacccattggtgcaggtatatgcgctagttatcagactcagactaattctcctcggcgggcacgtagtgtagctagtcaatccatcattgcctacactatgtcacttggtgcagaaaattcagttgcttactctaataactctattgccatacccacaaattttactattagtgttaccacagaaattctaccagtgtctatgaccaagacatcagtagattgtacaatgtacatttgtggtgattcaactgaatgcagcaatcttttgttgcaatatggcagtttttgtacacaattaaaccgtgctttaactggaatagctgttgaacaagacaaaaacacccaagaagtttttgcacaagtcaaacaaatttacaaaacaccaccaattaaagattttggtggttttaatttttcacaaatattaccagatccatcaaaaccaagcaagaggtcatttattgaagatctacttttcaacaaagtgacacttgcagatgctggcttcatcaaacaatatggtgattgccttggtgatattgctgctagagacctcatttgtgcacaaaagtttaacggccttactgttttgccacctttgctcacagatgaaatgattgctcaatacacttctgcactgttagcgggtacaatcacttctggttggacctttggtgcaggtgctgcattacaaataccatttgctatgcaaatggcttataggtttaatggtattggagttacacagaatgttctctatgagaaccaaaaattgattgccaaccaatttaatagtgctattggcaaaattcaagactcactttcttccacagcaagtgcacttggaaaacttcaagatgtggtcaaccaaaatgcacaagctttaaacacgcttgttaaacaacttagctccaattttggtgcaatttcaagtgttttaaatgatatcctttcacgtcttgacaaagttgaggctgaagtgcaaattgataggttgatcacaggcagacttcaaagtttgcagacatatgtgactcaacaattaattagagctgcagaaatcagagcttctgctaatcttgctgctactaaaatgtcagagtgtgtacttggacaatcaaaaagagttgatttttgtggaaagggctatcatcttatgtccttccctcagtcagcacctcatggtgtagtcttcttgcatgtgacttatgtccctgcacaagaaaagaacttcacaactgctcctgccatttgtcatgatggaaaagcacactttcctcgtgaaggtgtctttgtttcaaatggcacacactggtttgtaacacaaaggaatttttatgaaccacaaatcattactacagacaacacatttgtgtctggtaactgtgatgttgtaataggaattgtcaacaacacagtttatgatcctttgcaacctgaattagactcattcaaggaggagttagataaatattttaagaatcatacatcaccagatgttgatttaggtgacatctctggcattaatgcttcagttgtaaacattcaaaaagaaattgaccgcctcaatgaggttgccaagaatttaaatgaatctctcatcgatctccaagaacttggaaagtatgagcagtatataaaatggccatggtacatttggctaggttttatagctggcttgattgccatagtaatggtgacaattatgctttgctgtatgaccagttgctgtagttgtctcaagggctgttgttcttgtggatcctgctgcaaatttgatgaagacgactctgagccagtgctcaaaggagtcaaattacattacacataattcctgatcttctggtctaaacgaactaaatattatattagtttttctgtttggaactttaattttagccatggcagattccaacggtactattaccgttgaagagcttaaaaagctccttgaacaatggaacctagtaataggtttcctattccttacatggatttgtcttctacaatttgcctatgccaacaggaataggtttttgtatataattaagttaattttcctctggctgttatggccagtaactttagcttgttttgtgcttgctgctgtttacagaataaattggatcaccggtggaattgctatcgcaatggcttgtcttgtaggcttgatgtggctcagctacttcattgcttctttcagactgtttgcgcgtacccgttccatgtggtcattcaatccagaaactaacattcttctcaacgtgccactccatggcactattctgaccagaccgcttctagaaagtgaactcgtaatcggagctgtgatccttcgtggacatcttcgtattgctggacaccatctaggacgctgtgacatcaaggacctgcctaaagaaatcactgttgctacatcacgaacgctttcttattacaaattgggagcttcgcagcgtgtagcaggtgactcaggttttgctgcatacagtcgctacaggattggcaactataaattaaacacagaccattccagtagcagtgacaatattgctttgcttgtacagtaagtgacaacagatgtttcatctcgttgactttcaggttactatagcagagatattactaattattatgaggacttttaaagtttccatttggaatcttgattacatcataaacctcataattaaaaatttatctaagtcactaactgagaataaatattctcaattagatgaagagcaaccaatggagattgattaattgttttagatttcatctaaacgaacaaactaaaatgtctgataatggaccccaaaatcagcgaaatgcaccccgcattacgtttggtggaccctcagattcaactggcagtaaccagaatggagaacgcagtggggcgcgatcaaaacaacgtcggccccaaggtttacccaataatactgcgtcttggttcaccgctctcactcaacatggcaaggaagaccttaaattccctcgaggacaaggcgttccaattaacaccaatagcagtccagatgaccaaattggctactaccgaagagctaccagacgaattcgtggtggtgacggtaaaatgaaagatctcagtccaagatggtatttctactacctaggaactgggccagaagctggacttccctatggtgctaacaaagacggcatcatatgggttgcaactgagggagccttgaatacaccaaaagatcacattggcacccgcaatcctgctaacaatgctgcaatcgtgctacaacttcctcaaggaacaacattgccaaaaggcttctacgcagaagggagcagaggcggcagtcaagcctcttctcgttcctcatcacgtagtcgcaacagttcaagaaattcaactccaggcagcagtaggggaacttctcctgctagaatggctggcaatggcggtgatgctgctcttgctttgctgctgcttgacagattgaaccagcttgagagcaaaatgtctggtaaaggccaacaacaacaaggccaaactgtcactaagaaatctgctgctgaggcttctaagaagcctcggcaaaaacgtactgccactaaagcatacaatgtaacacaagctttcggcagacgtggtccagaacaaacccaaggaaattttggggaccaggaactaatcagacaaggaactgattacaaacattggccgcaaattgcacaatttgcccccagcgcttcagcgttcttcggaatgtcgcgcattggcatggaagtcacaccttcgggaacgtggttgacctacacaggtgccatcaaattggatgacaaagatccaaatttcaaagatcaagtcattttgctgaataagcatattgacgcatacaaaacattcccaccaacagagcctaaaaaggacaaaaagaagaaggctgatgaaactcaagccttaccgcagagacagaagaaacagcaaactgtgactcttcttcctgctgcagatttggatgatttctccaaacaattgcaacaatccatgagcagtgctgactcaactcaggcctaaactcatgcagaccacacaaggcagatgggctatataaacgttttcgcttttccgtttacgatatatagtctactcttgtgcagaatgaattctcgtaactacatagcacaagtagatgtagttaactttaatctcacatagcaatctttaatcagtgtgtaacattagggaggacttgaaagagccaccacattttcaccgaggccacgcggagtacgatcgagtgtacagtgaacaatgctagggagagctgcctatatggaagagccctaatgtgtaaaattaattttagtagtgctatccccatgtgattttaatagcttcttaggagaatgacaaaaaaaaaaaaaaaaaaaaaaaaa

SEQ ID NO: 44 - DNA, 28308 bp, Coronaviridae
  source 1..28308: mol_type = other DNA
  misc_feature 1..28308: note = SARS-CoV-2-[3,E,6,8] polynucleotide sequence
attaaaggtttataccttcccaggtaacaaaccaaccaactttcgatctcttgtagatctgttctctaaacgaactttaaaatctgtgtggctgtcactcggctgcatgcttagtgcactcacgcagtataattaataactaattactgtcgttgacaggacacgagtaactcgtctatcttctgcaggctgcttacggtttcgtccgtgttgcagccgatcatcagcacatctaggtttcgtccgggtgtgaccgaaaggtaagatggagagccttgtccctggtttcaacgagaaaacacacgtccaactcagtttgcctgttttacaggttcgcgacgtgctcgtacgtggctttggagactccgtggaggaggtcttatcagaggcacgtcaacatcttaaagatggcacttgtggcttagtagaagttgaaaaaggcgttttgcctcaacttgaacagccctatgtgttcatcaaacgttcggatgctcgaactgcacctcatggtcatgttatggttgagctggtagcagaactcgaaggcattcagtacggtcgtagtggtgagacacttggtgtccttgtccctcatgtgggcgaaataccagtggcttaccgcaaggttcttcttcgtaagaacggtaataaaggagctggtggccatagttacggcgccgatctaaagtcatttgacttaggcgacgagcttggcactgatccttatgaagattttcaagaaaactggaacactaaacatagcagtggtgttacccgtgaactcatgcgtgagcttaacggaggggcatacactcgctatgtcgataacaacttctgtggccctgatggctaccctcttgagtgcattaaagaccttctagcacgtgctggtaaagcttcatgcactttgtccgaacaactggactttattgacactaagaggggtgtatactgctgccgtgaacatgagcatgaaattgcttggtacacggaacgttctgaaaagagctatgaattgcagacaccttttgaaattaaattggcaaagaaatttgacaccttcaatggggaatgtccaaattttgtatttcccttaaattccataatcaagactattcaaccaagggttgaaaagaaaaagcttgatggctttatgggtagaattcgatctgtctatccagttgcgtcaccaaatgaatgcaaccaaatgtgcctttcaactctcatgaagtgtgatcattgtggtgaaacttcatggcagacgggcgattttgttaaagccacttgcgaattttgtggcactgagaatttgactaaagaaggtgccactacttgtggttacttaccccaaaatgctgttgttaaaatttattgtccagcatgtcacaattcagaagtaggacctgagcatagtcttgccgaataccataatgaatctggcttgaaaaccattcttcgtaagggtggtcgcactattgcctttggaggctgtgtgttctcttatgttggttgccataacaagtgtgcctattgggttccacgtgctagcgctaacataggttgtaaccatacaggtgttgttggagaaggttccgaaggtcttaatgacaaccttcttgaaatactccaaaaagagaaagtcaacatcaatattgttggtgactttaaacttaatgaagagatcgccattattttggcatctttttctgcttccacaagtgcttttgtggaaactgtgaaaggtttggattataaagcattcaaacaaattgttgaatcctgtggtaattttaaagttacaaaaggaaaagctaaaaaaggtgcctggaatattggtgaacagaaatcaatactgagtcctctttatgcatttgcatcagaggctgctcgtgttgtacgatcaattttctcccgcactcttgaaactgctcaaaattctgtgcgtgttttacagaaggccgctataacaatactagatggaatttcacagtattcactgagactcattgatgctatgatgttcacatctgatttggctactaacaatctagttgtaatggcctacattacaggtggtgttgttcagttgacttcgcagtggctaactaacatctttggcactgtttatgaaaaactcaaacccgtccttgattggcttgaagagaagtttaaggaaggtgtagagtttcttagagacggttgggaaattgttaaatttatctcaacctgtgcttgtgaaattgtcggtggacaaattgtcacctgtgcaaaggaaattaaggagagtgttcagacattctttaagcttgtaaataaatttttggctttgtgtgctgactctatcattattggtggagctaaacttaaagccttgaatttaggtgaaacatttgtcacgcactcaaagggattgtacagaaagtgtgttaaatccagagaagaaactggcctactcatgcctctaaaagccccaaaagaaattatcttcttagagggagaaacacttcccacagaagtgttaacagaggaagttgtcttgaaaactggtgatttacaaccattagaacaacctactagtgaagctgttgaagctccattggttggtacaccagtttgtattaacgggcttatgttgctcgaaatcaaagacacagaaaagtactgtgcccttgcacctaatatgatggtaacaaacaataccttcacactcaaaggcggtgcaccaacaaaggttacttttggtgatgacactgtgatagaagtgcaaggttacaagagtgtgaatatcacttttgaacttgatgaaaggattgataaagtacttaatgagaagtgctctgcctatacagttgaactcggtacagaagtaaatgagttcgcctgtgttgtggcagatgctgtcataaaaactttgcaaccagtatctgaattacttacaccactgggcattgatttagatgagtggagtatggctacatactacttatttgatgagtctggtgagtttaaattggcttcacatatgtattgttctttctaccctccagatgaggatgaagaagaaggtgattgtgaagaagaagagtttgagccatcaactcaatatgagtatggtactgaagatgattaccaaggtaaacctttggaatttggtgccacttctgctgctcttcaacctgaagaagagcaagaagaagattggttagatgatgatagtcaacaaactgttggtcaacaagacggcagtgaggacaatcagacaactactattcaaacaattgttgaggttcaacctcaattagagatggaacttacaccagttgttcagactattgaagtgaatagttttagtggttatttaaaacttactgacaatgtatacattaaaaatgcagacattgtggaagaagctaaaaaggtaaaaccaacagtggttgttaatgcagccaatgtttaccttaaacatggaggaggtgttgcaggagccttaaataaggctactaacaatgccatgcaagttgaatctgatgattacatagctactaatggaccacttaaagtgggtggtagttgtgttttaagcggacacaatcttgctaaacactgtcttcatgttgtcggcccaaatgttaacaaaggtgaagacattcaacttcttaagagtgcttatgaaaattttaatcagcacgaagttctacttgcaccattattatcagctggtatttttggtgctgaccctatacattctttaagagtttgtgtagatactgttcgcacaaatgtctacttagctgtctttgataaaaatctctatgacaaacttgtttcaagctttttggaaatgaagagtgaaaagcaagttgaacaaaagatcgctgagattcctaaagaggaagttaagccatttataactgaaagtaaaccttcagttgaacagagaaaacaagatgataagaaaatcaaagcttgtgttgaagaagttacaacaactctggaagaaactaagttcctcacagaaaacttgttactttatattgacattaatggcaatcttcatccagattctgccactcttgttagtgacattgacatcactttcttaaagaaagatgctccatatatagtgggtgatgttgttcaagagggtgttttaactgctgtggttatacctactaaaaaggctggtggcactactgaaatgctagcgaaagctttgagaaaagtgccaacagacaattatataaccacttacccgggtcagggtttaaatggttacactgtagaggaggcaaagacagtgcttaaaaagtgtaaaagtgccttttacattctaccatctattatctctaatgagaagcaagaaattcttggaactgtttcttggaatttgcgagaaatgcttgcacatgcagaagaaacacgcaaattaatgcctgtctgtgtggaaactaaagccatagtttcaactatacagcgtaaatataagggtattaaaatacaagagggtgtggttgattatggtgctagattttacttttacaccagtaaaacaactgtagcgtcacttatcaacacacttaacgatctaaatgaaactcttgttacaatgccacttggctatgtaacacatggcttaaatttggaagaagctgctcggtatatgagatctctcaaagtgccagctacagtttctgtttcttcacctgatgctgttacagcgtataatggttatcttacttcttcttctaaaacacctgaagaacattttattgaaaccatctcacttgctggttcctataaagattggtcctattctggacaatctacacaactaggtatagaatttcttaagagaggtgataaaagtgtatattacactagtaatcctaccacattccacctagatggtgaagttatcacctttgacaatcttaagacacttctttctttgagagaagtgaggactattaaggtgtttacaacagtagacaacattaacctccacacgcaagttgtggacatgtcaatgacatatggacaacagtttggtccaacttatttggatggagctgatgttactaaaataaaacctcataattcacatgaaggtaaaacattttatgttttacctaatgatgacactctacgtgttgaggcttttgagtactaccacacaactgatcctagttttctgggtaggtacatgtcagcattaaatcacactaaaaagtggaaatacccacaagttaatggtttaacttctattaaatgggcagataacaactgttatcttgccactgcattgttaacactccaacaaatagagttgaagtttaatccacctgctctacaagatgcttattacagagcaagggctggtgaagctgctaacttttgtgcacttatcttagcctactgtaataagacagtaggtgagttaggtgatgttagagaaacaatgagttacttgtttcaacatgccaatttagattcttgcaaaagagtcttgaacgtggtgtgtaaaacttgtggacaacagcagacaacccttaagggtgtagaagctgttatgtacatgggcacactttcttatgaacaatttaagaaaggtgttcagataccttgtacgtgtggtaaacaagctacaaaatatctagtacaacaggagtcaccttttgttatgatgtcagcaccacctgctcagtatgaacttaagcatggtacatttacttgtgctagtgagtacactggtaattaccagtgtggtcactataaacatataacttctaaagaaactttgtattgcatagacggtgctttacttacaaagtcctcagaatacaaaggtcctattacggatgttttctacaaagaaaacagttacacaacaaccataaaaccagttacttataaattggatggtgttgtttgtacagaaattgaccctaagttggacaattattataagaaagacaattcttatttcacagagcaaccaattgatcttgtaccaaaccaaccatatccaaacgcaagcttcgataattttaagtttgtatgtgataatatcaaatttgctgatgatttaaaccagttaactggttataagaaacctgcttcaagagagcttaaagttacatttttccctgacttaaatggtgatgtggtggctattgattataaacactacacaccctcttttaagaaaggagctaaattgttacataaacctattgtttggcatgttaacaatgcaactaataaagccacgtataaaccaaatacctggtgtatacgttgtctttggagcacaaaaccagttgaaacatcaaattcgtttgatgtactgaagtcagaggacgcgcagggaatggataatcttgcctgcgaagatctaaaaccagtctctgaagaagtagtggaaaatcctaccatacagaaagacgttcttgagtgtaatgtgaaaactaccgaagttgtaggagacattatacttaaaccagcaaataatagtttaaaaattacagaagaggttggccacacagatctaatggctgcttatgtagacaattctagtcttactattaagaaacctaatgaattatctagagtattaggtttgaaaacccttgctactcatggtttagctgctgttaatagtgtcccttgggatactatagctaattatgctaagccttttcttaacaaagttgttagtacaactactaacatagttacacggtgtttaaaccgtgtttgtactaattatatgccttatttctttactttattgctacaattgtgtacttttactagaagtacaaattctagaattaaagcatctatgccgactactatagcaaagaatactgttaagagtgtcggtaaattttgtctagaggcttcatttaattatttgaagtcacctaatttttctaaactgataaatattataatttggtttttactattaagtgtttgcctaggttctttaatctactcaaccgctgctttaggtgttttaatgtctaatttaggcatgccttcttactgtactggttacagagaaggctatttgaactctactaatgtcactattgcaacctactgtactggttctataccttgtagtgtttgtcttagtggtttagattctttagacacctatccttctttagaaactatacaaattaccatttcatcttttaaatgggatttaactgcttttggcttagttgcagagtggtttttggcatatattcttttcactaggtttttctatgtacttggattggctgcaatcatgcaattgtttttcagctattttgcagtacattttattagtaattcttggcttatgtggttaataattaatcttgtacaaatggccccgatttcagctatggttagaatgtacatcttctttgcatcattttattatgtatggaaaagttatgtgcatgttgtagacggttgtaattcatcaacttgtatgatgtgttacaaacgtaatagagcaacaagagtcgaatgtacaactattgttaatggtgttagaaggtccttttatgtctatgctaatggaggtaaaggcttttgcaaactacacaattggaattgtgttaattgtgatacattctgtgctggtagtacatttattagtgatgaagttgcgagagacttgtcactacagtttaaaagaccaataaatcctactgaccagtcttcttacatcgttgatagtgttacagtgaagaatggttccatccatctttactttgataaagctggtcaaaagacttatgaaagacattctctctctcattttgttaacttagacaacctgagagctaataacactaaaggttcattgcctattaatgttatagtttttgatggtaaatcaaaatgtgaagaatcatctgcaaaatcagcgtctgtttactacagtcagcttatgtgtcaacctatactgttactagatcaggcattagtgtctgatgttggtgatagtgcggaagttgcagttaaaatgtttgatgcttacgttaatacgttttcatcaacttttaacgtaccaatggaaaaactcaaaacactagttgcaactgcagaagctgaacttgcaaagaatgtgtccttagacaatgtcttatctacttttatttcagcagctcggcaagggtttgttgattcagatgtagaaactaaagatgttgttgaatgtcttaaattgtcacatcaatctgacatagaagttactggcgatagttgtaataactatatgctcacctataacaaagttgaaaacatgacaccccgtgaccttggtgcttgtattgactgtagtgcgcgtcatattaatgcgcaggtagcaaaaagtcacaacattgctttgatatggaacgttaaagatttcatgtcattgtctgaacaactacgaaaacaaatacgtagtgctgctaaaaagaataacttaccttttaagttgacatgtgcaactactagacaagttgttaatgttgtaacaacaaagatagcacttaagggtggtaaaattgttaataattggttgaagcagttaattaaagttacacttgtgttcctttttgttgctgctattttctatttaataacacctgttcatgtcatgtctaaacatactgacttttcaagtgaaatcataggatacaaggctattgatggtggtgtcactcgtgacatagcatctacagatacttgttttgctaacaaacatgctgattttgacacatggtttagccagcgtggtggtagttatactaatgacaaagcttgcccattgattgctgcagtcataacaagagaagtgggttttgtcgtgcctggtttgcctggcacgatattacgcacaactaatggtgactttttgcatttcttacctagagtttttagtgcagttggtaacatctgttacacaccatcaaaacttatagagtacactgactttgcaacatcagcttgtgttttggctgctgaatgtacaatttttaaagatgcttctggtaagccagtaccatattgttatgataccaatgtactagaaggttctgttgcttatgaaagtttacgccctgacacacgttatgtgctcatggatggctctattattcaatttcctaacacctaccttgaaggttctgttagagtggtaacaacttttgattctgagtactgtaggcacggcacttgtgaaagatcagaagctggtgtttgtgtatctactagtggtagatgggtacttaacaatgattattacagatctttaccaggagttttctgtggtgtagatgctgtaaatttacttactaatatgtttacaccactaattcaacctattggtgctttggacatatcagcatctatagtagctggtggtattgtagctatcgtagtaacatgccttgcctactattttatgaggtttagaagagcttttggtgaatacagtcatgtagttgcctttaatactttactattccttatgtcattcactgtactctgtttaacaccagtttactcattcttacctggtgtttattctgttatttacttgtacttgacattttatcttactaatgatgtttcttttttagcacatattcagtggatggttatgttcacacctttagtacctttctggataacaattgcttatatcatttgtatttccacaaagcatttctattggttctttagtaattacctaaagagacgtgtagtctttaatggtgtttcctttagtacttttgaagaagctgcgctgtgcacctttttgttaaataaagaaatgtatctaaagttgcgtagtgatgtgctattacctcttacgcaatataatagatacttagctctttataataagtacaagtattttagtggagcaatggatacaactagctacagagaagctgcttgttgtcatctcgcaaaggctctcaatgacttcagtaactcaggttctgatgttctttaccaaccaccacaaacctctatcacctcagctgttttgcagagtggttttagaaaaatggcattcccatctggtaaagttgagggttgtatggtacaagtaacttgtggtacaactacacttaacggtctttggcttgatgacgtagtttactgtccaagacatgtgatctgcacctctgaagacatgcttaaccctaattatgaagatttactcattcgtaagtctaatcataatttcttggtacaggctggtaatgttcaactcagggttattggacattctatgcaaaattgtgtacttaagcttaaggttgatacagccaatcctaagacacctaagtataagtttgttcgcattcaaccaggacagactttttcagtgttagcttgttacaatggttcaccatctggtgtttaccaatgtgctatgaggcccaatttcactattaagggttcattccttaatggttcatgtggtagtgttggttttaacatagattatgactgtgtctctttttgttacatgcaccatatggaattaccaactggagttcatgctggcacagacttagaaggtaacttttatggaccttttgttgacaggcaaacagcacaagcagctggtacggacacaactattacagttaatgttttagcttggttgtacgctgctgttataaatggagacaggtggtttctcaatcgatttaccacaactcttaatgactttaaccttgtggctatgaagtacaattatgaacctctaacacaagaccatgttgacatactaggacctctttctgctcaaactggaattgccgttttagatatgtgtgcttcattaaaagaattactgcaaaatggtatgaatggacgtaccatattgggtagtgctttattagaagatgaatttacaccttttgatgttgttagacaatgctcaggtgttactttccaaagtgcagtgaaaagaacaatcaagggtacacaccactggttgttactcacaattttgacttcacttttagttttagtccagagtactcaatggtctttgttcttttttttgtatgaaaatgcctttttaccttttgctatgggtattattgctatgtctgcttttgcaatgatgtttgtcaaacataagcatgcatttctctgtttgtttttgttaccttctcttgccactgtagcttattttaatatggtctatatgcctgctagttgggtgatgcgtattatgacatggttggatatggttgatactagtttgtctggttttaagctaaaagactgtgttatgtatgcatcagctgtagtgttactaatccttatgacagcaagaactgtgtatgatgatggtgctaggagagtgtggacacttatgaatgtcttgacactcgtttataaagtttattatggtaatgctttagatcaagccatttccatgtgggctcttataatctctgttacttctaactactcaggtgtagttacaactgtcatgtttttggccagaggtattgtttttatgtgtgttgagtattgccctattttcttcataactggtaatacacttcagtgtataatgctagtttattgtttcttaggctatttttgtacttgttactttggcctcttttgtttactcaaccgctactttagactgactcttggtgtttatgattacttagtttctacacaggagtttagatatatgaattcacagggactactcccacccaagaatagcatagatgccttcaaactcaacattaaattgttgggtgttggtggcaaaccttgtatcaaagtagccactgtacagtctaaaatgtcagatgtaaagtgcacatcagtagtcttactctcagttttgcaacaactcagagtagaatcatcatctaaattgtgggctcaatgtgtccagttacacaatgacattctcttagctaaagatactactgaagcctttgaaaaaatggtttcactactttctgttttgctttccatgcagggtgctgtagacataaacaagctttgtgaagaaatgctggacaacagggcaaccttacaagctatagcctcagagtttagttcccttccatcatatgcagcttttgctactgctcaagaagcttatgagcaggctgttgctaatggtgattctgaagttgttcttaaaaagttgaagaagtctttgaatgtggctaaatctgaatttgaccgtgatgcagccatgcaacgtaagttggaaaagatggctgatcaagctatgacccaaatgtataaacaggctagatctgaggacaagagggcaaaagttactagtgctatgcagacaatgcttttcactatgcttagaaagttggataatgatgcactcaacaacattatcaacaatgcaagagatggttgtgttcccttgaacataatacctcttacaacagcagccaaactaatggttgtcataccagactataacacatataaaaatacgtgtgatggtacaacatttacttatgcatcagcattgtgggaaatccaacaggttgtagatgcagatagtaaaattgttcaacttagtgaaattagtatggacaattcacctaatttagcatggcctcttattgtaacagctttaagggccaattctgctgtcaaattacagaataatgagcttagtcctgttgcactacgacagatgtcttgtgctgccggtactacacaaactgcttgcactgatgacaatgcgttagcttactacaacacaacaaagggaggtaggtttgtacttgcactgttatccgatttacaggatttgaaatgggctagattccctaagagtgatggaactggtactatctatacagaactggaaccaccttgtaggtttgttacagacacacctaaaggtcctaaagtgaagtatttatactttattaaaggattaaacaacctaaatagaggtatggtacttggtagtttagctgccacagtacgtctacaagctggtaatgcaacagaagtgcctgccaattcaactgtattatctttctgtgcttttgctgtagatgctgctaaagcttacaaagattatctagctagtgggggacaaccaatcactaattgtgttaagatgttgtgtacacacactggtactggtcaggcaataacagttacaccggaagccaatatggatcaagaatcctttggtggtgcatcgtgttgtctgtactgccgttgccacatagatcatccaaatcctaaaggattttgtgacttaaaaggtaagtatgtacaaatacctacaacttgtgctaatgaccctgtgggttttacacttaaaaacacagtctgtaccgtctgcggtatgtggaaaggttatggctgtagttgtgatcaactccgcgaacccatgcttcagtcagctgatgcacaatcgtttttaaacgggtttgcggtgtaagtgcagcccgtcttacaccgtgcggcacaggcactagtactgatgtcgtatacagggcttttgacatctacaatgataaagtagctggttttgctaaattcctaaaaactaattgttgtcgcttccaagaaaaggacgaagatgacaatttaattgattcttactttgtagttaagagacacactttctctaactaccaacatgaagaaacaatttataatttacttaaggattgtccagctgttgctaaacatgacttctttaagtttagaatagacggtgacatggtaccacatatatcacgtcaacgtcttactaaatacacaatggcagacctcgtctatgctttaaggcattttgatgaaggtaattgtgacacattaaaagaaatacttgtcacatacaattgttgtgatgatgattatttcaataaaaaggactggtatgattttgtagaaaacccagatatattacgcgtatacgccaacttaggtgaacgtgtacgccaagctttgttaaaaacagtacaattctgtgatgccatgcgaaatgctggtattgttggtgtactgacattagataatcaagatctcaatggtaactggtatgatttcggtgatttcatacaaaccacgccaggtagtggagttcctgttgtagattcttattattcattgttaatgcctatattaaccttgaccagggctttaactgcagagtcacatgttgacactgacttaacaaagccttacattaagtgggatttgttaaaatatgacttcacggaagagaggttaaaactctttgaccgttattttaaatattgggatcagacataccacccaaattgtgttaactgtttggatgacagatgcattctgcattgtgcaaactttaatgttttattctctacagtgttcccacctacaagttttggaccactagtgagaaaaatatttgttgatggtgttccatttgtagtttcaactggataccacttcagagagctaggtgttgtacataatcaggatgtaaacttacatagctctagacttagttttaaggaattacttgtgtatgctgctgaccctgctatgcacgctgcttctggtaatctattactagataaacgcactacgtgcttttcagtagctgcacttactaacaatgttgcttttcaaactgtcaaacccggtaattttaacaaagacttctatgactttgctgtgtctaagggtttctttaaggaaggaagttctgttgaattaaaacacttcttctttgctcaggatggtaatgctgctatcagcgattatgactactatcgttataatctaccaacaatgtgtgatatcagacaactactatttgtagttgaagttgttgataagtactttgattgttacgatggtggctgtattaatgctaaccaagtcatcgtcaacaacctagacaaatcagctggttttccatttaataaatggggtaaggctagactttattatgattcaatgagttatgaggatcaagatgcacttttcgcatatacaaaacgtaatgtcatccctactataactcaaatgaatcttaagtatgccattagtgcaaagaatagagctcgcaccgtagctggtgtctctatctgtagtactatgaccaatagacagtttcatcaaaaattattgaaatcaatagccgccactagaggagctactgtagtaattggaacaagcaaattctatggtggttggcacaacatgttaaaaactgtttatagtgatgtagaaaaccctcaccttatgggttgggattatcctaaatgtgatagagccatgcctaacatgcttagaattatggcctcacttgttcttgctcgcaaacatacaacgtgttgtagcttgtcacaccgtttctatagattagctaatgagtgtgctcaagtattgagtgaaatggtcatgtgtggcggttcactatatgttaaaccaggtggaacctcatcaggagatgccacaactgcttatgctaatagtgtttttaacatttgtcaagctgtcacggccaatgttaatgcacttttatctactgatggtaacaaaattgccgataagtatgtccgcaatttacaacacagactttatgagtgtctctatagaaatagagatgttgacacagactttgtgaatgagttttacgcatatttgcgtaaacatttctcaatgatgatactctctgacgatgctgttgtgtgtttcaatagcacttatgcatctcaaggtctagtggctagcataaagaactttaagtcagttctttattatcaaaacaatgtttttatgtctgaagcaaaatgttggactgagactgaccttactaaaggacctcatgaattttgctctcaacatacaatgctagttaaacagggtgatgattatgtgtaccttccttacccagatccatcaagaatcctaggggccggctgttttgtagatgatatcgtaaaaacagatggtacacttatgattgaacggttcgtgtctttagctatagatgcttacccacttactaaacatcctaatcaggagtatgctgatgtctttcatttgtacttacaatacataagaaagctacatgatgagttaacaggacacatgttagacatgtattctgttatgcttactaatgataacacttcaaggtattgggaacctgagttttatgaggctatgtacacaccgcatacagtcttacaggctgttggggcttgtgttctttgcaattcacagacttcattaagatgtggtgcttgcatacgtagaccattcttatgttgtaaatgctgttacgaccatgtcatatcaacatcacataaattagtcttgtctgttaatccgtatgtttgcaatgctccaggttgtgatgtcacagatgtgactcaactttacttaggaggtatgagctattattgtaaatcacataaaccacccattagttttccattgtgtgctaatggacaagtttttggtttatataaaaatacatgtgttggtagcgataatgttactgactttaatgcaattgcaacatgtgactggacaaatgctggtgattacattttagctaacacctgtactgaaagactcaagctttttgcagcagaaacgctcaaagctactgaggagacatttaaactgtcttatggtattgctactgtacgtgaagtgctgtctgacagagaattacatctttcatgggaagttggtaaacctagaccaccacttaaccgaaattatgtctttactggttatcgtgtaactaaaaacagtaaagtacaaataggagagtacacctttgaaaaaggtgactatggtgatgctgttgtttaccgaggtacaacaacttacaaattaaatgttggtgattattttgtgctgacatcacatacagtaatgccattaagtgcacctacactagtgccacaagagcactatgttagaattactggcttatacccaacactcaatatctcagatgagttttctagcaatgttgcaaattatcaaaaggttggtatgcaaaagtattctacactccagggaccacctggtactggtaagagtcattttgctattggcctagctctctactacccttctgctcgcatagtgtatacagcttgctctcatgccgctgttgatgcactatgtgagaaggcattaaaatatttgcctatagataaatgtagtagaattatacctgcacgtgctcgtgtagagtgttttgataaattcaaagtgaattcaacattagaacagtatgtcttttgtactgtaaatgcattgcctgagacgacagcagatatagttgtctttgatgaaatttcaatggccacaaattatgatttgagtgttgtcaatgccagattacgtgctaagcactatgtgtacattggcgaccctgctcaattacctgcaccacgcacattgctaactaagggcacactagaaccagaatatttcaattcagtgtgtagacttatgaaaactataggtccagacatgttcctcggaacttgtcggcgttgtcctgctgaaattgttgacactgtgagtgctttggtttatgataataagcttaaagcacataaagacaaatcagctcaatgctttaaaatgttttataagggtgttatcacgcatgatgtttcatctgcaattaacaggccacaaataggcgtggtaagagaattccttacacgtaaccctgcttggagaaaagctgtctttatttcaccttataattcacagaatgctgtagcctcaaagattttgggactaccaactcaaactgttgattcatcacagggctcagaatatgactatgtcatattcactcaaaccactgaaacagctcactcttgtaatgtaaacagatttaatgttgctattaccagagcaaaagtaggcatactttgcataatgtctgatagagacctttatgacaagttgcaatttacaagtcttgaaattccacgtaggaatgtggcaactttacaagctgaaaatgtaacaggactctttaaagattgtagtaaggtaatcactgggttacatcctacacaggcacctacacacctcagtgttgacactaaattcaaaactgaaggtttatgtgttgacatacctggcatacctaaggacatgacctatagaagactcatctctatgatgggttttaaaatgaattatcaagttaatggttaccctaacatgtttatcacccgcgaagaagctataagacatgtacgtgcatggattggcttcgatgtcgaggggtgtcatgctactagagaagctgttggtaccaatttacctttacagctaggtttttctacaggtgttaacctagttgctgtacctacaggttatgttgatacacctaataatacagatttttccagagttagtgctaaaccaccgcctggagatcaatttaaacacctcataccacttatgtacaaaggacttccttggaatgtagtgcgtataaagattgtacaaatgttaagtgacacacttaaaaatctctctgacagagtcgtatttgtcttatgggcacatggctttgagttgacatctatgaagtattttgtgaaaataggacctgagcgcacctgttgtctatgtgatagacgtgccacatgcttttccactgcttcagacacttatgcctgttggcatcattctattggatttgattacgtctataatccgtttatgattgatgttcaacaatggggttttacaggtaacctacaaagcaaccatgatctgtattgtcaagtccatggtaatgcacatgtagctagttgtgatgcaatcatgactaggtgtctagctgtccacgagtgctttgttaagcgtgttgactggactattgaatatcctataattggtgatgaactgaagattaatgcggcttgtagaaaggttcaacacatggttgttaaagctgcattattagcagacaaattcccagttcttcacgacattggtaaccctaaagctattaagtgtgtacctcaagctgatgtagaatggaagttctatgatgcacagccttgtagtgacaaagcttataaaatagaagaattattctattcttatgccacacattctgacaaattcacagatggtgtatgcctattttggaattgcaatgtcgatagatatcctgctaattccattgtttgtagatttgacactagagtgctatctaaccttaacttgcctggttgtgatggtggcagtttgtatgtaaataaacatgcattccacacaccagcttttgataaaagtgcttttgttaatttaaaacaattaccatttttctattactctgacagtccatgtgagtctcatggaaaacaagtagtgtcagatatagattatgtaccactaaagtctgctacgtgtataacacgttgcaatttaggtggtgctgtctgtagacatcatgctaatgagtacagattgtatctcgatgcttataacatgatgatctcagctggctttagcttgtgggtttacaaacaatttgatacttataacctctggaacacttttacaagacttcagagtttagaaaatgtggcttttaatgttgtaaataagggacactttgatggacaacagggtgaagtaccagtttctatcattaataacactgtttacacaaaagttgatggtgttgatgtagaattgtttgaaaataaaacaacattacctgttaatgtagcatttgagctttgggctaagcgcaacattaaaccagtaccagaggtgaaaatactcaataatttgggtgtggacattgctgctaatactgtgatctgggactacaaaagagatgctccagcacatatatctactattggtgtttgttctatgactgacatagccaagaaaccaactgaaacgatttgtgcaccactcactgtcttttttgatggtagagttgatggtcaagtagacttatttagaaatgcccgtaatggtgttcttattacagaaggtagtgttaaaggtttacaaccatctgtgggtcccaaacaagctagtcttaatggagtcacattaattggagaagccgtaaaaacacagttcaattattataagaaagttgatggtgttgtccaacaattacctgaaacttactttactcagagtagaaatttacaagaatttaaacccaggagtcaaatggaaattgatttcttagaattagctatggatgaattcattgaacggtataaattagaaggctatgccttcgaacatatcgtttatggagattttagtcatagtcagttaggtggtttacatctactgattggactagctaaacgttttaaggaatcaccttttgaattagaagattttattcctatggacagtacagttaaaaactatttcataacagatgcgcaaacaggttcatctaagtgtgtgtgttctgttattgatttattacttgatgattttgttgaaataataaaatcccaagatttatctgtagtttctaaggttgtcaaagtgactattgactatacagaaatttcatttatgctttggtgtaaagatggccatgtagaaacattttacccaaaattacaatctagtcaagcgtggcaaccgggtgttgctatgcctaatctttacaaaatgcaaagaatgctattagaaaagtgtgaccttcaaaattatggtgatagtgcaacattacctaaaggcataatgatgaatgtcgcaaaatatactcaactgtgtcaatatttaaacacattaacattagctgtaccctataatatgagagttatacattttggtgctggttctgataaaggagttgcaccaggtacagctgttttaagacagtggttgcctacgggtacgctgcttgtcgattcagatcttaatgactttgtctctgatgcagattcaactttgattggtgattgtgcaactgtacatacagctaataaatgggatctcattattagtgatatgtacgaccctaagactaaaaatgttacaaaagaaaatgactctaaagagggttttttcacttacatttgtgggtttatacaacaaaagctagctcttggaggttccgtggctataaagataacagaacattcttggaatgctgatctttataagctcatgggacacttcgcatggtggacagcctttgttactaatgtgaatgcgtcatcatctgaagcatttttaattggatgtaattatcttggcaaaccacgcgaacaaatagatggttatgtcatgcatgcaaattacatattttggaggaatacaaatccaattcagttgtcttcctattctttatttgacatgagtaaatttccccttaaattaaggggtactgctgttatgtctttaaaagaaggtcaaatcaatgatatgattttatctcttcttagtaaaggtagacttataattagagaaaacaacagagttgttatttctagtgatgttcttgttaacaactaaacgaacaatgtttgtttttcttgttttattgccactagtctctagtcagtgtgttaatcttacaaccagaactcaattaccccctgcatacactaattctttcacacgtggtgtttattaccctgacaaagttttcagatcctcagttttacattcaactcaggacttgttcttacctttcttttccaatgttacttggttccatgctatacatgtctctgggaccaatggtactaagaggtttgataaccctgtcctaccatttaatgatggtgtttattttgcttccactgagaagtctaacataataagaggctggatttttggtactactttagattcgaagacccagtccctacttattgttaataacgctactaatgttgttattaaagtctgtgaatttcaattttgtaatgatccatttttgggtgtttattaccacaaaaacaacaaaagttggatggaaagtgagttcagagtttattctagtgcgaataattgcacttttgaatatgtctctcagccttttcttatggaccttgaaggaaaacagggtaatttcaaaaatcttagggaatttgtgtttaagaatattgatggttattttaaaatatattctaagcacacgcctattaatttagtgcgtgatctccctcagggtttttcggctttagaaccattggtagatttgccaataggtattaacatcactaggtttcaaactttacttgctttacatagaagttatttgactcctggtgattcttcttcaggttggacagctggtgctgcagcttattatgtgggttatcttcaacctaggacttttctattaaaatataatgaaaatggaaccattacagatgctgtagactgtgcacttgaccctctctcagaaacaaagtgtacgttgaaatccttcactgtagaaaaaggaatctatcaaacttctaactttagagtccaaccaacagaatctattgttagatttcctaatattacaaacttgtgcccttttggtgaagtttttaacgccaccagatttgcatctgtttatgcttggaacaggaagagaatcagcaactgtgttgctgattattctgtcctatataattccgcatcattttccacttttaagtgttatggagtgtctcctactaaattaaatgatctctgctttactaatgtctatgcagattcatttgtaattagaggtgatgaagtcagacaaatcgctccagggcaaactggaaagattgctgattataattataaattaccagatgattttacaggctgcgttatagcttggaattctaacaatcttgattctaaggttggtggtaattataattacctgtatagattgtttaggaagtctaatctcaaaccttttgagagagatatttcaactgaaatctatcaggccggtagcacaccttgtaatggtgttgaaggttttaattgttactttcctttacaatcatatggtttccaacccactaatggtgttggttaccaaccatacagagtagtagtactttcttttgaacttctacatgcaccagcaactgtttgtggacctaaaaagtctactaatttggttaaaaacaaatgtgtcaatttcaacttcaatggtttaacaggcacaggtgttcttactgagtctaacaaaaagtttctgcctttccaacaatttggcagagacattgctgacactactgatgctgtccgtgatccacagacacttgagattcttgacattacaccatgttcttttggtggtgtcagtgttataacaccaggaacaaatacttctaaccaggttgctgttctttatcaggatgttaactgcacagaagtccctgttgctattcatgcagatcaacttactcctacttggcgtgtttattctacaggttctaatgtttttcaaacacgtgcaggctgtttaataggggctgaacatgtcaacaactcatatgagtgtgacatacccattggtgcaggtatatgcgctagttatcagactcagactaattctcctcggcgggcacgtagtgtagctagtcaatccatcattgcctacactatgtcacttggtgcagaaaattcagttgcttactctaataactctattgccatacccacaaattttactattagtgttaccacagaaattctaccagtgtctatgaccaagacatcagtagattgtacaatgtacatttgtggtgattcaactgaatgcagcaatcttttgttgcaatatggcagtttttgtacacaattaaaccgtgctttaactggaatagctgttgaacaagacaaaaacacccaagaagtttttgcacaagtcaaacaaatttacaaaacaccaccaattaaagattttggtggttttaatttttcacaaatattaccagatccatcaaaaccaagcaagaggtcatttattgaagatctacttttcaacaaagtgacacttgcagatgctggcttcatcaaacaatatggtgattgccttggtgatattgctgctagagacctcatttgtgcacaaaagtttaacggccttactgttttgccacctttgctcacagatgaaatgattgctcaatacacttctgcactgttagcgggtacaatcacttctggttggacctttggtgcaggtgctgcattacaaataccatttgctatgcaaatggcttataggtttaatggtattggagttacacagaatgttctctatgagaaccaaaaattgattgccaaccaatttaatagtgctattggcaaaattcaagactcactttcttccacagcaagtgcacttggaaaacttcaagatgtggtcaaccaaaatgcacaagctttaaacacgcttgttaaacaacttagctccaattttggtgcaatttcaagtgttttaaatgatatcctttcacgtcttgacaaagttgaggctgaagtgcaaattgataggttgatcacaggcagacttcaaagtttgcagacatatgtgactcaacaattaattagagctgcagaaatcagagcttctgctaatcttgctgctactaaaatgtcagagtgtgtacttggacaatcaaaaagagttgatttttgtggaaagggctatcatcttatgtccttccctcagtcagcacctcatggtgtagtcttcttgcatgtgacttatgtccctgcacaagaaaagaacttcacaactgctcctgccatttgtcatgatggaaaagcacactttcctcgtgaaggtgtctttgtttcaaatggcacacactggtttgtaacacaaaggaatttttatgaaccacaaatcattactacagacaacacatttgtgtctggtaactgtgatgttgtaataggaattgtcaacaacacagtttatgatcctttgcaacctgaattagactcattcaaggaggagttagataaatattttaagaatcatacatcaccagatgttgatttaggtgacatctctggcattaatgcttcagttgtaaacattcaaaaagaaattgaccgcctcaatgaggttgccaagaatttaaatgaatctctcatcgatctccaagaacttggaaagtatgagcagtatataaaatggccatggtacatttggctaggttttatagctggcttgattgccatagtaatggtgacaattatgctttgctgtatgaccagttgctgtagttgtctcaagggctgttgttcttgtggatcctgctgcaaatttgatgaagacgactctgagccagtgctcaaaggagtcaaattacattacacataattcctgatcttctggtctaaacgaactaaatattatattagtttttctgtttggaactttaattttagccatggcagattccaacggtactattaccgttgaagagcttaaaaagctccttgaacaatggaacctagtaataggtttcctattccttacatggatttgtcttctacaatttgcctatgccaacaggaataggtttttgtatataattaagttaattttcctctggctgttatggccagtaactttagcttgttttgtgcttgctgctgtttacagaataaattggatcaccggtggaattgctatcgcaatggcttgtcttgtaggcttgatgtggctcagctacttcattgcttctttcagactgtttgcgcgtacccgttccatgtggtcattcaatccagaaactaacattcttctcaacgtgccactccatggcactattctgaccagaccgcttctagaaagtgaactcgtaatcggagctgtgatccttcgtggacatcttcgtattgctggacaccatctaggacgctgtgacatcaaggacctgcctaaagaaatcactgttgctacatcccgcacgctttcttattacaaattgggagcttcgcagcgtgtagcaggtgactcaggttttgctgcatacagtcgctacaggattggcaactataaattaaacacagaccattccagtagcagtgacaatattgctttgcttgtacagtaagtgacaacagaaccaatggagattgattaaacgaacatgaaaattattcttttcttggcactgataacactcgctacttgtgagctttatcactaccaagagtgtgttagaggtacaacagtacttttaaaagaaccttgctcttctggaacatacgagggcaattcaccatttcatcctctagctgataacaaatttgcactgacttgctttagcactcaatttgcttttgcttgtcctgacggcgtaaaacacgtctatcagttacgtgccagatcagtttcacctaaactgttcatcagacaagaggaagttcaagaactttactctccaatttttcttattgttgcggcaatagtgtttataacactttgcttcacactcaaaagaaagacagaatgattgaactttcattaattgacttctatttgtgctttttagcctttctgctattccttgttttaattatgcttattatcttttggttctcacttgaactgcaagatcataatgaaacttgtcacgcctaatgttttagatttcatctaaacgaacaaactaaaatgtctgataatggaccccaaaatcagcgaaatgcaccccgcattacgtttggtggaccctcagattcaactggcagtaaccagaatggagaacgcagtggggcgcgatcaaaacaacgtcggccccaaggtttacccaataatactgcgtcttggttcaccgctctcactcaacatggcaaggaagaccttaaattccctcgaggacaaggcgttccaattaacaccaatagcagtccagatgaccaaattggctactaccgaagagctaccagacgaattcgtggtggtgacggtaaaatgaaagatctcagtccaagatggtatttctactacctaggaactgggccagaagctggacttccctatggtgctaacaaagacggcatcatatgggttgcaactgagggagccttgaatacaccaaaagatcacattggcacccgcaatcctgctaacaatgctgcaatcgtgctacaacttcctcaaggaacaacattgccaaaaggcttctacgcagaagggagcagaggcggcagtcaagcctcttctcgttcctcatcacgtagtcgcaacagttcaagaaattcaactccaggcagcagtaggggaacttctcctgctagaatggctggcaatggcggtgatgctgctcttgctttgctgctgcttgacagattgaaccagcttgagagcaaaatgtctggtaaaggccaacaacaacaaggccaaactgtcactaagaaatctgctgctgaggcttctaagaagcctcggcaaaaacgtactgccactaaagcatacaatgtaacacaagctttcggcagacgtggtccagaacaaacccaaggaaattttggggaccaggaactaatcagacaaggaactgattacaaacattggccgcaaattgcacaatttgcccccagcgcttcagcgttcttcggaatgtcgcgcattggcatggaagtcacaccttcgggaacgtggttgacctacacaggtgccatcaaattggatgacaaagatccaaatttcaaagatcaagtcattttgctgaataagcatattgacgcatacaaaacattcccaccaacagagcctaaaaaggacaaaaagaagaaggctgatgaaactcaagccttaccgcagagacagaagaaacagcaaactgtgactcttcttcctgctgcagatttggatgatttctccaaacaattgcaacaatccatgagcagtgctgactcaactcaggcctaaactcatgcagaccacacaaggcagatgggctatataaacgttttcgcttttccgtttacgatatatagtctactcttgtgcagaatgaattctcgtaactacatagcacaagtagatgtagttaactttaatctcacatagcaatctttaatcagtgtgtaacattagggaggacttgaaagagccaccacattttcaccgaggccacgcggagtacgatcgagtgtacagtgaacaatgctagggagagctgcctatatggaagagccctaatgtgtaaaattaattttagtagtgctatccccatgtgattttaatagcttcttaggagaatgacaaaaaaaaaaaaaaaaaaaaaaaaa

SEQ ID NO: 45 - DNA, 940 bp, Coronaviridae
  source 1..940: mol_type = other DNA
  misc_feature 1..940: note = Fnsp1_A polynucleotide sequence
ggcgcgcctaagttgacattgattattgactagttattaatagtaatcaattacggggtcattagttcatagcccatatatggagttccgcgttacataacttacggtaaatggcccgcctggctgaccgcccaacgacccccgcccattgacgtcaataatgacgtatgttcccatagtaacgccaatagggactttccattgacgtcaatgggtggagtatttacggtaaactgcccacttggcagtacatcaagtgtatcatatgccaagtacgccccctattgacgtcaatgacggtaaatggcccgcctggcattatgcccagtacatgaccttatgggactttcctacttggcagtacatctacgtattagtcatcgctattaccatggtgatgcggttttggcagtacatcaatgggcgtggatagcggtttgactcacggggatttccaagtctccaccccattgacgtcaatgggagtttgttttggcaccaaaatcaacgggactttccaaaatgtcgtaacaactccgccccattgacgcaaatgggcggtaggcgtgtacggtgggaggtctatataagcagagctcgtttagtgaaccgtattaaaggtttataccttcccaggtaacaaaccaaccaactttcgatctcttgtagatctgttctctaaacgaactttaaaatctgtgtggctgtcactcggctgcatgcttagtgcactcacgcagtataattaataactaattactgtcgttgacaggacacgagtaactcgtctatcttctgcaggctgcttacggtttcgtccgtgttgcagccgatcatcagcacatctaggtttcgtccgggtgtgaccgaaaggtaagatggagagccttgtccctcaactcagtttgcctgttttacaggttcgcgacgtgctcgtacg

SEQ ID NO: 46 - DNA, 6340 bp, Coronaviridae
  source 1..6340: mol_type = other DNA
  misc_feature 1..6340: note = Fnsp1_[B,D] polynucleotide sequence
cgtacgtggctttggagactccgtggaggaggtcttatcagaggcacgtcaacatcttaaagatggcacttgtggcttagtagaagttgaaaaaggcgttttgcctcaacttgaacagccctatgtgttcatcaaacgttcggatgctcgaactgcagaactcgaaggcattcagtacggtcgtagtggtgagacacttggtgtccttgtccctcatgtgggcgaaataccagtggcttaccgcaaggttcttcttcgtaagaacggtaataaaggagctggtggccatagttacggcgccgatctaaagtcatttgacttaggcgacgagcttggcactgatccttatagcagtggtgttacccgtgaactcatgcgtgagcttaacggaggggcatacactcgctatgtcgataacaacttctgtggccctgatggctaccctcttgagtgcattaaagaccttctagcacgtgctggtaaagcttcatgcactttgtccgaacaactggactttattgacactaagaggggtgtatactgctgccgtgaacatgagcatgaaattgcttggtacacggaacgttctgaaaagagctatgaattgcagacaccttttgaaattaaattggcaaagaaatttgacaccttcaatggggaatgtccaaattttgtatttcccttaaattccataatcaagactattcaaccaagggttgaaaagaaaaagcttgatggctttatgggtagaattcgatctgtctatccagttgcgtcaccaaatgaatgcaaccaaatgtgcctttcaactctcatgaagtgtgatcattgtggtgaaacttcatggcagacgggcgattttgttaaagccacttgcgaattttgtggcactgagaatttgactaaagaaggtgccactacttgtggttacttaccccaaaatgctgttgttaaaatttattgtccagcatgtcacaattcagaagtaggacctgagcatagtcttgccgaataccataatgaatctggcttgaaaaccattcttcgtaagggtggtcgcactattgcctttggaggctgtgtgttctcttatgttggttgccataacaagtgtgcctattgggttccacgtgctagcgctaacataggttgtaaccatacaggtgttgttggagaaggttccgaaggtcttaatgacaaccttcttgaaatactccaaaaagagaaagtcaacatcaatattgttggtgactttaaacttaatgaagagatcgccattattttggcatctttttctgcttccacaagtgcttttgtggaaactgtgaaaggtttggattataaagcattcaaacaaattgttgaatcctgtggtaattttaaagttacaaaaggaaaagctaaaaaaggtgcctggaatattggtgaacagaaatcaatactgagtcctctttatgcatttgcatcagaggctgctcgtgttgtacgatcaattttctcccgcactcttgaaactgctcaaaattctgtgcgtgttttacagaaggccgctataacaatactagatggaatttcacagtattcactgagactcattgatgctatgatgttcacatctgatttggctactaacaatctagttgtaatggcctacattacaggtggtgttgttcagttgacttcgcagtggctaactaacatctttggcactgtttatgaaaaactcaaacccgtccttgattggcttgaagagaagtttaaggaaggtgtagagtttcttagagacggttgggaaattgttaaatttatctcaacctgtgcttgtgaaattgtcggtggacaaattgtcacctgtgcaaaggaaattaaggagagtgttcagacattctttaagcttgtaaataaatttttggctttgtgtgctgactctatcattattggtggagctaaacttaaagccttgaatttaggtgaaacatttgtcacgcactcaaagggattgtacagaaagtgtgttaaatccagagaagaaactggcctactcatgcctctaaaagccccaaaagaaattatcttcttagagggagaaacacttcccacagaagtgttaacagaggaagttgtcttgaaaactggtgatttacaaccattagaacaacctactagtgaagctgttgaagctccattggttggtacaccagtttgtattaacgggcttatgttgctcgaaatcaaagacacagaaaagtactgtgcccttgcacctaatatgatggtaacaaacaataccttcacactcaaaggcggtgcaccaacaaaggttacttttggtgatgacactgtgatagaagtgcaaggttacaagagtgtgaatatcacttttgaacttgatgaaaggattgataaagtacttaatgagaagtgctctgcctatacagttgaactcggtacagaagtaaatgagttcgcctgtgttgtggcagatgctgtcataaaaactttgcaaccagtatctgaattacttacaccactgggcattgatttagatgagtggagtatggctacatactacttatttgatgagtctggtgagtttaaattggcttcacatatgtattgttctttctaccctccagatgaggatgaagaagaaggtgattgtgaagaagaagagtttgagccatcaactcaatatgagtatggtactgaagatgattaccaaggtaaacctttggaatttggtgccacttctgctgctcttcaacctgaagaagagcaagaagaagattggttagatgatgatagtcaacaaactgttggtcaacaagacggcagtgaggacaatcagacaactactattcaaacaattgttgaggttcaacctcaattagagatggaacttacaccagttgttcagactattgaagtgaatagttttagtggttatttaaaacttactgacaatgtatacattaaaaatgcagacattgtggaagaagctaaaaaggtaaaaccaacagtggttgttaatgcagccaatgtttaccttaaacatggaggaggtgttgcaggagccttaaataaggctactaacaatgccatgcaagttgaatctgatgattacatagctactaatggaccacttaaagtgggtggtagttgtgttttaagcggacacaatcttgctaaacactgtcttcatgttgtcggcccaaatgttaacaaaggtgaagacattcaacttcttaagagtgcttatgaaaattttaatcagcacgaagttctacttgcaccattattatcagctggtatttttggtgctgaccctatacattctttaagagtttgtgtagatactgttcgcacaaatgtctacttagctgtctttgataaaaatctctatgacaaacttgtttcaagctttttggaaatgaagagtgaaaagcaagttgaacaaaagatcgctgagattcctaaagaggaagttaagccatttataactgaaagtaaaccttcagttgaacagagaaaacaagatgataagaaaatcaaagcttgtgttgaagaagttacaacaactctggaagaaactaagttcctcacagaaaacttgttactttatattgacattaatggcaatcttcatccagattctgccactcttgttagtgacattgacatcactttcttaaagaaagatgctccatatatagtgggtgatgttgttcaagagggtgttttaactgctgtggttatacctactaaaaaggctggtggcactactgaaatgctagcgaaagctttgagaaaagtgccaacagacaattatataaccacttacccgggtcagggtttaaatggttacactgtagaggaggcaaagacagtgcttaaaaagtgtaaaagtgccttttacattctaccatctattatctctaatgagaagcaagaaattcttggaactgtttcttggaatttgcgagaaatgcttgcacatgcagaagaaacacgcaaattaatgcctgtctgtgtggaaactaaagccatagtttcaactatacagcgtaaatataagggtattaaaatacaagagggtgtggttgattatggtgctagattttacttttacaccagtaaaacaactgtagcgtcacttatcaacacacttaacgatctaaatgaaactcttgttacaatgccacttggctatgtaacacatggcttaaatttggaagaagctgctcggtatatgagatctctcaaagtgccagctacagtttctgtttcttcacctgatgctgttacagcgtataatggttatcttacttcttcttctaaaacacctgaagaacattttattgaaaccatctcacttgctggttcctataaagattggtcctattctggacaatctacacaactaggtatagaatttcttaagagaggtgataaaagtgtatattacactagtaatcctaccacattccacctagatggtgaagttatcacctttgacaatcttaagacacttctttctttgagagaagtgaggactattaaggtgtttacaacagtagacaacattaacctccacacgcaagttgtggacatgtcaatgacatatggacaacagtttggtccaacttatttggatggagctgatgttactaaaataaaacctcataattcacatgaaggtaaaacattttatgttttacctaatgatgacactctacgtgttgaggcttttgagtactaccacacaactgatcctagttttctgggtaggtacatgtcagcattaaatcacactaaaaagtggaaatacccacaagttaatggtttaacttctattaaatgggcagataacaactgttatcttgccactgcattgttaacactccaacaaatagagttgaagtttaatccacctgctctacaagatgcttattacagagcaagggctggtgaagctgctaacttttgtgcacttatcttagcctactgtaataagacagtaggtgagttaggtgatgttagagaaacaatgagttacttgtttcaacatgccaatttagattcttgcaaaagagtcttgaacgtggtgtgtaaaacttgtggacaacagcagacaacccttaagggtgtagaagctgttatgtacatgggcacactttcttatgaacaatttaagaaaggtgttcagataccttgtacgtgtggtaaacaagctacaaaatatctagtacaacaggagtcaccttttgttatgatgtcagcaccacctgctcagtatgaacttaagcatggtacatttacttgtgctagtgagtacactggtaattaccagtgtggtcactataaacatataacttctaaagaaactttgtattgcatagacggtgctttacttacaaagtcctcagaatacaaaggtcctattacggatgttttctacaaagaaaacagttacacaacaaccataaaaccagttacttataaattggatggtgttgtttgtacagaaattgaccctaagttggacaattattataagaaagacaattcttatttcacagagcaaccaattgatcttgtaccaaaccaaccatatccaaacgcaagcttcgataattttaagtttgtatgtgataatatcaaatttgctgatgatttaaaccagttaactggttataagaaacctgcttcaagagagcttaaagttacatttttccctgacttaaatggtgatgtggtggctattgattataaacactacacaccctcttttaagaaaggagctaaattgttacataaacctattgtttggcatgttaacaatgcaactaataaagccacgtataaaccaaatacctggtgtatacgttgtctttggagcacaaaaccagttgaaacatcaaattcgtttgatgtactgaagtcagaggacgcgcagggaatggataatcttgcctgcgaagatctaaaaccagtctctgaagaagtagtggaaaatcctaccatacagaaagacgttcttgagtgtaatgtgaaaactaccgaagttgtaggagacattatacttaaaccagcaaataatagtttaaaaattacagaagaggttggccacacagatctaatggctgcttatgtagacaattctagtcttactattaagaaacctaatgaattatctagagtattaggtttgaaaacccttgctactcatggtttagctgctgttaatagtgtcccttgggatactatagctaattatgctaagccttttcttaacaaagttgttagtacaactactaacatagttacacggtgtttaaac

SEQ ID NO: 47 - DNA, 28636 bp, Coronaviridae
  source 1..28636: mol_type = other DNA
  misc_feature 1..28636: note = SARS-CoV-2-[3,E,6] polynucleotide sequence, containing two point substitutions (c.27041A>C and c.27044A>C) in comparison to SEQ ID NO: 1
attaaaggtttataccttcccaggtaacaaaccaaccaactttcgatctcttgtagatctgttctctaaacgaactttaaaatctgtgtggctgtcactcggctgcatgcttagtgcactcacgcagtataattaataactaattactgtcgttgacaggacacgagtaactcgtctatcttctgcaggctgcttacggtttcgtccgtgttgcagccgatcatcagcacatctaggtttcgtccgggtgtgaccgaaaggtaagatggagagccttgtccctggtttcaacgagaaaacacacgtccaactcagtttgcctgttttacaggttcgcgacgtgctcgtacgtggctttggagactccgtggaggaggtcttatcagaggcacgtcaacatcttaaagatggcacttgtggcttagtagaagttgaaaaaggcgttttgcctcaacttgaacagccctatgtgttcatcaaacgttcggatgctcgaactgcacctcatggtcatgttatggttgagctggtagcagaactcgaaggcattcagtacggtcgtagtggtgagacacttggtgtccttgtccctcatgtgggcgaaataccagtggcttaccgcaaggttcttcttcgtaagaacggtaataaaggagctggtggccatagttacggcgccgatctaaagtcatttgacttaggcgacgagcttggcactgatccttatgaagattttcaagaaaactggaacactaaacatagcagtggtgttacccgtgaactcatgcgtgagcttaacggaggggcatacactcgctatgtcgataacaacttctgtggccctgatggctaccctcttgagtgcattaaagaccttctagcacgtgctggtaaagcttcatgcactttgtccgaacaactggactttattgacactaagaggggtgtatactgctgccgtgaacatgagcatgaaattgcttggtacacggaacgttctgaaaagagctatgaattgcagacaccttttgaaattaaattggcaaagaaatttgacaccttcaatggggaatgtccaaattttgtatttcccttaaattccataatcaagactattcaaccaagggttgaaaagaaaaagcttgatggctttatgggtagaattcgatctgtctatccagttgcgtcaccaaatgaatgcaaccaaatgtgcctttcaactctcatgaagtgtgatcattgtggtgaaacttcatggcagacgggcgattttgttaaagccacttgcgaattttgtggcactgagaatttgactaaagaaggtgccactacttgtggttacttaccccaaaatgctgttgttaaaatttattgtccagcatgtcacaattcagaagtaggacctgagcatagtcttgccgaataccataatgaatctggcttgaaaaccattcttcgtaagggtggtcgcactattgcctttggaggctgtgtgttctcttatgttggttgccataacaagtgtgcctattgggttccacgtgctagcgctaacataggttgtaaccatacaggtgttgttggagaaggttccgaaggtcttaatgacaaccttcttgaaatactccaaaaagagaaagtcaacatcaatattgttggtgactttaaacttaatgaagagatcgccattattttggcatctttttctgcttccacaagtgcttttgtggaaactgtgaaaggtttggattataaagcattcaaacaaattgttgaatcctgtggtaattttaaagttacaaaaggaaaagctaaaaaaggtgcctggaatattggtgaacagaaatcaatactgagtcctctttatgcatttgcatcagaggctgctcgtgttgtacgatcaattttctcccgcactcttgaaactgctcaaaattctgtgcgtgttttacagaaggccgctataacaatactagatggaatttcacagtattcactgagactcattgatgctatgatgttcacatctgatttggctactaacaatctagttgtaatggcctacattacaggtggtgttgttcagttgacttcgcagtggctaactaacatctttggcactgtttatgaaaaactcaaacccgtccttgattggcttgaagagaagtttaaggaaggtgtagagtttcttagagacggttgggaaattgttaaatttatctcaacctgtgcttgtgaaattgtcggtggacaaattgtcacctgtgcaaaggaaattaaggagagtgttcagacattctttaagcttgtaaataaatttttggctttgtgtgctgactctatcattattggtggagctaaacttaaagccttgaatttaggtgaaacatttgtcacgcactcaaagggattgtacagaaagtgtgttaaatccagagaagaaactggcctactcatgcctctaaaagccccaaaagaaattatcttcttagagggagaaacacttcccacagaagtgttaacagaggaagttgtcttgaaaactggtgatttacaaccattagaacaacctactagtgaagctgttgaagctccattggttggtacaccagtttgtattaacgggcttatgttgctcgaaatcaaagacacagaaaagtactgtgcccttgcacctaatatgatggtaacaaacaataccttcacactcaaaggcggtgcaccaacaaaggttacttttggtgatgacactgtgatagaagtgcaaggttacaagagtgtgaatatcacttttgaacttgatgaaaggattgataaagtacttaatgagaagtgctctgcctatacagttgaactcggtacagaagtaaatgagttcgcctgtgttgtggcagatgctgtcataaaaactttgcaaccagtatctgaattacttacaccactgggcattgatttagatgagtggagtatggctacatactacttatttgatgagtctggtgagtttaaattggcttcacatatgtattgttctttctaccctccagatgaggatgaagaagaaggtgattgtgaagaagaagagtttgagccatcaactcaatatgagtatggtactgaagatgattaccaaggtaaacctttggaatttggtgccacttctgctgctcttcaacctgaagaagagcaagaagaagattggttagatgatgatagtcaacaaactgttggtcaacaagacggcagtgaggacaatcagacaactactattcaaacaattgttgaggttcaacctcaattagagatggaacttacaccagttgttcagactattgaagtgaatagttttagtggttatttaaaacttactgacaatgtatacattaaaaatgcagacattgtggaagaagctaaaaaggtaaaaccaacagtggttgttaatgcagccaatgtttaccttaaacatggaggaggtgttgcaggagccttaaataaggctactaacaatgccatgcaagttgaatctgatgattacatagctactaatggaccacttaaagtgggtggtagttgtgttttaagcggacacaatcttgctaaacactgtcttcatgttgtcggcccaaatgttaacaaaggtgaagacattcaacttcttaagagtgcttatgaaaattttaatcagcacgaagttctacttgcaccattattatcagctggtatttttggtgctgaccctatacattctttaagagtttgtgtagatactgttcgcacaaatgtctacttagctgtctttgataaaaatctctatgacaaacttgtttcaagctttttggaaatgaagagtgaaaagcaagttgaacaaaagatcgctgagattcctaaagaggaagttaagccatttataactgaaagtaaaccttcagttgaacagagaaaacaagatgataagaaaatcaaagcttgtgttgaagaagttacaacaactctggaagaaactaagttcctcacagaaaacttgttactttatattgacattaatggcaatcttcatccagattctgccactcttgttagtgacattgacatcactttcttaaagaaagatgctccatatatagtgggtgatgttgttcaagagggtgttttaactgctgtggttatacctactaaaaaggctggtggcactactgaaatgctagcgaaagctttgagaaaagtgccaacagacaattatataaccacttacccgggtcagggtttaaatggttacactgtagaggaggcaaagacagtgcttaaaaagtgtaaaagtgccttttacattctaccatctattatctctaatgagaagcaagaaattcttggaactgtttcttggaatttgcgagaaatgcttgcacatgcagaagaaacacgcaaattaatgcctgtctgtgtggaaactaaagccatagtttcaactatacagcgtaaatataagggtattaaaatacaagagggtgtggttgattatggtgctagattttacttttacaccagtaaaacaactgtagcgtcacttatcaacacacttaacgatctaaatgaaactcttgttacaatgccacttggctatgtaacacatggcttaaatttggaagaagctgctcggtatatgagatctctcaaagtgccagctacagtttctgtttcttcacctgatgctgttacagcgtataatggttatcttacttcttcttctaaaacacctgaagaacattttattgaaaccatctcacttgctggttcctataaagattggtcctattctggacaatctacacaactaggtatagaatttcttaagagaggtgataaaagtgtatattacactagtaatcctaccacattccacctagatggtgaagttatcacctttgacaatcttaagacacttctttctttgagagaagtgaggactattaaggtgtttacaacagtagacaacattaacctccacacgcaagttgtggacatgtcaatgacatatggacaacagtttggtccaacttatttggatggagctgatgttactaaaataaaacctcataattcacatgaaggtaaaacattttatgttttacctaatgatgacactctacgtgttgaggcttttgagtactaccacacaactgatcctagttttctgggtaggtacatgtcagcattaaatcacactaaaaagtggaaatacccacaagttaatggtttaacttctattaaatgggcagataacaactgttatcttgccactgcattgttaacactccaacaaatagagttgaagtttaatccacctgctctacaagatgcttattacagagcaagggctggtgaagctgctaacttttgtgcacttatcttagcctactgtaataagacagtaggtgagttaggtgatgttagagaaacaatgagttacttgtttcaacatgccaatttagattcttgcaaaagagtcttgaacgtggtgtgtaaaacttgtggacaacagcagacaacccttaagggtgtagaagctgttatgtacatgggcacactttcttatgaacaatttaagaaaggtgttcagataccttgtacgtgtggtaaacaagctacaaaatatctagtacaacaggagtcaccttttgttatgatgtcagcaccacctgctcagtatgaacttaagcatggtacatttacttgtgctagtgagtacactggtaattaccagtgtggtcactataaacatataacttctaaagaaactttgtattgcatagacggtgctttacttacaaagtcctcagaatacaaaggtcctattacggatgttttctacaaagaaaacagttacacaacaaccataaaaccagttacttataaattggatggtgttgtttgtacagaaattgaccctaagttggacaattattataagaaagacaattcttatttcacagagcaaccaattgatcttgtaccaaaccaaccatatccaaacgcaagcttcgataattttaagtttgtatgtgataatatcaaatttgctgatgatttaaaccagttaactggttataagaaacctgcttcaagagagcttaaagttacatttttccctgacttaaatggtgatgtggtggctattgattataaacactacacaccctcttttaagaaaggagctaaattgttacataaacctattgtttggcatgttaacaatgcaactaataaagccacgtataaaccaaatacctggtgtatacgttgtctttggagcacaaaaccagttgaaacatcaaattcgtttgatgtactgaagtcagaggacgcgcagggaatggataatcttgcctgcgaagatctaaaaccagtctctgaagaagtagtggaaaatcctaccatacagaaagacgttcttgagtgtaatgtgaaaactaccgaagttgtaggagacattatacttaaaccagcaaataatagtttaaaaattacagaagaggttggccacacagatctaatggctgcttatgtagacaattctagtcttactattaagaaacctaatgaattatctagagtattaggtttgaaaacccttgctactcatggtttagctgctgttaatagtgtcccttgggatactatagctaattatgctaagccttttcttaacaaagttgttagtacaactactaacatagttacacggtgtttaaaccgtgtttgtactaattatatgccttatttctttactttattgctacaattgtgtacttttactagaagtacaaattctagaattaaagcatctatgccgactactatagcaaagaatactgttaagagtgtcggtaaattttgtctagaggcttcatttaattatttgaagtcacctaatttttctaaactgataaatattataatttggtttttactattaagtgtttgcctaggttctttaatctactcaaccgctgctttaggtgttttaatgtctaatttaggcatgccttcttactgtactggttacagagaaggctatttgaactctactaatgtcactattgcaacctactgtactggttctataccttgtagtgtttgtcttagtggtttagattctttagacacctatccttctttagaaactatacaaattaccatttcatcttttaaatgggatttaactgcttttggcttagttgcagagtggtttttggcatatattcttttcactaggtttttctatgtacttggattggctgcaatcatgcaattgtttttcagctattttgcagtacattttattagtaattcttggcttatgtggttaataattaatcttgtacaaatggccccgatttcagctatggttagaatgtacatcttctttgcatcattttattatgtatggaaaagttatgtgcatgttgtagacggttgtaattcatcaacttgtatgatgtgttacaaacgtaatagagcaacaagagtcgaatgtacaactattgttaatggtgttagaaggtccttttatgtctatgctaatggaggtaaaggcttttgcaaactacacaattggaattgtgttaattgtgatacattctgtgctggtagtacatttattagtgatgaagttgcgagagacttgtcactacagtttaaaagaccaataaatcctactgaccagtcttcttacatcgttgatagtgttacagtgaagaatggttccatccatctttactttgataaagctggtcaaaagacttatgaaagacattctctctctcattttgttaacttagacaacctgagagctaataacactaaaggttcattgcctattaatgttatagtttttgatggtaaatcaaaatgtgaagaatcatctgcaaaatcagcgtctgtttactacagtcagcttatgtgtcaacctatactgttactagatcaggcattagtgtctgatgttggtgatagtgcggaagttgcagttaaaatgtttgatgcttacgttaatacgttttcatcaacttttaacgtaccaatggaaaaactcaaaacactagttgcaactgcagaagctgaacttgcaaagaatgtgtccttagacaatgtcttatctacttttatttcagcagctcggcaagggtttgttgattcagatgtagaaactaaagatgttgttgaatgtcttaaattgtcacatcaatctgacatagaagttactggcgatagttgtaataactatatgctcacctataacaaagttgaaaacatgacaccccgtgaccttggtgcttgtattgactgtagtgcgcgtcatattaatgcgcaggtagcaaaaagtcacaacattgctttgatatggaacgttaaagatttcatgtcattgtctgaacaactacgaaaacaaatacgtagtgctgctaaaaagaataacttaccttttaagttgacatgtgcaactactagacaagttgttaatgttgtaacaacaaagatagcacttaagggtggtaaaattgttaataattggttgaagcagttaattaaagttacacttgtgttcctttttgttgctgctattttctatttaataacacctgttcatgtcatgtctaaacatactgacttttcaagtgaaatcataggatacaaggctattgatggtggtgtcactcgtgacatagcatctacagatacttgttttgctaacaaacatgctgattttgacacatggtttagccagcgtggtggtagttatactaatgacaaagcttgcccattgattgctgcagtcataacaagagaagtgggttttgtcgtgcctggtttgcctggcacgatattacgcacaactaatggtgactttttgcatttcttacctagagtttttagtgcagttggtaacatctgttacacaccatcaaaacttatagagtacactgactttgcaacatcagcttgtgttttggctgctgaatgtacaatttttaaagatgcttctggtaagccagtaccatattgttatgataccaatgtactagaaggttctgttgcttatgaaagtttacgccctgacacacgttatgtgctcatggatggctctattattcaatttcctaacacctaccttgaaggttctgttagagtggtaacaacttttgattctgagtactgtaggcacggcacttgtgaaagatcagaagctggtgtttgtgtatctactagtggtagatgggtacttaacaatgattattacagatctttaccaggagttttctgtggtgtagatgctgtaaatttacttactaatatgtttacaccactaattcaacctattggtgctttggacatatcagcatctatagtagctggtggtattgtagctatcgtagtaacatgccttgcctactattttatgaggtttagaagagcttttggtgaatacagtcatgtagttgcctttaatactttactattccttatgtcattcactgtactctgtttaacaccagtttactcattcttacctggtgtttattctgttatttacttgtacttgacattttatcttactaatgatgtttcttttttagcacatattcagtggatggttatgttcacacctttagtacctttctggataacaattgcttatatcatttgtatttccacaaagcatttctattggttctttagtaattacctaaagagacgtgtagtctttaatggtgtttcctttagtacttttgaagaagctgcgctgtgcacctttttgttaaataaagaaatgtatctaaagttgcgtagtgatgtgctattacctcttacgcaatataatagatacttagctctttataataagtacaagtattttagtggagcaatggatacaactagctacagagaagctgcttgttgtcatctcgcaaaggctctcaatgacttcagtaactcaggttctgatgttctttaccaaccaccacaaacctctatcacctcagctgttttgcagagtggttttagaaaaatggcattcccatctggtaaagttgagggttgtatggtacaagtaacttgtggtacaactacacttaacggtctttggcttgatgacgtagtttactgtccaagacatgtgatctgcacctctgaagacatgcttaaccctaattatgaagatttactcattcgtaagtctaatcataatttcttggtacaggctggtaatgttcaactcagggttattggacattctatgcaaaattgtgtacttaagcttaaggttgatacagccaatcctaagacacctaagtataagtttgttcgcattcaaccaggacagactttttcagtgttagcttgttacaatggttcaccatctggtgtttaccaatgtgctatgaggcccaatttcactattaagggttcattccttaatggttcatgtggtagtgttggttttaacatagattatgactgtgtctctttttgttacatgcaccatatggaattaccaactggagttcatgctggcacagacttagaaggtaacttttatggaccttttgttgacaggcaaacagcacaagcagctggtacggacacaactattacagttaatgttttagcttggttgtacgctgctgttataaatggagacaggtggtttctcaatcgatttaccacaactcttaatgactttaaccttgtggctatgaagtacaattatgaacctctaacacaagaccatgttgacatactaggacctctttctgctcaaactggaattgccgttttagatatgtgtgcttcattaaaagaattactgcaaaatggtatgaatggacgtaccatattgggtagtgctttattagaagatgaatttacaccttttgatgttgttagacaatgctcaggtgttactttccaaagtgcagtgaaaagaacaatcaagggtacacaccactggttgttactcacaattttgacttcacttttagttttagtccagagtactcaatggtctttgttcttttttttgtatgaaaatgcctttttaccttttgctatgggtattattgctatgtctgcttttgcaatgatgtttgtcaaacataagcatgcatttctctgtttgtttttgttaccttctcttgccactgtagcttattttaatatggtctatatgcctgctagttgggtgatgcgtattatgacatggttggatatggttgatactagtttgtctggttttaagctaaaagactgtgttatgtatgcatcagctgtagtgttactaatccttatgacagcaagaactgtgtatgatgatggtgctaggagagtgtggacacttatgaatgtcttgacactcgtttataaagtttattatggtaatgctttagatcaagccatttccatgtgggctcttataatctctgttacttctaactactcaggtgtagttacaactgtcatgtttttggccagaggtattgtttttatgtgtgttgagtattgccctattttcttcataactggtaatacacttcagtgtataatgctagtttattgtttcttaggctatttttgtacttgttactttggcctcttttgtttactcaaccgctactttagactgactcttggtgtttatgattacttagtttctacacaggagtttagatatatgaattcacagggactactcccacccaagaatagcatagatgccttcaaactcaacattaaattgttgggtgttggtggcaaaccttgtatcaaagtagccactgtacagtctaaaatgtcagatgtaaagtgcacatcagtagtcttactctcagttttgcaacaactcagagtagaatcatcatctaaattgtgggctcaatgtgtccagttacacaatgacattctcttagctaaagatactactgaagcctttgaaaaaatggtttcactactttctgttttgctttccatgcagggtgctgtagacataaacaagctttgtgaagaaatgctggacaacagggcaaccttacaagctatagcctcagagtttagttcccttccatcatatgcagcttttgctactgctcaagaagcttatgagcaggctgttgctaatggtgattctgaagttgttcttaaaaagttgaagaagtctttgaatgtggctaaatctgaatttgaccgtgatgcagccatgcaacgtaagttggaaaagatggctgatcaagctatgacccaaatgtataaacaggctagatctgaggacaagagggcaaaagttactagtgctatgcagacaatgcttttcactatgcttagaaagttggataatgatgcactcaacaacattatcaacaatgcaagagatggttgtgttcccttgaacataatacctcttacaacagcagccaaactaatggttgtcataccagactataacacatataaaaatacgtgtgatggtacaacatttacttatgcatcagcattgtgggaaatccaacaggttgtagatgcagatagtaaaattgttcaacttagtgaaattagtatggacaattcacctaatttagcatggcctcttattgtaacagctttaagggccaattctgctgtcaaattacagaataatgagcttagtcctgttgcactacgacagatgtcttgtgctgccggtactacacaaactgcttgcactgatgacaatgcgttagcttactacaacacaacaaagggaggtaggtttgtacttgcactgttatccgatttacaggatttgaaatgggctagattccctaagagtgatggaactggtactatctatacagaactggaaccaccttgtaggtttgttacagacacacctaaaggtcctaaagtgaagtatttatactttattaaaggattaaacaacctaaatagaggtatggtacttggtagtttagctgccacagtacgtctacaagctggtaatgcaacagaagtgcctgccaattcaactgtattatctttctgtgcttttgctgtagatgctgctaaagcttacaaagattatctagctagtgggggacaaccaatcactaattgtgttaagatgttgtgtacacacactggtactggtcaggcaataacagttacaccggaagccaatatggatcaagaatcctttggtggtgcatcgtgttgtctgtactgccgttgccacatagatcatccaaatcctaaaggattttgtgacttaaaaggtaagtatgtacaaatacctacaacttgtgctaatgaccctgtgggttttacacttaaaaacacagtctgtaccgtctgcggtatgtggaaaggttatggctgtagttgtgatcaactccgcgaacccatgcttcagtcagctgatgcacaatcgtttttaaacgggtttgcggtgtaagtgcagcccgtcttacaccgtgcggcacaggcactagtactgatgtcgtatacagggcttttgacatctacaatgataaagtagctggttttgctaaattcctaaaaactaattgttgtcgcttccaagaaaaggacgaagatgacaatttaattgattcttactttgtagttaagagacacactttctctaactaccaacatgaagaaacaatttataatttacttaaggattgtccagctgttgctaaacatgacttctttaagtttagaatagacggtgacatggtaccacatatatcacgtcaacgtcttactaaatacacaatggcagacctcgtctatgctttaaggcattttgatgaaggtaattgtgacacattaaaagaaatacttgtcacatacaattgttgtgatgatgattatttcaataaaaaggactggtatgattttgtagaaaacccagatatattacgcgtatacgccaacttaggtgaacgtgtacgccaagctttgttaaaaacagtacaattctgtgatgccatgcgaaatgctggtattgttggtgtactgacattagataatcaagatctcaatggtaactggtatgatttcggtgatttcatacaaaccacgccaggtagtggagttcctgttgtagattcttattattcattgttaatgcctatattaaccttgaccagggctttaactgcagagtcacatgttgacactgacttaacaaagccttacattaagtgggatttgttaaaatatgacttcacggaagagaggttaaaactctttgaccgttattttaaatattgggatcagacataccacccaaattgtgttaactgtttggatgacagatgcattctgcattgtgcaaactttaatgttttattctctacagtgttcccacctacaagttttggaccactagtgagaaaaatatttgttgatggtgttccatttgtagtttcaactggataccacttcagagagctaggtgttgtacataatcaggatgtaaacttacatagctctagacttagttttaaggaattacttgtgtatgctgctgaccctgctatgcacgctgcttctggtaatctattactagataaacgcactacgtgcttttcagtagctgcacttactaacaatgttgcttttcaaactgtcaaacccggtaattttaacaaagacttctatgactttgctgtgtctaagggtttctttaaggaaggaagttctgttgaattaaaacacttcttctttgctcaggatggtaatgctgctatcagcgattatgactactatcgttataatctaccaacaatgtgtgatatcagacaactactatttgtagttgaagttgttgataagtactttgattgttacgatggtggctgtattaatgctaaccaagtcatcgtcaacaacctagacaaatcagctggttttccatttaataaatggggtaaggctagactttattatgattcaatgagttatgaggatcaagatgcacttttcgcatatacaaaacgtaatgtcatccctactataactcaaatgaatcttaagtatgccattagtgcaaagaatagagctcgcaccgtagctggtgtctctatctgtagtactatgaccaatagacagtttcatcaaaaattattgaaatcaatagccgccactagaggagctactgtagtaattggaacaagcaaattctatggtggttggcacaacatgttaaaaactgtttatagtgatgtagaaaaccctcaccttatgggttgggattatcctaaatgtgatagagccatgcctaacatgcttagaattatggcctcacttgttcttgctcgcaaacatacaacgtgttgtagcttgtcacaccgtttctatagattagctaatgagtgtgctcaagtattgagtgaaatggtcatgtgtggcggttcactatatgttaaaccaggtggaacctcatcaggagatgccacaactgcttatgctaatagtgtttttaacatttgtcaagctgtcacggccaatgttaatgcacttttatctactgatggtaacaaaattgccgataagtatgtccgcaatttacaacacagactttatgagtgtctctatagaaatagagatgttgacacagactttgtgaatgagttttacgcatatttgcgtaaacatttctcaatgatgatactctctgacgatgctgttgtgtgtttcaatagcacttatgcatctcaaggtctagtggctagcataaagaactttaagtcagttctttattatcaaaacaatgtttttatgtctgaagcaaaatgttggactgagactgaccttactaaaggacctcatgaattttgctctcaacatacaatgctagttaaacagggtgatgattatgtgtaccttccttacccagatccatcaagaatcctaggggccggctgttttgtagatgatatcgtaaaaacagatggtacacttatgattgaacggttcgtgtctttagctatagatgcttacccacttactaaacatcctaatcaggagtatgctgatgtctttcatttgtacttacaatacataagaaagctacatgatgagttaacaggacacatgttagacatgtattctgttatgcttactaatgataacacttcaaggtattgggaacctgagttttatgaggctatgtacacaccgcatacagtcttacaggctgttggggcttgtgttctttgcaattcacagacttcattaagatgtggtgcttgcatacgtagaccattcttatgttgtaaatgctgttacgaccatgtcatatcaacatcacataaattagtcttgtctgttaatccgtatgtttgcaatgctccaggttgtgatgtcacagatgtgactcaactttacttaggaggtatgagctattattgtaaatcacataaaccacccattagttttccattgtgtgctaatggacaagtttttggtttatataaaaatacatgtgttggtagcgataatgttactgactttaatgcaattgcaacatgtgactggacaaatgctggtgattacattttagctaacacctgtactgaaagactcaagctttttgcagcagaaacgctcaaagctactgaggagacatttaaactgtcttatggtattgctactgtacgtgaagtgctgtctgacagagaattacatctttcatgggaagttggtaaacctagaccaccacttaaccgaaattatgtctttactggttatcgtgtaactaaaaacagtaaagtacaaataggagagtacacctttgaaaaaggtgactatggtgatgctgttgtttaccgaggtacaacaacttacaaattaaatgttggtgattattttgtgctgacatcacatacagtaatgccattaagtgcacctacactagtgccacaagagcactatgttagaattactggcttatacccaacactcaatatctcagatgagttttctagcaatgttgcaaattatcaaaaggttggtatgcaaaagtattctacactccagggaccacctggtactggtaagagtcattttgctattggcctagctctctactacccttctgctcgcatagtgtatacagcttgctctcatgccgctgttgatgcactatgtgagaaggcattaaaatatttgcctatagataaatgtagtagaattatacctgcacgtgctcgtgtagagtgttttgataaattcaaagtgaattcaacattagaacagtatgtcttttgtactgtaaatgcattgcctgagacgacagcagatatagttgtctttgatgaaatttcaatggccacaaattatgatttgagtgttgtcaatgccagattacgtgctaagcactatgtgtacattggcgaccctgctcaattacctgcaccacgcacattgctaactaagggcacactagaaccagaatatttcaattcagtgtgtagacttatgaaaactataggtccagacatgttcctcggaacttgtcggcgttgtcctgctgaaattgttgacactgtgagtgctttggtttatgataataagcttaaagcacataaagacaaatcagctcaatgctttaaaatgttttataagggtgttatcacgcatgatgtttcatctgcaattaacaggccacaaataggcgtggtaagagaattccttacacgtaaccctgcttggagaaaagctgtctttatttcaccttataattcacagaatgctgtagcctcaaagattttgggactaccaactcaaactgttgattcatcacagggctcagaatatgactatgtcatattcactcaaaccactgaaacagctcactcttgtaatgtaaacagatttaatgttgctattaccagagcaaaagtaggcatactttgcataatgtctgatagagacctttatgacaagttgcaatttacaagtcttgaaattccacgtaggaatgtggcaactttacaagctgaaaatgtaacaggactctttaaagattgtagtaaggtaatcactgggttacatcctacacaggcacctacacacctcagtgttgacactaaattcaaaactgaaggtttatgtgttgacatacctggcatacctaaggacatgacctatagaagactcatctctatgatgggttttaaaatgaattatcaagttaatggttaccctaacatgtttatcacccgcgaagaagctataagacatgtacgtgcatggattggcttcgatgtcgaggggtgtcatgctactagagaagctgttggtaccaatttacctttacagctaggtttttctacaggtgttaacctagttgctgtacctacaggttatgttgatacacctaataatacagatttttccagagttagtgctaaaccaccgcctggagatcaatttaaacacctcataccacttatgtacaaaggacttccttggaatgtagtgcgtataaagattgtacaaatgttaagtgacacacttaaaaatctctctgacagagtcgtatttgtcttatgggcacatggctttgagttgacatctatgaagtattttgtgaaaataggacctgagcgcacctgttgtctatgtgatagacgtgccacatgcttttccactgcttcagacacttatgcctgttggcatcattctattggatttgattacgtctataatccgtttatgattgatgttcaacaatggggttttacaggtaacctacaaagcaaccatgatctgtattgtcaagtccatggtaatgcacatgtagctagttgtgatgcaatcatgactaggtgtctagctgtccacgagtgctttgttaagcgtgttgactggactattgaatatcctataattggtgatgaactgaagattaatgcggcttgtagaaaggttcaacacatggttgttaaagctgcattattagcagacaaattcccagttcttcacgacattggtaaccctaaagctattaagtgtgtacctcaagctgatgtagaatggaagttctatgatgcacagccttgtagtgacaaagcttataaaatagaagaattattctattcttatgccacacattctgacaaattcacagatggtgtatgcctattttggaattgcaatgtcgatagatatcctgctaattccattgtttgtagatttgacactagagtgctatctaaccttaacttgcctggttgtgatggtggcagtttgtatgtaaataaacatgcattccacacaccagcttttgataaaagtgcttttgttaatttaaaacaattaccatttttctattactctgacagtccatgtgagtctcatggaaaacaagtagtgtcagatatagattatgtaccactaaagtctgctacgtgtataacacgttgcaatttaggtggtgctgtctgtagacatcatgctaatgagtacagattgtatctcgatgcttataacatgatgatctcagctggctttagcttgtgggtttacaaacaatttgatacttataacctctggaacacttttacaagacttcagagtttagaaaatgtggcttttaatgttgtaaataagggacactttgatggacaacagggtgaagtaccagtttctatcattaataacactgtttacacaaaagttgatggtgttgatgtagaattgtttgaaaataaaacaacattacctgttaatgtagcatttgagctttgggctaagcgcaacattaaaccagtaccagaggtgaaaatactcaataatttgggtgtggacattgctgctaatactgtgatctgggactacaaaagagatgctccagcacatatatctactattggtgtttgttctatgactgacatagccaagaaaccaactgaaacgatttgtgcaccactcactgtcttttttgatggtagagttgatggtcaagtagacttatttagaaatgcccgtaatggtgttcttattacagaaggtagtgttaaaggtttacaaccatctgtgggtcccaaacaagctagtcttaatggagtcacattaattggagaagccgtaaaaacacagttcaattattataagaaagttgatggtgttgtccaacaattacctgaaacttactttactcagagtagaaatttacaagaatttaaacccaggagtcaaatggaaattgatttcttagaattagctatggatgaattcattgaacggtataaattagaaggctatgccttcgaacatatcgtttatggagattttagtcatagtcagttaggtggtttacatctactgattggactagctaaacgttttaaggaatcaccttttgaattagaagattttattcctatggacagtacagttaaaaactatttcataacagatgcgcaaacaggttcatctaagtgtgtgtgttctgttattgatttattacttgatgattttgttgaaataataaaatcccaagatttatctgtagtttctaaggttgtcaaagtgactattgactatacagaaatttcatttatgctttggtgtaaagatggccatgtagaaacattttacccaaaattacaatctagtcaagcgtggcaaccgggtgttgctatgcctaatctttacaaaatgcaaagaatgctattagaaaagtgtgaccttcaaaattatggtgatagtgcaacattacctaaaggcataatgatgaatgtcgcaaaatatactcaactgtgtcaatatttaaacacattaacattagctgtaccctataatatgagagttatacattttggtgctggttctgataaaggagttgcaccaggtacagctgttttaagacagtggttgcctacgggtacgctgcttgtcgattcagatcttaatgactttgtctctgatgcagattcaactttgattggtgattgtgcaactgtacatacagctaataaatgggatctcattattagtgatatgtacgaccctaagactaaaaatgttacaaaagaaaatgactctaaagagggttttttcacttacatttgtgggtttatacaacaaaagctagctcttggaggttccgtggctataaagataacagaacattcttggaatgctgatctttataagctcatgggacacttcgcatggtggacagcctttgttactaatgtgaatgcgtcatcatctgaagcatttttaattggatgtaattatcttggcaaaccacgcgaacaaatagatggttatgtcatgcatgcaaattacatattttggaggaatacaaatccaattcagttgtcttcctattctttatttgacatgagtaaatttccccttaaattaaggggtactgctgttatgtctttaaaagaaggtcaaatcaatgatatgattttatctcttcttagtaaaggtagacttataattagagaaaacaacagagttgttatttctagtgatgttcttgttaacaactaaacgaacaatgtttgtttttcttgttttattgccactagtctctagtcagtgtgttaatcttacaaccagaactcaattaccccctgcatacactaattctttcacacgtggtgtttattaccctgacaaagttttcagatcctcagttttacattcaactcaggacttgttcttacctttcttttccaatgttacttggttccatgctatacatgtctctgggaccaatggtactaagaggtttgataaccctgtcctaccatttaatgatggtgtttattttgcttccactgagaagtctaacataataagaggctggatttttggtactactttagattcgaagacccagtccctacttattgttaataacgctactaatgttgttattaaagtctgtgaatttcaattttgtaatgatccatttttgggtgtttattaccacaaaaacaacaaaagttggatggaaagtgagttcagagtttattctagtgcgaataattgcacttttgaatatgtctctcagccttttcttatggaccttgaaggaaaacagggtaatttcaaaaatcttagggaatttgtgtttaagaatattgatggttattttaaaatatattctaagcacacgcctattaatttagtgcgtgatctccctcagggtttttcggctttagaaccattggtagatttgccaataggtattaacatcactaggtttcaaactttacttgctttacatagaagttatttgactcctggtgattcttcttcaggttggacagctggtgctgcagcttattatgtgggttatcttcaacctaggacttttctattaaaatataatgaaaatggaaccattacagatgctgtagactgtgcacttgaccctctctcagaaacaaagtgtacgttgaaatccttcactgtagaaaaaggaatctatcaaacttctaactttagagtccaaccaacagaatctattgttagatttcctaatattacaaacttgtgcccttttggtgaagtttttaacgccaccagatttgcatctgtttatgcttggaacaggaagagaatcagcaactgtgttgctgattattctgtcctatataattccgcatcattttccacttttaagtgttatggagtgtctcctactaaattaaatgatctctgctttactaatgtctatgcagattcatttgtaattagaggtgatgaagtcagacaaatcgctccagggcaaactggaaagattgctgattataattataaattaccagatgattttacaggctgcgttatagcttggaattctaacaatcttgattctaaggttggtggtaattataattacctgtatagattgtttaggaagtctaatctcaaaccttttgagagagatatttcaactgaaatctatcaggccggtagcacaccttgtaatggtgttgaaggttttaattgttactttcctttacaatcatatggtttccaacccactaatggtgttggttaccaaccatacagagtagtagtactttcttttgaacttctacatgcaccagcaactgtttgtggacctaaaaagtctactaatttggttaaaaacaaatgtgtcaatttcaacttcaatggtttaacaggcacaggtgttcttactgagtctaacaaaaagtttctgcctttccaacaatttggcagagacattgctgacactactgatgctgtccgtgatccacagacacttgagattcttgacattacaccatgttcttttggtggtgtcagtgttataacaccaggaacaaatacttctaaccaggttgctgttctttatcaggatgttaactgcacagaagtccctgttgctattcatgcagatcaacttactcctacttggcgtgtttattctacaggttctaatgtttttcaaacacgtgcaggctgtttaataggggctgaacatgtcaacaactcatatgagtgtgacatacccattggtgcaggtatatgcgctagttatcagactcagactaattctcctcggcgggcacgtagtgtagctagtcaatccatcattgcctacactatgtcacttggtgcagaaaattcagttgcttactctaataactctattgccatacccacaaattttactattagtgttaccacagaaattctaccagtgtctatgaccaagacatcagtagattgtacaatgtacatttgtggtgattcaactgaatgcagcaatcttttgttgcaatatggcagtttttgtacacaattaaaccgtgctttaactggaatagctgttgaacaagacaaaaacacccaagaagtttttgcacaagtcaaacaaatttacaaaacaccaccaattaaagattttggtggttttaatttttcacaaatattaccagatccatcaaaaccaagcaagaggtcatttattgaagatctacttttcaacaaagtgacacttgcagatgctggcttcatcaaacaatatggtgattgccttggtgatattgctgctagagacctcatttgtgcacaaaagtttaacggccttactgttttgccacctttgctcacagatgaaatgattgctcaatacacttctgcactgttagcgggtacaatcacttctggttggacctttggtgcaggtgctgcattacaaataccatttgctatgcaaatggcttataggtttaatggtattggagttacacagaatgttctctatgagaaccaaaaattgattgccaaccaatttaatagtgctattggcaaaattcaagactcactttcttccacagcaagtgcacttggaaaacttcaagatgtggtcaaccaaaatgcacaagctttaaacacgcttgttaaacaacttagctccaattttggtgcaatttcaagtgttttaaatgatatcctttcacgtcttgacaaagttgaggctgaagtgcaaattgataggttgatcacaggcagacttcaaagtttgcagacatatgtgactcaacaattaattagagctgcagaaatcagagcttctgctaatcttgctgctactaaaatgtcagagtgtgtacttggacaatcaaaaagagttgatttttgtggaaagggctatcatcttatgtccttccctcagtcagcacctcatggtgtagtcttcttgcatgtgacttatgtccctgcacaagaaaagaacttcacaactgctcctgccatttgtcatgatggaaaagcacactttcctcgtgaaggtgtctttgtttcaaatggcacacactggtttgtaacacaaaggaatttttatgaaccacaaatcattactacagacaacacatttgtgtctggtaactgtgatgttgtaataggaattgtcaacaacacagtttatgatcctttgcaacctgaattagactcattcaaggaggagttagataaatattttaagaatcatacatcaccagatgttgatttaggtgacatctctggcattaatgcttcagttgtaaacattcaaaaagaaattgaccgcctcaatgaggttgccaagaatttaaatgaatctctcatcgatctccaagaacttggaaagtatgagcagtatataaaatggccatggtacatttggctaggttttatagctggcttgattgccatagtaatggtgacaattatgctttgctgtatgaccagttgctgtagttgtctcaagggctgttgttcttgtggatcctgctgcaaatttgatgaagacgactctgagccagtgctcaaaggagtcaaattacattacacataattcctgatcttctggtctaaacgaactaaatattatattagtttttctgtttggaactttaattttagccatggcagattccaacggtactattaccgttgaagagcttaaaaagctccttgaacaatggaacctagtaataggtttcctattccttacatggatttgtcttctacaatttgcctatgccaacaggaataggtttttgtatataattaagttaattttcctctggctgttatggccagtaactttagcttgttttgtgcttgctgctgtttacagaataaattggatcaccggtggaattgctatcgcaatggcttgtcttgtaggcttgatgtggctcagctacttcattgcttctttcagactgtttgcgcgtacccgttccatgtggtcattcaatccagaaactaacattcttctcaacgtgccactccatggcactattctgaccagaccgcttctagaaagtgaactcgtaatcggagctgtgatccttcgtggacatcttcgtattgctggacaccatctaggacgctgtgacatcaaggacctgcctaaagaaatcactgttgctacatcccgcacgctttcttattacaaattgggagcttcgcagcgtgtagcaggtgactcaggttttgctgcatacagtcgctacaggattggcaactataaattaaacacagaccattccagtagcagtgacaatattgctttgcttgtacagtaagtgacaacagaaccaatggagattgattaaacgaacatgaaaattattcttttcttggcactgataacactcgctacttgtgagctttatcactaccaagagtgtgttagaggtacaacagtacttttaaaagaaccttgctcttctggaacatacgagggcaattcaccatttcatcctctagctgataacaaatttgcactgacttgctttagcactcaatttgcttttgcttgtcctgacggcgtaaaacacgtctatcagttacgtgccagatcagtttcacctaaactgttcatcagacaagaggaagttcaagaactttactctccaatttttcttattgttgcggcaatagtgtttataacactttgcttcacactcaaaagaaagacagaatgattgaactttcattaattgacttctatttgtgctttttagcctttctgctattccttgttttaattatgcttattatcttttggttctcacttgaactgcaagatcataatgaaacttgtcacgcctaaacgaacatgaaatttcttgttttcttaggaatcatcacaactgtagctgcatttcaccaagaatgtagtttacagtcatgtactcaacatcaaccatatgtagttgatgacccgtgtcctattcacttctattctaaatggtatattagagtaggagctagaaaatcagcacctttaattgaattgtgcgtggatgaggctggttctaaatcacccattcagtacatcgatatcggtaattatacagtttcctgtttaccttttacaattaattgccaggaacctaaattgggtagtcttgtagtgcgttgttcgttctatgaagactttttagagtatcatgacgttcgtgttgttttagatttcatctaaacgaacaaactaaaatgtctgataatggaccccaaaatcagcgaaatgcaccccgcattacgtttggtggaccctcagattcaactggcagtaaccagaatggagaacgcagtggggcgcgatcaaaacaacgtcggccccaaggtttacccaataatactgcgtcttggttcaccgctctcactcaacatggcaaggaagaccttaaattccctcgaggacaaggcgttccaattaacaccaatagcagtccagatgaccaaattggctactaccgaagagctaccagacgaattcgtggtggtgacggtaaaatgaaagatctcagtccaagatggtatttctactacctaggaactgggccagaagctggacttccctatggtgctaacaaagacggcatcatatgggttgcaactgagggagccttgaatacaccaaaagatcacattggcacccgcaatcctgctaacaatgctgcaatcgtgctacaacttcctcaaggaacaacattgccaaaaggcttctacgcagaagggagcagaggcggcagtcaagcctcttctcgttcctcatcacgtagtcgcaacagttcaagaaattcaactccaggcagcagtaggggaacttctcctgctagaatggctggcaatggcggtgatgctgctcttgctttgctgctgcttgacagattgaaccagcttgagagcaaaatgtctggtaaaggccaacaacaacaaggccaaactgtcactaagaaatctgctgctgaggcttctaagaagcctcggcaaaaacgtactgccactaaagcatacaatgtaacacaagctttcggcagacgtggtccagaacaaacccaaggaaattttggggaccaggaactaatcagacaaggaactgattacaaacattggccgcaaattgcacaatttgcccccagcgcttcagcgttcttcggaatgtcgcgcattggcatggaagtcacaccttcgggaacgtggttgacctacacagctgccatcaaattggatgacaaagatccaaatttcaaagatcaagtcattttgctgaataagcatattgacgcatacaaaacattcccaccaacagagcctaaaaaggacaaaaagaagaaggctgatgaaactcaagccttaccgcagagacagaagaaacagcaaactgtgactcttcttcctgctgcagatttggatgatttctccaaacaattgcaacaatccatgagcagtgctgactcaactcaggcctaaactcatgcagaccacacaaggcagatgggctatataaacgttttcgcttttccgtttacgatatatagtctactcttgtgcagaatgaattctcgtaactacatagcacaagtagatgtagttaactttaatctcacatagcaatctttaatcagtgtgtaacattagggaggacttgaaagagccaccacattttcaccgaggccacgcggagtacgatcgagtgtacagtgaacaatgctagggagagctgcctatatggaagagccctaatgtgtaaaattaattttagtagtgctatccccatgtgattttaatagcttcttaggagaatgac

SEQ ID NO: 48 - DNA, 28430 bp, Coronaviridae
  source 1..28430: mol_type = other DNA
  misc_feature 1..28430: note = SARS-CoV-2-[3,E,7] polynucleotide sequence
attaaaggtttataccttcccaggtaacaaaccaaccaactttcgatctcttgtagatctgttctctaaacgaactttaaaatctgtgtggctgtcactcggctgcatgcttagtgcactcacgcagtataattaataactaattactgtcgttgacaggacacgagtaactcgtctatcttctgcaggctgcttacggtttcgtccgtgttgcagccgatcatcagcacatctaggtttcgtccgggtgtgaccgaaaggtaagatggagagccttgtccctggtttcaacgagaaaacacacgtccaactcagtttgcctgttttacaggttcgcgacgtgctcgtacgtggctttggagactccgtggaggaggtcttatcagaggcacgtcaacatcttaaagatggcacttgtggcttagtagaagttgaaaaaggcgttttgcctcaacttgaacagccctatgtgttcatcaaacgttcggatgctcgaactgcacctcatggtcatgttatggttgagctggtagcagaactcgaaggcattcagtacggtcgtagtggtgagacacttggtgtccttgtccctcatgtgggcgaaataccagtggcttaccgcaaggttcttcttcgtaagaacggtaataaaggagctggtggccatagttacggcgccgatctaaagtcatttgacttaggcgacgagcttggcactgatccttatgaagattttcaagaaaactggaacactaaacatagcagtggtgttacccgtgaactcatgcgtgagcttaacggaggggcatacactcgctatgtcgataacaacttctgtggccctgatggctaccctcttgagtgcattaaagaccttctagcacgtgctggtaaagcttcatgcactttgtccgaacaactggactttattgacactaagaggggtgtatactgctgccgtgaacatgagcatgaaattgcttggtacacggaacgttctgaaaagagctatgaattgcagacaccttttgaaattaaattggcaaagaaatttgacaccttcaatggggaatgtccaaattttgtatttcccttaaattccataatcaagactattcaaccaagggttgaaaagaaaaagcttgatggctttatgggtagaattcgatctgtctatccagttgcgtcaccaaatgaatgcaaccaaatgtgcctttcaactctcatgaagtgtgatcattgtggtgaaacttcatggcagacgggcgattttgttaaagccacttgcgaattttgtggcactgagaatttgactaaagaaggtgccactacttgtggttacttaccccaaaatgctgttgttaaaatttattgtccagcatgtcacaattcagaagtaggacctgagcatagtcttgccgaataccataatgaatctggcttgaaaaccattcttcgtaagggtggtcgcactattgcctttggaggctgtgtgttctcttatgttggttgccataacaagtgtgcctattgggttccacgtgctagcgctaacataggttgtaaccatacaggtgttgttggagaaggttccgaaggtcttaatgacaaccttcttgaaatactccaaaaagagaaagtcaacatcaatattgttggtgactttaaacttaatgaagagatcgccattattttggcatctttttctgcttccacaagtgcttttgtggaaactgtgaaaggtttggattataaagcattcaaacaaattgttgaatcctgtggtaattttaaagttacaaaaggaaaagctaaaaaaggtgcctggaatattggtgaacagaaatcaatactgagtcctctttatgcatttgcatcagaggctgctcgtgttgtacgatcaattttctcccgcactcttgaaactgctcaaaattctgtgcgtgttttacagaaggccgctataacaatactagatggaatttcacagtattcactgagactcattgatgctatgatgttcacatctgatttggctactaacaatctagttgtaatggcctacattacaggtggtgttgttcagttgacttcgcagtggctaactaacatctttggcactgtttatgaaaaactcaaacccgtccttgattggcttgaagagaagtttaaggaaggtgtagagtttcttagagacggttgggaaattgttaaatttatctcaacctgtgcttgtgaaattgtcggtggacaaattgtcacctgtgcaaaggaaattaaggagagtgttcagacattctttaagcttgtaaataaatttttggctttgtgtgctgactctatcattattggtggagctaaacttaaagccttgaatttaggtgaaacatttgtcacgcactcaaagggattgtacagaaagtgtgttaaatccagagaagaaactggcctactcatgcctctaaaagccccaaaagaaattatcttcttagagggagaaacacttcccacagaagtgttaacagaggaagttgtcttgaaaactggtgatttacaaccattagaacaacctactagtgaagctgttgaagctccattggttggtacaccagtttgtattaacgggcttatgttgctcgaaatcaaagacacagaaaagtactgtgcccttgcacctaatatgatggtaacaaacaataccttcacactcaaaggcggtgcaccaacaaaggttacttttggtgatgacactgtgatagaagtgcaaggttacaagagtgtgaatatcacttttgaacttgatgaaaggattgataaagtacttaatgagaagtgctctgcctatacagttgaactcggtacagaagtaaatgagttcgcctgtgttgtggcagatgctgtcataaaaactttgcaaccagtatctgaattacttacaccactgggcattgatttagatgagtggagtatggctacatactacttatttgatgagtctggtgagtttaaattggcttcacatatgtattgttctttctaccctccagatgaggatgaagaagaaggtgattgtgaagaagaagagtttgagccatcaactcaatatgagtatggtactgaagatgattaccaaggtaaacctttggaatttggtgccacttctgctgctcttcaacctgaagaagagcaagaagaagattggttagatgatgatagtcaacaaactgttggtcaacaagacggcagtgaggacaatcagacaactactattcaaacaattgttgaggttcaacctcaattagagatggaacttacaccagttgttcagactattgaagtgaatagttttagtggttatttaaaacttactgacaatgtatacattaaaaatgcagacattgtggaagaagctaaaaaggtaaaaccaacagtggttgttaatgcagccaatgtttaccttaaacatggaggaggtgttgcaggagccttaaataaggctactaacaatgccatgcaagttgaatctgatgattacatagctactaatggaccacttaaagtgggtggtagttgtgttttaagcggacacaatcttgctaaacactgtcttcatgttgtcggcccaaatgttaacaaaggtgaagacattcaacttcttaagagtgcttatgaaaattttaatcagcacgaagttctacttgcaccattattatcagctggtatttttggtgctgaccctatacattctttaagagtttgtgtagatactgttcgcacaaatgtctacttagctgtctttgataaaaatctctatgacaaacttgtttcaagctttttggaaatgaagagtgaaaagcaagttgaacaaaagatcgctgagattcctaaagaggaagttaagccatttataactgaaagtaaaccttcagttgaacagagaaaacaagatgataagaaaatcaaagcttgtgttgaagaagttacaacaactctggaagaaactaagttcctcacagaaaacttgttactttatattgacattaatggcaatcttcatccagattctgccactcttgttagtgacattgacatcactttcttaaagaaagatgctccatatatagtgggtgatgttgttcaagagggtgttttaactgctgtggttatacctactaaaaaggctggtggcactactgaaatgctagcgaaagctttgagaaaagtgccaacagacaattatataaccacttacccgggtcagggtttaaatggttacactgtagaggaggcaaagacagtgcttaaaaagtgtaaaagtgccttttacattctaccatctattatctctaatgagaagcaagaaattcttggaactgtttcttggaatttgcgagaaatgcttgcacatgcagaagaaacacgcaaattaatgcctgtctgtgtggaaactaaagccatagtttcaactatacagcgtaaatataagggtattaaaatacaagagggtgtggttgattatggtgctagattttacttttacaccagtaaaacaactgtagcgtcacttatcaacacacttaacgatctaaatgaaactcttgttacaatgccacttggctatgtaacacatggcttaaatttggaagaagctgctcggtatatgagatctctcaaagtgccagctacagtttctgtttcttcacctgatgctgttacagcgtataatggttatcttacttcttcttctaaaacacctgaagaacattttattgaaaccatctcacttgctggttcctataaagattggtcctattctggacaatctacacaactaggtatagaatttcttaagagaggtgataaaagtgtatattacactagtaatcctaccacattccacctagatggtgaagttatcacctttgacaatcttaagacacttctttctttgagagaagtgaggactattaaggtgtttacaacagtagacaacattaacctccacacgcaagttgtggacatgtcaatgacatatggacaacagtttggtccaacttatttggatggagctgatgttactaaaataaaacctcataattcacatgaaggtaaaacattttatgttttacctaatgatgacactctacgtgttgaggcttttgagtactaccacacaactgatcctagttttctgggtaggtacatgtcagcattaaatcacactaaaaagtggaaatacccacaagttaatggtttaacttctattaaatgggcagataacaactgttatcttgccactgcattgttaacactccaacaaatagagttgaagtttaatccacctgctctacaagatgcttattacagagcaagggctggtgaagctgctaacttttgtgcacttatcttagcctactgtaataagacagtaggtgagttaggtgatgttagagaaacaatgagttacttgtttcaacatgccaatttagattcttgcaaaagagtcttgaacgtggtgtgtaaaacttgtggacaacagcagacaacccttaagggtgtagaagctgttatgtacatgggcacactttcttatgaacaatttaagaaaggtgttcagataccttgtacgtgtggtaaacaagctacaaaatatctagtacaacaggagtcaccttttgttatgatgtcagcaccacctgctcagtatgaacttaagcatggtacatttacttgtgctagtgagtacactggtaattaccagtgtggtcactataaacatataacttctaaagaaactttgtattgcatagacggtgctttacttacaaagtcctcagaatacaaaggtcctattacggatgttttctacaaagaaaacagttacacaacaaccataaaaccagttacttataaattggatggtgttgtttgtacagaaattgaccctaagttggacaattattataagaaagacaattcttatttcacagagcaaccaattgatcttgtaccaaaccaaccatatccaaacgcaagcttcgataattttaagtttgtatgtgataatatcaaatttgctgatgatttaaaccagttaactggttataagaaacctgcttcaagagagcttaaagttacatttttccctgacttaaatggtgatgtggtggctattgattataaacactacacaccctcttttaagaaaggagctaaattgttacataaacctattgtttggcatgttaacaatgcaactaataaagccacgtataaaccaaatacctggtgtatacgttgtctttggagcacaaaaccagttgaaacatcaaattcgtttgatgtactgaagtcagaggacgcgcagggaatggataatcttgcctgcgaagatctaaaaccagtctctgaagaagtagtggaaaatcctaccatacagaaagacgttcttgagtgtaatgtgaaaactaccgaagttgtaggagacattatacttaaaccagcaaataatagtttaaaaattacagaagaggttggccacacagatctaatggctgcttatgtagacaattctagtcttactattaagaaacctaatgaattatctagagtattaggtttgaaaacccttgctactcatggtttagctgctgttaatagtgtcccttgggatactatagctaattatgctaagccttttcttaacaaagttgttagtacaactactaacatagttacacggtgtttaaaccgtgtttgtactaattatatgccttatttctttactttattgctacaattgtgtacttttactagaagtacaaattctagaattaaagcatctatgccgactactatagcaaagaatactgttaagagtgtcggtaaattttgtctagaggcttcatttaattatttgaagtcacctaatttttctaaactgataaatattataatttggtttttactattaagtgtttgcctaggttctttaatctactcaaccgctgctttaggtgttttaatgtctaatttaggcatgccttcttactgtactggttacagagaaggctatttgaactctactaatgtcactattgcaacctactgtactggttctataccttgtagtgtttgtcttagtggtttagattctttagacacctatccttctttagaaactatacaaattaccatttcatcttttaaatgggatttaactgcttttggcttagttgcagagtggtttttggcatatattcttttcactaggtttttctatgtacttggattggctgcaatcatgcaattgtttttcagctattttgcagtacattttattagtaattcttggcttatgtggttaataattaatcttgtacaaatggccccgatttcagctatggttagaatgtacatcttctttgcatcattttattatgtatggaaaagttatgtgcatgttgtagacggttgtaattcatcaacttgtatgatgtgttacaaacgtaatagagcaacaagagtcgaatgtacaactattgttaatggtgttagaaggtccttttatgtctatgctaatggaggtaaaggcttttgcaaactacacaattggaattgtgttaattgtgatacattctgtgctggtagtacatttattagtgatgaagttgcgagagacttgtcactacagtttaaaagaccaataaatcctactgaccagtcttcttacatcgttgatagtgttacagtgaagaatggttccatccatctttactttgataaagctggtcaaaagacttatgaaagacattctctctctcattttgttaacttagacaacctgagagctaataacactaaaggttcattgcctattaatgttatagtttttgatggtaaatcaaaatgtgaagaatcatctgcaaaatcagcgtctgtttactacagtcagcttatgtgtcaacctatactgttactagatcaggcattagtgtctgatgttggtgatagtgcggaagttgcagttaaaatgtttgatgcttacgttaatacgttttcatcaacttttaacgtaccaatggaaaaactcaaaacactagttgcaactgcagaagctgaacttgcaaagaatgtgtccttagacaatgtcttatctacttttatttcagcagctcggcaagggtttgttgattcagatgtagaaactaaagatgttgttgaatgtcttaaattgtcacatcaatctgacatagaagttactggcgatagttgtaataactatatgctcacctataacaaagttgaaaacatgacaccccgtgaccttggtgcttgtattgactgtagtgcgcgtcatattaatgcgcaggtagcaaaaagtcacaacattgctttgatatggaacgttaaagatttcatgtcattgtctgaacaactacgaaaacaaatacgtagtgctgctaaaaagaataacttaccttttaagttgacatgtgcaactactagacaagttgttaatgttgtaacaacaaagatagcacttaagggtggtaaaattgttaataattggttgaagcagttaattaaagttacacttgtgttcctttttgttgctgctattttctatttaataacacctgttcatgtcatgtctaaacatactgacttttcaagtgaaatcataggatacaaggctattgatggtggtgtcactcgtgacatagcatctacagatacttgttttgctaacaaacatgctgattttgacacatggtttagccagcgtggtggtagttatactaatgacaaagcttgcccattgattgctgcagtcataacaagagaagtgggttttgtcgtgcctggtttgcctggcacgatattacgcacaactaatggtgactttttgcatttcttacctagagtttttagtgcagttggtaacatctgttacacaccatcaaaacttatagagtacactgactttgcaacatcagcttgtgttttggctgctgaatgtacaatttttaaagatgcttctggtaagccagtaccatattgttatgataccaatgtactagaaggttctgttgcttatgaaagtttacgccctgacacacgttatgtgctcatggatggctctattattcaatttcctaacacctaccttgaaggttctgttagagtggtaacaacttttgattctgagtactgtaggcacggcacttgtgaaagatcagaagctggtgtttgtgtatctactagtggtagatgggtacttaacaatgattattacagatctttaccaggagttttctgtggtgtagatgctgtaaatttacttactaatatgtttacaccactaattcaacctattggtgctttggacatatcagcatctatagtagctggtggtattgtagctatcgtagtaacatgccttgcctactattttatgaggtttagaagagcttttggtgaatacagtcatgtagttgcctttaatactttactattccttatgtcattcactgtactctgtttaacaccagtttactcattcttacctggtgtttattctgttatttacttgtacttgacattttatcttactaatgatgtttcttttttagcacatattcagtggatggttatgttcacacctttagtacctttctggataacaattgcttatatcatttgtatttccacaaagcatttctattggttctttagtaattacctaaagagacgtgtagtctttaatggtgtttcctttagtacttttgaagaagctgcgctgtgcacctttttgttaaataaagaaatgtatctaaagttgcgtagtgatgtgctattacctcttacgcaatataatagatacttagctctttataataagtacaagtattttagtggagcaatggatacaactagctacagagaagctgcttgttgtcatctcgcaaaggctctcaatgacttcagtaactcaggttctgatgttctttaccaaccaccacaaacctctatcacctcagctgttttgcagagtggttttagaaaaatggcattcccatctggtaaagttgagggttgtatggtacaagtaacttgtggtacaactacacttaacggtctttggcttgatgacgtagtttactgtccaagacatgtgatctgcacctctgaagacatgcttaaccctaattatgaagatttactcattcgtaagtctaatcataatttcttggtacaggctggtaatgttcaactcagggttattggacattctatgcaaaattgtgtacttaagcttaaggttgatacagccaatcctaagacacctaagtataagtttgttcgcattcaaccaggacagactttttcagtgttagcttgttacaatggttcaccatctggtgtttaccaatgtgctatgaggcccaatttcactattaagggttcattccttaatggttcatgtggtagtgttggttttaacatagattatgactgtgtctctttttgttacatgcaccatatggaattaccaactggagttcatgctggcacagacttagaaggtaacttttatggaccttttgttgacaggcaaacagcacaagcagctggtacggacacaactattacagttaatgttttagcttggttgtacgctgctgttataaatggagacaggtggtttctcaatcgatttaccacaactcttaatgactttaaccttgtggctatgaagtacaattatgaacctctaacacaagaccatgttgacatactaggacctctttctgctcaaactggaattgccgttttagatatgtgtgcttcattaaaagaattactgcaaaatggtatgaatggacgtaccatattgggtagtgctttattagaagatgaatttacaccttttgatgttgttagacaatgctcaggtgttactttccaaagtgcagtgaaaagaacaatcaagggtacacaccactggttgttactcacaattttgacttcacttttagttttagtccagagtactcaatggtctttgttcttttttttgtatgaaaatgcctttttaccttttgctatgggtattattgctatgtctgcttttgcaatgatgtttgtcaaacataagcatgcatttctctgtttgtttttgttaccttctcttgccactgtagcttattttaatatggtctatatgcctgctagttgggtgatgcgtattatgacatggttggatatggttgatactagtttgtctggttttaagctaaaagactgtgttatgtatgcatcagctgtagtgttactaatccttatgacagcaagaactgtgtatgatgatggtgctaggagagtgtggacacttatgaatgtcttgacactcgtttataaagtttattatggtaatgctttagatcaagccatttccatgtgggctcttataatctctgttacttctaactactcaggtgtagttacaactgtcatgtttttggccagaggtattgtttttatgtgtgttgagtattgccctattttcttcataactggtaatacacttcagtgtataatgctagtttattgtttcttaggctatttttgtacttgttactttggcctcttttgtttactcaaccgctactttagactgactcttggtgtttatgattacttagtttctacacaggagtttagatatatgaattcacagggactactcccacccaagaatagcatagatgccttcaaactcaacattaaattgttgggtgttggtggcaaaccttgtatcaaagtagccactgtacagtctaaaatgtcagatgtaaagtgcacatcagtagtcttactctcagttttgcaacaactcagagtagaatcatcatctaaattgtgggctcaatgtgtccagttacacaatgacattctcttagctaaagatactactgaagcctttgaaaaaatggtttcactactttctgttttgctttccatgcagggtgctgtagacataaacaagctttgtgaagaaatgctggacaacagggcaaccttacaagctatagcctcagagtttagttcccttccatcatatgcagcttttgctactgctcaagaagcttatgagcaggctgttgctaatggtgattctgaagttgttcttaaaaagttgaagaagtctttgaatgtggctaaatctgaatttgaccgtgatgcagccatgcaacgtaagttggaaaagatggctgatcaagctatgacccaaatgtataaacaggctagatctgaggacaagagggcaaaagttactagtgctatgcagacaatgcttttcactatgcttagaaagttggataatgatgcactcaacaacattatcaacaatgcaagagatggttgtgttcccttgaacataatacctcttacaacagcagccaaactaatggttgtcataccagactataacacatataaaaatacgtgtgatggtacaacatttacttatgcatcagcattgtgggaaatccaacaggttgtagatgcagatagtaaaattgttcaacttagtgaaattagtatggacaattcacctaatttagcatggcctcttattgtaacagctttaagggccaattctgctgtcaaattacagaataatgagcttagtcctgttgcactacgacagatgtcttgtgctgccggtactacacaaactgcttgcactgatgacaatgcgttagcttactacaacacaacaaagggaggtaggtttgtacttgcactgttatccgatttacaggatttgaaatgggctagattccctaagagtgatggaactggtactatctatacagaactggaaccaccttgtaggtttgttacagacacacctaaaggtcctaaagtgaagtatttatactttattaaaggattaaacaacctaaatagaggtatggtacttggtagtttagctgccacagtacgtctacaagctggtaatgcaacagaagtgcctgccaattcaactgtattatctttctgtgcttttgctgtagatgctgctaaagcttacaaagattatctagctagtgggggacaaccaatcactaattgtgttaagatgttgtgtacacacactggtactggtcaggcaataacagttacaccggaagccaatatggatcaagaatcctttggtggtgcatcgtgttgtctgtactgccgttgccacatagatcatccaaatcctaaaggattttgtgacttaaaaggtaagtatgtacaaatacctacaacttgtgctaatgaccctgtgggttttacacttaaaaacacagtctgtaccgtctgcggtatgtggaaaggttatggctgtagttgtgatcaactccgcgaacccatgcttcagtcagctgatgcacaatcgtttttaaacgggtttgcggtgtaagtgcagcccgtcttacaccgtgcggcacaggcactagtactgatgtcgtatacagggcttttgacatctacaatgataaagtagctggttttgctaaattcctaaaaactaattgttgtcgcttccaagaaaaggacgaagatgacaatttaattgattcttactttgtagttaagagacacactttctctaactaccaacatgaagaaacaatttataatttacttaaggattgtccagctgttgctaaacatgacttctttaagtttagaatagacggtgacatggtaccacatatatcacgtcaacgtcttactaaatacacaatggcagacctcgtctatgctttaaggcattttgatgaaggtaattgtgacacattaaaagaaatacttgtcacatacaattgttgtgatgatgattatttcaataaaaaggactggtatgattttgtagaaaacccagatatattacgcgtatacgccaacttaggtgaacgtgtacgccaagctttgttaaaaacagtacaattctgtgatgccatgcgaaatgctggtattgttggtgtactgacattagataatcaagatctcaatggtaactggtatgatttcggtgatttcatacaaaccacgccaggtagtggagttcctgttgtagattcttattattcattgttaatgcctatattaaccttgaccagggctttaactgcagagtcacatgttgacactgacttaacaaagccttacattaagtgggatttgttaaaatatgacttcacggaagagaggttaaaactctttgaccgttattttaaatattgggatcagacataccacccaaattgtgttaactgtttggatgacagatgcattctgcattgtgcaaactttaatgttttattctctacagtgttcccacctacaagttttggaccactagtgagaaaaatatttgttgatggtgttccatttgtagtttcaactggataccacttcagagagctaggtgttgtacataatcaggatgtaaacttacatagctctagacttagttttaaggaattacttgtgtatgctgctgaccctgctatgcacgctgcttctggtaatctattactagataaacgcactacgtgcttttcagtagctgcacttactaacaatgttgcttttcaaactgtcaaacccggtaattttaacaaagacttctatgactttgctgtgtctaagggtttctttaaggaaggaagttctgttgaattaaaacacttcttctttgctcaggatggtaatgctgctatcagcgattatgactactatcgttataatctaccaacaatgtgtgatatcagacaactactatttgtagttgaagttgttgataagtactttgattgttacgatggtggctgtattaatgctaaccaagtcatcgtcaacaacctagacaaatcagctggttttccatttaataaatggggtaaggctagactttattatgattcaatgagttatgaggatcaagatgcacttttcgcatatacaaaacgtaatgtcatccctactataactcaaatgaatcttaagtatgccattagtgcaaagaatagagctcgcaccgtagctggtgtctctatctgtagtactatgaccaatagacagtttcatcaaaaattattgaaatcaatagccgccactagaggagctactgtagtaattggaacaagcaaattctatggtggttggcacaacatgttaaaaactgtttatagtgatgtagaaaaccctcaccttatgggttgggattatcctaaatgtgatagagccatgcctaacatgcttagaattatggcctcacttgttcttgctcgcaaacatacaacgtgttgtagcttgtcacaccgtttctatagattagctaatgagtgtgctcaagtattgagtgaaatggtcatgtgtggcggttcactatatgttaaaccaggtggaacctcatcaggagatgccacaactgcttatgctaatagtgtttttaacatttgtcaagctgtcacggccaatgttaatgcacttttatctactgatggtaacaaaattgccgataagtatgtccgcaatttacaacacagactttatgagtgtctctatagaaatagagatgttgacacagactttgtgaatgagttttacgcatatttgcgtaaacatttctcaatgatgatactctctgacgatgctgttgtgtgtttcaatagcacttatgcatctcaaggtctagtggctagcataaagaactttaagtcagttctttattatcaaaacaatgtttttatgtctgaagcaaaatgttggactgagactgaccttactaaaggacctcatgaattttgctctcaacatacaatgctagttaaacagggtgatgattatgtgtaccttccttacccagatccatcaagaatcctaggggccggctgttttgtagatgatatcgtaaaaacagatggtacacttatgattgaacggttcgtgtctttagctatagatgcttacccacttactaaacatcctaatcaggagtatgctgatgtctttcatttgtacttacaatacataagaaagctacatgatgagttaacaggacacatgttagacatgtattctgttatgcttactaatgataacacttcaaggtattgggaacctgagttttatgaggctatgtacacaccgcatacagtcttacaggctgttggggcttgtgttctttgcaattcacagacttcattaagatgtggtgcttgcatacgtagaccattcttatgttgtaaatgctgttacgaccatgtcatatcaacatcacataaattagtcttgtctgttaatccgtatgtttgcaatgctccaggttgtgatgtcacagatgtgactcaactttacttaggaggtatgagctattattgtaaatcacataaaccacccattagttttccattgtgtgctaatggacaagtttttggtttatataaaaatacatgtgttggtagcgataatgttactgactttaatgcaattgcaacatgtgactggacaaatgctggtgattacattttagctaacacctgtactgaaagactcaagctttttgcagcagaaacgctcaaagctactgaggagacatttaaactgtcttatggtattgctactgtacgtgaagtgctgtctgacagagaattacatctttcatgggaagttggtaaacctagaccaccacttaaccgaaattatgtctttactggttatcgtgtaactaaaaacagtaaagtacaaataggagagtacacctttgaaaaaggtgactatggtgatgctgttgtttaccgaggtacaacaacttacaaattaaatgttggtgattattttgtgctgacatcacatacagtaatgccattaagtgcacctacactagtgccacaagagcactatgttagaattactggcttatacccaacactcaatatctcagatgagttttctagcaatgttgcaaattatcaaaaggttggtatgcaaaagtattctacactccagggaccacctggtactggtaagagtcattttgctattggcctagctctctactacccttctgctcgcatagtgtatacagcttgctctcatgccgctgttgatgcactatgtgagaaggcattaaaatatttgcctatagataaatgtagtagaattatacctgcacgtgctcgtgtagagtgttttgataaattcaaagtgaattcaacattagaacagtatgtcttttgtactgtaaatgcattgcctgagacgacagcagatatagttgtctttgatgaaatttcaatggccacaaattatgatttgagtgttgtcaatgccagattacgtgctaagcactatgtgtacattggcgaccctgctcaattacctgcaccacgcacattgctaactaagggcacactagaaccagaatatttcaattcagtgtgtagacttatgaaaactataggtccagacatgttcctcggaacttgtcggcgttgtcctgctgaaattgttgacactgtgagtgctttggtttatgataataagcttaaagcacataaagacaaatcagctcaatgctttaaaatgttttataagggtgttatcacgcatgatgtttcatctgcaattaacaggccacaaataggcgtggtaagagaattccttacacgtaaccctgcttggagaaaagctgtctttatttcaccttataattcacagaatgctgtagcctcaaagattttgggactaccaactcaaactgttgattcatcacagggctcagaatatgactatgtcatattcactcaaaccactgaaacagctcactcttgtaatgtaaacagatttaatgttgctattaccagagcaaaagtaggcatactttgcataatgtctgatagagacctttatgacaagttgcaatttacaagtcttgaaattccacgtaggaatgtggcaactttacaagctgaaaatgtaacaggactctttaaagattgtagtaaggtaatcactgggttacatcctacacaggcacctacacacctcagtgttgacactaaattcaaaactgaaggtttatgtgttgacatacctggcatacctaaggacatgacctatagaagactcatctctatgatgggttttaaaatgaattatcaagttaatggttaccctaacatgtttatcacccgcgaagaagctataagacatgtacgtgcatggattggcttcgatgtcgaggggtgtcatgctactagagaagctgttggtaccaatttacctttacagctaggtttttctacaggtgttaacctagttgctgtacctacaggttatgttgatacacctaataatacagatttttccagagttagtgctaaaccaccgcctggagatcaatttaaacacctcataccacttatgtacaaaggacttccttggaatgtagtgcgtataaagattgtacaaatgttaagtgacacacttaaaaatctctctgacagagtcgtatttgtcttatgggcacatggctttgagttgacatctatgaagtattttgtgaaaataggacctgagcgcacctgttgtctatgtgatagacgtgccacatgcttttccactgcttcagacacttatgcctgttggcatcattctattggatttgattacgtctataatccgtttatgattgatgttcaacaatggggttttacaggtaacctacaaagcaaccatgatctgtattgtcaagtccatggtaatgcacatgtagctagttgtgatgcaatcatgactaggtgtctagctgtccacgagtgctttgttaagcgtgttgactggactattgaatatcctataattggtgatgaactgaagattaatgcggcttgtagaaaggttcaacacatggttgttaaagctgcattattagcagacaaattcccagttcttcacgacattggtaaccctaaagctattaagtgtgtacctcaagctgatgtagaatggaagttctatgatgcacagccttgtagtgacaaagcttataaaatagaagaattattctattcttatgccacacattctgacaaattcacagatggtgtatgcctattttggaattgcaatgtcgatagatatcctgctaattccattgtttgtagatttgacactagagtgctatctaaccttaacttgcctggttgtgatggtggcagtttgtatgtaaataaacatgcattccacacaccagcttttgataaaagtgcttttgttaatttaaaacaattaccatttttctattactctgacagtccatgtgagtctcatggaaaacaagtagtgtcagatatagattatgtaccactaaagtctgctacgtgtataacacgttgcaatttaggtggtgctgtctgtagacatcatgctaatgagtacagattgtatctcgatgcttataacatgatgatctcagctggctttagcttgtgggtttacaaacaatttgatacttataacctctggaacacttttacaagacttcagagtttagaaaatgtggcttttaatgttgtaaataagggacactttgatggacaacagggtgaagtaccagtttctatcattaataacactgtttacacaaaagttgatggtgttgatgtagaattgtttgaaaataaaacaacattacctgttaatgtagcatttgagctttgggctaagcgcaacattaaaccagtaccagaggtgaaaatactcaataatttgggtgtggacattgctgctaatactgtgatctgggactacaaaagagatgctccagcacatatatctactattggtgtttgttctatgactgacatagccaagaaaccaactgaaacgatttgtgcaccactcactgtcttttttgatggtagagttgatggtcaagtagacttatttagaaatgcccgtaatggtgttcttattacagaaggtagtgttaaaggtttacaaccatctgtgggtcccaaacaagctagtcttaatggagtcacattaattggagaagccgtaaaaacacagttcaattattataagaaagttgatggtgttgtccaacaattacctgaaacttactttactcagagtagaaatttacaagaatttaaacccaggagtcaaatggaaattgatttcttagaattagctatggatgaattcattgaacggtataaattagaaggctatgccttcgaacatatcgtttatggagattttagtcatagtcagttaggtggtttacatctactgattggactagctaaacgttttaaggaatcaccttttgaattagaagattttattcctatggacagtacagttaaaaactatttcataacagatgcgcaaacaggttcatctaagtgtgtgtgttctgttattgatttattacttgatgattttgttgaaataataaaatcccaagatttatctgtagtttctaaggttgtcaaagtgactattgactatacagaaatttcatttatgctttggtgtaaagatggccatgtagaaacattttacccaaaattacaatctagtcaagcgtggcaaccgggtgttgctatgcctaatctttacaaaatgcaaagaatgctattagaaaagtgtgaccttcaaaattatggtgatagtgcaacattacctaaaggcataatgatgaatgtcgcaaaatatactcaactgtgtcaatatttaaacacattaacattagctgtaccctataatatgagagttatacattttggtgctggttctgataaaggagttgcaccaggtacagctgttttaagacagtggttgcctacgggtacgctgcttgtcgattcagatcttaatgactttgtctctgatgcagattcaactttgattggtgattgtgcaactgtacatacagctaataaatgggatctcattattagtgatatgtacgaccctaagactaaaaatgttacaaaagaaaatgactctaaagagggttttttcacttacatttgtgggtttatacaacaaaagctagctcttggaggttccgtggctataaagataacagaacattcttggaatgctgatctttataagctcatgggacacttcgcatggtggacagcctttgttactaatgtgaatgcgtcatcatctgaagcatttttaattggatgtaattatcttggcaaaccacgcgaacaaatagatggttatgtcatgcatgcaaattacatattttggaggaatacaaatccaattcagttgtcttcctattctttatttgacatgagtaaatttccccttaaattaaggggtactgctgttatgtctttaaaagaaggtcaaatcaatgatatgattttatctcttcttagtaaaggtagacttataattagagaaaacaacagagttgttatttctagtgatgttcttgttaacaactaaacgaacaatgtttgtttttcttgttttattgccactagtctctagtcagtgtgttaatcttacaaccagaactcaattaccccctgcatacactaattctttcacacgtggtgtttattaccctgacaaagttttcagatcctcagttttacattcaactcaggacttgttcttacctttcttttccaatgttacttggttccatgctatacatgtctctgggaccaatggtactaagaggtttgataaccctgtcctaccatttaatgatggtgtttattttgcttccactgagaagtctaacataataagaggctggatttttggtactactttagattcgaagacccagtccctacttattgttaataacgctactaatgttgttattaaagtctgtgaatttcaattttgtaatgatccatttttgggtgtttattaccacaaaaacaacaaaagttggatggaaagtgagttcagagtttattctagtgcgaataattgcacttttgaatatgtctctcagccttttcttatggaccttgaaggaaaacagggtaatttcaaaaatcttagggaatttgtgtttaagaatattgatggttattttaaaatatattctaagcacacgcctattaatttagtgcgtgatctccctcagggtttttcggctttagaaccattggtagatttgccaataggtattaacatcactaggtttcaaactttacttgctttacatagaagttatttgactcctggtgattcttcttcaggttggacagctggtgctgcagcttattatgtgggttatcttcaacctaggacttttctattaaaatataatgaaaatggaaccattacagatgctgtagactgtgcacttgaccctctctcagaaacaaagtgtacgttgaaatccttcactgtagaaaaaggaatctatcaaacttctaactttagagtccaaccaacagaatctattgttagatttcctaatattacaaacttgtgcccttttggtgaagtttttaacgccaccagatttgcatctgtttatgcttggaacaggaagagaatcagcaactgtgttgctgattattctgtcctatataattccgcatcattttccacttttaagtgttatggagtgtctcctactaaattaaatgatctctgctttactaatgtctatgcagattcatttgtaattagaggtgatgaagtcagacaaatcgctccagggcaaactggaaagattgctgattataattataaattaccagatgattttacaggctgcgttatagcttggaattctaacaatcttgattctaaggttggtggtaattataattacctgtatagattgtttaggaagtctaatctcaaaccttttgagagagatatttcaactgaaatctatcaggccggtagcacaccttgtaatggtgttgaaggttttaattgttactttcctttacaatcatatggtttccaacccactaatggtgttggttaccaaccatacagagtagtagtactttcttttgaacttctacatgcaccagcaactgtttgtggacctaaaaagtctactaatttggttaaaaacaaatgtgtcaatttcaacttcaatggtttaacaggcacaggtgttcttactgagtctaacaaaaagtttctgcctttccaacaatttggcagagacattgctgacactactgatgctgtccgtgatccacagacacttgagattcttgacattacaccatgttcttttggtggtgtcagtgttataacaccaggaacaaatacttctaaccaggttgctgttctttatcaggatgttaactgcacagaagtccctgttgctattcatgcagatcaacttactcctacttggcgtgtttattctacaggttctaatgtttttcaaacacgtgcaggctgtttaataggggctgaacatgtcaacaactcatatgagtgtgacatacccattggtgcaggtatatgcgctagttatcagactcagactaattctcctcggcgggcacgtagtgtagctagtcaatccatcattgcctacactatgtcacttggtgcagaaaattcagttgcttactctaataactctattgccatacccacaaattttactattagtgttaccacagaaattctaccagtgtctatgaccaagacatcagtagattgtacaatgtacatttgtggtgattcaactgaatgcagcaatcttttgttgcaatatggcagtttttgtacacaattaaaccgtgctttaactggaatagctgttgaacaagacaaaaacacccaagaagtttttgcacaagtcaaacaaatttacaaaacaccaccaattaaagattttggtggttttaatttttcacaaatattaccagatccatcaaaaccaagcaagaggtcatttattgaagatctacttttcaacaaagtgacacttgcagatgctggcttcatcaaacaatatggtgattgccttggtgatattgctgctagagacctcatttgtgcacaaaagtttaacggccttactgttttgccacctttgctcacagatgaaatgattgctcaatacacttctgcactgttagcgggtacaatcacttctggttggacctttggtgcaggtgctgcattacaaataccatttgctatgcaaatggcttataggtttaatggtattggagttacacagaatgttctctatgagaaccaaaaattgattgccaaccaatttaatagtgctattggcaaaattcaagactcactttcttccacagcaagtgcacttggaaaacttcaagatgtggtcaaccaaaatgcacaagctttaaacacgcttgttaaacaacttagctccaattttggtgcaatttcaagtgttttaaatgatatcctttcacgtcttgacaaagttgaggctgaagtgcaaattgataggttgatcacaggcagacttcaaagtttgcagacatatgtgactcaacaattaattagagctgcagaaatcagagcttctgctaatcttgctgctactaaaatgtcagagtgtgtacttggacaatcaaaaagagttgatttttgtggaaagggctatcatcttatgtccttccctcagtcagcacctcatggtgtagtcttcttgcatgtgacttatgtccctgcacaagaaaagaacttcacaactgctcctgccatttgtcatgatggaaaagcacactttcctcgtgaaggtgtctttgtttcaaatggcacacactggtttgtaacacaaaggaatttttatgaaccacaaatcattactacagacaacacatttgtgtctggtaactgtgatgttgtaataggaattgtcaacaacacagtttatgatcctttgcaacctgaattagactcattcaaggaggagttagataaatattttaagaatcatacatcaccagatgttgatttaggtgacatctctggcattaatgcttcagttgtaaacattcaaaaagaaattgaccgcctcaatgaggttgccaagaatttaaatgaatctctcatcgatctccaagaacttggaaagtatgagcagtatataaaatggccatggtacatttggctaggttttatagctggcttgattgccatagtaatggtgacaattatgctttgctgtatgaccagttgctgtagttgtctcaagggctgttgttcttgtggatcctgctgcaaatttgatgaagacgactctgagccagtgctcaaaggagtcaaattacattacacataattcctgatcttctggtctaaacgaactaaatattatattagtttttctgtttggaactttaattttagccatggcagattccaacggtactattaccgttgaagagcttaaaaagctccttgaacaatggaacctagtaataggtttcctattccttacatggatttgtcttctacaatttgcctatgccaacaggaataggtttttgtatataattaagttaattttcctctggctgttatggccagtaactttagcttgttttgtgcttgctgctgtttacagaataaattggatcaccggtggaattgctatcgcaatggcttgtcttgtaggcttgatgtggctcagctacttcattgcttctttcagactgtttgcgcgtacccgttccatgtggtcattcaatccagaaactaacattcttctcaacgtgccactccatggcactattctgaccagaccgcttctagaaagtgaactcgtaatcggagctgtgatccttcgtggacatcttcgtattgctggacaccatctaggacgctgtgacatcaaggacctgcctaaagaaatcactgttgctacatcacgaacgctttcttattacaaattgggagcttcgcagcgtgtagcaggtgactcaggttttgctgcatacagtcgctacaggattggcaactataaattaaacacagaccattccagtagcagtgacaatattgctttgcttgtacagtaagtgacaacagatgtttcatctcgttgactttcaggttactatagcagagatattactaattattatgaggacttttaaagtttccatttggaatcttgattacatcataaacctcataattaaaaatttatctaagtcactaactgagaataaatattctcaattagatgaagagcaaccaatggagattgattaattgaactttcattaattgacttctatttgtgctttttagcctttctgctattccttgttttaattatgcttattatcttttggttctcacttgaactgcaagatcataatgaaacttgtcacgcctaaacgaacatgaaatttcttgttttcttaggaatcatcacaactgtagctgcatttcaccaagaatgtagtttacagtcatgtactcaacatcaaccatatgtagttgatgacccgtgtcctattcacttctattctaaatggtatattagagtaggagctagaaaatcagcacctttaattgaattgtgcgtggatgaggctggttctaaatcacccattcagtacatcgatatcggtaattatacagtttcctgtttaccttttacaattaattgccaggaacctaaattgggtagtcttgtagtgcgttgttcgttctatgaagactttttagagtatcatgacgttcgtgttgttttagatttcatctaaacgaacaaactaaaatgtctgataatggaccccaaaatcagcgaaatgcaccccgcattacgtttggtggaccctcagattcaactggcagtaaccagaatggagaacgcagtggggcgcgatcaaaacaacgtcggccccaaggtttacccaataatactgcgtcttggttcaccgctctcactcaacatggcaaggaagaccttaaattccctcgaggacaaggcgttccaattaacaccaatagcagtccagatgaccaaattggctactaccgaagagctaccagacgaattcgtggtggtgacggtaaaatgaaagatctcagtccaagatggtatttctactacctaggaactgggccagaagctggacttccctatggtgctaacaaagacggcatcatatgggttgcaactgagggagccttgaatacaccaaaagatcacattggcacccgcaatcctgctaacaatgctgcaatcgtgctacaacttcctcaaggaacaacattgccaaaaggcttctacgcagaagggagcagaggcggcagtcaagcctcttctcgttcctcatcacgtagtcgcaacagttcaagaaattcaactccaggcagcagtaggggaacttctcctgctagaatggctggcaatggcggtgatgctgctcttgctttgctgctgcttgacagattgaaccagcttgagagcaaaatgtctggtaaaggccaacaacaacaaggccaaactgtcactaagaaatctgctgctgaggcttctaagaagcctcggcaaaaacgtactgccactaaagcatacaatgtaacacaagctttcggcagacgtggtccagaacaaacccaaggaaattttggggaccaggaactaatcagacaaggaactgattacaaacattggccgcaaattgcacaatttgcccccagcgcttcagcgttcttcggaatgtcgcgcattggcatggaagtcacaccttcgggaacgtggttgacctacacagctgccatcaaattggatgacaaagatccaaatttcaaagatcaagtcattttgctgaataagcatattgacgcatacaaaacattcccaccaacagagcctaaaaaggacaaaaagaagaaggctgatgaaactcaagccttaccgcagagacagaagaaacagcaaactgtgactcttcttcctgctgcagatttggatgatttctccaaacaattgcaacaatccatgagcagtgctgactcaactcaggcctaaactcatgcagaccacacaaggcagatgggctatataaacgttttcgcttttccgtttacgatatatagtctactcttgtgcagaatgaattctcgtaactacatagcacaagtagatgtagttaactttaatctcacatagcaatctttaatcagtgtgtaacattagggaggacttgaaagagccaccacattttcaccgaggccacgcggagtacgatcgagtgtacagtgaacaatgctagggagagctgcctatatggaagagccctaatgtgtaaaattaattttagtagtgctatccccatgtgattttaatagcttcttaggagaatgac

SEQ ID NO: 49 - DNA, 28449 bp, Coronaviridae
  source 1..28449: mol_type = other DNA
  misc_feature 1..28449: note = SARS-CoV-2-[3,E,8] polynucleotide sequence
attaaaggtttataccttcccaggtaacaaaccaaccaactttcgatctcttgtagatctgttctctaaacgaactttaaaatctgtgtggctgtcactcggctgcatgcttagtgcactcacgcagtataattaataactaattactgtcgttgacaggacacgagtaactcgtctatcttctgcaggctgcttacggtttcgtccgtgttgcagccgatcatcagcacatctaggtttcgtccgggtgtgaccgaaaggtaagatggagagccttgtccctggtttcaacgagaaaacacacgtccaactcagtttgcctgttttacaggttcgcgacgtgctcgtacgtggctttggagactccgtggaggaggtcttatcagaggcacgtcaacatcttaaagatggcacttgtggcttagtagaagttgaaaaaggcgttttgcctcaacttgaacagccctatgtgttcatcaaacgttcggatgctcgaactgcacctcatggtcatgttatggttgagctggtagcagaactcgaaggcattcagtacggtcgtagtggtgagacacttggtgtccttgtccctcatgtgggcgaaataccagtggcttaccgcaaggttcttcttcgtaagaacggtaataaaggagctggtggccatagttacggcgccgatctaaagtcatttgacttaggcgacgagcttggcactgatccttatgaagattttcaagaaaactggaacactaaacatagcagtggtgttacccgtgaactcatgcgtgagcttaacggaggggcatacactcgctatgtcgataacaacttctgtggccctgatggctaccctcttgagtgcattaaagaccttctagcacgtgctggtaaagcttcatgcactttgtccgaacaactggactttattgacactaagaggggtgtatactgctgccgtgaacatgagcatgaaattgcttggtacacggaacgttctgaaaagagctatgaattgcagacaccttttgaaattaaattggcaaagaaatttgacaccttcaatggggaatgtccaaattttgtatttcccttaaattccataatcaagactattcaaccaagggttgaaaagaaaaagcttgatggctttatgggtagaattcgatctgtctatccagttgcgtcaccaaatgaatgcaaccaaatgtgcctttcaactctcatgaagtgtgatcattgtggtgaaacttcatggcagacgggcgattttgttaaagccacttgcgaattttgtggcactgagaatttgactaaagaaggtgccactacttgtggttacttaccccaaaatgctgttgttaaaatttattgtccagcatgtcacaattcagaagtaggacctgagcatagtcttgccgaataccataatgaatctggcttgaaaaccattcttcgtaagggtggtcgcactattgcctttggaggctgtgtgttctcttatgttggttgccataacaagtgtgcctattgggttccacgtgctagcgctaacataggttgtaaccatacaggtgttgttggagaaggttccgaaggtcttaatgacaaccttcttgaaatactccaaaaagagaaagtcaacatcaatattgttggtgactttaaacttaatgaagagatcgccattattttggcatctttttctgcttccacaagtgcttttgtggaaactgtgaaaggtttggattataaagcattcaaacaaattgttgaatcctgtggtaattttaaagttacaaaaggaaaagctaaaaaaggtgcctggaatattggtgaacagaaatcaatactgagtcctctttatgcatttgcatcagaggctgctcgtgttgtacgatcaattttctcccgcactcttgaaactgctcaaaattctgtgcgtgttttacagaaggccgctataacaatactagatggaatttcacagtattcactgagactcattgatgctatgatgttcacatctgatttggctactaacaatctagttgtaatggcctacattacaggtggtgttgttcagttgacttcgcagtggctaactaacatctttggcactgtttatgaaaaactcaaacccgtccttgattggcttgaagagaagtttaaggaaggtgtagagtttcttagagacggttgggaaattgttaaatttatctcaacctgtgcttgtgaaattgtcggtggacaaattgtcacctgtgcaaaggaaattaaggagagtgttcagacattctttaagcttgtaaataaatttttggctttgtgtgctgactctatcattattggtggagctaaacttaaagccttgaatttaggtgaaacatttgtcacgcactcaaagggattgtacagaaagtgtgttaaatccagagaagaaactggcctactcatgcctctaaaagccccaaaagaaattatcttcttagagggagaaacacttcccacagaagtgttaacagaggaagttgtcttgaaaactggtgatttacaaccattagaacaacctactagtgaagctgttgaagctccattggttggtacaccagtttgtattaacgggcttatgttgctcgaaatcaaagacacagaaaagtactgtgcccttgcacctaatatgatggtaacaaacaataccttcacactcaaaggcggtgcaccaacaaaggttacttttggtgatgacactgtgatagaagtgcaaggttacaagagtgtgaatatcacttttgaacttgatgaaaggattgataaagtacttaatgagaagtgctctgcctatacagttgaactcggtacagaagtaaatgagttcgcctgtgttgtggcagatgctgtcataaaaactttgcaaccagtatctgaattacttacaccactgggcattgatttagatgagtggagtatggctacatactacttatttgatgagtctggtgagtttaaattggcttcacatatgtattgttctttctaccctccagatgaggatgaagaagaaggtgattgtgaagaagaagagtttgagccatcaactcaatatgagtatggtactgaagatgattaccaaggtaaacctttggaatttggtgccacttctgctgctcttcaacctgaagaagagcaagaagaagattggttagatgatgatagtcaacaaactgttggtcaacaagacggcagtgaggacaatcagacaactactattcaaacaattgttgaggttcaacctcaattagagatggaacttacaccagttgttcagactattgaagtgaatagttttagtggttatttaaaacttactgacaatgtatacattaaaaatgcagacattgtggaagaagctaaaaaggtaaaaccaacagtggttgttaatgcagccaatgtttaccttaaacatggaggaggtgttgcaggagccttaaataaggctactaacaatgccatgcaagttgaatctgatgattacatagctactaatggaccacttaaagtgggtggtagttgtgttttaagcggacacaatcttgctaaacactgtcttcatgttgtcggcccaaatgttaacaaaggtgaagacattcaacttcttaagagtgcttatgaaaattttaatcagcacgaagttctacttgcaccattattatcagctggtatttttggtgctgaccctatacattctttaagagtttgtgtagatactgttcgcacaaatgtctacttagctgtctttgataaaaatctctatgacaaacttgtttcaagctttttggaaatgaagagtgaaaagcaagttgaacaaaagatcgctgagattcctaaagaggaagttaagccatttataactgaaagtaaaccttcagttgaacagagaaaacaagatgataagaaaatcaaagcttgtgttgaagaagttacaacaactctggaagaaactaagttcctcacagaaaacttgttactttatattgacattaatggcaatcttcatccagattctgccactcttgttagtgacattgacatcactttcttaaagaaagatgctccatatatagtgggtgatgttgttcaagagggtgttttaactgctgtggttatacctactaaaaaggctggtggcactactgaaatgctagcgaaagctttgagaaaagtgccaacagacaattatataaccacttacccgggtcagggtttaaatggttacactgtagaggaggcaaagacagtgcttaaaaagtgtaaaagtgccttttacattctaccatctattatctctaatgagaagcaagaaattcttggaactgtttcttggaatttgcgagaaatgcttgcacatgcagaagaaacacgcaaattaatgcctgtctgtgtggaaactaaagccatagtttcaactatacagcgtaaatataagggtattaaaatacaagagggtgtggttgattatggtgctagattttacttttacaccagtaaaacaactgtagcgtcacttatcaacacacttaacgatctaaatgaaactcttgttacaatgccacttggctatgtaacacatggcttaaatttggaagaagctgctcggtatatgagatctctcaaagtgccagctacagtttctgtttcttcacctgatgctgttacagcgtataatggttatcttacttcttcttctaaaacacctgaagaacattttattgaaaccatctcacttgctggttcctataaagattggtcctattctggacaatctacacaactaggtatagaatttcttaagagaggtgataaaagtgtatattacactagtaatcctaccacattccacctagatggtgaagttatcacctttgacaatcttaagacacttctttctttgagagaagtgaggactattaaggtgtttacaacagtagacaacattaacctccacacgcaagttgtggacatgtcaatgacatatggacaacagtttggtccaacttatttggatggagctgatgttactaaaataaaacctcataattcacatgaaggtaaaacattttatgttttacctaatgatgacactctacgtgttgaggcttttgagtactaccacacaactgatcctagttttctgggtaggtacatgtcagcattaaatcacactaaaaagtggaaatacccacaagttaatggtttaacttctattaaatgggcagataacaactgttatcttgccactgcattgttaacactccaacaaatagagttgaagtttaatccacctgctctacaagatgcttattacagagcaagggctggtgaagctgctaacttttgtgcacttatcttagcctactgtaataagacagtaggtgagttaggtgatgttagagaaacaatgagttacttgtttcaacatgccaatttagattcttgcaaaagagtcttgaacgtggtgtgtaaaacttgtggacaacagcagacaacccttaagggtgtagaagctgttatgtacatgggcacactttcttatgaacaatttaagaaaggtgttcagataccttgtacgtgtggtaaacaagctacaaaatatctagtacaacaggagtcaccttttgttatgatgtcagcaccacctgctcagtatgaacttaagcatggtacatttacttgtgctagtgagtacactggtaattaccagtgtggtcactataaacatataacttctaaagaaactttgtattgcatagacggtgctttacttacaaagtcctcagaatacaaaggtcctattacggatgttttctacaaagaaaacagttacacaacaaccataaaaccagttacttataaattggatggtgttgtttgtacagaaattgaccctaagttggacaattattataagaaagacaattcttatttcacagagcaaccaattgatcttgtaccaaaccaaccatatccaaacgcaagcttcgataattttaagtttgtatgtgataatatcaaatttgctgatgatttaaaccagttaactggttataagaaacctgcttcaagagagcttaaagttacatttttccctgacttaaatggtgatgtggtggctattgattataaacactacacaccctcttttaagaaaggagctaaattgttacataaacctattgtttggcatgttaacaatgcaactaataaagccacgtataaaccaaatacctggtgtatacgttgtctttggagcacaaaaccagttgaaacatcaaattcgtttgatgtactgaagtcagaggacgcgcagggaatggataatcttgcctgcgaagatctaaaaccagtctctgaagaagtagtggaaaatcctaccatacagaaagacgttcttgagtgtaatgtgaaaactaccgaagttgtaggagacattatacttaaaccagcaaataatagtttaaaaattacagaagaggttggccacacagatctaatggctgcttatgtagacaattctagtcttactattaagaaacctaatgaattatctagagtattaggtttgaaaacccttgctactcatggtttagctgctgttaatagtgtcccttgggatactatagctaattatgctaagccttttcttaacaaagttgttagtacaactactaacatagttacacggtgtttaaaccgtgtttgtactaattatatgccttatttctttactttattgctacaattgtgtacttttactagaagtacaaattctagaattaaagcatctatgccgactactatagcaaagaatactgttaagagtgtcggtaaattttgtctagaggcttcatttaattatttgaagtcacctaatttttctaaactgataaatattataatttggtttttactattaagtgtttgcctaggttctttaatctactcaaccgctgctttaggtgttttaatgtctaatttaggcatgccttcttactgtactggttacagagaaggctatttgaactctactaatgtcactattgcaacctactgtactggttctataccttgtagtgtttgtcttagtggtttagattctttagacacctatccttctttagaaactatacaaattaccatttcatcttttaaatgggatttaactgcttttggcttagttgcagagtggtttttggcatatattcttttcactaggtttttctatgtacttggattggctgcaatcatgcaattgtttttcagctattttgcagtacattttattagtaattcttggcttatgtggttaataattaatcttgtacaaatggccccgatttcagctatggttagaatgtacatcttctttgcatcattttattatgtatggaaaagttatgtgcatgttgtagacggttgtaattcatcaacttgtatgatgtgttacaaacgtaatagagcaacaagagtcgaatgtacaactattgttaatggtgttagaaggtccttttatgtctatgctaatggaggtaaaggcttttgcaaactacacaattggaattgtgttaattgtgatacattctgtgctggtagtacatttattagtgatgaagttgcgagagacttgtcactacagtttaaaagaccaataaatcctactgaccagtcttcttacatcgttgatagtgttacagtgaagaatggttccatccatctttactttgataaagctggtcaaaagacttatgaaagacattctctctctcattttgttaacttagacaacctgagagctaataacactaaaggttcattgcctattaatgttatagtttttgatggtaaatcaaaatgtgaagaatcatctgcaaaatcagcgtctgtttactacagtcagcttatgtgtcaacctatactgttactagatcaggcattagtgtctgatgttggtgatagtgcggaagttgcagttaaaatgtttgatgcttacgttaatacgttttcatcaacttttaacgtaccaatggaaaaactcaaaacactagttgcaactgcagaagctgaacttgcaaagaatgtgtccttagacaatgtcttatctacttttatttcagcagctcggcaagggtttgttgattcagatgtagaaactaaagatgttgttgaatgtcttaaattgtcacatcaatctgacatagaagttactggcgatagttgtaataactatatgctcacctataacaaagttgaaaacatgacaccccgtgaccttggtgcttgtattgactgtagtgcgcgtcatattaatgcgcaggtagcaaaaagtcacaacattgctttgatatggaacgttaaagatttcatgtcattgtctgaacaactacgaaaacaaatacgtagtgctgctaaaaagaataacttaccttttaagttgacatgtgcaactactagacaagttgttaatgttgtaacaacaaagatagcacttaagggtggtaaaattgttaataattggttgaagcagttaattaaagttacacttgtgttcctttttgttgctgctattttctatttaataacacctgttcatgtcatgtctaaacatactgacttttcaagtgaaatcataggatacaaggctattgatggtggtgtcactcgtgacatagcatctacagatacttgttttgctaacaaacatgctgattttgacacatggtttagccagcgtggtggtagttatactaatgacaaagcttgcccattgattgctgcagtcataacaagagaagtgggttttgtcgtgcctggtttgcctggcacgatattacgcacaactaatggtgactttttgcatttcttacctagagtttttagtgcagttggtaacatctgttacacaccatcaaaacttatagagtacactgactttgcaacatcagcttgtgttttggctgctgaatgtacaatttttaaagatgcttctggtaagccagtaccatattgttatgataccaatgtactagaaggttctgttgcttatgaaagtttacgccctgacacacgttatgtgctcatggatggctctattattcaatttcctaacacctaccttgaaggttctgttagagtggtaacaacttttgattctgagtactgtaggcacggcacttgtgaaagatcagaagctggtgtttgtgtatctactagtggtagatgggtacttaacaatgattattacagatctttaccaggagttttctgtggtgtagatgctgtaaatttacttactaatatgtttacaccactaattcaacctattggtgctttggacatatcagcatctatagtagctggtggtattgtagctatcgtagtaacatgccttgcctactattttatgaggtttagaagagcttttggtgaatacagtcatgtagttgcctttaatactttactattccttatgtcattcactgtactctgtttaacaccagtttactcattcttacctggtgtttattctgttatttacttgtacttgacattttatcttactaatgatgtttcttttttagcacatattcagtggatggttatgttcacacctttagtacctttctggataacaattgcttatatcatttgtatttccacaaagcatttctattggttctttagtaattacctaaagagacgtgtagtctttaatggtgtttcctttagtacttttgaagaagctgcgctgtgcacctttttgttaaataaagaaatgtatctaaagttgcgtagtgatgtgctattacctcttacgcaatataatagatacttagctctttataataagtacaagtattttagtggagcaatggatacaactagctacagagaagctgcttgttgtcatctcgcaaaggctctcaatgacttcagtaactcaggttctgatgttctttaccaaccaccacaaacctctatcacctcagctgttttgcagagtggttttagaaaaatggcattcccatctggtaaagttgagggttgtatggtacaagtaacttgtggtacaactacacttaacggtctttggcttgatgacgtagtttactgtccaagacatgtgatctgcacctctgaagacatgcttaaccctaattatgaagatttactcattcgtaagtctaatcataatttcttggtacaggctggtaatgttcaactcagggttattggacattctatgcaaaattgtgtacttaagcttaaggttgatacagccaatcctaagacacctaagtataagtttgttcgcattcaaccaggacagactttttcagtgttagcttgttacaatggttcaccatctggtgtttaccaatgtgctatgaggcccaatttcactattaagggttcattccttaatggttcatgtggtagtgttggttttaacatagattatgactgtgtctctttttgttacatgcaccatatggaattaccaactggagttcatgctggcacagacttagaaggtaacttttatggaccttttgttgacaggcaaacagcacaagcagctggtacggacacaactattacagttaatgttttagcttggttgtacgctgctgttataaatggagacaggtggtttctcaatcgatttaccacaactcttaatgactttaaccttgtggctatgaagtacaattatgaacctctaacacaagaccatgttgacatactaggacctctttctgctcaaactggaattgccgttttagatatgtgtgcttcattaaaagaattactgcaaaatggtatgaatggacgtaccatattgggtagtgctttattagaagatgaatttacaccttttgatgttgttagacaatgctcaggtgttactttccaaagtgcagtgaaaagaacaatcaagggtacacaccactggttgttactcacaattttgacttcacttttagttttagtccagagtactcaatggtctttgttcttttttttgtatgaaaatgcctttttaccttttgctatgggtattattgctatgtctgcttttgcaatgatgtttgtcaaacataagcatgcatttctctgtttgtttttgttaccttctcttgccactgtagcttattttaatatggtctatatgcctgctagttgggtgatgcgtattatgacatggttggatatggttgatactagtttgtctggttttaagctaaaagactgtgttatgtatgcatcagctgtagtgttactaatccttatgacagcaagaactgtgtatgatgatggtgctaggagagtgtggacacttatgaatgtcttgacactcgtttataaagtttattatggtaatgctttagatcaagccatttccatgtgggctcttataatctctgttacttctaactactcaggtgtagttacaactgtcatgtttttggccagaggtattgtttttatgtgtgttgagtattgccctattttcttcataactggtaatacacttcagtgtataatgctagtttattgtttcttaggctatttttgtacttgttactttggcctcttttgtttactcaaccgctactttagactgactcttggtgtttatgattacttagtttctacacaggagtttagatatatgaattcacagggactactcccacccaagaatagcatagatgccttcaaactcaacattaaattgttgggtgttggtggcaaaccttgtatcaaagtagccactgtacagtctaaaatgtcagatgtaaagtgcacatcagtagtcttactctcagttttgcaacaactcagagtagaatcatcatctaaattgtgggctcaatgtgtccagttacacaatgacattctcttagctaaagatactactgaagcctttgaaaaaatggtttcactactttctgttttgctttccatgcagggtgctgtagacataaacaagctttgtgaagaaatgctggacaacagggcaaccttacaagctatagcctcagagtttagttcccttccatcatatgcagcttttgctactgctcaagaagcttatgagcaggctgttgctaatggtgattctgaagttgttcttaaaaagttgaagaagtctttgaatgtggctaaatctgaatttgaccgtgatgcagccatgcaacgtaagttggaaaagatggctgatcaagctatgacccaaatgtataaacaggctagatctgaggacaagagggcaaaagttactagtgctatgcagacaatgcttttcactatgcttagaaagttggataatgatgcactcaacaacattatcaacaatgcaagagatggttgtgttcccttgaacataatacctcttacaacagcagccaaactaatggttgtcataccagactataacacatataaaaatacgtgtgatggtacaacatttacttatgcatcagcattgtgggaaatccaacaggttgtagatgcagatagtaaaattgttcaacttagtgaaattagtatggacaattcacctaatttagcatggcctcttattgtaacagctttaagggccaattctgctgtcaaattacagaataatgagcttagtcctgttgcactacgacagatgtcttgtgctgccggtactacacaaactgcttgcactgatgacaatgcgttagcttactacaacacaacaaagggaggtaggtttgtacttgcactgttatccgatttacaggatttgaaatgggctagattccctaagagtgatggaactggtactatctatacagaactggaaccaccttgtaggtttgttacagacacacctaaaggtcctaaagtgaagtatttatactttattaaaggattaaacaacctaaatagaggtatggtacttggtagtttagctgccacagtacgtctacaagctggtaatgcaacagaagtgcctgccaattcaactgtattatctttctgtgcttttgctgtagatgctgctaaagcttacaaagattatctagctagtgggggacaaccaatcactaattgtgttaagatgttgtgtacacacactggtactggtcaggcaataacagttacaccggaagccaatatggatcaagaatcctttggtggtgcatcgtgttgtctgtactgccgttgccacatagatcatccaaatcctaaaggattttgtgacttaaaaggtaagtatgtacaaatacctacaacttgtgctaatgaccctgtgggttttacacttaaaaacacagtctgtaccgtctgcggtatgtggaaaggttatggctgtagttgtgatcaactccgcgaacccatgcttcagtcagctgatgcacaatcgtttttaaacgggtttgcggtgtaagtgcagcccgtcttacaccgtgcggcacaggcactagtactgatgtcgtatacagggcttttgacatctacaatgataaagtagctggttttgctaaattcctaaaaactaattgttgtcgcttccaagaaaaggacgaagatgacaatttaattgattcttactttgtagttaagagacacactttctctaactaccaacatgaagaaacaatttataatttacttaaggattgtccagctgttgctaaacatgacttctttaagtttagaatagacggtgacatggtaccacatatatcacgtcaacgtcttactaaatacacaatggcagacctcgtctatgctttaaggcattttgatgaaggtaattgtgacacattaaaagaaatacttgtcacatacaattgttgtgatgatgattatttcaataaaaaggactggtatgattttgtagaaaacccagatatattacgcgtatacgccaacttaggtgaacgtgtacgccaagctttgttaaaaacagtacaattctgtgatgccatgcgaaatgctggtattgttggtgtactgacattagataatcaagatctcaatggtaactggtatgatttcggtgatttcatacaaaccacgccaggtagtggagttcctgttgtagattcttattattcattgttaatgcctatattaaccttgaccagggctttaactgcagagtcacatgttgacactgacttaacaaagccttacattaagtgggatttgttaaaatatgacttcacggaagagaggttaaaactctttgaccgttattttaaatattgggatcagacataccacccaaattgtgttaactgtttggatgacagatgcattctgcattgtgcaaactttaatgttttattctctacagtgttcccacctacaagttttggaccactagtgagaaaaatatttgttgatggtgttccatttgtagtttcaactggataccacttcagagagctaggtgttgtacataatcaggatgtaaacttacatagctctagacttagttttaaggaattacttgtgtatgctgctgaccctgctatgcacgctgcttctggtaatctattactagataaacgcactacgtgcttttcagtagctgcacttactaacaatgttgcttttcaaactgtcaaacccggtaattttaacaaagacttctatgactttgctgtgtctaagggtttctttaaggaaggaagttctgttgaattaaaacacttcttctttgctcaggatggtaatgctgctatcagcgattatgactactatcgttataatctaccaacaatgtgtgatatcagacaactactatttgtagttgaagttgttgataagtactttgattgttacgatggtggctgtattaatgctaaccaagtcatcgtcaacaacctagacaaatcagctggttttccatttaataaatggggtaaggctagactttattatgattcaatgagttatgaggatcaagatgcacttttcgcatatacaaaacgtaatgtcatccctactataactcaaatgaatcttaagtatgccattagtgcaaagaatagagctcgcaccgtagctggtgtctctatctgtagtactatgaccaatagacagtttcatcaaaaattattgaaatcaatagccgccactagaggagctactgtagtaattggaacaagcaaattctatggtggttggcacaacatgttaaaaactgtttatagtgatgtagaaaaccctcaccttatgggttgggattatcctaaatgtgatagagccatgcctaacatgcttagaattatggcctcacttgttcttgctcgcaaacatacaacgtgttgtagcttgtcacaccgtttctatagattagctaatgagtgtgctcaagtattgagtgaaatggtcatgtgtggcggttcactatatgttaaaccaggtggaacctcatcaggagatgccacaactgcttatgctaatagtgtttttaacatttgtcaagctgtcacggccaatgttaatgcacttttatctactgatggtaacaaaattgccgataagtatgtccgcaatttacaacacagactttatgagtgtctctatagaaatagagatgttgacacagactttgtgaatgagttttacgcatatttgcgtaaacatttctcaatgatgatactctctgacgatgctgttgtgtgtttcaatagcacttatgcatctcaaggtctagtggctagcataaagaactttaagtcagttctttattatcaaaacaatgtttttatgtctgaagcaaaatgttggactgagactgaccttactaaaggacctcatgaattttgctctcaacatacaatgctagttaaacagggtgatgattatgtgtaccttccttacccagatccatcaagaatcctaggggccggctgttttgtagatgatatcgtaaaaacagatggtacacttatgattgaacggttcgtgtctttagctatagatgcttacccacttactaaacatcctaatcaggagtatgctgatgtctttcatttgtacttacaatacataagaaagctacatgatgagttaacaggacacatgttagacatgtattctgttatgcttactaatgataacacttcaaggtattgggaacctgagttttatgaggctatgtacacaccgcatacagtcttacaggctgttggggcttgtgttctttgcaattcacagacttcattaagatgtggtgcttgcatacgtagaccattcttatgttgtaaatgctgttacgaccatgtcatatcaacatcacataaattagtcttgtctgttaatccgtatgtttgcaatgctccaggttgtgatgtcacagatgtgactcaactttacttaggaggtatgagctattattgtaaatcacataaaccacccattagttttccattgtgtgctaatggacaagtttttggtttatataaaaatacatgtgttggtagcgataatgttactgactttaatgcaattgcaacatgtgactggacaaatgctggtgattacattttagctaacacctgtactgaaagactcaagctttttgcagcagaaacgctcaaagctactgaggagacatttaaactgtcttatggtattgctactgtacgtgaagtgctgtctgacagagaattacatctttcatgggaagttggtaaacctagaccaccacttaaccgaaattatgtctttactggttatcgtgtaactaaaaacagtaaagtacaaataggagagtacacctttgaaaaaggtgactatggtgatgctgttgtttaccgaggtacaacaacttacaaattaaatgttggtgattattttgtgctgacatcacatacagtaatgccattaagtgcacctacactagtgccacaagagcactatgttagaattactggcttatacccaacactcaatatctcagatgagttttctagcaatgttgcaaattatcaaaaggttggtatgcaaaagtattctacactccagggaccacctggtactggtaagagtcattttgctattggcctagctctctactacccttctgctcgcatagtgtatacagcttgctctcatgccgctgttgatgcactatgtgagaaggcattaaaatatttgcctatagataaatgtagtagaattatacctgcacgtgctcgtgtagagtgttttgataaattcaaagtgaattcaacattagaacagtatgtcttttgtactgtaaatgcattgcctgagacgacagcagatatagttgtctttgatgaaatttcaatggccacaaattatgatttgagtgttgtcaatgccagattacgtgctaagcactatgtgtacattggcgaccctgctcaattacctgcaccacgcacattgctaactaagggcacactagaaccagaatatttcaattcagtgtgtagacttatgaaaactataggtccagacatgttcctcggaacttgtcggcgttgtcctgctgaaattgttgacactgtgagtgctttggtttatgataataagcttaaagcacataaagacaaatcagctcaatgctttaaaatgttttataagggtgttatcacgcatgatgtttcatctgcaattaacaggccacaaataggcgtggtaagagaattccttacacgtaaccctgcttggagaaaagctgtctttatttcaccttataattcacagaatgctgtagcctcaaagattttgggactaccaactcaaactgttgattcatcacagggctcagaatatgactatgtcatattcactcaaaccactgaaacagctcactcttgtaatgtaaacagatttaatgttgctattaccagagcaaaagtaggcatactttgcataatgtctgatagagacctttatgacaagttgcaatttacaagtcttgaaattccacgtaggaatgtggcaactttacaagctgaaaatgtaacaggactctttaaagattgtagtaaggtaatcactgggttacatcctacacaggcacctacacacctcagtgttgacactaaattcaaaactgaaggtttatgtgttgacatacctggcatacctaaggacatgacctatagaagactcatctctatgatgggttttaaaatgaattatcaagttaatggttaccctaacatgtttatcacccgcgaagaagctataagacatgtacgtgcatggattggcttcgatgtcgaggggtgtcatgctactagagaagctgttggtaccaatttacctttacagctaggtttttctacaggtgttaacctagttgctgtacctacaggttatgttgatacacctaataatacagatttttccagagttagtgctaaaccaccgcctggagatcaatttaaacacctcataccacttatgtacaaaggacttccttggaatgtagtgcgtataaagattgtacaaatgttaagtgacacacttaaaaatctctctgacagagtcgtatttgtcttatgggcacatggctttgagttgacatctatgaagtattttgtgaaaataggacctgagcgcacctgttgtctatgtgatagacgtgccacatgcttttccactgcttcagacacttatgcctgttggcatcattctattggatttgattacgtctataatccgtttatgattgatgttcaacaatggggttttacaggtaacctacaaagcaaccatgatctgtattgtcaagtccatggtaatgcacatgtagctagttgtgatgcaatcatgactaggtgtctagctgtccacgagtgctttgttaagcgtgttgactggactattgaatatcctataattggtgatgaactgaagattaatgcggcttgtagaaaggttcaacacatggttgttaaagctgcattattagcagacaaattcccagttcttcacgacattggtaaccctaaagctattaagtgtgtacctcaagctgatgtagaatggaagttctatgatgcacagccttgtagtgacaaagcttataaaatagaagaattattctattcttatgccacacattctgacaaattcacagatggtgtatgcctattttggaattgcaatgtcgatagatatcctgctaattccattgtttgtagatttgacactagagtgctatctaaccttaacttgcctggttgtgatggtggcagtttgtatgtaaataaacatgcattccacacaccagcttttgataaaagtgcttttgttaatttaaaacaattaccatttttctattactctgacagtccatgtgagtctcatggaaaacaagtagtgtcagatatagattatgtaccactaaagtctgctacgtgtataacacgttgcaatttaggtggtgctgtctgtagacatcatgctaatgagtacagattgtatctcgatgcttataacatgatgatctcagctggctttagcttgtgggtttacaaacaatttgatacttataacctctggaacacttttacaagacttcagagtttagaaaatgtggcttttaatgttgtaaataagggacactttgatggacaacagggtgaagtaccagtttctatcattaataacactgtttacacaaaagttgatggtgttgatgtagaattgtttgaaaataaaacaacattacctgttaatgtagcatttgagctttgggctaagcgcaacattaaaccagtaccagaggtgaaaatactcaataatttgggtgtggacattgctgctaatactgtgatctgggactacaaaagagatgctccagcacatatatctactattggtgtttgttctatgactgacatagccaagaaaccaactgaaacgatttgtgcaccactcactgtcttttttgatggtagagttgatggtcaagtagacttatttagaaatgcccgtaatggtgttcttattacagaaggtagtgttaaaggtttacaaccatctgtgggtcccaaacaagctagtcttaatggagtcacattaattggagaagccgtaaaaacacagttcaattattataagaaagttgatggtgttgtccaacaattacctgaaacttactttactcagagtagaaatttacaagaatttaaacccaggagtcaaatggaaattgatttcttagaattagctatggatgaattcattgaacggtataaattagaaggctatgccttcgaacatatcgtttatggagattttagtcatagtcagttaggtggtttacatctactgattggactagctaaacgttttaaggaatcaccttttgaattagaagattttattcctatggacagtacagttaaaaactatttcataacagatgcgcaaacaggttcatctaagtgtgtgtgttctgttattgatttattacttgatgattttgttgaaataataaaatcccaagatttatctgtagtttctaaggttgtcaaagtgactattgactatacagaaatttcatttatgctttggtgtaaagatggccatgtagaaacattttacccaaaattacaatctagtcaagcgtggcaaccgggtgttgctatgcctaatctttacaaaatgcaaagaatgctattagaaaagtgtgaccttcaaaattatggtgatagtgcaacattacctaaaggcataatgatgaatgtcgcaaaatatactcaactgtgtcaatatttaaacacattaacattagctgtaccctataatatgagagttatacattttggtgctggttctgataaaggagttgcaccaggtacagctgttttaagacagtggttgcctacgggtacgctgcttgtcgattcagatcttaatgactttgtctctgatgcagattcaactttgattggtgattgtgcaactgtacatacagctaataaatgggatctcattattagtgatatgtacgaccctaagactaaaaatgttacaaaagaaaatgactctaaagagggttttttcacttacatttgtgggtttatacaacaaaagctagctcttggaggttccgtggctataaagataacagaacattcttggaatgctgatctttataagctcatgggacacttcgcatggtggacagcctttgttactaatgtgaatgcgtcatcatctgaagcatttttaattggatgtaattatcttggcaaaccacgcgaacaaatagatggttatgtcatgcatgcaaattacatattttggaggaatacaaatccaattcagttgtcttcctattctttatttgacatgagtaaatttccccttaaattaaggggtactgctgttatgtctttaaaagaaggtcaaatcaatgatatgattttatctcttcttagtaaaggtagacttataattagagaaaacaacagagttgttatttctagtgatgttcttgttaacaactaaacgaacaatgtttgtttttcttgttttattgccactagtctctagtcagtgtgttaatcttacaaccagaactcaattaccccctgcatacactaattctttcacacgtggtgtttattaccctgacaaagttttcagatcctcagttttacattcaactcaggacttgttcttacctttcttttccaatgttacttggttccatgctatacatgtctctgggaccaatggtactaagaggtttgataaccctgtcctaccatttaatgatggtgtttattttgcttccactgagaagtctaacataataagaggctggatttttggtactactttagattcgaagacccagtccctacttattgttaataacgctactaatgttgttattaaagtctgtgaatttcaattttgtaatgatccatttttgggtgtttattaccacaaaaacaacaaaagttggatggaaagtgagttcagagtttattctagtgcgaataattgcacttttgaatatgtctctcagccttttcttatggaccttgaaggaaaacagggtaatttcaaaaatcttagggaatttgtgtttaagaatattgatggttattttaaaatatattctaagcacacgcctattaatttagtgcgtgatctccctcagggtttttcggctttagaaccattggtagatttgccaataggtattaacatcactaggtttcaaactttacttgctttacatagaagttatttgactcctggtgattcttcttcaggttggacagctggtgctgcagcttattatgtgggttatcttcaacctaggacttttctattaaaatataatgaaaatggaaccattacagatgctgtagactgtgcacttgaccctctctcagaaacaaagtgtacgttgaaatccttcactgtagaaaaaggaatctatcaaacttctaactttagagtccaaccaacagaatctattgttagatttcctaatattacaaacttgtgcccttttggtgaagtttttaacgccaccagatttgcatctgtttatgcttggaacaggaagagaatcagcaactgtgttgctgattattctgtcctatataattccgcatcattttccacttttaagtgttatggagtgtctcctactaaattaaatgatctctgctttactaatgtctatgcagattcatttgtaattagaggtgatgaagtcagacaaatcgctccagggcaaactggaaagattgctgattataattataaattaccagatgattttacaggctgcgttatagcttggaattctaacaatcttgattctaaggttggtggtaattataattacctgtatagattgtttaggaagtctaatctcaaaccttttgagagagatatttcaactgaaatctatcaggccggtagcacaccttgtaatggtgttgaaggttttaattgttactttcctttacaatcatatggtttccaacccactaatggtgttggttaccaaccatacagagtagtagtactttcttttgaacttctacatgcaccagcaactgtttgtggacctaaaaagtctactaatttggttaaaaacaaatgtgtcaatttcaacttcaatggtttaacaggcacaggtgttcttactgagtctaacaaaaagtttctgcctttccaacaatttggcagagacattgctgacactactgatgctgtccgtgatccacagacacttgagattcttgacattacaccatgttcttttggtggtgtcagtgttataacaccaggaacaaatacttctaaccaggttgctgttctttatcaggatgttaactgcacagaagtccctgttgctattcatgcagatcaacttactcctacttggcgtgtttattctacaggttctaatgtttttcaaacacgtgcaggctgtttaataggggctgaacatgtcaacaactcatatgagtgtgacatacccattggtgcaggtatatgcgctagttatcagactcagactaattctcctcggcgggcacgtagtgtagctagtcaatccatcattgcctacactatgtcacttggtgcagaaaattcagttgcttactctaataactctattgccatacccacaaattttactattagtgttaccacagaaattctaccagtgtctatgaccaagacatcagtagattgtacaatgtacatttgtggtgattcaactgaatgcagcaatcttttgttgcaatatggcagtttttgtacacaattaaaccgtgctttaactggaatagctgttgaacaagacaaaaacacccaagaagtttttgcacaagtcaaacaaatttacaaaacaccaccaattaaagattttggtggttttaatttttcacaaatattaccagatccatcaaaaccaagcaagaggtcatttattgaagatctacttttcaacaaagtgacacttgcagatgctggcttcatcaaacaatatggtgattgccttggtgatattgctgctagagacctcatttgtgcacaaaagtttaacggccttactgttttgccacctttgctcacagatgaaatgattgctcaatacacttctgcactgttagcgggtacaatcacttctggttggacctttggtgcaggtgctgcattacaaataccatttgctatgcaaatggcttataggtttaatggtattggagttacacagaatgttctctatgagaaccaaaaattgattgccaaccaatttaatagtgctattggcaaaattcaagactcactttcttccacagcaagtgcacttggaaaacttcaagatgtggtcaaccaaaatgcacaagctttaaacacgcttgttaaacaacttagctccaattttggtgcaatttcaagtgttttaaatgatatcctttcacgtcttgacaaagttgaggctgaagtgcaaattgataggttgatcacaggcagacttcaaagtttgcagacatatgtgactcaacaattaattagagctgcagaaatcagagcttctgctaatcttgctgctactaaaatgtcagagtgtgtacttggacaatcaaaaagagttgatttttgtggaaagggctatcatcttatgtccttccctcagtcagcacctcatggtgtagtcttcttgcatgtgacttatgtccctgcacaagaaaagaacttcacaactgctcctgccatttgtcatgatggaaaagcacactttcctcgtgaaggtgtctttgtttcaaatggcacacactggtttgtaacacaaaggaatttttatgaaccacaaatcattactacagacaacacatttgtgtctggtaactgtgatgttgtaataggaattgtcaacaacacagtttatgatcctttgcaacctgaattagactcattcaaggaggagttagataaatattttaagaatcatacatcaccagatgttgatttaggtgacatctctggcattaatgcttcagttgtaaacattcaaaaagaaattgaccgcctcaatgaggttgccaagaatttaaatgaatctctcatcgatctccaagaacttggaaagtatgagcagtatataaaatggccatggtacatttggctaggttttatagctggcttgattgccatagtaatggtgacaattatgctttgctgtatgaccagttgctgtagttgtctcaagggctgttgttcttgtggatcctgctgcaaatttgatgaagacgactctgagccagtgctcaaaggagtcaaattacattacacataattcctgatcttctggtctaaacgaactaaatattatattagtttttctgtttggaactttaattttagccatggcagattccaacggtactattaccgttgaagagcttaaaaagctccttgaacaatggaacctagtaataggtttcctattccttacatggatttgtcttctacaatttgcctatgccaacaggaataggtttttgtatataattaagttaattttcctctggctgttatggccagtaactttagcttgttttgtgcttgctgctgtttacagaataaattggatcaccggtggaattgctatcgcaatggcttgtcttgtaggcttgatgtggctcagctacttcattgcttctttcagactgtttgcgcgtacccgttccatgtggtcattcaatccagaaactaacattcttctcaacgtgccactccatggcactattctgaccagaccgcttctagaaagtgaactcgtaatcggagctgtgatccttcgtggacatcttcgtattgctggacaccatctaggacgctgtgacatcaaggacctgcctaaagaaatcactgttgctacatcacgaacgctttcttattacaaattgggagcttcgcagcgtgtagcaggtgactcaggttttgctgcatacagtcgctacaggattggcaactataaattaaacacagaccattccagtagcagtgacaatattgctttgcttgtacagtaagtgacaacagatgtttcatctcgttgactttcaggttactatagcagagatattactaattattatgaggacttttaaagtttccatttggaatcttgattacatcataaacctcataattaaaaatttatctaagtcactaactgagaataaatattctcaattagatgaagagcaaccaatggagattgattaaacgaacatgaaaattattcttttcttggcactgataacactcgctacttgtgagctttatcactaccaagagtgtgttagaggtacaacagtacttttaaaagaaccttgctcttctggaacatacgagggcaattcaccatttcatcctctagctgataacaaatttgcactgacttgctttagcactcaatttgcttttgcttgtcctgacggcgtaaaacacgtctatcagttacgtgccagatcagtttcacctaaactgttcatcagacaagaggaagttcaagaactttactctccaatttttcttattgttgcggcaatagtgtttataacactttgcttcacactcaaaagaaagacagaatgattgaactttcattaattgacttctatttgtgctttttagcctttctgctattccttgttttaattatgcttattatcttttggttctcacttgaactgcaagatcataatgaaacttgtcacgcctaatgttttagatttcatctaaacgaacaaactaaaatgtctgataatggaccccaaaatcagcgaaatgcaccccgcattacgtttggtggaccctcagattcaactggcagtaaccagaatggagaacgcagtggggcgcgatcaaaacaacgtcggccccaaggtttacccaataatactgcgtcttggttcaccgctctcactcaacatggcaaggaagaccttaaattccctcgaggacaaggcgttccaattaacaccaatagcagtccagatgaccaaattggctactaccgaagagctaccagacgaattcgtggtggtgacggtaaaatgaaagatctcagtccaagatggtatttctactacctaggaactgggccagaagctggacttccctatggtgctaacaaagacggcatcatatgggttgcaactgagggagccttgaatacaccaaaagatcacattggcacccgcaatcctgctaacaatgctgcaatcgtgctacaacttcctcaaggaacaacattgccaaaaggcttctacgcagaagggagcagaggcggcagtcaagcctcttctcgttcctcatcacgtagtcgcaacagttcaagaaattcaactccaggcagcagtaggggaacttctcctgctagaatggctggcaatggcggtgatgctgctcttgctttgctgctgcttgacagattgaaccagcttgagagcaaaatgtctggtaaaggccaacaacaacaaggccaaactgtcactaagaaatctgctgctgaggcttctaagaagcctcggcaaaaacgtactgccactaaagcatacaatgtaacacaagctttcggcagacgtggtccagaacaaacccaaggaaattttggggaccaggaactaatcagacaaggaactgattacaaacattggccgcaaattgcacaatttgcccccagcgcttcagcgttcttcggaatgtcgcgcattggcatggaagtcacaccttcgggaacgtggttgacctacacagctgccatcaaattggatgacaaagatccaaatttcaaagatcaagtcattttgctgaataagcatattgacgcatacaaaacattcccaccaacagagcctaaaaaggacaaaaagaagaaggctgatgaaactcaagccttaccgcagagacagaagaaacagcaaactgtgactcttcttcctgctgcagatttggatgatttctccaaacaattgcaacaatccatgagcagtgctgactcaactcaggcctaaactcatgcagaccacacaaggcagatgggctatataaacgttttcgcttttccgtttacgatatatagtctactcttgtgcagaatgaattctcgtaactacatagcacaagtagatgtagttaactttaatctcacatagcaatctttaatcagtgtgtaacattagggaggacttgaaagagccaccacattttcaccgaggccacgcggagtacgatcgagtgtacagtgaacaatgctagggagagctgcctatatggaagagccctaatgtgtaaaattaattttagtagtgctatccccatgtgattttaatagcttcttaggagaatgac

SEQ ID NO: 50 - DNA, 28283 bp, Coronaviridae
  source 1..28283: mol_type = other DNA
  misc_feature 1..28283: note = SARS-CoV-2-[3,E,6,8] polynucleotide sequence, containing two point substitutions (c.27041A>C and c.27044A>C) in comparison to SEQ ID NO: 1
attaaaggtttataccttcccaggtaacaaaccaaccaactttcgatctcttgtagatctgttctctaaacgaactttaaaatctgtgtggctgtcactcggctgcatgcttagtgcactcacgcagtataattaataactaattactgtcgttgacaggacacgagtaactcgtctatcttctgcaggctgcttacggtttcgtccgtgttgcagccgatcatcagcacatctaggtttcgtccgggtgtgaccgaaaggtaagatggagagccttgtccctggtttcaacgagaaaacacacgtccaactcagtttgcctgttttacaggttcgcgacgtgctcgtacgtggctttggagactccgtggaggaggtcttatcagaggcacgtcaacatcttaaagatggcacttgtggcttagtagaagttgaaaaaggcgttttgcctcaacttgaacagccctatgtgttcatcaaacgttcggatgctcgaactgcacctcatggtcatgttatggttgagctggtagcagaactcgaaggcattcagtacggtcgtagtggtgagacacttggtgtccttgtccctcatgtgggcgaaataccagtggcttaccgcaaggttcttcttcgtaagaacggtaataaaggagctggtggccatagttacggcgccgatctaaagtcatttgacttaggcgacgagcttggcactgatccttatgaagattttcaagaaaactggaacactaaacatagcagtggtgttacccgtgaactcatgcgtgagcttaacggaggggcatacactcgctatgtcgataacaacttctgtggccctgatggctaccctcttgagtgcattaaagaccttctagcacgtgctggtaaagcttcatgcactttgtccgaacaactggactttattgacactaagaggggtgtatactgctgccgtgaacatgagcatgaaattgcttggtacacggaacgttctgaaaagagctatgaattgcagacaccttttgaaattaaattggcaaagaaatttgacaccttcaatggggaatgtccaaattttgtatttcccttaaattccataatcaagactattcaaccaagggttgaaaagaaaaagcttgatggctttatgggtagaattcgatctgtctatccagttgcgtcaccaaatgaatgcaaccaaatgtgcctttcaactctcatgaagtgtgatcattgtggtgaaacttcatggcagacgggcgattttgttaaagccacttgcgaattttgtggcactgagaatttgactaaagaaggtgccactacttgtggttacttaccccaaaatgctgttgttaaaatttattgtccagcatgtcacaattcagaagtaggacctgagcatagtcttgccgaataccataatgaatctggcttgaaaaccattcttcgtaagggtggtcgcactattgcctttggaggctgtgtgttctcttatgttggttgccataacaagtgtgcctattgggttccacgtgctagcgctaacataggttgtaaccatacaggtgttgttggagaaggttccgaaggtcttaatgacaaccttcttgaaatactccaaaaagagaaagtcaacatcaatattgttggtgactttaaacttaatgaagagatcgccattattttggcatctttttctgcttccacaagtgcttttgtggaaactgtgaaaggtttggattataaagcattcaaacaaattgttgaatcctgtggtaattttaaagttacaaaaggaaaagctaaaaaaggtgcctggaatattggtgaacagaaatcaatactgagtcctctttatgcatttgcatcagaggctgctcgtgttgtacgatcaattttctcccgcactcttgaaactgctcaaaattctgtgcgtgttttacagaaggccgctataacaatactagatggaatttcacagtattcactgagactcattgatgctatgatgttcacatctgatttggctactaacaatctagttgtaatggcctacattacaggtggtgttgttcagttgacttcgcagtggctaactaacatctttggcactgtttatgaaaaactcaaacccgtccttgattggcttgaagagaagtttaaggaaggtgtagagtttcttagagacggttgggaaattgttaaatttatctcaacctgtgcttgtgaaattgtcggtggacaaattgtcacctgtgcaaaggaaattaaggagagtgttcagacattctttaagcttgtaaataaatttttggctttgtgtgctgactctatcattattggtggagctaaacttaaagccttgaatttaggtgaaacatttgtcacgcactcaaagggattgtacagaaagtgtgttaaatccagagaagaaactggcctactcatgcctctaaaagccccaaaagaaattatcttcttagagggagaaacacttcccacagaagtgttaacagaggaagttgtcttgaaaactggtgatttacaaccattagaacaacctactagtgaagctgttgaagctccattggttggtacaccagtttgtattaacgggcttatgttgctcgaaatcaaagacacagaaaagtactgtgcccttgcacctaatatgatggtaacaaacaataccttcacactcaaaggcggtgcaccaacaaaggttacttttggtgatgacactgtgatagaagtgcaaggttacaagagtgtgaatatcacttttgaacttgatgaaaggattgataaagtacttaatgagaagtgctctgcctatacagttgaactcggtacagaagtaaatgagttcgcctgtgttgtggcagatgctgtcataaaaactttgcaaccagtatctgaattacttacaccactgggcattgatttagatgagtggagtatggctacatactacttatttgatgagtctggtgagtttaaattggcttcacatatgtattgttctttctaccctccagatgaggatgaagaagaaggtgattgtgaagaagaagagtttgagccatcaactcaatatgagtatggtactgaagatgattaccaaggtaaacctttggaatttggtgccacttctgctgctcttcaacctgaagaagagcaagaagaagattggttagatgatgatagtcaacaaactgttggtcaacaagacggcagtgaggacaatcagacaactactattcaaacaattgttgaggttcaacctcaattagagatggaacttacaccagttgttcagactattgaagtgaatagttttagtggttatttaaaacttactgacaatgtatacattaaaaatgcagacattgtggaagaagctaaaaaggtaaaaccaacagtggttgttaatgcagccaatgtttaccttaaacatggaggaggtgttgcaggagccttaaataaggctactaacaatgccatgcaagttgaatctgatgattacatagctactaatggaccacttaaagtgggtggtagttgtgttttaagcggacacaatcttgctaaacactgtcttcatgttgtcggcccaaatgttaacaaaggtgaagacattcaacttcttaagagtgcttatgaaaattttaatcagcacgaagttctacttgcaccattattatcagctggtatttttggtgctgaccctatacattctttaagagtttgtgtagatactgttcgcacaaatgtctacttagctgtctttgataaaaatctctatgacaaacttgtttcaagctttttggaaatgaagagtgaaaagcaagttgaacaaaagatcgctgagattcctaaagaggaagttaagccatttataactgaaagtaaaccttcagttgaacagagaaaacaagatgataagaaaatcaaagcttgtgttgaagaagttacaacaactctggaagaaactaagttcctcacagaaaacttgttactttatattgacattaatggcaatcttcatccagattctgccactcttgttagtgacattgacatcactttcttaaagaaagatgctccatatatagtgggtgatgttgttcaagagggtgttttaactgctgtggttatacctactaaaaaggctggtggcactactgaaatgctagcgaaagctttgagaaaagtgccaacagacaattatataaccacttacccgggtcagggtttaaatggttacactgtagaggaggcaaagacagtgcttaaaaagtgtaaaagtgccttttacattctaccatctattatctctaatgagaagcaagaaattcttggaactgtttcttggaatttgcgagaaatgcttgcacatgcagaagaaacacgcaaattaatgcctgtctgtgtggaaactaaagccatagtttcaactatacagcgtaaatataagggtattaaaatacaagagggtgtggttgattatggtgctagattttacttttacaccagtaaaacaactgtagcgtcacttatcaacacacttaacgatctaaatgaaactcttgttacaatgccacttggctatgtaacacatggcttaaatttggaagaagctgctcggtatatgagatctctcaaagtgccagctacagtttctgtttcttcacctgatgctgttacagcgtataatggttatcttacttcttcttctaaaacacctgaagaacattttattgaaaccatctcacttgctggttcctataaagattggtcctattctggacaatctacacaactaggtatagaatttcttaagagaggtgataaaagtgtatattacactagtaatcctaccacattccacctagatggtgaagttatcacctttgacaatcttaagacacttctttctttgagagaagtgaggactattaaggtgtttacaacagtagacaacattaacctccacacgcaagttgtggacatgtcaatgacatatggacaacagtttggtccaacttatttggatggagctgatgttactaaaataaaacctcataattcacatgaaggtaaaacattttatgttttacctaatgatgacactctacgtgttgaggcttttgagtactaccacacaactgatcctagttttctgggtaggtacatgtcagcattaaatcacactaaaaagtggaaatacccacaagttaatggtttaacttctattaaatgggcagataacaactgttatcttgccactgcattgttaacactccaacaaatagagttgaagtttaatccacctgctctacaagatgcttattacagagcaagggctggtgaagctgctaacttttgtgcacttatcttagcctactgtaataagacagtaggtgagttaggtgatgttagagaaacaatgagttacttgtttcaacatgccaatttagattcttgcaaaagagtcttgaacgtggtgtgtaaaacttgtggacaacagcagacaacccttaagggtgtagaagctgttatgtacatgggcacactttcttatgaacaatttaagaaaggtgttcagataccttgtacgtgtggtaaacaagctacaaaatatctagtacaacaggagtcaccttttgttatgatgtcagcaccacctgctcagtatgaacttaagcatggtacatttacttgtgctagtgagtacactggtaattaccagtgtggtcactataaacatataacttctaaagaaactttgtattgcatagacggtgctttacttacaaagtcctcagaatacaaaggtcctattacggatgttttctacaaagaaaacagttacacaacaaccataaaaccagttacttataaattggatggtgttgtttgtacagaaattgaccctaagttggacaattattataagaaagacaattcttatttcacagagcaaccaattgatcttgtaccaaaccaaccatatccaaacgcaagcttcgataattttaagtttgtatgtgataatatcaaatttgctgatgatttaaaccagttaactggttataagaaacctgcttcaagagagcttaaagttacatttttccctgacttaaatggtgatgtggtggctattgattataaacactacacaccctcttttaagaaaggagctaaattgttacataaacctattgtttggcatgttaacaatgcaactaataaagccacgtataaaccaaatacctggtgtatacgttgtctttggagcacaaaaccagttgaaacatcaaattcgtttgatgtactgaagtcagaggacgcgcagggaatggataatcttgcctgcgaagatctaaaaccagtctctgaagaagtagtggaaaatcctaccatacagaaagacgttcttgagtgtaatgtgaaaactaccgaagttgtaggagacattatacttaaaccagcaaataatagtttaaaaattacagaagaggttggccacacagatctaatggctgcttatgtagacaattctagtcttactattaagaaacctaatgaattatctagagtattaggtttgaaaacccttgctactcatggtttagctgctgttaatagtgtcccttgggatactatagctaattatgctaagccttttcttaacaaagttgttagtacaactactaacatagttacacggtgtttaaaccgtgtttgtactaattatatgccttatttctttactttattgctacaattgtgtacttttactagaagtacaaattctagaattaaagcatctatgccgactactatagcaaagaatactgttaagagtgtcggtaaattttgtctagaggcttcatttaattatttgaagtcacctaatttttctaaactgataaatattataatttggtttttactattaagtgtttgcctaggttctttaatctactcaaccgctgctttaggtgttttaatgtctaatttaggcatgccttcttactgtactggttacagagaaggctatttgaactctactaatgtcactattgcaacctactgtactggttctataccttgtagtgtttgtcttagtggtttagattctttagacacctatccttctttagaaactatacaaattaccatttcatcttttaaatgggatttaactgcttttggcttagttgcagagtggtttttggcatatattcttttcactaggtttttctatgtacttggattggctgcaatcatgcaattgtttttcagctattttgcagtacattttattagtaattcttggcttatgtggttaataattaatcttgtacaaatggccccgatttcagctatggttagaatgtacatcttctttgcatcattttattatgtatggaaaagttatgtgcatgttgtagacggttgtaattcatcaacttgtatgatgtgttacaaacgtaatagagcaacaagagtcgaatgtacaactattgttaatggtgttagaaggtccttttatgtctatgctaatggaggtaaaggcttttgcaaactacacaattggaattgtgttaattgtgatacattctgtgctggtagtacatttattagtgatgaagttgcgagagacttgtcactacagtttaaaagaccaataaatcctactgaccagtcttcttacatcgttgatagtgttacagtgaagaatggttccatccatctttactttgataaagctggtcaaaagacttatgaaagacattctctctctcattttgttaacttagacaacctgagagctaataacactaaaggttcattgcctattaatgttatagtttttgatggtaaatcaaaatgtgaagaatcatctgcaaaatcagcgtctgtttactacagtcagcttatgtgtcaacctatactgttactagatcaggcattagtgtctgatgttggtgatagtgcggaagttgcagttaaaatgtttgatgcttacgttaatacgttttcatcaacttttaacgtaccaatggaaaaactcaaaacactagttgcaactgcagaagctgaacttgcaaagaatgtgtccttagacaatgtcttatctacttttatttcagcagctcggcaagggtttgttgattcagatgtagaaactaaagatgttgttgaatgtcttaaattgtcacatcaatctgacatagaagttactggcgatagttgtaataactatatgctcacctataacaaagttgaaaacatgacaccccgtgaccttggtgcttgtattgactgtagtgcgcgtcatattaatgcgcaggtagcaaaaagtcacaacattgctttgatatggaacgttaaagatttcatgtcattgtctgaacaactacgaaaacaaatacgtagtgctgctaaaaagaataacttaccttttaagttgacatgtgcaactactagacaagttgttaatgttgtaacaacaaagatagcacttaagggtggtaaaattgttaataattggttgaagcagttaattaaagttacacttgtgttcctttttgttgctgctattttctatttaataacacctgttcatgtcatgtctaaacatactgacttttcaagtgaaatcataggatacaaggctattgatggtggtgtcactcgtgacatagcatctacagatacttgttttgctaacaaacatgctgattttgacacatggtttagccagcgtggtggtagttatactaatgacaaagcttgcccattgattgctgcagtcataacaagagaagtgggttttgtcgtgcctggtttgcctggcacgatattacgcacaactaatggtgactttttgcatttcttacctagagtttttagtgcagttggtaacatctgttacacaccatcaaaacttatagagtacactgactttgcaacatcagcttgtgttttggctgctgaatgtacaatttttaaagatgcttctggtaagccagtaccatattgttatgataccaatgtactagaaggttctgttgcttatgaaagtttacgccctgacacacgttatgtgctcatggatggctctattattcaatttcctaacacctaccttgaaggttctgttagagtggtaacaacttttgattctgagtactgtaggcacggcacttgtgaaagatcagaagctggtgtttgtgtatctactagtggtagatgggtacttaacaatgattattacagatctttaccaggagttttctgtggtgtagatgctgtaaatttacttactaatatgtttacaccactaattcaacctattggtgctttggacatatcagcatctatagtagctggtggtattgtagctatcgtagtaacatgccttgcctactattttatgaggtttagaagagcttttggtgaatacagtcatgtagttgcctttaatactttactattccttatgtcattcactgtactctgtttaacaccagtttactcattcttacctggtgtttattctgttatttacttgtacttgacattttatcttactaatgatgtttcttttttagcacatattcagtggatggttatgttcacacctttagtacctttctggataacaattgcttatatcatttgtatttccacaaagcatttctattggttctttagtaattacctaaagagacgtgtagtctttaatggtgtttcctttagtacttttgaagaagctgcgctgtgcacctttttgttaaataaagaaatgtatctaaagttgcgtagtgatgtgctattacctcttacgcaatataatagatacttagctctttataataagtacaagtattttagtggagcaatggatacaactagctacagagaagctgcttgttgtcatctcgcaaaggctctcaatgacttcagtaactcaggttctgatgttctttaccaaccaccacaaacctctatcacctcagctgttttgcagagtggttttagaaaaatggcattcccatctggtaaagttgagggttgtatggtacaagtaacttgtggtacaactacacttaacggtctttggcttgatgacgtagtttactgtccaagacatgtgatctgcacctctgaagacatgcttaaccctaattatgaagatttactcattcgtaagtctaatcataatttcttggtacaggctggtaatgttcaactcagggttattggacattctatgcaaaattgtgtacttaagcttaaggttgatacagccaatcctaagacacctaagtataagtttgttcgcattcaaccaggacagactttttcagtgttagcttgttacaatggttcaccatctggtgtttaccaatgtgctatgaggcccaatttcactattaagggttcattccttaatggttcatgtggtagtgttggttttaacatagattatgactgtgtctctttttgttacatgcaccatatggaattaccaactggagttcatgctggcacagacttagaaggtaacttttatggaccttttgttgacaggcaaacagcacaagcagctggtacggacacaactattacagttaatgttttagcttggttgtacgctgctgttataaatggagacaggtggtttctcaatcgatttaccacaactcttaatgactttaaccttgtggctatgaagtacaattatgaacctctaacacaagaccatgttgacatactaggacctctttctgctcaaactggaattgccgttttagatatgtgtgcttcattaaaagaattactgcaaaatggtatgaatggacgtaccatattgggtagtgctttattagaagatgaatttacaccttttgatgttgttagacaatgctcaggtgttactttccaaagtgcagtgaaaagaacaatcaagggtacacaccactggttgttactcacaattttgacttcacttttagttttagtccagagtactcaatggtctttgttcttttttttgtatgaaaatgcctttttaccttttgctatgggtattattgctatgtctgcttttgcaatgatgtttgtcaaacataagcatgcatttctctgtttgtttttgttaccttctcttgccactgtagcttattttaatatggtctatatgcctgctagttgggtgatgcgtattatgacatggttggatatggttgatactagtttgtctggttttaagctaaaagactgtgttatgtatgcatcagctgtagtgttactaatccttatgacagcaagaactgtgtatgatgatggtgctaggagagtgtggacacttatgaatgtcttgacactcgtttataaagtttattatggtaatgctttagatcaagccatttccatgtgggctcttataatctctgttacttctaactactcaggtgtagttacaactgtcatgtttttggccagaggtattgtttttatgtgtgttgagtattgccctattttcttcataactggtaatacacttcagtgtataatgctagtttattgtttcttaggctatttttgtacttgttactttggcctcttttgtttactcaaccgctactttagactgactcttggtgtttatgattacttagtttctacacaggagtttagatatatgaattcacagggactactcccacccaagaatagcatagatgccttcaaactcaacattaaattgttgggtgttggtggcaaaccttgtatcaaagtagccactgtacagtctaaaatgtcagatgtaaagtgcacatcagtagtcttactctcagttttgcaacaactcagagtagaatcatcatctaaattgtgggctcaatgtgtccagttacacaatgacattctcttagctaaagatactactgaagcctttgaaaaaatggtttcactactttctgttttgctttccatgcagggtgctgtagacataaacaagctttgtgaagaaatgctggacaacagggcaaccttacaagctatagcctcagagtttagttcccttccatcatatgcagcttttgctactgctcaagaagcttatgagcaggctgttgctaatggtgattctgaagttgttcttaaaaagttgaagaagtctttgaatgtggctaaatctgaatttgaccgtgatgcagccatgcaacgtaagttggaaaagatggctgatcaagctatgacccaaatgtataaacaggctagatctgaggacaagagggcaaaagttactagtgctatgcagacaatgcttttcactatgcttagaaagttggataatgatgcactcaacaacattatcaacaatgcaagagatggttgtgttcccttgaacataatacctcttacaacagcagccaaactaatggttgtcataccagactataacacatataaaaatacgtgtgatggtacaacatttacttatgcatcagcattgtgggaaatccaacaggttgtagatgcagatagtaaaattgttcaacttagtgaaattagtatggacaattcacctaatttagcatggcctcttattgtaacagctttaagggccaattctgctgtcaaattacagaataatgagcttagtcctgttgcactacgacagatgtcttgtgctgccggtactacacaaactgcttgcactgatgacaatgcgttagcttactacaacacaacaaagggaggtaggtttgtacttgcactgttatccgatttacaggatttgaaatgggctagattccctaagagtgatggaactggtactatctatacagaactggaaccaccttgtaggtttgttacagacacacctaaaggtcctaaagtgaagtatttatactttattaaaggattaaacaacctaaatagaggtatggtacttggtagtttagctgccacagtacgtctacaagctggtaatgcaacagaagtgcctgccaattcaactgtattatctttctgtgcttttgctgtagatgctgctaaagcttacaaagattatctagctagtgggggacaaccaatcactaattgtgttaagatgttgtgtacacacactggtactggtcaggcaataacagttacaccggaagccaatatggatcaagaatcctttggtggtgcatcgtgttgtctgtactgccgttgccacatagatcatccaaatcctaaaggattttgtgacttaaaaggtaagtatgtacaaatacctacaacttgtgctaatgaccctgtgggttttacacttaaaaacacagtctgtaccgtctgcggtatgtggaaaggttatggctgtagttgtgatcaactccgcgaacccatgcttcagtcagctgatgcacaatcgtttttaaacgggtttgcggtgtaagtgcagcccgtcttacaccgtgcggcacaggcactagtactgatgtcgtatacagggcttttgacatctacaatgataaagtagctggttttgctaaattcctaaaaactaattgttgtcgcttccaagaaaaggacgaagatgacaatttaattgattcttactttgtagttaagagacacactttctctaactaccaacatgaagaaacaatttataatttacttaaggattgtccagctgttgctaaacatgacttctttaagtttagaatagacggtgacatggtaccacatatatcacgtcaacgtcttactaaatacacaatggcagacctcgtctatgctttaaggcattttgatgaaggtaattgtgacacattaaaagaaatacttgtcacatacaattgttgtgatgatgattatttcaataaaaaggactggtatgattttgtagaaaacccagatatattacgcgtatacgccaacttaggtgaacgtgtacgccaagctttgttaaaaacagtacaattctgtgatgccatgcgaaatgctggtattgttggtgtactgacattagataatcaagatctcaatggtaactggtatgatttcggtgatttcatacaaaccacgccaggtagtggagttcctgttgtagattcttattattcattgttaatgcctatattaaccttgaccagggctttaactgcagagtcacatgttgacactgacttaacaaagccttacattaagtgggatttgttaaaatatgacttcacggaagagaggttaaaactctttgaccgttattttaaatattgggatcagacataccacccaaattgtgttaactgtttggatgacagatgcattctgcattgtgcaaactttaatgttttattctctacagtgttcccacctacaagttttggaccactagtgagaaaaatatttgttgatggtgttccatttgtagtttcaactggataccacttcagagagctaggtgttgtacataatcaggatgtaaacttacatagctctagacttagttttaaggaattacttgtgtatgctgctgaccctgctatgcacgctgcttctggtaatctattactagataaacgcactacgtgcttttcagtagctgcacttactaacaatgttgcttttcaaactgtcaaacccggtaattttaacaaagacttctatgactttgctgtgtctaagggtttctttaaggaaggaagttctgttgaattaaaacacttcttctttgctcaggatggtaatgctgctatcagcgattatgactactatcgttataatctaccaacaatgtgtgatatcagacaactactatttgtagttgaagttgttgataagtactttgattgttacgatggtggctgtattaatgctaaccaagtcatcgtcaacaacctagacaaatcagctggttttccatttaataaatggggtaaggctagactttattatgattcaatgagttatgaggatcaagatgcacttttcgcatatacaaaacgtaatgtcatccctactataactcaaatgaatcttaagtatgccattagtgcaaagaatagagctcgcaccgtagctggtgtctctatctgtagtactatgaccaatagacagtttcatcaaaaattattgaaatcaatagccgccactagaggagctactgtagtaattggaacaagcaaattctatggtggttggcacaacatgttaaaaactgtttatagtgatgtagaaaaccctcaccttatgggttgggattatcctaaatgtgatagagccatgcctaacatgcttagaattatggcctcacttgttcttgctcgcaaacatacaacgtgttgtagcttgtcacaccgtttctatagattagctaatgagtgtgctcaagtattgagtgaaatggtcatgtgtggcggttcactatatgttaaaccaggtggaacctcatcaggagatgccacaactgcttatgctaatagtgtttttaacatttgtcaagctgtcacggccaatgttaatgcacttttatctactgatggtaacaaaattgccgataagtatgtccgcaatttacaacacagactttatgagtgtctctatagaaatagagatgttgacacagactttgtgaatgagttttacgcatatttgcgtaaacatttctcaatgatgatactctctgacgatgctgttgtgtgtttcaatagcacttatgcatctcaaggtctagtggctagcataaagaactttaagtcagttctttattatcaaaacaatgtttttatgtctgaagcaaaatgttggactgagactgaccttactaaaggacctcatgaattttgctctcaacatacaatgctagttaaacagggtgatgattatgtgtaccttccttacccagatccatcaagaatcctaggggccggctgttttgtagatgatatcgtaaaaacagatggtacacttatgattgaacggttcgtgtctttagctatagatgcttacccacttactaaacatcctaatcaggagtatgctgatgtctttcatttgtacttacaatacataagaaagctacatgatgagttaacaggacacatgttagacatgtattctgttatgcttactaatgataacacttcaaggtattgggaacctgagttttatgaggctatgtacacaccgcatacagtcttacaggctgttggggcttgtgttctttgcaattcacagacttcattaagatgtggtgcttgcatacgtagaccattcttatgttgtaaatgctgttacgaccatgtcatatcaacatcacataaattagtcttgtctgttaatccgtatgtttgcaatgctccaggttgtgatgtcacagatgtgactcaactttacttaggaggtatgagctattattgtaaatcacataaaccacccattagttttccattgtgtgctaatggacaagtttttggtttatataaaaatacatgtgttggtagcgataatgttactgactttaatgcaattgcaacatgtgactggacaaatgctggtgattacattttagctaacacctgtactgaaagactcaagctttttgcagcagaaacgctcaaagctactgaggagacatttaaactgtcttatggtattgctactgtacgtgaagtgctgtctgacagagaattacatctttcatgggaagttggtaaacctagaccaccacttaaccgaaattatgtctttactggttatcgtgtaactaaaaacagtaaagtacaaataggagagtacacctttgaaaaaggtgactatggtgatgctgttgtttaccgaggtacaacaacttacaaattaaatgttggtgattattttgtgctgacatcacatacagtaatgccattaagtgcacctacactagtgccacaagagcactatgttagaattactggcttatacccaacactcaatatctcagatgagttttctagcaatgttgcaaattatcaaaaggttggtatgcaaaagtattctacactccagggaccacctggtactggtaagagtcattttgctattggcctagctctctactacccttctgctcgcatagtgtatacagcttgctctcatgccgctgttgatgcactatgtgagaaggcattaaaatatttgcctatagataaatgtagtagaattatacctgcacgtgctcgtgtagagtgttttgataaattcaaagtgaattcaacattagaacagtatgtcttttgtactgtaaatgcattgcctgagacgacagcagatatagttgtctttgatgaaatttcaatggccacaaattatgatttgagtgttgtcaatgccagattacgtgctaagcactatgtgtacattggcgaccctgctcaattacctgcaccacgcacattgctaactaagggcacactagaaccagaatatttcaattcagtgtgtagacttatgaaaactataggtccagacatgttcctcggaacttgtcggcgttgtcctgctgaaattgttgacactgtgagtgctttggtttatgataataagcttaaagcacataaagacaaatcagctcaatgctttaaaatgttttataagggtgttatcacgcatgatgtttcatctgcaattaacaggccacaaataggcgtggtaagagaattccttacacgtaaccctgcttggagaaaagctgtctttatttcaccttataattcacagaatgctgtagcctcaaagattttgggactaccaactcaaactgttgattcatcacagggctcagaatatgactatgtcatattcactcaaaccactgaaacagctcactcttgtaatgtaaacagatttaatgttgctattaccagagcaaaagtaggcatactttgcataatgtctgatagagacctttatgacaagttgcaatttacaagtcttgaaattccacgtaggaatgtggcaactttacaagctgaaaatgtaacaggactctttaaagattgtagtaaggtaatcactgggttacatcctacacaggcacctacacacctcagtgttgacactaaattcaaaactgaaggtttatgtgttgacatacctggcatacctaaggacatgacctatagaagactcatctctatgatgggttttaaaatgaattatcaagttaatggttaccctaacatgtttatcacccgcgaagaagctataagacatgtacgtgcatggattggcttcgatgtcgaggggtgtcatgctactagagaagctgttggtaccaatttacctttacagctaggtttttctacaggtgttaacctagttgctgtacctacaggttatgttgatacacctaataatacagatttttccagagttagtgctaaaccaccgcctggagatcaatttaaacacctcataccacttatgtacaaaggacttccttggaatgtagtgcgtataaagattgtacaaatgttaagtgacacacttaaaaatctctctgacagagtcgtatttgtcttatgggcacatggctttgagttgacatctatgaagtattttgtgaaaataggacctgagcgcacctgttgtctatgtgatagacgtgccacatgcttttccactgcttcagacacttatgcctgttggcatcattctattggatttgattacgtctataatccgtttatgattgatgttcaacaatggggttttacaggtaacctacaaagcaaccatgatctgtattgtcaagtccatggtaatgcacatgtagctagttgtgatgcaatcatgactaggtgtctagctgtccacgagtgctttgttaagcgtgttgactggactattgaatatcctataattggtgatgaactgaagattaatgcggcttgtagaaaggttcaacacatggttgttaaagctgcattattagcagacaaattcccagttcttcacgacattggtaaccctaaagctattaagtgtgtacctcaagctgatgtagaatggaagttctatgatgcacagccttgtagtgacaaagcttataaaatagaagaattattctattcttatgccacacattctgacaaattcacagatggtgtatgcctattttggaattgcaatgtcgatagatatcctgctaattccattgtttgtagatttgacactagagtgctatctaaccttaacttgcctggttgtgatggtggcagtttgtatgtaaataaacatgcattccacacaccagcttttgataaaagtgcttttgttaatttaaaacaattaccatttttctattactctgacagtccatgtgagtctcatggaaaacaagtagtgtcagatatagattatgtaccactaaagtctgctacgtgtataacacgttgcaatttaggtggtgctgtctgtagacatcatgctaatgagtacagattgtatctcgatgcttataacatgatgatctcagctggctttagcttgtgggtttacaaacaatttgatacttataacctctggaacacttttacaagacttcagagtttagaaaatgtggcttttaatgttgtaaataagggacactttgatggacaacagggtgaagtaccagtttctatcattaataacactgtttacacaaaagttgatggtgttgatgtagaattgtttgaaaataaaacaacattacctgttaatgtagcatttgagctttgggctaagcgcaacattaaaccagtaccagaggtgaaaatactcaataatttgggtgtggacattgctgctaatactgtgatctgggactacaaaagagatgctccagcacatatatctactattggtgtttgttctatgactgacatagccaagaaaccaactgaaacgatttgtgcaccactcactgtcttttttgatggtagagttgatggtcaagtagacttatttagaaatgcccgtaatggtgttcttattacagaaggtagtgttaaaggtttacaaccatctgtgggtcccaaacaagctagtcttaatggagtcacattaattggagaagccgtaaaaacacagttcaattattataagaaagttgatggtgttgtccaacaattacctgaaacttactttactcagagtagaaatttacaagaatttaaacccaggagtcaaatggaaattgatttcttagaattagctatggatgaattcattgaacggtataaattagaaggctatgccttcgaacatatcgtttatggagattttagtcatagtcagttaggtggtttacatctactgattggactagctaaacgttttaaggaatcaccttttgaattagaagattttattcctatggacagtacagttaaaaactatttcataacagatgcgcaaacaggttcatctaagtgtgtgtgttctgttattgatttattacttgatgattttgttgaaataataaaatcccaagatttatctgtagtttctaaggttgtcaaagtgactattgactatacagaaatttcatttatgctttggtgtaaagatggccatgtagaaacattttacccaaaattacaatctagtcaagcgtggcaaccgggtgttgctatgcctaatctttacaaaatgcaaagaatgctattagaaaagtgtgaccttcaaaattatggtgatagtgcaacattacctaaaggcataatgatgaatgtcgcaaaatatactcaactgtgtcaatatttaaacacattaacattagctgtaccctataatatgagagttatacattttggtgctggttctgataaaggagttgcaccaggtacagctgttttaagacagtggttgcctacgggtacgctgcttgtcgattcagatcttaatgactttgtctctgatgcagattcaactttgattggtgattgtgcaactgtacatacagctaataaatgggatctcattattagtgatatgtacgaccctaagactaaaaatgttacaaaagaaaatgactctaaagagggttttttcacttacatttgtgggtttatacaacaaaagctagctcttggaggttccgtggctataaagataacagaacattcttggaatgctgatctttataagctcatgggacacttcgcatggtggacagcctttgttactaatgtgaatgcgtcatcatctgaagcatttttaattggatgtaattatcttggcaaaccacgcgaacaaatagatggttatgtcatgcatgcaaattacatattttggaggaatacaaatccaattcagttgtcttcctattctttatttgacatgagtaaatttccccttaaattaaggggtactgctgttatgtctttaaaagaaggtcaaatcaatgatatgattttatctcttcttagtaaaggtagacttataattagagaaaacaacagagttgttatttctagtgatgttcttgttaacaactaaacgaacaatgtttgtttttcttgttttattgccactagtctctagtcagtgtgttaatcttacaaccagaactcaattaccccctgcatacactaattctttcacacgtggtgtttattaccctgacaaagttttcagatcctcagttttacattcaactcaggacttgttcttacctttcttttccaatgttacttggttccatgctatacatgtctctgggaccaatggtactaagaggtttgataaccctgtcctaccatttaatgatggtgtttattttgcttccactgagaagtctaacataataagaggctggatttttggtactactttagattcgaagacccagtccctacttattgttaataacgctactaatgttgttattaaagtctgtgaatttcaattttgtaatgatccatttttgggtgtttattaccacaaaaacaacaaaagttggatggaaagtgagttcagagtttattctagtgcgaataattgcacttttgaatatgtctctcagccttttcttatggaccttgaaggaaaacagggtaatttcaaaaatcttagggaatttgtgtttaagaatattgatggttattttaaaatatattctaagcacacgcctattaatttagtgcgtgatctccctcagggtttttcggctttagaaccattggtagatttgccaataggtattaacatcactaggtttcaaactttacttgctttacatagaagttatttgactcctggtgattcttcttcaggttggacagctggtgctgcagcttattatgtgggttatcttcaacctaggacttttctattaaaatataatgaaaatggaaccattacagatgctgtagactgtgcacttgaccctctctcagaaacaaagtgtacgttgaaatccttcactgtagaaaaaggaatctatcaaacttctaactttagagtccaaccaacagaatctattgttagatttcctaatattacaaacttgtgcccttttggtgaagtttttaacgccaccagatttgcatctgtttatgcttggaacaggaagagaatcagcaactgtgttgctgattattctgtcctatataattccgcatcattttccacttttaagtgttatggagtgtctcctactaaattaaatgatctctgctttactaatgtctatgcagattcatttgtaattagaggtgatgaagtcagacaaatcgctccagggcaaactggaaagattgctgattataattataaattaccagatgattttacaggctgcgttatagcttggaattctaacaatcttgattctaaggttggtggtaattataattacctgtatagattgtttaggaagtctaatctcaaaccttttgagagagatatttcaactgaaatctatcaggccggtagcacaccttgtaatggtgttgaaggttttaattgttactttcctttacaatcatatggtttccaacccactaatggtgttggttaccaaccatacagagtagtagtactttcttttgaacttctacatgcaccagcaactgtttgtggacctaaaaagtctactaatttggttaaaaacaaatgtgtcaatttcaacttcaatggtttaacaggcacaggtgttcttactgagtctaacaaaaagtttctgcctttccaacaatttggcagagacattgctgacactactgatgctgtccgtgatccacagacacttgagattcttgacattacaccatgttcttttggtggtgtcagtgttataacaccaggaacaaatacttctaaccaggttgctgttctttatcaggatgttaactgcacagaagtccctgttgctattcatgcagatcaacttactcctacttggcgtgtttattctacaggttctaatgtttttcaaacacgtgcaggctgtttaataggggctgaacatgtcaacaactcatatgagtgtgacatacccattggtgcaggtatatgcgctagttatcagactcagactaattctcctcggcgggcacgtagtgtagctagtcaatccatcattgcctacactatgtcacttggtgcagaaaattcagttgcttactctaataactctattgccatacccacaaattttactattagtgttaccacagaaattctaccagtgtctatgaccaagacatcagtagattgtacaatgtacatttgtggtgattcaactgaatgcagcaatcttttgttgcaatatggcagtttttgtacacaattaaaccgtgctttaactggaatagctgttgaacaagacaaaaacacccaagaagtttttgcacaagtcaaacaaatttacaaaacaccaccaattaaagattttggtggttttaatttttcacaaatattaccagatccatcaaaaccaagcaagaggtcatttattgaagatctacttttcaacaaagtgacacttgcagatgctggcttcatcaaacaatatggtgattgccttggtgatattgctgctagagacctcatttgtgcacaaaagtttaacggccttactgttttgccacctttgctcacagatgaaatgattgctcaatacacttctgcactgttagcgggtacaatcacttctggttggacctttggtgcaggtgctgcattacaaataccatttgctatgcaaatggcttataggtttaatggtattggagttacacagaatgttctctatgagaaccaaaaattgattgccaaccaatttaatagtgctattggcaaaattcaagactcactttcttccacagcaagtgcacttggaaaacttcaagatgtggtcaaccaaaatgcacaagctttaaacacgcttgttaaacaacttagctccaattttggtgcaatttcaagtgttttaaatgatatcctttcacgtcttgacaaagttgaggctgaagtgcaaattgataggttgatcacaggcagacttcaaagtttgcagacatatgtgactcaacaattaattagagctgcagaaatcagagcttctgctaatcttgctgctactaaaatgtcagagtgtgtacttggacaatcaaaaagagttgatttttgtggaaagggctatcatcttatgtccttccctcagtcagcacctcatggtgtagtcttcttgcatgtgacttatgtccctgcacaagaaaagaacttcacaactgctcctgccatttgtcatgatggaaaagcacactttcctcgtgaaggtgtctttgtttcaaatggcacacactggtttgtaacacaaaggaatttttatgaaccacaaatcattactacagacaacacatttgtgtctggtaactgtgatgttgtaataggaattgtcaacaacacagtttatgatcctttgcaacctgaattagactcattcaaggaggagttagataaatattttaagaatcatacatcaccagatgttgatttaggtgacatctctggcattaatgcttcagttgtaaacattcaaaaagaaattgaccgcctcaatgaggttgccaagaatttaaatgaatctctcatcgatctccaagaacttggaaagtatgagcagtatataaaatggccatggtacatttggctaggttttatagctggcttgattgccatagtaatggtgacaattatgctttgctgtatgaccagttgctgtagttgtctcaagggctgttgttcttgtggatcctgctgcaaatttgatgaagacgactctgagccagtgctcaaaggagtcaaattacattacacataattcctgatcttctggtctaaacgaactaaatattatattagtttttctgtttggaactttaattttagccatggcagattccaacggtactattaccgttgaagagcttaaaaagctccttgaacaatggaacctagtaataggtttcctattccttacatggatttgtcttctacaatttgcctatgccaacaggaataggtttttgtatataattaagttaattttcctctggctgttatggccagtaactttagcttgttttgtgcttgctgctgtttacagaataaattggatcaccggtggaattgctatcgcaatggcttgtcttgtaggcttgatgtggctcagctacttcattgcttctttcagactgtttgcgcgtacccgttccatgtggtcattcaatccagaaactaacattcttctcaacgtgccactccatggcactattctgaccagaccgcttctagaaagtgaactcgtaatcggagctgtgatccttcgtggacatcttcgtattgctggacaccatctaggacgctgtgacatcaaggacctgcctaaagaaatcactgttgctacatcccgcacgctttcttattacaaattgggagcttcgcagcgtgtagcaggtgactcaggttttgctgcatacagtcgctacaggattggcaactataaattaaacacagaccattccagtagcagtgacaatattgctttgcttgtacagtaagtgacaacagaaccaatggagattgattaaacgaacatgaaaattattcttttcttggcactgataacactcgctacttgtgagctttatcactaccaagagtgtgttagaggtacaacagtacttttaaaagaaccttgctcttctggaacatacgagggcaattcaccatttcatcctctagctgataacaaatttgcactgacttgctttagcactcaatttgcttttgcttgtcctgacggcgtaaaacacgtctatcagttacgtgccagatcagtttcacctaaactgttcatcagacaagaggaagttcaagaactttactctccaatttttcttattgttgcggcaatagtgtttataacactttgcttcacactcaaaagaaagacagaatgattgaactttcattaattgacttctatttgtgctttttagcctttctgctattccttgttttaattatgcttattatcttttggttctcacttgaactgcaagatcataatgaaacttgtcacgcctaatgttttagatttcatctaaacgaacaaactaaaatgtctgataatggaccccaaaatcagcgaaatgcaccccgcattacgtttggtggaccctcagattcaactggcagtaaccagaatggagaacgcagtggggcgcgatcaaaacaacgtcggccccaaggtttacccaataatactgcgtcttggttcaccgctctcactcaacatggcaaggaagaccttaaattccctcgaggacaaggcgttccaattaacaccaatagcagtccagatgaccaaattggctactaccgaagagctaccagacgaattcgtggtggtgacggtaaaatgaaagatctcagtccaagatggtatttctactacctaggaactgggccagaagctggacttccctatggtgctaacaaagacggcatcatatgggttgcaactgagggagccttgaatacaccaaaagatcacattggcacccgcaatcctgctaacaatgctgcaatcgtgctacaacttcctcaaggaacaacattgccaaaaggcttctacgcagaagggagcagaggcggcagtcaagcctcttctcgttcctcatcacgtagtcgcaacagttcaagaaattcaactccaggcagcagtaggggaacttctcctgctagaatggctggcaatggcggtgatgctgctcttgctttgctgctgcttgacagattgaaccagcttgagagcaaaatgtctggtaaaggccaacaacaacaaggccaaactgtcactaagaaatctgctgctgaggcttctaagaagcctcggcaaaaacgtactgccactaaagcatacaatgtaacacaagctttcggcagacgtggtccagaacaaacccaaggaaattttggggaccaggaactaatcagacaaggaactgattacaaacattggccgcaaattgcacaatttgcccccagcgcttcagcgttcttcggaatgtcgcgcattggcatggaagtcacaccttcgggaacgtggttgacctacacagctgccatcaaattggatgacaaagatccaaatttcaaagatcaagtcattttgctgaataagcatattgacgcatacaaaacattcccaccaacagagcctaaaaaggacaaaaagaagaaggctgatgaaactcaagccttaccgcagagacagaagaaacagcaaactgtgactcttcttcctgctgcagatttggatgatttctccaaacaattgcaacaatccatgagcagtgctgactcaactcaggcctaaactcatgcagaccacacaaggcagatgggctatataaacgttttcgcttttccgtttacgatatatagtctactcttgtgcagaatgaattctcgtaactacatagcacaagtagatgtagttaactttaatctcacatagcaatctttaatcagtgtgtaacattagggaggacttgaaagagccaccacattttcaccgaggccacgcggagtacgatcgagtgtacagtgaacaatgctagggagagctgcctatatggaagagccctaatgtgtaaaattaattttagtagtgctatccccatgtgattttaatagcttcttaggagaatgac